European Patent Application EP 4 640 057 A1, published October 29, 2025. Title: ISOLATED BACTERIOPHAGE AGAINST XYLELLA FASTIDIOSA. Applicant: BIOLINE AGROSCIENCES FRANCE. The sequence listing filed with the application follows.

SEQUENCE LISTING (63 sequences)

SEQ ID NO: 1 - DNA, 45510 bp, unidentified
  source 1..45510: mol_type = genomic DNA
atgaatcaggccgtaagtgacgaaatcgaagttgtatggcgtccaatcgaaggaacgtcgcaagagcttgcgattgattcgcgagcgcatcacacgttgtacgaaggcgcgcgcggtccaggcaaaaccctaacgcagttgatgcgttttcgccgtcgtgttggcttgggctatggccgatattggaaaggcgtaattttcgaccgtgagtttgacaatctttccggcttggttactgagtcgaagaaatggtttagcaaattcaacgacggcgcggtgtttcttgaatctgcatcgtcttacaaatgggtttggcctactggcgaagaactgttattccgccatgtaaaaaagatcggcgattatgacggttttcacggccacgaatacccgttcattggctggaacgaacttactcgttattcaaacggcgatttgtacgacaaatttatgtcgtgcaatcgctgtacgtttacgcctgaacgtgatacgcctcacagggttgtgcgccagggcgataaagacattctcgacgcgtttaagtgcgcagacggaacgtatcgcgttttcgatacgccggatagaaagccgctgccgcagattccgcttgaagtgttttcgacaaccaaccctgacggccccggccacaattgggtaaaagcacgtttcatcgacattgcgcctcgcggcgttttggtttcgactactacgcgcgtattcaatccgcagacgcagcaagacgaagacgtaaccaaaactcagattacgctgttcggttcgtatcgcgaaaacaaatacctcacgccggaatacgttgcggagcttgaaaagatcaccgacccgaatttgcgcaaagcttggctgttcggcgattgggatatttcggcaggcgacgccttcggcgatctttggaattcggcctatcatgttatcccgcgctttgcgatcccgaaggggtggagcatcgaccgagcgtttgactggggtagttcccagccttacagtgtgggctggtgggccgaagcaaatggcgaagaagccaaagtaaagatcggcaacgaatggtttacgttctgtcccccggcaggaagcctaattcagttctttgaagactacagcgcgcccaagattgaagagaacaagggcaataagctttcagcaaagaacaccgcaaaacgcattatcgaaattgaaaaatcgctaaaagaaaatggctgggttgaaggtgaaattttccctggaccggccgacaacgcaatcagcaatgttacagagtcggacaccgaaaccattgaaaagaaaatggctgacaacggcgtaacttggcaagagtcggataaatcgaaaggcagccgaactaacggcttccaattgttccgcgacaggcttgaagcagtgttggaaaacgaagggccgggcatatactttatgcaaaattgcacggccagcatttccaccattcccaagcttccgcgcgatcctgttaaagttgacgacgtagacactaccgcaattgaccacccttgggatatgacgcggtatcgggttttgaaaagttcgaatcgtttggctcgtagtattaaagtaaaattctaattaaagggcaattcaatggccgttcgcagcgttcccaatacccctaacgtaactttcattcatccggccctttctcagaaaatggccgagtacgcagtaattcgcgactgcatcgcgggcgagacggcagtaaaggctaagcgcgaagcgtatttgccgttccctgatgaatcgcggctcgaaatggacccggacgtagttaaggaaggcaaagcgcgttacgatgcgtatttgacgcgcgctgtgttttacaacgctacgcggcgaaccctggacggcttgaccggccaagttttcatgcgcgatccggtttgtgaaattccggcgcaaatgtctgcactgaaggctgacgtttccggcaccggaattagccttttccagtctgccgaaatgtcattgcaggaagttgtttcgtattcgcgcgctggcgtgttcgtagactttcccgacactacggaacggggcgcatcggccgacgatgttgcaagcgggcgcatccgcccgactttgtattcgtacaatacgtttgaaattttgaactggcgagtcaaagaaatcgattcgtctgaagttctgtcgcttgtcgttctaatggaaggcttccccatgaacgacgatgggtttgaagtcaaatacggtccgcaggttcgcgtgcttcgtttgaacgaagctaacgaatacgttcaagaaatttggcggcaagttaagccgactgagtggagcctgggggccaaaattccaaagggcaacgaattccgtttgcattcgacgtattacccgacaatggcagatggaagccgagccaagcgcattccgttttggtttatcggtagtcgcaataacgatgcgaatccggaaaatccgaacttctacgatcttgcgagcttgaacattgcgcattatcgaaacagcgctgactacgaagaatgctgcttcctgctgggccagcccacactagttgtaacgggaatgcagcaaaaatggctgactgaagttctgaaaggaaagcttaacttcggttcgcgcggcggcattccacttgaagccgagtcggacgctaagctaatcactgctgaagaaaacagcatgattaaggaagcgatggacgacaaagtaaagcagatgaaagggcttggcgctaagcttgttgaagagcgtggcgttcaacgcaccgcaacggagacgcgcagcgacaatgcttcggaaagttccgttctggcttcgtgtgcgaataacgtaagcgttgcctataccgctgcgcttgtttacgctgcggagcttatggggttgggcacaaacggcatcaagttcgaattgaacaaggatttcgatctgtcggcaatgtcgcccgaagagcaacggcttatcgtagagctttggcaaaagggcgcaattagctggcccgaaatgcgaactgcgctgcgcagggcaggtaaggcttttgaagacgacaacaaggttaaggccgaaatcgaagctgacactctgaagcaaatggaaatggccgcatctgttgaaggggctgcgccgacgggggccgagtaatggccgcgaaggacgcgttgcgactgtttgatttgacggtaagaactgcactgctggtcgaaggcgtaaagctgggccagcagcgcgaattaaatgctgttgtcgctgaagcggaaaaggaatttcgcaaagttatgcagcgagtaaaatatgaaaagctcggccagctaacaaaggccgagcttttgaatttgcttaaagcggttcgcgcatcgcaatccaaagtttacggggcttacgttaagcacttcattaaacagcttgaagagtttatgaaggagaagactaagcttgacgcaatcattttggggactaacagctacgatcccgaagaagctgaaccgcttagcccgaccaaggctttcaaccacattgagcgcacgcaaaaagaaaagcgaacttggcccattttcggattgctgtttttgcccgcatccgcgccactgctttggagtcgtattcgaaatacaccgattccggcaaacggaatattgccggaaaagctgattgcgggctttgcaacaactgcacaggtttctattgaaaacgaagtgcgaaaggcatatgcaaacaatatgcagcttcaggaagctatcgaaacaatcgcactgagccgtagtgctacggcgcgacgccagggaacggcagcagtggaaacgacagtggggttcgtatcggaaactgtttaccaagccgtggcgtcggcgatccacacgttctacaagtggatttcggttatcgacaacgctacaactgacatttgccgaagccgcaacttgcgcattttccgttacggcgtcgggccaattcccccggcacattacaactgccgaagcactacggttccacttgcgcctgaagtggatgactttaaagttccaacgctttacacttggcttcgcgaacagccccgcgaatatctggacgaccttgtgggcagcaaagcagcggacgccatcgaaaatgggggaattactgcggctaatttcaacattgcaacaatcgtaaaacctgccgcaatcaacgggctttccaacaaggcaaagtcaattctaactcgccgatccgatggattggcttaaaggtcgaagacaatggcactgaagcgcaagattaccaaagatcagtacgaagcccttgccgaaaatattcgtttcgaatacaaggcgggcgaaagtgacggcgaattcgtccttcagactgaaggcgacgaagacattggcgcgctgaagcgtgcccatacgcgaaccaaggacgcgcttgcgcagtctgaagcaaagcgcgacgagcttgaaatcagaatcgaaaagatggaaagcaaccccgctcgcaagaccggtgacattgaagcactggaacgccagtggaacgccgaaaaggcagaatccgacggcaaattcactgcgaagatttctgcgcttagctcgcgcattatcgatagcgcgcttaacaccgctgcgatgggtctttccgaaaagatcgcaacgacaggcaatgcgaagattctccttccccacattaaggcccgcatttcggccgagcttgacgataacgacaacgttgttgtcaaggtgttgggccaggacggcaagccgtccgatttgaccattgacaaactcggcgaagagtttgttgcaaacaaggattattcgggtatcatccagggcacaaaggccagcggcggtgccggggcttcgaataacggcggtgccgtccacaccagcaacagcggcaacaatggtggcggcaaacttcttgcagacttgtcgccgcaggaactcgctgagcgcttcggcgcgaagtaaccctttcgaagtcaactcccaaaaggcaaaacgatggcactttccgacctgaaggtctattccgaaaccgcgtacagtgttgcgactgaaattcttcaggagcaaaccgacctgttcaatgcagcgtccaacggcgcaatcgtcctgggcagcgcagcacaccaaggcgatttcagcgaaatcgcgttcttccagaaaatcgcgggcggcaccgttcgtcgtcgcaacccgtatggcaacggcgatgttgcaatgaagtcgctggcgcatatcgccgacgtaatggttaaggtcgcgagcggcacgttcccgattgacctgtccccggcgcagttccgttggattcagttgaatccgcaggttgccggtgccgcattcggccagcagttggctaaggatacgatggcggatatgctgcgcatcggcctgggttcggcgcatgcggccgtcgtcaatcagggccgtatgctctacgacgcaaccaccgacgcggcaaacaccacgccggattccaagaccatgacttggctcaatcaggccaaggccgcagccctgttcggcgacgcatcggaccgcattcgcgtttgggcgatgcactcgggcgcttcgcacaagctgtatcagaacaacttgatgaacgtcgagcgcctgttcaacttcggcaccgtcaacgtgatgcgcgatccgatgggccgtgtaattctcgttagcgacaacccttcgcttgttaccccggcagcgggccagaacccggccaagttccattcgctgggcctgggcgcatcggcaatcgtaattcagcagaacaacgatttcgacgccaacgaagaaacgaagaacggcaaggaaaatatccagcgcacttaccaggctgaatggtcgtatcagcttggcctggacggctattcttgggacaagcagacgggcggcaaggctccgaccgacgctgcgctgctgtcgggcgcgaattgggaccagcattcgaccagcgacaaggacacgttgggcgtcgtactggaaaccaactaaccgacgtaagccggggcgtaattgccccggctttccccgtctcgcattacaaggaaacattcgatgaaaggcccgcatattctgtatttcgttgacggtcccgcaccgtcagccgcgcagcttgacgaagccgccgaaattaacggcattgtccagtatcgcaacgttcgtgccgtcgatctgagcaacccgcttgaaaaggcagacggcgtagccggtgaagtgccggacgcttacaagcactacccgtcgcccgaagaagccgttgaaaagttcaaggccgaagcccgcaagcgtcgcggtgcgatgggcgacaagcccgcgccgggaagcaacgccgaaaagctcgccaagagtgacggcgaaacctctcagccgggcgcaggcgagccgccgagcggtggccccgctactacccccgatgccgacgccgcgaagggcggtgacgcgcctgccgggggtgcctggggtaagccgcagtaaccggcgcaacgccaacaaaagccggggcaaaaccccggctttttcttaacctaaaaaggctatcgaaatgaccgataaaattctttacttcacggctgggcgcattccgaccaccgccgaaaaggccgaaatcgctgcaatcgaagcgctgtgcgttgtgccgtattccgttggcgttcgcaatcccatcgattcgccgaactacggcacgccggaagaagccgactacgttgcggggaccgttcccgaagaagagccttacgcatcgctgccggaattcgacccggccgacccgccgaaccccagcttgcccgcagacaaagcaattgtgggcaatggcgatagctatcccgtaaccggcggcactgtttccgtcgcagtcgccgggggcgttccgaccttcactttcaccccgactccgtaaggctaagcaatggctattcaaatcatcgttgaagacggaagtattgttgccggggcaaacagctacgttagcattgctgacgcacgaatctacgcggcaaatcgcggcgtacagcttccggctaatgacgatgacgttgcggccatgttgattaaagcaaccgactaccttgaagcgcaaggatgccgcttcaagggtcgtaaagttgactgcgatcaaccgttgcaatggccgcgaaaaggcgtctatctgtgctgcgatccgtatccgtcagaccgcattccgaaagaccttatcgcggcgcaagttaagcttgcaatggcggcaagcgaaggaatcgtattgcagccgaactacagtgcggcggatatggttatcgaagaaacggttgacgtaatcacaaccaaatatgccgatccaacttcgttgggttatgaaacgacgtttaccggcgttcaagctttgctttcgtcgcttgttacggatggaagctgcggcgggatttctcttcgcggtcggcgggtttaattatggctggccgctttgatcgtcaaattgcaacggccgcgcgcctaattcaaaagaatgggcagcttgtcgatttcgtcagtcgcgtaaaatcgattgatgacaatttcaatgaaattgtttctgaagttcgccataaagtatggatttgctttattccatataaaagcgacattaagcaattcatggcatacatttcagggaaagaacttaaaagcggaaccgtcttaggcttgatggccggtaatgttcctttcgctccggacctcacagacttcgttgaaagggatggcgttcgcattgaaattttgcgagtcggcaagcttagccctaacggccaatcaatcctttacaagttggagcttaaagaatgacttcgacttacaaccattcaaccgacgcaatgcgagcgcgatttaaggcggcgatgcaatccgccgccgcagtcgcagcaaacctgggcaatcctgtcgaattggccttttccggcatcgaagggaatgctaagcttccccgcgataaggtttgcgcaaggttggatgttcagcatattttggacgaccaacagacgctttcaaattgcgtcgaagagcctttcaaaaagcggtatcttgtttcgggaatgttgtttgtcgaattctacgccccgaaaaccacggtcaacgccgcaaagataattggcgaattggcagagattgcaaaagcagcttttcgcggtagggaaatgaacggaaacattacctttcgtagaacaaggattgtaacagcaccgaaggaagacgatttttaccggctcgacgtgtcttcggattttgaatataaccaaataggctaaaggaaaagataatggcccgtatctgtgataatgaaggcattgacggcggcttgaccggccttcggattgctgaagaagtttgcttgaaagaactgcccacacaagcaatcgacggtttcgacccgacgtggcacacccgcgaaccgaattcgtattccgatttcggcggcgacgttacgcttgttgcgcgcgaaatcatcgacccgtcccgccaaaacaaaaagggtcgtccgaccgacctcgacgcgtcgggcggctggaatgaagacctgacgcaaagcaatatcggctggcttgcacaaggctttttcttcgccaacgctcgcgaagccggttcgactgacccgtttgacccgacgaagaagattgcaattaccgccgtaacttcggcggataagcgctatgccgccgcgtcgggcctggatgccatctttgccgaaggccagcttgtaaaggccagcggcttcgcatctgccagcaacaacggcctgaagcgcgttactgccgtcgccgctggttatatcgaagtcgccgaagcgctgattgctgaagcgtcgccgtcggccaaggccaaggttgaagttgttggcgggcagttcgaagcgggcgatgtttcgattgcggtggttgacggcattccgtcgctggtttccaccgctaccgacttcaccactttccccggcttgatccccggcaagtggctgttcctgggcggcgatgttgcgaattcggcgttcgtaaacaacaccggctttgctcgcatcgcaagcgtttcggcaaacgcaatcgttttcgatgacaccacttggcagcctgtgaacgaagctggcgcgggtctgtcggtgcagttcttcagcggcccgctgattcgtaacgaaaaggagcgcgccctaatcaagcgtcggtcgtacacgattgagcgcaccctcggcgaagacgaagccacttcggaaaatcccggcgacgaacagggcgaatatttgctcggcgcagtgccgaacgaattgaccttgaacattcccgtcgcggaaaagttcaatgtcgattacaccttcgttgcctgcgataacgatttccgttcgggcgcggccggtgacaagctgcgttcccttgtgggcaccgttattccggcccttggcgaagatttcatcaatacgtcgagcgatatttaccgcatcaagatgaacattcttgacccggcaacttcgaatccgactggcctgttcgcctggatcactgaaggcaacatcgcaatcaacaacggtattacgccgaccaaggttgtcggcaagttcggcgcaggtagcgtgtcggccgataactttgccgttacgggcgaagttactgccctgttcaccagcgttgcggcctgccgtgcgattcgtgaaagcaaggatgttggctttaacgtaattgctgcttacaacaatgcgggcatgatttgggatttgccgctcgtttcgttgggcggcggtcgcctgaacgttgaaaagggtcagccggtgtcgattccgttgaacacttcggcggcagaaaacgtctacggttatacggcaatgctttgcctgttcccgtacctgcccgacgctgcaatgccgaagtaactggcagcgccacaaccgatgcgatacactgaaagggccgggcattccggccctttctttcattcaaaacacaggcagaaaacaatgtccctttcccgttcgtttttgatcgacaacaacgccgcagaaaaaggcttcgagttcgccattggcgaaaagaacgaagacggtacgcagccaaccattctcattgcgcgcgctggatacaacaaccgccagtatcaaagcggtatcgcaaaggcttacgaaaagtttgctttgcaggatcgcgcaggaatcgacagcacgcttgaaaaggccaaggctcgcattccggtaattgcaaagcatatcgtcaagggctgggccaacattcccctcggcgacgtgaccggcgaagacggtttgcagggccgcgcatttgccgaaggctatgccgatttcagccccgaaaacgcaatcaagcttttcgaacgtctgccggaactgttcgcaattgtcgaagtgcagtcgcacgaaacgtcgaacttccttgtcgcatcgcgcgaggaagcagcaaaaaactaacggaagttttgctgtatgtgcttgatttcggcgaatcggaattgacgataatcaagcaggctttgcgatgcggcgagccagttcctgaccgcatcgcaaaagctccaaggctattcagcgggcaggatttctatttaaatgcgttcttcgaactaggaacggagcgaagcgcaggggattctagcatcgggccgataccctggggcagcattcaacgatacggcgaaactttcggccttgattttgatgcaatggaatcgctccattatcacataaggcaattagataacgcctaccttaaacgcgaaagcgccaagatggaagccaaggtgaagcatggcaaatctgcacgatctggcaaagcgtcttcgcggaaaggccggggcaattgaaaaggaagcaagccgatgcgccgttgaaatggccatcggcttcgttcgtgaagtggcatacagcacaccggttgacacgtcgcaggcgttgtcaagttggatagtaactattgacgatccgaccgcagataaaaacccgccgcattttaggggtaaaggcggttcgacaagaaatataagcgcggccgaaaccgtggcgcaagctaggcaagttcttgcgactaagcggcctgggcaacctatttacattcaaaacaaccagccctatatcagaaagctaaacgacggcggacattctaagcagcctggacgctttcttgaaaaagggctgtttgtaatgcgaagtgttcgcgcaaatttcaagttcaacattgggtgacgtatggctgacgataacattcaagtagtcgttgaagataaaattgctgctggcgtaactaccaagcttaacagcatggcagacgcggccgacaaagccgggtcgaaagttgacgcgctcgttaagtcactcggcaaggtaaaagtaagcgcgtttgaccaagccgcaatttctgccgaaaagcttcgcgaagcaactgccaaagccgatgttgccgaacaacgccgtcagcagcaaattgcaaaaactgaagcttcgattgccaaaatgattgaagctgaaaacaatcaacgagtttctacgcagaaattgcagcaggagcttgcgaaaacagacaaggcattgcttgatgttgcaaccggcgaagaaaagcttcgcggcgaaactcagaaaactcagcagcaaatggcaagaactgagtcttcgctagcaaaactagttgaaggcgaaaatcgcgttgcgcaggccaaggaaaaatccgcagaaagctcacgcaaagcacaagctaaaatttcggatgctgagcaaaaggcggcaaaaaagatagccgacgcgcagcaggccgcagcggatgctgccgccgccgcagccgccgccgaagtcgaaagaaccgaacgtatcagcgcaatggttgatgcgtctttgcgcgaagttgaagccagaaacgaagctaatcgggcaagcttggcagcggccgagtcttcttcggaaaatgctaaggctattcgtagcgaagccgatgcaatggccgaacgcgttgcagcgatgcaaaaggctgaaaaagctgccgaagaaaacgcggcggttgttgccgagcttaatcgacagttggcggtaggcgtaaagactaccgaagacgttgcaagagttgaagccctgctagaccgtgcaatggctaagggcgctctttccactgagcagcaggccaaggcgcttgcaaatctggacaagcaagcttccaaaatcaaaaacgtttcaaacgaagttcagaatttgggcggcgttagcgcgcagacaagccgccagataacttcaatgatcgtaaatcttgcgcagggtcaatgggccgctgcgcgagccaacattgtgggcatggctcagtctaccggcctactcaatggaacgctcacgggcctgggcactgcggccggtggtgctgcggcgggccttgctgggctgcttgcgtatgtcgcattgatcggtgcggcagcattgaagagccgcaacgaatacgacgaattcaataatagcctgcttacaaacggtcgtatttccggtgcaactgctggcgaacttgctgttttgtcttcgcgcatcggtgagattacccacaattacgaagaagctcgcggtgctgtaaacgctttggcgcgagacggccgcgtttcggcggatcagcttcaagctgttgcaacttccgcagcatccttcgcaaagctttcgggcaccgaagttaaggaaatttcgaaggagcttcttaccgtattcgatgacccggttaaagctgcggccgagcttaacgcaaagtatagcttccttactgtcgcaacgtataagcaagttgcggcgttgcaggagcaaggcgataagcaagccgccgcaactcggttgcttgaagagtttggcgcaacttctagcaagcggctcgccgaagcaactaacgacactaacgggcttgctgccgcttggcaaaaagttggcaacacgattgaatgggcaatgcagcgctttaaggaagaaagcgcgatccttaccggttcagcaagcaagatggaagagcttgcagttcttcagcagcgcatggcgaagttcaacgaacaacccgcttgggtcaaggggcttacccccgacgcgttgattgaaaagaacacgaagcgaattaaggaacttacggattcaattgaagctgagcaaaaggcagcacgcgaagccgccaaggctcagcaggttcacgacaaggcaattgccgcaactgactcgttgaaggctcgcgaacttcagcttgacaagacggcacagaaaactaaggaactgaaagaccttaacgccgaactgacggccgcttacattggcggcaattccggcataacaatggatgacaacggcaacttcaacgatgctcgttcgttgaagcttattgctgcgatcaacgaaaagtataaagacaagggtgccgaacgcgccgcgaaggctgctgccaaggctgaagaaactcgcgcaggtgccctggcaaaagtaaacgcacagcttgacaacgaaattgcccgcatgggaatgcttggcagcgaacgtgaagcgcaagagcaattcgataaggttagcgaggctctaatgggccgtcgcatcacccttaccgaacaagaaaagaacgcaattcgcgaaaaggtcgatttgcttgcaaaggctcgcgacgaacaggccgcgatggatcgcatttatcagcaggcaaccggcccgcttcgtgatttcaacgcaacgcttgatgctgcaaacaagcttgtcgaaaagggcgctatcacttggcagcagtttttcggcgtcactgcgcaggccgaagaagcttacaagtcagcaatcgatccgctgtatcaaatcaacaaggggcttgacgaacaaaccaagcttcttgcgcttaattcgcagcagcgagaaattgaaacgcagctaattgccgctcagaatcaggcaattgcaagcggtcaaaagattcgcgacgaagaccttgcgcagcttcgcgcacggcttaccgtcatgcaagaattgcagcgcgtttcggctattgaagattcgattcgccagggaagcgggagccagcgcaagcaggattcgcaagatcggattaaggcggcaacgaatgtcgccggtcagggtggtgtcgatccgaccgatattgtgggcatgatggctcagcagaacgcagggcttcaagcgacgcaggcgtatacgcaatatcaagtcgaatcgtatacgcaaatgtatgccgaaattgacgctttgcgtcaggctgatttgcttagcgatactgacgcacagcttgcaaagttcgcagtgttccagcagcaatcgcaacagtatttgactgccgcaagcactgtgtttagcagcctgtcaaccctgcaaagttctgaaaacaaaaaacaagcggctatcggcaaaaaggcggcaattgcgcaaaccctgattcaaacttaccaaagcgctacgtcgtcgtttagcgcaatgtcgggtattccttacattggcccaatcctgggcgttgcagcagcagcggcagcaatcgcggcaggcatggcaaacgttcaaaagattcgcgcaacgaacgcgggctttatggacggcggctataccggtaacatgccgcgcacgtccattgctggcccggtgcatggtcaggaatacgtgttcgacgctgcggccactcagcgcatcggtgttggcaacctggaagccctgcgcaggggtagggtgcccacacagattgcggcgcaggctgaggggcaggggagcggccagcgggccaatttcgcgccgacgatcaacgttaacgtcgaaggcggtcgcatggatcgtcgcacgccggaacaaattgctcgcgcaacgcgaacgggcgtttccaaagaatacgaacggagctactaagctatgggaaagattacaaaggcattcgacccgtcattttcctacggtttcgaaggcgggcctagctacgaaagcgaagtcgttgcattggaaaacggctttgaacaagtcgatagtgcctggcaatatgccaggcatcgctatacggccaaggccgaagcgattgacgacgaacagaaagaatattacacggccgtgtttcatgcttgccggggccgcttgcattcgttccaatttttggattggaacgattacattgcaaaccgcgagcctttgaaggtgagcgccggaacaacaaagaaagttcagctttacaaaacgtatacgttcggaaacgccaaaacgattcgccctgtgcaagccttggttccggccgatcctaataaccgcgatccgaatttccgccaagctggccctaaagtatacacggcgggcggaaacgaagttgcaggcactttcgattttatgacaggcgaatttacgccgtctgaaatatggggaagcggcgattacacttggtcgggatggttttatgtttgggttcgcttcgacagcgacgacaacacaatgactatcaacagttggaacaacagcggcttttcaatttctctaattgaaaagaagtttgaaattactgcggataacatgccgcaaagctgggtaggataatgcctaagcaaattccgttggcgctaaagcttgaatattcgaaaagttcaacttcgacggcttatgcggtaaggattgaatctgttaaaactggcgaagtcgcaggcttcactagctgcgattcaactttgcgatttgacgacggcgacgggttggttgcgtattcgccggtcgaagagcttgcgccgcaaaactttcaaacttcggcagatatggccgtagacaacacaaagttagttgggtggtttagcgatgcgttggaaaaacgttttcttgcgggcgttttcgattccgcgaagataactatttaccgcgtagcctatttgaatttgggcgctggatttgaaattgtaggctacggtaacgtcggtgaagtcgattacgcatcggacgcaaaagaacgtcgcaaagtagaatttcgcgggcttacccaaattctcgcggctagcacaaatcagctttacagtcttacatgccgtgcgaatttcggtgattcgaaatgccgaatgccgctggcctgggaagctgcaaccgtaaccgagctaggctcaaacgctcagttgaaatttaaagtaggcagtataagccgacctcctgggtattttgagcttggcgttgtcaactttattgatggcgacaacgcaggtgcggatcttgaaattgaatcttgggaagccgacgggtctgtgaaacttagctacgcaaccccttacgcaattactgtaggcactaaagttaggcttcgtcgcgattgcgataaaaccgaaactaattgcaaagcttacggcaacattgttaacatgcgagccgaacacttgaccccgaccgaagatcaatcgcttatggttccgggtgcgtatatcaaaaatcggaatgcgctatgaaagaacgaattgaacgcgccagggcaatgctaggggttccgtttttgcatcaagggcaaaacgaaaagggcattgattgcgttgggctattggctcacgcaatggcctttccgtttagtcgagttcctgcgtatcctcgcgatccccatcaaggaaagcttgaagctaccttgactgagcttttcggcccgccgctaattacgaaccccgaaagcgccgatgttttgcagcccggcgatttcgtcgcgatgcagtatcgcggccccgtccgtcatgtgggcatcgtaacagactatcccggcgctgtcggccttatccataccgattcaatggtaggcgaagttaccgaacatcgcttagatgaaaaatggctgcgccgaattgtttacgtgtggcgcgtataaatggctggcctgtttggttccattacaatcaagggaaacagacttaccgagtttgcttcgcaaactgcgacggtaggcgttccaattccttacggcttcggtcgttttccgtgcgaaggcaacgttattttcgcgccgatgccgccgaaagaacacgtcaagaaaaagaaacagggtaaaggcggcgtaaaaagtgaagaatacagctatacgctatcttacgctgtcgcattttgcgaaggtccgattttcggctttttgacgatcaaacgaaacggcaaagttgtttggacgcaagaccctaacgcatccgttgatgatagaacctatgccgcaaaatggaaaagaaaggcaacgttctattacggcacagaaacgcagcttcccgattcaacaattgaaagctatcgcggcgtcggacaggtttcagcgtttcgcggcattgcttatattgttgttgaagacgacgacgttacggacggcggcggcgctgtgcccacatatgaagctgtagtcattgcatcgccgcctgacgcgtaccttacttcgcggccgtacccaagcgatatggctcccgaatcgcttggaactacgtttgccgtaatgcctggaatgctaaggcagacttcgcacgtaggttattcatccgatcttgtcggggcaaacgtgtctcttgccgaaggacagctttggacgcctttggtaaaagttaacgcagaaaccgacgaagttcaaagctcaatttcagttggcgaaggcaggctttacaatcccttggtttcagctaacgccgaaattgacacagttaatgccgttggaattcgtccgctttctggcgttcttgcagttaagcttattacatacacatattggcctgccgaatcggtcaattcaaacataactttgccttcgggcggatacttgggagtttgatatgttggaaccgattaacattaaacgcgaagtcggcggcttttatactttcgttaagcacaagaacgacagcgacggcaatcctattccaggcaccgccgaaattgtcggtatggccgatacaccgaacttgctgactaattacggcatgaattcgtttgccgggtcgcagtttatgagtttttctagcaacggaactgcttgctgcgtcggcagcggaaatcaaacgccgcagtttaccgatacgcaacttcagtcgcaggttgcacagacccaaaaccagccgagcggcatcggcgcggcgagcggcattgtgcttaccgatacggccaaccgttacggctttcttcgcaatgtgtggcgctttggcgacggcttggccgctggcaatcttcaggaagttggaatcaggggttatcctgttgatgggaatagcttcaatactgcgccgctaatgtccagggcgctaattcgcgacgtaaacggaaatccaacgtcaattaccgttttgagcgacgaaacgcttgatgttttctacgaaattcgttcttacattccgaacgatgacgttaccggctctatcgtgctggacggcattacttacaactacactgcccggcccgttgacgtaggggcggagaattacggggcgtggtggtatcagattgcgtcgggtcgagcgattatgtcaggagcgcgaaatgatttctcctggcagtctgcgccgtacaatcaatatataactactacttcaaatcttacgctatacccccaaactcagcgagcttatgaacttttggctaacggtcaagcgcccgcaaatgttctaaaatctgcgtatgcgcaaaactcttaccaattggacctgactcttgttttcgggttgcttgaaggcaatttggcgcaaggggttggaacaattttggcttcgactggaatgttcggcggctatcaaattgtgttcgacaaaagaattcccaaagacgggacaaagaaatggaaccagccgattcggatttcctgggcgcgtaggtaaatacaatgatccccgaaggtacactttcaacgaagtctgtagttagcgcgacggccgacccggttaaacaaccgggcgactttcttgttgattgggagcgcgccgggaaaaatttgaatgatccgtctgaaggcttgcttgtaaagctttggacgctttctgtcgacactgttgacgaagttcaacaggttaaagtttcagcccccggcgtagatgaaattgttttgtttaccggaactgaaattaccgaagcttcgctagcattcgatcaaaatatgcggccgtttgttgcctttgttcaagcgaaccaagccaaaatttattggtacgatagttctgtccctgggcaaattacgacagttctcccggccggaatcaaaacgccgcgttgcactacagatgaaaagcgcgaatggcacacagcaatttccgatattgttcttagctacattcgggccgggaatctttgcgttcgctatcagcgcgagcgctatcaaatcgaacacgtcttgaagggggtcggatcgaccgccgagcttgtcagtgtgggcgtaaacgcaggcggaaggctccaatttaggtgtcgtaaagtctcaaacatcgacagccaattttcggtaaacgcagacccgtaccttgccgatgttgtaatggccctttgcctgcgttccggaatttctcccgaacgaatcaacgtttccgaactgtacgaccaagccgtaattggctacaagataaacacgaaagacggaaccaatgcgcgaattgacgcgttgcgaaagattttctttttcgataaaagcgagcgcgatggaatactattcttcccacgtaggggtcgcgagattagcgcgcgcattccttacgtgcatcttgttgccgatgatccttcggcgcttggcgtcacgctagttcaagaaagcgaacttcctgccgaagttaacgttacgcatttggacccggaaggcggttttgcaaacaacaagcagaccgttcgccgtaaaagcaatttggtaaaaaccacaaagaaaattgatgttgaaagcgaagtggttttgaccgcagaccaagcagcaacaacagcgctaatcactagcgtttctgcctggggcgagccgcaaaaattcaagttcaaaacaggcttgcaatatgcggaattggttgctgccgataccgtagaagtcgaagacaaaaacggcaattggcatatcgtccgaatcactgaacgaaatgaagaccgcagcgtaatcgggtttgaaggcgtttcggatgcgcaggagctttacgcgtctttgggcgtaggaaggccgctaacgccgccagtatccacaacccccggcttgatcggccctacgcgcattgaaattttgaacattccgtgccttcgcgatcaagacgatgaactaggcgtttacctgggcgtatgcggggaatcttcaggttggtacgggtcttcgattttggtcgctaccgatggtgcgaactttaccgaagctttgacaattgaaaccccggcaacaataggggacacaacaaccgaaatgcttgccgaaattagcgccgagtatccaggcaaccaagctgtcgaagttttgacaaactacccgctagaatcggtttcttatgaaaatttgcttagcggaatgaaccggtgcgtaatcggcgatgaagttttgcaattccaattcgcaaatttccttggaatgtccggcgcgctgtatcattacaagctggtcggattggttcgcgggcgctatgctacaggcgtcgaggcttggccgcaaaatactcgcttcgttttgctcgacagcagtattgcgttcatgcaagctcagcaatggatgctggggcgcgagatacaaataaagccggtaagcttgggcttgacggaagacgaaacaatagaaactgaatatgactacagcgaaggcgtgtcgcaacgtgaattccctgtaacgcaagtaactgcaactcgcgacggaagcaacaacgtttcagttgcgttcgtaggtcgtccccggctgggaattgaaaccgccccgcgaaacggcaagtattttgcaggctatcgcgtaaagtttagcaacggaaacacgatagacacgttcgaaatggcggcttcttaccctagcgctccggcaggaatttcggtgcaaatttgtgcgcttaattctgtgactggcgaaggcccgtattcaaccccgataatggtgtaacaatggcgactaccccgaacctcgatttgcctcagattccgcaaaatgctcttcaaatttctacgccgtataacgaagcaatgcaaacgctcgacggcgttgttcagtgcggcgtcatcgacgttttgaacgatcctcctgcaactgccaacgcagacattggccgatgctggcttgtgggcactgccccgacaggtgcgtttgtttcgcattcaaacagccttgcaatgtgcgtaggcgaaaatttgtggaagttctttgcgccaggaactcaagtaaaatactttttgaatttggcgaacggcggattttataaatacgaagctgcgtcgcaatcctgggtgcttgctggcggattgggcgacgcgccgaacgacgataaaacctatgggcgcaaatcccaaggttgggtcgaagttggaagttcggcagcggttcaaagtatttctgccggaactggcattggcgtcgatagctcaaatccggccgagcctgaagtttcgcttttgcttgaagctgggagtaatgtcgaacttgttccggggtctgcccccaattcaatcaagatcaacgcgaccggcggatcgggcgggggcattcctgaagccccaacagacggaaagcagtatgctcggcagaatgggcaatggacggaagttgtaagcggcggcgatgttgcgcgaagccttacagtaaccaccactggaaccgacgacccctattcgaagtattccgaatgggaaacggccttcggattttctccaggctcaaacgattacccagcaattgcagcagtcacagacgacgccgcgtttttgctttcaattggcggtcagcaaaagccggggtttccgccattcctttcgctagggtccgaagggcatctttggtacgaatttcccggttcgccgggtatcgcatcgcaggcacctacgccgcttccgcctgatacaaatcgtgcgtattggagcacgtctccgcatccgcgaaaaggaatttgcttccatcctgacggatcggacgccgaatccaaaaactgcatcgcaaaatatacgccaaacggagtaattattcgaggcttaattgccttcccgcgagggggcacaaacggcgtaaagtttgcggcaaaatttgatggcggaagctgggagctttatctcgcaaacaatttgcttaccgagcaatgctctttcatgtttttggaaataagcggcccggacagcgcgccaacctatagctatattggagcgcaccccaaaattccggtaggcggattccttaaagccgaatacaagtaaaaacaacgggccgaaaggcccgttgttttatgcaaataacgttggctgagcttttggagtaaagccaatgtccgatagaatcttttggcccaactgaacgtatttgtcgtaatcaatatcttgcgggaatgacgggggaaggtcttgcaaaggctttgccccgtcgctttttccaaccttggaacctttgccgatatactcaattgggccgtgcgaatctgcggcgtaataccaacgaacaaccttgcccacatagaccccgttcttttgcgcaccgccgttcacttggcgaatcgttgtgaatctgcgaatgtctttgcaagcctggatcgtttcgtgaagtggaaccccatcaacgatcatcttgattacggcgtcggtacagataaggttttccgcattctttgaaagcacgctgttcaatgcgctacctacttccgcatacgcacctttaaccttgcagcccattcggtccgcgaacgtcttgcccttcgggtcgaaatcaatttcgccaggaatgaatcgctttgcttccttgtcaaacttcagcttgaatgcaagatagttgttaacgtcgcggctgtaggtcgaatggtattgcgtttcttcagtttcgaagttggtaatacgttcccaaagtgcaacaacgtcgttcagttcgttgtagcggttcgccgggcacttgataataatgccatcggtgttacctgacacaaccgggattccgtgatgctcaatcatttcaatcagcattagcaacgcaagctgaccggtgatagttaccttcagcagcagctccggcgaatacaccttcgaatggcgattgccaagtttgccgaaaagaccgttaataacaatcttcagcgagtttgcgatctttttgttgccgacagctttagcctgaagacgctttgtaacaaggtaatcgtatacttcaaggaaagcccgcccaaggtgtttcgggaaaagcttttcgttcaagataattcgcggatagaagcttgcaacgtcgcgatcaataagcaacaggtcttccgacgcaacatgctttacgcacgattcggaagagtgcaagccgcccatgccgagcttgtatgtgctgctgccgatctttacgctaagctgccaaacttccttgccgttcttatctttgacaagttcgcccaagcctttaggccaaaccggcgaaccgttcgcgtctagcatgaattcggcggattcgatgctatcaacaacgtcgcgaagctctttagacacaaagcctacccagccaggggctttgtatttgacgctgtaaatttcgtctgtgttgtcctttggatagctgccggtgattcgctttagctcctggcaaaccactgcttccgcgatctgagcatctgacttgctgcgaaggtctagcttgtattgctcgcctagctcttcgcgcaacttcaattcacccgcaagctcttcccaaagaatacgggtcaagtgaaggtcgttgacgttgtaatgctttacttccaatgcttcctgacggctaaggtttgcacctacagggtacggcaaatcttgcaagcggtcagcttgcagccttgcgccatacagcttcaagccgcccgacaacggggcaacttcaataaggtcgatatggttaaatctgtcccaatcgattccaaagccaaacattttcgcaacgtcttttgctttatacaagggcttgttattctcgcccttttccataagcttttgcgtcacaaggaacagcaattcggcgtcgaagcccttcagtgctgcgaagataattggaatatcgtatttgcgcgaattgaagcctatgcaacaaaacttttccatcatccattgcaaaacgccggtattaaaccggccatccgggcttatctcaaaatgaacaacctttttgctaatagggtcgaggaaaccgacgcaccaatagttgccgtaagattcaacgtcaaacagcatcgggtggtttgtgggcagcgcaattagttcgtccggcgtaaattcttcaaacgccttcagttcaattgccggtttcacaagtttgtgatatggcgttcctttcggcccgcctgttcgcttttccgtgaattctgcggcatcgaatttgaacattaacgaagccccttgattacgcctcgcgtgttgccatcttcgctaagaaacatcaaagccgattcgtcagttgccaagtcaatgcgatgcaataccgacattgaaattttcaaaaagtcaatgttgaaccgtctgttcggcggaagcccttcgatttcgaaagccccgctttcggtgcgcccgtcttcggcaaacacgcgcattccttcgctagtgaattcaactacgttagtgcttgccttcgaaaaggtttcaattgccttaatgccttcaaagaatccgtcgggcaaaggccaatagttgcagttgtccgaaaatacggcgcgatagtctggatattgtccgctgaacaactggctcttaataaagcttccgtcttcgtagtaaaacgttacggaattttgagaaaagccgaattgcgccagcttcttagggcactttgaaatcgcaagggctgttgcgcggggaaccatgattccgggcggcaagtcaatgccgtggaacgtttcaatcagcattgcgccattgcttccgaccattgtatttgcctgaagcaatacggcggtttgcaggacgcgaggggcggtgtcttccagcatcggggccagcaggccaaagccgaccttcaggcggtcatccaccaccgcgcaggctgcgtcaggctccacgttcggggcatggcctgggggtaggcaagggacagtcgcccggaatcggccagaacgcacgctgagggtggtttctgaagcctgggtaattgcgatcttgtccccacatttggaaattgctgcggcgagcaggccggtattcgggcacgcgctgaagtcttcttcaatctgcattcccgccgcgaagattccgttaaagccaatcagccagttgttttcaattcggcaatgtgattgccaaggctcgccgtctttcttttgagcgggtagcacgaaggccaaggctgcggcaagccctggtgctgcggacgatttaggtttacgtgcgcgagttgatgcggccattgtgtttgcctcagaacggaatatcgtcgtcgtgatcggggcagccgcttacgataatgtgaggcggcggaactgcgcggaattttccgcaaccttcgctagctttatcccattcaatgcaattcaggcaagttttccacattccaacccttaccgcaaagtcttgcatttcaagctgcaattctgcgctgagctttttatgtcttgaaaaatcaagtttagaattcatggctcaaaatctccggatactttggggcaacgtcaacgcgaattgctacaggctcccgaagctggcttgttagctgcaaagcttcatatgtcgttgctggcgggtctacgcccattcgctgccgccaccagttacgtgcgcgtcttgacgttgcgccagggtgttcaaggcaaacccattcgctaaacatcaacagccctgcccaatacgtgaccttgatagacgggggtttgccttccttagtgtgcagactatagacggtcttgtgtacgtcataccgttcaatttgctgcttggtatcgccgcgcatcacttcaacgtcgctagattgctcttcaatctttacgtcaaacttaaattccattccgcaattttcgcagaaccgaattttaggatggttgtagcagtcgcagccgtcagtgtgccataccttttcgccgttcttcattcgccaaccttccttgcaaattcggatcggcatatcgccgccgcccttgccgggcttgttgggaattctaatatcgttgataggtccgtgcatttcgcagttcgaaccgtagtcaaggaatacgcaatttcgtttgaacgtcggaaatgcgagcgggtcaacttcgcccggccgcgcaggatcgtaagggcgcgttccacgtcccgcaatctgcacaaacattccaggcgatttggtcttgcgaagcattccaattagatcggtcggagtgtgatcgaagccggtcgtatatttcgacatattgaccaaggcttgaacttgaccactcttgaacgcctttaggttttcgtcgttttcgtccgggtgcagcttagaatggcttagcacaatttcaacgccagcgccgcgcataatatcgcgaatgaactcggcgttcttaatgctgctaccaaacaacagccaggacaaacgattctgaccgatgttgtagatttcttcgcaagccttttcggtgattgcgttggcacgctcgcccatttggttttgattgaagtcgccgcccgaagacgaaacgcccttcatatccatttggacggcaccgcgcttagtcacaagtggcgcaagatagccttcgaagacaagtcggttaaagctgttgaagtcggtaatgtcgtagcaaatatgggtgaagattccgccatcggtaatcatccctagcttcatacgatatggcgttgcagtgaatccgataacgcgcatgtaaggattcgttttaagaatctctgcgatgattgcttgataaaccgtgtcttcctggggcgaaagcaagtggcattcgtcaataatcaaaaggtcgatatggccgaatgccggaacagcatttcgcacgctcagcacaccgccgaacgtgatcggaaaaacggattgcttttgcttcaggcccgcgctgtaaatacctagcggggcagtcggccaaatttgcgtgagctttgccgcgttctgagcaatcaattcctttacgtgcgtcagcatcataattcgctgaccgcgatacatgcgaaacacgcgttcaaggaaacgcgcgataacaacgcttttgcctgtccctgtgggcatggctacaaccggattgcctacccggttgtgatcgaagaaatcaaaaattgcgtcaacggcttcgacctgataccaacgatcttcaaattgcgccggtagctgcatatttactcaatcgccttgtgcatgttgcagccgattacgataacgtctttcggaattgggccgttgtccgggtaaagattgcaacgccatttcgcgccttcaattggctcggcgtgttggcagctacggcagtttatttcgacaggctcgccgcgatggcaaacgccagcaaactcgcattgtgaacattcgtagctgtcggcaaccaatgagattttgggcggcggtgtttgcgagcgaataatgccgtcagccttttgaatcatttgctgacccaaggtgtgattaagctccaccacttcgacgtgcaagttatcatcgtttttgcagatattcaaatagacgcaatagcggaaattatacttgtatccgtaaacgccagtctgcgcataatgctgtggcttagcttttgccatgcccttttcgacaagcttgttgaagcttgaaccggtgccgttggtcttgaactcgaccaaaacaggctcttcgattccccattcgggcggaagaattgcaatgccgtccagggagccgccaaagtggcccattacgtcgcttacgcggtattgcgggaatttcaagccctgagcttttgccatacccacatgggtacggtaatactcgttgtcttccgtaattagatcgcaatcaaggcgcagttcttcgccgggctgcaaaatgccgtaagtttcgctgccaccgtgataatagaagccttcgcggttttcgaaccacactttgaagccgatgccttcaagccattcaatgaaacgttcttcttcgcgatggccgcgattgaacaggcgttgcatacggccgctgtgaatgtggtgcttgacccaacggaaaatgtaaaacagcttacggcggcagtctccgccgataagggacgcgcccaaatggttgcggtggccgtcgtcgtaagctgtttggcaatagctgtcaattgcttcagcgattcgcttttccagcgcgcgagctacgccgggtgcgccaagttcaatcttctttacgttatcgttcatcgccttgtcctattaaaaacatggcggcattacgccgccatgttgtttgccgatgttgcaggcagcttagttgcgctggccccacgacgggccaccattgccgccgttgccgccctggccctgctgccaaccaccattgccgccaccgttaccgccggtattgccctggtcgttgttgccgccgttattggcgttgttgccgttcgaattccaaccgccaccgccctgaccctgctggctgttgtcctgcgaaccctggttgctgtcgttgctgttggcgttgttctgcccctggccgtttccccagccgccgcccgagttgccgccgttgttctggccctggtttgcgttggaattgttgttgccccaaccaccgccgttgccgccctggttctgcgtctgctggttgttctgctgcggagcctgtccgccgccctggcccgacttgcccggctcgttaccgtgaatgtcgtacagctttttgatttcggtgtagcccttggcgtcttcgccatcggtcgccgggttgtggccgcgctgatagccaacgtccacgacgaaaggcttgttgaacaactgcgacaggtccgttccctgcgcgccaaggcggaacgtctgcgttgcgtggcacattgcggacaggtcgcgacgcgcaaaattgcgagccttttcgctttcgtgatacaggttcaggttccaaaaacccttgtagcccttttccggcccgtcgatcacttccagggtgaacgaagccatgccgttgtttccgtctttggttgccttgacttcaacaccggttgcgacgaccggatgacggcccagcggccagccgccgctaccctgggtcgggtcgacctgggtcgggtcaaacgcttcagtcagaaaatgcgaattgttggacattgtttttacctttgacttttcgaaaagtctttgcctttatacggcggcaaagttcaccgttgggcggggacgttttagcctataaactaaccgcccgagattggcgggcgtgcccttgtgccggaatcgaaccgagcttcttccccaaaacttttacgacaacgccttgcgaacaagattgccgaaatgcggcggttcaaattcgtccagcttgccgaaccggtcgcgggccataacatcatcgccgcgcgtttgaatggcaagcaccttgccattttgccccattactgtggttcgtgcaacacgcaaaattgcatcgaacaaatgcggcatctttacgttcaggtcttgccctgggaagaacggaactcgcttgctaatgccttgctcttcgcgcccgctttccttgcaaatcaaatacatgtgtttctgcggcatgtaaaacagcttattcgccacgtccattacgtgttcagacattgcgccgtaagccttcaggccgtgcgaatgcttcttcaggtagtaagcaagcacaagctcagcgtattgcgaaaacgaatcgacgcagcacgtatcgaacttcttcgcttccgccgagttgaacagccacttgaagaactcgtctgccccggccatcgtcaagccgtcccatgcggggatattgtgggcatcgcgcatcgaacccatgcccggctcacaaatcaacagaaccgggttgatggtcgttttaatcagcggcgtcttgccttcccctggcggaccgtaaacgatggctttatagccgttcgccagtgcgaaggaagatgcgggccgcagctttgaattgccgaagttctgtgccattgcttattccttcgggaaaatgcttttgcgaaccataatgccgaccggggcgggccttgcgcaccatgcgtaatgccaaacacggccgaagaacaacgcagagaatcgttcccgccacgtcattttccaatgcgaaacgatcacttcgccgtcgctgaaagtttcaagatcgacgcagttttccattccgggcggagccttccacgttttgttagcctggggaaaaggttgcggttccattgtaatcctcgcttggtagtctttgaagtggctcgctcgaccgtttacgaactgcctagctggcaacgtttaccgtcttcgaacaagccacttcaaagactgcgcccgaaggcgcagccgtattgcttacttcttcgccttcggcgcgatgatttcaagcgtcggagcgccgctgtcgatggtcagaaccggggacaacaacgccttgatttctgcaccgcgcgggtgttcatcaagcgccttgtattccgacaccgaaaggtctgcggtccacttcaccagccggtcggcgataaaacggccttcgtcgccgagcgcttcgattttctgcaaggctgcatcaacagcatcgcgagccgaaacgccttcgacatttgacccaagcttgtagttgacctttttgacggtcttggctttgtagccattgccaaggtcaacgttttcggttccgctgatcttgtcggcctgggtggcaaccgcgacgaacttcttgcgaagttccatttcggtttccttggcggcgtcaaggtctttctttgcctgctcccaatccgcaaggatttcgttgcggtagcgaatgaatcgcgggtcttccttgtcgagcgctgcaagctcttcttcggtcatcccgctatctttgtaatacttgatttcgttcatgttcggcctgttggctgttgtgacggggttattcaagcacagcttttcagcactgtcaagcctggggcttgtcgatgccgaaaacgcgagaaatgttaacttcttcaattacgccaacgcgcttcgaagtgcgctcttccaaaattacgcgctcgccgaacaggtcgcggttgttcgcgtcgaattcgttgaacttgtcagggaagcgcttgcgcagctttgcgatgttgattcgctgagcttcgtcaaacgtcattccgacggcactaagcccggccgcatcgtaccaaaggccgtcgccaatttcttcaacgaaattggtagcgtcaaattccttatccttgaacagaacgccataaagcagttcgccaagttcggtggcttcggtgatcttgccgatgattgcgtgaaagatcgtttcgcccctgacggcatcgccagggcaaatcttttcgccgatgaacatgcaattcggttcgtcggcatagcgttcatattcttgcaggtcgcggccgtagaagattgctttcttcagttcgtcggcatggttgccgttctgaatcagccattccagaacgttgcgcaacagcctcgcggggattgctccaccgtggaagttgtttgaaagcgttacggcggcttcggcctgatagtggaacggcggttttgcgtcggtcatgtggtgttctgcctgtgatagcccggtgatgggccgggaccgtcaccctacgcccgtccatgtgggctgtcaacaacattctgtatcttgacgacagaatcttgaaggggtagccttcacggcatcctaatgcccacatgatgcgatccaatggccgtcaccgacaaagcgcaccccattttgattgagacaatagccaggattcgccgtagaccctgcaccatttccattgaagagcttgccgcatcggctggccttggcgtgcgttgggttggctcgttctcccgatccgaaattgctgacccgtcatttaacaaagtgatggcaatcaaagaatgcctagacaatcttggcatcaagtaagggcgcgtaatgcttgataacattccaaacgaaatgcggacctatccgcattgggtcatgtggcggtatgaagaccgcgacggcccgaagccaacgaaagttccttactcgcctagaagtcacaaacgcgctgacgtgagcaagcctgaaacctgggcggactacgacacggccgttgcctgtttgaacagcgggcaatacagcggtattggattcgtgcttagcgagcacgacccctataccatgattgaccttgatgacgtatttagcgatacgtccggcgttcgtggtgaagaagcacagcgcaaagcgtttgagcttcagaaagaagtgttcaacgaattcaacagctattcggaattctcgccatccggcaaaggcttgcacgtaattgtgaaaggccaagttccttgcggccgtcgtcgtagctgcatcgaagtctattcgaacgttcgctttatgacgatgaccggcaatgttcatcgcaatgcaccgattgccgaacggcacgacttgttgcaagtgctgcacaaggaaatgtcaaagggtaaagaagcggccgtattctatgcgggcgcaaacgaaatcaagttcagcgacgaagaagttttgaagatggcggctgaagctgccaacggcgaaaagttttctgatctgttctatgaaggcaactggcagaaatactacccgtcgcaatcggaagccgatttcgccctggtcaatatcatcgcgttctatagcgaaaaccgttggcaggttcaaaacctgttcctacggtcgaagcttgccgagcgcgaaaaatcgcgcgcgcaataccgcattgaatacatgctcgcgcgctgcttcgataggatgttgccgcctgtagacattgacggtctgcaaaatctgctagaggaatacatgcaatcccgcaagcaggcggacattgtaaagacacaggccgagcctgttcaagttggcgagttgaaaccgcaaaagagcatctattcggttcctcccggcttgactggcgaaatcgcaaaattcgtctacgcccaagcaccgcgacctgttgccgaaattgccatcgtcgcagcgctgggccttatgtccggcatcatagggcgagcttacaacgtcagcggaaccgggctgaattcctatctgcttttgctggctccgacaggcacaggcaaagaagccatcgcaagcggcattgaaaagctaatgagcgctgttggcgtgagcgtgccgaccgcaagcgaattcattggccctggcgaaatttcgtcgtcgcctgctttgattaaacaacttgcaattacgccgtcgtgcttgtccctggttggcgaattcggcctttacttccgcaacatgtgcgccgaacatgcgccgccgcatttggttggcttgcgtcgatcattgcttgacctgttcaacaagtcaggctttggcaacgtagttcgcccgatggtttacagcgaccgcgacaaaaacactcgctccgttctgtccccggcgtttaccgtcgtaggcgaaagcacgccggaacgcttttacgacgtgcttaacgaaagcatgattagcgaaggcttgttgccccgatttacgataattgaatacaacggcccgcgtgttgaaaacaacgaaaatcgcggcatggttaagccttccgacgaactcgttgacaagctcgcaaccctttgcgctttcgcgatgcagttgaattcgaacaaccgtgttatcgacgttgcgcttgatgacaacgccgataggatgttccgtgatttcgataagcattgcgatgccaatatcaacacggccgaccgcgagattcgccgccacctttggaaccgtgcccatctgcgtgcaatgaagctggccgcagtgttggccgtaggcaacgacccgtatcaccccacaattgatagtgaggctgcgacctgggcgattaaccttgtcgtggccgacgtgcgcaatatcctcggcaagttcgatgcaggcgaaattggcatcgacaacgacgaaacaaagcagcttcagactgtagtgcataacgtccgcagctacattctgtcgccgtttagtgaagttgaaaagtatgtcaacggaatggcgaacctgcatagcgaacgaatcatcccgtattcgttccttcagcgtaagctagtctctgtcgcaatcttccgtaaggataagcttggcgcaaccaacgcaattaagcgcgcgctgaagactcttgaagagcgaggcgacattcagctagtatcgcgcaaagacctgtcaacgaaatacaagacaagttcagtcgcatacatgattagcaacccaaaggcgttcgacctgtgagcaagccagttatcaactatcgcaagacgcaaccggttctaggcgggcgcaggatcgtaacgccgagcgacactgttcgtaccgtgcggcatatcatgcgcgaacatcttgcattccatcggatgacgttaacttatgacctgtcagcaatgctcggcatcgccaatcgtagcgccgtaaccatgatgaacaaaaagtatccgattgctccccagcatatcgacgcgttcattgaaggaatgaagcttgacgaattcgatgccctggaactgcgcttgcagggagcaattgaatacgggtggcaactcacaccgctaaagaaatacgcaaaggtataaacgaaaaacccggctttcgccgggttttgtttttcactgcgatgtagtttcgtatgtctgcccgaatatgtcaggcttgcacgggtagaattcaccagcaacgccgcgaatgatccagtcaccggccgacgccttaacggttccttcaagcgtgtttattgcaatatgctcttcggaatgtacgacgccaccaccccaagcggtttcttcgtcgtgatagcgagccgtcccgccctggctaagcacccaatcaattacgggtgatgcttcggtggcggtgccaatccaacgcatcgcctcaattacaacgggcttctttcggaacttggttggttgcattttctatactccaatgaattgaaactcggggccggtcgtaaccagcgggaaaacatccatatcgttgaaccggcgcgtatccgtcgcagcttcagccgggctatatttcgaccggccttcgctaatcgcaatcatgcacggcgtcagcttgaatcctggcgattctagtgtgggcatcggtgccggttctgccctgggctgctgcctcacgccgggcggcacacgccccgccgtgacctgggctgaccctgacctagcggcgaacctgggcaaagggcgtggcgtgcgccgggcgagtcggtaggcttccccagcttcggtgcaggtgtgcaggattccgaacctatctgctaaccgccatttgcctgtactgattacgacccaatgaaacccgttgcgcttgcaatactgacattgcttgttagccattagattggttccttccaatgcttgatgcttttgaaatatgcaatgactttgcgacattcgggacaggtgataacttcccccggctgcgcaaattcaatcgtgcggtcatagtcgccagagtcatgcgcgtcaaatgcgatgccgcaaattgtgaactcgctgccttgccctgggtcagttccgtgcttcattgtccttgcccacgttaatgacgacttccagcttgaagaatgcgataaggccgcaatccatatagcgtgctgccctggccgtccaacgacgcgacgcattctttacgctgtcgtcttcgctcacgtcctgaacccaaatctgcatcacttcgccgcgaatgttgaacgtcgtcgttttgattgtgtaggttgccattagacaagctcccattcagtggacacaggaaacgacgaacgcttgccagcagtcttgttgcgcgattcgaaacgacgggccttggttgcaatctcttccgcgcgctgctgttcggcagtcttgcgcaggtccatcgtgctgacggtgcgggcgatcttcgacaagcggaacttgaagctttgcatgatggcgtgtcctgtgtgttgtggtgtgtgtctagattacgatggacgattacgatctgtcaatgccttcggctctacgacccgacgaacggtaggaattgttaaagtatagtgaagtttaatggccgtatagcacgcaagtgattgatttcaaagggaatatagcaaatataacaaatataacggtccggggtgtttccagggtgggtgtaacgtgtaagcgtgtaaattatacacattaaaccttacacacataaaagaagcttttaccattatatttattatatttattatatatgtatatatttcaatgacttaggcattctacgatcccttatatctgtataacggctatgtaacgtataattaagcgcttgacaccttgcatttaacgtgcaatgatggccttacattcacgcgaggcaagcaacatgacgtttgaaatcagggacagcagcccggccgcagtcgaagcagcaaaggccattgaaaacactggcgcaaagtatccgttcgatacgctggaagtaggcaagtcgttcacggccaacattgccgaagtcaattggaagtcgctgcgaacctgtgtgtcgcaacgtaacacccgtgagcgtgccaacgtgggcaccggcaaagtgttcaagttcatcaagcatgatgacctgggccttgtcgaagtcgcgaggcttgcgtaatggctaacgataagccgttttcaattggcgaagcattcactacaaggcgttacttctatgacgtaacgcttaggcttcgtggctgtacgaaccttgcaatattttcttccgttctggcagagagccaagagcaggccgctaagcttgcaaagaacatgctaagcaatcccaattcctgggaagtgctggaagctaggcaagtaacaatcacagtcaaacggccgggagcctgaaatgattagcgacaaagagaaagcgtttcgcgaagagcttgccgcgttgttcaacaagcacggattcgaagtagcttcttgcgggtgctgcggtggaaccatcattgttgaattcgacccggctaacgatcttcgcagcccggcaaccctgggcaacgtagacggccgctaaccgcctgcatcaatgtgggcagcacaggagcaaggcatgaaaattcgtgttgaaatttgaacgtagacggccgctaaccgcctgcatcaatgtgggcagcacaggagcaaggcatgaaaattcgtgttgaaatttgggccagcattcaggcgatgaatgacgcaaccgtaacgcttatgagtgacgcgagcgttgatgttggcgatttggcttatcgtgtttacgatatgaaccatgatgacgctaagcagcgtcgcgttctgggcgaacagtgccgtaacgcattcgaagctgggcagtgcgtcgtaacctatccgatcaagggctgagcaatgaaaactattcttcgctttagtagagggcacatgttttcttcgtataacggtgagcctttggcgtctcttgttattgacggtcatccctgttgcattgggcaattgaagagtattgatttcggtgcgggcgcttgtttgactcgcgttgaaacggaaagctacgtctatgtcctggtcgaaggggaaggcgaatgaacaagaaagagttgcttgaaatgcttgacaacgccattcccgacgaacccggtttcgtcaacatcgaagtcgagttctatgcggatgcagcggaccgcaaaacaagccttgaatacttggccgagcttaacgaaggccacttcggcggcaatgttcgcattgaaactgagcatgtgccgagcaatggcacgctgcgctttcgcttcggggtgccgtaatgaaaaacgcagggcatgttagctcaattgggctggaagccatcgcaaagctgttcaggcggcagcttcagttttacaaaacgcagaaagcgttttatgaatacgttggaattagcaaggctgcttttaacgcaattatgacgggcaaaggttccataagcgcaaagtcgcttatggctgttcgtgcttacgcttcgcgatttactaaaccgcttgttgacaagcaaccacccatcgtataagctgttagtaatccacacagcagggcacaggcaatggctaacgaaaaacgatggcaggttaaactcgccaacgggaagagtgttactgtttgggaaagcgtcttgtcgacgcacgacattcaggaatccacttttgagcgcgttcaaacaatgaacgtaggtgaaatctacgaagacattggcggcaacacttgggagcgcaagcaatgaaggatcgtatttggctggccgtgcttgtgaccctgtttgccggtgcggttgttgccggtgcaattgtcggtcacgaactgtatcaagccagggctgaagcaaagagactgaagccgaccaatctcgcaatgtggcagggcattgcgccgcaaacctatgtgcagtatgatcgtgagcaaggcatcatctgccttgccactggcgaaagcctggaagctgcattgaaagccaaaacctaccgttgcgagcgtgccgaatgagcaataagctaaagccccatcaacgcgagacgattgacgccgtaatgaccttggcggcgctggggttgattccccaaccgctcgtaggtgctgggaagtcaagtagattcaaaacaggcggttacaccagcgcaaagcctgaaggtgtgccgatgcaagtaacaaacggcagcgcatacgtagaagtaatcaagcctaagccgcgtctcgtttggagcaaaatgcttaagcggtggaaatacaatgcccaatcacatgcttcaattgaaaggctgaagtacgctgtagaccgcaagctttattgggatttcgaaattcaccttaacgttcgtaatgggttagaataatgactgaagaattcgaaattcaggacgcagcctgtccgccccgcaagcccatcgtcttgaacgctcccgctagcgtagacaaggcttgcattgcgcacgaagaagcttacaagaaagtcttcggcgtagttcctacaggctacacttacgacgtagattcgcgtatgatttacgtcggaagtgacgcaggtgtaagcctgaagcgtttgaaagaactgactcgcatgttgaattggcgggcgtaatggacaaattcgaacaggaaggttacgacgcattcgttgaagctttgtgcaacatgccaaagcacgcaatgccgtcgttttcgcacgctcacaatctgttgccgggcaactatctgcaaggctctgaagagcgtcaaggctgggttcgcggctggctgaaagccagggaggaagcatgagcaagagacagcgcaagaccgacgcgcgaattgccgcctcatgggatcggcacgacaccgacagcattagcaccgaaaggctgttcgcaatggtgtctgacgatacgggatgcgatacggatcgaatcatcgaagctatggttcgattgggccacttcaaaccggtagagccgaaatgagcaagcagcttccacgcatttggcttgaacattaccctaaatcgaagcgtagctattggcgggtgtcgccgcttcctggcaaatgggccagggttagcgacgaagtaaaagcccgctgggaagctgcgcacaagttcaaacaggcaatgaacgcaaagcgcaatgtctgcgaatgttgcggaaaggagttgtaatgccaaccgtaaagctgctaggcggaagccacaacaacaagaccgtcgaagacgatcctaagcaaaaggtgatcgtctacggcggcgaactgttcagcctgggcgacctggggccgaacggctggcgctatcatgtgggcaatgcccctgctggcgcatgtgatacagtcgccaagcccgccacgtctggatgggtcagcggtccggctgttaccggatggggcaatgggcgtggctgagcgcatcaacttcgaacgctacaaagacaaatcgaaatacacccgcgaaatcaatgccggaatggcggcaggctatgacggggccaaggttgacgacaatccgtatttcccgagggattcggaacaagcgcaggcttggcactacggctggaagggttcgcaaaacaagcttaacggttcagaaaagctttgcccgacgtgcttgcgttaggcaaagctttgtcgtaatctggctacgcaaacagcgaggcttatatgaacaagcgcaagcttgaaatcgtgctaagtcggttgcgcagggccagggacggttctaactggcaaggcaagttcactgccgaagtaaggcaggcgacaatggggcatcgtagggacgaaatagccgttccgcttgacgatgcgattaaattggtagaagctgagcttgatcgtattgagcgcaagcgaagcaaaaggcgatccgaaccgggtcgccttccgtatgtcgataactaggggaattgggatggccgacgaaattgacgtaacgaacgaacgggttgaaaacgaaactgcattgctggtggccgacgcagccaggaaagccgcaagcattcccaagggctatgcaggcgagtgctatttctgcggcgaagaaaaggcccgcgttgtgccggtgttcgttccgacaacacagcaggttgaagacgtgtgcggcggatgccgtgacaggcgggggctgccatgagcaatgttcgcagaattgacggcaacagtgttgacgcaatacaagcaggccataccgcagatagcgaaggcattgaaagcggcatggtcttgggatacgataaagacggtcgagtttgcgttataggattcggcggaacaaaagtagccgacggctttttcatggttgaagctttcaagcacaacgttttgacgggagcaaacgaatgaagctgttcgtaaacaccgaaaacctgggcgagattgacgaacaagacattgccgaagacgacgaccttaccgagtatgacgccgaacgaattttagccttagccgtaggccaaggttataccgattggcctggacgcaagtggaggcgcgtgcaatgaagatttccgaattgatggaacgcctaggcgaattgcagggcgagcatggcgatttggttgttgtcgcatttggcggcaatgaagaagtcggcgaagtcactgaagcaacgccagtcgcaaacaatgaaggcgaagcgccaacacaggtgcttttgctatgattacgccatcctcgctagcaaaatcggggacagaaagcggccatcaaagggccgttttctgttgggcggcaattgccattcatcacggcttcgacgtagccgataacttcgatgcgatgggcaaggaagcattcaaatattcgccgaagatcggcattcctgaattgaagtggcttcacgccgtacccaatggcggatcgcgcggcgatacggctgacagccgagccattcgcggcggacaaatgaaagccgaaggcgtaaaggttggcgttagcgacattttcttgccagtcaagcgcgggcagttctccgggctgtatatcgaaatgaagaagcctggaaacattcgcggtacgtctgccgagcaaaaggaattcggcgaattcgtcttgtcgcagggcttcgggttcatcgtatgcgattcctggcaaatggccgtccgcgtgattcgggagtatctagaacatggctgagtgcgtgcgatgcgaaattgcgcgagctaagttcagcgcaatcattcgttataacctgggcgatacccccgaccaaatcgtaagccgattgaacgataagccgacaggctatttcttcagcaggcaggacaacgggcgaattgtgatcgtaagatcgtcaacactggaacaatggcgagccaaggaaggaatcgacgtaatttctttctgaaagtgcttgacaaggccaaatgaccgtcgtaatgtgtgttcgtggctgacgtagctatatcgtaaagcaacgcgattcccattcatcgggcgcgtagggtagtagggtcgttccctaccgtcagccatttaattaagcccacaatggaaacggcaatgcaccgcatggtattcattgacgaaggattcgcctacgacgacattgaaagaatgtctagacttagcgaaaagctgaaggccgaaggctttcacgtaatcaacgcaattcatcccgaggataacgaaatgcacaattcccgcacccgtttgatgattactgctggccttgcggccctgggcaatctgttcatcgatgccgccgcgaacccaatgccttcgttcgctggccgctacggcaacaacccgaagagcctgaacgggtcgtatcgccagaacagcaacgcggccaagcagaaacgcgctgccgtcaagcgccgcaacatcgcaaagcacggccgctgatatgaaggtccgaaccgccgtcggcttggtaatcatcctggccgctgccctacttgtgggcatcaccaacaagcaggaagtcgattcgcaacgcgatcaatactgtgaaatggtgggcggcggttactggccggactaccaccattcatacaaggctgaatgtggcggtaaagacccgccaaagtttttgaaagaaaatcgctgaaatttgttgacttcgaaattcatgctgctatagtgaagcctcacaacgcagcacccacccagcgaggataaggcaatggcaaagagcaagttcgacctgtcggcgatcatcgccgcgacttccggcagcaatgccggtgccctggttcacaccagcgcaaagcagttttccaacccgaaggcttacgaaaaggcaatcgaagatggcctgatcgaagtcaatccgtccatgaccaatgcgaatggcgaagtcgccacccgcgcaactgaaaagggcatcgccagcatgaccgaatccaccaccgcaacccccgccgccgaaaagtctgccgcaccggccttcgaaatccaggacggcgcgaccctgaccccgattgatcgcggcaccggccttaccggcggcaccgagcgttacccgttcagcaagctgggcgttggtcagtcgttcttcgtcgctgcaaccgccgaaaacgccgacccggcgaagtcgatggcttccaccgtgtcgagcgcttcgaagcgttacgcgaccgaaaccggcgaaaccaagcagcgcggcgacaagaccgttccggttctggcctacgaacgcaagttcgaactgcgccgtcgtaccgccgagcaggaacaggccgacggcttcaagccgcaggctggcgtgcgcatctaccgcaccaagtaatcgcgcctggaacatgggcctgaaataacggccccaccgggtgaaagaccggattgaaagcccccgcaaatcgggggctttctttttgccgcagcaggcggtatgctggccctgccacggctcctgcctgtgccctggctctcctgtgatgggttggttgtggaaccccgcttagcgcacgctaggcggggtttttgctatgtgataagctccgcccatcttggggatcacgtttcagcgaatggacgaatcaaagatgaacgttgacccggcacaatttactgtcgtagtcgaacgtctaggcgaaatgcgcgaagacgcgaaagcaacaatgaaaagccttcacgcaatcgaactgactcttgccgagttcaagggcgttcctgggcagcttgaagcgctgaaatccaccgttgcacagcagggcgaagaattgacccagcacaaaacgttggttcgaatcatggccgcaattctgagcattagcgttggcctgatcggctggggctggaaggaatacagcgcagccaagcatttcgatatgcaaaccgaccgccgcctttacttgatcgaattcaagttaggcttgccgccaccttccgccgatggaaagcccgaatgaaaaaggtcgtcacgaaagtagttgcaccgaactggcgcgatgttgtaaagcgttggtcattctggctttcgactgctggaactgtcgtagtcagctgggcaatttccgcgccggaaactgtcttgcacgtttggcttatgatgcctgacgacctgaaagcagttctgccgccgaatttcgttaagcaattcggcatcggtcttttcattgcgtcgaatgtcgcaatgatcctgaagcagagcaggagcgagaaatgaagcacttcaaaattgcagagttttgcaagagcgcaacggcggatcgaatggggattaagatcgttcccaacgccgaagaaacgaaagcgcttgaagccctggttgcaaacgtgcttgaccctctgcgcgaaaagctgggaaagccggttaacgtaaccagcggccttcgccccaaaaaggtgaatattgccgtaggcggaaccggcacgtcgcagcacgtaaagggtgaagcggcagacattcaagtcaagggtatgaccccgattgaactgtgtcgtttcatcgttgccgctggcctgccgttcgatcaactgattgaagaaggcacctggacccatgtgagctttggcccgcgcaatcgtcgccaagtgctgacaatgcgcaacggcaaatacaccgaagggctgcggccgtgatcggcgcatggctgtcccgagtaggggctacagtgtgggcatggatcgttgcggccggggctgtagctgcgtcaatcctggggctgtatttcctggcaaaaggcaaaggtaaagccgaggctgaagtaaaggaagcaaagagcgaaacagaacgccaagccgaagacttcgcagttgaacgcgaagcaattgaaacccgaactgaaaccgtaaaggtggccgaaaatgtcgcgagtgaagttaatcgcattgctcctggcgatgctgctgagcgcttgcgcgatgaatggacgcgcgattaagtcggtagtaatcgataccgcttgtgattgggtatcgccgatttacataagcaaatccgacgttttgacagacggcaccgctcgacaaatccttacccataatgaaaagtggaaacggatttgcacaaagcctagcaattgaaccgaaggcccgctatagtccattgcgacgatagcgggctttcttttatgacttggcaaccggatcacgacattctgaagcgcttcgcccaagctcttttacgtaacgagcctgggatgaacggccgtttcaaggcggcttgcgaagtgacgccggacacaagtcatgccttgctgctcgcaaatcaattctacgaaaacgacattgttctaactgagattgaaaatatctctgagcgtgctaaagacgaagggcttgacgcactagggacaaaattcgatttcgcaaaagaagttttgagccgcgcgcgaagctgtaccgaagacactgacgcgcataagtttttcaaactgtattcggatattcgcggttggaccggaccgaaggaaaccaacgttaacattgatgcccgcaagcaaacggttatgatagtaaccgatatgggcactaatgacgaatgggccgacaaggccgcacgccaacaacgccaattgatgaatcaga

SEQ ID NO: 2 - DNA, 44570 bp, unidentified
  source 1..44570: mol_type = genomic DNA
gcttgcgagtaacatcgtcgtcgctaagacgattaactttgtcggtttcatcctttgcgcctttgatagtttcgacttcgtgtgcggcctgcgtttgggctgcttcgacacggcgcacggcttcgccgtcaatgcgcttaacttcggcttcggcgtgttcttgcttcgcgttcaattcgcctttgcgcttggcgttctgatagaatccgaagacaactaacgccgctgcgccgatggccgccagccatgcccacaattcagcccctttctttgccagccatgcgctaatcacggcttgcccgccgcgtcaataagcacgtcggccacggccttggccgcaagccacttgcgagcgtcgtacgacgcaagatcgtttgcgcttgtgatgaacagcacttcaacgatgatgccgccggactggacaaatgccaaccggctgtgctggcccgatgcttcgggctttgcaccacgattacggatcaccagcgcgtcagaaatcgcctgcgcgatacgaccgcctaacgccatgtctttcggccctgacagcgtttcaacgccggttgcagtggccgggcctgcattgcagtggaattcaaccgcaatcggatggcgctttgcagcggccgcagcttgacgcaacggcaggttttgtgtaccgcttccatccagttcgtgcggaacgtttgcccgttgcaaatagaacgaaaccatgttacggaattcaaccgcaatgtcagcttctttgcggccgaaggctactgcgccgggatcgtcgttgctgtgaccggctgaaacgtaaatgcttttcattgcggcttcttcctttggcggatgaacgtggcggcttggcccgcgatcaacagtcccaaaccaaaccacttgacaaaatcaggcggaagcgctgcctttaaatccatcggcattgcaacccaaacctgtaacgccacgtcaggaaccgcgacagcaaagccggtaatcagcgtgccgattacgccgagtcgaacggaccaacgtttcttgacttcgcgccagttcggcacgacaaccttttcaacggtctgtttcatttcgatgatccttcgacgggtgcggctggcaagcctaacttgaattcaatcaaataaaggcggcggtcggcgtcttggtcgcgagcatagaagcctttagcttccgtccagccccaaccaatcaagccgacgcacagcgccaaaaccgtcccgcaaatctttatgactaatgaatgatttgcaattgtcttggcttgcgattcgacttggatgcgcaatgcggccatttcagcggggacttgttcaatgcgagcaagggagagttgaatgtttcccaattggccgcgcatttctttagagtccgtcaacaagttgttcacccggtcaatcaacacggcgaattgttgcgggtcaacattcatgtcgttttcgctcactttgcctgttccggtggccccaattcccggcactatacacgcgcacagggcgcaggcaaagaaaaaccccggccgaagccggggtttcctgtcagcggggcgcagcgcgcggctgcggccggcttacgcggtgcgccagacgcgtgcgccgccttcgacggcacgaacgacgaacttgcgggtttccttgatggccggaacggtgttgcccttgcgatcaacgcgggtttcgccggggatttcttcggcataacgacgggttgcgctggaaacggtggaagccagcgacttggcaacgttcggcttgtcgtcgctgttcggaacgaagaacgactggccgacttgcagcaggtcgaacgggtaggtttcgccgccacgaccgcgaccggtcacgggggccagtgcgatgccgtcttcgatctggaaggacggctttgcggccggggtgctggccggagcggcctgctgggtgttctgcgctgcgttcatgctttcgatgcccttggtggtggcgcgggttgccagttcacccgcttcattggtcatggactcgttgacttcgacaagcccatcttcaagcgcgctggcgtgcgcttcgcgggaagtatacacgaaactaccggcgttggtagcggcgataacggcggacaggtcgaaagatgcggtcttcgacttcggggcgggcttacgggccatgttcgtttctcctagctaggtgagttctgcggaatgcaggatttgaatactacaggtttcggcaggcgtgtcaacaactatttcgttaaatcttcgtggaactttggcgggttcttaccgccgcattcaagcttgtaacggccgggttcatagtccggccaaacgccgtcacgaacattgttgcaataacgctgctgttcaagttcggcgtcttgcttatccatgatccccacaacaatgaatgccgtgaggatcgcgattagtccgacagcctgccggaccttcacgcgcgcttactcgacttggcccgcacgttgcgacgcttcttcgctgcgcgcttttgtgctgcggcattgctgttcagaagatgcgagccgttcaggctgcgcgggttgttgccgtagcgctgggaaaacgacgacagcatgttgctgttggcaactgcaacgtcggtgagtgcggcggcacctgcgccaaggccaccggccagtgcagacagggcggaaacaagaacattgcgacgattgtgcatgacactttcctctgttttgtaatcgatgatttcaatttcgccgttaagctttcttctaacggcgtccagtgctgcgacgttgattgtactttcgtcgcctattaaaagcaacttcattcgcggccccacttaaattcgttgtcgcggcgatggcctgcgcgctgcggcggttcacggtaagaattgcggcgcatatcagcaacgtggcgttcgtagttcaaacgggcttgcacgtcatcggtacgcgccttgttacgaatcaggcgcacagcgttggcgatagcaagtgctgcaataatccaaaacagtgcggccatgatcctttctccttagtaatcgtagcgcgaacgttcgtattcttcgcgctgtttagaaagcgcttcccaaattgcgtcgtaagtatcctgccatttatctagcttgtcaagcttggattcaagccaattcaaccggctttcgttctttacgttatgaagcgtaacgtcttccaagccttccgacatgataccgacagaacggtctgactcggttacgctcccgcgagctatgcaaggaatgccaagagtcttgatttcgacttcaaatgacattacggcgtcccttcgtcttagtgtgggaatagaatacgacgctgtttttcgcttgtcaactacttttcgtcagaaaaaccaaatctcaattgcgggtgcgattgggttgtcgttacgacgatagactgcggccccgtgttcattgcgcctaacgaaatattcaccttcgtagcggccgctaaggtctacggccagtgcttccgggctaaggcccatattgaaatagaagatagcgcgaatcttagcccgcgctatctcacaacgtacgcacttcatttgtcccatcccggtatgatcttgttgggatcgccgcccgctgctttgaatccgcgcgtgtacgatgcggccatgcgtgcgtccatagttccgccgcagttgcaacaatccaccttcaaccctaaatggccgcttatgttcaacggccaagttggaaaatgatgctgcttgcatccgtcaagcaacgcttgatttgcgcggatttcttcaagcatgacctttggatcaatgttcattgccatgatagatactcctgcaagaccttaactgcatcttcccagttgtcgcacacgatccagccgaagccttgcgccttgacaaactcgccgaattccttttgctctttcgacgtggttttgatcttgccgggcttcttcatttcaatgtaaaggccgctgtattcgccgcgcttcactggcaaaaacaaatcagctacgccaacctttacgccttcggccttcaacgcattaccgcgaatggcgcgcgtcttttcgtcgtcgcctcgcgcaccgccgttcggtatgtgatgcagccaacgtagctcaggccattgcgtaatgtgcaacgccgcccatgcgaaaacggcccgctggtggccgctttcggttccgcttttagctaggtcagcgggcttcattgtgcttcgcccgcttttcagcgtcctgcttgcgcttcaattcgacgcgcatttcgtgcaactgcctttgcagttccggcagcttatcgcgttgcttggctcgctgcaactgaacaacgcgaacattcaatgcgttgacacaagacgccaattcgttgcaggtcatgcctgcccattccttgccgttcattccaagccccttttatcgcggcacccgccgcaacattcttcgcctacggactcgacgtaaacaacacgggcgaaatgctccccacaatagaagcaatcgcccggctgtccagtcgggatagcggcggccttacgtgaaacgtctgcaaccaacaatgcggtttcattttcaacgcggtcattggttacgtcgatttcgtcagccacggtaattcccctgttcgttattgatgttagtgagtgttgccgcgcggcttgcggttctgcaacgtggcaagcaagtcggcgaattcttcggccgaaccaacttccacgatgcgaacttcaaggccattcgccgacacgccctgttcggtggtgtccggggcttcctgcttgacgaagcgcgaaaggcggtcatacaccttttgttcttcggcgtcaagtgacatggccttgcccttgatcttttcgatcaactggaatgcttcgaccaatgcggcggtcgtttccagcacttgcgactgaacatcgaccatcatttcacgattcttacatgcgatgcacatggctaatcatccttatacggtagtcgctgcggtgttgcagcgtgtctatgatgcggccttcgattgcgcttgtcaagcgctttttgaaccaaaccgataacttcttcaatcggtttggctatttcttcaatgcgatgcgtcacggttgcctgcctaatttcggccgtgaacttcccttgccagttcgatgcgtcgcgcgcactgcgcagcctgttcaacgcgcgttctagttcggacttgcgcatagcattcactcctaaagcccggccattgctgaccgggcttcgttaattagttcggatcgctacgatctaccgaaatcccgtgcatcattccaacgcacaagtctacgtaatcgtctttccctgctgtgtaattgcctttcagccatcctgcgttcagaccgttggcggtttcgccagctacagacctgcacacttcgcgcagcaggatcgttttagaaccgtcggtttctttcattgctacgaaatgcgtaccgtctccgtatgcgccttcgtagaagtattcgacgttaacgttcttcatttgctgtactcggttagttccttgctggaacaactatagaatacgataaagctctacgacagtcaagactatttttctgaacggttaatcttgcttgggttcgtccaacgcttcgacttcgtgactaacgcctgacgctgacaccgcttcttcaagcgatatgacgcccttttcaaccaacagttcagccaaacgaccgaacgcttcggcagtcttttgcgtcaagcgttccatactttcagagcggccgtcacattcatatgcgtcaatatacggcgtcaaagcatacgacaagaacgtttcgcgtgtgccatgccaagttttaactttaactttcattgcaaggttccttccaatgtctaatgcttttgaaataggcgattactttgcggcattcggggcaagtgattgtctcgccgggactcgcaaaccttgttggttcgtcaacgtctcccgaatcaaaagcgtcaaatgcaataccgcaaatcgtaaattctccaccctgcgacgggtcgcttccatgtcgcattgttcaatcctcgctaatggtgaatacggaccgcttgccacacgtcttgttcttacgctcaaacttttcacagcgaaccttacgcgtttcgtcgtcggtacgaagatcaagcgtcgtatacgatttgaagaagcggctaagacgttgcttgaaagtttgcatggcatcgttcctttgctgttgggcggtcaacggccgggaacgacccggctaccctacgtgcccatttaagggtgtcacgttgctttacgatatagctacgctgaccatgtgcaaagaatacgacgcctgacacgacatgtcaagcgttcattcaatccgatttataaatacgttcagttatcccgtattgctttctccacccattcaatcgggttatgcaaatcgttaacgtccttgttcaacgtttcaagacgttgggctatgcgccaaagcaagccgcaaacaccccataacaacagaacgatcattgccagcagtgcaacaattaaatacgtcacggtagcttactccctgcgtgatggcgaacgccaagctgcttgtttgcgcccagttcgtacagttcaatgcttgcaacgttgccgtttacgtcatacagattcagttcaacaacctgtgctgtgcccacaattgggccgttcttgccattgagcgggccgccgactaggaagcaatcgacggtcggcacgccgttcttgtcgtacgtcgtttcggctggatagcgcttgccaaactcgcgcactgcgacggattcaacgacaggttcgctagtccatccgtcatccgttacggtgacaggttctttgaacttagtggtgacaactacaccacttgaccaaccgcttgcgtcgcctacttcgctaattggccccttggcccatgtatcgggcttgtcaggttgcggcaatggcacgtcgtcatcaatgcgaatggtcattacgccctcgctatgcggaagcctaaacgcgcttcgccgggttcaacggttgtttcaatcttgccgttggtcagcatttcatgcggcccaacttcggcaaggtacttcaacgttgtttcgcggtcttcatgttccgcatacatttcaacgttgatttcaatgaacagcgccttatcaggaatggcgttgttcaacagttcaagcaactgtgctttgttcatcgtcaatactcctagctgaaagttccttgccgcagtgcgagcataccacacgtttggcgttcatcgcttctttgaacttgtgtgccttgttccaacgctcctttacttcttcgcttacgcgattccatttgccgggcagcggcgaaacgcgccaatagctacgcttcgacttcgggtagtgctgcaaccaaatacgcggcttgttcatggcatgtactcctgcggcgcatcgtcatcgccagaattcggcaacttattgtaaatgcttgcgggcacaccttcaatggtgtcttcggtgtaaacgcggcggtattgatcgccagcgcgaacgcccatcgctttaacccatgcgcggcctttgtcggcatgaccatacttcgcagggtacgcccgttcggccatgtgttcgcgccagtctgcccgatcaatgcgactaaccatgcgatggcgatttgacgtgcgtgcgtaacctttggctttcaattgctccaaagtgtacggaaatttgttagccatcatccagccctcaattcaagctgacgggtcatttccttcaagcgcataagcgatacgccgccgctgttgccaatgcggatgaacttcgttgccttgtcatacgtgaagttgtccggggtgatcccaaacactttcttgtatgcctcgctgtatgctttgaatgcagcgtgaacgctgtccgggcacttgcgcgctttctttacgcgcggtgctttgatgtgtgagtcaattttatacatgacgattcgccttattcagttcaatcataaacttaccatagattgcctgctcgcgcttatcgcatacgctaacgattcgcctgaatgactcttccgtaaaacaccaatgaccgttgcgaaggcgaagacgtggcttgtttcccttacgccatgcgcggccaagcatctgcggcatgaatggaaactctttacgattgagtccatcaagcgcacctttaaaaccacccggtggcggtgcgacaatgattgtggcctttccgatagctggatcgtcaaagccttcggtcaaatcagccatgttagttccccttgatgggataggtaacaacgcactgaccggcttcaaacgcatttcggcactgttcgcccaaaacacgacgttctgctgcgtcatcgtggttcatgatgtaacacgcaatcatcgggcttttaaacacaaggtcgtaatctgcataaacaataacgcgaactttcatttcgcttgctcctgttggatggcctatcttacggatatacggcgacgattgcaatagccagtacggcgaaatacaacgctttgaattcttctttacgtcgccatgcaagaatcgaacgaatcaatacgacgattgcgacggcttgcagcatgtaatagagcgtcattgcgcatgtccctgtgatgcccacattgggcggttattcgcggcgggcgacttcaaagcagttgttcggcgcgtcgtgcttgatgaccctgaatttgcccggtcctttcttgttgcgtcggctaactgccatgcgaatttgcgactcgcttacgacgctaaacggtacaacaaacgacttgcctacgtcaagcgaatcaaacgggtattcgatgcggccttgcttcttatcgtcttccttggcttgcggcgatgaatcgacaattgcaaacgtcacgggtctgtctcctgctgttagtgagttataacaacataacgttatcaccgttataacgatatgtcaagcataacagggtcattcactcggtataagggtctgtatagtagctaagtagttgaaatcattgaaaatataataaatataataaatataataaaataagatcgtattgtaatgtaacggacctaacgtataacgatgtaacggaatcacgtataacacaggggtggtatggggtagaccattatatttgttatatccattcaactgactgattttgctagggttttgcgttatacttgcgttatatcccgttataccgtattcacacaacgtaaggttcagcgtatgacatgtgcaaaacaggtggttgaagctacgatcatcgcaacggatggaacaacgtatgtcggtcgtaacgactgtgcgaatccgcaggctgtctgtccccgtggttcgatgccgtctaatgtgggctaccacctgtgccggtcggtgtgtcgtcaggcggggcacgcggaagtgatggcgattgaagcggctggcgaacacgcggaaggcgctacgttgatcctgcgcggccatgttgcggtgtgtcctgagtgcatgaaagcatgtaacgccgcaggtattgcacgcattgaagttgtgtagtagggtacaacttccaaccgaaggagcgcgcaatgtacctcgcacttaacatcgcagtggtggtattggttttgtacgccgcacactggacaacgctggccctgtcaactgatccaaaagaaaagccccgctaaatgcggggcttcttcgttacaggccaaaggttttcggtacgtttatcatgtaagcgactgctgacgttttgtattggttgtgcatgttagcgcgtgatacctcgctaatgtcaccacgttcaactaacgtcttcaatgcccgtttgattgcgtagcttgatcccatcttgtctttgcggtagatggcaacggatgcaagtttgcgttgaaggaaggcgtagggtatgacgcgttccgaatgaaggttgcccatgttcggaatgtacttttcaacttcactgaacggtgcagttacatacgtcttgattgtgttgatgatgttttgaagctgcttcgtttcgtcgttgtcaataccgatttcgccagcgtcgaacttagcgagcaagttgcgaacgtctgcaactacgaagttgattgcccatgtcgcatgttcgctgttaatcgtcgggtgatatggatcgcagcccacagcaatcaatgcggccagcttcattgccttgacgtgtgcgcggttccaaaggtggcggcgaacttcgcggtctgcgccgttgatgttgtcgtcggcgtgttggttcaactgcttcaacaatgcttgtgcgtcttcgtcaacctgtacgtgaatcgctttgttctgcgaattcaattgcagcgagaacgcgcacagttcgcccaactgttgaatcaactggaatgacggccgggccaacatgtgtgcttcgttcaacggcggacgcgggccagtgtattcaatcatcgaaaagcgcggcaacaggcccgacgcaatcatgccttcattcaacacgttgtagaacgtttcggccgtcgattcgccaagcatggtgaaagcaggcgcgagcaatgcggttgtgttcttttctttgtcgctgtagatcgtcggacgcagaacgttgccttcgccagacttgttgaacagttcaagatacgaacgaagcagactgaccaaatgcgggggcgcattctcgttgcacatttgtttgaagtacaaaccgaactcgccaacgattgacacgaagctaggcgacgaccggccaaggtgcttaatcaacgccggggctgaactcacttcggccgggcctacgaagtcagttgcggcaggaacaccgcgttgtacttcggtcatcaacttgtcaatgcctcgcgcaatagcttccttacccgatccggttggagcgagcaacagaatgtattgattcaatccggttccgctaatgttgtagctgcggccaatgattccactgaccaaaccgattgcgccagccaatgcaatttctgcaacctgacgcggcgcttgtgcgtagataaactgcgcaatttcgccaaccaatccgggcggcggactgtatacggatcggctggggttcaaaggtgcgacagggaccggtgcaggttccagcgtgggcgcgttccctgtcaccggctcctgtcgctttgcttcaatagcttcgttcaacatgttgcgcagtccatcaatgtcaaccggcggcaacatcctgtcgaagcaacgatcaagcatgtaattaatacgatactgcgcgcgtgacttttcacgctggcccagtgccgaacgcaagaacaggttttgaacctgaaagcggttttcgctatagaacgcaagaatgtcaacaagggcaaagtccgcttcggattgcgaagggtaatacttttgccaattgccgtcataaaacaaatcgctgaacttttctgcgttggctgcgcggccagccatttctagcacttcttcgtcgcgcaacttcgcctgttcaagcccagcgtaaaacattgctgcgcccttgccttcggacatttgcccgtgcaagacctgcaacatttgattgtgttcgttgatcggtgcgttgcggtaaacattgccggtcatcgtcatgtatcgctgcgacgaatagacttcaatgtaactacggcgacggccggaaggcaccttgccctttacgatgatgtgcagacccgcgccagacggcgacagttccgcatagctatcaaattcattgaacactttgatctgacgatcaagcgattgttgatcgcctttcgtgtcgtcaagatcgataaaggtatacgggtcgttgtcggtcagaacgaagccaatgcctgcgtaccaactcgtttccattgcggcaactgcatcatcaaagcttccccaagttgcgggatcgcttacggatgccatgcggtttgaagctggtgaatacggaaccttagtcggtttgtctgcgtcgcggtcttcgtaccgccaaacaacccactgcttataggtccgcatttcgttagggatattcccaaacatgcggccttattccttcggttcggtggtctgctgacgcatgaaatcgcggactcgcatcacgcgattaaacgacgggtcatcgatcttgccgcgcgcaaagtgcgacagccaaccgacgctaacgttcgcaccatcggcgacagcttcaagggtgagagtacgcggccgattcgccaacaacttcaacgtttcggttagttcgggatgcgtcgcaacatcaagcgaagtcatgcggtgacaccttgtttatatgggccgaagttcggcaagatggcgcacatgatgacccgcaaaataattcgcgtcaagcgcaaaatttgcttgacagccgtgacggccgtgtctagcctatgcttccacactggcccgtcgccaagcggtcaaggcaccgggttttgatcccggcatcgtaggttcgattcctaccgggccagccagtcaaatcaacgcaaggaacgtcgcatgtcgaacgcaccgattcacccggccggatcatccgaagcattcaactacattgcggaagcgaacgttaccgcatcgaacaactatcacggccacgctgtttcgcatcacgaagcgttcggcatcatcacaagttcggtgatggcgttgaaccaactggacaagttgaaaaaggcactgttttacggccgcaaccttgaagacttttccaccggcaacgaagttcgcgcgagcatggcgacgtggcctgaaatcattcagcaaggcaacccgaacaaaggcgaattccttttgcacgccattgtgggcatcgctactgaatccggtgaactgcttgaagcgctgttgaagtcagttgaccgggctgacccgaaagagtttgacgaagtgaacttcgttgaagaacttggcgacgttctttggtacgttgcgattggccttggcgcaattggcgtatcgtttgaagaagtgcagcgccgcaacattgccaagctgcggcatcgcttcccgcaaaagttcaccgagtacgacgccaacaatcgtgacctgttcggcgaacgcaagattcttgaaatgcacggcgcaggtacaccggaaggctaccgaatgccgctgactgacggcgaagggcatgttatcgaagttacttcgccgaacggatacgtcaagattggcccggatgacatgcgcgaagcttggtcatgcaagattggcaacacgaacggggtaaacattcccaacggcgccgatttgccaatgcgtgaagctgtgcgcgaagcttacgcgcgtatcactggcgaacagcccgaagcaatctttagcggctggggcgcaacgttcaccgaaccggagcgggcagtaattgaaaaccgtttgccggtagttgacaagccgaaataagcgtgttttaattgcgcaacggtcgaacaacggccgttgcaacccaacccaaacaggtgatcgcatggacaacggatggactcaaacgcccccggccgcactggtcaaaggcaccccggaatggctggccgaacgtgaccgcatccttgcggcatgggaacagtcgaaaaaggatcttgacaaggcgaaagaagacgaaatgaatctgcgtaagcagttcgttgttttctctttcgacaatgaaaagttgtcaggaaccgaacgcatccagttgaacaacggctatgaagcaaaggccgttaagaagctgaacttcaagttcgtttcgcgtgacgaaaacgtcaaggttgttgacgcagttgacgcagcgcttacgcagattgaagcgcttggccccgaagcaacgttcatgggggatcgtcttgttaagtggtcggctgacctgtcgttgaccgaatacaaggcgttgactgaaacggaaatcggccgcaaggtcaagtcgatcattgacggcgttattgaaacgaccgaaggtgcgccgacgctggaaatcatcgaaccgaagtcgaagaagtaaaaatgattctaattttgttgatcgctgcggtgctgtttgccttggggcgttttgttgccgaacgctttgacaaggcccagccaatcgcagcccaaaacgccggggcacgcgtgcccacatggaccgagcgatgtagaacgccgggtttcaagggcaaattaagcgcgtatgccttaacttgaaatctggcgaccgttcacaatcaggccgcgatgccgtcgcttaacggcggcatcgcatttaatctttagaatgagttcgttaggatttattctaaagactaaaggggcacagcatgaacgcacgaattccaagcaagccgggcaactactattggtcggaatggaaatgcgttgttgaagtcaagcagcgcgggcagcagctttacgtaacaccgccgaatggcgttgaagtcaagatcacggccaaaattgcaggccgcttcgtggagcaatcataatgcaaatgaaagacttgaagcccgcatcaagcttcgcaaagaactacggcttcaaagcgctggcctacggtccgcccggcgaaggcaaaacgccgttgattatgaccgccccccggcccgtaatgctggtgtgtgaacccggcatgttgtcgatgcgcaacgcacacaacgtcgccgcatgggaaggcgacacgccggagcgctgcgccgaattctttacgtggttaaattcttcgcacgaagctaagaacttcgatactgcgtgtgtcgatagcttttcgcaatacgccgaaatcgtgttgaagcgcgcgcttgaaaagaatacgcacgggcttaaagcttacggcgtcatggctgaaacggtcaatgaaacggcgcacaaactctattacatgcgcgaaaagcacatgtatttgatttgcaaagaaaccgtcattgacgaaggcggaatgaagaagcgcaaaccttatttccccggtcaagacctgaacgtaaagatgccgcatcttttcgattcaatcttgcatgtcgcaagggcacagattcccggcatcatcaaaccgacgcttgcaattcgcacgttcggtacttccgacattatggctcgcattcgcacaagcaatcccggtttgtttaacgaactggaaccgccggatttgacggcgttgattgccaaggtgatgcagaactaagacacgccccgttggcgaaattggtagacgcaccggacttaaaatccgttgccgcaaggcatgtcggttcgattccgacacggggcaccaaaacggcaaagctttcggccgtattaaacgaaggcacactttgcaaaggtgacgaaaatggtacagcttttgaacggtttcaacccgttggattacgacccggcacagggcggcggtacttggccgctcggcaagcacccggttgtgatcgaatcggccgaagtaaaagcgacgcaggacaacagcagcggctatctgcaactgaactgcgttatcactgagggtccgtccgccggattcaagggcgcgtatcgcctgaatctctacaatcagtcggcgaaggctgctgaaatcgcacacaagcaactgtcggcgatttgccacgtcttgcaggtgttcgcactgccgaacaacggcacggacattaccccgctgtttggtcgcccgtttgttgtcgaagtcggctatcaaaagggtgaagaacccagcccgaccaacccggacgcgaagggctacaccgaagtcaagcgcgtgtttgacatgaacggcaacgaaccgaaaaagggcggttcggtcgatcagcagccgcaaggcttcggcggtcagcagcagaacggcggcttcaatcagcagcagccgcagcagcaagcaccgcaacagcagccccagcagggcggcgcgggtgcatggggtgcaggtggtcagggcggtggcgcaccgcagggccagcagcagccgcaggccgggggttggggccagcagggccagcagggccagcagccccagcagcagccgccgcagcagaacccccagcagcaggcaccgcagggtggcggctggcagcagggccagcagcagggcaacggcggtgcgccgcagcagccgtcctggggtcagcgctaagagcgtcgcagtaaacaacgtgtgaccaatacggccgggtgaaaatccggccgtatttctaacaggggaaagccgcatgtcagaccgggttaaaaacccattaccaataccggaacaatgcgacaactgcgcgtcgtttgatattgcgtttgttgggaacgaagcgctatacggtagacctttcggcgactggccgttttgctatttctgttcaggatgcggcgcagcagttggatgccatccgaacacacgcattccacttggccggatggctgacaagaaaacacggcaactgcgtgcggaagcgcataggcattttgacccgctttggaaatccggcggaatgtcaagaaccgacgcgtatcagatgctcgcaaggcatctgaacataccgcatgaaaaatgtcacatatcgcaaatgaacgtcgaacagttgcaatatgtgatcgaacaatgcaaaggcttggaattcgacaacaccgccaaagtggttcaacgccggaaggacaaaaaagatgcaaaacgaaataaacgggctgaacgagaaaagcgaaaccgctaccacaacggaaagcggatcgaaggtccaaaccctttctttagacgcgcccggcgtggcgaacaaaattgcagcgagggttttgaaggagattgatgcgtattgcgtgcaaacgtatgacggcggccaccgaacgcatttaggcgcttcgttgatcggtcgtaactgcaaacgttacctttggtacgttttccgctggtgtctacgcgccgcgacagacggacgcaagcaacgcctgttcaatcgtgggcatcgtgaagaagcccgcttcgttgaatggcttgaaggtatcggcatcaaagtttggtttgaaaaccgcgaaggcttttactaccacgcagaaagcgacgcgtacggtatcgcagttgatggcgaaatgccggatgcgctttgcacaccgatactcgaaagcaaccccgaatatttgcgtcacgttgcccgtgcaaaagctgacgggttggaatttccgcaataccgtattagcgacgtaaacggccacttcggcggatcgctcgacggcattgccgtcttgccgccgcactggggtattgacgaaccggtattgcttgaattcaaaacgcacggaaccggacacaagtttgtcaagttgaaagaaaacaagatgcctgttgaaaagcaagagcattttgcgcaaacttcaacgtacggcttgaagtacgggtttcgctacgtcttgtatttttccatatgcaagaacgatgacgatttgcatgttgaagttgcaaagctagatcatgcgacaggccaacaaatgattttaaaggctgaaagcataatcaattcgcagactccgccgccaaagctttcggaaagcccaacgtatagcgaatgcggatattgcgacatgcgcagcatttgccacggtggcgaacctgttgaacgcaactgccgaagctgcattcacgcaacgccaatcgaaaacgcgcaatggcactgtgcggtgcatagcccgacgaatggcccgataccgaagcaagtaattccaaccggatgccctgattacaaggctattgtgtaatgtttgaaaatagttcgatgattgcgccagttgattttgaggcgcgttggtatcaagccgaagcggagcaatcaattttcgactatttcgaccgtggcggccggggaaacccggtcgttgccatgcccacgggtacgggcaaaagcgtcgtaatcgcgaacttccttcgcagggtttatcgatactggcccggtcagcgcattatgatgctgacgcacgttaaagagttgatcgaacagaacgcaaagaaagtgatgcaggtttggccgactgcaccactgggtatttatagcgccggattgaagcgtcgcgatttgatgttgccacttacgttcggcggtgtcgctagcgtcaagaatgtcattcgccagtttggccgcatcgatctgctgttgattgacgaatgccatttgctttcgccgaacgatgacacgatgtatcaggtaatcattgccgaactgttggcgatgaatccttttatgaaagtcattggcttcactgcaacgccgttccgaatgaagcagggcatgattacggacggtggcattttcaccgacatttgctatgacattaccgattacgaatcattcaatcgtttggttgcggaaggctttatttcgccgctaattccaaagcgaactaacattgaaattgacgtgtcgaacgtcggtctttctggcggagatttcaatcgcaaggcgcttaacgaagttagcgacaaggacgaaatcacatgggcggcttgcaaagaaatggcggagctaggctataaccgcgcttcgtggttgaccttcgcaaacagcgttgaacacgccgaacatgttgccgcgatgctgcaaagcttcggcattacagcggtcgcaagccatagcaaactgcccggcaacgaaaacgataagcgtgttgaagcattcaagcgtggcgaaattcgctgcttggtcaacatgggtaagtatacaaccggcttcgatcatcccccgattgatttaattagcatgttgcgcgccacggcatcgcccggtttatgggtgcagatgcttggccgtggtacgcgtccgttcggcggcgatggcttcttccctcaaaaggacaactgcctagttttagacttcgcgggcaatacgcgtaggcttggccctatcaatgacccggtgattccgcgcaagccgggtcagggcggcggtgacgccccggttcgcatttgcgaaaactgcggtgcatacaaccacacgaaggttaggttttgctgcaactgcggaacagaatttacgttcaataccaagcttgttagaagcgccgcaacgcaagaagtaatgaagtcggatgcaccgcaggttgaatatttcaacgttagccgtgtgctttacaacctgcatgaaaagcgcggcgcggctggcgaattgctgtcgccgccttcgatcaaagtttcgtacatttgcggtctgcacatgtttaacgaatggattttgcttgaacactcgggaatggcaggaaagcgggcgcgggactggtggcggcaacgaatgggaacggaaccaccgccgtcaacgtacgaagctttgttgtccgtccataagtcgcgcgtaccttcaaagattcgcgttcatgtcaataaaaaatacccggagattttaggccatgagttttaaggacgtgatgaacagcaagttgcgcaatgacgatgaaaacgaacttgtcatagcaattcaagacggtgcagtaaaggcccaccgctggatgacttgcgttaactgtttgcattggcatcgcaataacacaagcgcaggcgaagaaggttgcgataaatttgcagctatgccgccaccgcatattatcgttagcggctgcaaagaccatgagtttgatattccgttctgaggctaaagccatgaataacatttgctggtgcaattcctgctatgctcgccgcttcaatgatgacgacagccgcaagtttgacgactgcgaaattcagcaggctttagatacagcgtacgaagaaaacgaaaagctgcgtgtgcagcttgaagaagaacgtatgtggaatcaacacgggaatcaaagcaatggctaagaccgcaggcgcgcgacgcgcacgcaagcccaaagatgccgccaatggcgcggcgtctttaattgaggcgttaaagttcattgcattggcgcagcaaaaggaaggcacgccagtgcaaacgcattgcgtcgttagcagcgggcgagctatggcgttcaacggcatattcgcaaccgggcatttagtcgaggatgatttatcggcgtgcccacatacgattaggctgcttgacgcgttaggcaagtgcggcgaaaccctgtcgattacgcagcttgatagcggccgactttccattaagtcaggtgcgttcaaagcattcattcagtgcataccgttcggcgaagtgccgatgattgaacccgattcaccgtgcgcaacgattgatgatcgtttgaaagcagggttcgatttaatcgcgccgttgttgaacgaaaccgcaccgcgtccgatctttgcaagcgcgctgctgcaaagcgggtccattgtgggcacaaacggtcacgttctgatagagcattggcacggcatcgatttgccgcccggtttgcttattccgaaggcgtcattgcaagctgtgacgaagacggctaagaagcttgcgcgttttggtttctcgcaaaactcggcaacattcttctttgaagacgacagctttattaagacgcagctttattcggaagcttacccggactatgccgcactgtttccgcagcaggtcaacccttggccgcttccgcaaggcttctttgacggtatccgcaagattcagtctttgtcggatgacaaaatcgcgtatttcgatgaaagtggattttcggtaaaggacgcgcaaaagaaccaagcaggttcgtttgaaatcgaaggtttgcacaaaggtcttgcgtttaacatggattacttgtctatcgttgaaccgattttcaagcaagttgattttgaaaccgaaccgggcaaagcggtgttctttggcgataattcgcgcggtatgctaatgggggttcgttcgtaatgttcttcgacagcgaggaatttacacgtcgtatggctaaaggcaaatccaaagggattgaccttagcacgcttgcccggccgacattaacccttcgcccattcgttgaattcactggcgaagaattggcgcgtatgcctgtcggctcgccaatgatctacgacgttgaatgttacccgaacttcttttgcgtatcgttcaagtgccctgaaactggcaaggttgtttattttgagcgttcgccgcgttctgattttgacggcgaagaactgcgatggatgatgtttaagttttgcacggttggtttcaacaatcttgcatacgacgtgaacatggtttttgccgcagcacagggcttcgattgcgcaaagcttaaagcgctttccaacgcaatgatcggcgatggcatgtggccgcgcgaagcacaaaaagaattcggtttccgcgtaccgtttgacttactaaaccaaattgatttgatcgaagtggccccgcttgaagggtcgctaaagctgtacgccgcacgtatgcaggccgcaaggctgcaagatttaccatttgaacacacccggcaccttgacgaagaagaagccgatattgtcaagtattacaatatcaacgatgacgacaacaccattcttttgtataaggaactgttgccagaaatcaagcttcgcgaaactctaggcaaggaatacaaccaagaccttcgcagccgttccgatgcgcagattgcagaagccgtaattgcaagcgagctaaccaagcttaccggtaagtatccgtcaaagcctaagactaacgttttaaacgtaaagtacgaagcgccgcactggattggctacgtgtcgccagaattgcgaagcatcgttgaccggatcgaagcggccacattcccgcttgacggcaacggttcgcctatgtggccggaagggctgggcgaaaaagaaaagacgaaaagcggatacacttgggtattaaaagcccgcatcggccagtcagtttataagcttggcatgggcggcctgcattcgtccgaacagaacgttgcacacgtagcgacggctgacacgttgctaattgatcgtgacgttgcaagctactacccgcgaattatcctaaacgaacgtctttaccctaagcacttaggcgaagcgttcttgcaggtttacgaagcgctagttaacaagcgtctggccgctaaaaaggcaggcaacaagacaattgccaacgcattgaagatcaccattaacggtggtttcggcaagttcggcaacctgtattcattgctgtattcgcccaagctgcttttgcaagtaaccattaccgggcagcttgcactgttaatgctaattgaaatgatccagcaccacggcatacccgtcgtgtccggcaatacagacggcatcgtaattaaatgcccggttgaccgctacgacgaacttaacgcgatcattgcaatgtgggaacagattacaggatttgaaacggaagaaacccgctacaaagctttgtattgccgtgacgttaacaactattttgcagtaaaggaaaaaggcgacgaaggcgctaagttgctgtcggataggctgggcgtaaaaatcaaaggatcgtatgccgaagtaggcagcgcgcttaacagcgtgttgtctaagaacgccgaacatttgatttgcagcgacgcagttgttcatgcaataactagcggcaagcctgtgcgcgaaacaatcgaagcctgccgcgatattcgcagatttactacggtgcgcaaggttaacggcggcgcagaaaaagacggcgtttttatcggcaagattattcgttggtattacgcgcaggacattaacgggcaaattcgttacattgccactggcaacgccgttccaaaaagtgagggggctaaacccttgatggatttgccccctaagtttccttcggatattgattacaattggtacgtagatcaagccgaagacactttagaaaagatcggctttaagccaaagaaacaacaaccgctgttcttttaaggaacagcggtccaagtcccggccatgttcctgtattcgataccgtccgcaatgttgtacgcaacgatgtaaggcggtggcaggatgaacacccacaagccgacccccgtacacagcgccacctgaccggccttcccggcccatgccccggtagccccggccgcaggtatccagcgcttgcccgcgtcgcctgtgcccgtgctgggcggcgcggtgagggccatagattcgacggccaagggcaacaacgcgtcgatggtctgcattgcttggttgaatggcacagacggctgaaaactgttctgcggcatttcgggaaggtttgcattcggtgttgacattttcggcccttacgtgctaattgcggtggaatacggcccttcgccggttacggtgttcaaagcgcaaacttgaaccgtaatgcctgccggggcgctgttataaactgcggtcatgttctgcgtgtcaatcacattgccattgctgaacttaatgcgatagccagcgaaatacttaccgttacgcggtgccgtttcaatgccaagccgcccgcgtccaacaaatgtgacagtgacgttgtttgagccgtcgcgcactgcggtaacgctatgcaccgggaattcgcgttgcgacacgccttcaagatagtcatacccggttgcaactgtttcgtcttcggtaaggccaagactgaccggcttgatttggatttcttgaccaagcatccattgttgcgcctgcaaaaacgcgatacttgaatcaagtaaaacaaagcgggttcctgtcggccaatcttcaacggaagttgcgtaacgaccgcgaaccaatccgctgagacggtagcggtaatgcccgtcaaccataccaagcagaaccgcaaattgaaattgcatcaattcatcgccgacaacacaacgattgacgttgttcaacaggttttcatacgtgaccgattcaagcgcaaagtttaccagcacttcaaagctttggttggctggatattccgcgctgatttcgtctttaatatcagttagcgtttcacccaaagttgcaggcgtttcaatttgcatggcttcgtagaagttaacaccgccgtcagtgctgataaggatttgcgatccgtaccacgctgacgaagcgcccgccactgcaatatagacgcctaattcatcgtcttgatcgcgcaatgtgggaatgttcaagatttcaagcgttgtttcaccgaccaagcccggcgttgtcgaagtaggaggcggcaacgactggcctacgccaagcgttgcgtatacgtcctgccctgcgtcctgtacgccttcaaacttaatgatcgggtgattgtcgttgcgttcggtgatacgcacgcgataccaattgccgcgcttgtcttcgacttccacaacgtcagttgaaacaacttgcgcgtacttcaacgttgttgcaaacttaaaagtctgcaattcatgccaagcaattttaagcttgattgacgccgctgtcattgcttggtctgcggttaaaacaacttcgctttcaaccgtttggtctttctttgccttgatgatgttactgcgacggcgtgcggtttgcttattcgtagcaaagccgccagccgggtcaaggtgattgaccgacacagaacgggcgagttccttttcttgcagacgtgtttgttcaagcgccgatggatcatccgcaacaagatcgcgatacggaatacgaacaacaaccggtcgcccgcgtcgagtaaacgctagcttcttatcggcttcggctttgtcgaagaagaacatttcacgcaacgcatcgatgcgcttgttaactccgtcatcggtgttcagcttgtaaccgataacgttagcgtcgtaaagttcgcgcacgtctacggcttcggggttgattccagcacgaacacaaagcgctaaaacaatgtccgctaagaatgggtcaacgttaacagcgaactgactatcaagcgcagtaactttgcggcatcggaattgcaaacgtccgccagcattgatgcccacacagacaagctcggccgtcgaaccaaccggctttaaaacgtgttcggtttgataacgttcgcgctgataacgaacgcacaggttgcccgcgcgaacgtaacctaaaacaatgtcagaaatcgccgtatgccattcgcgccgttcgtccattgtgcaacgcggcgtgcgaagatcggtgccaagggtcgtgatagtctggcccggaatcgtcggatcgtaccaccacattttagtggtggtattttccaagtaaactacaaacgggcgcatgttttggtcaaacgacaaagacgcttctttaacgttggccgccgcaaacagaaattgtctaccgttcgcaggggattcaacataaaaattccactgcgttattacaaccggatcgcgttcaacttttagcgtccatagctgaactaacaacccctgcgaaggatcgtttaacgcgatgccgccacgttcgtaatcaattaagaagtcaccgggtgtttttaccgggtcaacgaacgcactaacgaacgcggtggtagacaactggccgttatcgggcagcatttaattatctccgggccacggtaaagattacgtcttgtgaccacttaaattggttcgtcttaggtactttggcgttggtaaacgtgattttatagccgccaaggccagcggaaataaataagctacctacgccacccggcacgttaccctgcggcaagttgaacaggatagttccggtgcgagtaaagctattgtcaacgtagggtttcagcgtccacgactgggcgttttcgacgttaccccaaatggccgacgcattttgttccttcgggtacagcgtttgcaccggggaagcgaacaccgatgtttggtaatagcttgaccatcgctgttgacccataatgctagtgtcaagtgcggtcataccgccagtgtcacccgtgcctgtttgccacgcgttgtattgcgcaggcagaaaatcgattggacgaatgttgtaatcgtaactcacgccgttaagcgtaatcgatcccgttacttcggctggcgggtaataccgaatttcataataaatgtctaacgtttcgtcaggctgaattgcaatcgaagtagggttgccgcccgaatcgagaataagcgcgcgcgaacacataatgttcggacgggtgggactgcttgccatacctgccgcaaatatgccgacttcttgaatgttgttataggccgccagaccatcggcaaaacgaaacacccagcgccgccacgtatacgaagaatccgccgcgtaaccgctagtttgcaagtcgtaaggcttaccggaattaccgctagtcccttgaccaacatacacaaggaacgattgcagggcggtatctgtaaccgtcggggtctgattgccgcttccaattgcgcagttgtaaccgtaggtgtttctaccgcttatgtccttgctgagtaagcagttaagcccggtgttggtaatcaaatttttgaattcagcaaccttgcggcgcgtacccgcaatttcattgccgtcagcatcttgtttgaaagcttcaaacgtaaagtaaccggcaataccgcattctaaaagaagtggttcgggctttttcatcatgttcatatttacggtcctaaagtaccttcgccaagagacgcagacatattaacggattccggcggataccggtcatagttcacaagcgcaacacgtagccagccatatggaatgtccgccgaaaggttaatgctttcttgtggcacattatacggcctaattggatcgtaaagcctaccggcgccaagcgcaatatcattgcttatgctttcagcaagaacattgtaaggaacgattggcgttctaaaatcgccaaaaccaagcgttagcgcaaggtcaaccgattcggtgtaatgttcttcaaacagcagcggccgcagttcgcccgcgctaagacccaagcccatttgcaccgattcgggggccatgtcgttcggatacggccgcgaagtcaaatatgcgtcaggcggcgaagcgatgataacggcttcgtatgtgggtactgcgccgccgttgtctgtaacgtcatcgtcttcaactacgatgtacgcaacgccgcgatgtgcagaaaccttgccagcacctttatacgattcaatcgttgaatctggcaattgcgtttcagtgccgtaatagaacgtcgcctttcttgcccatttggccgcgtaagcgcgatcatcaaccgatgcgctagggtcttgcgtccaaacaattttgccgtttcgtttgatcgtccaatagccgaagatcgggccttcgcagaacgcaatggcatacgaaagcgtgtagctgtattcttcggttttaacgccgcctttaccttgtttctttttctttacatgttccttcggcggcatcggcgcaaagataatgttgccttcgcacgggaacttaccaaagccgaaaggcataggaataccgactgtcgaagtttgcgatgcaaactccgtaagccgatttcctttgattgtgattgaaccgaataagcctgccatttcgtattaacctaaacgccagactttttcaatgcgacgtagccatttcgcatctaatatatgctcggtaacttttccaaccattgaatcggtgtgaattaaagacagcacaccgggaagcgtcggatgattaagcacgatgcccacatgacggattgggccgcgatattgcatcgccgctaggtcgccttcctgcaattggtcaatcgtaggtttcaacagcaaaggcggcccgaaggccgcttgcattgcgttttcaagttcgctgttgtacggatcgcgagggtacggcgggatttggtcgaacggaaattgaattgcgtaagccattaagccgacgcaatcaattccgttttcgttccgtccttgatgcacaaacggtacgtcttttaaagcccttgcacgttccgcaatgtcggtcatagcgcgttctgcgatttaatgtatgcgcccggcaccatcaaagattgatcttcggtcggggtcaggtgttcagcccgcatattaactatgttgccgtatgacatgcaatcagtttcggttttgccgcagtctttgcgtagccgaaccgcagtgccgttcgctacaggatacggggaaagataactaagcttcactgtgccgtctgcggcccagctttcaatttcccagtctgcgccttcgttgtcgccgctatcgaaatggattacgcccaattcaaagtaacccgccggttgcgaaatgccggtaactttgaaaacaagctgtgcgttttcgttcggtataagctgcactgttcctgcgaaccaaataagcggcatttggcacttggaatcgccaaactgcgcccggcatgtcaggctgtaatattggtttgtgtttacggtcaactgctgcgtcaaactgcggaattcaacaccgcgcttgctcttgccgtcactgttgtaatcaatttcgccaactgtgccgtagcctacgacttcgtagccgtaagcaagacgcaaatacgacacgcgataaatggtgatttcggcagaatcgaacgcacctgaaataaccttgcgttcaactgcttctttaaaccaaccgagcagtttggtattgtcaaccgtcatgtcggccgacgactgaatgttttgcggccgcaattcttcgtccggcaaatacgatacttcgccaaggccgtcgttgaaccttacgacaaaatctgcggtggtgaacgcaaaaatgccgtcttctttagtgacgatcttaataagaaagcacgtcgaagttccgggcttgccgaattgaagttgcagcgcaattggaatttgcttaggcattattcttcccagctatccggcatattggttgcagtaataaggcgcttaccttccatcaattcgacctttgcggtattcgcacgccaactgttaatggtcatgctgttatagtccgcgtcgaaacgaacccaaacgtaaaactcgccggaccacgtatgcgtgccgctggcccaattagcagacggtgtaaacatgcccgtttcagtgtcgagcgttccggcaaccgcgtttccgcccggcgttttgatgacggcgctttttattgcttggattggtcgcacggtccaagcgggccaagctacgccggtaactgggtctttcggttgataggttttgtaaagttgaaccggcttcgtggtgcccgcttcgacctgcaagggttcatcaactgcaagaaaatcgttccagtctttgaacttgaaatagtgacgacgacccttgcaagcgtgaaacgctgcaatgatatagtcgcggtcttcgtcagtaatattgccgaagcttgccgaatacctatggcgcggatacgcccatgcgctatcaatgtattcgtagccgttttcaaggtctacgatttcgttggcgtattcgggaccgccttcaaaaccgtaatcaacctgttcgtctaaaactgcgttaatgtgacccattagccaccactcctaataagttcgcgcgtcgattgcgtgcgaatcgcccgcgcttcctgttcagcggtgcgacgatcacgcttgcccgcgacggtaacgttgacggtttggttgtagttaatctgatcgctgcccacacgggtaggggtcggcgaagcgtcggttactgcgccgctttgaccggtgccaagcgaatcaaccgggatacggccgcgtcgcagcgcttcaaggttgccgacgccaatgcgtgcggttgccggtgcgtcgaacacgtattctttaccatgcacagggccagcgattgagtttgtggggatattacccgtatagccgccttccttgaagcctgcgttctgtgcgcggatttgctggacgtttgccatacctgccgcaatggccgcagccgcagcggccgcgcccaagaacggaccgacgtacggaatgcctgccattgcgctgaacgctgcggtcgcactttgataggtttgaatcaaagtctgtgcaattgccgctttcttgccgattgcagcttgctttttgttctgcgaattttgcagcgttgctaaagcgccaagcgcagtggttgcgccttcaatttgcttagaatactgctgctggaacagttccattcgcgcttgaatcgccgacgtttcgctaatcaagtcggcttggcgaagcgcatcaatttgcgcgtacatatccgtatacgacgcaatagtttgctgctggaattcgcgcgtcgcttcaagcgccgggttttcttgcgccaacgcactgatagcgtcgcccccagtgaagccgttgttgccgacttcaccgattgcagtttgcgtgcgggtcgcagtgttgaccgaacgttgcgcttgactaccttgttgcagttcatcgcgcattgatgaaacaatgttcaactgctgcacaagcttcaacttttcacgcagcgctttaatttcgtcatcgcgcagcggcttgccttcctgcaatgccttgttcatggcttgcagaacttgttgttcaacttcacgttgcggacccaacatgccaagcagcttgatttgttcgtcaagttccttgttcatatcgtgcaacggatcggaagccgacgcgaaagcttctttcgcccggttcacttccgcaacatactgcgcctgcgaaattgcgcccatctttacaagcttgtcagccgcagcaagcgaagcgttgtattcgcgcagcgggccggtggcgttttgatagatgcggtcaaattgcgtttgaacttccttggcgtcattcaacgcctgaattttcttacgcagcgaatcaatttcttcttcgcgtagcggctggccttccttagcaaaacgcaatgcaatttcatccgcgcggttagctgcatcgcgcgccgtagccagaacaaacatgttcttagcttgcgaatcaagttctgcgttgatttgcgcaagttccttggcgcggtcaaagcctcgcgacttcttacccttgctgtcgtcttcgcctgccgcagctttcaagcggtcttgcgcgttcttcaacgcttgcgcgcgaacgtcgttaccgaacttggtaacgattgtgtcagcctgcttgtaaccgttaacgattgcgtctttaacgtcgctttgcatgttcttagcatctgcgctaagttcaagacgcggcaacttgatttcaaccggcccactcatgccgagcagcttaccgagcggactatctgcaactgctttgctgatttggttgattgcaaactcaatgatggaaattgcgccgtttgctgcgccctttgcagcagcttcaacggcggcgggaatgtccttccaaacggccttgattacgttagcgaacgaaagccacatgccgagttggatgcgtacccacactgaaaaggccgtggtgatgaaatcgagcgccttgttccaccacttgacgacccattctgtcacaggcttaaaatactgcgtagcatactggccgataacttggaaggtggctttaaacgtatcgccgaaggtcacgcgcgtttcttcgcccgacttcttcaatttcttcaattgatcttcggtaagctttaagccgtcaacaagctttttggaatcaacgcccttgttaaattcgcgagtaaacagcgcaaagggcgcggtcacaacaccgatgacagcggcgaaagctaacagcggcggaattaaacgcgcgacgatgccgcctaactgacgcaagattgcgccagcgcctacgccggacgtgccgaagatttggccaatttgcgcaccctgttgcaagaacacttgcatcggcttttggccagaacctaacgacacaacaacgtcgttaacttggtacgcgagattctgcaattcgtggcgagctaaacccgacttcttagcggtttcttctaagcccttcgtaaagttctgttgatatttcgggttgcgagcaagcaccgcattaaagcggtcgtgaatgccgctaatgcgttcaacttctttatcttgccccagcatacgcatttgcgaattgagccgttcaagggctgcgctttgctggtccgccgaaattgcacccttcgccatagcccggtctaacaggtcttcggcgcggtacatttcttcaatgcttttaacgccacggtctaacgtagcgttaagttctgcaaccattctacgttggtcggcggtcgcctttgcggtcgcttcgacgcttgcacgcaaacgcgattcggccgaagctgcatcattcgcaacgcgtgcgcccgccgattcggcttgttcaagcttccaacgttctgacgtttcgtttttcaatgcttccgctttgcggatagactcttgaaccatgttgcgaatgcgatccgcacgggcctgttccgccccggccgcctgctgggcggcggcagcttccgccttggccgccgctgcaacgcgtgcgctggcgtctgccgcgcgtttctgcgcagcttcaagggagagggtagcttgggcggcgcgtgcctgctgctgggccgcctgcgcggccgcagtggcggtcttggcctgttcggttgcaagacgttgcgccgaaatggccgcctgttgcatttggcgttcggcgttgcttacgacgctgctaaactgcgcgattgcggtaggctttacgcggttaagctgacgaacaagcttttcaacattctgataagcgctgcgtgcctgacttgaaatttcagacaggttacgcgaaatgtttttgtcaacactgtcttttacttcaattacaacaggctggtcagacatgtttatttcctaagcttgaacttagctttcgttttacgcccaagtaaaatggcgcgttcgataaagcctgccggaacttgttccgaatacccgtcattcaaacggcgaatatacggaaggttgtttgcaatgtagatgacttcgccgggctttttgttcttcaacgtttcttttgcaacgtttaaagcttgtgcggcgctttgttgctgtgtcgaaccgtgcttaccggcgacgtatgggccgtgcggatcgtccatcggtgcccctatcgtaacgtcccagttcgacagggcttgcgatgtatcaaccggtgtgtgataaaccaagtcgccgacaatggttagcgccgtcttaactgcatggtcgctagcagcttgcgaaatttcaccgccgagcttgtcaatgtcatttgctaaatcaagtagcgagcgggccatcacttcaccttttggctttagattccttttcaagccgtttcatgtgggcattgtccaaagctttaacgaagaaaaacaagtcttcggtcaaatcgctatcgaacgaataagcctgcgaatagtctttaatcttgctccacggtatagggccgatagaaaagcctgcttggcgttccgtgtctaaatcaaaaaacgcattcaagaacagttctagaccgatgtgaagttcaggagcatttgctatccgggcgggtattggttgacctgcccggatagcttgcttggcaatggactgttcgtgcggccccatttcaagcaaatactctaaaacttccgtcagttttttgcggattcctcgcgcgtcgcttcaaggaacaggcttgccgaactggcctgttcttgcaggaaatcgtagagttccggcagacgttcaaacagtgcctttgcgttctgcttgttgaattcgatatagccctcgtcgctcgccacgccggtcatatcggccttcggaacgttcgaccaaccgcgcaaaacggtatcgcaaaacacgtccatgaaagctttttcaagctgggcggaaacgtcaatcttcaactgaatctgacgttgaaacggtgcggcagccttggtaagcgcggcctgataaaccttgttggtcttgctcgcgcgtgcgagaacaaacgtcggatagcttccgtctttgttcacgtcgccgacttcgatttcaacgccgttggtttcgcggtcggtgtcggtcttgtattgactggaaaggcccattttgtattcaccttttaagttaaggaaaaggccggggcaatcccggcctttccagtgtatcgcgtttaatgcggccgggctacattaacccggcattgcgacgttcggcaggaagacgaacgattcaaacagcatggtatagccgttcgggttttcagcaccggccggttcaagcggaacggtaatcggcgcatccttttcaacgttgatacgaccgccacccaaaccgagcaacggaatgtcgaaaatgaaaccggcgttcttcgacgcagcgatgatcgaaaggccaacgtcagcattggcgcggacagccttcacagcggcaaccgaagtgaagtaagccgtaatcgaaccgccgacagtgaagttcgcagcgctggtatcgaaagcacccaacacgccaacagccttgttcggcgtaacgccgttgttaatcgaaacgttcgcttcggaaacaaaaccaaacagcggcgaaggcgcagacgttgacggatcaacaatcgccatcttgatccggtaaatgtcagacgaagtattgaaagcatcttcgcccggcgcagaaaccaaggttccaagggttgacgatttgattttgttttcgtcacccgccgcaccgctgcgataggtgttgtcgcacgcaacgaaagtcaaatccgcgttgatcttgtcggcctgcggaatgttgacggtcagttcattgcaaactgcaccgatcaaatattcggcctgttgatcgccggggttttcagcttccgggccttcgcccaacgtgcgttcgatttgatacgaacggcgcttgattaaagcagcaagcttttcgttcttgatcgaaataccggcgaagaagcgaatgcttttaccggtgccagcttcgttaaccggtgcccaagtcgtgtcgtcaaacgtgatcgaattcgcagacacagctttgatgcgagcaaagcccacattgttgacgaagcggtttgcggtagcgtcgccaccgatgaacagccacttgcccgcaaacaagttcgggaaggtgctaaagtcggtggttgtcgaaacaagcgacggaatgccgtcaacaactgcgaaggaaacatcgcccgcaatcagttcgccgccaacgcgctggaacttggcaccggccgggggagcggcttcgtcaacgacagtttccgcaacaacgacggtcgttgcggtcgatgcggtgacgcgcttcaaaccgttgtttgcggcgttcgcaaaacctgcggccaaaatcaattggcccgctgcgaagttggttccaccgcttgcaatggtgtaagtcttatcagcagccgttacgccagtgatggcgatacgcgggccgttcatcggaacagtcgatgcgggttcgcgcgcgtctgcgaagaagaagccttgcagaatgcgcgtcatgttcgacttggtaaaatcggtgttgtaaccaccgcttgcatcaagatcggtaacggttcctttcttgttctggcgcgacggatcaatcggcgcgcgtgcaacggtggtcaggtcgccgccaaaatccgaatagctattcggttcctgaccgtaccatgtggggtcaaagccatcaaccgccaaaacgggaagctgctttaagcaaacttcttcggcgatgctaaggccagtgatgttggaatcaatcttgacaacttcgcaaaccatgtgaatatctcctagcctagttcgtcgtaatcgtattcggcgacaacgttgatgcgataaaacagttcttcggggtcaagcccgtcgttgatacgtacattgtggaacgtaacgccaccgtctgactttttgccccggtacgcgtttcttgcaaccttcgccagcgtacgccctttgattaaagcattcgcaatcgtcttgggcaagaacaattggacgaagattaagcctgcaccattccagcggcgaacgtatggtttatctacgcaggttgatagcgtcgcctgttcttcggtaacgttctgcgttgaaaacctgacccatactttcgtgcgatctactttggtactcgcttctttaccgttccacacaatttgcggaatgtatccaaacacagcaccggcattggcttgccaagccgtgttaaatattacttccatttccgcaactgcttggtcgaattcgacggtcatcccttaaactctactgtataaagaatcttttgcccgttcggcgaaagcaagtcgatgttcaaaatttcaagagttacgccgtcgcgcaatacgtagtctgctgcgtcaggcgtaaaagaaacattgcccattaagccgattaccgaaccaattttaacgtcattggttccgcgaagatacgcgataaactctttagtatctttattgaccggaagaaagcaaatataaacgtcgtggtctaccggatcgttttcaatgacagcagcagggttattcggatcgtcttcgcgttgcaattgccgccacttaacaagctggccgttcttttgaatcaaacgaagcgcggttgcaatttgtcggtcaaagcgcgccatgattaaacccttacagtacgaagcgcgaatgcctgcccacatgatgcgtagaacagcggattaagcagcgaatcaagcgccgtgaacgtcgctgaaatgccagcttgaatcgggttcgcatatttggttgtgattggcccgacagtttcttcaatgacgtaatccgctgcggttacgttcggttgcagaactaagccttcattttgaatcaggacggccgaagcttgcgcagatttcaattgcttggggatcgcgttcgacgggtaatcgtcgcagcacatgacgacaccggttcgcggccattgcaatgattgctcgcaatcagtcttgcggccttgatacttgcaagcaaacgattctaaataatcggtcgccttgataatcatggatgcaactgcatcatcgtcggatggaagcgacacgccgcgctgcgcggcatactgccgcacttcgtcaaccgtgacgtatgaattagcgttagcgatgccgcttccatcttcgacgatgatttcaatagccattttgtagccttacgctgccggggtaacggtgatgccgcgaatggcaccgcccgaaacttcaaaggtgtacttgttgccgccgactgttacctctgcggcgttctttacgatgcaagccgtggcttcaagaacagcgttgcaagttccgtttgcaaacacgttcgcggttccatccgcagcgacgccaccttgatcgttcacgcccatatagccgccggtcgtgttcgtggtggtgtttgccggaagttgcaaccgggtgatcgcgctgtttgcaacgacaatcgttgcgtcagcatacgttgcggttccgtcaagcgtggtgacttgtgcggtatcgccgttcgttacgataagcttggtcggcggcaacacgatttcaggcgggttatcggggtcaatgaccggcacgtcttcgtatgcagtcggaatcgttccggccacataatccgcagcttcaagcggaccgcccgacgacatgggacgaacggcactgcgaacgccaacgtcatacggcgacactgccagttcgttcaacttttgaatgtccgccttttcagcggtagttgctacgtcgcctgcggtgaaataaattactttgttctttgcggccattgtcgcgattcctgcgttgaataccgatagaaaaacggggcgggttttacgccgccccgttcaacggcttagttgttcgacttccaagccgcgccggttgcgccttccggtgcgtgccccggcgctgcggccttcgcggcgtcaaggtcggccggcggcggggtggactggccttcgtctttcgacacgtcgtccttgccagcctgcgcgggcgcacggcccttgtcggccggtgcggggttcggcttcaccggcttacctgcggcgtcgttgttggccgttgcgttcatttcgcgcacctttgtggcgtgcgtcttgatggcctgtgcggcggtcggaagcttgctatacggggcgggaaccttgcctgctacgccgtcacaagcttcaagcgaaccgtcagccggaactgcgcgagcattgcggaaaacgacatgcgcgttgatttcgctggccgcttcaacatcggctgcggtcggtgccatgccgtcaacgaaaaaaagaatcttcggtactttcattgtggttgccttatcggttcgtgttgaaaagccggggccgcaatggccccggctacgtcactaagcgttgcgcttagtgggtcttcaacaggacgccagccaagtccttttcagacgtggaatagcggtcccagttcgtgccttgcaggattgcggcatcgttcggcgacttgccgccattcgccttgtcccaagcgaagcccatgatgcccagttcatacgaccattccgcttgatacgtgcggatgatgttttcgtcgccgttctttgtttcttcgttggcgtcgaagtcgttgttctgatccaccatgattgcgcccggcacaaggcccaacgtgttgtaaacgttgggggtgccagcggcaacaagattcggcgagtcggtcatcacgtaaacgcggccgaacggatcacgcacgacgttgacgctgccgtaggtgaaaagacgctcgttgttcgtcaacgcattcttgtaaagctggtgcatgggcttgctgtgcataacccaagcttgaatgcggctggacatgtcaccgaacttcgccgacgcatcggtttgtgcgataaacgacatttgatcgtccggggcagttgcgccggtaatgtcgtgaaccacggccggaacgccggacagtgctgcgacggttgcgccgagcgaagtgttcagcatgtcggcgagagtatcgacggcaagctgctggcccagtgcgacgcccgcgacttccgggttctgctgaatccaacggaactgacccggatcaatgcgaatcggcggcgtgcccgccgcaatcttgaccatcgtgtcaacaagatgcttcaagctcttttcgctgacagcgcccgaaccgtaggcgttacgacgacggacaacgccgcctgcgatctttgcgaagaaagcaacgtcgctgaaatcgccttgatgcgcggccgattgcaggacaatggttccgccagacgcagcgttgaacaggttcaactgctgttgcagaacttcggtaaacgacgaatacgcgtattcgctgtaaacggctaaatcagaaagtgccatgttggcgcgtccttactcggtgggtgattgttcggcctttcttgccttcaactgttccgccaactcgcgcggattcattgaagccatgttcggcggttgttcgcccggctgctgcgcgggggaaggtttgacggcaccgccgttactggaaggcgaaccggcaccgccggacgcttttgttacgcggatgatagacgaaaaatccttgtttgcaacaaattcttcgcccagcttgtcaagcgtcagattcgacaccttgccctgcgcgtccagcaccttgacaaccggcgcatcgccatccatgtcaaccgtcaagcggcgttcaatgtggggacgaatgacgcccggtgcagtgctaaccttgctagcaagagacgccgcagcgttttcaagcaacgtcgttttgatgaaaccgtttgccttttcaagcttgcccgcaacttccgcaacggcgtcgtctttatctttcgcccattgacgttcaagcgcgtcaatgtcgccctgctttcgcgcggggttcgtattgatcttttccaactttccggcaagatcgtcattggaattttccaacgtcgtcacttgatccttcaagcgtgcgtttgcgcgcttcaacgcgccaacgtcttcatcgccggtggtttgcagcgtaaagctgtcgccatcggcggcgtattcaaatttgatattgtccggcagactgtcgaacttttctttcgtgattttgcgtgcaagtgccatgtcttcgactcctactgattcaccgaatcaggttgaaaggatcaagccagttttcgacttgaattgattaaggtcaagcggttttcctacaacaacggatgcaaactcctttgaagacatttgccccgaatctatcaagcctgcaaccttatcgccaacgaactgcgcgattactgctttaggttgccgcttgaaccaagcatataacgtcggcggtgaaaagtcatcaaactgtgatgcgaggggtacggttgtgctgcgacatttgtaatgcgctggcggaattggcccttccccgtaacgataaatgtttttatcgtgttcaatacaaaactgcgtcgtctgactatcaataaccgaaatccacatatagcgcgaatagatcgccgaactaatagcggccgcgctgatttggtcaacgtgtgcaaacgacgtttcaataaccgcgttagcttgattacgaagcttggcaaactgagacgaaaaaccttgcgcagttttaggcgcgaacagttcaagcaacgtagcgtcaacgctctgacgattcgcataagcacgtcgaattgtattttcaacgctggcttgcgcagaccgcgaaaacgttgaaatgaagggaagcagatacaagccgtttgctggaatcggtgcgttcttgatcgaagaccaaagcgatttgctgccactaggtaaaatggcagataaaccaaatagcgctgcgaacggcaaaatgctgttctgttcttcaatgtattcgtaagattggtcttcgcttagttcttcgtcagacccagttgcaaattgatgcctaaccgtggcataagccacggcgctaacgtcaagacgaatttgcataaaatcctgcaacgtcttgataagcttttcggtgtaagcgctataaacgcgaagttgcgactttcgcattgcaagcaacagcctatttaattcagccttgctcaatccgtctaaagtcctgtatttgactcgactaaatatctttcgcaagtcttcttcgactactgcaagaactgcgccgaattcttgcatttgaccaagcttgacgttttcaacaaacagcgccaagcgtgtcgttatatcaaacagacggccggtttcggtaagtgccattgtcagatgcccacattaagcggacgcaggcgggttgccgccgttgtcgttttggttatattgcgggtcattttcggcaagcagcgtcattgcttcaacctgttcgtcggcaatcttcttcttagcttcttcgtcgtcttccgtagccagaccatagcggcgaagatcggcgcgcatttcggcccaagtaatggcgcccttttgccacgcttcaatagccatacgaacttgctcaggcgtaagcgctgcaatttcaaaatcaatgtttaaggcgtattcgatttctgcgccttccgcacccatcaacattgcggcgtatgccaacgcagaacggtacgcttcgcttacgttgtttgcactcgacgtaagaacggaattttcagcggccttgtcctgcgaagattcggttgcggtacgctgcacttcacgctgttcaacaagctttgcgccaagggccgtcatctgacgttccttggtgtccatagcttctttaatcatcgtgttggcttcggcttgcaacagttcggccgtagctcctacgggcaacggaatgccgccgcgcgaaccgaacgccaattggccgccaagtacgttcttaacccattcttcggttaagccagttgcaaccggtgtgggctgtcctacgacgtagcacgattcttcgtaatcagcgctgttgcgataatgcgcgatattcaaagacgccatatcgtacatgttcgggttatccgggttaacgtcgttgttttgactaccgataaaccaaaacggaatttcgcgcagcggcttgccatccgggccagtcggcttaatggtatgcgaaagctggaagttgcctttcttcggaacgctaaagccgtcccatttattcgggtcaggttccttccaaatttcttgaacgtagttacctgcgtcatcaagcttcaaaacgcggaactgcggcgcattcttgatttcaaagccatcgtctgaaaccggatagccttcaagcaaaacgacgagcgaaagcacttcgtttgcgccgcgctcggttactcgccagttgataatttcaagcggcgaatacgcgtacattgtcgggcggatttcgcccgcttcaacttgggctgcgcttgcgccgccttgcgccgaagtatcagggaaatcaacgaacaggccgcttcgcgaatacgcgatgttgtggcctaagctgatttcggcaagctgattcaagctagttcctgtaccggttgcgttggcaatcatcgggtcaagaaccgatggaagctttacggccgggtcttgtccgaaaacttgaccaatcaagcccatgacagttcgacgcgtaacgttgtaaaacactgcgcgtaaaaggtaggcttcgtaacgtgcgcggttttccggcgacttgtccgacgcgttaggcatcggcaaatacttcattcgccggtctttgattaccgtttcgcccgcgatgcaatcacggatcaattcgtattgcggcaacagccttgctaattcaggccgaatgaacgcaacgttcggatttccaacaacagtgcggcgaatggctgcggtcatttgcgtaaccttttaagtaggcattgaaactttaattgaacgggcgacacgatgactgccctttaaaacacgatagcgtgtcatgtcccaacagtgatcttcggtcgtagtgtctacgtcgtcaatcttgatcggatcgcgcggaagctttggaattaggctaatactagcacggcagttttccataaagtaaaccgctgggccttcacctttcttcgcattcgacaatcgttcgcggaacaattccattccgtttttacgcgaacccggcgacttatccgattcttcccagttaatgccgaacttctgcattttcttttcaatcgtgtcaacatcgctttcgcgaacatcgcgaatttggttatcggctggaccgggccaaggctgcgatttgatccagccattgaacattaacgcagtttcaatttccctaattttctctgcgatttcaccggctggctttttcaagcctttattcgttccgatcttttcagttccgtagtattcaaagaactgaattaacgaacccggctgcggacagaaagtaaatacttgatcgccgataataaccttagcttcttcaccgtttgcttcggcccaccaacccacactgaacgggtgcgaactaccccagtcaaacgaccggtcaatattccaacctgctggaataacgaagcgcggcacgacatgatatttcttgtcccatacgtcgccgaaagcgtcaccggctacaacgtcccaatcgccgtacagccaagccttgcgcaagttttcgtcggtgatggattcaagttcagcaacatattccggcggaagatatttgttttcacgatacgaaccgaagatcgcaacttgcgtgcgaatgactttatcgttttcttgcgtctgaggattgaatacctcgacttcggttcgtacgacagtcccgcgcggtgccggatcaatgaaacgatccttaacccagttgtgccccggaccggccgggttggtcgtgctgaacacttccaacggaatcggcggcaacggtaaaccgttcggcgtcaaatagcggccggtcttcgggtctttcggcgtgtctcgttcggggtcaaacgtcgaacgattgaccgacatgaacttgttataaagtgcgtcggttgcgtgcttggttaattcgttccaaccaagaaacgggtattcgtgaccgtggaagccttcgtaatccgcaatcttttttacgtgacgaaatagcagttcttcgccagtcggccaaacccatttgtattgcgacggagattcaaggaaaacagccccatcgccaaacttcttaaaccatttctttgattcggcgaccaaacctgctaaatggtcaaactccaaatcaaagataacgccgcgccaatattggccgtaaccaataccaacgcggcgacgaaaacgcattaactgcgttaaagttttgccgggaccgcgcgcaccttcgtacagggtatgatggcaccgggaatcaatcgcaagttcttgcgaagttccgggcagtggttgccaaataacctcaaacggttgcgcttcggtttcagtgtcgggatgcgctaacatcaatcaaattccgctgttgctgttgcgctttgcgttcccaatcgtcgtcagttcccatgtccttaacaaccatgacgcggttgttattgacttgaacgttaacgttcgtatccggctttgcaataaagcctcgcacttcggcataaagcttgaagaacttaatcttcgtttcgccgtcccattgcgcgcgggcttcggttaacagttcgcgtgcaaaatcagccttagtgccaatgaagttcaaatcgccttcgtcagcacctttaagcaaacgcgtttgttctgcgacaacaaaaggatcatcaagccacttgttcgccatgacaagggctttaccagtatcggaagtaaccgacagggccgccgcaaacctgccttcaaggtcttgcggatgcttcaacagcgcattagcaaatgccagctttaagcgctgttcttcgtcaacagaaacggccgggatagtgtccatgcggagactataaccggccgtctgattatttggaagcagcgccgcaattacgccgccatgcttcattgtgggcaagtatttgccgggctgtttcgggtgataaaacgtcttcggtcttgcttatgtaaatcggtgttacccatttacaggcagtgtctacgacgaccgtttcaggtattcgatcaatcccgcgcccagtcgtcatgca

SEQ ID NO: 3 - DNA, 44570 bp, unidentified
  source 1..44570: mol_type = genomic DNA
ttcagcttcttaacggcctttgcttcatagccgttgttcaactggatgcgttcggttcctgacaacttttcattgtcgaaagagaaaacaacgaactgcttacgcagattcatttcgtcttctttcgccttgtcaagatcctttttcgactgttcccatgccgcaaggatgcggtcacgttcggccagccattccggggtgcctttgaccagtgcggccgggggcgtttgagtccatccgttgtccatgcgatcacctgtttgggttgggttgcaacggccgttgttcgaccgttgcgcaattaaaacacgcttatttcggcttgtcaactaccggcaaacggttttcaattactgcccgctccggttcggtgaacgttgcgccccagccgctaaagattgcttcgggctgttcgccagtgatacgcgcgtaagcttcgcgcacagcttcacgcattggcaaatcggcgccgttgggaatgtttaccccgttcgtgttgccaatcttgcatgaccaagcttcgcgcatgtcatccgggccaatcttgacgtatccgttcggcgaagtaacttcgataacatgcccttcgccgtcagtcagcggcattcggtagccttccggtgtacctgcgccgtgcatttcaagaatcttgcgttcgccgaacaggtcacgattgttggcgtcgtactcggtgaacttttgcgggaagcgatgccgcagcttggcaatgttgcggcgctgcacttcttcaaacgatacgccaattgcgccaaggccaatcgcaacgtaccaaagaacgtcgccaagttcttcaacgaagttcacttcgtcaaactctttcgggtcagcccggtcaactgacttcaacagcgcttcaagcagttcaccggattcagtagcgatgcccacaatggcgtgcaaaaggaattcgcctttgttcgggttgccttgctgaatgatttcaggccacgtcgccatgctcgcgcgaacttcgttgccggtggaaaagtcttcaaggttgcggccgtaaaacagtgcctttttcaacttgtccagttggttcaacgccatcaccgaacttgtgatgatgccgaacgcttcgtgatgcgaaacagcgtggccgtgatagttgttcgatgcggtaacgttcgcttccgcaatgtagttgaatgcttcggatgatccggccgggtgaatcggtgcgttcgacatgcgacgttccttgcgttgatttgactggctggcccggtaggaatcgaacctacgatgccgggatcaaaacccggtgccttgaccgcttggcgacgggccagtgtggaagcataggctagacacggccgtcacggctgtcaagcaaattttgcgcttgacgcgaattattttgcgggtcatcatgtgcgccatcttgccgaacttcggcccatataaacaaggtgtcaccgcatgacttcgcttgatgttgcgacgcatcccgaactaaccgaaacgttgaagttgttggcgaatcggccgcgtactctcacccttgaagctgtcgccgatggtgcgaacgttagcgtcggttggctgtcgcactttgcgcgcggcaagatcgatgacccgtcgtttaatcgcgtgatgcgagtccgcgatttcatgcgtcagcagaccaccgaaccgaaggaataaggccgcatgtttgggaatatccctaacgaaatgcggacctataagcagtgggttgtttggcggtacgaagaccgcgacgcagacaaaccgactaaggttccgtattcaccagcttcaaaccgcatggcatccgtaagcgatcccgcaacttggggaagctttgatgatgcagttgccgcaatggaaacgagttggtacgcaggcattggcttcgttctgaccgacaacgacccgtatacctttatcgatcttgacgacacgaaaggcgatcaacaatcgcttgatcgtcagatcaaagtgttcaatgaatttgatagctatgcggaactgtcgccgtctggcgcgggtctgcacatcatcgtaaagggcaaggtgccttccggccgtcgccgtagttacattgaagtctattcgtcgcagcgatacatgacgatgaccggcaatgtttaccgcaacgcaccgatcaacgaacacaatcaaatgttgcaggtcttgcacgggcaaatgtccgaaggcaagggcgcagcaatgttttacgctgggcttgaacaggcgaagttgcgcgacgaagaagtgctagaaatggctggccgcgcagccaacgcagaaaagttcagcgatttgttttatgacggcaattggcaaaagtattacccttcgcaatccgaagcggactttgcccttgttgacattcttgcgttctatagcgaaaaccgctttcaggttcaaaacctgttcttgcgttcggcactgggccagcgtgaaaagtcacgcgcgcagtatcgtattaattacatgcttgatcgttgcttcgacaggatgttgccgccggttgacattgatggactgcgcaacatgttgaacgaagctattgaagcaaagcgacaggagccggtgacagggaacgcgcccacgctggaacctgcaccggtccctgtcgcacctttgaaccccagccgatccgtatacagtccgccgcccggattggttggcgaaattgcgcagtttatctacgcacaagcgccgcgtcaggttgcagaaattgcattggctggcgcaatcggtttggtcagtggaatcattggccgcagctacaacattagcggaaccggattgaatcaatacattctgttgctcgctccaaccggatcgggtaaggaagctattgcgcgaggcattgacaagttgatgaccgaagtacaacgcggtgttcctgccgcaactgacttcgtaggcccggccgaagtgagttcagccccggcgttgattaagcaccttggccggtcgtcgcctagcttcgtgtcaatcgttggcgagttcggtttgtacttcaaacaaatgtgcaacgagaatgcgcccccgcatttggtcagtctgcttcgttcgtatcttgaactgttcaacaagtctggcgaaggcaacgttctgcgtccgacgatctacagcgacaaagaaaagaacacaaccgcattgctcgcgcctgctttcaccatgcttggcgaatcgacggccgaaacgttctacaacgtgttgaatgaaggcatgattgcgtcgggcctgttgccgcgcttttcgatgattgaatacactggcccgcgtccgccgttgaacgaagcacacatgttggcccggccgtcattccagttgattcaacagttgggcgaactgtgcgcgttctcgctgcaattgaattcgcagaacaaagcgattcacgtacaggttgacgaagacgcacaagcattgttgaagcagttgaaccaacacgccgacgacaacatcaacggcgcagaccgcgaagttcgccgccacctttggaaccgcgcacacgtcaaggcaatgaagctggccgcattgattgctgtgggctgcgatccatatcacccgacgattaacagcgaacatgcgacatgggcaatcaacttcgtagttgcagacgttcgcaacttgctcgctaagttcgacgctggcgaaatcggtattgacaacgacgaaacgaagcagcttcaaaacatcatcaacacaatcaagacgtatgtaactgcaccgttcagtgaagttgaaaagtacattccgaacatgggcaaccttcattcggaacgcgtcataccctacgccttccttcaacgcaaacttgcatccgttgccatctaccgcaaagacaagatgggatcaagctacgcaatcaaacgggcattgaagacgttagttgaacgtggtgacattagcgaggtatcacgcgctaacatgcacaaccaatacaaaacgtcagcagtcgcttacatgataaacgtaccgaaaacctttggcctgtaacgaagaagccccgcatttagcggggcttttcttttggatcagttgacagggccagcgttgtccagtgtgcggcgtacaaaaccaataccaccactgcgatgttaagtgcgaggtacattgcgcgctccttcggttggaagttgtaccctactacacaacttcaatgcgtgcaatacctgcggcgttacatgctttcatgcactcaggacacaccgcaacatggccgcgcaggatcaacgtagcgccttccgcgtgttcgccagccgcttcaatcgccatcacttccgcgtgccccgcctgacgacacaccgaccggcacaggtggtagcccacattagacggcatcgaaccacggggacagacagcctgcggattcgcacagtcgttacgaccgacatacgttgttccatccgttgcgatgatcgtagcttcaaccacctgttttgcacatgtcatacgctgaaccttacgttgtgtgaatacggtataacgggatataacgcaagtataacgcaaaaccctagcaaaatcagtcagttgaatggatataacaaatataatggtctaccccataccacccctgtgttatacgtgattccgttacatcgttatacgttaggtccgttacattacaatacgatcttattttattatatttattatatttattatattttcaatgatttcaactacttagctactatacagacccttataccgagtgaatgaccctgttatgcttgacatatcgttataacggtgataacgttatgttgttataactcactaacagcaggagacagacccgtgacgtttgcaattgtcgattcatcgccgcaagccaaggaagacgataagaagcaaggccgcatcgaatacccgtttgattcgcttgacgtaggcaagtcgtttgttgtaccgtttagcgtcgtaagcgagtcgcaaattcgcatggcagttagccgacgcaacaagaaaggaccgggcaaattcagggtcatcaagcacgacgcgccgaacaactgctttgaagtcgcccgccgcgaataaccgcccaatgtgggcatcacagggacatgcgcaatgacgctctattacatgctgcaagccgtcgcaatcgtcgtattgattcgttcgattcttgcatggcgacgtaaagaagaattcaaagcgttgtatttcgccgtactggctattgcaatcgtcgccgtatatccgtaagataggccatccaacaggagcaagcgaaatgaaagttcgcgttattgtttatgcagattacgaccttgtgtttaaaagcccgatgattgcgtgttacatcatgaaccacgatgacgcagcagaacgtcgtgttttgggcgaacagtgccgaaatgcgtttgaagccggtcagtgcgttgttacctatcccatcaaggggaactaacatggctgatttgaccgaaggctttgacgatccagctatcggaaaggccacaatcattgtcgcaccgccaccgggtggttttaaaggtgcgcttgatggactcaatcgtaaagagtttccattcatgccgcagatgcttggccgcgcatggcgtaagggaaacaagccacgtcttcgccttcgcaacggtcattggtgttttacggaagagtcattcaggcgaatcgttagcgtatgcgataagcgcgagcaggcaatctatggtaagtttatgattgaactgaataaggcgaatcgtcatgtataaaattgactcacacatcaaagcaccgcgcgtaaagaaagcgcgcaagtgcccggacagcgttcacgctgcattcaaagcatacagcgaggcatacaagaaagtgtttgggatcaccccggacaacttcacgtatgacaaggcaacgaagttcatccgcattggcaacagcggcggcgtatcgcttatgcgcttgaaggaaatgacccgtcagcttgaattgagggctggatgatggctaacaaatttccgtacactttggagcaattgaaagccaaaggttacgcacgcacgtcaaatcgccatcgcatggttagtcgcattgatcgggcagactggcgcgaacacatggccgaacgggcgtaccctgcgaagtatggtcatgccgacaaaggccgcgcatgggttaaagcgatgggcgttcgcgctggcgatcaataccgccgcgtttacaccgaagacaccattgaaggtgtgcccgcaagcatttacaataagttgccgaattctggcgatgacgatgcgccgcaggagtacatgccatgaacaagccgcgtatttggttgcagcactacccgaagtcgaagcgtagctattggcgcgtttcgccgctgcccggcaaatggaatcgcgtaagcgaagaagtaaaggagcgttggaacaaggcacacaagttcaaagaagcgatgaacgccaaacgtgtggtatgctcgcactgcggcaaggaactttcagctaggagtattgacgatgaacaaagcacagttgcttgaactgttgaacaacgccattcctgataaggcgctgttcattgaaatcaacgttgaaatgtatgcggaacatgaagaccgcgaaacaacgttgaagtaccttgccgaagttgggccgcatgaaatgctgaccaacggcaagattgaaacaaccgttgaacccggcgaagcgcgtttaggcttccgcatagcgagggcgtaatgaccattcgcattgatgacgacgtgccattgccgcaacctgacaagcccgatacatgggccaaggggccaattagcgaagtaggcgacgcaagcggttggtcaagtggtgtagttgtcaccactaagttcaaagaacctgtcaccgtaacggatgacggatggactagcgaacctgtcgttgaatccgtcgcagtgcgcgagtttggcaagcgctatccagccgaaacgacgtacgacaagaacggcgtgccgaccgtcgattgcttcctagtcggcggcccgctcaatggcaagaacggcccaattgtgggcacagcacaggttgttgaactgaatctgtatgacgtaaacggcaacgttgcaagcattgaactgtacgaactgggcgcaaacaagcagcttggcgttcgccatcacgcagggagtaagctaccgtgacgtatttaattgttgcactgctggcaatgatcgttctgttgttatggggtgtttgcggcttgctttggcgcatagcccaacgtcttgaaacgttgaacaaggacgttaacgatttgcataacccgattgaatgggtggagaaagcaatacgggataactgaacgtatttataaatcggattgaatgaacgcttgacatgtcgtgtcaggcgtcgtattctttgcacatggtcagcgtagctatatcgtaaagcaacgtgacacccttaaatgggcacgtagggtagccgggtcgttcccggccgttgaccgcccaacagcaaaggaacgatgccatgcaaactttcaagcaacgtcttagccgcttcttcaaatcgtatacgacgcttgatcttcgtaccgacgacgaaacgcgtaaggttcgctgtgaaaagtttgagcgtaagaacaagacgtgtggcaagcggtccgtattcaccattagcgaggattgaacaatgcgacatggaagcgacccgtcgcagggtggagaatttacgatttgcggtattgcatttgacgcttttgattcgggagacgttgacgaaccaacaaggtttgcgagtcccggcgagacaatcacttgccccgaatgccgcaaagtaatcgcctatttcaaaagcattagacattggaaggaaccttgcaatgaaagttaaagttaaaacttggcatggcacacgcgaaacgttcttgtcgtatgctttgacgccgtatattgacgcatatgaatgtgacggccgctctgaaagtatggaacgcttgacgcaaaagactgccgaagcgttcggtcgtttggctgaactgttggttgaaaagggcgtcatatcgcttgaagaagcggtgtcagcgtcaggcgttagtcacgaagtcgaagcgttggacgaacccaagcaagattaaccgttcagaaaaatagtcttgactgtcgtagagctttatcgtattctatagttgttccagcaaggaactaaccgagtacagcaaatgaagaacgttaacgtcgaatacttctacgaaggcgcatacggagacggtacgcatttcgtagcaatgaaagaaaccgacggttctaaaacgatcctgctgcgcgaagtgtgcaggtctgtagctggcgaaaccgccaacggtctgaacgcaggatggctgaaaggcaattacacagcagggaaagacgattacgtagacttgtgcgttggaatgatgcacgggatttcggtagatcgtagcgatccgaactaattaacgaagcccggtcagcaatggccgggctttaggagtgaatgctatgcgcaagtccgaactagaacgcgcgttgaacaggctgcgcagtgcgcgcgacgcatcgaactggcaagggaagttcacggccgaaattaggcaggcaaccgtgacgcatcgcattgaagaaatagccaaaccgattgaagaagttatcggtttggttcaaaaagcgcttgacaagcgcaatcgaaggccgcatcatagacacgctgcaacaccgcagcgactaccgtataaggatgattagccatgtgcatcgcatgtaagaatcgtgaaatgatggtcgatgttcagtcgcaagtgctggaaacgaccgccgcattggtcgaagcattccagttgatcgaaaagatcaagggcaaggccatgtcacttgacgccgaagaacaaaaggtgtatgaccgcctttcgcgcttcgtcaagcaggaagccccggacaccaccgaacagggcgtgtcggcgaatggccttgaagttcgcatcgtggaagttggttcggccgaagaattcgccgacttgcttgccacgttgcagaaccgcaagccgcgcggcaacactcactaacatcaataacgaacaggggaattaccgtggctgacgaaatcgacgtaaccaatgaccgcgttgaaaatgaaaccgcattgttggttgcagacgtttcacgtaaggccgccgctatcccgactggacagccgggcgattgcttctattgtggggagcatttcgcccgtgttgtttacgtcgagtccgtaggcgaagaatgttgcggcgggtgccgcgataaaaggggcttggaatgaacggcaaggaatgggcaggcatgacctgcaacgaattggcgtcttgtgtcaacgcattgaatgttcgcgttgttcagttgcagcgagccaagcaacgcgataagctgccggaactgcaaaggcagttgcacgaaatgcgcgtcgaattgaagcgcaagcaggacgctgaaaagcgggcgaagcacaatgaagcccgctgacctagctaaaagcggaaccgaaagcggccaccagcgggccgttttcgcatgggcggcgttgcacattacgcaatggcctgagctacgttggctgcatcacataccgaacggcggtgcgcgaggcgacgacgaaaagacgcgcgccattcgcggtaatgcgttgaaggccgaaggcgtaaaggttggcgtagctgatttgtttttgccagtgaagcgcggcgaatacagcggcctttacattgaaatgaagaagcccggcaagatcaaaaccacgtcgaaagagcaaaaggaattcggcgagtttgtcaaggcgcaaggcttcggctggatcgtgtgcgacaactgggaagatgcagttaaggtcttgcaggagtatctatcatggcaatgaacattgatccaaaggtcatgcttgaagaaatccgcgcaaatcaagcgttgcttgacggatgcaagcagcatcattttccaacttggccgttgaacataagcggccatttagggttgaaggtggattgttgcaactgcggcggaactatggacgcacgcatggccgcatcgtacacgcgcggattcaaagcagcgggcggcgatcccaacaagatcataccgggatgggacaaatgaagtgcgtacgttgtgagatagcgcgggctaagattcgcgctatcttctatttcaatatgggccttagcccggaagcactggccgtagaccttagcggccgctacgaaggtgaatatttcgttaggcgcaatgaacacggggccgcagtctatcgtcgtaacgacaacccaatcgcacccgcaattgagatttggtttttctgacgaaaagtagttgacaagcgaaaaacagcgtcgtattctattcccacactaagacgaagggacgccgtaatgtcatttgaagtcgaaatcaagactcttggcattccttgcatagctcgcgggagcgtaaccgagtcagaccgttctgtcggtatcatgtcggaaggcttggaagacgttacgcttcataacgtaaagaacgaaagccggttgaattggcttgaatccaagcttgacaagctagataaatggcaggatacttacgacgcaatttgggaagcgctttctaaacagcgcgaagaatacgaacgttcgcgctacgattactaaggagaaaggatcatggccgcactgttttggattattgcagcacttgctatcgccaacgctgtgcgcctgattcgtaacaaggcgcgtaccgatgacgtgcaagcccgtttgaactacgaacgccacgttgctgatatgcgccgcaattcttaccgtgaaccgccgcagcgcgcaggccatcgccgcgacaacgaatttaagtggggccgcgaatgaagttgcttttaataggcgacgaaagtacaatcaacgtcgcagcactggacgccgttagaagaaagcttaacggcgaaattgaaatcatcgattacaaaacagaggaaagtgtcatgcacaatcgtcgcaatgttcttgtttccgccctgtctgcactggccggtggccttggcgcaggtgccgccgcactcaccgacgttgcagttgccaacagcaacatgctgtcgtcgttttcccagcgctacggcaacaacccgcgcagcctgaacggctcgcatcttctgaacagcaatgccgcagcacaaaagcgcgcagcgaagaagcgtcgcaacgtgcgggccaagtcgagtaagcgcgcgtgaaggtccggcaggctgtcggactaatcgcgatcctcacggcattcattgttgtggggatcatggataagcaagacgccgaacttgaacagcagcgttattgcaacaatgttcgtgacggcgtttggccggactatgaacccggccgttacaagcttgaatgcggcggtaagaacccgccaaagttccacgaagatttaacgaaatagttgttgacacgcctgccgaaacctgtagtattcaaatcctgcattccgcagaactcacctagctaggagaaacgaacatggcccgtaagcccgccccgaagtcgaagaccgcatctttcgacctgtccgccgttatcgccgctaccaacgccggtagtttcgtgtatacttcccgcgaagcgcacgccagcgcgcttgaagatgggcttgtcgaagtcaacgagtccatgaccaatgaagcgggtgaactggcaacccgcgccaccaccaagggcatcgaaagcatgaacgcagcgcagaacacccagcaggccgctccggccagcaccccggccgcaaagccgtccttccagatcgaagacggcatcgcactggcccccgtgaccggtcgcggtcgtggcggcgaaacctacccgttcgacctgctgcaagtcggccagtcgttcttcgttccgaacagcgacgacaagccgaacgttgccaagtcgctggcttccaccgtttccagcgcaacccgtcgttatgccgaagaaatccccggcgaaacccgcgttgatcgcaagggcaacaccgttccggccatcaaggaaacccgcaagttcgtcgttcgtgccgtcgaaggcggcgcacgcgtctggcgcaccgcgtaagccggccgcagccgcgcgctgcgccccgctgacaggaaaccccggcttcggccggggtttttctttgcctgcgccctgtgcgcgtgtatagtgccgggaattggggccaccggaacaggcaaagtgagcgaaaacgacatgaatgttgacccgcaacaattcgccgtgttgattgaccgggtgaacaacttgttgacggactctaaagaaatgcgcggccaattgggaaacattcaactctcccttgctcgcattgaacaagtccccgctgaaatggccgcattgcgcatccaagtcgaatcgcaagccaagacaattgcaaatcattcattagtcataaagatttgcgggacggttttggcgctgtgcgtcggcttgattggttggggctggacggaagctaaaggcttctatgctcgcgaccaagacgccgaccgccgcctttatttgattgaattcaagttaggcttgccagccgcacccgtcgaaggatcatcgaaatgaaacagaccgttgaaaaggttgtcgtgccgaactggcgcgaagtcaagaaacgttggtccgttcgactcggcgtaatcggcacgctgattaccggctttgctgtcgcggttcctgacgtggcgttacaggtttgggttgcaatgccgatggatttaaaggcagcgcttccgcctgattttgtcaagtggtttggtttgggactgttgatcgcgggccaagccgccacgttcatccgccaaaggaagaagccgcaatgaaaagcatttacgtttcagccggtcacagcaacgacgatcccggcgcagtagccttcggccgcaaagaagctgacattgcggttgaattccgtaacatggtttcgttctatttgcaacgggcaaacgttccgcacgaactggatggaagcggtacacaaaacctgccgttgcgtcaagctgcggccgctgcaaagcgccatccgattgcggttgaattccactgcaatgcaggcccggccactgcaaccggcgttgaaacgctgtcagggccgaaagacatggcgttaggcggtcgtatcgcgcaggcgatttctgacgcgctggtgatccgtaatcgtggtgcaaagcccgaagcatcgggccagcacagccggttggcatttgtccagtccggcggcatcatcgttgaagtgctgttcatcacaagcgcaaacgatcttgcgtcgtacgacgctcgcaagtggcttgcggccaaggccgtggccgacgtgcttattgacgcggcgggcaagccgtgattagcgcatggctggcaaagaaaggggctgaattgtgggcatggctggcggccatcggcgcagcggcgttagttgtcttcggattctatcagaacgccaagcgcaaaggcgaattgaacgcgaagcaagaacacgccgaagccgaagttaagcgcattgacggcgaagccgtgcgccgtgtcgaagcagcccaaacgcaggccgcacacgaagtcgaaactatcaaaggcgcaaaggatgaaaccgacaaagttaatcgtcttagcgacgacgatgttactcgcaagctgcatgacgactgggcgcgggattgatcgaatacctgaaacggtcgtcgtagacactgcctgtaaatgggtaacaccgatttacataagcaagaccgaagacgttttatcacccgaaacagcccggcaaatacttgcccacaatgaagcatggcggcgtaattgcggcgctgcttccaaataatcagacggccggttatagtctccgcatggacactatcccggccgtttctgttgacgaagaacagcgcttaaagctggcatttgctaatgcgctgttgaagcatccgcaagaccttgaaggcaggtttgcggcggccctgtcggttacttccgatactggtaaagcccttgtcatggcgaacaagtggcttgatgatccttttgttgtcgcagaacaaacgcgtttgcttaaaggtgctgacgaaggcgatttgaacttcattggcactaaggctgattttgcacgcgaactgttaaccgaagcccgcgcgcaatgggacggcgaaacgaagattaagttcttcaagctttatgccgaagtgcgaggctttattgcaaagccggatacgaacgttaacgttcaagtcaataacaaccgcgtcatggttgttaaggacatgggaactgacgacgattgggaacgcaaagcgcaacagcaacagcggaatttgattgatgttagcgcatcccgacactgaaaccgaagcgcaaccgtttgaggttatttggcaaccactgcccggaacttcgcaagaacttgcgattgattcccggtgccatcataccctgtacgaaggtgcgcgcggtcccggcaaaactttaacgcagttaatgcgttttcgtcgccgcgttggtattggttacggccaatattggcgcggcgttatctttgatttggagtttgaccatttagcaggtttggtcgccgaatcaaagaaatggtttaagaagtttggcgatggggctgttttccttgaatctccgtcgcaatacaaatgggtttggccgactggcgaagaactgctatttcgtcacgtaaaaaagattgcggattacgaaggcttccacggtcacgaatacccgtttcttggttggaacgaattaaccaagcacgcaaccgacgcactttataacaagttcatgtcggtcaatcgttcgacgtttgaccccgaacgagacacgccgaaagacccgaagaccggccgctatttgacgccgaacggtttaccgttgccgccgattccgttggaagtgttcagcacgaccaacccggccggtccggggcacaactgggttaaggatcgtttcattgatccggcaccgcgcgggactgtcgtacgaaccgaagtcgaggtattcaatcctcagacgcaagaaaacgataaagtcattcgcacgcaagttgcgatcttcggttcgtatcgtgaaaacaaatatcttccgccggaatatgttgctgaacttgaatccatcaccgacgaaaacttgcgcaaggcttggctgtacggcgattgggacgttgtagccggtgacgctttcggcgacgtatgggacaagaaatatcatgtcgtgccgcgcttcgttattccagcaggttggaatattgaccggtcgtttgactggggtagttcgcacccgttcagtgtgggttggtgggccgaagcaaacggtgaagaagctaaggttattatcggcgatcaagtatttactttctgtccgcagccgggttcgttaattcagttctttgaatactacggaactgaaaagatcggaacgaataaaggcttgaaaaagccagccggtgaaatcgcagagaaaattagggaaattgaaactgcgttaatgttcaatggctggatcaaatcgcagccttggcccggtccagccgataaccaaattcgcgatgttcgcgaaagcgatgttgacacgattgaaaagaaaatgcagaagttcggcattaactgggaagaatcggataagtcgccgggttcgcgtaaaaacggaatggaattgttccgcgaacgattgtcgaatgcgaagaaaggtgaaggcccagcggtttactttatggaaaactgccgtgctagtattagcctaattccaaagcttccgcgcgatccgatcaagattgacgacgtagacactacgaccgaagatcactgttgggacatgacacgctatcgtgttttaaagggcagtcatcgtgtcgcccgttcaattaaagtttcaatgcctacttaaaaggttacgcaaatgaccgcagccattcgccgcactgttgttggaaatccgaacgttgcgttcattcggcctgaattagcaaggctgttgccgcaatacgaattgatccgtgattgcatcgcgggcgaaacggtaatcaaagaccggcgaatgaagtatttgccgatgcctaacgcgtcggacaagtcgccggaaaaccgcgcacgttacgaagcctaccttttacgcgcagtgttttacaacgttacgcgtcgaactgtcatgggcttgattggtcaagttttcggacaagacccggccgtaaagcttccatcggttcttgacccgatgattgccaacgcaaccggtacaggaactagcttgaatcagcttgccgaaatcagcttaggccacaacatcgcgtattcgcgaagcggcctgttcgttgatttccctgatacttcggcgcaaggcggcgcaagcgcagcccaagttgaagcgggcgaaatccgcccgacaatgtacgcgtattcgccgcttgaaattatcaactggcgagtaaccgagcgcggcgcaaacgaagtgctttcgctcgtcgttttgcttgaaggctatccggtttcagacgatggctttgaaatcaagaatgcgccgcagttccgcgttttgaagcttgatgacgcaggtaactacgttcaagaaatttggaaggaacctgacccgaataaatgggacggctttagcgttccgaagaaaggcaacttccagctttcgcataccattaagccgactggcccggatggcaagccgctgcgcgaaattccgttttggtttatcggtagtcaaaacaacgacgttaacccggataacccgaacatgtacgatatggcgtctttgaatatcgcgcattatcgcaacagcgctgattacgaagaatcgtgctacgtcgtaggacagcccacaccggttgcaactggcttaaccgaagaatgggttaagaacgtacttggcggccaattggcgttcggttcgcgcggcggcattccgttgcccgtaggagctacggccgaactgttgcaagccgaagccaacacgatgattaaagaagctatggacaccaaggaacgtcagatgacggcccttggcgcaaagcttgttgaacagcgtgaagtgcagcgtaccgcaaccgaatcttcgcaggacaaggccgctgaaaattccgttcttacgtcgagtgcaaacaacgtaagcgaagcgtaccgttctgcgttggcatacgccgcaatgttgatgggtgcggaaggcgcagaaatcgaatacgccttaaacattgattttgaaattgcagcgcttacgcctgagcaagttcgtatggctattgaagcgtggcaaaagggcgccattacttgggccgaaatgcgcgccgatcttcgccgctatggtctggctacggaagacgacgaagaagctaagaagaagattgccgacgaacaggttgaagcaatgacgctgcttgccgaaaatgacccgcaatataaccaaaacgacaacggcggcaacccgcctgcgtccgcttaatgtgggcatctgacaatggcacttaccgaaaccggccgtctgtttgatataacgacacgcttggcgctgtttgttgaaaacgtcaagcttggtcaaatgcaagaattcggcgcagttcttgcagtagtcgaagaagacttgcgaaagatatttagtcgagtcaaatacaggactttagacggattgagcaaggctgaattaaataggctgttgcttgcaatgcgaaagtcgcaacttcgcgtttatagcgcttacaccgaaaagcttatcaagacgttgcaggattttatgcaaattcgtcttgacgttagcgccgtggcttatgccacggttaggcatcaatttgcaactgggtctgacgaagaactaagcgaagaccaatcttacgaatacattgaagaacagaacagcattttgccgttcgcagcgctatttggtttatctgccattttacctagtggcagcaaatcgctttggtcttcgatcaagaacgcaccgattccagcaaacggcttgtatctgcttcccttcatttcaacgttttcgcggtctgcgcaagccagcgttgaaaatacaattcgacgtgcttatgcgaatcgtcagagcgttgacgctacgttgcttgaactgttcgcgcctaaaactgcgcaaggtttttcgtctcagtttgccaagcttcgtaatcaagctaacgcggttattgaaacgtcgtttgcacacgttgaccaaatcagcgcggccgctattagttcggcgatctattcgcgctatatgtggatttcggttattgatagtcagacgacgcagttttgtattgaacacgataaaaacatttatcgttacggggaagggccaattccgccagcgcattacaaatgtcgcagcacaaccgtacccctcgcatcacagtttgatgacttttcaccgccgacgttatatgcttggttcaagcggcaacctaaagcagtaatcgcgcagttcgttggcgataaggttgcaggcttgatagattcggggcaaatgtcttcaaaggagtttgcatccgttgttgtaggaaaaccgcttgaccttaatcaattcaagtcgaaaactggcttgatcctttcaacctgattcggtgaatcagtaggagtcgaagacatggcacttgcacgcaaaatcacgaaagaaaagttcgacagtctgccggacaatatcaaatttgaatacgccgccgatggcgacagctttacgctgcaaaccaccggcgatgaagacgttggcgcgttgaagcgcgcaaacgcacgcttgaaggatcaagtgacgacgttggaaaattccaatgacgatcttgccggaaagttggaaaagatcaatacgaaccccgcgcgaaagcagggcgacattgacgcgcttgaacgtcaatgggcgaaagataaagacgacgccgttgcggaagttgcgggcaagcttgaaaaggcaaacggtttcatcaaaacgacgttgcttgaaaacgctgcggcgtctcttgctagcaaggttagcactgcaccgggcgtcattcgtccccacattgaacgccgcttgacggttgacatggatggcgatgcgccggttgtcaaggtgctggacgcgcagggcaaggtgtcgaatctgacgcttgacaagctgggcgaagaatttgttgcaaacaaggatttttcgtctatcatccgcgtaacaaaagcgtccggcggtgccggttcgccttccagtaacggcggtgccgtcaaaccttcccccgcgcagcagccgggcgaacaaccgccgaacatggcttcaatgaatccgcgcgagttggcggaacagttgaaggcaagaaaggccgaacaatcacccaccgagtaaggacgcgccaacatggcactttctgatttagccgtttacagcgaatacgcgtattcgtcgtttaccgaagttctgcaacagcagttgaacctgttcaacgctgcgtctggcggaaccattgtcctgcaatcggccgcgcatcaaggcgatttcagcgacgttgctttcttcgcaaagatcgcaggcggcgttgtccgtcgtcgtaacgcctacggttcgggcgctgtcagcgaaaagagcttgaagcatcttgttgacacgatggtcaagattgcggcgggcacgccgccgattcgcattgatccgggtcagttccgttggattcagcagaacccggaagtcgcgggcgtcgcactgggccagcagcttgccgtcgatactctcgccgacatgctgaacacttcgctcggcgcaaccgtcgcagcactgtccggcgttccggccgtggttcacgacattaccggcgcaactgccccggacgatcaaatgtcgtttatcgcacaaaccgatgcgtcggcgaagttcggtgacatgtccagccgcattcaagcttgggttatgcacagcaagcccatgcaccagctttacaagaatgcgttgacgaacaacgagcgtcttttcacctacggcagcgtcaacgtcgtgcgtgatccgttcggccgcgtttacgtgatgaccgactcgccgaatcttgttgccgctggcacccccaacgtttacaacacgttgggccttgtgccgggcgcaatcatggtggatcagaacaacgacttcgacgccaacgaagaaacaaagaacggcgacgaaaacatcatccgcacgtatcaagcggaatggtcgtatgaactgggcatcatgggcttcgcttgggacaaggcgaatggcggcaagtcgccgaacgatgccgcaatcctgcaaggcacgaactgggaccgctattccacgtctgaaaaggacttggctggcgtcctgttgaagacccactaagcgcaacgcttagtgacgtagccggggccattgcggccccggcttttcaacacgaaccgataaggcaaccacaatgaaagtaccgaagattctttttttcgttgacggcatggcaccgaccgcagccgatgttgaagcggccagcgaaatcaacgcgcatgtcgttttccgcaatgctcgcgcagttccggctgacggttcgcttgaagcttgtgacggcgtagcaggcaaggttcccgccccgtatagcaagcttccgaccgccgcacaggccatcaagacgcacgccacaaaggtgcgcgaaatgaacgcaacggccaacaacgacgccgcaggtaagccggtgaagccgaaccccgcaccggccgacaagggccgtgcgcccgcgcaggctggcaaggacgacgtgtcgaaagacgaaggccagtccaccccgccgccggccgaccttgacgccgcgaaggccgcagcgccggggcacgcaccggaaggcgcaaccggcgcggcttggaagtcgaacaactaagccgttgaacggggcggcgtaaaacccgccccgtttttctatcggtattcaacgcaggaatcgcgacaatggccgcaaagaacaaagtaatttatttcaccgcaggcgacgtagcaactaccgctgaaaaggcggacattcaaaagttgaacgaactggcagtgtcgccgtatgacgttggcgttcgcagtgccgttcgtcccatgtcgtcgggcggtccgcttgaagctgcggattatgtggccggaacgattccgactgcatacgaagacgtgccggtcattgaccccgataacccgcctgaaatcgtgttgccgccgaccaagcttatcgtaacgaacggcgataccgcacaagtcaccacgcttgacggaaccgcaacgtatgctgacgcaacgattgtcgttgcaaacagcgcgatcacccggttgcaacttccggcaaacaccaccacgaacacgaccggcggctatatgggcgtgaacgatcaaggtggcgtcgctgcggatggaaccgcgaacgtgtttgcaaacggaacttgcaacgctgttcttgaagccacggcttgcatcgtaaagaacgccgcagaggtaacagtcggcggcaacaagtacacctttgaagtttcgggcggtgccattcgcggcatcaccgttaccccggcagcgtaaggctacaaaatggctattgaaatcatcgtcgaagatggaagcggcatcgctaacgctaattcatacgtcacggttgacgaagtgcggcagtatgccgcgcagcgcggcgtgtcgcttccatccgacgatgatgcagttgcatccatgattatcaaggcgaccgattatttagaatcgtttgcttgcaagtatcaaggccgcaagactgattgcgagcaatcattgcaatggccgcgaaccggtgtcgtcatgtgctgcgacgattacccgtcgaacgcgatccccaagcaattgaaatctgcgcaagcttcggccgtcctgattcaaaatgaaggcttagttctgcaaccgaacgtaaccgcagcggattacgtcattgaagaaactgtcgggccaatcacaaccaaatatgcgaacccgattcaagctggcatttcagcgacgttcacggcgcttgattcgctgcttaatccgctgttctacgcatcatgtgggcaggcattcgcgcttcgtactgtaagggtttaatcatggcgcgctttgaccgacaaattgcaaccgcgcttcgtttgattcaaaagaacggccagcttgttaagtggcggcaattgcaacgcgaagacgatccgaataaccctgctgctgtcattgaaaacgatccggtagaccacgacgtttatatttgctttcttccggtcaataaagatactaaagagtttatcgcgtatcttcgcggaaccaatgacgttaaaattggttcggtaatcggcttaatgggcaatgtttcttttacgcctgacgcagcagactacgtattgcgcgacggcgtaactcttgaaattttgaacatcgacttgctttcgccgaacgggcaaaagattctttatacagtagagtttaagggatgaccgtcgaattcgaccaagcagttgcggaaatggaagtaatatttaacacggcttggcaagccaatgccggtgctgtgtttggatacattccgcaaattgtgtggaacggtaaagaagcgagtaccaaagtagatcgcacgaaagtatgggtcaggttttcaacgcagaacgttaccgaagaacaggcgacgctatcaacctgcgtagataaaccatacgttcgccgctggaatggtgcaggcttaatcttcgtccaattgttcttgcccaagacgattgcgaatgctttaatcaaagggcgtacgctggcgaaggttgcaagaaacgcgtaccggggcaaaaagtcagacggtggcgttacgttccacaatgtacgtatcaacgacgggcttgaccccgaagaactgttttatcgcatcaacgttgtcgccgaatacgattacgacgaactaggctaggagatattcacatggtttgcgaagttgtcaagattgattccaacatcactggccttagcatcgccgaagaagtttgcttaaagcagcttcccgttttggcggttgatggctttgaccccacatggtacggtcaggaaccgaatagctattcggattttggcggcgacctgaccaccgttgcacgcgcgccgattgatccgtcgcgccagaacaagaaaggaaccgttaccgatcttgatgcaagcggtggttacaacaccgattttaccaagtcgaacatgacgcgcattctgcaaggcttcttcttcgcagacgcgcgcgaacccgcatcgactgttccgatgaacggcccgcgtatcgccatcactggcgtaacggctgctgataagacttacaccattgcaagcggtggaaccaacttcgcagcgggccaattgattttggccgcaggttttgcgaacgccgcaaacaacggtttgaagcgcgtcaccgcatcgaccgcaacgaccgtcgttgttgcggaaactgtcgttgacgaagccgctcccccggccggtgccaagttccagcgcgttggcggcgaactgattgcgggcgatgtttccttcgcagttgttgacggcattccgtcgcttgtttcgacaaccaccgactttagcaccttcccgaacttgtttgcgggcaagtggctgttcatcggtggcgacgctaccgcaaaccgcttcgtcaacaatgtgggctttgctcgcatcaaagctgtgtctgcgaattcgatcacgtttgacgacacgacttgggcaccggttaacgaagctggcaccggtaaaagcattcgcttcttcgccggtatttcgatcaagaacgaaaagcttgctgctttaatcaagcgccgttcgtatcaaatcgaacgcacgttgggcgaaggcccggaagctgaaaaccccggcgatcaacaggccgaatatttgatcggtgcagtttgcaatgaactgaccgtcaacattccgcaggccgacaagatcaacgcggatttgactttcgttgcgtgcgacaacacctatcgcagcggtgcggcgggtgacgaaaacaaaatcaaatcgtcaacccttggaaccttggtttctgcgccgggcgaagatgctttcaatacttcgtctgacatttaccggatcaagatggcgattgttgatccgtcaacgtctgcgccttcgccgctgtttggttttgtttccgaagcgaacgtttcgattaacaacggcgttacgccgaacaaggctgttggcgtgttgggtgctttcgataccagcgctgcgaacttcactgtcggcggttcgattacggcttacttcacttcggttgccgctgtgaaggctgtccgcgccaatgctgacgttggcctttcgatcatcgctgcgtcgaagaacgccggtttcattttcgacattccgttgctcggtttgggtggcggtcgtatcaacgttgaaaaggatgcgccgattaccgttccgcttgaaccggccggtgctgaaaacccgaacggctataccatgctgtttgaatcgttcgtcttcctgccgaacgtcgcaatgccgggttaatgtagcccggccgcattaaacgcgatacactggaaaggccgggattgccccggccttttccttaacttaaaaggtgaatacaaaatgggcctttccagtcaatacaagaccgacaccgaccgcgaaaccaacggcgttgaaatcgaagtcggcgacgtgaacaaagacggaagctatccgacgtttgttctcgcacgcgcgagcaagaccaacaaggtttatcaggccgcgcttaccaaggctgccgcaccgtttcaacgtcagattcagttgaagattgacgtttccgcccagcttgaaaaagctttcatggacgtgttttgcgataccgttttgcgcggttggtcgaacgttccgaaggccgatatgaccggcgtggcgagcgacgagggctatatcgaattcaacaagcagaacgcaaaggcactgtttgaacgtctgccggaactctacgatttcctgcaagaacaggccagttcggcaagcctgttccttgaagcgacgcgcgaggaatccgcaaaaaactgacggaagttttagagtatttgcttgaaatggggccgcacgaacagtccattgccaagcaagctatccgggcaggtcaaccaatacccgcccggatagcaaatgctcctgaacttcacatcggtctagaactgttcttgaatgcgttttttgatttagacacggaacgccaagcaggcttttctatcggccctataccgtggagcaagattaaagactattcgcaggcttattcgttcgatagcgatttgaccgaagacttgtttttcttcgttaaagctttggacaatgcccacatgaaacggcttgaaaaggaatctaaagccaaaaggtgaagtgatggcccgctcgctacttgatttagcaaatgacattgacaagctcggcggtgaaatttcgcaagctgctagcgaccatgcagttaagacggcgctaaccattgtcggcgacttggtttatcacacaccggttgatacatcgcaagccctgtcgaactgggacgttacgataggggcaccgatggacgatccgcacggcccatacgtcgccggtaagcacggttcgacacagcaacaaagcgccgcacaagctttaaacgttgcaaaagaaacgttgaagaacaaaaagcccggcgaagtcatctacattgcaaacaaccttccgtatattcgccgtttgaatgacgggtattcggaacaagttccggcaggctttatcgaacgcgccattttacttgggcgtaaaacgaaagctaagttcaagcttaggaaataaacatgtctgaccagcctgttgtaattgaagtaaaagacagtgttgacaaaaacatttcgcgtaacctgtctgaaatttcaagtcaggcacgcagcgcttatcagaatgttgaaaagcttgttcgtcagcttaaccgcgtaaagcctaccgcaatcgcgcagtttagcagcgtcgtaagcaacgccgaacgccaaatgcaacaggcggccatttcggcgcaacgtcttgcaaccgaacaggccaagaccgccactgcggccgcgcaggcggcccagcagcaggcacgcgccgcccaagctaccctctcccttgaagctgcgcagaaacgcgcggcagacgccagcgcacgcgttgcagcggcggccaaggcggaagctgccgccgcccagcaggcggccggggcggaacaggcccgtgcggatcgcattcgcaacatggttcaagagtctatccgcaaagcggaagcattgaaaaacgaaacgtcagaacgttggaagcttgaacaagccgaatcggcgggcgcacgcgttgcgaatgatgcagcttcggccgaatcgcgtttgcgtgcaagcgtcgaagcgaccgcaaaggcgaccgccgaccaacgtagaatggttgcagaacttaacgctacgttagaccgtggcgttaaaagcattgaagaaatgtaccgcgccgaagacctgttagaccgggctatggcgaagggtgcaatttcggcggaccagcaaagcgcagcccttgaacggctcaattcgcaaatgcgtatgctggggcaagataaagaagttgaacgcattagcggcattcacgaccgctttaatgcggtgcttgctcgcaacccgaaatatcaacagaactttacgaagggcttagaagaaaccgctaagaagtcgggtttagctcgccacgaattgcagaatctcgcgtaccaagttaacgacgttgttgtgtcgttaggttctggccaaaagccgatgcaagtgttcttgcaacagggtgcgcaaattggccaaatcttcggcacgtccggcgtaggcgctggcgcaatcttgcgtcagttaggcggcatcgtcgcgcgtttaattccgccgctgttagctttcgccgctgtcatcggtgttgtgaccgcgccctttgcgctgtttactcgcgaatttaacaagggcgttgattccaaaaagcttgttgacggcttaaagcttaccgaagatcaattgaagaaattgaagaagtcgggcgaagaaacgcgcgtgaccttcggcgatacgtttaaagccaccttccaagttatcggccagtatgctacgcagtattttaagcctgtgacagaatgggtcgtcaagtggtggaacaaggcgctcgatttcatcaccacggccttttcagtgtgggtacgcatccaactcggcatgtggctttcgttcgctaacgtaatcaaggccgtttggaaggacattcccgccgccgttgaagctgctgcaaagggcgcagcaaacggcgcaatttccatcattgagtttgcaatcaaccaaatcagcaaagcagttgcagatagtccgctcggtaagctgctcggcatgagtgggccggttgaaatcaagttgccgcgtcttgaacttagcgcagatgctaagaacatgcaaagcgacgttaaagacgcaatcgttaacggttacaagcaggctgacacaatcgttaccaagttcggtaacgacgttcgcgcgcaagcgttgaagaacgcgcaagaccgcttgaaagctgcggcaggcgaagacgacagcaagggtaagaagtcgcgaggctttgaccgcgccaaggaacttgcgcaaatcaacgcagaacttgattcgcaagctaagaacatgtttgttctggctacggcgcgcgatgcagctaaccgcgcggatgaaattgcattgcgttttgctaaggaaggccagccgctacgcgaagaagaaattgattcgctgcgtaagaaaattcaggcgttgaatgacgccaaggaagttcaaacgcaatttgaccgcatctatcaaaacgccaccggcccgctgcgcgaatacaacgcttcgcttgctgcggctgacaagcttgtaaagatgggcgcaatttcgcaggcgcagtatgttgcggaagtgaaccgggcgaaagaagctttcgcgtcggcttccgatccgttgcacgatatgaacaaggaacttgacgaacaaatcaagctgcttggcatgttgggtccgcaacgtgaagttgaacaacaagttctgcaagccatgaacaaggcattgcaggaaggcaagccgctgcgcgatgacgaaattaaagcgctgcgtgaaaagttgaagcttgtgcagcagttgaacattgtttcatcaatgcgcgatgaactgcaacaaggtagtcaagcgcaacgttcggtcaacactgcgacccgcacgcaaactgcaatcggtgaagtcggcaacaacggcttcactgggggcgacgctatcagtgcgttggcgcaagaaaacccggcgcttgaagcgacgcgcgaattccagcagcaaactattgcgtcgtatacggatatgtacgcgcaaattgatgcgcttcgccaagccgacttgattagcgaaacgtcggcgattcaagcgcgaatggaactgttccagcagcagtattctaagcaaattgaaggcgcaaccactgcgcttggcgctttagcaacgctgcaaaattcgcagaacaaaaagcaagctgcaatcggcaagaaagcggcaattgcacagactttgattcaaacctatcaaagtgcgaccgcagcgttcagcgcaatggcaggcattccgtacgtcggtccgttcttgggcgcggccgctgcggctgcggccattgcggcaggtatggcaaacgtccagcaaatccgcgcacagaacgcaggcttcaaggaaggcggctatacgggtaatatccccacaaactcaatcgctggccctgtgcatggtaaagaatacgtgttcgacgcaccggcaaccgcacgcattggcgtcggcaaccttgaagcgctgcgacgcggccgtatcccggttgattcgcttggcaccggtcaaagcggcgcagtaaccgacgcttcgccgacccctacccgtgtgggcagcgatcagattaactacaaccaaaccgtcaacgttaccgtcgcgggcaagcgtgatcgtcgcaccgctgaacaggaagcgcgggcgattcgcacgcaatcgacgcgcgaacttattaggagtggtggctaatgggtcacattaacgcagttttagacgaacaggttgattacggttttgaaggcggtcccgaatacgccaacgaaatcgtagaccttgaaaacggctacgaatacattgatagcgcatgggcgtatccgcgccataggtattcggcaagcttcggcaatattactgacgaagaccgcgactatatcattgcagcgtttcacgcttgcaagggtcgtcgtcactatttcaagttcaaagactggaacgattttcttgcagttgatgaacccttgcaggtcgaagcgggcaccacgaagccggttcaactttacaaaacctatcaaccgaaagacccagttaccggcgtagcttggcccgcttggaccgtgcgaccaatccaagcaataaaaagcgccgtcatcaaaacgccgggcggaaacgcggttgccggaacgctcgacactgaaacgggcatgtttacaccgtctgctaattgggccagcggcacgcatacgtggtccggcgagttttacgtttgggttcgtttcgacgcggactataacagcatgaccattaacagttggcgtgcgaataccgcaaaggtcgaattgatggaaggtaagcgccttattactgcaaccaatatgccggatagctgggaagaataatgcctaagcaaattccaattgcgctgcaacttcaattcggcaagcccggaacttcgacgtgctttcttattaagatcgtcactaaagaagacggcatttttgcgttcaccaccgcagattttgtcgtaaggttcaacgacggccttggcgaagtatcgtatttgccggacgaagaattgcggccgcaaaacattcagtcgtcggccgacatgacggttgacaataccaaactgctcggttggtttaaagaagcagttgaacgcaaggttatttcaggtgcgttcgattctgccgaaatcaccatttatcgcgtgtcgtatttgcgtcttgcttacggctacgaagtcgtaggctacggcacagttggcgaaattgattacaacagtgacggcaagagcaagcgcggtgttgaattccgcagtttgacgcagcagttgaccgtaaacacaaaccaatattacagcctgacatgccgggcgcagtttggcgattccaagtgccaaatgccgcttatttggttcgcaggaacagtgcagcttataccgaacgaaaacgcacagcttgttttcaaagttaccggcatttcgcaaccggcgggttactttgaattgggcgtaatccatttcgatagcggcgacaacgaaggcgcagactgggaaattgaaagctgggccgcagacggcacagtgaagcttagttatctttccccgtatcctgtagcgaacggcactgcggttcggctacgcaaagactgcggcaaaaccgaaactgattgcatgtcatacggcaacatagttaatatgcgggctgaacacctgaccccgaccgaagatcaatctttgatggtgccgggcgcatacattaaatcgcagaacgcgctatgaccgacattgcggaacgtgcaagggctttaaaagacgtaccgtttgtgcatcaaggacggaacgaaaacggaattgattgcgtcggcttaatggcttacgcaattcaatttccgttcgaccaaatcccgccgtaccctcgcgatccgtacaacagcgaacttgaaaacgcaatgcaagcggccttcgggccgcctttgctgttgaaacctacgattgaccaattgcaggaaggcgacctagcggcgatgcaatatcgcggcccaatccgtcatgtgggcatcgtgcttaatcatccgacgcttcccggtgtgctgtctttaattcacaccgattcaatggttggaaaagttaccgagcatatattagatgcgaaatggctacgtcgcattgaaaaagtctggcgtttaggttaatacgaaatggcaggcttattcggttcaatcacaatcaaaggaaatcggcttacggagtttgcatcgcaaacttcgacagtcggtattcctatgcctttcggctttggtaagttcccgtgcgaaggcaacattatctttgcgccgatgccgccgaaggaacatgtaaagaaaaagaaacaaggtaaaggcggcgttaaaaccgaagaatacagctacacgctttcgtatgccattgcgttctgcgaaggcccgatcttcggctattggacgatcaaacgaaacggcaaaattgtttggacgcaagaccctagcgcatcggttgatgatcgcgcttacgcggccaaatgggcaagaaaggcgacgttctattacggcactgaaacgcaattgccagattcaacgattgaatcgtataaaggtgctggcaaggtttctgcacatcgcggcgttgcgtacatcgtagttgaagacgatgacgttacagacaacggcggcgcagtacccacatacgaagccgttatcatcgcttcgccgcctgacgcatatttgacttcgcggccgtatccgaacgacatggcccccgaatcggtgcaaatgggcttgggtcttagcgcgggcgaactgcggccgctgctgtttgaagaacattacaccgaatcggttgaccttgcgctaacgcttggttttggcgattttagaacgccaatcgttccttacaatgttcttgctgaaagcataagcaatgatattgcgcttggcgccggtaggctttacgatccaattaggccgtataatgtgccacaagaaagcattaacctttcggcggacattccatatggctggctacgtgttgcgcttgtgaactatgaccggtatccgccggaatccgttaatatgtctgcgtctcttggcgaaggtactttaggaccgtaaatatgaacatgatgaaaaagcccgaaccacttcttttagaatgcggtattgccggttactttacgtttgaagctttcaaacaagatgctgacggcaatgaaattgcgggtacgcgccgcaaggttgctgaattcaaaaatttgattaccaacaccgggcttaactgcttactcagcaaggacataagcggtagaaacacctacggttacaactgcgcaattggaagcggcaatcagaccccgacggttacagataccgccctgcaatcgttccttgtgtatgttggtcaagggactagcggtaattccggtaagccttacgacttgcaaactagcggttacgcggcggattcttcgtatacgtggcggcgctgggtgtttcgttttgccgatggtctggcggcctataacaacattcaagaagtcggcatatttgcggcaggtatggcaagcagtcccacccgtccgaacattatgtgttcgcgcgcgcttattctcgattcgggcggcaaccctacttcgattgcaattcagcctgacgaaacgttagacatttattatgaaattcggtattacccgccagccgaagtaacgggatcgattacgcttaacggcgtgagttacgattacaacattcgtccaatcgattttctgcctgcgcaatacaacgcgtggcaaacaggcacgggtgacactggcggtatgaccgcacttgacactagcattatgggtcaacagcgatggtcaagctattaccaaacatcggtgttcgcttccccggtgcaaacgctgtacccgaaggaacaaaatgcgtcggccatttggggtaacgtcgaaaacgcccagtcgtggacgctgaaaccctacgttgacaatagctttactcgcaccggaactatcctgttcaacttgccgcagggtaacgtgccgggtggcgtaggtagcttatttatttccgctggccttggcggctataaaatcacgtttaccaacgccaaagtacctaagacgaaccaatttaagtggtcacaagacgtaatctttaccgtggcccggagataattaaatgctgcccgataacggccagttgtctaccaccgcgttcgttagtgcgttcgttgacccggtaaaaacacccggtgacttcttaattgattacgaacgtggcggcatcgcgttaaacgatccttcgcaggggttgttagttcagctatggacgctaaaagttgaacgcgatccggttgtaataacgcagtggaatttttatgttgaatcccctgcgaacggtagacaatttctgtttgcggcggccaacgttaaagaagcgtctttgtcgtttgaccaaaacatgcgcccgtttgtagtttacttggaaaataccaccactaaaatgtggtggtacgatccgacgattccgggccagactatcacgacccttggcaccgatcttcgcacgccgcgttgcacaatggacgaacggcgcgaatggcatacggcgatttctgacattgttttaggttacgttcgcgcgggcaacctgtgcgttcgttatcagcgcgaacgttatcaaaccgaacacgttttaaagccggttggttcgacggccgagcttgtctgtgtgggcatcaatgctggcggacgtttgcaattccgatgccgcaaagttactgcgcttgatagtcagttcgctgttaacgttgacccattcttagcggacattgttttagcgctttgtgttcgtgctggaatcaaccccgaagccgtagacgtgcgcgaactttacgacgctaacgttatcggttacaagctgaacaccgatgacggagttaacaagcgcatcgatgcgttgcgtgaaatgttcttcttcgacaaagccgaagccgataagaagctagcgtttactcgacgcgggcgaccggttgttgttcgtattccgtatcgcgatcttgttgcggatgatccatcggcgcttgaacaaacacgtctgcaagaaaaggaactcgcccgttctgtgtcggtcaatcaccttgacccggctggcggctttgctacgaataagcaaaccgcacgccgtcgcagtaacatcatcaaggcaaagaaagaccaaacggttgaaagcgaagttgttttaaccgcagaccaagcaatgacagcggcgtcaatcaagcttaaaattgcttggcatgaattgcagacttttaagtttgcaacaacgttgaagtacgcgcaagttgtttcaactgacgttgtggaagtcgaagacaagcgcggcaattggtatcgcgtgcgtatcaccgaacgcaacgacaatcacccgatcattaagtttgaaggcgtacaggacgcagggcaggacgtatacgcaacgcttggcgtaggccagtcgttgccgcctcctacttcgacaacgccgggcttggtcggtgaaacaacgcttgaaatcttgaacattcccacattgcgcgatcaagacgatgaattaggcgtctatattgcagtggcgggcgcttcgtcagcgtggtacggatcgcaaatccttatcagcactgacggcggtgttaacttctacgaagccatgcaaattgaaacgcctgcaactttgggtgaaacgctaactgatattaaagacgaaatcagcgcggaatatccagccaaccaaagctttgaagtgctggtaaactttgcgcttgaatcggtcacgtatgaaaacctgttgaacaacgtcaatcgttgtgttgtcggcgatgaattgatgcaatttcaatttgcggttctgcttggtatggttgacgggcattaccgctaccgtctcagcggattggttcgcggtcgttacgcaacttccgttgaagattggccgacaggaacccgctttgttttacttgattcaagtatcgcgtttttgcaggcgcaacaatggatgcttggtcaagaaatccaaatcaagccggtcagtcttggccttaccgaagacgaaacagttgcaaccgggtatgactatcttgaaggcgtgtcgcaacgcgaattcccggtgcatagcgttaccgcagtgcgcgacggctcaaacaacgtcactgtcacatttgttggacgcgggcggcttggcattgaaacggcaccgcgtaacggtaagtatttcgctggctatcgcattaagttcagcaatggcaatgtgattgacacgcagaacatgaccgcagtttataacagcgccccggcaggcattacggttcaagtttgcgctttgaacaccgtaaccggcgaagggccgtattccaccgcaattagcacgtaagggccgaaaatgtcaacaccgaatgcaaaccttcccgaaatgccgcagaacagttttcagccgtctgtgccattcaaccaagcaatgcagaccatcgacgcgttgttgcccttggccgtcgaatctatggccctcaccgcgccgcccagcacgggcacaggcgacgcgggcaagcgctggatacctgcggccggggctaccggggcatgggccgggaaggccggtcaggtggcgctgtgtacgggggtcggcttgtgggtgttcatcctgccaccgccttacatcgttgcgtacaacattgcggacggtatcgaatacaggaacatggccgggacttggaccgctgttccttaaaagaacagcggttgttgtttctttggcttaaagccgatcttttctaaagtgtcttcggcttgatctacgtaccaattgtaatcaatatccgaaggaaacttagggggcaaatccatcaagggtttagccccctcactttttggaacggcgttgccagtggcaatgtaacgaatttgcccgttaatgtcctgcgcgtaataccaacgaataatcttgccgataaaaacgccgtctttttctgcgccgccgttaaccttgcgcaccgtagtaaatctgcgaatatcgcggcaggcttcgattgtttcgcgcacaggcttgccgctagttattgcatgaacaactgcgtcgctgcaaatcaaatgttcggcgttcttagacaacacgctgttaagcgcgctgcctacttcggcatacgatcctttgatttttacgcccagcctatccgacagcaacttagcgccttcgtcgcctttttcctttactgcaaaatagttgttaacgtcacggcaatacaaagctttgtagcgggtttcttccgtttcaaatcctgtaatctgttcccacattgcaatgatcgcgttaagttcgtcgtagcggtcaaccgggcatttaattacgatgccgtctgtattgccggacacgacgggtatgccgtggtgctggatcatttcaattagcattaacagtgcaagctgcccggtaatggttacttgcaaaagcagcttgggcgaatacagcaatgaatacaggttgccgaacttgccgaaaccaccgttaatggtgatcttcaatgcgttggcaattgtcttgttgcctgcctttttagcggccagacgcttgttaactagcgcttcgtaaacctgcaagaacgcttcgcctaagtgcttagggtaaagacgttcgtttaggataattcgcgggtagtagcttgcaacgtcacgatcaattagcaacgtgtcagccgtcgctacgtgtgcaacgttctgttcggacgaatgcaggccgcccatgccaagcttataaactgactggccgatgcgggcttttaatacccaagtgtatccgcttttcgtcttttctttttcgcccagcccttccggccacataggcgaaccgttgccgtcaagcgggaatgtggccgcttcgatccggtcaacgatgcttcgcaattctggcgacacgtagccaatccagtgcggcgcttcgtactttacgtttaaaacgttagtcttaggctttgacggatacttaccggtaagcttggttagctcgcttgcaattacggcttctgcaatctgcgcatcggaacggctgcgaaggtcttggttgtattccttgcctagagtttcgcgaagcttgatttctggcaacagttccttatacaaaagaatggtgttgtcgtcatcgttgatattgtaatacttgacaatatcggcttcttcttcgtcaaggtgccgggtgtgttcaaatggtaaatcttgcagccttgcggcctgcatacgtgcggcgtacagctttagcgacccttcaagcggggccacttcgatcaaatcaatttggtttagtaagtcaaacggtacgcggaaaccgaattctttttgtgcttcgcgcggccacatgccatcgccgatcattgcgttggaaagcgctttaagctttgcgcaatcgaagccctgtgctgcggcaaaaaccatgttcacgtcgtatgcaagattgttgaaaccaaccgtgcaaaacttaaacatcatccatcgcagttcttcgccgtcaaaatcagaacgcggcgaacgctcaaaataaacaaccttgccagtttcagggcacttgaacgatacgcaaaagaagttcgggtaacattcaacgtcgtagatcattggcgagccgacaggcatacgcgccaattcttcgccagtgaattcaacgaatgggcgaagggttaatgtcggccgggcaagcgtgctaaggtcaatccctttggatttgcctttagccatacgacgtgtaaattcctcgctgtcgaagaacattacgaacgaacccccattagcataccgcgcgaattatcgccaaagaacaccgctttgcccggttcggtttcaaaatcaacttgcttgaaaatcggttcaacgatagacaagtaatccatgttaaacgcaagacctttgtgcaaaccttcgatttcaaacgaacctgcttggttcttttgcgcgtcctttaccgaaaatccactttcatcgaaatacgcgattttgtcatccgacaaagactgaatcttgcggataccgtcaaagaagccttgcggaagcggccaagggttgacctgctgcggaaacagtgcggcatagtccgggtaagcttccgaataaagctgcgtcttaataaagctgtcgtcttcaaagaagaatgttgccgagttttgcgagaaaccaaaacgcgcaagcttcttagccgtcttcgtcacagcttgcaatgacgccttcggaataagcaaaccgggcggcaaatcgatgccgtgccaatgctctatcagaacgtgaccgtttgtgcccacaatggacccgctttgcagcagcgcgcttgcaaagatcggacgcggtgcggtttcgttcaacaacggcgcgattaaatcgaaccctgctttcaaacgatcatcaatcgttgcgcacggtgaatcgggttcaatcatcggcacttcgccgaacggtatgcactgaatgaatgctttgaacgcacctgacttaatggaaagtcggccgctatcaagctgcgtaatcgacagggtttcgccgcacttgcctaacgcgtcaagcagcctaatcgtatgtgggcacgccgataaatcatcctcgactaaatgcccggttgcgaatatgccgttgaacgccatagctcgcccgctgctaacgacgcaatgcgtttgcactggcgtgccttccttttgctgcgccaatgcaatgaactttaacgcctcaattaaagacgccgcgccattggcggcatctttgggcttgcgtgcgcgtcgcgcgcctgcggtcttagccattgctttgattcccgtgttgattccacatacgttcttcttcaagctgcacacgcagcttttcgttttcttcgtacgctgtatctaaagcctgctgaatttcgcagtcgtcaaacttgcggctgtcgtcatcattgaagcggcgagcatagcaggaattgcaccagcaaatgttattcatggctttagcctcagaacggaatatcaaactcatggtctttgcagccgctaacgataatatgcggtggcggcatagctgcaaatttatcgcaaccttcttcgcctgcgcttgtgttattgcgatgccaatgcaaacagttaacgcaagtcatccagcggtgggcctttactgcaccgtcttgaattgctatgacaagttcgttttcatcgtcattgcgcaacttgctgttcatcacgtccttaaaactcatggcctaaaatctccgggtattttttattgacatgaacgcgaatctttgaaggtacgcgcgacttatggacggacaacaaagcttcgtacgttgacggcggtggttccgttcccattcgttgccgccaccagtcccgcgcccgctttcctgccattcccgagtgttcaagcaaaatccattcgttaaacatgtgcagaccgcaaatgtacgaaactttgatcgaaggcggcgacagcaattcgccagccgcgccgcgcttttcatgcaggttgtaaagcacacggctaacgttgaaatattcaacctgcggtgcatccgacttcattacttcttgcgttgcggcgcttctaacaagcttggtattgaacgtaaattctgttccgcagttgcagcaaaacctaaccttcgtgtggttgtatgcaccgcagttttcgcaaatgcgaaccggggcgtcaccgccgccctgacccggcttgcgcggaatcaccgggtcattgatagggccaagcctacgcgtattgcccgcgaagtctaaaactaggcagttgtccttttgagggaagaagccatcgccgccgaacggacgcgtaccacggccaagcatctgcacccataaaccgggcgatgccgtggcgcgcaacatgctaattaaatcaatcgggggatgatcgaagccggttgtatacttacccatgttgaccaagcagcgaatttcgccacgcttgaatgcttcaacacgcttatcgttttcgttgccgggcagtttgctatggcttgcgaccgctgtaatgccgaagctttgcagcatcgcggcaacatgttcggcgtgttcaacgctgtttgcgaaggtcaaccacgaagcgcggttatagcctagctccgccatttctttgcaagccgcccatgtgatttcgtccttgtcgctaacttcgttaagcgccttgcgattgaaatctccgccagaaagaccgacgttcgacacgtcaatttcaatgttagttcgctttggaattagcggcgaaataaagccttccgcaaccaaacgattgaatgattcgtaatcggtaatgtcatagcaaatgtcggtgaaaatgccaccgtccgtaatcatgccctgcttcattcggaacggcgttgcagtgaagccaatgactttcataaaaggattcatcgccaacagttcggcaatgattacctgatacatcgtgtcatcgttcggcgaaagcaaatggcattcgtcaatcaacagcagatcgatgcggccaaactggcgaatgacattcttgacgctagcgacaccgccgaacgtaagtggcaacatcaaatcgcgacgcttcaatccggcgctataaatacccagtggtgcagtcggccaaacctgcatcactttctttgcgttctgttcgatcaactctttaacgtgcgtcagcatcataatgcgctgaccgggccagtatcgataaaccctgcgaaggaagttcgcgattacgacgcttttgcccgtacccgtgggcatggcaacgaccgggtttccccggccgccacggtcgaaatagtcgaaaattgattgctccgcttcggcttgataccaacgcgcctcaaaatcaactggcgcaatcatcgaactattttcaaacattacacaatagccttgtaatcagggcatccggttggaattacttgcttcggtatcgggccattcgtcgggctatgcaccgcacagtgccattgcgcgttttcgattggcgttgcgtgaatgcagcttcggcagttgcgttcaacaggttcgccaccgtggcaaatgctgcgcatgtcgcaatatccgcattcgctatacgttgggctttccgaaagctttggcggcggagtctgcgaattgattatgctttcagcctttaaaatcatttgttggcctgtcgcatgatctagctttgcaacttcaacatgcaaatcgtcatcgttcttgcatatggaaaaatacaagacgtagcgaaacccgtacttcaagccgtacgttgaagtttgcgcaaaatgctcttgcttttcaacaggcatcttgttttctttcaacttgacaaacttgtgtccggttccgtgcgttttgaattcaagcaataccggttcgtcaataccccagtgcggcggcaagacggcaatgccgtcgagcgatccgccgaagtggccgtttacgtcgctaatacggtattgcggaaattccaacccgtcagcttttgcacgggcaacgtgacgcaaatattcggggttgctttcgagtatcggtgtgcaaagcgcatccggcatttcgccatcaactgcgataccgtacgcgtcgctttctgcgtggtagtaaaagccttcgcggttttcaaaccaaactttgatgccgataccttcaagccattcaacgaagcgggcttcttcacgatgcccacgattgaacaggcgttgcttgcgtccgtctgtcgcggcgcgtagacaccagcggaaaacgtaccaaaggtaacgtttgcagttacgaccgatcaacgaagcgcctaaatgcgttcggtggccgccgtcatacgtttgcacgcaatacgcatcaatctccttcaaaaccctcgctgcaattttgttcgccacgccgggcgcgtctaaagaaagggtttggaccttcgatccgctttccgttgtggtagcggtttcgcttttctcgttcagcccgtttatttcgttttgcatcttttttgtccttccggcgttgaaccactttggcggtgttgtcgaattccaagcctttgcattgttcgatcacatattgcaactgttcgacgttcatttgcgatatgtgacatttttcatgcggtatgttcagatgccttgcgagcatctgatacgcgtcggttcttgacattccgccggatttccaaagcgggtcaaaatgcctatgcgcttccgcacgcagttgccgtgttttcttgtcagccatccggccaagtggaatgcgtgtgttcggatggcatccaactgctgcgccgcatcctgaacagaaatagcaaaacggccagtcgccgaaaggtctaccgtatagcgcttcgttcccaacaaacgcaatatcaaacgacgcgcagttgtcgcattgttccggtattggtaatgggtttttaacccggtctgacatgcggctttcccctgttagaaatacggccggattttcacccggccgtattggtcacacgttgtttactgcgacgctcttagcgctgaccccaggacggctgctgcggcgcaccgccgttgccctgctgctggccctgctgccagccgccaccctgcggtgcctgctgctgggggttctgctgcggcggctgctgctggggctgctggccctgctggccctgctggccccaacccccggcctgcggctgctgctggccctgcggtgcgccaccgccctgaccacctgcaccccatgcacccgcgccgccctgctggggctgctgttgcggtgcttgctgctgcggctgctgctgattgaagccgccgttctgctgctgaccgccgaagccttgcggctgctgatcgaccgaaccgccctttttcggttcgttgccgttcatgtcaaacacgcgcttgacttcggtgtagcccttcgcgtccgggttggtcgggctgggttcttcacccttttgatagccgacttcgacaacaaacgggcgaccaaacagcggggtaatgtccgtgccgttgttcggcagtgcgaacacctgcaagacgtggcaaatcgccgacagttgcttgtgtgcgatttcagcagccttcgccgactgattgtagagattcaggcgatacgcgcccttgaatccggcggacggaccctcagtgataacgcagttcagttgcagatagccgctgctgttgtcctgcgtcgcttttacttcggccgattcgatcacaaccgggtgcttgccgagcggccaagtaccgccgccctgtgccgggtcgtaatccaacgggttgaaaccgttcaaaagctgtaccattttcgtcacctttgcaaagtgtgccttcgtttaatacggccgaaagctttgccgttttggtgccccgtgtcggaatcgaaccgacatgccttgcggcaacggattttaagtccggtgcgtctaccaatttcgccaacggggcgtgtcttagttctgcatcaccttggcaatcaacgccgtcaaatccggcggttccagttcgttaaacaaaccgggattgcttgtgcgaatgcgagccataatgtcggaagtaccgaacgtgcgaattgcaagcgtcggtttgatgatgccgggaatctgtgcccttgcgacatgcaagattgaatcgaaaagatgcggcatctttacgttcaggtcttgaccggggaaataaggtttgcgcttcttcattccgccttcgtcaatgacggtttctttgcaaatcaaatacatgtgcttttcgcgcatgtaatagagtttgtgcgccgtttcattgaccgtttcagccatgacgccgtaagctttaagcccgtgcgtattcttttcaagcgcgcgcttcaacacgatttcggcgtattgcgaaaagctatcgacacacgcagtatcgaagttcttagcttcgtgcgaagaatttaaccacgtaaagaattcggcgcagcgctccggcgtgtcgccttcccatgcggcgacgttgtgtgcgttgcgcatcgacaacatgccgggttcacacaccagcattacgggccggggggcggtcataatcaacggcgttttgccttcgccgggcggaccgtaggccagcgctttgaagccgtagttctttgcgaagcttgatgcgggcttcaagtctttcatttgcattatgattgctccacgaagcggcctgcaattttggccgtgatcttgacttcaacgccattcggcggtgttacgtaaagctgctgcccgcgctgcttgacttcaacaacgcatttccattccgaccaatagtagttgcccggcttgcttggaattcgtgcgttcatgctgtgcccctttagtctttagaataaatcctaacgaactcattctaaagattaaatgcgatgccgccgttaagcgacggcatcgcggcctgattgtgaacggtcgccagatttcaagttaaggcatacgcgcttaatttgcccttgaaacccggcgttctacatcgctcggtccatgtgggcacgcgtgccccggcgttttgggctgcgattggctgggccttgtcaaagcgttcggcaacaaaacgccccaaggcaaacagcaccgcagcgatcaacaaaattagaatcatttttacttcttcgacttcggttcgatgatttccagcgtcggcgcaccttcggtcgtttcaataacgccgtcaatgatcgacttgaccttgcggccgatttccgtttcagtcaacgccttgtattcggtcaacgacaggtcagccgaccacttaacaagacgatcccccatgaacgttgcttcggggccaagcgcttcaatctgcgtaagcgctgcgtcaactgcgtcaacaaccttgacgttttcgtcacgcgaaacgaacttgaag

SEQ ID NO: 4 - DNA, 45433 bp, unidentified
  source 1..45433: mol_type = genomic DNA
ccttcaggctttgcgctggtgtaaccgcctgttttgaatctacttgacttcccagcacctacgagcggttggggaatcaaccccagcgccgccaaggtcattacggcgtcaatcgtctcgcgttgatggggctttagcttattgctcattcggcacgctcgcaacggtaggttttggctttcaatgcagcttccaggctttcgccagtggcaaggcagatgatgccttgctcacgatcatactgcacataggtttgcggcgcaatgccctgccacattgcgagattggtcggcttcagtctctttgcttcagccctggcttgatacagttcgtgaccgacaattgcaccggcaacaaccgcaccggcaaacagggtcacaagcacggccagccaaatacgatccttcattgcttgcgctcccaagtgttgccgccaatgtcttcgtagatttcacctacgttcattgtttgaacgcgctcaaaagtggattcctgaatgtcgtgcgtcgacaagacgctttcccaaacagtaacactcttcccgttggcgagtttaacctgccatcgtttttcgttagccattgcctgtgccctgctgtgtggattactaacagcttatacgatgggtggttgcttgtcaacaagcggtttagtaaatcgcgaagcgtaagcacgaacagccataagcgactttgcgcttatggaacctttgcccgtcataattgcgttaaaagcagccttgctaattccaacgtattcataaaacgctttctgcgttttgtaaaactgaagctgccgcctgaacagctttgcgatggcttccagcccaattgagctaacatgccctgcgtttttcattacggcaccccgaagcgaaagcgcagcgtgccattgctcggcacatgctcagtttcaatgcgaacattgccgccgaagtggccttcgttaagctcggccaagtattcaaggcttgttttgcggtccgctgcatccgcatagaactcgacttcgatgttgacgaaaccgggttcgtcgggaatggcgttgtcaagcatttcaagcaactctttcttgttcattcgccttccccttcgaccaggacatagacgtagctttccgtttcaacgcgagtcaaacaagcgcccgcaccgaaatcaatactcttcaattgcccaatgcaacagggatgaccgtcaataacaagagacgccaaaggctcaccgttatacgaagaaaacatgtgccctctactaaagcgaagaatagttttcattgctcagcccttgatcggataggttacgacgcactgcccagcttcgaatgcgttacggcactgttcgcccagaacgcgacgctgcttagcgtcatcatggttcatatcgtaaacacgataagccaaatcgccaacatcaacgctcgcgtcactcataagcgttacggttgcgtcattcatcgcctgaatgctggcccaaatttcaacacgaattttcatgccttgctcctgtgctgcccacattgatgcaggcggttagcggccgtctacgttgcccagggttgccgggctgcgaagatcgttagccgggtcgaattcaacaatgatggttccaccgcagcacccgcaagaagctacttcgaatccgtgcttgttgaacaacgcggcaagctcttcgcgaaacgctttctctttgtcgctaatcatttcaggctcccggccgtttgactgtgattgttacttgcctagcttccagcacttcccaggaattgggattgcttagcatgttctttgcaagcttagcggcctgctcttggctctctgccagaacggaagaaaatattgcaaggttcgtacagccacgaagcctaagcgttacgtcatagaagtaacgccttgtagtgaatgcttcgccaattgaaaacggcttatcgttagccattacgcaagcctcgcgacttcgacaaggcccaggtcatcatgcttgatgaacttgaacactttgccggtgcccacgttggcacgctcacgggtgttacgttgcgacacacaggttcgcagcgacttccaattgacttcggcaatgttggccgtgaacgacttgcctacttccagcgtatcgaacggatactttgcgccagtgttttcaatggcctttgctgcttcgactgcggccgggctgctgtccctgatttcaaacgtcatgttgcttgcctcgcgtgaatgtaaggccatcattgcacgttaaatgcaaggtgtcaagcgcttaattatacgttacatagccgttatacagatataagggatcgtagaatgcctaagtcattgaaatatatacatatataataaatataataaatataatggtaaaagcttcttttatgtgtgtaaggtttaatgtgtataatttacacgcttacacgttacacccaccctggaaacaccccggaccgttatatttgttatatttgctatattccctttgaaatcaatcacttgcgtgctatacggccattaaacttcactatactttaacaattcctaccgttcgtcgggtcgtagagccgaaggcattgacagatcgtaatcgtccatcgtaatctagacacacaccacaacacacaggacacgccatcatgcaaagcttcaagttccgcttgtcgaagatcgcccgcaccgtcagcacgatggacctgcgcaagactgccgaacagcagcgcgcggaagagattgcaaccaaggcccgtcgtttcgaatcgcgcaacaagactgctggcaagcgttcgtcgtttcctgtgtccactgaatgggagcttgtctaatggcaacctacacaatcaaaacgacgacgttcaacattcgcggcgaagtgatgcagatttgggttcaggacgtgagcgaagacgacagcgtaaagaatgcgtcgcgtcgttggacggccagggcagcacgctatatggattgcggccttatcgcattcttcaagctggaagtcgtcattaacgtgggcaaggacaatgaagcacggaactgacccagggcaaggcagcgagttcacaatttgcggcatcgcatttgacgcgcatgactctggcgactatgaccgcacgattgaatttgcgcagccgggggaagttatcacctgtcccgaatgtcgcaaagtcattgcatatttcaaaagcatcaagcattggaaggaaccaatctaatggctaacaagcaatgtcagtattgcaagcgcaacgggtttcattgggtcgtaatcagtacaggcaaatggcggttagcagataggttcggaatcctgcacacctgcaccgaagctggggaagcctaccgactcgcccggcgcacgccacgccctttgcccaggttcgccgctaggtcagggtcagcccaggtcacggcggggcgtgtgccgcccggcgtgaggcagcagcccagggcagaaccggcaccgatgcccacactagaatcgccaggattcaagctgacgccgtgcatgattgcgattagcgaaggccggtcgaaatatagcccggctgaagctgcgacggatacgcgccggttcaacgatatggatgttttcccgctggttacgaccggccccgagtttcaattcattggagtatagaaaatgcaaccaaccaagttccgaaagaagcccgttgtaattgaggcgatgcgttggattggcaccgccaccgaagcatcacccgtaattgattgggtgcttagccagggcgggacggctcgctatcacgacgaagaaaccgcttggggtggtggcgtcgtacattccgaagagcatattgcaataaacacgcttgaaggaaccgttaaggcgtcggccggtgactggatcattcgcggcgttgctggtgaattctacccgtgcaagcctgacatattcgggcagacatacgaaactacatcgcagtgaaaaacaaaacccggcgaaagccgggtttttcgtttatacctttgcgtatttctttagcggtgtgagttgccacccgtattcaattgctccctgcaagcgcagttccagggcatcgaattcgtcaagcttcattccttcaatgaacgcgtcgatatgctggggagcaatcggatactttttgttcatcatggttacggcgctacgattggcgatgccgagcattgctgacaggtcataagttaacgtcatccgatggaatgcaagatgttcgcgcatgatatgccgcacggtacgaacagtgtcgctcggcgttacgatcctgcgcccgcctagaaccggttgcgtcttgcgatagttgataactggcttgctcacaggtcgaacgcctttgggttgctaatcatgtatgcgactgaacttgtcttgtatttcgttgacaggtctttgcgcgatactagctgaatgtcgcctcgctcttcaagagtcttcagcgcgcgcttaattgcgttggttgcgccaagcttatccttacggaagattgcgacagagactagcttacgctgaaggaacgaatacgggatgattcgttcgctatgcaggttcgccattccgttgacatacttttcaacttcactaaacggcgacagaatgtagctgcggacgttatgcactacagtctgaagctgctttgtttcgtcgttgtcgatgccaatttcgcctgcatcgaacttgccgaggatattgcgcacgtcggccacgacaaggttaatcgcccaggtcgcagcctcactatcaattgtggggtgatacgggtcgttgcctacggccaacactgcggccagcttcattgcacgcagatgggcacggttccaaaggtggcggcgaatctcgcggtcggccgtgttgatattggcatcgcaatgcttatcgaaatcacggaacatcctatcggcgttgtcatcaagcgcaacgtcgataacacggttgttcgaattcaactgcatcgcgaaagcgcaaagggttgcgagcttgtcaacgagttcgtcggaaggcttaaccatgccgcgattttcgttgttttcaacacgcgggccgttgtattcaattatcgtaaatcggggcaacaagccttcgctaatcatgctttcgttaagcacgtcgtaaaagcgttccggcgtgctttcgcctacgacggtaaacgccggggacagaacggagcgagtgtttttgtcgcggtcgctgtaaaccatcgggcgaactacgttgccaaagcctgacttgttgaacaggtcaagcaatgatcgacgcaagccaaccaaatgcggcggcgcatgttcggcgcacatgttgcggaagtaaaggccgaattcgccaaccagggacaagcacgacggcgtaattgcaagttgtttaatcaaagcaggcgacgacgaaatttcgccagggccaatgaattcgcttgcggtcggcacgctcacgccaacagcgctcattagcttttcaatgccgcttgcgatggcttctttgcctgtgcctgtcggagccagcaaaagcagataggaattcagcccggttccgctgacgttgtaagctcgccctatgatgccggacataaggcccagcgctgcgacgatggcaatttcggcaacaggtcgcggtgcttgggcgtagacgaattttgcgatttcgccagtcaagccgggaggaaccgaatagatgctcttttgcggtttcaactcgccaacttgaacaggctcggcctgtgtctttacaatgtccgcctgcttgcgggattgcatgtattcctctagcagattttgcagaccgtcaatgtctacaggcggcaacatcctatcgaagcagcgcgcgagcatgtattcaatgcggtattgcgcgcgcgatttttcgcgctcggcaagcttcgaccgtaggaacaggttttgaacctgccaacggttttcgctatagaacgcgatgatattgaccagggcgaaatcggcttccgattgcgacgggtagtatttctgccagttgccttcatagaacagatcagaaaacttttcgccgttggcagcttcagccgccatcttcaaaacttcttcgtcgctgaacttgatttcgtttgcgcccgcatagaatacggccgcttctttaccctttgacatttccttgtgcagcacttgcaacaagtcgtgccgttcggcaatcggtgcattgcgatgaacattgccggtcatcgtcataaagcgaacgttcgaatagacttcgatgcagctacgacgacggccgcaaggaacttggcctttcacaattacgtgcaagcctttgccggatggcgagaattccgaatagctgttgaattcgttgaacacttctttctgaagctcaaacgctttgcgctgtgcttcttcaccacgaacgccggacgtatcgctaaatacgtcatcaaggtcaatcatggtataggggtcgtgctcgctaagcacgaatccaataccgctgtattgcccgctgttcaaacaggcaacggccgtgtcgtagtccgcccaggtttcaggcttgctcacgtcagcgcgtttgtgacttctaggcgagtaaggaactttcgttggcttcgggccgtcgcggtcttcataccgccacatgacccaatgcggataggtccgcatttcgtttggaatgttatcaagcattacgcgcccttacttgatgccaagattgtctaggcattctttgattgccatcactttgttaaatgacgggtcagcaatttcggatcgggagaacgagccaacccaacgcacgccaaggccagccgatgcggcaagctcttcaatggaaatggtgcagggtctacggcgaatcctggctattgtctcaatcaaaatggggtgcgctttgtcggtgacggccattggatcgcatcatgtgggcattaggatgccgtgaaggctaccccttcaagattctgtcgtcaagatacagaatgttgttgacagcccacatggacgggcgtagggtgacggtcccggcccatcaccgggctatcacaggcagaacaccacatgaccgacgcaaaaccgccgttccactatcaggccgaagccgccgtaacgctttcaaacaacttccacggtggagcaatccccgcgaggctgttgcgcaacgttctggaatggctgattcagaacggcaaccatgccgacgaactgaagaaagcaatcttctacggccgcgacctgcaagaatatgaacgctatgccgacgaaccgaattgcatgttcatcggcgaaaagatttgccctggcgatgccgtcaggggcgaaacgatctttcacgcaatcatcggcaagatcaccgaagccaccgaacttggcgaactgctttatggcgttctgttcaaggataaggaatttgacgctaccaatttcgttgaagaaattggcgacggcctttggtacgatgcggccgggcttagtgccgtcggaatgacgtttgacgaagctcagcgaatcaacatcgcaaagctgcgcaagcgcttccctgacaagttcaacgaattcgacgcgaacaaccgcgacctgttcggcgagcgcgtaattttggaagagcgcacttcgaagcgcgttggcgtaattgaagaagttaacatttctcgcgttttcggcatcgacaagccccaggcttgacagtgctgaaaagctgtgcttgaataaccccgtcacaacagccaacaggccgaacatgaacgaaatcaagtattacaaagatagcgggatgaccgaagaagagcttgcagcgctcgacaaggaagacccgcgattcattcgctaccgcaacgaaatccttgcggattgggagcaggcaaagaaagaccttgacgccgccaaggaaaccgaaatggaacttcgcaagaagttcgtcgcggttgccacccaggccgacaagatcagcggaaccgaaaacgttgaccttggcaatggctacaaagccaagaccgtcaaaaaggtcaactacaagcttgggtcaaatgtcgaaggcgtttcggctcgcgatgctgttgatgcagccttgcagaaaatcgaagcgctcggcgacgaaggccgttttatcgccgaccggctggtgaagtggaccgcagacctttcggtgtcggaatacaaggcgcttgatgaacacccgcgcggtgcagaaatcaaggcgttgttgtccccggttctgaccatcgacagcggcgctccgacgcttgaaatcatcgcgccgaaggcgaagaagtaagcaatacggctgcgccttcgggcgcagtctttgaagtggcttgttcgaagacggtaaacgttgccagctaggcagttcgtaaacggtcgagcgagccacttcaaagactaccaagcgaggattacaatggaaccgcaaccttttccccaggctaacaaaacgtggaaggctccgcccggaatggaaaactgcgtcgatcttgaaactttcagcgacggcgaagtgatcgtttcgcattggaaaatgacgtggcgggaacgattctctgcgttgttcttcggccgtgtttggcattacgcatggtgcgcaaggcccgccccggtcggcattatggttcgcaaaagcattttcccgaaggaataagcaatggcacagaacttcggcaattcaaagctgcggcccgcatcttccttcgcactggcgaacggctataaagccatcgtttacggtccgccaggggaaggcaagacgccgctgattaaaacgaccatcaacccggttctgttgatttgtgagccgggcatgggttcgatgcgcgatgcccacaatatccccgcatgggacggcttgacgatggccggggcagacgagttcttcaagtggctgttcaactcggcggaagcgaagaagttcgatacgtgctgcgtcgattcgttttcgcaatacgctgagcttgtgcttgcttactacctgaagaagcattcgcacggcctgaaggcttacggcgcaatgtctgaacacgtaatggacgtggcgaataagctgttttacatgccgcagaaacacatgtatttgatttgcaaggaaagcgggcgcgaagagcaaggcattagcaagcgagttccgttcttcccagggcaagacctgaacgtaaagatgccgcatttgttcgatgcaattttgcgtgttgcacgaaccacagtaatggggcaaaatggcaaggtgcttgccattcaaacgcgcggcgatgatgttatggcccgcgaccggttcggcaagctggacgaatttgaaccgccgcatttcggcaatcttgttcgcaaggcgttgtcgtaaaagttttggggaagaagctcggttcgattccggcacaagggcacgcccgccaatctcgggcggttagtttataggctaaaacgtccccgcccaacggtgaactttgccgccgtataaaggcaaagacttttcgaaaagtcaaaggtaaaaacaatgtccaacaattcgcattttctgactgaagcgtttgacccgacccaggtcgacccgacccagggtagcggcggctggccgctgggccgtcatccggtcgtcgcaaccggtgttgaagtcaaggcaaccaaagacggaaacaacggcatggcttcgttcaccctggaagtgatcgacgggccggaaaagggctacaagggtttttggaacctgaacctgtatcacgaaagcgaaaaggctcgcaattttgcgcgtcgcgacctgtccgcaatgtgccacgcaacgcagacgttccgccttggcgcgcagggaacggacctgtcgcagttgttcaacaagcctttcgtcgtggacgttggctatcagcgcggccacaacccggcgaccgatggcgaagacgccaagggctacaccgaaatcaaaaagctgtacgacattcacggtaacgagccgggcaagtcgggccagggcggcggacaggctccgcagcagaacaaccagcagacgcagaaccagggcggcaacggcggtggttggggcaacaacaattccaacgcaaaccagggccagaacaacggcggcaactcgggcggcggctggggaaacggccaggggcagaacaacgccaacagcaacgacagcaaccagggttcgcaggacaacagccagcagggtcagggcggtggcggttggaattcgaacggcaacaacgccaataacggcggcaacaacgaccagggcaataccggcggtaacggtggcggcaatggtggttggcagcagggccagggcggcaacggcggcaatggtggcccgtcgtggggccagcgcaactaagctgcctgcaacatcggcaaacaacatggcggcgtaatgccgccatgtttttaataggacaaggcgatgaacgataacgtaaagaagattgaacttggcgcacccggcgtagctcgcgcgctggaaaagcgaatcgctgaagcaattgacagctattgccaaacagcttacgacgacggccaccgcaaccatttgggcgcgtcccttatcggcggagactgccgccgtaagctgttttacattttccgttgggtcaagcaccacattcacagcggccgtatgcaacgcctgttcaatcgcggccatcgcgaagaagaacgtttcattgaatggcttgaaggcatcggcttcaaagtgtggttcgaaaaccgcgaaggcttctattatcacggtggcagcgaaacttacggcattttgcagcccggcgaagaactgcgccttgattgcgatctaattacggaagacaacgagtattaccgtacccatgtgggtatggcaaaagctcagggcttgaaattcccgcaataccgcgtaagcgacgtaatgggccactttggcggctccctggacggcattgcaattcttccgcccgaatggggaatcgaagagcctgttttggtcgagttcaagaccaacggcaccggttcaagcttcaacaagcttgtcgaaaagggcatggcaaaagctaagccacagcattatgcgcagactggcgtttacggatacaagtataatttccgctattgcgtctatttgaatatctgcaaaaacgatgataacttgcacgtcgaagtggtggagcttaatcacaccttgggtcagcaaatgattcaaaaggctgacggcattattcgctcgcaaacaccgccgcccaaaatctcattggttgccgacagctacgaatgttcacaatgcgagtttgctggcgtttgccatcgcggcgagcctgtcgaaataaactgccgtagctgccaacacgccgagccaattgaaggcgcgaaatggcgttgcaatctttacccggacaacggcccaattccgaaagacgttatcgtaatcggctgcaacatgcacaaggcgattgagtaaatatgcagctaccggcgcaatttgaagatcgttggtatcaggtcgaagccgttgacgcaatttttgatttcttcgatcacaaccgggtaggcaatccggttgtagccatgcccacagggacaggcaaaagcgttgttatcgcgcgtttccttgaacgcgtgtttcgcatgtatcgcggtcagcgaattatgatgctgacgcacgtaaaggaattgattgctcagaacgcggcaaagctcacgcaaatttggccgactgccccgctaggtatttacagcgcgggcctgaagcaaaagcaatccgtttttccgatcacgttcggcggtgtgctgagcgtgcgaaatgctgttccggcattcggccatatcgaccttttgattattgacgaatgccacttgctttcgccccaggaagacacggtttatcaagcaatcatcgcagagattcttaaaacgaatccttacatgcgcgttatcggattcactgcaacgccatatcgtatgaagctagggatgattaccgatggcggaatcttcacccatatttgctacgacattaccgacttcaacagctttaaccgacttgtcttcgaaggctatcttgcgccacttgtgactaagcgcggtgccgtccaaatggatatgaagggcgtttcgtcttcgggcggcgacttcaatcaaaaccaaatgggcgagcgtgccaacgcaatcaccgaaaaggcttgcgaagaaatctacaacatcggtcagaatcgtttgtcctggctgttgtttggtagcagcattaagaacgccgagttcattcgcgatattatgcgcggcgctggcgttgaaattgtgctaagccattctaagctgcacccggacgaaaacgacgaaaacctaaaggcgttcaagagtggtcaagttcaagccttggtcaatatgtcgaaatatacgaccggcttcgatcacactccgaccgatctaattggaatgcttcgcaagaccaaatcgcctggaatgtttgtgcagattgcgggacgtggaacgcgcccttacgatcctgcgcggccgggcgaagttgacccgctcgcatttccgacgttcaaacgaaattgcgtattccttgactacggttcgaactgcgaaatgcacggacctatcaacgatattagaattcccaacaagcccggcaagggcggcggcgatatgccgatccgaatttgcaaggaaggttggcgaatgaagaacggcgaaaaggtatggcacactgacggctgcgactgctacaaccatcctaaaattcggttctgcgaaaattgcggaatggaatttaagtttgacgtaaagattgaagagcaatctagcgacgttgaagtgatgcgcggcgataccaagcagcaaattgaacggtatgacgtacacaagaccgtctatagtctgcacactaaggaaggcaaacccccgtctatcaaggtcacgtattgggcagggctgttgatgtttagcgaatgggtttgccttgaacaccctggcgcaacgtcaagacgcgcacgtaactggtggcggcagcgaatgggcgtagacccgccagcaacgacatatgaagctttgcagctaacaagccagcttcgggagcctgtagcaattcgcgttgacgttgccccaaagtatccggagattttgagccatgaattctaaacttgatttttcaagacataaaaagctcagcgcagaattgcagcttgaaatgcaagactttgcggtaagggttggaatgtggaaaacttgcctgaattgcattgaatgggataaagctagcgaaggttgcggaaaattccgcgcagttccgccgcctcacattatcgtaagcggctgccccgatcacgacgacgatattccgttctgaggcaaacacaatggccgcatcaactcgcgcacgtaaacctaaatcgtccgcagcaccagggcttgccgcagccttggccttcgtgctacccgctcaaaagaaagacggcgagccttggcaatcacattgccgaattgaaaacaactggctgattggctttaacggaatcttcgcggcgggaatgcagattgaagaagacttcagcgcgtgcccgaataccggcctgctcgccgcagcaatttccaaatgtggggacaagatcgcaattacccaggcttcagaaaccaccctcagcgtgcgttctggccgattccgggcgactgtcccttgcctacccccaggccatgccccgaacgtggagcctgacgcagcctgcgcggtggtggatgaccgcctgaaggtcggctttggcctgctggccccgatgctggaagacaccgcccctcgcgtcctgcaaaccgccgtattgcttcaggcaaatacaatggtcggaagcaatggcgcaatgctgattgaaacgttccacggcattgacttgccgcccggaatcatggttccccgcgcaacagcccttgcgatttcaaagtgccctaagaagctggcgcaattcggcttttctcaaaattccgtaacgttttactacgaagacggaagctttattaagagccagttgttcagcggacaatatccagactatcgcgccgtattttcggacaactgcaactattggcctttgcccgacggattctttgaaggcattaaggcaattgaaaccttttcgaaggcaagcactaacgtagttgaattcactagcgaaggaatgcgcgtgtttgccgaagacgggcgcaccgaaagcggggctttcgaaatcgaagggcttccgccgaacagacggttcaacattgactttttgaaaatttcaatgtcggtattgcatcgcattgacttggcaactgacgaatcggctttgatgtttcttagcgaagatggcaacacgcgaggcgtaatcaaggggcttcgttaatgttcaaattcgatgccgcagaattcacggaaaagcgaacaggcgggccgaaaggaacgccatatcacaaacttgtgaaaccggcaattgaactgaaggcgtttgaagaatttacgccggacgaactaattgcgctgcccacaaaccacccgatgctgtttgacgttgaatcttacggcaactattggtgcgtcggtttcctcgaccctattagcaaaaaggttgttcattttgagataagcccggatggccggtttaataccggcgttttgcaatggatgatggaaaagttttgttgcataggcttcaattcgcgcaaatacgatattccaattatcttcgcagcactgaagggcttcgacgccgaattgctgttccttgtgacgcaaaagcttatggaaaagggcgagaataacaagcccttgtataaagcaaaagacgttgcgaaaatgtttggctttggaatcgattgggacagatttaaccatatcgaccttattgaagttgccccgttgtcgggcggcttgaagctgtatggcgcaaggctgcaagctgaccgcttgcaagatttgccgtaccctgtaggtgcaaaccttagccgtcaggaagcattggaagtaaagcattacaacgtcaacgaccttcacttgacccgtattctttgggaagagcttgcgggtgaattgaagttgcgcgaagagctaggcgagcaatacaagctagaccttcgcagcaagtcagatgctcagatcgcggaagcagtggtttgccaggagctaaagcgaatcaccggcagctatccaaaggacaacacagacgaaatttacagcgtcaaatacaaagcccctggctgggtaggctttgtgtctaaagagcttcgcgacgttgttgatagcatcgaatccgccgaattcatgctagacgcgaacggttcgccggtttggcctaaaggcttgggcgaacttgtcaaagataagaacggcaaggaagtttggcagcttagcgtaaagatcggcagcagcacatacaagctcggcatgggcggcttgcactcttccgaatcgtgcgtaaagcatgttgcgtcggaagacctgttgcttattgatcgcgacgttgcaagcttctatccgcgaattatcttgaacgaaaagcttttcccgaaacaccttgggcgggctttccttgaagtatacgattaccttgttacaaagcgtcttcaggctaaagctgtcggcaacaaaaagatcgcaaactcgctgaagattgttattaacggtcttttcggcaaacttggcaatcgccattcgaaggtgtattcgccggagctgctgctgaaggtaactatcaccggtcagcttgcgttgctaatgctgattgaaatgattgagcatcacggaatcccggttgtgtcaggtaacaccgatggcattattatcaagtgcccggcgaaccgctacaacgaactgaacgacgttgttgcactttgggaacgtattaccaacttcgaaactgaagaaacgcaataccattcgacctacagccgcgacgttaacaactatcttgcattcaagctgaagtttgacaaggaagcaaagcgattcattcctggcgaaattgatttcgacccgaagggcaagacgttcgcggaccgaatgggctgcaaggttaaaggtgcgtatgcggaagtaggtagcgcattgaacagcgtgctttcaaagaatgcggaaaaccttatctgtaccgacgccgtaatcaagatgatcgttgatggggttccacttcacgaaacgatccaggcttgcaaagacattcgcagattcacaacgattcgccaagtgaacggcggtgcgcaaaagaacggggtctatgtgggcaaggttgttcgttggtattacgccgcagattcgcacggcccaattgagtatatcggcaaaggttccaaggttggaaaaagcgacggggcaaagcctttgcaagaccttcccccgtcattcccgcaagatattgattacgacaaatacgttcagttgggccaaaagattctatcggacattggctttactccaaaagctcagccaacgttatttgcataaaacaacgggcctttcggcccgttgtttttacttgtattcggctttaaggaatccgcctaccggaattttggggtgcgctccaatatagctataggttggcgcgctgtccgggccgcttatttccaaaaacatgaaagagcattgctcggtaagcaaattgtttgcgagataaagctcccagcttccgccatcaaattttgccgcaaactttacgccgtttgtgccccctcgcgggaaggcaattaagcctcgaataattactccgtttggcgtatattttgcgatgcagtttttggattcggcgtccgatccgtcaggatggaagcaaattccttttcgcggatgcggagacgtgctccaatacgcacgatttgtatcaggcggaagcggcgtaggtgcctgcgatgcgatacccggcgaaccgggaaattcgtaccaaagatgcccttcggaccctagcgaaaggaatggcggaaaccccggcttttgctgaccgccaattgaaagcaaaaacgcggcgtcgtctgtgactgctgcaattgctgggtaatcgtttgagcctggagaaaatccgaaggccgtttcccattcggaatacttcgaataggggtcgtcggttccagtggtggttactgtaaggcttcgcgcaacatcgccgccgcttacaacttccgtccattgcccattctgccgagcatactgctttccgtctgttggggcttcaggaatgcccccgcccgatccgccggtcgcgttgatcttgattgaattgggggcagaccccggaacaagttcgacattactcccagcttcaagcaaaagcgaaacttcaggctcggccggatttgagctatcgacgccaatgccagttccggcagaaatactttgaaccgctgccgaacttccaacttcgacccaaccttgggatttgcgcccataggttttatcgtcgttcggcgcgtcgcccaatccgccagcaagcacccaggattgcgacgcagcttcgtatttataaaatccgccgttcgccaaattcaaaaagtattttacttgagttcctggcgcaaagaacttccacaaattttcgcctacgcacattgcaaggctgtttgaatgcgaaacaaacgcacctgtcggggcagtgcccacaagccagcatcggccaatgtctgcgttggcagttgcaggaggatcgttcaaaacgtcgatgacgccgcactgaacaacgccgtcgagcgtttgcattgcttcgttatacggcgtagaaatttgaagagcattttgcggaatctgaggcaaatcgaggttcggggtagtcgccattgttacaccattatcggggttgaatacgggccttcgccagtcacagaattaagcgcacaaatttgcaccgaaattcctgccggagcgctagggtaagaagccgccatttcgaacgtgtctatcgtgtttccgttgctaaactttacgcgatagcctgcaaaatacttgccgtttcgcggggcggtttcaattcccagccggggacgacctacgaacgcaactgaaacgttgttgcttccgtcgcgagttgcagttacttgcgttacagggaattcacgttgcgacacgccttcgctgtagtcatattcagtttctattgtttcgtcttccgtcaagcccaagcttaccggctttatttgtatctcgcgccccagcatccattgctgagcttgcatgaacgcaatactgctgtcgagcaaaacgaagcgagtattttgcggccaagcctcgacgcctgtagcatagcgcccgcgaaccaatccgaccagcttgtaatgatacagcgcgccggacattccaaggaaatttgcgaattggaattgcaaaacttcatcgccgattacgcaccggttcattccgctaagcaaattttcataagaaaccgattctagcgggtagtttgtcaaaacttcgacagcttggttgcctggatactcggcgctaatttcggcaagcatttcggttgttgtgtcccctattgttgccggggtttcaattgtcaaagcttcggtaaagttcgcaccatcggtagcgaccaaaatcgaagacccgtaccaacctgaagattccccgcatacgcccaggtaaacgcctagttcatcgtcttgatcgcgaaggcacggaatgttcaaaatttcaatgcgcgtagggccgatcaagccgggggttgtggatactggcggcgttagcggccttcctacgcccaaagacgcgtaaagctcctgcgcatccgaaacgccttcaaacccgattacgctgcggtcttcatttcgttcagtgattcggacgatatgccaattgccgtttttgtcttcgacttctacggtatcggcagcaaccaattccgcatattgcaagcctgttttgaacttgaatttttgcggctcgccccaggcagaaacgctagtgattagcgctgttgttgctgcttggtctgcggtcaaaaccacttcgctttcaacatcaattttctttgtggtttttaccaaattgcttttacggcgaacggtctgcttgttgtttgcaaaaccgccttccgggtccaaatgcgtaacgttaacttcggcaggaagttcgctttcttgaactagcgtgacgccaagcgccgaaggatcatcggcaacaagatgcacgtaaggaatgcgcgcgctaatctcgcgacccctacgtgggaagaatagtattccatcgcgctcgcttttatcgaaaaagaaaatctttcgcaacgcgtcaattcgcgcattggttccgtctttcgtgtttatcttgtagccaattacggcttggtcgtacagttcggaaacgttgattcgttcgggagaaattccggaacgcaggcaaagggccattacaacatcggcaaggtacgggtctgcgtttaccgaaaattggctgtcgatgtttgagactttacgacacctaaattggagccttccgcctgcgtttacgcccacactgacaagctcggcggtcgatccgacccccttcaagacgtgttcgatttgatagcgctcgcgctgatagcgaacgcaaagattcccggcccgaatgtagctaagaacaatatcggaaattgctgtgtgccattcgcgcttttcatctgtagtgcaacgcggcgttttgattccggccgggagaactgtcgtaatttgcccagggacagaactatcgtaccaataaattttggcttggttcgcttgaacaaaggcaacaaacggccgcatattttgatcgaatgctagcgaagcttcggtaatttcagttccggtaaacaaaacaatttcatctacgccgggggctgaaactttaacctgttgaacttcgtcaacagtgtcgacagaaagcgtccaaagctttacaagcaagccttcagacggatcattcaaatttttcccggcgcgctcccaatcaacaagaaagtcgcccggttgtttaaccgggtcggccgtcgcgctaactacagacttcgttgaaagtgtaccttcggggatcattgtatttacctacgcgcccaggaaatccgaatcggctggttccatttctttgtcccgtctttgggaattcttttgtcgaacacaatttgatagccgccgaacattccagtcgaagccaaaattgttccaaccccttgcgccaaattgccttcaagcaacccgaaaacaagagtcaggtccaattggtaagagttttgcgcatacgcagattttagaacatttgcgggcgcttgaccgttagccaaaagttcataagctcgctgagtttgggggtatagcgtaagatttgaagtagtagttatatattgattgtacggcgcagactgccaggagaaatcatttcgcgctcctgacataatcgctcgacccgacgcaatctgataccaccacgccccgtaattctccgcccctacgtcaacgggccgggcagtgtagttgtaagtaatgccgtccagcacgatagagccggtaacgtcatcgttcggaatgtaagaacgaatttcgtagaaaacatcaagcgtttcgtcgctcaaaacggtaattgacgttggatttccgtttacgtcgcgaattagcgccctggacattagcggcgcagtattgaagctattcccatcaacaggataacccctgattccaacttcctgaagattgccagcggccaagccgtcgccaaagcgccacacattgcgaagaaagccgtaacggttggccgtatcggtaagcacaatgccgctcgccgcgccgatgccgctcggctggttttgggtctgtgcaacctgcgactgaagttgcgtatcggtaaactgcggcgtttgatttccgctgccgacgcagcaagcagttccgttgctagaaaaactcataaactgcgacccggcaaacgaattcatgccgtaattagtcagcaagttcggtgtatcggccataccgacaatttcggcggtgcctggaataggattgccgtcgctgtcgttcttgtgcttaacgaaagtataaaagccgccgacttcgcgtttaatgttaatcggttccaacatatcaaactcccaagtatccgcccgaaggcaaagttatgtttgaattgaccgattcggcaggccaatatgtgtatgtaataagcttaactgcaagaacgccagaaagcggacgaattccaacggcattaactgtgtcaatttcggcgttagctgaaaccaagggattgtaaagcctgccttcgccaactgaaattgagctttgaacttcgtcggtttctgcgttaacttttaccaaaggcgtccaaagctgtccttcggcaagagacacgtttgccccgacaagatcggatgaataacctacgtgcgaagtctgccttagcattccaggcattacggcaaacgtagttccaagcgattcgggagccatatcgcttgggtacggccgcgaagtaaggtacgcgtcaggcggcgatgcaatgactacagcttcatatgtgggcacagcgccgccgccgtccgtaacgtcgtcgtcttcaacaacaatataagcaatgccgcgaaacgctgaaacctgtccgacgccgcgatagctttcaattgttgaatcgggaagctgcgtttctgtgccgtaatagaacgttgcctttcttttccattttgcggcataggttctatcatcaacggatgcgttagggtcttgcgtccaaacaactttgccgtttcgtttgatcgtcaaaaagccgaaaatcggaccttcgcaaaatgcgacagcgtaagatagcgtatagctgtattcttcactttttacgccgcctttaccctgtttctttttcttgacgtgttctttcggcggcatcggcgcgaaaataacgttgccttcgcacggaaaacgaccgaagccgtaaggaattggaacgcctaccgtcgcagtttgcgaagcaaactcggtaagtctgtttcccttgattgtaatggaaccaaacaggccagccatttatacgcgccacacgtaaacaattcggcgcagccatttttcatctaagcgatgttcggtaacttcgcctaccattgaatcggtatggataaggccgacagcgccgggatagtctgttacgatgcccacatgacggacggggccgcgatactgcatcgcgacgaaatcgccgggctgcaaaacatcggcgctttcggggttcgtaattagcggcgggccgaaaagctcagtcaaggtagcttcaagctttccttgatggggatcgcgaggatacgcaggaactcgactaaacggaaaggccattgcgtgagccaatagcccaacgcaatcaatgcccttttcgttttgcccttgatgcaaaaacggaacccctagcattgccctggcgcgttcaattcgttctttcatagcgcattccgatttttgatatacgcacccggaaccataagcgattgatcttcggtcggggtcaagtgttcggctcgcatgttaacaatgttgccgtaagctttgcaattagtttcggttttatcgcaatcgcgacgaagcctaactttagtgcctacagtaattgcgtaaggggttgcgtagctaagtttcacagacccgtcggcttcccaagattcaatttcaagatccgcacctgcgttgtcgccatcaataaagttgacaacgccaagctcaaaatacccaggaggtcggcttatactgcctactttaaatttcaactgagcgtttgagcctagctcggttacggttgcagcttcccaggccagcggcattcggcatttcgaatcaccgaaattcgcacggcatgtaagactgtaaagctgatttgtgctagccgcgagaatttgggtaagcccgcgaaattctactttgcgacgttcttttgcgtccgatgcgtaatcgacttcaccgacgttaccgtagcctacaatttcaaatccagcgcccaaattcaaataggctacgcggtaaatagttatcttcgcggaatcgaaaacgcccgcaagaaaacgtttttccaacgcatcgctaaaccacccaactaactttgtgttgtctacggccatatctgccgaagtttgaaagttttgcggcgcaagctcttcgaccggcgaatacgcaaccaacccgtcgccgtcgtcaaatcgcaaagttgaatcgcagctagtgaagcctgcgacttcgccagttttaacagattcaatccttaccgcataagccgtcgaagttgaacttttcgaatattcaagctttagcgccaacggaatttgcttaggcattatcctacccagctttgcggcatgttatccgcagtaatttcaaacttcttttcaattagagaaattgaaaagccgctgttgttccaactgttgatagtcattgtgttgtcgtcgctgtcgaagcgaacccaaacataaaaccatcccgaccaagtgtaatcgccgcttccccatatttcagacggcgtaaattcgcctgtcataaaatcgaaagtgcctgcaacttcgtttccgcccgccgtgtatactttagggccagcttggcggaaattcggatcgcggttattaggatcggccggaaccaaggcttgcacagggcgaatcgttttggcgtttccgaacgtatacgttttgtaaagctgaactttctttgttgttccggcgctcaccttcaaaggctcgcggtttgcaatgtaatcgttccaatccaaaaattggaacgaatgcaagcggccccggcaagcatgaaacacggccgtgtaatattctttctgttcgtcgtcaatcgcttcggccttggccgtatagcgatgcctggcatattgccaggcactatcgacttgttcaaagccgttttccaatgcaacgacttcgctttcgtagctaggcccgccttcgaaaccgtaggaaaatgacgggtcgaatgcctttgtaatctttcccatagcttagtagctccgttcgtattctttggaaacgcccgttcgcgttgcgcgagcaatttgttccggcgtgcgacgatccatgcgaccgccttcgacgttaacgttgatcgtcggcgcgaaattggcccgctggccgctcccctgcccctcagcctgcgccgcaatctgtgtgggcaccctacccctgcgcagggcttccaggttgccaacaccgatgcgctgagtggccgcagcgtcgaacacgtattcctgaccatgcaccgggccagcaatggacgtgcgcggcatgttaccggtatagccgccgtccataaagcccgcgttcgttgcgcgaatcttttgaacgtttgccatgcctgccgcgattgctgccgctgctgctgcaacgcccaggattgggccaatgtaaggaatacccgacattgcgctaaacgacgacgtagcgctttggtaagtttgaatcagggtttgcgcaattgccgcctttttgccgatagccgcttgttttttgttttcagaactttgcagggttgacaggctgctaaacacagtgcttgcggcagtcaaatactgttgcgattgctgctggaacactgcgaactttgcaagctgtgcgtcagtatcgctaagcaaatcagcctgacgcaaagcgtcaatttcggcatacatttgcgtatacgattcgacttgatattgcgtatacgcctgcgtcgcttgaagccctgcgttctgctgagccatcatgcccacaatatcggtcggatcgacaccaccctgaccggcgacattcgttgccgccttaatccgatcttgcgaatcctgcttgcgctggctcccgcttccctggcgaatcgaatcttcaatagccgaaacgcgctgcaattcttgcatgacggtaagccgtgcgcgaagctgcgcaaggtcttcgtcgcgaatcttttgaccgcttgcaattgcctgattctgagcggcaattagctgcgtttcaatttctcgctgctgcgaattaagcgcaagaagcttggtttgttcgtcaagccccttgttgatttgatacagcggatcgattgctgacttgtaagcttcttcggcctgcgcagtgacgccgaaaaactgctgccaagtgatagcgcccttttcgacaagcttgtttgcagcatcaagcgttgcgttgaaatcacgaagcgggccggttgcctgctgataaatgcgatccatcgcggcctgttcgtcgcgagcctttgcaagcaaatcgaccttttcgcgaattgcgttcttttcttgttcggtaagggtgatgcgacggcccattagagcctcgctaaccttatcgaattgctcttgcgcttcacgttcgctgccaagcattcccatgcgggcaatttcgttgtcaagctgtgcgtttacttttgccagggcacctgcgcgagtttcttcagccttggcagcagccttcgcggcgcgttcggcacccttgtctttatacttttcgttgatcgcagcaataagcttcaacgaacgagcatcgttgaagttgccgttgtcatccattgttatgccggaattgccgccaatgtaagcggccgtcagttcggcgttaaggtctttcagttccttagttttctgtgccgtcttgtcaagctgaagttcgcgagccttcaacgagtcagttgcggcaattgccttgtcgtgaacctgctgagccttggcggcttcgcgtgctgccttttgctcagcttcaattgaatccgtaagttccttaattcgcttcgtgttcttttcaatcaacgcgtcgggggtaagccccttgacccaagcgggttgttcgttgaacttcgccatgcgctgctgaagaactgcaagctcttccatcttgcttgctgaaccggtaaggatcgcgctttcttccttaaagcgctgcattgcccattcaatcgtgttgccaactttttgccaagcggcagcaagcccgttagtgtcgttagttgcttcggcgagccgcttgctagaagttgcgccaaactcttcaagcaaccgagttgcggcggcttgcttatcgccttgctcctgcaacgccgcaacttgcttatacgttgcgacagtaaggaagctatactttgcgttaagctcggccgcagctttaaccgggtcatcgaatacggtaagaagctccttcgaaatttccttaacttcggtgcccgaaagctttgcgaaggatgctgcggaagttgcaacagcttgaagctgatccgccgaaacgcggccgtctcgcgccaaagcgtttacagcaccgcgagcttcttcgtaattgtgggtaatctcaccgatgcgcgaagacaaaacagcaagttcgccagcagttgcaccggaaatacgaccgtttgtaagcaggctattattgaattcgtcgtattcgttgcggctcttcaatgctgccgcaccgatcaatgcgacatacgcaagcagcccagcaaggcccgccgcagcaccaccggccgcagtgcccaggcccgtgagcgttccattgagtaggccggtagactgagccatgcccacaatgttggctcgcgcagcggcccattgaccctgcgcaagatttacgatcattgaagttatctggcggcttgtctgcgcgctaacgccgcccaaattctgaacttcgtttgaaacgtttttgattttggaagcttgcttgtccagatttgcaagcgccttggcctgctgctcagtggaaagagcgcccttagccattgcacggtctagcagggcttcaactcttgcaacgtcttcggtagtctttacgcctaccgccaactgtcgattaagctcggcaacaaccgccgcgttttcttcggcagctttttcagccttttgcatcgctgcaacgcgttcggccattgcatcggcttcgctacgaatagccttagcattttccgaagaagactcggccgctgccaagcttgcccgattagcttcgtttctggcttcaacttcgcgcaaagacgcatcaaccattgcgctgatacgttcggttctttcgacttcggcggcggctgcggcggcggcagcatccgctgcggcctgctgcgcgtcggctatcttttttgccgccttttgctcagcatccgaaattttagcttgtgctttgcgtgagctttctgcggatttttccttggcctgcgcaacgcgattttcgccttcaactagttttgctagcgaagactcagttcttgccatttgctgctgagttttctgagtttcgccgcgaagcttttcttcgccggttgcaacatcaagcaatgccttgtctgttttcgcaagctcctgctgcaatttctgcgtagaaactcgttgattgttttcagcttcaatcattttggcaatcgaagcttcagtttttgcaatttgctgctgacggcgttgttcggcaacatcggctttggcagttgcttcgcgaagcttttcggcagaaattgcggcttggtcaaacgcgcttacttttaccttgccgagtgacttaacgagcgcgtcaactttcgacccggctttgtcggccgcgtctgccatgctgttaagcttggtagttacgccagcagcaattttatcttcaacgactacttgaatgttatcgtcagccatacgtcacccaatgttgaacttgaaatttgcgcgaacacttcgcattacaaacagccctttttcaagaaagcgtccaggctgcttagaatgtccgccgtcgtttagctttctgatatagggctggttgttttgaatgtaaataggttgcccaggccgcttagtcgcaagaacttgcctagcttgcgccacggtttcggccgcgcttatatttcttgtcgaaccgcctttacccctaaaatgcggcgggtttttatctgcggtcggatcgtcaatagttactatccaacttgacaacgcctgcgacgtgtcaaccggtgtgctgtatgccacttcacgaacgaagccgatggccatttcaacggcgcatcggcttgcttccttttcaattgccccggcctttccgcgaagacgctttgccagatcgtgcagatttgccatgcttcaccttggcttccatcttggcgctttcgcgtttaaggtaggcgttatctaattgccttatgtgataatggagcgattccattgcatcaaaatcaaggccgaaagtttcgccgtatcgttgaatgctgccccagggtatcggcccgatgctagaatcccctgcgcttcgctccgttcctagttcgaagaacgcatttaaatagaaatcctgcccgctgaatagccttggagcttttgcgatgcggtcaggaactggctcgccgcatcgcaaagcctgcttgattatcgtcaattccgattcgccgaaatcaagcacatacagcaaaacttccgttagttttttgctgcttcctcgcgcgatgcgacaaggaagttcgacgtttcgtgcgactgcacttcgacaattgcgaacagttccggcagacgttcgaaaagcttgattgcgttttcggggctgaaatcggcatagccttcggcaaatgcgcggccctgcaaaccgtcttcgccggtcacgtcgccgaggggaatgttggcccagcccttgacgatatgctttgcaattaccggaatgcgagccttggccttttcaagcgtgctgtcgattcctgcgcgatcctgcaaagcaaacttttcgtaagcctttgcgataccgctttgatactggcggttgttgtatccagcgcgcgcaatgagaatggttggctgcgtaccgtcttcgttcttttcgccaatggcgaactcgaagcctttttctgcggcgttgttgtcgatcaaaaacgaacgggaaagggacattgttttctgcctgtgttttgaatgaaagaaagggccggaatgcccggccctttcagtgtatcgcatcggttgtggcgctgccagttacttcggcattgcagcgtcgggcaggtacgggaacaggcaaagcattgccgtataaccgtagacgttttctgccgccgaagtgttcaacggaatcgacaccggctgacccttttcaacgttcaggcgaccgccgcccaacgaaacgagcggcaaatcccaaatcatgcccgcattgttgtaagcagcaattacgttaaagccaacatccttgctttcacgaatcgcacggcaggccgcaacgctggtgaacagggcagtaacttcgcccgtaacggcaaagttatcggccgacacgctacctgcgccgaacttgccgacaaccttggtcggcgtaataccgttgttgattgcgatgttgccttcagtgatccaggcgaacaggccagtcggattcgaagttgccgggtcaagaatgttcatcttgatgcggtaaatatcgctcgacgtattgatgaaatcttcgccaagggccggaataacggtgcccacaagggaacgcagcttgtcaccggccgcgcccgaacggaaatcgttatcgcaggcaacgaaggtgtaatcgacattgaacttttccgcgacgggaatgttcaaggtcaattcgttcggcactgcgccgagcaaatattcgccctgttcgtcgccgggattttccgaagtggcttcgtcttcgccgagggtgcgctcaatcgtgtacgaccgacgcttgattagggcgcgctccttttcgttacgaatcagcgggccgctgaagaactgcaccgacagacccgcgccagcttcgttcacaggctgccaagtggtgtcatcgaaaacgattgcgtttgccgaaacgcttgcgatgcgagcaaagccggtgttgtttacgaacgccgaattcgcaacatcgccgcccaggaacagccacttgccggggatcaagccggggaaagtggtgaagtcggtagcggtggaaaccagcgacggaatgccgtcaaccaccgcaatcgaaacatcgcccgcttcgaactgcccgccaacaacttcaaccttggccttggccgacggcgacgcttcagcaatcagcgcttcggcgacttcgatataaccagcggcgacggcagtaacgcgcttcaggccgttgttgctggcagatgcgaagccgctggcctttacaagctggccttcggcaaagatggcatccaggcccgacgcggcggcatagcgcttatccgccgaagttacggcggtaattgcaatcttcttcgtcgggtcaaacgggtcagtcgaaccggcttcgcgagcgttggcgaagaaaaagccttgtgcaagccagccgatattgctttgcgtcaggtcttcattccagccgcccgacgcgtcgaggtcggtcggacgaccctttttgttttggcgggacgggtcgatgatttcgcgcgcaacaagcgtaacgtcgccgccgaaatcggaatacgaattcggttcgcgggtgtgccacgtcgggtcgaaaccgtcgattgcttgtgtgggcagttctttcaagcaaacttcttcagcaatccgaaggccggtcaagccgccgtcaatgccttcattatcacagatacgggccattatcttttcctttagcctatttggttatattcaaaatccgaagacacgtcgagccggtaaaaatcgtcttccttcggtgctgttacaatccttgttctacgaaaggtaatgtttccgttcatttccctaccgcgaaaagctgcttttgcaatctctgccaattcgccaattatctttgcggcgttgaccgtggttttcggggcgtagaattcgacaaacaacattcccgaaacaagataccgctttttgaaaggctcttcgacgcaatttgaaagcgtctgttggtcgtccaaaatatgctgaacatccaaccttgcgcaaaccttatcgcggggaagcttagcattcccttcgatgccggaaaaggccaattcgacaggattgcccaggtttgctgcgactgcggcggcggattgcatcgccgccttaaatcgcgctcgcattgcgtcggttgaatggttgtaagtcgaagtcattctttaagctccaacttgtaaaggattgattggccgttagggctaagcttgccgactcgcaaaatttcaatgcgaacgccatccctttcaacgaagtctgtgaggtccggagcgaaaggaacattaccggccatcaagcctaagacggttccgcttttaagttctttccctgaaatgtatgccatgaattgcttaatgtcgcttttatatggaataaagcaaatccatactttatggcgaacttcagaaacaatttcattgaaattgtcatcaatcgattttacgcgactgacgaaatcgacaagctgcccattcttttgaattaggcgcgcggccgttgcaatttgacgatcaaagcggccagccataattaaacccgccgaccgcgaagagaaatcccgccgcagcttccatccgtaacaagcgacgaaagcaaagcttgaacgccggtaaacgtcgtttcataacccaacgaagttggatcggcatatttggttgtgattacgtcaaccgtttcttcgataaccatatccgccgcactgtagttcggctgcaatacgattccttcgcttgccgccattgcaagcttaacttgcgccgcgataaggtctttcggaatgcggtctgacggatacggatcgcagcacagatagacgccttttcgcggccattgcaacggttgatcgcagtcaactttacgacccttgaagcggcatccttgcgcttcaaggtagtcggttgctttaatcaacatggccgcaacgtcatcgtcattagccggaagctgtacgccgcgatttgccgcgtagattcgtgcgtcagcaatgctaacgtagctgtttgccccggcaacaatacttccgtcttcaacgatgatttgaatagccattgcttagccttacggagtcggggtgaaagtgaaggtcggaacgcccccggcgactgcgacggaaacagtgccgccggttacgggatagctatcgccattgcccacaattgctttgtctgcgggcaagctggggttcggcgggtcggccgggtcgaattccggcagcgatgcgtaaggctcttcttcgggaacggtccccgcaacgtagtcggcttcttccggcgtgccgtagttcggcgaatcgatgggattgcgaacgccaacggaatacggcacaacgcacagcgcttcgattgcagcgatttcggccttttcggcggtggtcggaatgcgcccagccgtgaagtaaagaattttatcggtcatttcgatagcctttttaggttaagaaaaagccggggttttgccccggcttttgttggcgttgcgccggttactgcggcttaccccaggcacccccggcaggcgcgtcaccgcccttcgcggcgtcggcatcgggggtagtagcggggccaccgctcggcggctcgcctgcgcccggctgagaggtttcgccgtcactcttggcgagcttttcggcgttgcttcccggcgcgggcttgtcgcccatcgcaccgcgacgcttgcgggcttcggccttgaacttttcaacggcttcttcgggcgacgggtagtgcttgtaagcgtccggcacttcaccggctacgccgtctgccttttcaagcgggttgctcagatcgacggcacgaacgttgcgatactggacaatgccgttaatttcggcggcttcgtcaagctgcgcggctgacggtgcgggaccgtcaacgaaatacagaatatgcgggcctttcatcgaatgtttccttgtaatgcgagacggggaaagccggggcaattacgccccggcttacgtcggttagttggtttccagtacgacgcccaacgtgtccttgtcgctggtcgaatgctggtcccaattcgcgcccgacagcagcgcagcgtcggtcggagccttgccgcccgtctgcttgtcccaagaatagccgtccaggccaagctgatacgaccattcagcctggtaagtgcgctggatattttccttgccgttcttcgtttcttcgttggcgtcgaaatcgttgttctgctgaattacgattgccgatgcgcccaggcccagcgaatggaacttggccgggttctggcccgctgccggggtaacaagcgaagggttgtcgctaacgagaattacacggcccatcggatcgcgcatcacgttgacggtgccgaagttgaacaggcgctcgacgttcatcaagttgttctgatacagcttgtgcgaagcgcccgagtgcatcgcccaaacgcgaatgcggtccgatgcgtcgccgaacagggctgcggccttggcctgattgagccaagtcatggtcttggaatccggcgtggtgtttgccgcgtcggtggttgcgtcgtagagcatacggccctgattgacgacggccgcatgcgccgaacccaggccgatgcgcagcatatccgccatcgtatccttagccaactgctggccgaatgcggcaccggcaacctgcggattcaactgaatccaacggaactgcgccggggacaggtcaatcgggaacgtgccgctcgcgaccttaaccattacgtcggcgatatgcgccagcgacttcattgcaacatcgccgttgccatacgggttgcgacgacgaacggtgccgcccgcgattttctggaagaacgcgatttcgctgaaatcgccttggtgtgctgcgctgcccaggacgattgcgccgttggacgctgcattgaacaggtcggtttgctcctgaagaatttcagtcgcaacactgtacgcggtttcggaatagaccttcaggtcggaaagtgccatcgttttgccttttgggagttgacttcgaaagggttacttcgcgccgaagcgctcagcgagttcctgcggcgacaagtctgcaagaagtttgccgccaccattgttgccgctgttgctggtgtggacggcaccgccgttattcgaagccccggcaccgccgctggcctttgtgccctggatgatacccgaataatccttgtttgcaacaaactcttcgccgagtttgtcaatggtcaaatcggacggcttgccgtcctggcccaacaccttgacaacaacgttgtcgttatcgtcaagctcggccgaaatgcgggccttaatgtggggaaggagaatcttcgcattgcctgtcgttgcgatcttttcggaaagacccatcgcagcggtgttaagcgcgctatcgataatgcgcgagctaagcgcagaaatcttcgcagtgaatttgccgtcggattctgccttttcggcgttccactggcgttccagtgcttcaatgtcaccggtcttgcgagcggggttgctttccatcttttcgattctgatttcaagctcgtcgcgctttgcttcagactgcgcaagcgcgtccttggttcgcgtatgggcacgcttcagcgcgccaatgtcttcgtcgccttcagtctgaaggacgaattcgccgtcactttcgcccgccttgtattcgaaacgaatattttcggcaagggcttcgtactgatctttggtaatcttgcgcttcagtgccattgtcttcgacctttaagccaatccatcggatcggcgagttagaattgactttgccttgttggaaagcccgttgattgcggcaggttttacgattgttgcaatgttgaaattagccgcagtaattcccccattttcgatggcgtccgctgctttgctgcccacaaggtcgtccagatattcgcggggctgttcgcgaagccaagtgtaaagcgttggaactttaaagtcatccacttcaggcgcaagtggaaccgtagtgcttcggcagttgtaatgtgccgggggaattggcccgacgccgtaacggaaaatgcgcaagttgcggcttcggcaaatgtcagttgtagcgttgtcgataaccgaaatccacttgtagaacgtgtggatcgccgacgccacggcttggtaaacagtttccgatacgaaccccactgtcgtttccactgctgccgttccctggcgtcgcgccgtagcactacggctcagtgcgattgtttcgatagcttcctgaagctgcatattgtttgcatatgcctttcgcacttcgttttcaatagaaacctgtgcagttgttgcaaagcccgcaatcagcttttccggcaatattccgtttgccggaatcggtgtatttcgaatacgactccaaagcagtggcgcggatgcgggcaaaaacagcaatccgaaaatgggccaagttcgcttttctttttgcgtgcgctcaatgtggttgaaagccttggtcgggctaagcggttcagcttcttcgggatcgtagctgttagtccccaaaatgattgcgtcaagcttagtcttctccttcataaactcttcaagctgtttaatgaagtgcttaacgtaagccccgtaaactttggattgcgatgcgcgaaccgctttaagcaaattcaaaagctcggcctttgttagctggccgagcttttcatattttactcgctgcataactttgcgaaattccttttccgcttcagcgacaacagcatttaattcgcgctgctggcccagctttacgccttcgaccagcagtgcagttcttaccgtcaaatcaaacagtcgcaacgcgtccttcgcggccattactcggcccccgtcggcgcagccccttcaacagatgcggccatttccatttgcttcagagtgtcagcttcgatttcggccttaaccttgttgtcgtcttcaaaagccttacctgccctgcgcagcgcagttcgcatttcgggccagctaattgcgcccttttgccaaagctctacgataagccgttgctcttcgggcgacattgccgacagatcgaaatccttgttcaattcgaacttgatgccgtttgtgcccaaccccataagctccgcagcgtaaacaagcgcagcggtataggcaacgcttacgttattcgcacacgaagccagaacggaactttccgaagcattgtcgctgcgcgtctccgttgcggtgcgttgaacgccacgctcttcaacaagcttagcgccaagccctttcatctgctttactttgtcgtccatcgcttccttaatcatgctgttttcttcagcagtgattagcttagcgtccgactcggcttcaagtggaatgccgccgcgcgaaccgaagttaagctttcctttcagaacttcagtcagccatttttgctgcattcccgttacaactagtgtgggctggcccagcaggaagcagcattcttcgtagtcagcgctgtttcgataatgcgcaatgttcaagctcgcaagatcgtagaagttcggattttccggattcgcatcgttattgcgactaccgataaaccaaaacggaatgcgcttggctcggcttccatctgccattgtcgggtaatacgtcgaatgcaaacggaattcgttgccctttggaattttggcccccaggctccactcagtcggcttaacttgccgccaaatttcttgaacgtattcgttagcttcgttcaaacgaagcacgcgaacctgcggaccgtatttgacttcaaacccatcgtcgttcatggggaagccttccattagaacgacaagcgacagaacttcagacgaatcgatttctttgactcgccagttcaaaatttcaaacgtattgtacgaatacaaagtcgggcggatgcgcccgcttgcaacatcgtcggccgatgcgccccgttccgtagtgtcgggaaagtctacgaacacgccagcgcgcgaatacgaaacaacttcctgcaatgacatttcggcagactggaaaaggctaattccggtgccggaaacgtcagccttcagtgcagacatttgcgccggaatttcacaaaccggatcgcgcatgaaaacttggccggtcaagccgtccagggttcgccgcgtagcgttgtaaaacacagcgcgcgtcaaatacgcatcgtaacgcgctttgccttccttaactacgtccgggtccatttcgagccgcgattcatcagggaacggcaaatacgcttcgcgcttagcctttactgccgtctcgcccgcgatgcagtcgcgaattactgcgtactcggccattttctgagaaagggccggatgaatgaaagttacgttaggggtattgggaacgctgcgaacggccattgaattgccctttaattagaattttactttaatactacgagccaaacgattcgaacttttcaaaacccgataccgcgtcatatcccaagggtggtcaattgcggtagtgtctacgtcgtcaactttaacaggatcgcgcggaagcttgggaatggtggaaatgctggccgtgcaattttgcataaagtatatgcccggcccttcgttttccaacactgcttcaagcctgtcgcggaacaattggaagccgttagttcggctgcctttcgatttatccgactcttgccaagttacgccgttgtcagccattttcttttcaatggtttcggtgtccgactctgtaacattgctgattgcgttgtcggccggtccagggaaaatttcaccttcaacccagccattttcttttagcgatttttcaatttcgataatgcgttttgcggtgttctttgctgaaagcttattgcccttgttctcttcaatcttgggcgcgctgtagtcttcaaagaactgaattaggcttcctgccgggggacagaacgtaaaccattcgttgccgatctttactttggcttcttcgccatttgcttcggcccaccagcccacactgtaaggctgggaactaccccagtcaaacgctcggtcgatgctccaccccttcgggatcgcaaagcgcgggataacatgataggccgaattccaaagatcgccgaaggcgtcgcctgccgaaatatcccaatcgccgaacagccaagctttgcgcaaattcgggtcggtgatcttttcaagctccgcaacgtattccggcgtgaggtatttgttttcgcgatacgaaccgaacagcgtaatctgagttttggttacgtcttcgtcttgctgcgtctgcggattgaatacgcgcgtagtagtcgaaaccaaaacgccgcgaggcgcaatgtcgatgaaacgtgcttttacccaattgtggccggggccgtcagggttggttgtcgaaaacacttcaagcggaatctgcggcagcggctttctatccggcgtatcgaaaacgcgatacgttccgtctgcgcacttaaacgcgtcgagaatgtctttatcgccctggcgcacaaccctgtgaggcgtatcacgttcaggcgtaaacgtacagcgattgcacgacataaatttgtcgtacaaatcgccgtttgaataacgagtaagttcgttccagccaatgaacgggtattcgtggccgtgaaaaccgtcataatcgccgatcttttttacatggcggaataacagttcttcgccagtaggccaaacccatttgtaagacgatgcagattcaagaaacaccgcgccgtcgttgaatttgctaaaccatttcttcgactcagtaaccaagccggaaagattgtcaaactcacggtcgaaaattacgcctttccaatatcggccatagcccaagccaacacgacggcgaaaacgcatcaactgcgttagggttttgcctggaccgcgcgcgccttcgtacaacgtgtgatgcgctcgcgaatcaatcgcaagctcttgcgacgttccttcgattggacgccatacaacttcgatttcgtcacttacggcctgattcattctgattcatcaattggcgttgttggcgtgcggccttgtcggcccattcgtcattagtgcccatatcggttactatcataaccgtttgcttgcgggcatcaatgttaacgttggtttccttcggtccggtccaaccgcgaatatccgaatacagtttgaaaaacttatgcgcgtcagtgtcttcggtacagcttcgcgcgcggctcaaaacttcttttgcgaaatcgaattttgtccctagtgcgtcaagcccttcgtctttagcacgctcagagatattttcaatctcagttagaacaatgtcgttttcgtagaattgatttgcgagcagcaaggcatgacttgtgtccggcgtcacttcgcaagccgccttgaaacggccgttcatcccaggctcgttacgtaaaagagcttgggcgaagcgcttcagaatgtcgtgatccggttgccaagtcataaaagaaagcccgctatcgtcgcaatggactatagcgggccttcggttcaattgctaggctttgtgcaaatccgtttccacttttcattatgggtaaggatttgtcgagcggtgccgtctgtcaaaacgtcggatttgcttatgtaaatcggcgatacccaatcacaagcggtatcgattactaccgacttaatcgcgcgtccattcatcgcgcaagcgctcagcagcatcgccaggagcaatgcgattaacttcactcgcgacattttcggccacctttacggtttcagttcgggtttcaattgcttcgcgttcaactgcgaagtcttcggcttggcgttctgtttcgctctttgcttcctttacttcagcctcggctttacctttgccttttgccaggaaatacagccccaggattgacgcagctacagccccggccgcaacgatccatgcccacactgtagcccctactcgggacagccatgcgccgatcacggccgcagcccttcggtgtatttgccgttgcgcattgtcagcacttggcgacgattgcgcgggccaaagctcacatgggtccaggtgccttcttcaatcagttgatcgaacggcaggccagcggcaacgatgaaacgacacagttcaatcggggtcatacccttgacttgaatgtctgccgcttcaccctttacgtgctgcgacgtgccggttccgcctacggcaatattcacctttttggggcgaaggccgctggttacgttaaccggctttcccagcttttcgcgcagagggtcaagcacgtttgcaaccagggcttcaagcgctttcgtttcttcggcgttgggaacgatcttaatccccattcgatccgccgttgcgctcttgcaaaactctgcaattttgaagtgcttcatttctcgctcctgctctgcttcaggatcattgcgacattcgacgcaatgaaaagaccgatgccgaattgcttaacgaaattcggcggcagaactgctttcaggtcgtcaggcatcataagccaaacgtgcaagacagtttccggcgcggaaattgcccagctgactacgacagttccagcagtcgaaagccagaatgaccaacgctttacaacatcgcgccagttcggtgcaactactttcgtgacgacctttttcattcgggctttccatcggcggaaggtggcggcaagcctaacttgaattcgatcaagtaaaggcggcggtcggtttgcatatcgaaatgcttggctgcgctgtattccttccagccccagccgatcaggccaacgctaatgctcagaattgcggccatgattcgaaccaacgttttgtgctgggtcaattcttcgccctgctgtgcaacggtggatttcagcgcttcaagctgcccaggaacgcccttgaactcggcaagagtcagttcgattgcgtgaaggcttttcattgttgctttcgcgtcttcgcgcatttcgcctagacgttcgactacgacagtaaattgtgccgggtcaacgttcatctttgattcgtccattcgctgaaacgtgatccccaagatgggcggagcttatcacatagcaaaaaccccgcctagcgtgcgctaagcggggttccacaaccaacccatcacaggagagccagggcacaggcaggagccgtggcagggccagcataccgcctgctgcggcaaaaagaaagcccccgatttgcgggggctttcaatccggtctttcacccggtggggccgttatttcaggcccatgttccaggcgcgattacttggtgcggtagatgcgcacgccagcctgcggcttgaagccgtcggcctgttcctgctcggcggtacgacggcgcagttcgaacttgcgttcgtaggccagaaccggaacggtcttgtcgccgcgctgcttggtttcgccggtttcggtcgcgtaacgcttcgaagcgctcgacacggtggaagccatcgacttcgccgggtcggcgttttcggcggttgcagcgacgaagaacgactgaccaacgcccagcttgctgaacgggtaacgctcggtgccgccggtaaggccggtgccgcgatcaatcggggtcagggtcgcgccgtcctggatttcgaaggccggtgcggcagacttttcggcggcgggggttgcggtggtggattcggtcatgctggcgatgcccttttcagttgcgcgggtggcgacttcgccattcgcattggtcatggacggattgacttcgatcaggccatcttcgattgccttttcgtaagccttcgggttggaaaactgctttgcgctggtgtgaaccagggcaccggcattgctgccggaagtcgcggcgatgatcgccgacaggtcgaacttgctctttgccattgccttatcctcgctgggtgggtgctgcgttgtgaggcttcactatagcagcatgaatttcgaagtcaacaaatttcagcgattttctttcaaaaactttggcgggtctttaccgccacattcagccttgtatgaatggtggtagtccggccagtaaccgccgcccaccatttcacagtattgatcgcgttgcgaatcgacttcctgcttgttggtgatgcccacaagtagggcagcggccaggatgattaccaagccgacggcggttcggaccttcatatcagcggccgtgctttgcgatgttgcggcgcttgacggcagcgcgtttctgcttggccgcgttgctgttctggcgatacgacccgttcaggctcttcgggttgttgccgtagcggccagcgaacgaaggcattgggttcgcggcggcatcgatgaacagattgcccagggccgcaaggccagcagtaatcatcaaacgggtgcgggaattgtgcatttcgttatcctcgggatgaattgcgttgattacgtgaaagccttcggccttcagcttttcgctaagtctagacattctttcaatgtcgtcgtaggcgaatccttcgtcaatgaataccatgcggtgcattgccgtttccattgtgggcttaattaaatggctgacggtagggaacgaccctactaccctacgcgcccgatgaatgggaatcgcgttgctttacgatatagctacgtcagccacgaacacacattacgacggtcatttggccttgtcaagcactttcagaaagaaattacgtcgattccttccttggctcgccattgttccagtgttgacgatcttacgatcacaattcgcccgttgtcctgcctgctgaagaaatagcctgtcggcttatcgttcaatcggcttacgatttggtcgggggtatcgcccaggttataacgaatgattgcgctgaacttagctcgcgcaatttcgcatcgcacgcactcagccatgttctagatactcccgaatcacgcggacggccatttgccaggaatcgcatacgatgaacccgaagccctgcgacaagacgaattcgccgaattccttttgctcggcagacgtaccgcgaatgtttccaggcttcttcatttcgatatacagcccggagaactgcccgcgcttgactggcaagaaaatgtcgctaacgccaacctttacgccttcggctttcatttgtccgccgcgaatggctcggctgtcagccgtatcgccgcgcgatccgccattgggtacggcgtgaagccacttcaattcaggaatgccgatcttcggcgaatatttgaatgcttccttgcccatcgcatcgaagttatcggctacgtcgaagccgtgatgaatggcaattgccgcccaacagaaaacggccctttgatggccgctttctgtccccgattttgctagcgaggatggcgtaatcatagcaaaagcacctgtgttggcgcttcgccttcattgtttgcgactggcgttgcttcagtgacttcgccgacttcttcattgccgccaaatgcgacaacaaccaaatcgccatgctcgccctgcaattcgcctaggcgttccatcaattcggaaatcttcattgcacgcgcctccacttgcgtccaggccaatcggtataaccttggcctacggctaaggctaaaattcgttcggcgtcatactcggtaaggtcgtcgtcttcggcaatgtcttgttcgtcaatctcgcccaggttttcggtgtttacgaacagcttcattcgtttgctcccgtcaaaacgttgtgcttgaaagcttcaaccatgaaaaagccgtcggctacttttgttccgccgaatcctataacgcaaactcgaccgtctttatcgtatcccaagaccatgccgctttcaatgccttcgctatctgcggtatggcctgcttgtattgcgtcaacactgttgccgtcaattctgcgaacattgctcatggcagcccccgcctgtcacggcatccgccgcacacgtcttcaacctgctgtgttgtcggaacgaacaccggcacaacgcgggccttttcttcgccgcagaaatagcactcgcctgcatagcccttgggaatgcttgcggctttcctggctgcgtcggccaccagcaatgcagtttcgttttcaacccgttcgttcgttacgtcaatttcgtcggccatcccaattcccctagttatcgacatacggaaggcgacccggttcggatcgccttttgcttcgcttgcgctcaatacgatcaagctcagcttctaccaatttaatcgcatcgtcaagcggaacggctatttcgtccctacgatgccccattgtcgcctgccttacttcggcagtgaacttgccttgccagttagaaccgtccctggccctgcgcaaccgacttagcacgatttcaagcttgcgcttgttcatataagcctcgctgtttgcgtagccagattacgacaaagctttgcctaacgcaagcacgtcgggcaaagcttttctgaaccgttaagcttgttttgcgaacccttccagccgtagtgccaagcctgcgcttgttccgaatccctcgggaaatacggattgtcgtcaaccttggccccgtcatagcctgccgccattccggcattgatttcgcgggtgtatttcgatttgtctttgtagcgttcgaagttgatgcgctcagccacgcccattgccccatccggtaacagccggaccgctgacccatccagacgtggcgggcttggcgactgtatcacatgcgccagcaggggcattgcccacatgatagcgccagccgttcggccccaggtcgcccaggctgaacagttcgccgccgtagacgatcaccttttgcttaggatcgtcttcgacggtcttgttgttgtggcttccgcctagcagctttacggttggcattacaactcctttccgcaacattcgcagacattgcgctttgcgttcattgcctgtttgaacttgtgcgcagcttcccagcgggcttttacttcgtcgctaaccctggcccatttgccaggaagcggcgacacccgccaatagctacgcttcgatttagggtaatgttcaagccaaatgcgtggaagctgcttgctcatttcggctctaccggtttgaagtggcccaatcgaaccatagcttcgatgattcgatccgtatcgcatcccgtatcgtcagacaccattgcgaacagcctttcggtgctaatgctgtcggtgtcgtgccgatcccatgaggcggcaattcgcgcgtcggtcttgcgctgtctcttgctcatgcttcctccctggctttcagccagccgcgaacccagccttgacgctcttcagagccttgcagatagttgcccggcaacagattgtgagcgtgcgaaaacgacggcattgcgtgctttggcatgttgcacaaagcttcaacgaatgcgtcgtaaccttcctgttcgaatttgtccattacgcccgccaattcaacatgcgagtcagttctttcaaacgcttcaggcttacacctgcgtcacttccgacgtaaatcatacgcgaatctacgtcgtaagtgtagcctgtaggaactacgccgaagactttcttgtaagcttcttcgtgcgcaatgcaagccttgtctacgctagcgggagcgttcaagacgatgggcttgcggggcggacaggctgcgtcctgaatttcgaattcttcagtcattattctaacccattacgaacgttaaggtgaatttcgaaatcccaataaagcttgcggtctacagcgtacttcagcctttcaattgaagcatgtgattgggcattgtatttccaccgcttaagcattttgctccaaacgagacgcggcttaggcttgattacttctacgtatgcgctgccgtttgttacttgcatcggcaca

SEQ ID NO: 5 - DNA, 42979 bp, unidentified
  source 1..42979: mol_type = genomic DNA
gatttgacgatttatcgtttccagcgcgacgccgcgacgtatgttccgtattggaaagggccggtcgcttcaatcatcattaacggcgaagaagcgacattgcgcacgccaagcaagttcggcaatatcttgcaaggcaatatcccgaacgtgtacgtacaaccgccgtgcaataacgttttgttcgacgaacgttgcaaggtaagtcgcgtatctaattcgctggatactgtcgtatctgcgataagttcggacggcttgcaaatcagcatcccgtcgattggttcgtttccgaacggatggtttgtcggcggcgaaatcgcaattccggcacgcaacgaacgccgaatgatcgttgcgcaagctggcgcaattctaacggtcaactatggattttcgcgtatttctgtcggcacgtcgattcaagttacggcgggctgcgatcatagcttcacaagcgcgaacggttgtccaaagttcaacaaccaaataaacttcggcggttgcccgtttgttccgggcgaatcgaataacccatttacgaacggaattagctaatatgtgggtcgcaatcgttatcgcggtaatcgcgttgcttatggtcgcgtttatgccgaaaccgaacgtcgaaaacgcgcgggcggcgaagcttggcgacttccaagttccccggtcgaaatacggcgatcccatgcccttagtgtggggaactgttcgccaaaagtcgccgattacattttggttcggtgacttccgcccggttccgattaagaagaaagtttcttcgggcttgttcagttcgaagaaggttattacgggttataaaaactacgtcggtatcgactgctgtttgtgccttgggccgggcgtcgtacttcgtaagttttgggccggtacgtatcttgtttggactggcaccgcttcgggcattacgaatatcgtaatcaatcaaccgaacttgtttggcggcgaagatcaacgcggcgggctgcaaggtacgttcacgttttacgatggccgttacgatccgccgcgcgattcgtacttggcttcggttcttgatccaaacgttccggcgtacaacggttttgcgcgtgccttgtttaagtcgttttatatcggcacgacgactaatcttgaaatgttcagcttcgaaatttcgcgtatgacttccggtcttcacgcgacgtattcgattatgccgaacggtcttgatttgaacccgatggaaattgcatatgacgccattacgcagaagttcgggcgcttcggcaatttgccttcggttttggacttgccttcgttcgttgcgtgcgcgcaaacgctgtataacgaacaaatgggcatgtctatggccgcgcaatcggccattacgggcaaagacctgttagaagaaattatgcggcaatgcgacggcttgctgtatcaagacccggcaacttcaaagattgttgcgaagttgattcgccaagactacgacattaacactttgccggttcttgacgaatccatcattaaggatttgaagaacttttcgaaaacgacttgggatagtacgttcaatcaatgccgcgttacgttcaaggatcgcgcaggcgattacgacgacagcgtagccattgcccaagacttcgcaaatatcaactatcaacagcgcgtcaagtctaccgaaatttcttcgccgggctgtacgactgccgaagttgcaaacaagcttgcagcgcgtcaactttcgttgattagcgttccgctgtataagtgcgacattacttgcaatcgcaaggcttcgacgcttcgtccgggcgacgtgttcgttctgaattgggggccgttcaacctgcaaaaaatggtcatgcgagtttcgaaaatcgaccttggcgaacttacgtcgggggaagtgaagatttcttgcgttcaagaccgattcgctacggcgacacctacgtttgcgccgcctgattcttcgaactggacgccgattaacacaagcgcaaatgccgtgacggtgcgtagcttctttacgccgccgcacttcttggcgcgccttactccgaacgaagccctttcgacgttcgacagtcaaggccggttgtatatcttggctaaggggccgtcgtcggcgtctatttcgttcgatgccatgttcagcggcgacaacttcgctaccgatcccacactagccattgaagcggccccgtacaacggcggcggcacgctgtcggctgcatatgcgaacacggttgcggcagacacgcgacacgacacgacgggcgctttcaatgttcaaggcgtgtcgtcggcagacattgcgaacttgcagcaatatacgacacttgaccaagcgcgcgacggttccgcgttgcttatggtcaataacgaactgttcgtttatgtcggcttcgttgataacggcgacggttccgttactttcccgaacctatatcgcggcgttctggacaccgtaccggcaagccatgcggcaggcgaccgcgtttggttcgttggcggcatcgacggtttgattccgcagcttgtgaacaatagtgcgacaggttacgttaagctgttggatacgacgacttcggacaagttgccgctgtcgtccgccccgaccgtatccgccgcgcagaatggccgcgcacgcctgccgtatcagccgcagaaccttacccttgacggtagccgtacccctgccccagccacgggcgcaacgtcgatcacggcggcatgggcacgccgcagccgcgaagcgcaagccctgtccgtcttcaacgacgccgacgccgggctagaaaccgggacgcaaacgcgcgtgcggtggcgcgtcggcggtggcggatatactacggtcatggtttccggcacttcgacgacgcttaacgtaaccggccttgtcggtacgttggaagttatcgtagatacgcaaatcacggcaagcgggctgttcagtacgaacagcgaacgcttgaccatgacgctatcttaaaagaacgcaagttcgccgttcttggctttcttcaaacgtccgcagtcgtacagcatttcgaccgcttcgtttatgtaccagtcgtaatttatatcgtcgggaaattcggtcggcaagtccattacagggcgcgcgccgtccgttttcccgactttgtttccgctggcaacgtaagcgatatacccggcttcgttcttcgggtaataccaacgaacgaccttgcccaagaaacgcccgttcttttcgccgccgccatgaacgttcttcacgcatacgaagcgccgaaagtcgcggcattccttaatcgtcttttctactggcgttccttcgacaagaaaccgaataaccgcgtccgaacatatcaaagcttcggggttcttcgacagaatcgaattaagcgcggaaccgcgttcgcaataagcgcccttcgtcttagcgcctaatttttcatccaagaaacgcgcttcggcgtcgccgccgtcgtccttgattgcgacatagctattaacgtcgcgcgaatatacggccttgtatcgcgtttcttcggtcttgtatcccgtatgcgcttcccatgctgcaatcaaattgcggacttcttcatgccgcgacttgtgatatttcgaaatgaagccgtctgtattgccggaaatgacttcgacgccgattccttcgattgcttcgataagcataagcaatacaagctgtccggtaatcgtcacttgcaacataagttgcggcgcgtacagcgtcgaatatttgttgccaagtttgccgaagcttccgttaatcgtaatcttcaagctgtcggcaattaccttccatttcttcgcgcctttacggtcgccttctttcttgcacttcgccgccattgccttagcgtgaattcgcgtttcgacgatcttgttataaaccatcaagaacgcttcgcccaagtgcggcgggaacagcttttgattaaggattgtgcgcggatagaacgattctacgtcgttatccgctagaataatatcttcggttgcgacatgcgcggtcttcttttctgtcgaatgaaggccgcccattccaagtttatacgtcgatttgccgatagttactttcagcttttcaatttcggtcggcatgatgggcgaacccaagccgtccagatagaacgccgcgccgcgcacgacttctaacatttgctgtaactgcggcgtctggaaacaaacgaagtccggtacgttgtaatacaacgggccgtcgtctgttagtgtgggcttcttcggatagtaacccaacaccttttcaagttctttattgattaccgcttcggctacctgcgcatcggatttcgaccgaagttctacgccgtattcttccgacatttcggcccgcaacttcaattcgggcgcaagttcgttaaacagaagttccgtattcgcaaggtcgttgcagcagtacgggcgaacgattgcggcatcttcgcgcgtcaatacgtgcgtttcgggaaatggcaagtcctgcatacgttcgcaatgcagccgaccggcgtacagcttcaacgatgccgggcgcgcagtaacgccgccgttcaccgggcaaacgttgaacaagtcgatatggttgtagcggccaatttgtacgccgtacttcttttcgaagtcgaacggcgtaaccttcttcgtaccgtaggccgggccgcttttaatgatgaagtccgaagcttctttaagcttggcgcacgatgcaccgcgcgccgcaagttcgatcatgggcaagtcatacgatgcgctgttgaagcccacaatacagaatcgccaaagcatccaaagaagcttcgtcgggttaaagtcatggtcgggcgaacgttcaaacgcgacgaactttccggtatcaagcgacttaaacgcgacataccaaaaattgatatacgtttcaacgtcaaagacgaagacgcttccagcgggaagcgccattagttcttcgtccgacatgaattcgacaggccgcaaagcatggcgaatgcttgcggccaacttatcgacgacgcggcttttcttggcaacgatgaagccttgttcgttcaacatatgacagccccttagaacggtatatcgtccgaatacggatcatccgaagttcggttaatgtacgtatcttccgactgttcagtatacgacgcttcggttccaaggtcaagccccataactgcgccgcgcacgttgtcgccgtagaaaattactttgttcgtttcggcgtcgaaatgcgctttcttgaatgcgtgttcgacggaaagcaaaagctttgcactgaaccccattcgttccggcaagccttcaatacgatacgtcgaagcttcttctttgtgcatacgcgacaataccgcgccatcttcgaagaagacatggccgttcggactgaacgattcgatagcacgaacgccccggtaaaagtcttcggggatcggccaaaggttcagattcggaacgtccagaaccgaagcgtaattcgggtaacgttcgccgtaaagctgcgacttgataaacgaaccgtcttcgaaatagaacgtcgccgacgactgcgaatagccgaacccggtaagcgccttcgacgccttcgcaatggccgacgctgcggccttcggaagcataaggccgggcggaaggtcgatgccgtgccacgcttccagcagggccgccccgttcgtcgctacggcgcttccagcttgcagcaggacggcggcataggtcgcattcggcgcgccgtccgttgccagccctgcgaccgcagccaaggccgctttaacccggtcgtcgatcacggcgcattgcggatcgggcggcatgatgggcacttcgtcgaacgctacgcacggcacaagcgcccggaatacgccggacgatacggcaagcgtgttcgccgtaagttgcgtaatcgacagttcgtcgctagccttcgacagtgcgtcgataaactgcaacgtatgcggacacgcggtcaagtcttcttcaattggcgcggccacggtcaagacgccatcgaaggccgccgcccaattgtgggcaatgtggccgaactgaatatttaccggcccggccttcttctgcgcgaccgaaataaacttcaatgctgcgataagcgaagcggcggggttcgccgtcttcttcgctgtcgtgccttcggcttgcttgcgtgcgcggcttttgcgcttcggcttttccggcgttgcaggaatcggaacgtcgttttcaatttgcgttgtcatagtttcaccattcagcggaaagaacttcgggatacttcttgttcacccaaacgcgaagccttgcgggcgttcgaagttcggatacacgttgcaaagcctgatacgtcgtcggcggcggttcttcgcggtgccgctgtcgccaccagtcccgcgaacgtttcgccgcaagtccggggtgttcaagcatcacaaattcgttaaacatttggaagccgcaaaagtacgatactttaatcatcggcggctttgtcaagttgccttgtgcgtcgcgtttttcgtgaaggttgtatatcaccttttgtacgtcgaaatattcgactatcggcgcatcgctgcgcaacggttcagcaacgcccggcgtcgcaaacaactttgtttcgaagctgaattcggcaccgcagttaatgcactggcgcgcggcagcatggttgtatacgccgcaaacttcgcaaatgcgaaccggcgcgtcgccgccacctttgccgggacgattcggaatacgcgggtcgttgatcgggccaaggcgacgaatgttcgccgcgaagtcgccgacaagacaattcatcttgccagtttcagggcttgggcgcgttccgcgtccgtacttctgtacgtgtttgcccggcgatagcgtcgggttcaaatcgccgatgaagtcgattgccggatggtcgaaacccgttgtaagtttctgcccggatacgatgccgcgaagttcgcccgctttgaatgcgcgcaaacgttcggtattaactttgtctttcaactttgaatgcacgggcaatacttccagcccgtaagactgaatcacgtttgcgacgtgttcggtattgtcaatgccagttgcgaagacaagccaagtcgaacggttatacgccatttccatcatttcgcggacggcgttaaacactacgtcgtcatcgtctgcggccttttcaagctgtttcgaattgaattcgccgccgactacaccaacgccggaaatgtcgatttcggttttcgtcgggcgcgcgataagcggcgacaagtacccttcggcgatcaaccgattaaacgattcaacgccggtaatgtcgtaacaaatatcggtgaagattccgttatcggtaatcatgcccattttcatacgatagggcgttgcggtgaatccgataactttaagatgcgggttaatcgcgcgcaattcggcgataatgtactgatagaacgaatcttctttatccgaaagcaaatggcattcgtcaatcaacagcaagtcgcgccatccgaaatggcgaagatgcggcgggcgtccatcgttctgttcaagcgcctttttaatcgccggggctacggactgaacgccgccgaatacgataggcataatcatttcgcggctgttcaagcctgcggaatagataccaaggggcgcagtcggccaaaccgacattagcttttcggcgttctgttcgatcaattctttaacgtgcgtcaacatcattattcgctgattcggccaaagtccgaaaatgcgacgaatgaagttagcaattacaacagatttgccggttccggtcggcatagcgacgaccgggtttccgacgtttccgcgctggaaatagtcgaagatcgaatattcggcttcgtcctgataccagcgcggtacgtagatactagacattttgcgttgtcgccgtgataggtacgtaagacgggcaagcctgcggtacgaagtcgcggggaattacgccgttatgcacgtcgcaaaaccattcgccattttcgaccggacgggccgccttgcagctacgacagttcttttcaggaatcgcgcctttgtggcaaatgtccttcgccgcgcaatacgtgcaatccttgaacgtcggattatcggaaagacgcggcggcggttcctgcgacagaatgatttgttcggccttttcccgcatttgctggcctaaccgatgatccaacttcacaagttcgacgtgtaacgaatcgtcgttcttgttaatgttgaagtacagtacgtaacggaatccgtatgccgcgtcgcttccatacgttgaagtttggcaaaaatgctgcggcttcgcaacaggcataccggcttcgccaagcttgttaaagcctgcgccggttccgttcgtcttgaattccagcaatacgggttcgtcgattccgtagcgcgccggaagctttgcgataccgtcaagcgatccgccgaaatgcccattcaccgccgacacgcgatattgtgggaattccaagccgtccgccttagcgcgtgcgacgtgttgcgtatagtacggatgttccttcgtaatcggtgacgaaaggccgtcgccttcttcgccgggcttcgcaatccaatacgaatcgctttcggcgtgatacataagaccgtcgcggttttcgtaccaaacttcggccccgatgccttccagccattcgataaagcgggcttcttcacgatgcccacgattaaacagccgttgcttgcgtccgtccgtctgttcgcggaacgtccagcggaacagataccaaagcttgcgcttgcagccgtcgccgatcaacgacgcgccaaggtgccagcggtggccgccgtcataggtgcgaacgcaatattcgtctatgtcttcaaggatgcgcttagaaagcgccttcgctacgccgggcgcgtcaagtgcgacgttttgttttccggcgtcgggcttcgtcgctggcgcgtcgttcagcgttaattgcgcgttcggttcgcttttcttgcttggcatcgttcttcacctttcgccggacaagtgcggcgtaattgttcgttagatagtcggcggaaagcgtcgcaacgtctttaagttgatccttcgataaccaactgatatggcattcggaagcgtctatgccaagttgcgccgcaagccaattgtacgccttcgaccgtgacattgagccagtttgccaaagacggtcgaattcgtcatgcgcttttgttcgaagctgtcgcgtagcacggtcggccatacgaccaagcggaataaacgtgccgggatgacagccgacagcggcgcgacagtcgttgcagaaataaatatgcggccaatcgccgtaacggcgaccgtaaatccggtcgtttgttgttagttcgatgttgaatgaacaacaggtatcgcattgttcgggtacgggcaatgcgtctttgattttcgacatacttacgcttttccccataaaagaacgccggggccggtgaaagccccggcgatgttacgccgctacgctagttcgtcttagcgtgcgccccaaggtgcggcaccgccagccggtgcgccgccctgcggttgctgctgccagccgcccggctgtccgccctgcggggccgcgttctgctgcggctgctggccgccccaagctgcgccgttgccctgcggctgctgcggctgctgttggggctgctggccccatgccgcgccgccttgggccggttgctgctgcgcgggctgctgctggccctgcggctggccgccccatgcgccgccctgcgcgggctgttgctgcggctgttgaccgaagccgccttggccctgcggctgctgtccgaagcctgcggcggcctgctgcggctgcgccggggctgcgccctgtccggccttgcccggttcgttgccgttcatgtcgaacacctttttaacttcggtgtactgcgggtcgttcttctgcggcccgacttcgataaggaacgggattccgtgaagctgcgacgaatcgttgatttggaacacgccgataacgtggcagactgcggacaactggcggtgcgcgatttcgaccgtctgttggttcgtatggtacaggttcaggcgatacgcgccggtcgtgccagcctgcgggccgtcgataatccgcaagttcagttgcagataaccgccgtcgttcgccttgttcgccttcacttcggaagtttcgacgataaccggatgcttgccgatgggcaggcttccgacgccttgggtcgggtcgtattgctgcgcgttgaaaggttgaatcagttgcatggtatttaccttttcgaaaagtcttcgccgttggttacggtggcaaagttaccgtttttggctgcgccggtaggattcgaacctacgaatgccggaatcaaaatccggtgccttaccgcttggcgacggcgcaaaagcttattgcatcgctttcgtgaaaagcgccgacaaatcgggcggttcaagttcgcccaagttgcccaaacgatcacgcgcgaacacttcgggaatttccttcgtccgcaacgcccgaaccggcttcggctggcccggtacgatagcttcgcccaagtgcaacacgttgtcgaacaggtgcggaacctttacgttaaggtctttgccggggaagaacggtcgcttttgcatgatcggttcgtatacgacttcgccgccctgcaagatggtttgccgtccgttttccatgacgccttgtttcgcaatcattacgatatgcttttgcggcatgtaatacaagtcgttgcaaattttcatcgtgcgttcggacatattgccgtatgccttcatgccgtgtttaaccttcgacagttcttcggccaagatgatttcggcaatgttcgaaatactgtcaatgcccaaggtgtcgaagttcgcggcttcgcgcgacttcataaaccattcgaagaattcggtaatcagcgccggggaatacgcttcccatgcgggcacgttcgaaccgcgcatggacaacatgccgggttcagtgaccaacagcacggggcgcggtgcggtgttgataagcggcgtcttgcccgaaccgggcgaaccgaatacgacggactttacgccatagcgtcgggccagttgcgacgccggtttaagctgcgacatttgcattttgtttactccgattaaagcggcattattgacgacgccgacgctttcgctttcccgactgtccgttatggcactatgcgacgcgatgcgcggcccggactttcgatgccgtcaagaatgccgccttgattgtgggcaaggcggcaagtacgttacttcttcgccttcggttccttgatttcaagggtcggcgtaccttccgacgtaacgataacgtcgtcaatgatcttgcggaagttgtcgggaagttgcttgtattcggtaagcgaaagttccggcgtccacttaaccaaacgttcggcgatcaattcgccagcttgtccggtcttttcgatcttcgacaacgccttttcaatgcgcgccttgtcggtcttgccttcggcgttctggacgaagccgtagcgaaccggaaccttcatcgtcgctttgtaaccgccgccaagttcgacgttttcggtcgtgccggacttcgccggatcgtgcatgaacatcacggccagcttgcgggcttccaattcggcttctttggcgacttcaagcgcggccttcttcgcctgccaatcgaccaacagacggtcgcgttcggcgatatattcggcttcgctgtagttcttgacttcgcccgtttccgggttcgttacctgaatgatattcggggtcatctttgcacctttcttcgttgggccgccgcacgttgcgccggtatgtgcgtaatgtacgacggcccgtttcggttgtcaagccttttgttcaagaatttttcgttcttcgaacaagtcccgattgttcgcgtcgtgttcggtgaacttctgcgggaaccgcttacgaagcttggcgatgttcacggcctgcgcttcgccgaagttcgaaccgatggcgcgaagcaacagcgcatcgtaccaaaagccgtcgccgacttcttcaagcgcgttcacgtcgtcgaatacggcaccttcggcggtcgccgacagggcttccagcagttcgcccgcttcggtcgctttgccgatgattgcatgaacgatattgacggcgcgcgcgttggcttcgtcggtgccatcggtggcgatccagtcgggcagcttggcaagcgtgccggtgttgtcgccgggggcaggaacgccgcagtcgcggccatagaaaagcgtcttcttgatcgcgtccagcttcaccagtgcggcgacagcttcggcgatggtttcgcggaagtagccaagcgacacgcggtcgccgtgatagctacccgacgcggttacgtgcgcttcttcgatatagtcgaaggtcttttcgggttcgttcattgcttgcacctttcaaagtcgccgggcaccgcgccgcagcgttccgacactgtagcgccgggcgtgttgcctgtcaacaaaattttgtcttgcctgctagaattttgtcgggtatagtgtcgttcattttgcccacattgaaccggaaacatggtgcgaacatggccgaaattacgaagctgcgggatgaaacccgcgaactgttgttgaaccgtccggcttcgctggctgttggcactattgccgaagctatgggcgtgtcgaagtcttggcttaatgccttcgcgcgcggcgacattgaaaaccccggcgtcgttacgattgaaacgcttaacgtctatttgaagaagtttgcgaagaaggcaaattgacaatgtatcaaaacatacctatcgaaatgcggacttatccgcaatgggttatgtggcggtacgaagacacggattcgaagaaacctactaaggttccgtattccgcccgtaccggcgcactcgccagcgttacagacgcgaacacttggggaacatttgacgaatgtttgcacgcgcttaattccggctggtataacggaatcgggttcgtgttgaccgatgccgacccgtattcatttatcgaccttgacgacacgaaaggcgatcaaacggcgcttgatcgtcaaatcaaaatctacaacgaattcgacagctacgccgaacgttcgccgtccggttcggggctgcatatcatcgtaaagggcgcggttcctgctggccgtcgtcggtcgtttatcgaagtgtattcgtcgcttcgttatatgaccatgacgggcgacatttaccgtaatgcgccgatcaaagaacaaaacgaactgttgaacattctttgggggcaaatggggcaaggttctgtcgccgttgcgcattacgcaggcgtcgccgaagccaaggaaaccgacgaacaggtttataaccgtgccgtcgccgcagccaacggggataagttcgccgaactgttcgcgggtaaatgggaaggcatgtacgcttcgcagtccgaagccgacttcgcattggtcgatattatcgcgttctatacgcagaaccgggcgcagattgcccgcatgttccgactgtccggcttgggccagcgtgacaaggcgaagcgtgacgattacgtatcgtacatgcttaacaaatgctttgaccgcatgttgccgcccgtcgatattgacggactgaaaaacaagcttgacgaagcaatagccgcaaaagaagcccgcgaccgtgccgaagccgcatcgttgaataccaacgttccgcaagcgccaatcgtcgcgccatccattcccgaaacgtcgaaggtgtattcagtgccgcccggacttgtcggcgaaatcgcccaatatatctacgcacaagcgccccgcccggttcccgaaattgcgttggctggcgcgcttggtcttgtcgctggcatcgtaggccgtgcgtacaatatcagcggcaccggccttaatcagtacgtattgctgttggccccgaccggaacgggtaaagaagccatcgcatccggcattgacaagctaatggcgcaagttatccgcaccgtaccggctgcaagcgacttcatcggccccggtgaaatcgcatcggcgcaagcgatcattaaatatatgtcgaaggggccaacgtcgtttgtatcgttggtcggcgaattcggcatctatcttcaacaaatggcaagcttgaacgcgccgccgcatcttttggggctgcgtcgtttcatgctggacgcttacaacaaatccggcgaaggcaaggttcttcgtccgtccatctattcggacaaggacaagaacactaccgcagttcttgcgccgtcgttttcgttgcttggcgaatcaacgcccgaaaagttttacgaaggcttgcacgaaggtttgattaccgaaggtcttttgccgcgctttacgatgattgaatatcatggtcaagtgccgccgttgaacaaggccggggcgcgcgtgcaaccgtcgttcgaacttatcgaccgtctttcgacgctttgcgcgcattcgcttatgttgaacagccaacataaagcgatccatgttcaatttgccgaaggcgtcgaacaagcttccgacaagttcgaagaacattgccgcaataacgtaaacagtagcgaccgcgacgttaagcgccaactatggtcgcgcgcccatatgaaggctttaaagctggccggtatcgtagcggtcggcaataacccatacgaccccgttattacgtcggacgttctgtcatgggcaaccggcgtaatcgttgcagacgtgcgcaacttgcttgcacgcttcgacgctggcgaaattggcgtagacaacgacgaaacgaaacagcttgcgaaggttattgcgacggttaaagatttcgtcgtatcgccttggccggaagttgcgaagtatgcaggcgaaggcgcaagcaacttgcattcgaaccgcattgttccgtatagctacgtacagcgtcggcttgccgccgtgtcggtcttccgtaaagatcgcatcggcgcgtctggcgcaatcaagcgtgcattgaagacgctatgcgaacggggcgacctgcaagaagtgtcgcgggctacgctgtcgaaggactacggaacgtccgccgtcgcgtacatgatcgcgcatcccggcgtcttcggcctgtagcggggccgggtagtgtgggcagaactggccgccttcgggcggctttttcatgccttaacgaaagttgaacgtatttcccgacgaacggtcgaaaagttgttgacgaagcttcgaagtcggcgtagtatttaatccatcgaagcaacgaacacgacgaaggagttacgaacatgaacaaccaagaaacctttttcgaagaactgcaacgcatcggcgaaattcgccaaggtaacgcagttcttaccaaagaccgcgaaggcttccatttccgcaacgcgcgcaatctgttttcgaagttccgtcacgacttgccagccgacgccagcgccgaacgtgtcgaagcgcattggaacggctttgtcgccaacatgcgcgcagcgaacgcagcttaaccccgtaagccagccccggcccttggcgcacgctaggggccgcgcagcctgcccacaatgaccgaaggtgcaaccatgaacctagaagccgcagacgtgcgcgtagacacgttccgcaagcccggcgcgtccgcatgggtcgccagccccgaaacctgcgttcgcgtgacgcacattccgaccggcgtttttgtcgaacgctgcgaccttcgttcggcgcacgctaacaagtccgcagcaatggcagaccttcgcaagaagcttgacaaactgccgaagatcaaaccgcgtatttattggcagtattacccgaagtcccgtcgcggttactggaaggtttcgcatatgccgaagccttggaagccggaagacgcgccgttttgggataaggcgcacgaattcgcccgccgtttgaatgacgcgataaccgcgaagattgaacaggaacgcgcaagctatcccgtcgtcgatacggtcgaacagttggacaacctgccgcccggaacgtatatcgtcaccggctgcgcatccgaagaaatggcgcgtcgcatggcgttgcatctattaaagaaggagttatcgaagttggcgctggcgttctggcgtctggccgctactgcattcgaagccgcttactactgcgcaaagaacggcgaacgttcgaaggcatggcgcttcatccttcgcggcatcttctgcgcgttttggctttcgctaatgattgcgcccgtcgttcgtttcttcgatagcttcgacgtgattagcatagacgaagcgccgcctatggttgcgccgaagcgttcgacagaccttcgcgtataatagacgatggaaagtataagggggctgtagaacacgcaaagccttgtgccataagggtttcagccgaaatttaacgaatataaagtataacgctgattcccccggttccccgcacactttatatattaagtcattctttatacataatgatttttaggtattatacttattaaacttattatatattcttatttttcaaggacttaggcattcttcgaccccttcaattcgtataacggccatttcacgttataaagttgttgacatacaaaatttatatggtatgcttgcggctgtagatcaacgaaaggggcttgaaatggcatacgaagtcatcgaatgttcgccgaaggcgcgcggtaaaatcgcatccttcgaagacgcaatcggaactgaaaccgaactgtcgcaccagcgttcgaagtatccttggccgttgctgaaaatcggccagtcgttcacggtgccgcttgcagaaggtaacgaagcatcgttgcgcaacggcgcggcgcagtacgcaaagaagaccggcaagaaatttaccgtcattcgtcacggcgaatacgcttgcttcgaagttgcgcggatcgcatgaacgcgcgggccaatgtgggcaacaaccgaaggggcaaccgatgaacaagattgcacaagcatttgaccgcctgaacgaagcaacgaagggcgcaaccgaagcaatgcagaacttcaccgcagcttatgcggttgaagacgggcacaagatgccgaaggcgcgtcgcaaggctggaagcgaaccgccagcggtgaagactgcatttaacgaatacgcggacgcatacaaagctgtttacggcgtgcgtccgctgtcgtatacttacgacgtaacgacgaagtttattcgcatcgaaaacagcggcggcgtaagcttgtcgcgtttgcgcgaaatgacgaagcaacttcgttaccgcaaaggttgacagcttcgaagtttaatcgtagtattgcaatgcgaaccgggcgcttcccggcaattgaaaggagttaacgaaatgtgcatcgtttgtgacattaagcgcatgaacccgtcgcccgaagttatggcgaaggtcgaagaattggcgcgcggtctggatactgctttgaccgtggcgcaagaagtcgccgaagcgaaccccggcgcgttcaacgatgaacagcgcgaccgtatgcagtccgccgccgacctgctgaatcagcgcgaaggcggcatcggcgggcttgccgcgatccttgcggccatccttggcggcgcgcgtgtcgaagttgcgcacgtcgaattgcgcgacggcgaaagccccgaagacgccgtagaacgctacatggccgaaaagaaggccgaagcgtcgaagaacgaaaccaagcgttgaccgaaagccccggctagtgtatagtcggggcttcttcgtaggggaacgaaaccaacatggccgacgaaatagacgcaacagccgaccgcatggacaacgaactagcgttgaccatcgccaacacttgccgcattgccgccgcgattccgaaaggctatcccggcgaatgcttcttttgcggcgaagacttcgcccgcgtcgtcgaagtgaccgacccgcgcagcggcgaacgtgtcgattcctgcgggcgctgtcgtgacgcaaggggtataaaatgacaccgaacaaacttgcgaaggaatccgaacattcgcaacaggtcgcattgttcgcatacgtagctgtcgcgtatcttcacggcttcgacgtagcggacgaatggtgtaagaccggcaagctaccgaagcgcgatccgaacgcaccgcccgccgtcccggcgcttgaatggttccacgcgatcccgaacggcggtagccgtggcgacgacgaacagtcgcgcaagatacgcggcggccagatgaaggccgaaggcgcacggcagggcatcgccgatacgttcttgccttggccggtctacgaacaaagcccgaccgattcgcaacaaatggtcgtaaaatggtgcggcctttatatcgaaatgaagaagccatcgcttcgcccgaagtcggaaacggcgaagggcggcgcatcggacgaacaaatagccttcggccagtacgcgcagcgcgtcggctacgggtgggccgtctgctatgattgggaacaggccgtttgttaccttcgtagctatatcgaatgggggcagaaatgaacaaagacgaagccgccgcactgttcgaacaagtcaaggcgaaccgtgctaagattgacggatgccgaaaacaccgcttcgacattggcgacccgccgtatcgcttcggacagaagttcgtatgcgccaactgcgggggcgaaatggacgccgtacaggcgttccgctactgccaaggctacgaagcggcgggcggcgacccgaacgaagtaataccgggcttccgctaatggattgcctgaaatgcgaactaacccgcgcgaagcttaaaacggctggcctgctaattgtgggctggccgttgtcgcgtattgctgaacacctttccgactgctacggcgaacgttactacgtcgaaggcgacaagctgtaccgggcgtcgaagcttccgccgtatgaaccgcacttgataaggagtaacgaaaatgacacttgacgaagccaagaagaaggcgcgcgaacatcgttgtttcatcgtgacgaaggccgattgtttcttgctgtaccgcgaatcggtgccgaagaacgtatgcgtcggcaaacggaaggacgaaaaaggcatcatcgcgctagtgaaaaaagcttgcgcgaccgcttgacgtagcttcgaaaccgtcgtagactatgcccatagtcaacgaacaaggggcacgaaatgggcgcatacaccgtaaaaactgaattcgaaatgaacgacggtcgcattctgtcgtgcgaatacggcgtatcgttcacgccgggcaactattccggtctgcccgaaaactgctaccccgacgaaagcgaagcgggcgaaccgacgtactatatcgacggcgaagaagtcgattacaaggacttgccgaaaggtcttgacaagatcgccgacaagttgtacgaagccgggccgggcgaatacggctacagcgaaaccgaaccggactacgacggcccggactacgaacccgacgactattattgaaggagtaaccgcaatgcctaccattgccgaactgttttggcacttcgtcacgctttccagcggcgtaaccattggcctaatgttggccgcatggttgcgtatgcaatcgaaagtcaccgaagaaacttacgacaccgattgcgaattcgtaaccgaatatatcgccaacatggaaagcggcccgaagatcattcgtcgcccgctgtcgcaatggccgatatgggcggacagcattaacccggccaagacgaacccgcccgaacctgaaccgccgattcgtattgaacgaaattttatcggcaaaaaggattgacaaccgttcggaaccgtcgtagtcttgttcgtaccaactggcaacctaaaggaatcgccgccatgtacgcacttattcttatcgcttgcaccgtcgttgctgtcgctattcacttagggcttgtccgtcccgtaatgcacgccatcgaacgccagagcgaagaatcgcggcgtcgtgcggcgcttgaagctggcttggccgctgcggcgcgcttgcaggcgttcaacgcccgtaagccgtcgaaccatcgcggcgcaaagctgaatgccgaacgcgaatggcggtcgcaggaatgaagcgcggtcacgttatttacacgcacccggacgaactgtcgaaatgggatcgccggtttatcgaactggcggaacaagtcgcgtcatggtcgaaggggccgcgcaagcgcataggcgcggccatcgtccggcctgataggtctatcgcgtcgcttggctacaacggcccgccgcgcggcttcgacgatgaagccttcttgcgcatgacgcgcgaagaacaacacgccgtcgtaattcacgccgaagcgaacgccattgcgcaggcgcacgacggcgaagccttggacggttacacgctgtacgtgtcgccgctgttcccgtgcgccgtctgcgcccgtcgcatcgttgacgcaggcattcggcgcgttgtcgcctattgtgggcacatttccccggactggcgcgcgtctgccgatgaagccgaagaagtcttcatcgctgcgggcgtcgaatgtctgttcagcatggattaacgaatatgacgcttgaccattcgcaaatcgaaggactgttgttcttcgaagaccccgtaacgcataacgtaatcggcgcagctaaggccgcaccgctggacttgtccgggcatttcgtcgcattcgggccgcgtattaccgttgatccgcagttgaagaacttgtttcttgctgcgccgacgttgtatcaaacgctgtcgcagcagtaccaagcgattcaaggtcttatcgaaatcgccgaaggcttgccgcagacgccggaacttgataagctgcaacggtcgttcgtcgaaatgcaaaacggcatgttaatggcgcagcttgtcgcacaaaaaggcatcgaagaagttgcgaattcgcttgacaagccgccgaagtagtcgtagactgtcaaacatcgaaacaacgaactaaggtgcccacgatgaagcgtaatgttaaagtcctgttggcgattgccgccattgttgccgctttcggcgtcgttggttcgatggactaccgcgacgaagtgcgcgaacagctttcatattgtgagaatgtgaagaacggcgtatggccggacttcaaggaatggggcgaaactgaatgccgccccgaacgcatcgcagaacttgaaaatattttgcgttgatcgcttgacacgtcgaacgaacagcgtaaaattacccctgtcgcaataacgcgacgttaactttccttcgaaggagtttcaaaaatggccaagtccaagaagtccaccgctaccgctgccgcttccgccgctgccgtgatcggtcttgctgaaatcgttgcagccggtgcaaacgggctgtatactacccccgaagttcacggcccgcttgtcgaagctggcatggtcgaactgaaccccgtcgggccgaacgaagccggcgaaactctcacccgcgccacgcagaaaggtatcgaatccatgaacaccgcaaccaacaccgccccggccaccgtcgccgctgctgccccgtcgtccttcgccatcgaagacggcatcgccatgccgaccgcttccggtcgcggtcgtggcggcaacgtgtaccccttcgacgccctgaacgtcggccaatcgttcttcgtcccgaacaccgaagacaagccgaacgccgccaagtcgctggcttcgaccgtttccagcgcgaccgcgcgttacgccgaagtcgtcgaaggccagttcaagacgaacaagaagggcgaacaggtgcccgtgacccgcgaaacccgcaagttcgttgttcgcagcgtagaaggcggcgcgcgcgtctggcgtaccgcctaagcgccccggcgtgcggcctacgggccgcgctacggccagaacgaagccccggcactgtccggggcttctttttgcctttctgctggcctacggccattttttcgggtactatcgggacaattcggggcgcagttcgccccttgcgcgtattaaggggctacgtagtgccattgaacaacgaagcgggacaggatatgaacgaacgtccgcagaagatcatagacgcaaaattgccgttaccttggcttatcggttcggcttgcgccgtagtcttttcaatgggcggcgtattcgtcaaactggacgccgtaggcgcatcgcttacgaagctggaagcgaagaccgacacgcgcgacgaacgaatttcaacgcttgcgcaatcgttgatacagcaggccggaaagaacgatacgcaggacgcgcaaattacccgcaacgccgcagacattaccgacttgaaacgcgacgttgaagacatacgcaagtcgcaacgttggatgccgaagtaatgaaaaagaaagtcgaactaatcgaagattggcgcaccgcccataagctttggtcggttcgactgtcggccatcggtgccgccgtaatgggcgtgtttaccgtatggcccgaatccgcgttgtatctttggtcggccatgccgtccgaagtgcgcgcgttgatccccgaacggttcgtatccggcatcgcgcttttcgtattcaccatgtccgcactgtcgcggatcgtcaagcaaaggccgaagaatgaacgaatcgaacgaaagcccgcagaagaaacagccgaataaaaagacgcttgcgggcgtccttggcgcaggtgccgccgcaatcctgctaggcgtagccgggcaaaccggctttaccgaacgcttcgaaggcatggttcttcgcggctaccttgaccctatcggcgttccgacgaagtgcgcaggcgatacatacggcgtcgaagtcggcaagcgatacaccatcgaagaatgccgcgaatcgctggaacagggtttgattaaacacgccgaacccgtgttgaagtgcgcgccgaacctgcgaacgcaaggctaccccttcgcactggccgccgcagtcgatcataactaccatttcggcacgttctgcggaacttcaatcgacgcagcgtttaagcgcggcgactatcgtacaggctgcgcacgcttcaacgaaaacgccgcaggccgcccgcaatgggtgtacgtcaaggacggcaagggcggttacaagacccttcccggccttatcacgcgggccgcagcgcgccgcgaactttgcatgaaaggggccggataatgtgggctatcatcgtagcgggcgcaaagcgtttcggcggctggattctggccgcattgtcgtttctggcgatgctggcgacaatttggcttacgtcccgaaaagtcggtaagtccgaagggcaagccgaagcggcggaacagcgcgcagccgaccgcgaagctatcgcagtacgcgaagttaacgaagcgcgcgaagcttccgaacgtcaaacaaaggcggtgcaaaatgcgaacgaagttgcttccgataatgctgttcttgacgatgacggcgtttctaagcggctgcgcgacgaatggtcgcgcgactaagccgccgcaatccatcgccgaaaccgtgcaaacgaagcccgtagtaatcgacacggcttgcgattgggtgcgggcgatttgggtttcgaagtcggacgacataacgcccggcacggcgcgccaaatcctgaaccataatcaagccgtcgtaaagaactgcgggccgcagaaaccgcccaaggtcgattcgccttaacagaacgtcggccttgcggtatagtgaaggcaaatgcgaatgacaggccgacgccatgaccgaccaacgtaacgaatccgaagaaaaggccgcatatgcggccttgcttttgaaggaacgcgaccccttcaaggctgcgcttcaactgttccccgacaacacgaatcgcgccctatgggtggcgaatcattggccgattgacgccgaagtaaaggccgaacaagaacggttaatgggcgaagacgacggttcgtcgttccttccgtcgaaggccgaacttgcccgcgacatttggcaacgtatgcagggcacgacccttgcaaacggcgtgaccattccgccgacccccgaagaatacgcgaagcttgcgaagctttacgcggacgttcgcgggttcatcgaaaagccgcaaacgaatgtgaacgtaacgacgaacgtacagcgtgtcgtcgaagttcccgttttccaaagcgaaagcgaatgggaaaacgccgccgcacgtcaacagcgggaattgttagaaaatgcccgcactcgccattaaagcgcccgaagcgccgccgctgattctacagaaagcgccgccaatcgaagtcgtatttaagccgcttcccggttcgcagactatcgcgctttgttcgcacgctgcgcataccctgtacgaaggcgcacgcggccccggcaaaactctaacgcagttaatgcgttattaccgtaacgtcggcaaaggttacggtaagttttggcgcggcgttatcttcgatcttgaattcgaccatttggccggacttgtcgccgaatctaaaaaatggttcggcgacaatggtaagttgaaagatggggcgaagttcttagaatcgccgtcccaatacaaatgggtttggccgactggcgaagaactgttgtttcggcacgttaagaagctgtcggattacgaaggcttccacggtcacgaatacccgtttatcggttggaacgaacttacgaagcatccaagcggcgacctttacgacaaatttatgtcggtcaaccgctgtacgttcgacccgataaaagacacgccgaaagacccgaaaaccgggcgttatttgacgcctaacggcctgccgttgcccgaaattaagtgcgaagtgttcagcacgacgaacccaagcggccccggtcataattgggtgaagaaacggtttattacgattgcgccgcgcggcactgtcgttcgtcgtagtatccagatttataacccgaagaccgaacaagaagaaacgcacgtaattacgcaaattgcgatcttcggttcatacaaggaaaacccgtatcttccggcgtcatatattgccgaactggaaagcattaaagaaccgaaccttcgcaaagcttggttgtatggcgattgggacgttaccgcaggcggcgcaatcgacgacctttggcaatcgcatatacacgttgtaccgcgctttgtcgtaccgccaagctggcgcatcgaccgcacatacgacgacggcagttcgcacccgtttagtgtgggctggtgggcggaagcggacggcaccgaagcgactatcgttctttccgatggaaccgaattcgtgttctgtccgcaaccgggttcgttgattcagatattcgaatggtacggatgcaagaaggacgaaaagggcgaattcttgccgaacgtcggtcttaaaatatcggcgtcggacgtagcgcaaggcattatcgaccgcgaagtttcgatgatggcgaacggctggatttcgtcgcagccttggcccggccctgcggataatcgcattcgacaagttatcgacgttgaactagacacgaccgaaaagcttatgtcgaagaagggcgttcgctggatggaatcggacaaatcgtcgggttcgcgtgttatcggcctacagcttttccgcgaccgactagaagcgtctgttaaacgcgaagggccgggggtatacttcatgtcgaattgcgttgcaagcattgatattttgcccacattgccccgcgacgaaaagaaaatcgacgacgtagacacaagcgcagaagatcacgtttacgacatggtgcgttatcgtgtattgaaaggcgcgaacaaagcggctacgaaagtcaaagtatcaatgccaacttaaaggaatcgaaatcatgccgaacgtatcttttgtgcgtcctgaactgtcgaagttgcttcccatgtactaccttattcgggacgcaatcgcaggcgaaccaacggttaaagaagcgcggacgaagtatcttccgatgccgaacgcttccgaccaatcgaaggaaaacaaggcgcgttatgatgcgtatatcgcgcgggccgtgttctacaacgtagcccgtcgaaccctgttcggtcttatcggacaggtgtttatgcgcgatccggtcgtaaaggttccggcgctgctgaacccgcttgtcgcaaacgcgaccggatcgggcattaaccttacgcagctttcgaagaaggccgtatcgttgaacttggcgtattcgcgcgccggaattttggtcgattacccgacgaccgaaggacagggcggcgcgtcggttgccgaactggaagcgggcaagattcgcccgacgctgtacgtctatgcgccgaccgaaattatcaattggcggacgattgatcgcggcgcggaagaagttttgtcgttggtcgttatctttgaaacgtggtgcgttcaagatgacggcttcgaaatgaagaacagcggtcaattccgcgttttgcgtttggacgacgaaggttattacgtccatgaaatttggcgcgaaccgaacccgaccaaggcggacggtacgaagattccgcgcggcaattaccaacttcacgaagttttcaaacctaccgacgcgaacgggaatcgtcttgacgaaatcccgtttatgtttatgggttccgaaaacaacgacgttaacccggataacccgaacttctacgatcttgcgtcgctgaacttggcgcattatcgcaacagcgcggattacgaagaatcgtgctacgtcgtaggccagccgacgcccgtacttatcggcctaacggaagaatgggttaacaacgttctgaaaggaacggtcaacttcggatcgcgcggcggcattccgcttccgaccggggccgacgcaaagctgttgcaggccgaaccgaacaccatgcttaaagaagcaatggacacaaaagaacgccaaatggtcgcacttggcgcaaagcttgtcgaacagaaagaagtacagcgcaccgcaaccgaagccgaattggaagcggcgtcggaaggttctacgctgtccagcgcaacgaagaacgttagcgccgcgttcgaatgggcgttgaaatgggcggcgcgctggatcggcgcgggcgacgctggcgttaagttcgaactgaatacagatttcgacattgcccgcatgacgccggacgaacgccgccagattatcgaagaatggcagaagggcgcgattacctttaccgaaatgcgtacagggcttcggaaggctggcattgccaccgaagacgacgcgaaggcgaaggccgacattgccaaggacaccgccgaagcgatggcccttgccatgccggacaacgtaccgggcgacggcaacacgcccccggctggtaatgtgggcaacgggggtgcgtaatcatggcgctatcggataacaagcgcctatacgacatttcaacgcggcttgccgtatatgtcgaaggcgtcaaagttcagcagtcccgccaattcaacttcgtattgcgcgatattagcgaagttctgaaaaagcttcttggtcgtgttcgttacaagacccttgacggtctttcgaaggcgcaactaaataagcttgtcgcagaactgcgcgaatcgcaatcgaagatttacagcgcgtacacgtcgcagcttatcgaacagcttaaagcgttcatggctgcggacttggaagtaaaccgccgcgcatgggttacggggtatatcgaacttgacggcgattcgccggacgaaattatttcggacgaagacgcaatacagttcttaatcgaagccaacgacagcggcgcaaatccgttgttcggcatcgcggccattactggcggcgacgaacgtatttggtcgcaagttacgaattcgccgcttccagcgaacggcctttatcttctgccgtttatcaagacgtttacaacttcggcgcaagcgtcaatcgaaagcattattcgcaaggcatgggcgaaccgctggactgttgacgaaaccttgcgcgaaatcatcggcgaagaaggcgcacgccaaggcacgccgtcgcagcttgcgcggatcaacaatcaagccgcgtcggttatccataccgccttcgcgcatactgcggcaatcgtagcggctggcgtagcgtctgcggttttcagttggtacgtttggttttcggttatggatggcaacacgaccgaaatttgccgaagccgcaatcgcaagcgttatcggtttggggccgggccgttgccgcctgcgcacattcgttgccggtcgcatactgccccggcgaatacggctagtgacctaatcgacgaaacgttttatacttggcttgcgcgtcaaccgctggaagtgcaagacgatatattgggcaccgaaggcggcgaagctttacgcgatggcaaattgaaagcttccgatattccgaagtacgaagccgacgaaccgctaacgcttgacgaattccgacgcaagattaaacagattctttcccgctgatacggtgtatcggcataacctgtaggagtcctacgaaatggcactgaaaaagcgtattaccaaagaagaacattcgaagcttgccgacgcgctgaaattcgaatacgtcgaagacggcgacggtttccgtctggacgttgacggcgacgaagacaccggcccgcttcgccgcgcgaaagaccgcgaagcgcagttgcgccgcgatgctgaaaagcgcgccaaagaagccgaagaccgtttggccgaactggaaggcgacgacgcccgcaaaaagggcgacattgctacgcttgaaaaatcgtggcaaaagaagcttgacgacgcgaacgccgcatcgcaagccaaaatcgacaagcttacgtcgcatacgacgaaaacccttgtcgataacgtcgcgctatcgatcgcaaccaaaatcagcaacgcgccgtcgatcatccttccccacattcgcgcgcgcctgcaagcgaatttcgacggcgacgaaccgacgaccgttgttcttggcaaggacggcaagccttccgcaatgaccatcgacgaactgtcggcggaatttgttgcaaacaaggatttttctgctatcatcacgggcagtaaggcgtccggcggtgccggtaagccttcgcaaaacggcggcggtgccccgaagatttccggtcaatccgacaaacccgccgacctttcgaagatgaatccgcaagaacttgcggcgcatctgaaagaagcgaaggctactactgaataaggacgctttatcatggcactttccgacctcgcggtttactccgaatacgcctattcttcgttctccgaagtcctgcggcagcaaatcgacctgttcaacgctgcaacgggcggcgcgatcatccttcaaggtgcggcgcaccaaggcgactttagcgacgtggcgtttttcgccaaggttgcgggcggccttgtccgtcgtcgtaacgcctacggttccggcgctgtcgccgaaaaggtgatgaaacaccttgtcgatacttcggtgaaggttgcggcaggtacgccgccgattcgccttgaccccggccaattccgttggattcagcagaacccggaagtcgcgggcgctgcgatgggccaacagcttgccgtcgatacgatggccgacatgctgaataccggccttggcgcgacttacgccgcgcttacgcaggttgcggcggtcaagtacgacgccaccggcaacaccgcgccggacgacggcccgacttggaacaacctcaacaacggccaagcgaagttcggcgaccagtcgtcgcagattgcggcatggatcatgcacagcacgcccatgcacaagctgtacggcaacaacctgaacaactccgaacgcctgttcacctacggcaccgtcaacgtgattcgtgatccgttcggcaagctgctggtgatgaccgacagtccgaacctgtttgcggcgggtacgccgaacgtctatcacattcttggccttgtgccgggtgcggtgatgatcggccagaacaacgacttcgacgcgatggaagaaggcaagaccggcgacgaaaacctgattcgggtttaccaagccgaatggtcgtacaacgtcggcgttcgcggcttcgcatgggacaagggcaacggcggcaagtcgccgaccgacgcggccctgttcacttcgacgaattgggatcgttacgccacgtccgaaaaggatttggcgggcgtgatcgtcgaagttcattaaccaacgaacaaacgggcggggcttcggccccgttcgtttaacgttcccaaacgaaggagttacgaagcatgaaacctgcaaagattctgtttttcgtcgatggcccggccccgacccccgaagatttcgccgcagccgccgaactgaacgcaagcgtttcgttccgcaacgcacgcgccgtaccgtccgaagcgcattcgctggaaatctgcgacggcgtggcgggcgcagttccgccgatctacgccgaaaagttccccgacgccgccgaagctatcaagaagaaggccgccgaactgaaagaacttacttcgaaggtcggcgacagcccggcaccgaaggccaagggcggcaagaccggccagcaagcgccgcagcagccgcagaccccggcccccgcaactggcggccagcagcccgcagcgggccagcaaggcggcggcgcgccgtcgtggaacccgaacccggcgcagtaaggccgggcgcagcgtagggcgcggcctgttcgcctagtgtgggcaggccgtttttataggcgcaacgaaaggacaaacgaacatgcaacgcattgtctattttaccgcaggcattaccccgacttcgggcgaactggcagatattgcaaagttgaacgcagccgccgaagccgcctacgaagtcaccgtagttaatggcgcagcgaatgcgaagtacggcgaaacgaaccgtcttattccgtgcgatttggtcgcgggcaccattccgaccatttacaacgcgaaagaagttatcgaccccgacgcaatcccggcgcgcggtttggccgctaccgaagcaatcgtacagaccggaacccccatcgctgtaactggcggaactgtaacgtttaccgtcgttgatagcgaaatcacgggcggcgttttcaccccgacaccgtaaggatttggcatcatggcaattactatcgtagtcgaagacggaagcggcgtagccaacgcgaacagttacgtaagcgtcgcggatgcgcgcgtatacgcggccaatcgcggcaccgaacttccgttggacgacaacgaagtagccgcgatgttgattcgtgcgacggactacctagaagcgcaggaatgccggtatcaaggcaaacgcacgtcgccgacgcaggcgcttgcgtggccgcgtaccggcgtattcctgaactgcgatgaagtcccgtcgaacgttattccgaaatcgcttatcgccgcacaaacgcaattggcgatggcgattaacgcaggcttcgacctgcaaccgaacatttcgccgcaggattacgtaacgcgcgaaaaagtcggcccaatcgaaacggaatacgccgacccggtagccgttggcattatgcccacgtttaccgcagcgaacgcgcttcttgcgccgctgtttggcgaatgcgcttcgaacaagtttgcacttcggacaattcgggtttgacgtatggcacgctttgaccgcgcgattcaaacggcgttgcgattgatcgcaaagaacggcgaaaaggtgaaatggcgcgttattgacgacgcagccgcgcccgatccgtcgcagccgtggaaccccggcccggcaacgcccgaagacaaggacgtaactatttgcttcttgccggttgatcggcaaacgatggaaacatttacgtttatcaaaggcaccgaagttccgaaaggttcagtaatggggcttatgggaaacgtgccgtttaatccgaacttgaaagacgtagttattcgggatggcgtagaacttcgaatcgcaaatatcgacgttctttcgccgaatgggcaaaaggtactttacacggtagtttttcaagcatgattgaatttgaccaagcccgcgacgaaatcaatacgctgtttcttacggcgtggaacgctaacgcgggcgcggtcgtcggctatgttcccgaaattcgttggcagggcgtacagtaccgcgatttgccggacggttcgaagttttgggttcgcgtgtcgaaacaaaccgttttcgaagaacaaacaacgctttcaacttgcgaaggaaaaccgggacaaaaacgttatacggcgtcggggcttgttttcgtgcaagtgttttgcccgaaatcgaatacgcaagctttcgcacttggtcaaacgctggcgaagattgcccgcaatgcttttcgcggaaagactacgccggggaagatttggtttcgaaatgttcgcataaacgaacttgaccccgaagaactgtacgaacggtttaacgtcgttaccgaatttgaatacgacgaattaggttgaaggagttacgaaaatggccgattgcgctatcaacaaaatcgactcgaacattaccggactggcgtatgccgaagaagaatgcttgaagcaacttccggcgtccgtcacttggtacggactggaaccgaacagctattcggacttcggcggcgaactgtccaccgtagcccgtgcgcctatcgacccgtcgcgccagaacaagaagggcacgattaccgatcttgacgcatcgggcggcttcaattcggactttacgaagtcgaaccttacccgcatcctgcaagggttcttcttcgcagacgcgcgcgaactgccgtctactgcgccgatgaacgccgccgctatcgcaatttcggctgtcgatgctgcgacgaagacctataccgttgcaagcggcggcgcggcgttcgctgcgaatatgcttgtcaacgcaaccggcttcgccaacgctgcgaacaacggccttaaaaccgtagcttcgtccaccgcaacgaccgtcgttgttaacgaaacccttatcgacgaagccgcgccgcccgctggcgtgaaactggaagtcgtcgggcgtcaactggccgcagccgatgcgaacatcgccgttacttccggcgtcgcttcgttggtcgtcaccgctggcgactttacgaccatgcccgaactgttccccggtcgttgggtgttcatcggcggcgacgcggcgtcgaaccgctttgcaaataatgtgggctacgctcgcattaagtcggtttcggcgaaggcgcttgttttcgacgatacgaccttcgcggctgcgaccgaaaccggaaccggcaagtcgattcgtctgttcgtcggcgtcgttatcaagaacgaaaaagacccggcccttatcaagcgtcgttcgtacaacatcgaacgcacgttgggcaacggcgaaaacggcgttcaatgcgaatacttggaaggcgcggtagccaacgaatttacgttgaacattccgcaggccgacaagctgaacgccgatcttacgttcatcgcgtgcgacaacacgcaccgcagcggcgaccccggcgacgaacaaaaggccggtacgcgcatttcggcaccgggcgaagatgcgtacaacacttcgtcggatatttaccgtatcaagatggcggttcacgacgacgcttcgtcgaatcccgccgccctgttcggttacgtgtccgaagcgaacgtttcgattaacaacaacgtttcgccgaacaaggccgtcggtatcttgggcgcgttcgacacgacggcgggtaacttcgaagtcggcggttcgattaccgcttactttacgaccgtcgcagcggtaaaggcggttcgtgcgaatgccgacgttggtttgtcggttatcagcgcggcgaagaacgccggtttcatcttcgatattccgttgcttggtttgggcggcggtcggttgaacgtcgaaaaggacgcgccgattaccgttccgcttgaacccgcaggcgcggaaaacgaaaacggttatacgatgctgtacgaagtgttttcgtacctgccaacggtagccatgcccgattaagtcgggtacacttgaagggccggacttttccggcccttctttcatccatcggagtaaatcaaatgtctggactgtttaagcaattcaaaacgaattcggcgaaggaaaccgaaggcgtcgaaatcgaatttcccgaagcgcagaacgacgacggcaccgttcccacgttcatcatttcgcgcatgggcaagtcgaacaaagcgtattccaagtcgctggaagccgcgacccgcccgtatcgccgacaggtcgaattgggcaccatgaaaaacgaagtcgccgaacagcttttcatgggcgttttcgtcgataccatcctgcgcggctggaagaacgttcaggacgaaaagggcgaagccatcgcctattcgaaggacgcggcaatttcgcttctgtccgaactgcccgacgtttacgaacgtctgcaagaagaagccaagttgtcggccaacttccgcgattcggtgttggaaaccgaatcgggaaactgatagaagttctagcgtatctgttcgaactaggcccgcacgaacagaccatagcaaaacaggcgatgcgggcgggccagccgttacccgaccgcatcgccaacgcgccagaacttgaaccgggcttgcagttgtatttgcaagccttcttcgatttggatagcgaacgaacgcacgcaatgggattgacgccgattccttggacaagtattgcggcgtatgcgtcggcattcgaattcgacgaagaacagcgggaagacttgttttattttgttcgtaaactggattcggaacatttgaagaaactggaagcaaagcataaggcgaataaaggcaatggcaaacgaccttctaagtctggccgttagtctggaacgcaaggctaaggcaatcgacgaagcggcttctaaaacagccgtcgatactgcaatggctattgtgggcgacttggcgtataagacgcccgtagatacttcgcaagctttgtcgaactggcgcgttacgcttgattcgccagcaaccgggacgattgcaccgcattaccccggcattcaaggttcgtcgcaacgggcaagcgcagccgaaacgatcaacgcggcaaaaagcgtacttgcaaacaagaagcccggtcaagcgatttttattacgaacaaccttccgtatatcaaacggcttaacgacggatattcagcgcaagcgcctgcgggattcgtcgaacgtgcggtattgattggccgcaagatgcttgcgaagttcaagattaaggattaagacgaaatggccgaaaacatcgaaattaaagtacaagataaagtcgattcgtccatttcgaccaagcttaaaggcatcgcttcggatgcccgcaccgccgacagcgccgtaaaggcgttgcaatcgtcgttgaagtcgatttcggcttcgtccggtctttcgcgccttcaaagcgaacttgcacgtaccgccattctacagcagaagcttgccaccgaaacgcagaaaacgcaagtcgcaatggcgaacgttgaagcggcgttgcaacgtgccatcgcagccgaagccaaggcgaacgccgcgattaaccaactttccgccgcgcaatcgaaggccgccaccgaagcgcaacgtttggcaacagcgcagcagcagaccgccgccgcagcagcgcaggcgcaagccgcacaagcgaacttgaccgcagcgcagaccaacagcgcgaccgcatcgcagcggcttgccacggcgcagcaacagacgaccgcagcaacggccaacgccgccgcagcgcagacgcgcgcggctacggcgcaggtacagggccagaccgccgcgcagaaccttgcagcggccaccacgcgcgccagcacggcccaaacgcagggggcgaacgctgcgcagcggcttgccaccgaacagcagcgtacagccgtccagacggccaacgcggcagcggccaacgaccgggcggcccttgcagccctgcggctggcccaagcgcagcagcgggccgggcaggcgtcgcagaccgcaggccagcaaatcgccggatacgtcaaagccgccgcaggcatcgcaggcgtaacgctgtcggctggcgctattctcgcatcggcggacgcatatacgacgctgcaaaacaagttgcagaacgtcaccgaatcgcaatcgcaagtcgtaacgcttacgaaagaattgttcgacttggcgaaccgcacgcgcgcgggcgtcgaagaaaccgcgacggcgtttacgcgctttgatcgtgcgttgaagttcatgggcaaatcgcaagaagattcgttgcgtttgaccgaaaccattaacaaagcccttatcgtttccggcgcaactgcgcaagaagcgtcgtcggctttgttgcagctttcgcagggcttcaacgccggtaagctgcaaggcgacgaattccgcgccgtatccgaaaatatgccgatggttcttgacgcagtagcgaaggcgcttaacgtgcctatcaaccgcgttaagcaactttcgaccgaaggcaaaatcacgtccgaagttctgtttaacgcattccagcttatacagaagtcggtcgatgacacgttcgcaaaaacgacgcccacaatcggccaaagccttaccgtcttgaagaatagcgcaatcgaattcttcggcgaattgaacaaggcgaccggcgttacggctgcgctgtcgaaggcgattctttggcttgccgacaacatgaagaccgttgccgtcgtagttacggcgcttggaacggcgatgcttcttgcattcgggccgcagattgtcgcggctatcgtttccgcaacgactgccgtaaaggcgttcaccgtcgcgcttgcgtcgaacccgattggccttatcgccgtcgcactggcaaccgtcattgcgtaccttacgctgttccgcgacgaaattaacttgggaatcgacgacgttacgacgttgggcgatttcttccgcgcgacctttgaaggcatcgggcaggttattagcgacgtgaccttgattgtcggccaattgtgggcagacatgaccgaaggcgcgtccggggcgcttggcgaaatttcgtcgttcgttggcgatgctgtttccggctggacggaagactatacgtcgttcttccagaccgaacgcaccggatgggccgccgcgctggaaaacaccgcgaaagttcttgacgcaatcgccggattcattaccggccttgcaacgttcgccggtcgtgctatggccgaagtcgtgattaccgttcaaaacggaatcgcaaacggctataactatatcgtcggatggattgaacgggttacgaatctggcgattgaatcggcgaacaaacttcgcgcgatggtcggcaagtcggcatacgaacttgtcaacttcgaacgcatgggccaagccggacaaactgaattcgaatcttggggcaagctttgggccgaatcgctggaagacggctttaagtcccaaggcggcgcaatgcaaaaggtcgtcgaaggtcttatgacgcgcgcgcagcaaatcggcgcgaatcgtcgcgcaagcgaaaacgcttcgcttcgcggcgcaggtgcgaaccaacttagcgcagctaccgacgacaaggcggcgaaggccgcagaacgtcgcggcttggctttggaaaagatcaatacgcaacttgataacgaattgaaccgtatgtttacgcttcaaccgcaacgcgaagcgcaagcgaaaatggatcaaatcgaagaatcgttgattcaacgtaaaatcaagcttaccgaagacgaacgcgcttcgatcatggcgaagattcaggccgtccagcaagcgcaaatcgtgcaacagaagttcgacgcgatttataacgaagctgtcggcccgcaacgcgattacaccgccacgcttgaagcttcgaaaaagcttcttgaccttggcgcgatttcgcaagaacagtattcgcgcgcagtaacgaaggcgaccgaagaattcaagaacgcgcaagacccgatgcgcgcgtataaccgcgaccttgaccaacagttgcagcttttgcagttgttgccgaagcaacgcgaaatcgaacagcaggttatgcaagtgcaaaacgacctgttgacgaagggcattacgcttaatgccgaagaacttacgcaactgcgcgaacggcttacgctgttgcagcaggcgaacgcgcttgcgcagcaagaagccgcgttaatggacgcaagcgttacgaagcgtcaacagtatatcgaccaattgaaggcgattaacgcgcttaaaaacaatccgcaaagcggcttcacgcaaggcgacgcagctaacgccgtaatgaacgcgaatagcgatcttgacttcacgaataccgatacgtatttcgaaggtcaagcgcagaaatacgaagatatgtattcgcgtatcgaccaattgcggcaacaggatttgattagcgaacaaaccgccgcgacgctgcgccaacgtatttggctggatcaacagaaccaaacgcttaacgccgcgtcgggtttcttcggacaaatggcgcaattgcagaagtccgaaaatagcaagatggccgccgttggcaaggccgcagctatcgcgcaagccatgattaacacgtatcaggctgcgaccggcgcgtattcgtcgcttgcgtcgattccttacgtcggcccggcgttgggtgcggctgcggctgcggctgcgattgccgcaggcttggcgaacgtccaacaaatccggtcgcaaaataccgggttcatgtcgggcggttacactggcgacattccgacgaatgccgtagcgggtgccgtgcatggtcaagaattcgtaatgaacgcagcttcgacgaaccgcattggcgttgataacctgcaagccctgcaaagcggcgcggccagcgtccagcgcaacggggataatgtgggcaccggccaagcggccccggctgctgcgcccgaagtaaatgtaactacgccggtaactgccgtcgtggtacaatcgaaagaagccgccttggctgcgatgaagtctagcgaaggcaaggcatttgttatcgaaactatcgaagaaaacggcggcaccgtcgcccgaatcgtaggggttaaataatgggatacgcaatcggaacccttgcaaaaggtggcggcgacgactgccattatcaattgcttggcgtattgaagacgcttgccgaagcgaacggatggacgacgcttcggtatgtcaacactggcaccgaccgcgaattgattttgaagggcgtaggtctgtccggcaccgaagaaattttcatcggatggaagacctatcaaagcgtcggcgcggattactacaatctgaattgcgcaacgtttgtcggatacgtcgccggaaataccttcgaaacgcaaccgggcggcaagtacagcggttgccctgcccacaataacgcaattacgtatttcatcacggcaaatgcgcaacgcatcgcgttttgcctgaaagtcggtacgccggtttatacgcattgctacgtcggcaagctgtttccgtatgcacgtccgggcgaatatccgtcgccgttggtcgttgcttcgatgttcaacgggccagccgcaacgcgcttcgacaatacggcgtattattttccgtatccgggtgaaggctattcgacttcgtgttttatgtggctgcgcgacgctgcgggcaactggaataagtgttattcgtatcctttcacgaatgcgaacagtagcacgaacgcacttgccgggccgcaaggatcgaatacgcttgttccgtccgacgtgtattaccagcttgaaccgattattcttcaacagttggacacgtccgttaacccttcgaatgtatggggtgaactggacggcgttactttctgttccgggttcaacaacggccccgaaaacgtcgttcaaatgggcggaagttcaaccgtagatcaaaccggaatgaccgtacttcaagcggttgacgcaatccgggcagtcggcgggcgcgcgttcgtagtttgccagaacgtgcgctttacttcttggcgcgattatatcactttggaaatgtcgtaatggcctacgttaacggaagtgccgcaagttttgcggatttgaaaacagcaatcgaaaacgcagcggtcgccgcaggctggacgctttctagcggtgttctgtccaagaacggcgcgtttatcaagcttacgaacaatacagcaagcccgccgcgcttggaagttcaaggcggcacggcgcaaagcggttcgacgctaacgaacccttccggttcaccgtcgattgttaacccgacttcgaacggcactatatcttttccggtcacgtatgaaattcatacttttacgaacccggacgaagtttattgcttcattaactacaattcggattattaccagcatctttgtttcggcaaatcggatatgccgggcgtaggtcttggcgcatggctaacggcaagttggccggtttcgccgactactggcggcggtttgaatttgtcggtaagcaaaactagcgttagtgcgtttccgtttgtaaattcgcaaaacgtcggccttttttgcgacggtagttggggaagtacggaaaattgcacctacattcgaacttcgcttgattccgaagcttggcgttcgcctgccaatgcaggccaaatgacaaacgcttgcagcgtaacggcttcgctgttgaccgcacttccgaacttgtcgaatcaagcaaccgttttgcttccgataaaaggcgtgcaaaagcgcacttctggcggactcactaccgttgtcgatttgcaaaatgcacgtatttgtcgtattgacaacttgacgcccggcgatcttgtcacatacggcccggatcaatggaaagtttatccgtggtatcggaaagacattaacaatcgcaacggcgcgaatacttcagtgtcaaccccgcgcccgacgcatagcggaacgtttggcttcgcaatcaaatacaccgggacgtaattagatggctggacgactcgccgcaccggaaatgcaacggcctgtatatggcgaagtcaacgctaatatatcggtcgaattgaacgaactaaccccggcggactacgatccgaccgggtatccgacgcgccttttcaaactttggggcgtgtatcaatcctatcgaatggcggcccgcacgggatggcctattgtgggcgcgcgccaacatagcttcttcgaagattattactttcgcattcacgtaacaccgcaagaaatcgaccttcaaacggtcgcaagtacgcaggtgcgcgaagttgaagtatggaacgcatatccgtacagttccgcaatccttcaagacattttggttagtaatcctgtcggcattaacgtaaatgggccgaacccttatacttttccgccgcttgtcgaacagacttacgaaattgaagtaggtacttccggcccggcgaatattgaccttcaaattcaattcgatttttctaacgtaacaaatccgcttccggtacttgtgaccggcacgcgcgctgttaagttcgacattatccccgaaacgccagtaacggaagaatggcaatggcttaccgataatatcgtagccgttgacggcaccgaacagcgtatcgcgctgcgcggtgaaatgccgcgtgttgaagaaaatttgaaagttattttcgacgattcgacgaagattcggaagttttatagcgatcttatggccgcagtcggtcggctttggattcccgaatttcagtatgcaacgcgcacgctttcggccagcgtaacgggcggctttaacctttacttcgacacgtcgaagactgacattcgcgcaggcgaatacgtcttgattcaaacgccgttgaccgctgcgcttgtcgaaattgacgtattgaccgtaacgggcgctaccgtaacttcagctttgacgtttgatattccgaagggttcgcttatcatgccgggttcgcccgcgctgttgaatgacggttcggggctgtcgcgctatgctgttaacgaagttgccgaaacgacgttggtttgcaagatgcttcgccagcgtgcgcagcttgtgcgccccggatcaaccgtcacgcttccgacatatcttggcgttccggtcttcgaaaagcgaccgcttgccgatgaaatggtagacgacaacgtatctaccggccaacagtcaatcgacaatcaaaccggattgccggacattatttcgcgttgggattatagccgtattggcggcgcacgttcgtataaagtgaaccgcattcaacgtcccgaagaaatggactattggaaaacgctattcgcgtatatgcgcggtgcggcgcgtaaagtttgggtgcccacataccgaaccgacatgcgcgttaccgtccagcctgccgaagaaacttcgacgttcacgattgaaggcaccgaatacgccgaaaagctgtttccgattgtcacgcatcgttatatcgaagttgaaacggcttccggtattcatcgtgccaacgtaattggtgcaagcgtaagcggcgtcggttcgattatcctgtttaaccccggccttccggctggcgcaggctggacggacattaagcgaatttcgttcctgttgcctatgcgaatggcagaagacaaggtaacatggaagcattacggattagaaagtttacttcaactttcgttgattacggcggaaccttaaatgtccgattacgacgacaaagaaataagccagcaagacggcgcgccatacgaactttacgaatgggtcggaacttaccgtagttattacatgactacggacagcataccgcacgttttcaacagtgcgacgtacaatcctgtttcgggtttgaagcgcagtacgttaaaagccggtacgcacgaagaagacaatatcgaccttacgattatagttcccattaccgaacaaatcgtaaaagactacggttttcaaactacgccgcccgcgctg

SEQ ID NO: 6 - DNA, 41878 bp, unidentified
  source 1..41878: mol_type = genomic DNA
tagaaccgtcttcaactgtaattgttatcgccatttttaaaccttcgttcgttacggttgccgcctgcccacactaggcgggcaggctgcgacttattgcggcgcgttgggcgtccatgccggggcgctggcgggctttgcaggctgcgccggggcttgggccttggctgcggttgcgggcgcgttggcgggcttggccggggctttcggggccgggctgtcgcctaccttcttcgccagcttcgccagcttggcggcgtgcgccttaatcgcttcgtcggcttccgggtaggcttccgcgtaggtcggcggaaccttgcccgttacgccgtcgcattcttccaacgcaccttcgggcggaacagcgcgggcattgcggaacacgacttgcgcttgcatcttcgaagcggcttcgaagtcttccggggtcggcgaaacgccatccacgaaataaagaatctttgcgggtttcatagttgaaattccttcgaattaagtttgcatggaagaaaggggccgaagccccttccgtcgttcgccttacttggttttgacaacaaccccggcaaggtctttatgcgaagttgcgtacttgtcccaattggtcgaagtcagcaacgcggcatcgttcggcgacttgccgccgttagccttgtcccaagcgaagcccttaacgccgacgttatacgaccattcggcttgataggtgcgaatgatgttttcgccgccgttcttcgcttcttcgttggccgtaaagtcgttgttttggtcgataatcacgccgcccggcacaaggccaagcgaagcgtagtaatcgacgccaacgccgcccgcttcgtcaaggaacagcgcgggcgaatcggtcataatcaacagcttgccgaacgggtcgcgaataacattcacggttccgtaagtgaaaagcgacgcgctgttggtaaggttcttcccgtaaaggtcgaacatcgctttcgagtgcataacccaagccgaaatcatagaagcttggtcgccgaacttcgcttgacccttgttcaagttcaggaacgacatggtatcttcgggcgcagtcaagcccgtagcgtcatgcacgacggcggattgcgcggaaagcgcggcgtaggtcgcaccaaggccggtattcagcatatcggccatcgtatcgacggcgagttgttgcccaagggccgcgcctgcgacttccgggttttgctgaatccatttgaattggccggggtcaaggcgaacgggcggcgtaccggctgcaaccttaaccatcgtatcgacaagatgcgccatgttcttttcggcgacgttgccggaaccgtaagcgttacggcgacgaacaagccccgaaattttggcgaaaaaggcaacgtcggaataatcgccttgatgcgcagccgcgcgaagttgaatcgccccgcccgttgcggcgttgaacaggtcgattttttggcgcaaaacttcggtcatcgaagaatatgcgtattcggaataaacggcaaggtcagaaagtgccatgataaagcttccttaatcggttgccttcgaagctttgatgtgttccgcaagttgtgcgggattcatcgaagcaaggtcggcgggtttgtcggattggttcggggcaccgccgccgttttgattcgaagaccgaccggcaccgccggaagcctttgatgcggtaattatagcggaaaaatctttgtttgcaacaaattccgccgacagttcttcgatggtcattgcagaaaccttgccgtctttgtccaaaatgcgcgtaaccggggcgtcgccttcgaaatcggcttgcaaacgcgccttgatgtggggaagaagcaacgccggggcgttggaaatcttcgaagcaatttgcgttgcaacgttatcgacaagctgtttttgcgtatgcgaagtaagcttgcccaacttgccttcgtattcggctttggtatcgtcaagcttcttttgccaagacttttcaagcgttgcaatgtcgcctttcttgcgggcgtcgtcgccgttgattcggtctagttcttcctgcgcttcgcgcaacttcgcttcggcatcgcggcgcaactgcgcttcgcggtcttttgcgcgcttcaaagcgcccgtatcttcgtcgccgtcaatatccagccggaagccgtcgccgtcttcgatgtattcggctttgatgtgttcggaaagcttttcgtattcagctttggtaagtttctttttaagtgccattgctaggactccttagcggttatgccgattcaccgaatcagcgggaaagaacttcgttaatcttacggcggaattcgtcaagggttaggggttgcttactttcaaacttcggcaaatccttttctttcaaatttccgtttcgcaattcgtcggctacgtcttcgcccaaaatgtcgttttgaacgtctgcgggctggcgaatggcccaagtataaaacgattcggcggctatgtcatctatgcccacaataggcgcgatatgcgaccggcaccgaatatgcgcgggcgggattgggccttgtccgaaacgataccgtttgcgatttcggcttatgcaaatttcggtcgtctttccgtccattacggaataccaaccgtaaaagccgaaaagcgccgacattaccgccgcgcctgtaatgcctgcgacgtgttgaactgcggttgcgacaacggcgcttgcttgaacgccgacgcgctgcaattgcgacgaagtaccttgcttattatcttcgccggttatttcttgcaatgtttcttcaaccgtccaaccattcgcccaagctttgcgaatcgtgttttcgacgcttgcttgtgctgatactgcgaaggtctttacgaacggcacaagataaagaccattcgccggaataggcgcgttcgttactgccgaccaaagccggtcgttattgccagtaattgcggccaatccgaacagcggaataaagttcgcttggttgttttcttctttaagaaacttgattgcccttgcatccgacggaatttgcggcttgccgtaacgttcttcgtcgaattcgaattttgcatagacgtaagcgcgacggttcatttccaaatcggcgcgcatgaagtcttttagctgtttcaaaatctgttgcgtgtatgcgctataaatcctagattgtgattcacgcaacgaaacgacaagcttgttcaattcggcttttgtcaaaccgtcaagggttttatacttgacgcgcgcaagggttcggctaatttccaagcgaagttcggccaagacaaagttaaattcgcgggcgtattgaactttaacgccttcgatataaacttggcttcgcgtcgctatgtcataaagccgcacattgtccgatagcgccatgattacgccccttggttattgtcgggcggcgtgttgccgtcgcccggtacgttggcaggggttgcaagcgccattgcggcggctgtttctgcggcaatcttcgtttttgccttttcgtcttcttcggttgccgtgccagacttgcgaagaaccgcgcgcatttcttcgaaggtaattgcgccgccttgccattctttaatcgcttgggcgcgttcttccggcgtcatacgggcaatgtcgaaatccgtattcagttcgaaagtaattgcggtatcaggaacgccgacaaactttgcgcaccatttcaacgcccaaacgtaagcggcttgaacgttcttcgcggtactggaaagcgtcgaaccttccgacgttgcttctaccttggcttcgaaggcggttcgttgaacttgcttttgttcgacaagctttgcgccaagtgctaccatttgccgttctttggcttccatcgcttctttaatcatcgtattttcgccagcctgcaacaacttagcgtcgccgccgacaggaagcggaatgccgccgcgcgaaccaaacgcgacggttcctttcaatacgtcttttacccattcttccgtaaggccggtaagaactggcgtcggttgtccgacgataaaacaagattcttcgtaatccgccgaattacgataatgcgcgacgttgatacttgccaaatcgtaaagattcgggttatcgggctgcgggtcgttgttttccgaacctacgaacgaaaacgggatttcgcgcaacggcaggccgtcggcacctttcgggcgaagttgcttcgtaagctggaaattgcctttcggcgtcttgcttccatcccatgccgacggctgcggttccgaccaaacttccattacatattcgccgttttcgtcaagcttcaagacgcggaattgcgccgcattcttcatttcaaagccatcatcggcgaacgtgtaagattcggccaatacgacaagcgacaagatttcttcggccccgcgttcggtcaaacgccaattgacgatttcttgcggcgaatacgtcgtaatggtcgggcgaacgcggcccgcttcaaggtcggcaatcgttgcgccgccttctggaacttcgggataatcgaccaacagcccggcgcgcgaatacgccagcgttagcgaaagcgtctttttcgattgttgcgtaagacttacgccggttccacttgcgttttcgacaaccgggttcaacagcgaaggaactttaacaaccgggtcgcgcatgaacacttgaccgacaaggccgttcaaagtgcgacgggttacgttatagaaaacggcgcgcttcaaataagaatcgtaacgcgctttattttccttcgattggtcttcggcgttcggcatcggcaaataaaccgttcgcgcgcctttaatcgtcggttcgcccgaaaggcaatcgcgaataaggtaatattgcggaagaagcttcgacaattcggggcgaataaacgcaacgttcggcattttgattttcctttaacttggcatgattactttaaacttcgacgcgctgcgcttcgaacccttcaagacgcgataacgaaccatatcataacaatggtcttccgccgtcgtatcaacatcgtcgattttctctttgtcgcgcggtaatgtgggcaaaagttctatcgaagcaacgcaatttgccataaagtatatacccggcccttcgtttttaacagcggcttctaacctatcgcgcaacaactgcaaaccgtttcgccgcgaaccgggcgatttgtcggattcaatccagcgaatgcccttcttcgacattttaagttcgattgtttcaacgtcggattcccgaacatcgcgaatctgattatcggcagggccgggccaaggctgcgacgaaatccagccgtttgccatcatcgaaacttcgcggtcgataataccttgcgcaacgtctggcgcggaaagcttcaaacctttattcgtaccgatttcggttgcgccgtaccattcgaagatttgaataagcgaaccggcaggcgggcaaaacgaataaacttcgtcgccgattactatttgcgcttcttcgccgttggcttcggcaaaccaacccacactaaacggatgcgaactgccccaatccaaagccctatcaatgcgccagctttgcggaacaacgaagcgcggtacgacgtgaatatgcgattgccaaaggtcatcaagcgcaccgcctgcggtaacatcccaatcgccataaagccaagccttacgcaaattcgggtctttgatgctttccagttcggcaacgtatccgggcggaagatacttgttttcgcgatacgaaccgaagatagcgacttgggttcgaacgacggtttcgttttgttccgtttgcgggttatagatttcgacggaagtacgaacgacagtaccgcgcggggctacgttgataaaacgacgtttaacccaattatggccggggccgttcgggttcgtcgtactgaaaacttctagcggaatcggcggaagcggaagaccattcggcgttaaatattcgcctttgtcgttcttcggcgtgtttaatatcgggtcgaatgaacttcgattaaccgacataaacttatcgtaaagttccgacgaagcatgtttggttaattcgttccagcctagaaacgggtattcgtggccgtggaagccttcgtaatccgaaacctttttgacgtggcgaaacaacagttcttcgccagtaggccaaacccatttataagccgaagtcgattcgtagaacttcgcaccgtcgccaaacttgccgaaccattttttcgattcagcaacaagcccgcccaaatggtcaaattccaaatcgaagataacgccgcgccagaattggccgtagcctttcccgacgtggcgaaggaatcgcataagttgggtaacggtcttgccggggccgcgtgcgccttcgtacaacgtatggtcgcaacgcgaatcaatggcgattgattgcgaaccgggcaggggtcgccaaacgatttcaggtttcggggcgttcgccaatgccgccgacattcgcgccgacttaatggcgctttcggcgatttcgcccgcgcttttaatgtcggcttcggctaacattcagcaattcccgttgttgtgcggcggctgcggcttcccattcttcgttcgttccatgcgtcggaacttcgattgcgcgcgggattacgacttgcacggcggggccgctttgcggcttcttcgacaagccttttaaatccattagcttatcaagcgccttaattcggtcgtctggaaaacgtgcgttttcgatgatttcttttagtttttcttctacataacgttcgtcttccgatacgccagattcggcgatttcggctttcttcaattcggcaatcatcgccttaacttcggcgtcgttgtgccacattgaagcgatttgcgcggcccggttaaagttggcaggatgcaccaattgcccggcttctagcgggttcatattcgccgaaatcatcgcttgcgcgaatgcggctttttcttcggattcggtcatagcgggaagccttcaaatgtctttgcccaactataccgcaaacggccttgcctgtcagcctgttattgcttttcgcaattcttcgaccatgtttcgttatgtgccagaatttgccgcgcggttccgtcggttaatacgtctttcttcgaaatcaaaataggttgaacccatttgcaagcggtatcaattacgaccgtttttgtttcggttgcttctttaatcccgcgcccatttgtcgcgcaacttgttagcagcgtcgccagcgtcaagacgattaatattcgtttgaacatcatttgccccttttacggtttcgacttcggtttttgcggcgtcgcgtgcggcgtcgatttcgcgaactgcgatttcttcgttacgcttggtttccgcttgggcggcttctaccttggcttcggccttgcccacactacgcgaagaccgcatggcgacgaacagcgccccggcaagcgacaaagcggccagaatccagccgccaaagcgtttcaagcctgcaagaataattgcggtcataatgcgcccctatgcttcgttcgttgataccttgccgttcgatgccagcaacggcaacgaatagcgttcggcgttcggcgtactctttacggcggctttattctgccacatagacggccaaaaatagccagtaacgcgcgacgttgcgaagggcgcaatacttacggcgttcgattgattgccgcccaaaacaaggatattcccgcgcgcatctttgccgactacgaagccaacatgcccgccgccttcgcgtgtaaaagttacgatgcaaccgtaagccggttcgttaagcttcgtcatttccgacgattcccaagaccgcgcccggaaccattctttaactacgaagcgcccggcagttccaaggcaaaagccgacgaacagaccgcaccaaggcgtttcgtcgtcgtgccaccatgcgcgggattcgttcgaaaaactgcccattttatccagcatcgcaagcaacgtcggattatgggcagtcttcgaagtattttctttaaggccgatatatttacgggcttcggcaagccaaggaagttcattcatctttcggcccttctttctgttcaagcttcgtttgtttgattgcgcgggcaaccaacgaagcaacgaagataacgacgccaataagcggcatatagcgttcgggaattgccgccttcaagtcgccgggcatcatggcccaagccgacaaggcaacgtctggaaacgcgataagaacgccggtaatcgccgaaccgataatgccaagacgaaccgaccaaaagcgccagaaattgcgccaatcttcgataagttcaagtttaattttgttcatttgtcgattccttcgcgccaatgattcgacgatagacagtttcgaaacccgcaattgcgcgcgttcccatgtgccccgaaattgcgataagaaccgccgacattgtttcgctaatgcctgcggaacgacagaaataaaacgtaatcaatccggcgaacgttgaaacaacaaggtcaaaaatcaattctttaagttggaatttctttcgaccgcttcgaagcgtcgtaatatgattcacaaccccgccccaagttgaaagaaaaaacgtcgtaaggtacggcataaactggcgcaaccattcgacaaataacgccgtattgttcgggtctttttcgggcatgtttgaacgttccataattgattatcgcatttaaggcgaatgatacccgcatttaacacaatttggaacaaacaggcaataaaaagcccggcgcaatggccgggcctgttgtcgaatagccccgcgaagggctaccgggcgacgtttaggcggtacgccaaacacgcgcgcccttcacgccgttttcttcgacgctgcgaacgacgaacttacgggtttcgaccatgacgggcacgacttcgcctttcttgttggtcttggtcgcgccgtcttcgctggcaacggcgtaacgggcggttgcgctggaaacggtcgaagcaagcgacttcgcggcgttcggcttgtcttcgctgttggcaacgaagaaggattggccgacttccagttggtcgaacggatacacgttgccgccgcgaccgcgaccggaaatcgtaggaacgggaatgctatcttcaatcttaaacatggttttcaccttttcagttttgccggtttcggcggttgcggaagttgcttcggaagttgcattgttgccgatggtttcgccgttgtcaaggctttcgataccggcttgcgttgcgcgggtcgcgacgttgccgttatcatcggtcatggccggattgatttcgaccaagccagcttcgacaagcggggcatagacggattcgggaacaaacatgccattcgcgccagcggcgacgatttcagcaaggccgataacaacaacggcagttgcagcggttgcggcggtcttcttgcctgcggatttcttggtagccattttcaaaactccttcgaagggttaagttactgcggttaatgtcgcgattggtgcgacggttttaattctacgccattgcttccggttgtcaagcggtcaaagcgaagaattcgtaaattttttcggcttgccgtattcagcttcgcaaaccttcgcataagtgccttcgtagtccggccattggcccgactttacgttttcacaatatgaaatttcttcctgtttcgcgtcttcatagtcgaaatgtccgacaatcccgaacagcgcaacaactgcgacggcaataagaacggttttcgctttcatgtgggcaagcctttttcgttgaacatgcgatgatgttacggcaacttcggttgcttgtcaagcattacggcgacattttcgacgccttcgcgtgcgacctgttgcgttagaagaattgcgttttgcagttcgataaagtttcggattatcggattgttcggccctgttacggtttccgaaaggtcgataaggtcttgaagcgcgttgtattgtgccgttagttgctgatacattgcaccgcttgcgcgaagtacattgtaccattcaggcgctacgcttccttcggcaaaaacgatttttgccggttcggcttcttcggtattgaccgacaaaacgtttccttcgtcgtcgcgaataagccaatatttcgccaaatcttgatgattcatactaagccccttcaaacataaacaggcattcgatacccgcgttaataaatacctgttcggcggcttcggcggaagcgcgccaatctggcgatatgtgcccacaataggcaacgacgcggcttatcccggcccgcgctatcttttcggcgcatttgtcgcacggaaacaacggcgaaacgtacagggtataacctgcgaccgattcggcgtcgtgcgtttggcgcaatgcgttgtcttcggcatggattacgacggaatgttgttcgtcgcgcgtcatgcgcaaaaaggcttcgtcgtcaaagccgcgcggcgggccgttatagccaagcgacgcaatcgacttatccgggcgcacgataaccgcgccgatacgctttcgcgggcctttcgaccatgcggcgacgtgttcggccaattctaaaaagcgcgtatcccatttcgacaggctggcgcggtcagtataaattatcatacgacaagcctttttctttgcgcatacgaataaccgttgcgcgttcgacaagttcgcgcatcttcttagcctgccgaacttcgttatatttcagtcttgcggcgttgcaaagcgccgcgattgcgataagccaacagattgtcgaaagcattatatttgccccggtttgtttgttgccttaatcttcgttcaagttcgaagctttgtcaagtgctacgttcgaacttttcccgttgcgtcgcacatatcgcaatcgtgccaatcgttcgggccggtttcgtagcctgcgacgccttggcacttcgggcaggtttcgacgcaaggcgggtcgtttgcgcgcatcaatgcggcgataaaaaggccgatgcccgttccgatggaaagccaaataaacgcggcaagcgaaaagatttgttcaagcattgcaataactccttagtaatagtcgggttcgtcgaagtaatcgttctttgcgtcgtccatagcggcgtaaatagcttcttctatggccgtttcgtcgcgcttcgaaagacgcttataaatccaatcggcggattctttcttgcgaagtgggcgacctgcgatttcgcaaatcgaccaatcttcgaagtagtccgacataatacctacgtcgggttcggcactgcaagccgtaaattctacggtaatttccagaccgcctaaaactttaacgtttgtttgcatggcctgaactcctttgtttgttcgattggttcaatgatacgaacaaacttcgaagttgtcaagtggtgcgacaaacttttttcgttaaagctacgatgccttcgacgcttgaccgcctgccgacgcaaacgttcttcggttcgcattcccgaaacagcaagtaataatccggctttgttacgataaaacaacgatgtttgcgcgcaagttccttcgcttcgtgcaatgtcatttcatgccccttgttccatgtattgttcgataactgcggcggcgtcttcccaagaatagcaaacgcaccaaccgaagccctgcgattgaacgaacgcgccgaattcggcttggtcgtcgcttacgccgccttttgacgtagcttttaccggcttttcgctcggcttcttcatttcgatataaagacccgaccagccgccccggcgaacgggcaagcatacgtcggcaacgccagttcgcacgccctgcgccttcatttgcgaaccccggatagcgcgcgactttgcatcgtcgccccggcttccgccgttgggtatatggtgcaaccaacgaagttcgggccagcgtttgacctgcaacgcggcccaagcgaataatgccgtttggtgcgccgcttcgcttcctgattttgccaatgtttcgggcgtcatttcgaaaccccttacggcaacttatggcggtcgcgacaaggtgcgcaaacgccgttaattaaacgcggcatatcttcgccgcaaaggtcgcaaacgcccggaacgcctttcggtattgctgcggccttgcggcaaatttccgcaatgttcgcggcttcttcgacttccattaggtcggctgttttatccgcttcgtctgccattgttcgccctttgtcaaattgattataaaacaagtttaaagcattttaaacaagcgtgctgaacttttataagcttctttgcaaagattcggcggaagttctgaaagcaagccgctttctttagcttcttcaatagcacgctttacgcaagccgtttcgccgtctttgctgtttcgtgcgaccgacagtttggacaagcgtttgtgaagaaacgaatagcttacgatgttttcattcttcatttgttccgaaatagaagccttataccgtgccgcttcttcaaagctgaaatttcggtattcgtcaagtattgtttgcaaacattccaaggcgctttcttcaatttcgttattctgttcgatagacgcataaaacaacgaaacgtcgtcattattgccaagcctgcgaacttcgaagccgttttcttcgtggtcaattacgacaattcgtttcggcttatagctttcggccatcttgcgcaacatgcccacattgaaccccggcgcgattgcaaacgccttatataccggaacgcggcttgcgggttccatcgcttgcgcatggcgcataaattcgccgcctactggcgacggttccagccaaacaacgtcggcaggctttgcggattcgtctttaacttcgacttcttcgttcatgttcaaaactccttcggttaaggttcttcaagcatagccgaccttttgcagtctgtcaagcaattatgaggtattgcactacaagcggcaaggtacagatagaacagtttttatatcgtcttaatcattgatttatatacaaatacattaaatatatcttataccttaacttatatttttctaatagtatatagtgcatagtatggcagggtttgaacttttcatggtgttttatacagcatactacatactatgaggtatcctaggggtatagggtcggggaagtcgatatatttgatgtattgttttaaaatcaatgacttgcgcgctatattcgtacctaaacccatacctcaaaacaaataccgcataactcataccttacgacaaagaaaagaccgaacttctaacaaggttcggtcgtattttattttacaaaggccattcgcaagcataaaaagcgccgttgtattcatcgcactttttgcgaatatctggcggcaagtcttccgcttcgcatgttccttgcgccacgtcgtaacgtgaatcttcggcggattgttcgcaccatttataaaagtcttgcccgattgctttacgaacaaatcgggcctttgctgttccgggctttctgtattgggttcgaatcatggttgcaccttcgcggttcaatgtgggcaggcaagccccattccggggccgctggcggggttacaggaaggcgacggtatccgacaggccaagggcacgcgctacggccttgcggcgttcctgcgccttgtcattgggcgcgcttcgcatccaaatatcggcggcgcgttgggcgtgttccgggcctgcggttcgcatagacgcgatacggtgcgcttccttcgcttcgttcttcgtaacttcgacgacttggcggttaatactcattttgtgcatttggcttttcctttcggttgttggttacgacgattcaactttagttcgttaaaacttcgttgtcaagcttcgaacgaaaaaaaaccgcccgaaggcggcttgttgtcttttcgcaacgttgttcaatagttgataaggaattgctttacgaacttgcgacggtctttcgatgctatgcacaaatcgaccaaagggcgatattcaggttcgacgcgattacgaacgcgcttggcgaagttacgaatttctttgccgtctgcgccccaatggtacaaaagcgcgatacccaaagcaaaatcaagaatcgtaagttcgttcatagtccgaacgcctttgcgtttgaaatcatataacattgtgcggcggttgcgaacttatcatgcgccagctttggccccaacaattgcacgtcgccgcgttccgtaagcgtcttaattgcgcgtttaagtgcgccagtttcgccgatgcggtctttcttaaaagtcgcaagctttgttgcccgcttgtgcaaatacgaataaggaacgaccttttcggcgtgcatgttcgcggttccggccttatagcgcgaaatttccgaccaaggggctaaaatgtaatctttaataatcttcaacagttcggcaagctgtttcgtttcttcgttatcgccgccaatttcgccagcgttaaaacggtctagtaagttgcgaacatcggcgacaataaggttcgttgcccatgttgccccgtcgattgaaataatcgggtcgtaagggttgcagccaacagcaacaagcgcggcaagcttcattgccttaatatgcgcccggttccacaaatgccgctgaacttccgccgacgaactgttaatgttcaaatcgcaatgccggtcgaattcgtcaaacaatcctttggcttccggcgtcatttgaacatgaacggctttatgttggctgttcaacattaaagcatgtgcgcaaaccgtcgaaagcctgtcgataagttcgaagcttggttgcgcttggatatggtacggattcaaaggcgggcgttcgccgcgatattcgattgttgtaaaacgcggcaacaagccttcggctatcaatccttcgtgcaaaccttcgtaaaacttttccggggtcgattcgccaagcaacgtaaaagccggggcggtaactgccgacgtattcttttctttgtccgaataaatcgacgggcgcaaaacctttccttcgccgcttttattgtaggcatccaacaagaaacgacgaaggcccataaggtgcggcggggcgttatgcgcggccatttgttgaagataaataccgaattcgccgaccatcgaaacgaacgacgttggccccttcgacatatatttaattacggcttgcgacgatgcgatttcgcccggcccgatgaaatcaacggcggcgggtacggtgcggattacttgcgccatcaatttatcgacgccgcttgcgattgcttctttacctgttccggtcggcgctagaagcaagacgtattgattaagcccggttcccgaaacgttgtacgccctgcccacaataccggccagaaagccaagcgcgccagccaaagcgatttcggcaacagggcgcggcgcttgtgcgtaaatgaattgggcgatttcgccgacaaggccgggcggaaccgaataaacgttggtcgtcggggctggaattgcgacaggctgcggcgtttgttgcgttgcgtcgctttgtgccattgcgcgcgattgttcggccttcgcctttgcttcgattgcttcgttaagttggttgcgcaatccgtcaatatcaacgggcggcaacatgcggtcgaagcatttgttaagcatgtaattaacgtaatcgacgcgctttcctttttcgcgttggcccaaacccgacgcccgaaacattcgcgaaatctgcgcccggttttgggtatagaacgcgataatatcgaccaaggcaaagtcggcttcggattgcgacgggtaataatcttgccaacgaccggcgtaaaggtcggcgaatttgtcgccgtttgctgcggctgttgcacgcgctaaaatttcttcgtcggtttctttggcttcggcaacgccagcataaacagcggcggcaaccgaacccgaacccatttgcgaccaaagaacgttcaacagttcgccgcaatctttaatcggcgcattgcggtaaatgtcgccggtcatcgtcatataacgcgccgacgaatagacttcgataaaagaacgacgacggcccgacggcaaagcgcctttaacgatgatatgaagaccggaacccgacggcgaacgttcggcgtaactgtcaaattcgttaaagattttaacttggcggtctaacgctgtttggtcgccctttgtgtcgtcaaggtcgataaacgcgaacgggtcggcttcggtcaatacgaaaccaattccgctatacatgccggaattcgtcaaggcgtgcgcggcttcgtcaaagcttgcccaagtgttcgggtcggtaacgctggcaagtcttccgttcaacgctgaataaggaaccttcgtcggtttcggcccgtctgtatcttcgtaacgccaaacaacccattggcggaaaatccgcatttcttgcggtatattgtttaacattacttcgccgcctttttcttattcagatattcggaaagcgcaccaatataaaggatgcccggattgtctattttaccagcggcaagggtcttcaaccaaccaacgctaaacccgcacgcatcggaaatttccgcaaaggtcttatcctttggcttgccttcaatgtaggctttcaaatcggctatggtttcatcgcgccaccaagtcgaattcgcgataactggattcggtttcgccggttctttgcgttgcttcggtcggctggcaagcctgttaagaagcggcgacagttcgcgaaccaacttgcgttcgatttcggctatttcgtcttcgcttgcttcctgccattcaatgacggttgcgccgtgcatggcgaaggcgtcgcgccgatgatgcgacgcgaaacgctggcgtaacgtccaagtcgaaccgacgtaaagaacttcggtttcgttcctaacaacatagaccgccgaaacgttcggaaggcttcgccgttcttcgtatgaaattttttgcatgttcgcgcttcccggtttaggtgcaatgcttcgcatcttaacgccggttaaaatattggtcaagggcaaaaatgcttgacgggaaattttttcggatttatgatgctggaacgcttcggcatggggccgggcgaacttcaacgaagggccgaactatgaacgcaccgcaacccgtcttcgactatgtagccgaagcccatttgaccgcatcgccgaagttctacggcgaacttgtaccgctggcgcacttcgacgccgtactatcccaagcaatcgacgcccttaacgcgctcgaccgtgttaagaagtgccttttctacggtcgcgaacttggcccgctggccgaaggcgtcgaaaccggcgaagtgtatcaaaattgcaacggccttccgggctggatttccgaccgccccgaagacgacgaaaaagcccgcaatatcattcatgcaatcatcggtaaggcaaccgaagcgggcgaactgttggaagccttgcacgcaaccgccattcgtggcgaaaccttcgacgttgccaacgctggcgaagaaatcggcgacggcttttggtacgacgcccttttggcccgcgcttgtgggcttaccttcgacggcatccagcgaaccaatatcgccaagcttcgccatcgcttccccgaccgtttcaccgaatacgacgcgaacaatcgcgatttgttcggcgaacgtcgtattttggaagaaggcgaaaaaacttcgtcgtaacgcttgacaacatcgaaaagccgtcgtatagttcaaccataccggcgcaattgtgcggcggcttaaacgaaaggaaggaaattatgtcatttaacgaaaccgcaaatcgcgacgcaaagattattgcttgggaagccgcagttaaggcgcttgccgctgcgaaggatgccgaagccgcgttgcgtaaagaagtcttggccgaagctttcgcgtttgacccagaagcattgcgcgaaggaaccgaaaacttcgaacttggcaacggttacaagctgaaagccgttttcaagatttcgcgcaatttgaacaacgaaaacgaagccgtcgataaggtcttgtcgaagattgaaaagaccagccccgaaggtgcgtttatcgccgaacgtctggtaaaatggaagcctgaactttcggtttccgaatacaagaaacttcccgaaaagtttaaaaagctgttcgacgaagttgttacttcgaaagaagccatgccgtcgcttgaactggtagcgccgaagtcgaagtaatgcgaagacgggaagaacaatcggccttagcccttatcgaacgattcttgaaagataaaggcgggcttacttcctatcaattggccgaacttttgggtatcaacattcgaaacgttcggccatacatgaaaattttgcacgataggaagaccgtatttattcaggattggaaaacgccgaaacatgggcacggcccgaaggttccggtttggcgacttgacgaatacggcgacggcgacgacgaaccttatccgaaaccaactagcccacaacaacgggcgcgaatttacaggaagcgcaaaaatgcaaatgtccaatttaaaaccggcgtcggaactggcgcaacgcttcggcgttaaagcgttggtttatggcgggccgggcatgggcaaaacgcctatcatcaaaaccgccccgcgcccggtcttgtgcgtcgtcgaacccggcatgttgtctatgcgcgacgcgacgaatattccggcatgggatgcttacacgccggaacgaatcgacgaattctttaaatggcttttcacgtcgaacgaagcaaagaactttgatactgtcggcattgattcgatttcgcaacttgccgaaatcatcttgaccgaagaacttaaacgtaacaaagacggtcgcaaggcttacggcgaaatgtcgcgtcgtgttatggaaatcgttaatgccctgtactatttgccgaacaagcatatttatttgattggcaaacaggccgtagcagacgaaaacggcgtatcgacgaagcgcccgtatttccccggtcaagacttgaacgttaaggttccgcacctttacgacgaaatcttgcaccttggcgaagtcaatattccgggccagccgaaacccgttgtcggctttcgttgtctgccgacgttcggaatcatggcgcgcgaccgtagcgggcggcttaacgaaattgaaccgccgaatcttgacgcaatctttaaaaaatgtatgtcgtaacgcttgcaaagttttataaaagcgttatcatagcgaataggcgaattcgacggccttaaactgtcggaacttttcgaaaaggtgaattcaaatggcacaacttatccaagcgttcaacgcgcaacagtacgacccgacccaaggcggcggaagccttcccgttggccgtcatccggtcatcatcgaatcttccgaagtcaaggcgaacaaggcgaacgacggcggttatcttcaacttaacttgaagcttatcgacggcccgcaaatgggcacgaccggcgcttatcgcctgaacctgtaccattccaacccgcaaacggcagaaatcgcgcatcgccagctttccgcaatttgccacgttatcggcgttttcaacgtgcaagattcgcagcaattgcacaatatcccgtttatcgtcgaagttggtttgcaaaagggcgaagaagcggcgcaaaagggttataccgaagttaaaaaggtattcgacattaacggcaacgaaccgggcaaggccgggcagggcgcagccccggcgcagccgcaagcccaaggcggcttcggtcagcaacagcccgcccaacagccgcagcaaccccaaggcggcggggcatggggccagcaacccgcacaacagcccgcagcgcagccgcaaggcaacgccccggcttggggcggtcagccgcagcaaccggcgcagcaaccggcccaacagcccgccgcatggggccagccgcagcaacccgcagcccaaccgcagcaaccggcaggcaatgcgcccgcttggggccagcaacagggcggcgcagccccggcaggcggcgcaccttggggccaacgttaatcgttaggtcgtaacttcgtcggggcttcggccccggcgtcttttaaaggggctgaattatcgtatgtcaaacataaaagacgcattgccgacgcctacgcattgcgataactgttgttcggttaatatcgaactgacaacgaacgataagatttacgggcgcatttatggcgattggcccaagatttattattgcaatgattgccgcgcggctgtcggttgccatccggacaccgttattccgttgggtcgaatggcagatagggcgacgcgccagcttagaacaaaggcgcatgacgaattcgacaaactttggcgaagtggcttaatgtcaagggcgaaagcttataactggcttgctgcttctttggaaatcgacccgtcgcaatgtcatatttcatggcttagtaaagaccaattgaaagacgttgcgacgctttccgccgattaccttaaccgaaattacaacgcgcttttaaggcgcaaggaaaagcaagatgccaagcaaagaagacggttccagcaagacgaacaagacgaacagcgccgaacaagcgaccatattagacgccggaaagcaaagcgttaatcttgacgcgcctggcgttgcaaaggcgcttgcaaaacgcattcttgaagaaatcgacgaatattgcgttcgcacttacgacggcgggcaccgttcgcaccttggcgcaagtcttatcggtcgtgaatgcaagcgttatttgtggtatgtcttccgttggtgtttgcatgaaaagacgaccgggcgacaacaacggttgtttaatcgtgggcatcgcgaagaagcccgctttatcgaatggctggaaggcatcgggtttaaagtttggttcgaaaatcgcgacgaagcgccaaacgaaaagggcgaatatccgcaatatcgaatttccgacgttatggggcatttcggcgggtcgcttgacggcatcgcaattttgcccgaacgctacggaatcgccgaacccgtcttgttggaatttaaaacgaacggaacaggcgcgggatttaacaaacttgccgacgacggaatgccaatcgcaaagccggaacacttcgcgcaaacttcgacgtatggcaagaaatacaatttccgttattgcgtttatttgaacatcaataaaaacgacgattcgttgcatattgaagtcgtaaagctgagtcataatcttggcgaacaaatgatcatgaaagccgaacaaatcattatgtcgcagactgcgcccgcgcgactttcggacaatcccacatttcacaaatgcggctattgtcacatgaaagaagtttgccataaaggcgcggtcgttgaagtcaattgccgaagctgcgcattcgcccggcctgttgaaaacgccgaatggttttgcgacgttcacaacggcgtaattccgaaagactttataccgcaggcttgcccgtcttatattccgataacagcgagtgtttgatatgaaatacatgggttctaaatcgcgttttgctaaagcaatttatgccaaaatttgcgagatttcaccgcgcaatggtcgtgcatgggtcgaaccttttgctggcggcatgaatatgatttgcgaagttccgcctgaagatggcccgcgttatgccaacgattgcaatgaatatttaattgaattgtttaaagcggctgtcttaggttttgaatttccagaatttgttacaagcgaagaaagaaaatttataaaacaaaatcctgaaaaattcgccccgtggcaagttggctatgctggtttcatttgcggctttggcggcgattttaacggcggctttgccgggaaatcaaatacaaaaattggaacggttagaaactatcaagacgaaggtgcaagaagcttaaaaaagcaagcttctaaattgaaagacgttttcttttgcaatgcttcgtatgatgaaattctaattccagaaaattcaattgtttattgtgacccgccttatgatggagtgacaggctacggaattgaattcaatcattgcgaattctggaattgggttcgcaatatctcaaaagagcatgaagtatttatttctgaatacaacgcacccgaagattttgaatgcgtttggcaaagcgttgcgacaagctctctaagcgcgaacggaaaaagcggcggaagcaaacaaagcgttgaaaagctttttaggattgcaaagaataatgtctagtatttacgcgaatcgttggtatcaatcagaagcggaattttcgatattcgactatttccaacgcggcggggtcggaaaccccgtcgtcgccatgccgacaggaaccggaaagtctgtcgtaattgcgaatttcattcgtcgcattttcggatattggccgaatcagcgcgttatgatgctaacgcacgttaaaaagcttatttcgcaaaatgccgaaaagcttttgtcggtttggcctgtcgcaccaatgggcatttattccgctggcctgaatagccgcgaaatgattatgccaatcgtattcggcggcgtgcaatctgtcgcgcctgccattaaaaaatcgcttgaagcgaacgacggcaagccgccgcatttaaaacatttcggatggcgcgatttattgattatcgacgaagcgcatttgttaagcccttcggaagatacgcaataccaatatattatcgccgaacttcgcaagattaacccgcatttaaaagttatcggttttaccgcaacgccgtatcgtcttaaacaaggcatgattaccgaagacgacggtatttttaccgatatttgttacgacataacaggaatcgaagcgtttaaccgacttatcgccgaaggctatttggccccgctgatttcacgcccgacgacaacgaaaattgatacgtcgaaccttaatctttcgaacggcgattttaacggcaagcaagccgaagacgaagccgaaaaagtcatttacgaaggattgaaggaaacttgcgaacttggttacgaccgtcgccattggcttatttttgccgctggcgtcaagaatgccgaacatatcgcatctatgcttaattcgttcggaataagcgccgtcgccagtcattcgaagttaagtgaaaaggaaaacgacgcgcgcatggcggctttcgaagctggcgaattccgggcacttgtgggcatgaacaaatatacgacgggctacgacttcccggcaatcgacttaatcgccgactttcagcctactatgtcgcccggcaaacacgttcaaaaaggcgggcgcggaacgcgaccttcgccggatactggcaaagaaaattgcttgtttcttgacttcgccggaaacgttcgacggcttgggccgattaacgacccggttaagccgcgcaaacccggcaaaggtgcgccgggcgacgcgccggttcgtatttgcgaagtctgcggggtttataaccatgcttcggcccgtcattgcatggcgtgcggcaatgaatttacttttgaaacgaagttgtttgcaaattccttcggcggcgaaattctgcggtcggatgcgccaatagttgaatacttcaacgttcaaaaggttatttacggcttgcacgaaaagaaaaacgaacacggcgttttaacttcgccgccttctattaaagtttcgtatttctgcggctttcaaatgttcaatgaatggctttgcctagaacatccggggcttgcaggcaaacgggcgcgcgattggtggcggcaacgtcattcggaagaaccgccgccgactacttacgaagcattgcgccgcgtttcagaattgcgcgttccgtcgcgtattcgtgttcatacgaacaaaaaatatcccgaaattctttccgctgaatggtgaaatatgacgaacgaaattacgaaatcgcccgattcgaacgtagaaaagaaccgcgaaatgttgttgcaacgttccatcgtcgggcttgcgaaatacggcgtaacgaccgataataacccgcttacgttgcgggcttggctgcaacatgcgctagaagaagccttggatatggcgaactatcttcaagcggcgatttccaaacttgacgaagaaggggcaaaccatgacaacgcaaatcgacaataacgttccgattcctgccgacgaagcgccagccgtcgaagaaaagaccgaagccaaaccggaagcgccgaaaaagaaacatcgcgccagacgtgcaaaaacgaccgccgttaatcctgcggcgtctttgcttgcggcattgaagtttgttgccgtagcacaaaagaaggccggaacagttcaacagcaattcggcgtaatttctggcaattgggccgcagcgtcgaacggcgttcttactgtcgcaacaaaagtcgaagaagatttgtcggcttgcccacatacttaccaacttatcgacgcgctttccaaggtcggcgaagaactggcgattacgcaactttcgccgacttcgcttgcggtcgtttctggcgcattccgggccttgattccgtgcgtcggttttggcgacgttggtattaccggccccgacgaacgttgcgccgtaattgacgaccggattaaagccgcattcgaagcggtcttgccgcttgcgacagacggggcgcaacatgcgcaccttgccgccgtgctgttgcagtctggaagcgccgtcgcgacgaacgggcacgtcttggccgaatactggcacggcatagaccttccgccgatgctgattcccaaggcttcggcggttgccattttgaaggctggcaaggcgcttaccgggtttggctattccgggccgtcggcgacgttttggtttgaagacgattcgtttattaaaacgcaacttttcgccgaacaattcccgaactatcaaccgcttttcaactgcgaaagtttgaacccttggcctgttcccgatgaattttacaaggccgttcgttcgattgaatctttcagccgaagcggcgttgtgtattttgaaaacggcatgttggcttcgaacgaacaagaaacggaagcttcgacttataaaattgaaggtttgccggaaggtatgggatttaatgcgaagtatcttcttatggtcgaatcttcgtttaagaacgtacatttcgacgaacaatcgaataaagcgttcttctttggcgaaaacgtgcggggcgttcttatgggtattgaccgaaacagcgcaacgccgtataatcccgaagcaaacgaatttgaagacgacattccattttaagaaggttcgaatatgttagacgctaacggctttatcgtaacaaaagcaagccgcaaaattgacaaaatcgcgtcggcggttcgtatgttgcttcggcctgttgaatttatgacagacgaagaactaatgtcgattccagccggaagcgtcttcgttttcgacgttgaatgttaccgaaactttttttacgtcgcttttaagtgcctgtcgaatggaaagttcgtcgctttcgaaaggtcgcccgactttgattttcccgaattgaaattgcgttggatgctttggcgcttttgtcttgtgggcttcaattcggcaagttacgatattccaatggtcgaacttgccgcgaagggtcttagctgcaacgaacttaaagaagcttcggatttcatcattaaaagcggcataaactacggaacgaaaaaggttacgccgtttgatattgaaaagaaatataacgttcaaatcggcaaatacaaccatatcgacttatttaacgtatgcccggtaaatggcggcgtatctgctaacccggcgtcgctcaaactgtattccggtcgcttgcacgccgaacgaatgcaagatttgccgtttccagaatcgcacattttgacggcggaagatgccgcagtagttcgcccttattgttgcaacgacttagcgaataccgaacttctttttaacgaacttgcgcccgaactaaaattgcgcatggaaatgtcggaagaatacggtatagaccttcgcagccggtcggatgctcaaattgccgaagctgttattaacagcgaattgcaaaaagtcttaggatactatccgcgcaagcccacattagccgccgatttggtcttgcagtacaacgccccggatttcatttcgtaccgttcgcagcaattgcgcgatatgttcgaagtcgtcaagaatgcccgattttatcttgacggcttggggtcgccgattatgccggatgaaatcgacaagcttaaagtaaaaatcggaaacagcgtttataaacttggcatgggcgggcttcattcaacagaaaagaagactgcccataaagcaaccgacgaaatcattttggcagataacgacgtagaatcgttttatccgcgaatcatccttaaccaaaagcttttcccgccgcaccttggcgaagctttcttgcaggtctataaccaaatcgtcgaaacccgtattcatgccaaagcgcaagccgcagcatgtaagaaagcgggcgacaaggccggggcgaagaaatggaagactattgccgatagtttgaagattacgattaacggaagctttggcaaacttggcaacaaatattcaacgctttacgcgccgcaacttatgttgcaagttaccattaccgggcaacttgttttgcttatgcttatcgaaatgctagaagacgccggtatttcggttatttctggcaataccgacggcattgtttcgaaatatcacaaagacagacataacgacgttcgggccattattgccgaatgggaaaagcgaaccaacttcaagaccgaagaaacgcggtattctgccgtttatagtcgcgacgttaattcctatgtcgcaatcaagacagacggcggcgacgaagaagcgcgctttcttgatgaacgcctgggcgtcaaaaccaaaggcgcatattgcgaacgcggttcggcccttaattcgattctttcgaagaacccggaagctttggtatgttccgacgctgttatttcattcttgaagaacggaacgcctgtcgaaaaaacgattcgggaatgcaaagatattcgccgcttcgtatcagttaagaacgtcaaaggcggcggcgaaaagaacggcgtttatcttggcaaggtcgttcgctggtattacccgaaaggcgaaaccggccatatttcatacgtcggaagcggaaacaaagtcgggaagacagacggcgcacgccctttaatggatttgccgaccgaatttcccgacgatgttaattacgaatggtacattaacgaagccgtcgatatgctttacgattgcggcgggcttcgtaaagccgaaacggcttcgcttttcttttagttaagcgtcatcgtaagcgattcggaataagtcgaatatttactattcgaaataatttgcgaatctacgataacttccagcgtaccgacaaggccggtaacgttaagcgtcgtactgtttccggtcgtcgtaactgtcgtataaccgccagcccctacgcgccagcgaatccgggtttgcgttccgctttcccggttgtctgttgtgtcgccatagacgcgcaaggcggtatccgcgcggctgcggttgcgccatgctacggcaatcgacgttgcgcccgtctgcggggctggcgtgcggcttcctgcaagggttagatactgcggcggcaatggcaggcccgcccggttcgttacggcgctggaaaaggccgtagccgacccaatcggaagcgttgcgcttgtcgtttggtcaagaagtttaagataacccgtcgttccgaccgaaagaaggttaggaaccaagccgtcggcggaactaatgaaccaaacgcggtcgtttgccgcatggttcgccggtatcgtatccaaaacgccgcgatacagtttcgggaacgtaacttgcccgtttccattatcgacgaagcccacataaacgaacagttcgttattgaccatcaagaaagccgacccgtcgcgcgcttggtcaagggtcgtatattgcataagcttttcgatagcggattgcgcgacgcctgtaacaacaaacgtcgaacttgtgtcgtaacggtcagttgcggcaacggtcgaagcgtaagcgttcaacagcaagccgccgccgttgtaagacgcatcgtttagcgccaaagtcgggtcggttgcgaagttgtcaaggctaaacataccgtcgtaagaaatagacgcattgcccggcgcaacggctgcgcaatacaaccgcccggcgttgtcaaatgtcgccgtcgtttcgttgctatcgtttgaagacaggaaagcgggcggcgtgaaaagaagccgcgtaacgacgttttgcgcggcggtatttgtgggcatccatcccgaaccttcgggcggggcaaacgtaaccgtcgaagacgaaaagcggtcttgaacgcaagaaatcttgatttcgttcgaagttaattcgccgaaatcaattttcgtaacgcgcataaccatattcgaaatgccaaacggtttccagttcaaaacaaatacgcttccggggcgcaagttttgcgctttgcgattaactacaatatcgcatttataaagaggaacgttaagcaacgacaattgacgcgacgccaacacggaagcaaccgacgcaacagcgcagcccggaacgttaatttcagtcgatttaacgcggttttgaaaattgatatttgcgaagtcttgcgtaattgctacgctgtcatcgtagttatttgaacggtctttaaatgtaacgcgacattggttaaacgtattttcccaagtcgttttttgaaaattcttcaaagttgaaatgctagattcgtccaaaacaagcaagcttgaaattgtgtaatcttggcgaattaacttcgcaactatttttgccgtcgccgggtcttgatacaaaacgccgtcggcaacgcgcataacttcttctaaaacgtctttgccggtaattgcggattgaacaataagcgacattcctaaaccttcgttataaagagtttgggcgcaagctgtcaaagaaggcaaatcaagctcggttgctgaattaccaaaccggccccatttttgcgtaaaggcgtcgtaaataatttccatcggattaacgtcgtaaccgttcggcataagcgaataagtcgcatgaaggccagacgtaagacgcgacagttcgaagctaaacgcttttggcgtcgtactggttccgatataaaacgctttgaaaaccgcacgcgcaaagccgttataggctggaacgtttgcgccaatcttcgaaaccaaataagaatcttgcggcgggtcaaagcggccatcgtagaacgtcattgttccttgaagcccgccgccttccttttcgccgccgaacaaatcaggaaggttaatcgaaatatcgccggaagccatatttcccgaccaaatttggtaagtatccgcccaaaccttgcgaagctttacgccggggccaaggcacaaaatgcaatcaatgcccatataatttttgtagccgaccgtaacgcgcttcgaactgaaaaggcccgtcttaactttttcggtaatcgcaaccgggcgaaaatcgccgtaccaagccgtaatcggcgatttctggcgcaccgttccccacactaggggcatagggtcgccatgcttcgaccgtggaaattggaagtcgccaagcttcgccgcgcgggcgttttcaatgttcggcttcggggtaagcgccgcaaccaaaagaagggcgacgataaaaacgactaagtaccacatttatttaacccctgtaacgaatacgttattcgattcgcccggaacaaacgggcaaccaccgaagttgcgttgatttgcgaatttcgggcaaccgttcgcgcctgaataagaatggtcgcaacctgccgtaacttgaatcgaagtacctacggaaagtttgctaaattcataattgattgttagaaggcttcccgattgattaacaatcattcgacgttcgttgcgggcgggaattgcaatttcgccgccgataaaccaaccgttaggaaaaccgccaatggaaggaatgccaataacgcgaccttctatcgaagaaacttgcgtatcaagcgaattagcgacgcgggaaaccttgcaaagttcgtcaaacaaaacgttattgcatggcggttgaacatacacgttcgggatattgccttgcagaatcgaaccaaacttggaaggaatgcggaacgttgcgaattcgtcatttacagtaattgacgcaatcggccctttccagtaagcgacgtaagttccggcgtcgcgttgaagtcgataaatagtaaccgacaacgaaggcggcgtagtttgaaacgcataatctttaacgatttgttcgataattggaatatctatcgtaatatctacgttatcatcgtcatgcgttccgactttcaaaccgccgcgcttcatacctgcaacgggattaaacgtaaaggaattgaagatatgcggtattgcgtcggtcgtcatgtaataatttttgtacgttccgacgaattcgtaaagttcataaggcgcgctatccgaaacgctttcttctttaatatcgtaatcagacatatttaaacttccgccgttctaatggaaagattcaacagactttcaagcccgtaatgtttccattctatcttatcatcgttgattctgacaggtagcaaatacgaaatacgtttgacaacttgccaacccgcgcccgttggaattgcagggtcgaacaaaataacgctgttgccgcttgaaaccgaagcgccgattatgcttgttcgatgaatgccggaattggtttcgatttcgatataacgatgcgtcggaatcggataaatcttttcggcgtattgcgtgccttcgaccgtgtagttagttgcagcatcggcaggcgcgacaattactttcaaatcttggcgatatgtgggcatccaaaacttgcgggcttgaccgcgcgcataagctaaaacggtcttccaataatccatttcttccggcgcataaatgcgatttactttaaaagttcgcggcccgccgatgcggctataatcccaacgcgaaataatatcttgcgtgcccgtttgattgtctaatgaaacttgcccggtcgaaacttcgtctttaaccaattcgtcggcaagcggtcttttttcaacaaccggaacgcccaaaaactgcggtaatgaaacagccgacccggtacgggttaaaactgttctttgtcgcgttagctttgcattaaacgaaacttcggcaacgtcatcaacggcataacgacttaatgccgtttgattgtcgataagtgcgggcgaacccggcattatcaaagaatccgaaggaatgtcgaaaagcatattcgaagtaagaagcgccccgcttgcagtaagcgaagaaacttcaacaagcgcggcattgcttggcgtttgaatcaatacatattcgcccgccctaatgtctgttttcgtattgtcgtaataaagtacgttagttcccgccgtagttttggcggttgttcgcgtcgcatattgatattcaggaagccaaagacgaccaacagcggccaagaaatcgccgtaaaaacgccgtatttgttccttgctatcaaacacggccttaaacgacgtttcaatgcgcggaacttcgccgcgaagtgctatacgttgttccgttccgtctgttgcaatcattaaatccgacaaccattcccaagtttcagtaaccggaacttcgggcacaatgtcaaatttaacggcgcgggttccggtaataacaatcggcagagggtcggcaacgttggaaaaatcaaaaagaatttcgacgttaatattcggcgggcctgaaacgccgacagttacgttatagaaaatttccttaagcggattcatcgaaaacggcgtagcttcgcccgaaatttcaatgcctgcgggctggctaattgaaatttcgtcaagcgtcgccgaagtttttacatatgcgttccatacgctaacttcgcgggtttgcgaagaagcgatagtttgcaaatcaattttcaacggcaagacgtgaattcgattataaaaatcgtcgaaaaagtttggcgcttgctggcccggaattgcccacaaattagcgggcgcgattcgaaacggattgcgcgggccttgcgccttgcgtgtttccgaatcaaacggcgcggggtcgaacatgcgttgcccgaaggcgttgttatcgttagacaacgccgggttaatttcgggataattgcggtcgttcgttacttgtccaagtcttccggccatgatttaagttccagtgtaacgaatagcgtaaccgtaagttccggtatgattcggcggcgtcgaagtgctgttatctacgccgttgcgcgtcgttgcatctttgcgaagccaaggataaaccttccattggtcagcgctataagttacgatgcttcccggcgtcaaattgtcaagacggcaccagcgggcgttacgcggattaactacggtcgcgacgccgttgttcgtcatgttcttaacgcccttgattggaagaagaacggttgtcgaattgaatgcacttggcaaagaacccaacagcccggcgacaagacccgccgaaccgtttttaatgccgttcgtcgaatcgcccgcgccataccatcccggcgttccaagtgtcgtataaaaatacgaacttcctacttcgtccgaccaaaccccgcgattaaacaagccaacgccattcgttgaaaccgaataaaagcaataagaataaatgtcgctgaacgttgttgctacgttgcaaccgttattcgaagaagtgtaagtagaattatgcgccccggtaatccaagggccgtttcctgcgcccgcaacgtcggaagttccgaacgaaagttgttggtaatagtcggaattataattaacgaccatataaacttcgtcaggattcgtaaaaatatgaatttcgtatgtaacaggaaaagtcatatacgaaccgccaagtcttacgaagttcggcgaagctgtcgtaagcgttcccgaactttgacccaagccgcctttaagttcgacgaaatttccgcttgccgcaacgctgaaaaagcttgcgccttttgaaagaatatttccggcaggattcgcccaaccgttcgcgatacaagcgtttcgaagggctgcggccaagtctgaaatattggcggcggaacctgtaacgtatgccattgtttgaactccttacatttcaagcgcgacaaaatcgcgccaagacgtgcggttaatattttgacccattacgaaggcccgcccgccgaccgctttaattgcttgcacggcttgaagtacggtcattcccgtttggtcgattgttgaacttccgccagattgaacgacgttttcgacggcattgttaaaaccgcttacaaaataaacgccgtcaagttcgccccaaacgttgttcgtaatgccgacggttgctgttatatcgtgaagaataatcggttcgacttggtaataactgcctgccggaacttgacaattcgttgtcgccgggcctgcaaggcaactgttaaagttaccgtcggaaccatgcgaaaaaggccacattgcgggctgataccaagacccgtcaagccttcgcatataaaaattcgtgtaactggaaattgtgtcgccgtgatacgggaaaacttgttttgtatcactaaagcgcagcaattcggcaccgttaaagcttccggcgcaaacaagcgggttcgggaattcagccggtcgcgcatacggaaagaacttgcccaaatagccatgcgtataaaccggcgtgccgactttcaacataaacgcgatacgttgcgcgttcattgtcatgtaataagtaattgcgttattgtgggcaggaacgccagacaattgcgcgccgggttgcgtatcgaatgtatttccggcgacgtatccggtaaaagcgcccaaaagcaaattataataatcgcctgcaacgctttgataagttcgaatccctatgtaaatttcttcgttgccggataggcccaagcttttacctatccattcgcgattcgccgaagccgtattgtaacgaagcgttgtccatccgttagcttcggcaagggttttaatcgcggccaataattgataatggcaatcatcgccgccgcccttcgttaatgttccgattgcgtaacccattatttaacccctacgattttcgctaccgtcgaaccgttttgttcgatggtttcaataataaatgcttgaccttcggaagacttcaaaccggccaaggcggcttctttcgattgtaccactacggcattaaaaggaacattgacaatcggcgcgggcgctgcggcgggcgcgttgcccacactagccgccccggcctgttcgccgttccgttgcacgtttgccgcgccagcttgcaaggcttgcagatttgcgacgccgattcgtgccgttgcgtttgcgtccatgacgtattcgcgaccatgcacgacgcccgcaacttcattaacgccaattgacccggtataaccgccttctttaaatccggcgttttggctgcggatttgttgaacgttcgccaagcctgcggcaatggctgcggcggctgcggctgcgcccaacgccgggccgacgtaaggaatcgacgccatagcggcgtatgcgcttgttgcgctttggtaagtcgaaatcatggcttgcgcaattgcggcggctttgccaactgcggccattttcttgttaccggatttttgcaacgcggccaagtttccgaaaaagctattcgccgcgttcaaatgcacgttttggcgctgcaattcaatttgcattgaagccgaagcgtattcctgttccgtaattaagcgttcgtcatacatgcgcttaatttggtcgttatacgtttgatacattgccaattgtgcgtcgatattgctttggaagttcgttgtatcgacgcccattccttgcaacatggaattagtcgcgttagcttggtcgcccgcagtaaagcccgacgattgattggcgcgaaggttcttaatcgcggtcaattggtcgataaatgcttggcgcttggttacgctggcatccattaacgcggcttcctgttgcgaaacggcgttaagttgctgaataaccgtaagcttttcgcgaagtgcggcggtttccgcttgtgtcagtacgacgcccttttgcaaaaggtcgttactgatttgcataatttgctgttcgacttcgcgttgtttcggcaacatttgcaacaacgtttgttgttggtttaattccttgttgtactgataaagcgggtcggtcgcttgtttataagcttcgcccgctttggtaatctgttggttatattgctgttgcgtaataacgccttgcgacaacagcttttgcgctgcggtaagatttgcgttatagtcgcgttgcgggcctacggcttcttcgtaaatcctatcgtaagcttgttgaatatccttcgcttcctgaatcgccttaatcttttctttgattgcggcggcttcgtcttgcgaaagcttaattttcttacccaataactgttcttcgatttggtcgaaccgggcttgcgcttcgcgttccggcttcaacatatacatacgcgacaattcgttatcaagttcggcgttaatcttggcaagtgcggttgcgcgcttttccgcagcctttgcggccttttcgtcgattgcgttaggcgtcaagttcgggccagttccgcgcaatgccgaaccttggccttcggcggctttacgcttggcggcaatatcgcgggcgcgtgccatgaatgcgtttgcagcgtcgccgacgtaatctttattaaatgcgtcggtaaatgctttgccaacttcggcggctgcgcccttggcggcatcgccaacttgcatacgcggaagcttaattgttgcagcatcaagcgcagcgttaagacgcccggccatatccggcgcaacttcggccccaagttcggcaatcttgcgcaaaccaatttgccaagcattaacgacggtttcgaccgcacttgcgccgaaattaacgaccgatgcgaaaacgtattgcataacgtcggggaatttatcccaaataaccttaattgcgttgaatgcgccgacccaacttgcaattacgaaattaacgtagcctttgacaagcttaacgataacgtttccgacgttacggaactgttcgccccaaccttccgttttgctatttacccaatcaatcgccgtattccaaacgcttttaatccattcagcggcaacgcccgcagcatcgctaatataagcgaaggcggttcggaacatatctttaagcgtaacggatttatcggcggtaactgcgatttcgtcgccgaatacggtaatcgcggcaattgctgcggtaatgcccacaacaagcaacccgatagggtttgcagcaagcgcggcggtaaaggcccaaacagcggaagccgccgaactaatagccgcaaccaacgtcgggccgaacgcgaccaacagcgcagccccggcaatcgcagccgctacggcaagcgccttcatattttcggcaaggaagataattactttcgaaatgccggaagtaatgcccaattgtttgttaatttcgccgaacgtttgcgtcgcattgtttttaagaacggtcattgcctgcgacaatgtgggcaccgtctttccaaatttttcatcaatgccttttgcggcatcgttgaaagcatcgaccataacttgcgccgtaatcttgccttgcggggcaagcttcaacagttcgccgcgcgtaacgcccaagcgtttagcgattgcgtcggcggcattcggcataagttccataaccgaacggaattcgtcgccgtctaatttgcctttgttgaatgcctgcgaaagttgcagcaacgcggaaccggcttcggtagaagttgcgccagaaacgacaagcattttattaactgtttcggtaagccgcaacgaatcttgttgcgatttgccaaggtttttcaacgccatatcgaagcgcgtaaaagcttgcgccgtttcctgtaccggcgttcgcgttttgttggctacgttaaacagttcgttggtaagttccgtaacctgtcgttcggaatccgaaacgttttgcaacttgttttgaagtaccgtataagcgtcggcactttgcaaaatggcttgcgccgatagacctacgccgacaagcgcagccgccccgcgaacaaacgacataatcgacgacgccgcgcgctgcgacgattgcgcggccctgtcttgggcctgttgtagccgaagcgcagccaacgccgcccggtcgcttgccgccgccgcattggccgtttgcgtagccgtgcgggcctgttcggttgccagacgttgcgcggctgtctggccttgcgtttgggccgtattggcgcgcgtcgttgctgcggctaggttttgggctgcggtttgactttgcgttgctgcggtcgtaacgcgctgttgcgctgcggcggcttgcgcggctgcggttgcggttcgctgttgttcggtcgccagacgttgcgcggcgacggccccggcttgaagctggcgcgtagcgttggccgatgcgttgataagttgcgacaacccgccgacattgattgcggcaagttgtgtttgcagattcttaacggcggcgtcggcgcttcgggcttcggttgcgattcgattaagcttcgtcgaaatagaaggcgaaaccttatcggcaatttcgatgctaatattttcgtctgccatttcttagccctttatcttaaaattcttgcgcattttgcggccaattaaaaccgcacgttctacaaagcccgccggggcttgttttgaatatccgtcattcaaacgacgaatataaggaagattgttcgtaataaaaatccgttggccgggtttcttaccggctagaattttgcgcgcttggttgattgtttcggctgcgcttgccttttgagttgaaccgccttcgcccggaaaatgcggctttattttttcagacgaaggcgtttcaagtgttacaatccagttcgacaaagcttgcgaagtatcgacgggcgttttaaatgccaaatcgccgacaatggttaaggccgtatcgacggcgagtttagacgcggcttcgtcgattgccttagccttcttttctaaacttgccgccaaatccaataagccttttgccattacttcgccttttgttttgcttccattttcgccgaaatccgtttaaggtgttcgccgtccattctgcgaatgaaaaaatgcaaatcttccgtttgttcttcgtcgaactcaaaagcccttgcgtagtcttgcacgctagaccacggaatagcggtcggggccatagcgtgcgaacgttcgcaatccaaatcgaaaaaggcttgcatatacaactgcaagccctgttgaagttccggcgcgttggcgatgcggtcgggtattggttgcccggcgcgcatcgcctgtttcgctattgtctgttcgattgggccaagttccaacagatacgccaaaacttcgtttagttttttacttcttcttccaacgccgcatcgcggaagttcgccgacaacttggcttcttcctgcaaacgttcatacacttccggcaggtcggtaaaaagcttcacggctgcggctttggtgaattccaacggcttaccgtcttcgccgcgaacgttcttccagcccttcaagaccgtatcgacgaagacgcccataaagatttcttcggccttgtcgttgttcatcgtgccaagttcgatttgacgacgataagggcgggtcgcggcttcaagcgccttagaataacgcttgttcgacttgcccatgcgcgaaacaacgaaagtcggaatcgaaccgtcttcgttttcggcttcggtcatttgaacttcgacgccttccatttctttttcgctgttcgtagcgaattgcttataaagcgacatttgtttaactccttcgaaatttgagaaaaagggccggaacttcccggccctttaatgataccgcaattacttaggcattgccacattcggcagatacgaaaacgcttcgtaaagcatcgtatagccgttcgggttttccgcgcctgccggttccagcggaacagtaatcggcgcgtctttttcaacagccagacgaccgccgccaagaccaagcaaaggaatatcgaagacaaaaccggcattcttcgaagcgccgataacagataagccaacgtcggcattttggcgaaccgcgcgaacagccgaaaccgtcgtaaagtaagccgtaatggaaccgccgacttcgaagttacccgccgtcgtatcgaatgcgccaagaataccgacggccttgttcggcgaaacgttgttgttaatcgaaacgttcgcttcggaaacgtagccaaacagcgcggcggggttcgaagcggtagggtcgattaccgccattttgattcggtaaatgtccgaagacgtgttaaacgcatcttcgccagccgccgaaacgcgcgttcccgacttgatttcgtcgccagcttcgcccgatttgtgggtattgtcgcaagcgataaacgtaaggtcggcgttcaacttgtcggcctgcggaatgttcaacgtaaattcgttggctaccgcaccttccaagtattcggcttgggtcgaagttgggccgcttcccaactggcgttcgatgttgtacgaacgacgcttgataagcgacggcgttttttcgttcttaatgacagtaccgacgaaaagacgaatcgttttgcccgtaccggcttcggtcgccggggtaaaggtcgtatcgtcgaaaacgatagcctttgcagcaatcgacttaatgcgcgcgtagcccacattattagcgaaggccgttcccgcagcatcgccgccaatgaagacccaaagccccggaatcaggcccggcagggtcgtaaagtcggcggcggtagcgacaagcgacggaacgccagacgtaacagccatcgaaatatcgccgcttgcgaactggaagccgacggtttgaagctttgcagcggcgggcggggcggcttcgtcaataagcgtttcattaacgacaaccgttccagcggtcgaagaagcgacggttttaaggccgttgttcgtcgcattgctgaaaccgcttgcgtaaatcaattgaagcgcagcgaaggaaccaaggccggaagcggcggcgtaggtcttcgaagaagcggtaacgccggtaagcgcgaccgccgcagcgttaagcgccttcgtgttcggcagttcgcgcgcatcggcgaagaagaagccttgaagcaagcgcgtaagattcgacttcgtaaagtcgatattgaaaccgcccgaagcgtcaaggtcggtaatcgtacctttcttgttttgccgcgaagggtcgataggcgcacgcgcaacggtcgaaagttcgccgccgaaatccgaatagctgttgggttccagcccgtaccaaacgggcgtacccggaagcgttttcagcgtcgtttcttccgcgaatgcaaggccggtaatgttcgaatcaattttgttagccatttggcgaactcctttaacctaattcgtcgtattcaaattcggcaacgacgttaaaccgataaaacaaatcttcgggcgaaagttcgtttattcgggcattgcgaaaccaaaccttaccgggcgttgatttgccccggaatgaatttcgcgcaacttcggcaagcttccttccgatttcgccagcttgcgcaagcgacttcgggcaaaagatttgcacgaacaccagccccgaagaagtgtaacgcttttgaccgggcaagcccgcttcgtctgaaagcgtcgattgttcttcaaataccgtttgcgtcgaaacgcggccccaaaatttggaaccatccggcgtcgaaggttcttcgacgtattgccaacgaatttcgggaacatacccggcaaccgacgaagttttggccgaattccaatcttgccaaaaaacggcgttgatttcgtcgatagcattactataagttgttgtcatcctttgaacactaccgtataaagtatggtttgaccattcggcgaaagaacgtcgatattttccaaacgaagttctttgccgtcgcgaataacaacgtctttcaacgacggttcgaaattaaccgcgcccatataccccataaccgaacccgtcggcacttccgttccgcgaagatatgcgattgtttcgcgcatttctttgttaatcggaagaaagcaaatcgttacgtcgtgttcgacaggcgttgcgggttgcgtcggcttccaaggctgcgacgaatcgaccggggcaccgtcgcgaacaatccgccatttaacagcttggccgttcttcgcaataagcttcaatgccgttttaacttgtcggtcgaattggcccataatcaaacccgcaaagtacgaagcgcaaagccggttgcagttgaaccaaacagcggggccaacagcgaatcaacggcggttaatgtgggcacgataccaactttagtcgggtcggcgtatttggtcgtaatcggccctacggtttcttcggttacgaagttcgaagccgaataattcggcataatatcgacgccttcggcaattgccagaattgcggcgcattgtgccgatttaagttcttttggaattgcgttcgacggaaaagcgacttcgcttccgtacaaataaacgtcgattcgcggccattgcaaagcttggtcggcattcgtcatttcgccttgatagcgattcgcgaacgattccaaataatcttttgctttgataatttgaacggctacgtcgtcatcggtagccgacagggttacgccgcgttgcacggcatacgcccgcgcttcggcaatcgtaacgaacgaatttgcgttggctacgt

SEQ ID NO: 7 - DNA, 62014 bp, unidentified
  source 1..62014: mol_type = genomic DNA
cctcccgccgctggagcaggtccgggcgcactgggacaagaactttggaggcccgttcgagtggcccaaggtcgaaccgacccaggagcctctgaaggacggcccgaagtcggacaagccgccattctgaggacgcccccatgagcgagacgctggaagcaacgaagcgggagctggagggggcggggatcgcctacacggtggagctgggccggagacactacaaggtccgcttcaccgtgagggggaagcccctgatggtgacgtgctcgcggacttcctccgaccaccgcgcggccctcaacgcccgccttcaggtccggcgggaaatccgccgtgcgctggaattgacctgaaccgctttacttcttcggactgacccactatacttcttcacacgagtcgagaaatgaaccaaccccagacactgacaccgcgattcgagattggaaaggagctgacccatcatgaactacaagaagccttccgccgcatacacgggcacccaatcccgcgcggcgcaaaaccgcaagaagtcgcacgaggacttgctgcgcgaagcccgttgcgattcgagtttgaagtcaatcgccttcgaggctatgcgtgggacgctgacgaggttgagtgaccacgcccgctgggctgctccgcttgccttcgccgtcctgctgctctggggcctcgcgggggcctttgcggactacctggaccgcccggaggttcatatcagctacctgacccgggagtgtgtgcgcgtggtgaacgcggacggctcccccggatcgtgtggagccctcccggaccgctatgagcgagtgtgggtggagtaagattctgtttcaacaaccctgagaaaaggagtcacaacgtgatcatcttccgcaacaagggcgtcattgaccccaagtccatcaccaccttcggggtcagctcgaaggagaaccccggggccatcggcttcttcgggaccggcctcaagtacgccatcgccatcctcctccgcgaaggctgcgacatcaccattcacgccgggaagcgcaagctggagttcggcatcaagcgggatcgcgtccgggtcgatgacttcaacgtggtcacgatgaacaaacgccgtctgggcttcaccacggaggtcggcaagacctgggaattgtggcaagccttccgcgagctgtactgcaacacgatggacgaacgcggcgaagtgttcgaggccgatgaggtcccggaagtcgccgcggacgaaaccgtgattgtggtccggggcgaaaagttcctggatgtctgggcctcccgctctgacatcatcctgtccagcgagcctctggagcgacacgaggccgtccacatccatcccggcccgtcgcacttcgtgtactaccggggcgtgcgagcctaccggctggaccaaccctcgcagttcacctacaacatccagaagaaggtggacctgacggaggatcggaccatcaagtggtcctgggacatcagcgccgccgtccgccgcggcctgtgcgagtcgcagaccgccccgctgatcaagaaggccgtgaccgcgcccaaggggacgttcgagcaccagctggacttcgagggcgtggagccgtccaagcccttcctgtccatcgtctccgaactggcgcgcaacttcgactccagcctgagccggtcggcgctgaaggcgtcccaggtctggatcatggaccagctccacgaggaggcgaccccgatgcgcctgagcgagctggagcggacccggctggagaaggccgcgacgttctgcgagcggctgggcttcgccgtccaggagtacccgatcattgtcagcgagttcctgggcgaggaggtcctgggccgggctcatgagggcaaaatctacatcagcaagcgcaccttgatgatggggaccaagatgctggcagggacgctgattgaggagttcatccacctccgccaccagttgtacgacgaaacccgcaccatgcagaacttcctgatggacaccatcgtgtccttgggcgaacagatcaccggagaaccgctatgagcaagaccaccattcgccttaccggagacgccctgagcgccgcccggattgtccacggcatccaccaacaggctcacgcccagaaggcggagctggaacgtgagtatcaagaacgcctcaccgaactcgggaaggaggcccaggagcagatgagccgggcttggccggggctgatgcgtgccgcagacctcccgctggaggagctgggtgagtgggagctggacgcgagctatctggatgaccacggctgcgccttcctcactaagcgcgaggaggacgcccgcccctccctgggcgacctgctccagtccatgaccgcctcgaagcactgaggagcccgactatgaaaccgctgctgatcttcgtcctcgccctgctgcccctcgccacgcaggcggcaccggaggaccgccccctgtataacgcccaggagacggtccggcgtgcgcagattggcagcaattccccacgcctcgcccctccgtcccgggtcctcccggcggaggtcggggcgaagccggacccggcccgcttcgagcggctggagtgctggcacgatcccgcccgacccctgggcaaccgtattgtttgcgaacctcggagaacaaaatgagcaatgaaacccaagaatccatcacccgctgggctgacgaaaccttcggagtgaagcacccggcggaagtcgccgcccgtatgaacgtggaggtggcggagctggtcgctggcctcgccaccgtcgccgccgtcccggtcgaagatatggacccggagctggtccaggaactccagaaggagtgtgcggacgtgttcatcatgctcgcccaggtcgcggagaagctggacgtggaccttcagaccgtggtgaactacaagatgggggtgaaccgccgccgcaactggaccaagagcccgtccgggaagatgcagcatgttgagacgttcttggagccggggagcgggcttgagatggagctggacaagttctacatcctcagcgactcgggccacttctacactgaccggggcttcgagtccgcggacgccgccctgaactgggcccaatccgcggaggggatcgccgccggagccgaaggagcggtggtgccgaccttccgggccgggggcttcttcgagggccaggacggcgtgaacatctacctgggccgcgagctgcgcgccttctggaaagccaaccccctgaacgaaggagaacccgcatgacgacaacaatccagggcatccaggcccgcctcgggcgcaacccggaggacccccgcaagtaccaggtcacggtcctggtgtatagccaagtccgcccaggcctgaagtcctccacggacatcgaccccggccagtgcgcgaaccagcagcacctcctccagctgatcgggacggcgggggccgcttgcgcggagtacctgggcaacaactacggggacaacatcgaccccgtggccgcgtcccgggacgccatccgcgccttcggggaggagtgccggctgatggcggaactcgccaaggacgtacccgcgaagctgaagcgcctcgaaagcaacgtggcgaagctgtccaacgagaaccaggaacagttgcgccgcctccgctacctcgtggaccatcaggagaagctgctgcccaaggaggtcgcgtggctgaatcagcgcctcggggaactccacggaggtcagctgtgaaagacctggacgaagcggccctggccgttctgttcgaggagtaccggcaacgccttccggtcgcggactgggaggagttcctggtcatcgcccggggcgtccttgcctcggagcgggtccggtgccgagtccagcgccgggagtattttgtggaggactacctggaagccgatctgcgccgccattttgacacgctggcgcatcgtttcggatcgcccgccctggcgattcccggaccgcgaccgctccagctgaaggaactcccgtggtggaggcgctgggcgctgctcgccctcctcccgaagccggatgacgacaaaccctgatcaacacggagacaattgatgatcgagacgaacaacccgggccatggcttcttcggaacctacgccctgaagaagggcgaggaggccgcgcgcaaggcttgggccgtggccttcgaggcaatcgccgccgccgtaccctccgcgaagccggaggaggtccgcaactacctggacagcgtgtacgggcgtcacaccgcggatgaggtcctcagcggcccgtccgtcgcccaccaactccagttccgcgcggcccgcttccgtcgccacttcgcggagattcaacgccaaaccgcccgcggggccttcgaggactgaccatgataccatttgaccaagtcgaagcctacgtgggcgacttcctgagcgaactccacggacggggcctgggcgggaacatcgtgaaggactcccccgcccagctcatctacccggagcgggcgctgtggaccggggaagcgcaccagctcgccttcctgggcgagccgggggactaccgcctggagctgcgccggatcgaaggcgggcactgggaggcgatccgcgaggagcgcgacccggaccgcttcaacctgctgatcatcgacctctgcgtgaaggagggctgacgccatgaaccaagacccgaacaagcgccccaacgggacgtacaagcccaaggcggagcggttgccgcctcaacatttcaactgtcgctcctccctcccgccggtgaaccttgacgcggcgatccacgggggcctccgccttctcgccttcgccctgttccgccaggctatcgtggaggctatcgtggaccagcgcgagacggcccaaggtatcccgaccggcgacggctctgcggcgacctcctgggaggagctggagcgggtcctgggcaaggagacggtggacaggatgagggccggaacttgaaggaggaccggagctgggagctgtgctggatcgtcccgggaggttcccttcaaaccaagaaggtgacgggctacgcccgcgcctgtcaggaggccaagaacctccgattcaagatgcgcaagaccgaaggagtgagaatatggatcatgagcgagttctgagctggctgcggagcctgttcaggcggacgcccgccgccccgccgccggagtcgggaccgatcacctggcccgggatgatggccccgggcttcgaccaacaacccctaccggagaaacaccccttggaacttgatcatgaacagtggggcagcgtggtgaaaaacgacttcatcaggaccttcttgggcgaccgcctggggttcggagtcgcccgccaggtgtatgccctccacggacaaaccgcccttgtggctaaggtcgaaaccaccgcgcagtccttccagaatgtcgcggaatggcagatgtggcacgaggtccaattcaccccctgggcgcgctggttcgccccgtgtcgccgcatcagcccctgtggtatcgtcctgatccaggagcggacgcgacccctgccccatggcgaactgccgaaggagctgcccgacttcttcaccgacctgaagccggagaacttcggcctgatcgacgggcaggtggtgtgtcatgactacgccctccacctcgcctcctcgaactggttgggcaaggcgaagatgaagaaggtgaagaaggacgaatggcgactgcctgacgaagattgacaacccgacagaaacggagaacaaacatggaacatatcgacatgacggacgccgctgctgagttcatcgacaaccaaggcgtggctgacttcgcggacgcgatgcgccgcaagctggagaagaagagggcggagggccggggcggttggcacgaccccgaccagtgtcaactggacaccctcgcggtgatgctgctggatcacctggagaagggcgaccccgtggacatcggcaacttcgccatgatgttgtacaaccgcggcgacggagcggacggtcagccctccgtcctcggggcgaccttccgcgaatggctggatcaccagctcaaggcccgggacatcgtcgcctcgaacctccaagccgctctggacaaggccgcggcccggatcgcggagctggaggggatcgccggacgcctcgaaggcgagcgcaacgaggcccgccggtcgctggacaaggagcgggaggtgttccgcaaggagctgggggcggagcgggacgcccgccgccggtcggagctgaacctggcccgtgcccaagggtacatcgaccgcgtgacggaaggcgaaccgccgctgccgggagtgcgcaacgaggtccatgagcgggtcggacaggtcggggtcagctacatcagcggaccggatcgccgcggaccgcgccttgacctgggcgaacccctcagcgacccctatcaattccgctgatggcccgccggaaaccccgccgcggggagtacgtctgcacctgcggggcctatcggttcccgcaccgcttcggaggcggtcgctgctcgggctacttcatcgccgtggagcagtgggagtcgcactatgggaccggcgactgccgccactgtaactgcctcaaccggacggaggccgtgccctactgtgaagtggtggagggcggcgagtcggtccaggaatgccccgtgtggcaagagtttgtacgattcaatgagatcaaactgaagaaggagaagtgacatgagtgacgacaacacgatggacagcgtgatgattgacctggagacgatggcgaccggccccaacgccggggtcattcaggtcggggcgatcccgttcaacagccgaaccggattggtgaagccggacctgttcgaggtggacgtggacctccacagcgccctgatgctgggcggcgaggtcgatgcctccacggtccagttctggcgggaccggggcggactccagcccaagcgcccgccgaaggcgatgcgctccgcgctgaccgacctcgcccgctggttgggcaagtacccggacctgaagcgggtctgggcccaggggccgtcctttgacgtcgccattcttgagggttactatcgccgggcgggcgtcccgatcccgtggggatactccatgccgcgggacacccgcacagtgtatgacctggcgaaggagcggggctggtcgaagccggaagggacgcaagccgttcacaccagcctggaggactgccgccgccagatcatctgcctcatgagcgccctgaacgtcctccggggcaaccctgaaggagaacccaagattggctgacgaaatcgacttgagcaatgaccgcatcctccacgacacggaccgcgaagtggcccggatcgcggaggccgcggcgaagattccgcccggggagccgggcgactgtgacctgtgtggcgaatggagcgggaggctggtgggaggagtctgtgcgccctgtcgggaccgccacaagttgccgtgaatcgaagaaagttgtatgagggggctttacttcttcgggagcccccactatactttcttcacgttcaacaagaacggcaaccacagaaatggagaacatcatggcccgcaccgcttccttctacatcgaccgcgccaccgcccgcttcgaggctggtttcacctccaaggccgctcaacaagaagccctccgcgacctcaacagcgccttcgagctgctgaagcgcgacatcaccggcctggtcctggacatcgaccgggacgcccgcaccgcggatcatgatgacgtgtactggaacctggccgactacccccacaactggaaggccaagcactccgccctcgccctccgcgtgttcccggaagtcgccccgaccgtcgcccagatcgaagccctggtgaccttccgcgccgccgtgaaggccgccccggtggtgaaggtcgaacgcgccagcgacaccgccaagatcgaagccgtgaccaagtcggtccgcgacctgatggagctgcgccaggagcagtacaacaacgccctccgcctccacgacatcttcggcgggctcccggtccatgccaacgtccactacgtcaccaaccagcacggcaccaccttcctccgcgccttctactacctgaacggcgagctgaccccgctgggcatcatcatcgccgccgcggaggcgaaggcccgggaagccgaaggcaagtgagacgaagcgggagggctccggccctccccacccaagaaaaggagcccgatcatgtacaacatccacaaccgcaccctgaacccctccaccttcgtccccaccctgttcatcggagtcggggagctgggctgcttcttcaccctccgggagacgtacctgcacgccgtcccgggtcccggccccatgggcaacgcggtggtgaacggtgtgtatcagggcagcttcgaggtccgcagcagccacgtgaagaacctgagccaggaccctgacgaagccttcgagaaggcccaagaagcctcggagcgcatgggcctgaagctcacgacctcccgcgactccctgcgcgaggaaatgaacgcgattcaccgcgccaacgccgcggagctggagcgccgggagcgcgagcggaaggagcgcgaggaccgctgggccgcggaacgggccgcggaggaggaggagaagcgccagaccatcctgggcggcaagttcgccttcggaccctacgcgggcaaggagttccacgaggccccgcggggctacatcagctggttgatcgacaccctcccggacttcgaggaagggggcctgatgcgcctgaccgcccaggaggtcgcccgccgggtcccgcacctcgccctgccgaagccgaagcccgacctgtacgtgggcgagccgaagaagcgcatgaccttcgacgtgaccgtggttcgccgctacaccttcgcccgggacgcctggaacggctatggcatcgagacggtccacatcatcacgatgatcgaccgcgcgaccggggcctgcctcgtgtcgaagtccggggccttctacgcggaggaaggcgaggagctgaagatcaaggccaccgtgaaggagcacgcggagtaccgcggccaggcccaaaccgttgtccagcgaatcgcggtgatggaggactgactcatgcgccccaacctactcaaagccctccgcggaatgagcgaggcggagctgtacgcagccctgtaccaggaccccctcaccggggtcctgaaccgccgcgccttcgatgaagtccagtcggacgctatcgcgctggttgacctggactcgctgaagtgggtcaacgatacccacggccaccgcgccggggatcaagccattcaggagttggcggtgcggttggtcctcgccttcgggcctgacgccgtgtttcggatcgcgggcgatgagttcgtggtggtcaacgggaaccgggaggagctggccgaccgcctggagaaggtccgcgccgcgttccccggcttcagctttgggacgggcgcgacgttgtgcgaggcggaccgcgacctgagacacgacaaagcggagcgggagaagtccggcgaccgggcggcgaggggcgaacgaccgaagtgggtgccttgaacgcccggcggggctttacttcttcgggtcccgccactatactttcttcacctcaatcagaaatggagtaccccaacatgagcaagattaccgccacccgcatcgacaacgacgaacagcgcctcgaaatcctcccgaccttctttggcgcagacttcctccgggtcgaaatggccctgtacagccacctccagaagatgtgcgaggagtacaacggcgcgtactggtacatgtacaagctgtccaacggcgcgatgtacctggccccggcgattgagaaccggaagctgcgactgaccgtggacaccaatggctactcgggcgaggtcagcggggacgccgcgggcctgatcacctgtctgttcgtgttcaacgccctctgctggaagtacccccagcgcgaggacttcgtggacctgttctacaagctgcgtgacttcgccttcgaccacccggaggctgaggaaatcatcgccgccatcgactgaccaaccccctcggggcggatcggttccgccccgaacttcccagaaaaggagcaacaccatgaccaagaccacccccaagaccaacctcctggaggagaccatcaaccaaggtcgccaggacgtgaccgcccgccgcgtcctgtccctgggcgacttcaaggtgcgcctcacgatcaagtccgacagctacaagttccagtccttcgcccgggcggaagtctggaacccggcgaccctgagctggaaccaggtccactccatccactacgcggaaatggcgaccccggagggcctgtgctaccacccgaacaagtccggcctgaagatcacccacttcacccgcgacttcgaccgcctgctgacgatggtcaagcagatcatcctgtaaccttgtagaaaaggagcccgccatggccaacatgagctactgccgttgggagaacaccctcaacgacctccgcgactgcgcggaacacgtgaacgaccccctgggcggatcggaagcccgcgcccgggcgtccctcctcgaactcgccgcggacatgctggaggaggtcggggtgaccatcgaccgccgcgagctggacgaagccctgagcaacgccccgggaggtgaaggatgagcggacgctacaaggtcctggtcgggtcccaatccggccactgctgcttcgactacaccgtggtggacaccctcaagccccaccccgtgtatgcttcgcaaggtctgttcgatgcgatctgcgagacgttcagcgaggaggaagcccacgcggtcgcccgcgccctgaacgccgcgaccacgaaccaggcgaccctcgcccgggccgctcgcctgttcgaggaggccctgcccaagttcaactggggcgcgagcgccctggacgccaacgcgatccagctgctcaacgaggtcccgggcgaagtccgcgcggccctgaaggcttgcgccctgtgcggaggggaaggccacacggccccgaactgcccctgggcgaaggagggcggagcatgacccccgcaaaggctgacgccctgatccaggagttcatcgacctgggcgaacagatgaagcggctgaaggaccgccgggcgaagatcgcccaacagttcgccccgggacggacggaaggcgaccgcctggccctgtacgtcgccgggcggggctactcctcccgcttcgacgcggccctgctgcgccggtacgtgcccgccgccacgttggacctctgccgcgtgacgacctacaagaacggctccgcccgcgtggtgccgaagtcgaaaccaagacccaagaaggagaagcgcgcatgaagcggggaatctaccgcgtcccgatcccgcacctgatcggcaagaccgcgctgctgcgcgaggcgacccacggccatgtcgtggcgcagttcgatgactggagcctgacccggagcggcgacccgatcccagcggagaagcccgaaggcccgcccgcggacgccctgggctacggctggcacgccttcccggcggaggacttcgaggagaaccggacctgcccgacctgcgaggcgaccggctttcaacaaagcacgctgggtcccgaccgctgcaccttctgcgatgggacggaaggcgggaacccgccggaggaggacgcatgaacacgcccaacaccccgcccgaccgccgcgtgcggtccatgacctcctccgtgggcacgacccgcgacggctacctggtccgccaagtggttgtcgagtgcgaggacggcacgctgtggcgactctgcgacaacgaagccgggactgatcactgggtccggctcccggcgatcccggggaggtgagacgatggtgctggctgaaatcgagtcgcgcatcagcggcattccttgtataatcgccgtcacctactgggaaccctacgtgcccgcgaaggtgagcggaccccctgaacactgctacccggcggaaggcggatgcggtgaatgggaagtccgcgaccgccgcggacgccccgcgccctggctggagcgcaagatgacggaggcggaccgcgagcggattgaccaacaagtgttcgactacatggaggaccgctgatgaagcaacgcctgctcaagcgagcccaagaccgcatctgccgccgcctccgcgcccgcttcacgatggtgaagccggagccggtccaaggcatgttcaacttccgctgccacgagaactgcgtggagtacgtccgccgccacccggaggagaagctggccgtggtggagacgatctacattgacggcggcgagcccatcctacactacctggtccacgaccccgccgcgggccgctacctcgaagtgaccctgggctggcgggcggagcacctggaatactacgttgtcaggaccctacacccggacgatcaccaccacatcctcagcgagttccaacgctccctggacgattggacagaggagtacgtgggctggttcggtcggaaggtcctgggcatcacgagggtcctgtgatgaagcacctacacctcgaacgcctggaccaagcccttcaacacgccgtcgcggacggatgcgacccggcggacctcctcgcggaactcgccgcccgacacctgatgagcgatgaggcggacccggcccatgtcaacggcatcgccttcgcggaacggttcaacgccgccctcgcggcgaaggccggaggaggcgggacgtgacctgcatgcgcatcccgggcggcatcgtctgcctgtcgcccttcttccggctccgcctcgcggacggctcctgcgtgttcatggagtggcacaactactgcgggccaaccttcttccgcgaccgggcggcacgccgcatgattgacgagtggtgggacaaccccgcgatctgcgccgccctggactggttcatccaacgagggaagcgggcctgaccacccctcacgatcaatgccccgccgggcggcaatggtgccgacttcactacaggaggccgaaggctgcgggaaaaccggcggggctccctcctccttctccacttcgaccgggtgcgcttgggttacgggagtgcgcttgggttcggctccgaaaaagtatgaagcaaggcgtggcgggaagtcaagcccgtctggggttcccgcaccttgcgcttaggttacttgggattcttacctgaaataaattcgcccgacaaatcgacccggcggaccggcccaggagaatccttgttgaggctttctggtgtccgaagggctcccagggggttaaggtaagtaagttaagtaagttaagtatctatctatctatctatctataaagggctgttttatatggcctttttgcccgcttgactttttacttcttcggacgtggaagtgaagcgcgacccctcgaacctaagcggaggacgctgcctgcctgcttgggcaatccgctgccacacgctcctcgtgcctcccccgcgggcgagcgcgactcacccttggctaatgtacaagctcacgctatactcgcggcgaggatgtccttgggcgtgaggccggggacggatcgccgcgtgatgcgcgattgacgaacagtacacaccgaagggggagcgtgatgcacccgattgagaaactgaagccgaagccgatggtgcccttcacctcggaccgcaaggagcagtacctggagttgttccgcacgcatcccgacctgggtgggcggaagtacctgtgcgcggaggccgtgggcgtctccggctccaccatcgactatcatgtcaagaatgacccggagtttgcccaggctctggaggacgcccgccaagcgtggattgatgagcacctgttcagcgcggccctgaagcgggcgcgggacggcgtggagcgcccgatcatcggcgggaagttcaaggacgaaatcatcacctatgagcgggtgtacagcgattcgctgatggccatgatgctccgcgcccaccgtgcggagttcaaggacgggaaggacgcggccagcatgaccgcctcgggcaccggcggggtgctgatcgtcccgggggctccggccacgatcaacgactggcagaaccagtttggggacctcgcccgcgggaccgtgggccgtccgaccggggagggcagctgatgttcgcccagaccgaagtgagcaaggcggtcgccatcgccgcccgcccggactacccgattgagtggcgcgaggcggagcccggcgagctgcggggctactacgtggacccggagacggggaaggagtcggaggcgacctggtgcccgcagtacgggtcgcagctcgccttcctcatggcgcacccgatcttcgaggtgctgtatgaggggacgcgcggcccgggtaagaccgactgcctgctgatggacttcctccagcacgtggggaagggctacgggtcggagtggcgcggcatcttgttccgtcagacctacccccagctgtcggacgtgatcaacaaaaccaacaagtggttcaagcgcatcttcccgggggccaagtacaacaaggtggagcacaagtggaccttcccggacggcgaggagctgctgctgcgtcacatgaagtcgccggaggattattggaactaccacggccacgcatacccgtggattggctgggaagaactctgcaactgggccgatgacaagtgctacaccgtcatgatgtcctgctgccgctccacgaagccggggatgccccgctgctaccgggcgaccaccaacccctacggccccggccacaactgggtcaaggcccgcttccgcctcccccacatgcgcggtcgggtgatcctggacgcgatgcgagacggcgagcgcgaaccgccccgggtcgccattcacgggtccatctatgagaaccaaatcctgctccacgctgacccggagtacatcagcaagattcgagccgcggcccggaacccctccgaactcgccgcctggctccacggctcctgggacatcatcgcgggtgggatgtttgacgacatctaccgcggggacgtacacgtggtgccctccgtcccgttgtcggtgatcccgaagcggtggaagattgaccgcagcttcgactggggcagctccaagcccttcgccgtcctgtggtgggcggagtcgaatggggagccgttcgagtggaatggccgcgtgtacgggaaggtgcggggcgatctgtacctgatccaggagtggtacggctggaacggaacgcgcaacgagggcgtccgcatgctcgcctcggaggtcgcccaaggggtgaaggaccgggaggaggactgggcgctggaaggtcgggtcaagcccggccccgctgactcctccatcttcgacgtggagaacggcaacagcatcgccgtggacatggagaagaagggcgtgcgctggacgcccgcggacaagggcccaggctcgcgcaagcagggctgggagcaaatccgcaagctgctcaagggggcgttgcctccggcgggcgggggaccgcgcgaggtccctgggctgttcatcttcgactggtgtcagcagaccatcgagacggtccctgtgctgccccgcgatgacaaggacctggatgacgtgaacacggaggcggaggaccacattggtgacgcgatccgctaccgcgtgcgcaagaagctgcgtggcgtcaagcagggcaacatgtaatacaacttgccgggtcctcgccttcgggcgagaatccgcgaaccaggagaaccgaccatggccgacaaagacccaaagagccccgccacgaccagcggggcgtatgaccagatgctcccgcgctggcacgtcatcgagacgctgctgggcgggaccgaagcaatgcgcgaggcgggcgagacgtacctgccccgccaccaggaggagacggacacgggctatcaggagcgcctggcctccgccgtcctcctcaacatggtcgaacagacgctggacaccctgagcggcaagcccttcagcgagccgatcaagctcaacgaggacgtgcccaaggcgattgaggagacgatcctgcctgacgtggacctccaggggaacaacctggacgtgttcgcccgtcagtggttccgcgaaggcatggccaaggccctctgccacgtcctcatcgacatgccccgcccggccccgcgggaggacggccaaccccggaccctggcggatgaccgccgggagggcctgcgcccgtactgggtgatgatcaagccggagtgcctgctgttcgcccggtcggaggtgatcaacggggtcgaagtcctccagcacgtccgcatcatcgaacattacatggagcaggacggcttcgcggaggtctgcaagcgccgcatccgcgtcctggagccgggccttgtccagctctgggagccggtgaagaagtccaacgcccagaaggaggagtgggcgctggtggatgagtgggcgacggggttgaactacgtcccgctggtcaccttctacgcggaccgccaaggcttcatgatgggcaagcctccgctcctggacctggctcacctcaacgtggctcactggcagtccgcctccgaccaacgccacatcctcaccgtctcccgcttcccgatcctcgcctgctcgggggcgtccggggaggactcggacccggtggtggtcgggccgaacaaggtgctgtacaacccggacccgcaggggcggttctactacgtggagcacaccggccaagccatcgccgcgggccgcacggacctcaaggaccttgaggagcagatggcgggctatggcgcggagttcctgaagcgcaagaccggcgggcagacggcgaccgcccgggcgctggacagtgcggaggcgaccagcgacctgagcgcgatgactgggctgttcgaggacgccctggcccaggccctggacatcaccgcggactggctccgcctcgggccgaacggcggcaccgtggagctggtgaaggactatgacctggaggaaatggacgccccgggccttcaggccctccaagtcgcacgcgagaagcgcgacatcagccgcaagacctacctgaacggcctccgcctgcgcggggtcctcccggaggacttcgatgaggatgaggactgggaggagctgatggaggaaatcagcgaggcgatgggccgcgctggcttggacctggacccggcccagaagaacccgcccgaaggtggggagggtgagggtgagggcgaaggcgaaggcgagggcggcgaaggcggagaaggcggtggaaatccgggaggcgagtcatgaacgtctggcacttcttggggctttggctcctcctgagcatcgtcctcgccccgttgatcgggcgttgtatccacttcggcatgaacggacccaaagaaatggagaagcgggatgcccacattcaatgaggagtaccgggacgccgcgctgcgtcaccaaatcgacctgcgccgctacaccgcgggcgtcaccaagcgggtcgcccggctcctggaggaggcggaccgcgacctgaccgaacgcctgcgcacccggctcgcccgcttcgagggccgtgacctggacttcaccggcgaacgctggaaggccctgctcacggacatccgcggagcccgggccgcggccctcgcggagtacaagaccctggtgcgggacgaactcgggcagctcgccgtcctcgaaggccaggccgaaatcgacctgctgcagtcctccatcacgattgaggtgggcttcatggcggtgaacgcggaccagctccgggccatcgccacctcccgcccgttccagggccggttcctccgggactggttcagcaccctggaggcggtggaccagcagcggctgaccacggctcttcagctcgggatgacgaacggggagcccattgacgacatcgtgcggcgggtggtcgggacgcgcaagaacgcctatgcggacggcatcctgtcgatgacccggcgggacgcccaggggatcgtccgcaccgcggtgaaccacgtgtccaacaccgcgcggggctacgtctgggacgccaacagcgacatcatcacggcgaaggtctgggtgagcacgctggacggtcggaccacggctgtatgccgcgcccgggacggccacgggagccccgtgggcgacaatgagctgcccgcggacatccccctgctccagcccaaggacgcgaagcccccggcccacttcaactgccggtcggtgatggtcgcctacatcgacggcgtgggccttctgggcaatcgcccgaccgtgacggacacccggacccgcgccaagcgtgaaatcgacttccgccggatggcgaaggagcagggcaagccgatccaggacatcaggaaggcttgggccgcggagaacgtgggccgggttccggcggcgaccacatatcaggacttcttgaagcgccagcccgcctccttccaggatgaggtcctgggcaagaccaaggccaagctgttccgggaaggcgggctgaacgtggatcaatttgtggatcgggccggcaacgagctgaccctgtcccaactcgcggagcgcaagccggacgccttccgcaaggctggccttgaccctgaaaagttctgaggctacaatatgaaccgtgcgtgaggcacaacactggcgggtgatccgccgacaatgaggatacaattatggactttgaattcactccggtcgattccatcgacaaggtcccggaacagttccggggaatctacaagcagggcgatgatggcaagttcgtcccggacgaagcccacaaggggatcgtggaggccgtgactggcctgaaccgctccctcaaggctgctcgtgcggaggcgaaggccaagacctccgtggacctgaccccgctggctgacttcggtgcgacgccggaggaaatcaaggccaacatcaccgcgaagctgaccgaactccagaatgaactggccaagggcggcgaagccaagctgaacctggacaaggttcgccaggagctggccgatgcgcacgcgaaggacctgaagaaggccggagcccgcgccgaagccctccagaaccagctgtatgggctcctggtcgagaacgccgccactgccgccgttgcggagctgaagggcgtcccggaactcctgctgccattcatcaagaaccaggtcaaggtggtcgagcaggacggcgaattcaaggtgttcgtggtcgatgcccagggtgaccagcgttactcgggcgtgaccggccagcccatgaccatccgcgagctggtcagcgaaatgaaggccaacgagaagtatggccgcctgttcgagtcggaagccccggcgggcggcggcatgcctccgcgtggtggtcagacgcctccgcgccagcagggcaaggtcctgaccgccaacgaaaagatcgcccagggcctcgccaagggtcagttcaaggcgggccgcggtcgggcgtgacggatcggggaggcccccaagtttggccagggggcttcccttttccgcaacttggtactatactgacgtcacttttggttgtatagccagaggcgaaggcccacaggagtgattccgcgggccgcgacggaacaccgggtgatccggcacggctgaaaaccgcttgagtcatcaacttccgaaggagggccaatcatggcttctgttacccttgccgaaagcgccaagctggcccaggacgaactggttgctggcgtgatcgaaaacatcatcaccgtcaaccgcatgttcgacgtgctgcccttcgactccatcgaaggcaacagcctcgcgtacaaccgcgagaacgtccttggcgacgtcatcatggccggtgtcggcacgaccttctccggcgcgggtgctggtaaggccgctgcgaccttcaccaaggtcaactccaacctcaccaccatcatgggtgacgccgaagtgaacggcctgatccaggctacccgctccggcgacggcaacgaccagaccgctgtccagatcgcctccaaggcgaagtccgctggccgcaagtaccaggaccagctgatcaacggcaacggcgcgggcaacgagttcgcgggcctgatccagctctgcgcctcgggccagaaggccacgaccggcgcgaccggctccgccatcagcttcgccatcctggatgagctgatggacctcgtggtggacaaggacggccaggtggactacatcaccatgcatgcgcgtaccctgcgcagctacaaggcgctgctccgcgccctgggtggtgcgtccatcaacgaggttgtcgagctgcccagcggcgcggaggtcccggcctactcgggcaccccgatcttccgcaacgactacatcccgaccaaccagaccaagggcggcaccactggttgcaccaccatcttcgcgggtacgctggatgatggttcgcgcacccacggcatcgccggtctgaccgcgacccaggccgcgggcatccaggttgtggacgtgggcgagtcggaggactctgacgaacacatctggcgcgtcaagtggtactgcggcctggcgctgttcagcgagaagggcctggcctgcgctgacggcatcaccaactaaggcggcacccgccctccggggagggctctgccccgtagtacccgaagggcgggccggtctgagactggtccgcccttttgttttgaacgcactcaggagacgctatcatgcccgcttaccttgtaaccttggaccggaacaagtccggccacacccttgtccatggcgctgacgccatggttgtgttcgccgcctccgctactgccgccaagcaagctgccgcggcgaagtacgaaggcgacggcctggcctggctgaacgattcgaccgccaccgaaatcgttgccggcaccgactggtccggctggaccttccgcgtggcgatcctcggaggcttcggcaccggcggagacgaaccgcgcaccgtcgctgtcgtgggcgatgcgaccgacaacaccgtggacgaaatcgccgcggccctcgtggtggcgctgaacgccctggacgggatcgccaacgccgcctacaacgcgaccacgaacacgctgaccgtcgccgcggctgcggacgccctgggcgaccagaagctggaagtgtcgatcatccccccgggcggttcggcctccatcgcctccctcgtgggcacgatcacggatggcggagttgccgctgccgacctgaccgtggtgctcccggcggacaacgccgtgatcccgaacgtcctggcccccgtcgcccaggtctaacaccaaccccggagaactgtacaaatgtccaccatcatccaaacaacctttgtcctgaccggacccctggcgggccgcacgatccgcctgggcagtcagccctacccgttcgacaagggccgcttgaccatcaccgctccggcggaggaggtcgccctgcacgcccgcttcctcgaacgcaactggcaggcttacccggaaggacacccggccctgaaggaggtgcccgatggccagcgtgatcttcaagaaggcccccagccggacggccaacagccggtacacggcgacgttcagcccaacggggacgggactgaagccggtgacgcggcacctgtcagcggcggaggtgtcgaagccgaagccgggcaagccgggggtgtacccgatggggacggacaaccggaggtcctgaccgatccggcgaaggagccgaccctggagctgaacaccaagctccagaaggcggtcctgggcctggacccggcggatgacactcactggaccaaggacggaaagcccgcgatgaccgccgtggagaagctgtatggctccgccggcatcacccgcgctgacgtggaagccgtcgccccgggccatacccgcgacaaggcgaaggccgctcagtaacccaaccaactccgaaggagaagcatcatggcgaaatccggcaccaccaaggcaaccgcctcgaagatggtcaatgcctcgaagtctggcgtgcgtcacggccagaactcgaagaacgtggtcatgggcggcaagtccgctccggctccgtccggccccaccgccccgatcaagggcatggacaagggcggggtctgacccgtgttcggcttcccctcctccaaggtctgggctgcggcgggcgtcttgctcgccgtcgccttgatcgccctcgcgggctacggctacggctacggctccgggaaggcggacgcgaccgcggaggcggcggaggccatggacaaatacaaggaggaggtccgcgcccgggaacgggagcaggaacgcctcctggctgaggccaacgacaagaaccgtgaacaggagaaagcccatgaacagcgtgtcgcagacctccgggcggagttcgcccaacagcaagcggacgcccgggcgcgggatgagcgcactattgctgatctgcggtctggcaatcagcggctgcgcctccaagtctcctcttgtggtgcggcccgatccggtgcggctgagtccgcccccggcggagctgatggagccggaacagccgaacttgcgccagagacttcagcagctctctggggaatcgccgcagacggcgaccgggccatcaggaaactgaccgcccttcaggcttgggcgcggtccgccgtccagctgtgtaccctaccgcaaccggagaaccaacaatgaacatcgccgtcacccgcttcctcgcccgactgcgcaagcgcctcgcccccttcctggacctcacggcctgggtcctgctcatcgccagcatcgtcccgttgctgctgatcgacccggccatggtcgtgaccctcgcgcagtggacagcgtttgccctcgcgctggcggggatcaccgttgtgatcacccgtgtggtactaccccaggtgaacctatcggaatggctcgcgcgtgcccgggagggctccgtggccgggggcctcgtggtcctcgccgtcgccctgactatctgcttcaccttcttgggattggtgctatgggcaaaagcctgattcacttcgccttcgcggtcctctgctgggccttcggctccgtcgccctcgcccaggacgcccgcaccttcgtcccttcgggggcgaaggtgtacgcgccagtgctagtcgagaagcagcgggaggtctggccgcaagccccggagccctggaccctcgccggtctggtggagcaggaaagctgtatcagcctgactcactcccgctgctggaacccgcgggcggagctgcgcacccctcgtgaatacggcttcggcttcggtcaggtcacggtcgcctatcgcccggacggctccgaacgcatgaacgtgttcaacgaactgcgcaacacccacgcctccctccgcgactggacctgggagaaccgctatgacccgggcttccagctcacggccatcgtggaaatgaaccggagcctgtggcggaggatcgccgcgaacccgggcgcgacggtcacggaccagtgggccttcgtcctgtccagctacaacggcggggcggcgggcgtcctacaggatcgccgcctgtgctcgaacacccgcggatgcgacccggcccgttggtttgggcacgtagaacgcaccagcctcaagtcccgcgtccctcagcccgggtatgggaaccggagctggtatgagatcaaccggagccacgtgcggaacgtcctgacgatccgccgggccaaatatcaagccttctggaggacgtgatggccttgatcgtccaagacaacacgggagccgtcgccggggcgaacgcctacatcagcgtggaggagttcaagacctaccacaccgaccggggcaactccttcgcgggctccacggacccccagattgaggccgcgatcatccgcgcgaccgactacctggaccagcggttcaacttcgtgggcaagaagcggctgggccgcgaccagaccacggaatggccccggacggacgcctgggaccgtgaccgctactacatcaacgacatcccgccggaggtgaaggaagcctgctgtgagtacgccttgcgcgccctcgccgcggagctgaaccccgacccggagcggaacgcctcgggcgtggcggtcctgtcgaagtcggaagcggtcggacccatcagcgagtccgtcaccttcgtgggcggggccgtgttccagctgcccaaatacccggcggcggaccagaagctggtccgcgcgggccttgtccgctccggcggtacgttgctgcgggggtgatccatggcacggtttgactccgctatcgctctggccaagaagctgatcaagaagaacggccaggccgtgaccctccggggcttcaccgccggggccgctcccgatccgacgaagccgtggaagccgggcggcaacgtcgcggcggaccagcccattgaggcggtgttcctggactatgagcaacgctacatcgacggccagacgatccgcatgggcgaccagcgcgtgttcatgcctgcggagggtctggcggctccgccggaggtcgaaggcttggtgctgcggggcctggaggtctggaaggtcatcgccgtgaaaccgctgaacccgaacgggcaagcgatcatgtatgaattgcaggtgcgccaatgaccctcccgacctttgacagcgcccgcgacgaaatccttgggctgttcaacacgaagtggaccacggacaccccggccctcaacggcggggctccgatccgcgtggaatggcccggggtggacgcgggcgaccctccgcccgcggacaagccctatgcccgaatcacgttgcgtcacactatttcgcggcaggcgaccttcggaccaaccggcggtcgccgctttacccgtcccggactgatcacggtacaagttttcacaccgctgtccgggggacaaggcttgtctcttgctgaaaaatgcgcgataatcgcccgggacgccttcgaggggcgaggcaccgcgagcggcatttggttccgcaacgcacgcatccaggagattggcccggacggcgcgtggtatcagatgaacgtggtggtggagttcgagtatgacgaactgcgatgaaccccttgccacttgaattgaggagttacaaccatggctaacaagattgactcgaacgtcaccggcctccgctatgcggaggaggacacgatcaagaacctgcccgtgtcgccggtgtggtatccgctggagcccaacggctacaatgactttggtggtcagctgaccacggtcgcccggaaccccatcaacccgtcccgccagcgcaagaagggcgtgaccacggacctggacgcctcgggcggtttcggtcaggacctgacccagaacaacctgacccgcctgcttcagggcttcttcttcgcggacatccgcgagaaggccagcaacatcccgaccaacggaaccgccgtgcccttctccggcgtgacgggcaccagcaagacctacaccctgggctctggcacggtggggtcgcagttcctcgccggtgatctggtcctcgcctcgggcttcaaccaggcctcgaacaacggcttgaagaacgtcgccagctccaccgccgtgaccgtggtggtgactcaaaccgcagtggacgagacgcccccggcgaccgcgaagctgatcaaggtcggtttccagttcggctccgctgaaatgaacatcgacgtgtcgggcagctatccgcgcctggtccgcggctcgggcacgaaggacctgacgaccctgggcctgatcccgggcgagtgggtgttcatcggcggggacgcgacggctaccaaattcaccaacgccgccaacaacggcttcgcccgcgtccgggcggtcgctgccgcctacatcgagtttgacaagaccgccggcaccatggtggctgagacgggcacgggcaagaccatccggctgttctacggcaacgtgatcaagaacgagcgggacgcgaacctgatcaagcgccgcacctaccagctcgaacgtaccctgggccaggacgcgaacggcaccatgtcggagtacctggtgggagcggtcccgaatgaactgagcctccagattcgccaggccgacaaggtcacggttgatctgagcttcgtggcgaccgacaacgaacagcgcgacggctccgcgggcgtgaagtcgggcacccgtcccgacctcgtggatgcaccggccttcaacacctcctcggacttcagccggatcaagatgcacctgctgaccgcgggcaactcgaaccccactgcgctgttcgccttcctgacggagctgacgctgacgatcaacaacaacgtctcgcccaacaaggcggtcgctgtcctcggggccttcgacgtttccgcgggcaccttccaggtgtcgggcaacgtcacggcctacttcgcggacatcgcggcagtccaggcggtgcgcaacaactcggacgtgacgctggacttcgccttggtgaagaacaacgccggtctggtgtgggacatcccgctgctcgccctgggcgacggacgcctgaacgtggagcaggaccagccgatcaccctgcccctgtcggtggacgcggcggaaagcgcggcgggttacaccctgctgctcaatgaattcccttaccttccgaacgcggctgacgtataatcaacggagcccggggagggctccggccctcccttccctcaccctacgtggagaaacagagaatgagcctgtacaaactgttcaagaccaacgagaacctggaaacggacggcatctggctggagtacggccaaacggcggacggcaagccgattcgcatcaagatcgcgcgtgccgggggccacaacgtcgccttctcgaaggcgctggagaaggccacccgcccgtacaagaaggccatccagaccgggatgctggacaacaagaccgcggaccgcctgtacaaggaagtgttcgcggagacggtggtgctggattggatcaacgtggaaggcccggacggccagccgatggacttcaacaaggagaacgtcctgaagctgttcgaggacctgccggacctgttcgtggacctccgcgagcagtccgccaacgtggcgctgttccgcgatgaggtacgggagacggacctgggaaactctgggaagtcctctgctacggcttcgagcaaggcccagtagagcagaagatcatcgagcagtgtatgcggttcgggatgcccttgcccgaccgcatacagaacgccccggagttgacccttggttcggagctgtactacatcggatttttggacctgacgtcatgtaggcaaatcggcacgggcctgggacctatcccattgttggccatactggagtattgtatgatcaacgggatcgagggcgagcagcaggaggactttgtttggttcatccagcgacttgaccagaagtatctacagtggagcgcagcccgtgccaagtctaagtgagttcagccgacgcattaccctccggggccgaaaggtcgcggagggcgctgacgcgctcactcgcaaggtcgccctcgccgcggatcaagccgtggtgtctgggacgcccgtggacacgggccgcgcccgatccaactggatcgccgcgattggctccgccccctcctccgtgattgatgcttactcgcccggcgaggcgggcagcactgaagccgccaacactcaggccgcaatcgaccaagctgaatcggtcattcgcgggtacaattacggggaggagattcacatcaccaacaacctcccgtacatccaacgactgaatgacgggtattccgcccaagccccggcgaacttcgtggaacaggcggtgctcgaagccgtccaggttgtacagttcggaagggttgttgacggggacccggggagctgacggtggccgaagaacgcattgacatagtcatcactgaacgaggttcgcgtgtcgttcagcgaaacctggaggacatcggcaagtccgggcgaggagccgcgggcggggtggacttcctcaagaacgccctggcctccctgggcgcgtacctgtctgcgcgcgaactcgtgcgcctgctggacacctacaccaacctccagaaccgactccgggcgacgggccttgaagcccagaacctcggggcggtgtatcggtcgctgcttgacgtctcgaactccacccgccagtccctggagggtacggtggagacgtacagccgactggccaacagcgcgaaggacctgggcctgtcgcagcaggagctgatcgacttcacgaagtcgctgaaccaagccatcgccctgtccggcgcgagcgcgggcgaggctcaagctggtatgatccagctggcccagggcctcgcctcgggcgtcctccgcggcgatgaactgaactccgtcctggagcagctgccgaccgtcgcagacgtgatcgccaagcagctgaacgtgacccgcggcgaactccggcagatgggtcaggatggcaaaatcagcgctgacatcatcttcgacgccttcaagaacgcccggacggagctggaggaacggtttgccaagtccgtccccaccatcggccagtccttccaagtccttcagaacaacgtggtggacctggttggtaagttcgatgaggcgaccggcgcgagcgagctgctgtccaaggcgatcatgttcatcagcaataacctggacaccatcgccaaggtcctcctgtcggtgggcgcgggcttcgctatcgtcgccgggggcgcggctgcgttcaacgcggtccgcaccgcggtgatcgccctcaacgcggccatcgccgcgaaccccttgggcgcattcctgatcgtcctcacctccgtgatcaccgccctgaccctgttccgggacgaaatcaagctggggattgacgacacgaccactctgggcgatctgatgcgcgccgcctgggaggacattggcccgatcgtcaccggcctcgccaatacggtcggggagttcttcaactggctgaccggctccgcggcgacggcctatgagaacatgaccgaccaggccggggccagcgtacagaaccaggaagcctggtggttgaagctggtccgcaccgtcctccaggtgttcgacatgattggcgggacgatccggggcgtgatgcgcggggtcctcaatgtcgtgggctccgtcatcgacgccctcatgaacaacttccgccagctcgggaacgccctgaaggccgcagtggaccttgatgtggacggactgaaggccgcggtgaccagcaacctcgaaggttggaaggccgtgggcgccaacatcgggacgaactttgaggaaggattccgccaggaagtcctcgcccaatccgaaagcgggctggaggcgatgctggacagctggatcgaacgcgcccgcgacatttccaaggagcgggtcgccgcggctcaagtcgagacgccgaatctgggtggtgggggcggtcgccggacctccgggaaaggcgatgaggaggcggccaaggccctcaagaaacttcaggacgaactcaaccaactggtcgggtcctatgaccgtgtctgggcggctcagcaggagtacgccaacgccctcgccttgctcgacaaagcggagcgcgcgggcctgatcaccgcggagcgcaaggcccaggtcctggcgctgatcgaggagcagctgaaggacgccctggacccgatgggcgcgatcaaccgccagctggaggaggagcgcgagctgctgcgcctcacctcggagcagcgcgaggtcgaacagcagttgcgctacatcgaacaggacctgcgctatcagggcatcatcctcggggaccaggagctgaagcagctccgcgagaagctgaccctgattcaggcggaaacccgggcggcggaaacccgcaaccaggtccttcaggctatcctcggaccccagcaggagttcaccgcccagctcacggcgatcaatgagttgctggccgcgggggcgatcacgcaggcccaggcaaaccagttcctggtggagtccaacgcggaccttctcgcgggtacggtcgaagcccagcaggcgatgttgtcgcagtatgagcagatgtacgcgcggattgatgagatgcggcaagccgacctcatcagcgagcagaccgcccagcaattgaaggctcgggtccaggcacagatcactgagcagaacctgtccacccagcgcaacttcttctccaccctgtccgggctgtcccggtcggagaacaagaagctggcggccatcggtaaggccgcggctatcaccaccgcgaccatcgacggcgtgctggcggttcagaaggccctcgcctccgctccgcccccggccaactacgccctcgcggcggcgaccggcgcggtggcggcggcgaacgtcgcccagatcatcgcccagacgccgggctttgccttcggcggcgacttcaccgtgggcgggacgggcgggacggactcgcagctggtcgccttccgtgctacgcctggcgaacaggtgtctgtccgtactccgacccaggagcgggacgaagcgcgtcagggcggtggcgaggggcagcagggcggtgggtccgcgatccgggttgtgaacgtgatcgacccgaacctgatgcaggactacctgaccagctcctcgggcgagcgggtcctgctgaacgtaattcaacgcaacgctggcgcggtccgccaggttgtgaacaacggctgaggatgagacatggcacacgaaatcggaaccgcgacgaactttgaggacttcttcagcaagatcgtcgcctttcttaccacggacgcgaccctggtggcggcaggtcaggcttggcaggcgctgcgcgtccgccgggacaacatcgacacgtacaccaccagcctcccggactccttcacgggtaacggtcggaaacaaatccacacattccgctatgatccgcggtcgcttaacataaacaaccccgcccagaacggttcggagtccttctggtacaccaactcgggcttctccgccgggagcagctacggtcaatggaaactgcgacaggcgcgcgaagtcaagaccgtgcgcatcaaggcccccatcgggaccagctacgcgagctatgcccccaagtccttccggctccaatactcggatgacggaaccgcttggactacggccctgaccgtctcgaacgcgccgaactggtccgccggggagcagcgggacttcgccgtgcctggcacccccggttcgcacctgtattggaagatcatttgggacgctacccaggtggtgagctacatagggtggcaggaactcctcctgctcgaagcggacgggacggtggccaaccactttgggtcggaggtcatcctaaaggccctgggcaactcgggtctggatgaaatctacaccggcatccgggcggagtatgacagcgccgcaggctggtacaacctgttcatgaacgggtacactggctatgacgccaacgaaatgtcttggtttaaccaaccgggagccctcccgggatacggggcgcaatacactcgggcaaccccgatggtgccgctgtggaacaccaccatgccgtactggatggtggcttcgggccgctccttccggttctgcgtcaaggtcggtacgaactatgaggggggctatcttggtttcattctcccgtatgctacgcccaatcaatacccgtacccgctcgctgtcggtggttccctctgccccgtcaacgacagctcccggtccgcggagtggcgttattcatacgtgagcttcgcccacggcgtgtatcccgggccgggcactcagaactacccggaaagcgaagcgaactgggcgaccctttacctgcgcagcccggaaggagcctggaactaccacggcaaccgttctgcttacgcttcgtccaacagcgagggcgtagggggtccgaccgttagcagctcgcctccctacaacgtcgtcattaacaacgccggtttgcgcaacgtctggcctcactgcatgaacggccagtggtcctcgggccttcgcccctaccgcgagtgcttgggcggcgggtatattctccagccttgcgtgctgattcagcggtcgcctgcccaagtcctcggggagctggaggggacgtttgcaatcagcggctaccaaaacagcgcggagaacacgaccgtgttcaacggcaagactcacgtggtgttccagaatgcttaccgcaacacgatccacgagcactgggcgctgtcgatggattgagggagaactgaatcatggcttatgaaactgggtccgcgaccggaccgaacgacatgttgatcaagctgcgcgacttcgccgcggcccagggttggaccgtgaaccgggacgcggcggcgggctccgggcgcgagttgtgtctgagcaagggggcgtcctacgtcaatttgcgcagctaccagaacgaaacgatcatcatcaacggctcctccacctccgggcgatacgggatcgccatcaacggttcggacggctacagcgccggggcgacttgggaccgccagcccggctatccgctgtgcacttcgtcctcgggcggggaccaggcgcatgccaatcttccgctgcccatctacttcgggccgtttccgtcataccacttgtttgcgccggacagcaagaccatctacctggagctggaggtggcatccactatcttccagcgtctgggtttcggagccctggacttgtttaactccgcggccccgggcggggggcggttcttctacgccaccgggggctcgcacccggcaactactaccggaagcgccacttggctgggatcggacgtggagaactggagctattctctggaggaggtccccttcagggcggcagattacacgacctcctcaagtaccctttccgggtccttcctccgggcgcagttcgactccttcaacaactggtgtcactcctcgcgcagcccgaccaacacccaaaccggacaggcttgccaaggtggggcgattcacgataaagtattgatgtcgatgtctcccaaccccctgaacggggtcgggattctcctgcctcagatcgtgtctgtcaaccgcaacgaggagtacctgaacccggtcggagtcatgcctggtctgcgctatatggacatgaccctgtaccagccgggggaggagttcacgctggggtcggagacgtggaaagtgtttccgtggtaccagaagggcgggcggtccgtccaacggggaatcgcatacaagaaggtgacttgatatggcagtgatcaccacgcaagccttcgtggggctggataccctgcgagccccgacccctgattgggcggtcgggctggattcctatgcgtgggacgatcaaagcccgcccggaaagccatgggagcgaaccgcggacggcttcggctccgtccagaacaacctccccatcagcgaagccggggaggtttcgacgggctggcgcatgccgacctttctggacgactactacaaccgcatccatatccgcccctcgaacatcaacgtgggcaacctcgtgagtgagcagcagttcgcaatcgaggtgtggaacggctttttcaacagccgacaactccagaatatccaagttcagaacggcggcggtatttcccttgtgggggccgtcccgcccgcgacttgggcagctctggagaccaagacctatcagctgaccgtcaccacggacggaccacccgacatcaacgccatcttccattttgattgggatgggacggctgatgacggcgacctccgcgtgctgggctcgcgtatcgtcgccttgccgtacatcttcgaggcccccgccaaggaggtcctggagtggaaaacggacgtgctcacgaccaatgacgggtcggagcagcgggtgcgcctgcgcaagaagccccgccagtccttcaacgtcacctatccgatcccgtaccgggaaatggcccgggcggagaacctggtgtatggttggttgactcgccgttgggccgtcgccctctggtctgaggcccaacaggtcggaaccctgctggcgggcacgaccgtgatcaacatcgacacgaccgcctccgactaccgggacggcgcgctgatcatgatctgggagtccaaccgcaagagcgcgaccgctgacgtggggatcgtttccgccggggctttgacgctgaaccgaccgctggccgaaaccttcaacaacccctggatcgtgcccgtgcgccttgggcggatcgtcggcaacgtctcgcgggcaacctcgggctacaacggttcactggaaatgacctatgagttcagcgacaacatcgacctggacccgcccgcggctcccacgcagttcctcggatatgatgtgtattttgacgaggctctgaagaatggcgaggcgctgacggacagccttcaagcccgggttgatgtcgtggactacgggaccgcggcgggggccagcttctattcgccctggacctacacgcgaattggacgcccctacaagttcttgctacagggactccaggacatctggaacttccgcaagttccttcaccggcgtgcgggacgcctgcgcccgttctgggtcccaaccttcgagaacaacatgcgtgtcgcccagaccggcgagctgacccagagcatcgaggtgtatgctgacgactaccgcgaatttgcgccggagcgcactcacatcggcatcctcctggatgacggaacgtggttgctgcggacgatcaacgcggcgacggcctccgggacggacacggcggtgatcggtctggacgccccgatcaacatcaacgccaatcgcatccgccaaatcagcttcctgggcctgaagcgcctggacgcggatcgggtagaacttcagtggaactccaaccgggtccttgaatgtacggtccgcatgatggagattcaaccatgacgtatgacgcacgcgagcgaagcctgtttgaagcctacccggtcgagctgtacctgttcgcccggggcgcgcaatactggcgctacacctcagcggatgaagacaaggtggtggacggagtgacttacaactccgtccagatcaagcgcggggccttcgagcagaaccaggaaatgtcccggagcaacctgacgctgacgatggataagggcatcagcttccttaaccaattccgcggatcgccgcccaccgacatcgtccaactcaccattcagcggtatcacgagggtgacggacagctcgccgtcccgtgggtcgggcgagtggtgaacgtcaaattcacggagcgcgaggcggaggtgcgccttgagccggtatacacctccctgcgccgcccgaccctgcgccggatgtaccaaacaacttgtccccacgtcctgtacggggccgcgtgcggcctgtcctccgcgaacttccgggtggacgcgaccctcacgggcgtctcggggcgggacctcctgtcaccggccttctcctccttcgctgacggctacttcgccgggggctacgtggattgggaagtggccggggtcctggaacggcggttcatcgtcgcgcacgtggggcaggcgatcaccctcaatcttccgttggccggaatacccgccaacgcgacggtccgggcctatcccgggtgcgaccacaccttgaatacgtgtcacaacaagttcagtaacgtggacaactacgggggtcagccgttctacccgaagaagaacccgatgaacggcaccccgatcttttgaggaggaccccatcatggagtgggctgtatatctgatcatcttcatcgtcgcggcatacgcggcggtggccctcgccccgaagcaggccacccccaaacccgcttcgttggaggacttccaattcccaaccgcggagcccgggcgaccgatcccggttgtgttcgggaccgttaccgtgaagagcccgaacgtggtatggtacggggacttggccagcagtcccgtcaaaacggctggtggcaagtgatgaacaacgagccagtgatggtccgggtcgaacacgcccgcgccttgggctactgctcccgcggcatgcgcgccttcgccgcccgacacgggctggattggggccgcttcgtccacgagggcatcccggcggaggagctggaggcgaccggcgatcacatggcgctacaagtagtggagaaggcccgtgggcagcaaatctagtgtaacaattgggtacaagtattaccttggcgcccacctcgtgatctgtcacgggccggtcgattccgtccaggaaattgtcgtgggcgaccgaaccgcctggagcgggaacgtgactgcctcacagcaaatctacgtcaacaacccggagttgttcggtggcgagaagaaggaggggggtgtccagggttacgtggacatcatgatgggggaatcgaatcagggccgcaacagttacctccagtccaaactcggcacggtcatacccgctttccggggcgtcctgtccctggtccttcggaaggtgtacatgtgcgccatgtcgccctatccgaaggcttgggcgctgaaggtgaagcgcctcccgggcaaggcttggtacccggagaaggcggacatcaacggctccgcgaaccctgcccacgtcatctatgagacgctgacgaacccggactgggggatgggatacccgatcaacgccctggatgacgccgcctttcgcgctgcggcggacacccttcacgcggaaggcttgggcgtgtcgatgatcatgaccaagcaggactccatcgagtccttcatatacacggtgctgggccactgtaatggaatgctgtacacgcgacccgacaatggtcaattcgtggtgaagctgatccgcgaggactacgtggtggcggacctcccgctgttcaacgagtccaacacgatccggctggagtccttcgagcgcccgggctacgcggaaattgttaatgagatcgtggtgacctaccgcccgcaaggctccactgaggacgattccgtgaccgtccaggacctcgcggcgattcaagcacagcagggggtggtgagtcagacggtgaactatccggggattgacaccgcggcgaacgcggcgaagctggccatgcgcgacctccgccagaagtccaccccgttcgcgcgcatccgcatccgggtgaaccggaacgcatggaacctgaccctgggggacgtgttccgcttctcctgggatgagcacaacctcgtggacatcgtgttccgcgtcctcggggtgaactacggggagctgaccagcggcgaaatcgtggtggacgcggttgaggacatgtttggccttccgtcctccacctacatgggcaaccagggctcgggatgggtggacccggttcaagcgcccaacccgttcgccctccgccgtctggaggaggcgaactattgggacttggcgaacggtctgccctcgggcgacttccaggcgctggacaacacctccgccttcctgatcggcctgatgggcgagcccgcccagtacctccagaactatgaactgtggacgaagcccacgggcgggtcctacgcatacgcggccaccggcgaccccgcggcgcacgctacgctgacgaacgcgatcacgcccatacagacctccatccagctgtccaatctgtcctcccgcaccgaatttgcgcggacggggacctatgcgctgattgacaacgaaatcgtgcgcgtggacactatcgacctggtgaacgggatcgtgacggtgggtcgggggtgcttggataccgtctgcgcggaacacgcagccggggcgcggttttggttcgcggaggacgcccgcgtgcgcgaccgtcttgagtacaacagcggcgagaccatcgccgcgaagggcctgggccggtccggggtcggcattctggacctgtccgttgcgccggaggactcgaaggcactggtgggccgtttcgcacgcccctacgctcccgggaacttccgggtgaacagtctccagtatccttcggctatcctcggaggtctgagcctatcttgggcgcaccgcgaccggacccagcaggtggtccgtccgatcatcgaccactccgcggcgaacatcggcccggagccgggggtgacctaccgcgtggacatctacgcggccaacggcagcacgctcctgaagtcggagccgggcctgaccggcactagctggacctggaccaacgaggcgacggagaacaccgcgggccggaaccggatcaaggtcacggcggtccgcgacggcctggacagctaccaatcccacgattggtatgtggatcgggccggactcgggaacaatcttggaaattatcttggaggtttgtgatggctatcagtaacggcccgaacttgggcatcatggtgaacggcgcgctgggggaccagcactacaaccaattcatgtctttcctccgggcggtggacggccttctcatgggccacgcgaagtccgcgaccacgaccgcccaaccggcttcgcccgcggacggggacgtgtacgtgctcccggcgagcccgaccggcacgaactggtctggtcagggccaacggatcgcgcgctattcgagcgcggcgacggcctgggagttcttcgtgccgaagaaggggtggaccatttccgtggaggataccaacagcacctactggtatgacggcagcgcgtggaagttcctccgcggctacggcacgaccgcgaaccgcccggcggcgagcgccgccctgatcgggggccaatacttcgacaccaccctgggcaagccgatatggtccacgggctccgcctgggtggacgcgactgggttggccgtctaaaatttgccaagttgtcttgggtcccgtagaatacggcccaagatcatcttggtgcgaggaccccgatatgcccctgaccccggagcaagtcgaagacatcgccgttgcggctgcgacccgggcggcgaaactatccgtggaggacgcggcgaagcgagccgcggaaacggttgccatgtctcactcggagctgaacgacgtagtggccgaagcggtcaagcagacgttgatgcagctcggggtggacacgtccgacccgttcgccatgcagagggacttccaacacctccgccagtggcgcgagtccggggaggacctgaagcggaaggggaccgttgccctgctgggcatcttcttctccggtctggtctccctgatcctcctgggcctcaaggagtggttccaaaaatgagaatgcgcttgggctacttaccttcacacctgaagaagtatagaccccaagcgccatcgaaagcccagcgccgtaacagctccgaccctcctgcgcttaggttacttcactttctccagttcagttctacttcgcccgataaatcgcccggaccccctgcccagggaggcgaccggcgaccgttcctgctgttcggaggccgtccgggggtttaaggtaagtaagttaagtaagttaagaagaagaagaagaagaatatataaacccccagccccgctgggcttccctgcttactccacttcatacttcttcagcacacgaagtcgagcgttgggcccccgtcccaagcgcacatgattctccgctcgccttcgccgcccagctgggctatacttccgggcatcactatgagaaatggagccaccctatggaataccccttcaagaccgaacccttcaaccaccagcgtgaggagtggttgcgctcccgcgaagaagaagcccgcgcgatcttctgggaacagggcaccggcaagtccaagctgaccatcgacaccgcctgctggctctggctccgcgggctcatcgacggcgtgctggtggtcgccccgaacggcgtgcaccgcaactgggttgagaaggaaatcccggaccacgtacccgatgaggtgatcaagcacgtccgggccttccactaccagagcccgaaggccgacaccaagtggcacaagcaggcggtcaaggccgtcattgagcacaagggcttcgcctggctcaccatcagctatgaagccttcatgaccgcctccgggaagcgggcgctgattgacttcttcgacaagcgccgcctcctgtacgtcctggatgaggcgcactacatcaagaccccgaccgcggagcgcaccaagtccatcctccgctccgcgaagtacgcgccattcaggcgggtcctgaccgggactccgattgctcagggacccttcgacgcctacagccagatcaagttcttgattgacgactactggaacaagaaccagctggggaccttcacggagttcaagcagcacttcggcatctggaagaagggctggaacccgaccgccttcaaccccaagaccaagaagaacgatggcaacgagtatgacgtgctggtgggctatcgccgcctggacgccctgaacagcctccttcagcccgtctcctcccgcgtgacgaaggatgacgtgctggacctcccgccgaagctgtacagcaagcggttcttcccgatgaccccggagcagggcaagctgtatcgccagttgcgtgacgagtacatcgtgtggctggagacgggcgggattgagcgggacgcggaagcggtcgccgcggagccgtcgccggacgcctgcccgacctgcttgggcaaacgtgaggtggagtttgacggcttcatctacccctgccccgactgcggagacgcccctgacctgggcgcggagggcaccaccccggtcatcgccgccctcgccatcacccggctcctccgcctccagcagatcacctgcggctacctcccgaccgacgatgaagcggaacccgtgtacacaatcccggggccgaaccgtcgcctggacctgctctgtgagctgatcgaggagtcccagcacaaggtgatcgtctgggcccggttccagatggacatcaccctgatcatggacgccctccgcgagcgcggcatcagcgcggtccgctatgacgggctggtgaacgatgatgagcgggcggacgccaaggcccggttccagggcgagcgccccctgtaccacaacggacaggtggttgggcgcgaggccgtcccgccggaggagcaggcccgcgtgttcgtgggcaaccccgcggcgggggcgacgggtctgaccttgaccgcagccaagactgtcatttattattccaacagcttcaagctgattgaccgcctccagtcggaggaccgcgcccaccggatcggacagaccaacaacgtgctgtacatcgacctcgtggcggaggactccgtggatgagaaggtggttgaggctttgaggaacaaattcaacgtggcgagccagatcaccggcgaccgcctcaaagactggttgtgagactactatgagccgtgtatttgttgtacagaaccaacaccgctgggaccgcgacaagcagcggttcgagcccaaatttgatctgaccccggcggaggagttcggtgagctggtgtacttgctcagcccgaccgcggcccccttccgcccggagccgatcattgatgagctgaaggagaagctggccgacttcgggccgggggaccacctcctgctcgtgggcaatccggtcctgatcgggttcgccgtcgccatcgccgcggacgccaatgatggggacgtgtccctgctccagtggagcggcaaggaccaacgctacatcgcggtggacgcctcgggcctctttacttcttccgattgaccggctatacttcttcagcgtgattgggataccccctcaccgaagaaacggagaaccacatgtcaagtgaaaacgcatacctggactatgtccaacctcagaccgccggtggcgaactgagccaactcactcagctggccgaacaacaggccgctgcccagtcgaaggtcgcagacctcgaagcccagctcaacaaggcccgcgaagaactccgcgacatcgcggagcgccaggtgcccgaactcatggaccagatcggcattggcgagttcaagaccaccaccggcctgaagatcaagattgacgagacgatccgcgccagcatcccgaaggccaaggccccgctcgccttcgcctggctcaagcagcacggccacgccgcgatgatcaagcgcgtggtcgccgtcgccttcggcaagggcgaggacgagaaggctgacgaactgcgccagcgtctcgcggacgagttcgaggtggacgacaacgccagcgtccatccttcgacccttgccgctttcgtccgcgagaagctgcgtgaaggcgaggaagtccccctggacctgttcggggtccatcgtcagcgcgtgtccaagatcgaagtgtgaccagaatgccggaggacggccccgggccttcctcccgaccgaaccgccccgcgggtgacagcgggtacagccggtgagacggcagggctattcgaccgggggcccaatcgacccgctcacattgaaccgaaggagccacaccatggccaagaccgatagcaagaccaccgatgtcgcagtgaaggaacagaacaccgcaatggcggagtatggcgcatatgccgactacgcgggcgcgggtttcgagaaccagaccagcgatgactacagcatcccgttcctccagattcttcaggccctcagcccgcagctccaggagaacgacagcctgcgccagggcatgatcctgaacaccgtgaccggcgaagtctgggacggcaagaagggcattgccttcgtcccggcgaccacccagcacgtgtacgtggagtggaagccccgcgatgcgggcggcggtttcgtgggcatccacgaagtcaacagcgatctggtgaaccacgccaaggccgcgtcctcggagtatggcaagtacagcaccccggacggcaacgagctgatcgaaaccttctatgtgtacggcatcgcgctggatgatgacggcaacgcctcggaagcggtcctggccttcagctccacgaagatcaagaagtacaagggctggatgaccaaggccaagaccatccagattccgctgccggacggtcgccgcattccggctccgctgttcgcccaccgctaccgcctcaagaccgtgagcgagaagaacaacaagggccagttcttcaactgggacgccatcgccttcgacggcgagaacgcccaacaggctcgcctcctgcccgatgacccgctgttccagtccgccgtgaacatcaagtcgatgatcgagcagggcaaggcccgcgctgcctatgagtcgcaggctccgggctccgcggacgaagaagcccagggcgcaggcggcggcaagccggtgttctgatctaccgggaggaccgacccggacggcccgccccctcgggccgtaccttcagggggccttcgtggcccccttcttttcatcagaaacggagaacgatcatcatgtggagtccgcaacagcagaccgcgctggaccgggttgggcggtggctcaagacccgggacaagcccgtgttccagctcgccgggtacgccggaaccggcaagaccaccctggccaaacacctcgccgcgaccgtcaacggtcccgtgtacttcgccgcctacaccggcaaggccgctcacgtcctcacgaagtccggggcgaccaacgtgagcaccatccacaagctcatctacacgcccaaggacaagtcgcagcagcgcctgaaggaactccaagcggagcgggcgaagctgctaacccacaagcccgtcccggaaaccctcgtggagaaggtcgatgcggcgatcaaggcggagcagatcaacctcgcccgcccgatgttccagctcaacacggagtcgcccctgttcgaggccgcgctgctcgtggtggatgagtattccatgattgacgagcagatgggggaggacttgctcagcttcggttgcccgatcctcgccctgggcgatcccggacagctcccgcccgtgggcggcacccccttcttcaagaacaagcccgacatcctgctcacggagattcaccgccaggcccaggacaacccgatcatctggatgtccaaggaggtccgcgagggccgcgtgctccgccccggcgactacggcgccagccgcgtgattccctatggccgcctgccgcgcgaagaactccgggacatggtactgtccactgaccagctcctcgttggcaggaacgccacgagaatcacgagcaacggacgtgcccgtgaactcctcgggcggacgaacgccctgccgcaggaaggcgacaagctggtgtgcctccgcaacaaccacgaggtgggcctgctcaacggtcagctctggaaggtccgccgtgacacgatcttcgacggcgactatgtcatcatggacatcgaaggcgaggacggcgcgaaggtcgaagtcagcgcccacccccactacttccacggcagcaagccggagtattgggagcggaaggacgcggaggagttcgactatggctatgcgctcaccgtccacaagtcgcagggctcccagtggaacaacgtcctgctgtttgatgagtggtacgggaaggaccggaaggaatggttgtacaccgccattacccgggccgcggaacgcatcgacctcgttatgatgtagcccaagaacaggagcaacgatatgatagaaagccctcaacccttcaaggagactcgcaaaatgcacggtcctcaagtaccctactcacaagaactacacgcccagaagtaccgcggcagcggcgagtccttccgcgaggccatgaaccggatcgccgcggccctgaaggacgatgaccagcacttcgcggacttccgggacgccctcctgggcatgcgcttcctcccggcgggccgcatccagtccgcgatgggctccacccgccaagtcacaccctacaactgctatgtctccgggacgatcaacgacagcttcgtggacggcgaaggctccatcatggtccgggccgcggaagccgcagccacgatgcggatgggcggcgggatcggctatgacttcagcaccctccgtcctcgcggcgacctgatccgcaagctccagtcccactcctccggccccatcagcttcatgcacatcttcgacgcgatctgcaagtgcgtcgcctcctccggccatcgccgcggagcccagatgggggtgatgcgcgtggaccatcccgacatcgaggagttcattcacgccaagcaacccgggaaggacgttcagccgctctgggacctcgtggccgaactcccggagggagcccagaagcagcagttggtcatgtcccttcagcagaccctgaagctgaccggcttcaacgtctccgtcgccatcaccgacaagttcatggagtgcgtcgcctccggcgagccgttccccctcaccttcgagggccggacctaccgcgaagtggacgcccgggcgctgtgggacgcgatcatgcgcgggacctgggattgggcggagcccggggtgctgttcatcgacgcgatcaaccgcatgaacaacctctggtactgcgagaccatcgccgccacgaacccctgcggtgagcaaccgctcccgccctacggtgcctgcttgttgggctccttcaacctggtcaagtacatcttcaaggacggggcgggccgctacgccttcgactgggaccagtaccgcgaggacatcccgcaggtggtccgcgcgatggacaacgtggttgatcgcgcgatctacccgctgccgcagcagaagcaggaagccaaggacaagcgccgcatgggcctcgggatcaccggcctggccaacgctgccgaagccctgggccatgagtacggttcgcccgccttcctcgccttcgaggcggaggtgctggacacgctgcgtgatgagtcctacctggccagcgcccacatcgccaaggtcaagggctccttcccgaagttcgacaaggacaagtacctccagggccagttcatcaagaccctccgcgaggacgtgcgggacgccatcgccaaatacggcatccgcaactcccacctcacttccatcgccccgaccgggaccatcagcctgtgcgccgacaacgtcagctccgggattgagccggtgttcgcctacagcttcgaccgcaccgtgatcgagttcagcggcccgcgggtggagacggtggaggactacggtgcccgcgtgttcggggttcgcggcaaggcctgctcccgcgtcaccgtccaggaacacgtcgccgccctgaccgtcgccgcccagcgggtcgattccgcggtgagcaagacctgcaacgtgccttccgacatcagctgggaggacttcaagaacgtgtacgtgagcgcctgggaaggcggggcgaaaggctgcaccaccttccgtctgggcgggaagcggtcgggcatcctcgtggtgaaggatgacggcggcgagcccgaagcggacgccccggcggaggagccggcaagccagtgccgcatcgacccggccacgggacggagggagtgcgagtgaaagaactgagcctgaaggcggtcttgctgatcgccgccgggttcttgctcatgaccgggatgcgccttgctgaatgggccatcccggtcccggagcggaccctcaaactgaacgtcacccaagaaatggaggaacccgaagatgaacaagcccctgctgatcggtcaagcacccggacctaacacggacccggaccggcccctggctcccctcccgcggtcctccgcgggagggcgtctggcggagctggcgggcctatcgcccaaggactacctcaagaccttcgaccgcaccaacctgctccacaccttcccggggcgctggaagcgggacgacaagtggcccgcccgggacgcggggattgccgcagccgcgatgaagcccttgttgggcggtcggcacgtcatcctcgttgggcggaacgtcgcagaggctttcggctatccggcccagcacctggacttccaccagtggtttgcggatgatcgctggggcttcgaggtcgctgtggttccgcacacctcggggcgcaaccattggtacaggaagcctgggcacgaggacgccgcccgggccttctgggaagaagttgtacaacggttcgccctccgccgtccaacggttgttggccttcggacggggacctgaaaaagtttagtcaaaccactttacttcttcgggggctggggttaagattctctcacggtcgaacaagatcgcacctcaaccccagaaaaggagcctaccatgaacgccatcaacttcaacaacgtcgcctacaccgaagcctccctgagcgagctgtccggcccggccctggtcgagctgtacaacgaagtcatcggcaccttccgcaacggcgagtccgtcccgaacgtccgccgctttgccgacaagaccaccgccattgcccgcacctggaagatgcttcagcgttatgccgaagcgcacccggaagttgaggctgacgagcaggccgaaccccagaaggtcgaaaccgtgaacgaaaccgcaacccccgcccccgtcgctgctccgaaggcccagaaggctccgaagtccgcggaggagaagaaggcccgcgccccgcgcggcaccaacctggccgccccgggccacgccccgatcccctgccgcgagggctcgaagcaggccatgctcctggacatgctgtcccgcccgaacggtgcgaccatggctgaactgatcgaagccctgagtggcggcaacaagccctggaccgaagccaccgtgcgctccggcttcggttgggacatgaagctgaagggctacggggtccgctccgccttcgccgcggacggcactgagcggttccacatcgtggtccctgaaggccacgcgatcccggcccacaagccgctgaagtccgccccgaaggctgacgcccgccagacccgcctggttggctgaggcaagggtcatgggagcctcggagcgcacctatgactacctgatccgccgggtggagtacccggcggagcggggatacagaatggagcccttcaagctacctccgtggattcacgtggtgatcacggaggacggcgacagcaagtggctgacggtccattcccgtattcacgtcaacaaagaagtccgcatggagccttccttcagtcgccaattctctgattgggacatcttgaaggacctgagcgggaaaatcagtcacgcatacttgtgagaaaagattatgagcagaaactacccccggctggacatcgagacgtttggccgacatctgatcaccaccggcgatctggaccccatctacacggccctggttcgggcggagcaggcgggggacttctccgtgccgcagctctgtcgttggctccttggatattggtgctactaccacgccggggtcgcctccttcctgagtgagaaggagggcgaggagttctggcactggatgatggtcgcggcccgcaacgaggaggagacgcccgccggaggacgctggccccggggacacgagcgccgccactaccgggccaagatcgccgtggactccgtgacctccctccaggcccgctacggcgaccgcccggagaacatggccctgtacgtgggagcccgggcgacggaggatgagcgcctgcccttccgcaccgtctccgcccgcgcccaggagcacaacggcttcggtccgtggatcggcttcaagatcgcggacatgatggaccgggtgatggaggtcccggtggacttcgacaacgccgccgtgttcatgttcaaggacccggagaaggccgcgatgatgctgtgggagcagcgcgaggcgcacaagtacccggagaacgcgaagccgaagcgcgaggcgatcctgtccggggtcgcggactacctgattgggcggttcgcggacctcgccgccccgcccctgggcgaccgccccgtgaacatccaggaggtcgagacggtcctgtgtaaatggaagtcccacatgaatggccactacccgctctggaacgacatccgggaaatcaacggcgggctcgaaccgtgggcgggccgctgctccgccgcgcgggccttcctcaaccacatgcccaaggagcagtgagatgatcgtcaacaacaccccggtcgaaacctatgagctcaacggggtcccgatcctcgtgaagcgggaggacctgtgcgccccgctcccgggtccgtccttcagcaagattcgcggagttgtcgcccatatcaagaaccggcctgagaccaccatcggctgtctggacacgtaccactcgaaggcgggctgggcggtcgcctacgtctgccagcagctcgggaaacaggccgtggactactggccccgcttcaagcgcgacggggccgcggacgccccgcgcgtccaacagcagcacgctcgccagctcggggcggacctcgtggacatcccggcgggccgctccgcgatcctgtaccacacggccaagaagcacctgcgggagaactaccacgacagctacctgatgccgaacgccctgaagctcccggagtcgatcacggagaacgccgcggaggccgtccgcaccgccccgcacctcccggactccgggaccctggtcatcagtatcagctcggggacggtcgccgccggggtgctcaagggcttcgaggaggcgggcctgctccgcaactacaacgtcatcctccacatgggatactcgcggagccaggacgccacccgggagtacatcgagaaggccgcgggcctgaccctgggcgaccggatcaagttcattgacgagggctacgggtacgcggacgcggcccgggacgcctccgccccgttcccctgcaacccgttctatgatctgaaggcttggaagtggctgagtgacccgctcaacctggcttccgtccatccacgccccatcgtgttctggaacatcggggagtgacccaattcatagtgctttacttcttccgggtaaggcactagactttttcgcaatagatgaggagttgaactatggaccacgcagcatggctgaatgaagaaaccggcgaagccgctcaggaggcttacaagtatttcatgcgcccggacccgaaccaacgggagttcctgggcccaatcgaggaggaggatgacccgctgaccggcatgcgcgcgaagttccgcatggccaaggtggggatggtccgcaacgcgaaggatgacgacaagaaggaggtcaaggtgtatcttggcttcaatgacgtcacctacctcccgcacatccgcatcccgaacgccaagccccttcagggctggtaccaggacaagcacaacgacaagcgaggctcccgcgcccgcccctgcttcagcgaggcgatcctgacggagccttatgggggctactgcaccgtgggttgcgccttctgctacgtcaacagcgggttccggggctaccgcggcaccggcctcatcagcgtcccggtgaactacggcgagcaggtccgcaacatgctctcgaagtcccggacctccgccgcgggctacttctccagcttcacggaccccttcctgccgattgaggacgtgtaccacaacacccagcagggggcggaagccttcgtggagttgggcctgcccatcttcttcctgagccgtctcagctacccgtcctgggccatcgacctcctgaagcggaacccctacagctacgcccagaagtcgctgaacaccggcaacgaccgcgattggcacaagttgtcccccggggccatttccctccaggaccacattgacgaaatcgcggagctgcgccgtcagggcatctacacgtccattcaggtcaatccggtggtcccggggatcgtcacccatgacgacatccgccacctgttcgagcgcctggccgcggtcggcaacaaccacgtgatcgtgaagttcgtggaagcgggctacagctgggctccggcgatgatcgaacgtctccacaagcggttcggcccggagcgcaccaaagccttcatggacctgttcacggagaaccaggccggagcccaaaagaccatcgcggagccgtaccgggtcgaagcccaccagctgtaccggaagtgggcgacggagctgggcatgacctacgcgacgtgctatgagtaccgccgcgggaagcccggaaccggcgaaccggcctggctttcgatgggccgtgaaatgatcaccgcggaccagtgccacggccagcgcgtcccgatgttcacccggaccgatctgggccagcccttccaggaggtcaaggagtgcgcccccaccggctgtctccactgcgcggacgacaacgagggcaagccccgctgcggttcggaactgttcggggcggcgaaggctctgcgctcgcccgacttcaagaagatcgtggaaccgaccccgccggaggaggacggcggcgagcgcaagatcatcccgatcacgcagattgactgagcaacccgggcggggctccggctccgccgttttcaactgaaatggagaaccaagatgaagtacatcaacgtgcggggctgtaacggctccggcaagaccaccctgctgcgctgcctggcccgcgatccgctttgccgcgtcatcaacgtcatcgtcccggaccacaagccgatcccggtgacgtatgccccggacggcatcgccatcatcggggactacacccccgccgccgccggagcgaccaccgccggtctggaccggatcaagacccaagccgccgccaaggccgtcgcggagctggttgggcgggacccggacgtgaaggcggtcctgttcgagggcgtggtggtcagcaccatctacggtccgtggcaggagtggtcgaaggcgaacggcggaatgatctgggccttcctggacacaccgctcgaagtctgcctgaagcgcatccaggagcgcaacggcgggaagcccatcaaggaggaccaggtggccgacaagcaccgcaccatcgcccgggtccgcgacaaggccctggcggacggcgagacggtccgcgacatccactgggagacggccctgaaggacatcaaggccgtcatcgagaacttgggctgaggaccccgactatgaccacaccgcgcctcaacgacatcgccgccttcatgaaggcccggcacgacatctacttggaccgcaaggccgggaagcccggcccctggaccgcggacccggttctgcgtgatgggcggttctgcaacatcttccgggagctggacacggtgacgatctgggttgacaagcatatccgtcagccctacgcggaccacccgcacctctggttcatgctcgccatcgcccgctacatcaactggccggataccctcgcggagctgatccagaccaagcagtggcccgacaaccctgacttcgagccctcctggctcacgaccgctctggagcatcgcgccgtccgcggcgacaaggtgtacaccggagcctacatgatccgcgcggagtccgacccctccaaggagtggtacagctggaccaagcaccgctacatcgcggagattgtcctgggccgtctctgggaggaccgcgaggaatggcagcggatgctggaaaccactccgggcgtcctccggtccttcaaccggctcgaaaccgtctgggagaagttccagcagcaacgctacatcggctggggtccgttcatggcctatgaggtggtgaccgacctccgccacacccgctacctgcgcaacgccccggacatctgggcttgggccaacgccggtcccggggcgatccgcgggctcaaccgcctgtatgggcgcgacctcgccgcgaagccccgcccggagcagacgaacgcggaaatgatcgagctgatgcaggagctgaacgccctggacgcccggggcttcaacgaaaccttcggaccgccgcagctcgggagcccgcacgtggggccgcggttcgaggcccgggacattgaacacacgctgtgcgagttcgacaagtatgagcgcgtgcgcctgaacgaaggcaagatgcgctcgaagtatgactggcgcaaggcaaccaccctcgcctgatcgaaaccccgccgccggaccattccggcggcaccaacgaaatggagaaaccatcatggctgtacgtctgtccaattacatccgcgagcaggtccgtgacgcgatcctcgcccactccttctccgaccgcgagaaggccctggacgcccgcgagaaggagctggcgctggagttctacaacgacctgtacccggaagcggtccgcgcccacatgtacgccctgcccaacggcttcctcgaagtccgcagcagcatccgcgtccaggtggttggggagtcctaccactcgctggacctcccggagaagaagcgcgtggccgattgctgggcctcgaaccccggcaaggtctataacgcggaccacccgctgggcgagaagctgcgcacctacctgaaggaccgcgcccagttcaagcgcgagcgggaggaggccaagaccggagcctgggccgtcctcgaaagcgtgaccacggtcaacaagctgattcaggtctggccggaggtggagcagttcgcccgccccttcgcggttgaatcgccgtcccgggctatcgcgctgccgatcaaggacctgaacgcccgcctgggccttccgcctcagaccgcttcggcttaacaggagggggccatgatcttctcgccgttctggtggtactggagctggtggttggtctggctccctcgcccccgcgtccttcgccggaccggcaacgtcatcttcgtggagttcaacaagaaatgaaagtcatcaagacccgcaacgtacaacaggccctcccggaggccctgtatcaactgtccttcgagggcgtccgccgcgactcgcgcaacggccccgtgttcatgttcccggaacccgtcaccaccgtgtacctccgcccggcggagcgcgtgctgttctgggcggaacgggacgccaaccccttcttccacctgatggaaagcctctggatgctgggcggacgcaatgacgtggagtacgtcgcccgcttcgtggatcgcatgcgcagctactcggatgacggcctgaccttccacggggcctacggcttccgctggcgccagcacttcttcgaggaccagctgcccaagatcatcgccgccctgaaggcgaaccgcgatgaccgccgccaggtcctgtcgatgtgggacgcggacgcggacctgggccgccaaggcaaggacctcccctgcaaccttcaggccatcttccagatcgcctgtgacggtcgcctggacatgaccgtgaccaaccgctccaacgacctgatctggggagcctacggggccaacgcggtccacttcagctacctccatgagtacgtcgcccggagtgtcggggttgaacaaggcatctaccgccaagtcagcgccaacttccacgcctatgaggaggtgctggacaaggtcgccccgctcgcggaactcgccgccaacccgatgaccgggaaggagacgcccgacccctacgccgccgggatcgcggagccgtacccgctgatgtccacggacccggaggagtggaaccaggagctgatgatgttcctgagcgagccggacgccgtgggcttccgtgacccgttcttccgtcgcgtggcgatcccgatgttgaaggcccacaaggctttcaagcagacctccaacccctcccgctttgacgccgccttggcggagctggacaacgtcgccgccaccgactggaagctggccggggtggagtggatcgaacgccgccgcgccgccttcgaggctcgcaaggcccgggcgatggacgatggcgtggcgtatgagtgaggagacgcaataatgggaagcctgatgagcaagattcatgacgaggagcgcgaggcggaggagctgaaccgccgcgccgcccgcccgctcctgacccggatcgccgcgaccagggaggccgggacggtccgccggtgtcacatcgttccgcaccacggtcagtacaacatcgcccagcacagctacggggccgtgagcctcttgctgctgctccacccgcacccgtcgctgaacctgatcaaggcggtccagtggcacgactgcgcggagcgttggttgggcgacatcccggccccggcgaagtggacccactccgaactcgggaaggtgtatgaggaggcggaacgccgcgtgctggcgaccctgggcctgctcccgggccttctccctgacgaggaggactggttgaaggccgtggacaccctcgaactgtggttgtggtgccgggaggaagaagccctgggcaacgaagcggtcacggccatgcggagggcatgcgaggcggtgacggagaagcggggcctggagggtagcctgcccgaacccgtccgcgccttctacgtggcagcgaagcaccagccgcatggccgtctctcggacttcttcgaggaggtggtgcgcgatggacttggagaagctgcgacgtgattgggcggaggacccgcagctgaagttctacgccttcgacacggtggaagaactcgctgcgcacctccgcaaggtccatacagatatgatgaacggggagcacgggtgttttgggtacttgtaccgccagcagacactccggctccgggaactgatgaaggagttacaagatgagcgtgaacgaaaagcaagtgggcggtgagcactaccgctcgcccgttcaacactgggactacgtggagctgaacggcctccgctacaccgaaggctgcgcgaccaagtacgcgacccgcaaccgcaagaagcacgaggacccgcgccaggaccttgagaaggcgatccactacgtggagaaggtccaggacctgtaccgcaacggggtcctgctgccccgctccgcccccgtggtcattaccccggacgccttcgccgccgcgaacgggctgacggaggacgaagccgaagtggtccgcatcctcaccttctgggagtccgacccggagctgaccgcggccctgaacctcctgcgcaagatgattgaggaggtcggagcctgatgtcatacctccaaccacccctgttcacgaccgtctccagcgactgggtggccccggacctcaacaccctcccctcgtgggagggggccaagcgggtcgccatcgactgcgagacgcgggacccggacctgcgcaaactcggaccgggggcgggccgtcgcccgaacagctacatcaccggcatcagcttcgcaatcgaggacggcccgggcgggtacttgcccatcagacacgaaggcgggggcaacctcccgctggagggcgtgctggcctacctccgcgcccaggcaaaggtgttcaccggcgacctcgtgggggccaacctcccgtatgacctggacttcctcgccggggacggcatcgagttcgagcgggtccgctacttccgtgacatccagatcgctgacccgctgatctgcgaactccacgacagctacagcatgcaagctatcgcggagcggtggggcttccacggcaaggacgaagccctgctgcgcgccgccgcggtcgattatgggattgacccgaagaaggacatgtggatgctcccggccaagtttgtcgggaagtacgcggaggaggacacgcgcctgcctctgaacatcctccgccgtcaggagcgggagattgatgagcaggacctctggggcgtgtacaacctggagtccaagctgctcccgatcctcacgggccttcgccgccggggcgtccgaatcgactgcgaccgcctggacatgattgagcgttgggcgctggagaaggagacggaggccctggcccaagtccggtcgatcaccggccaccggatcgccgtgggcgatgtctggaagccggaggtgatcgcccccgccctcgaacacatcggcatcaagctgaacaagacctcccagggcaagcccaacatcgacaaggagctgctgggctcaatcgaccaccccgtggcggacctcctcgaacgcgcccggaaggtgaacaagctgcgcacgaccttcgccagctccgtccgggaccacatggtgaacggtcgcctccacgggacgttcaaccagctccgccgccagaaggatgacgaaagcgacgggaccgcgggcgctgcctacgggcgactgtccagcgaacacccgaacctccagcagcaaccggctcgggatgagttcgccatgatgtggcgggccatctacctcccggaggaaggccaacactgggcgtccaacgactacagccagcaggagccgcgcatggcggtccactacgcctgcttggcgaaggacctgattgggcaccaagcctggctgtccgcaatcgaagcccgggacaagtaccgcaacgacccgaacaccgacaaccaccagatgatggcggacatggcggggatcaagcgcaaggacgccaaggaaatctacctgggcctgtcctacgggatgggcggggcgaagatgtgccgcaagctcgggctcccgactatgatggccgtgcgcggcccccgcttccagctgttcgacgtgaacagcccggagggtcagcgcctggtcgcggaaggggcgcggaggttcgaggccgcggggccggagggtcaggccctcctggacaccttcgaccacaaggtgccgttcatcaagaagctggcgaaggcttgcgaagcccgggcgaaggccgtgggctacatcacgaccctgagcggtcgccgttgccgcttcccgaaggacaaggacgggaactatgactggacccacaagggactgaaccggctgattcagggctcctccgcggaccagaccaagatggcgatggtggcctgcgcggaagccggactggacatcatcatccaggtccacgatgagatcgccttcagcgtacacgacatgaaggaggccgcggaagccgcccacatcatgaggacgtgcacgccgctcgaactcccgtcaaaggtggacgtggagattgggcagagctggggtcattccatgggctgggacgggaacccaccatcatgaagttctgctatcaatgtgacgcgcaggtcacttacttgtttgcggacgcacgctgcgcaaagtgtacccgcctgaccccggaggaagtccggggcgaacccctggagaacgatatgcgccgcagcaacgacaacaccgtggacctcgaagtggtcatcaagcgcgagacagacaaggcatacctcatcgaccacggcggtgaggaggaagtctggatgcccaagtcacaggtccgcgcggtcgagaagaagggccgcacagcgaccctgacggtcaccgaatggatcgccaacgagaaggggctgatatgaacgacatcgccgtgcgctggacctcccggaagttctgggcggcgatgatctgggaggcggtcctggtttggctcctgtacatgggcaagttgccggtggacgccttcgagtccttgacctggctcctgctgggcggttacttcctcgggaacgtcgcccagaaggttttgctgaaggaggaggtgaaatgagcgaacgtcaagaccgctgggaccgccgctatgttgggctggcccaacacgtcgcgggctggagcaaggacccttccacgaaggtcggagccgtcctggttcggcccaacaacagcgtggcttcgaccgggttcaacggcttcccgcccgggcacgatgattcgccggagctgtacgctgaccgcgggtacaaataccagcacgttgttcacgcagaggtcaacgcactcaactttctgggctcgcctgcgactggcttcacgctctatacttctttcccctgctgtccgaactgtatggaggccgcggggaaggcgggcgtgaagcgggtcgccttcccgggcatcgactactcgggccgcgatccggggtgggttgctgagtggaatcaacgcattgatgaggctttggaagtcgcccgccgttacaacatcgaagtgaggtgggtagatgtctgaagccgcaatgtgggactccctccgccccgtcatccggtcgctggacccggtgcgcgtggagaaccccattgtgcccgggaccccggatgtgaactacaaccagggctggattgaattgaagttcgctgaacgctggccgcccaggggcggaccgcttcgagtggaccacttcacccgccagcagaggacctggctgacccgtcgccgcagggccgggggccgggccttcctcctgctgaaggtcggggagacggagtggttgctattcgatggagcggtggccgctgctatgctgggccgggttccgcgagaacgcctgtatgaggtctgtgtcgcacgttggacacgccttccaagaaccaaggagatttgtacatgtctgctacagtgacaccaaccaaaggcgaaagcctactgctacaccgccgccgcaagggcctcaatcagattgaggccgcgaaggagtacggggtgcacccggaccgctaccgtgaatgggaagcggaccgccgcctggacgatcaaccgcgccagcacctcggacaactgaagccccacgaggtctgcttgctgttccgccgccgctcgggtaagacccagcgcgaaatcgccgccgctctgggctgcactcgcctctgggtcatccagatggaggacgggaaagcgccggttgagcgccttcgtgaatattggggcttttgagggggatcggaaatggcggaactgccgaaacacaagaccaaggacgcaatcgacttcctgaagaagtggtgcccggaggggccgtgggtcctgacggccatcatcccggacgggaaaacggagacggtcacattcatgcccgaccgctggcagaaagccgcggagtggatcgaaggacatcagggcaagcgcaacctgtacttccacgtgaacccggtccgccgggcgatggacgtgaaagcctcgaaggaggacatggcccgcctcgcctggcttcacgtggacatcgacccgcgagccggggaggacttcgaggaggagcgggcgcgggcgctgaagctgctccagtcctacacgcccaagcccacggtcatcatcgactcgggcgggggctatcagggcttttggcgtctgaacccgtccgacaagctggacatcgccggatcggtggcgaaggctcaagagctggaagcctacaacatccagctggagaaggtgtttcaggcggaccactgccacaacgtggaccgcatcatgcgcctcccgggcacgatcaacatgcccaccgcgaagaaggtcaagaagggtcgccagccgaccctcgcccgtctcgtggagtggaatgaggccagctaccccatcgaacaattcacccccgcggttcgagtccagatggcggagcagggcctggccgggggccgtccgaaggtgaagatcacgggcaacgtcccggacatcggaacggaggagctgcgggagtgggcccatgagcacgggaaggctatcagcgaccacgtgctggcgctgattgctactgggcaggacccgctggacccgaccaagtacccctcccggtcggaagccctgttcaaggtctgctgcgacctcgtgcgggcggaggtccctgatgaaatgatcttcgcggtgatcaccggctccaacgaaatcgccgcgagcgtcagagacaagccgaactgggaaggctacgccctgcggcagatcgaacgtgcccacgaggaggcggtggacccttggctgcgcaagctcaacgagaagcacgccgtcatcgcggacatcggcgggaagtgccgcatcatcagcgaggtctgggacccggcgatgaagcggaccaaaatcagcaagcagtccttcgaggacttccgcaaccgctaccgccacatcaaggtagtggttgggcactcggaggagggcaagcccatcgagaaggccgcgggagccttctggattgatcacccccagcgccgccaatatgagaccatcgtgtttgcccccggccaggaggtcgaagaagcctacaacctctggcgcgggttcgcgtgcgactccctcccgggcgagaagcacatgcccttcctgaaccacatccgcgacaacgtctgctcagggaacccggagcactaccactacctggtcgggtggatggcgcggatggtccagcacccggacggcccgggcgaagtggccgtggtcctccgcggtcgccgcggcaccggcaagtccttcttcgccaaggtcctgggcgcgatgttcgggcgtcactacctccaagtcagcgactcgaagcacctggtgggctccttcaacgcccacctccgcgataccgtcctgctgttcggtgatgaggctttcttcgccggggacaagaagcacgaaagcgtgctcaagaccctcgtgaccgaagaacacctggtgatcgagggcaagggcgtggacgcggaagcggccccgaactatgtccacctggtcctcgcctcgaacgaagattgggtggtgcccgcgggtctggatgaacgccggttcttcgtcatggaggtgggtgagggacacaagcaggaccacgcctatttcaagcgcatcaaggacgatctggacaacggaggacttgagcacctgctccacttcctcctgacctatgacctgagcgccttcgaggttcgccaggttccccagacccgggcgctgcaggaccagaagatcatgagcatgtcgccggaaacccagtggatgtatgagaagctgtgggagggccggttgctcaagaccgaccaggactggcggaacaaggtggtgaaggacagcttgtatgacgactacgtgaacgacctccgcgaccagggccggaacttccgcatgagccgcaccggcttcggcaagtggcttgcccgggccttcccggacggctggccgcagtcgaagcaggaaatggcggagattccatggaccaatgaacacggcttcgaggtgatgatcaagaagcgcgtgtacatgtacca

SEQ ID NO: 8 - DNA, 63828 bp, unidentified
  source 1..63828: mol_type = genomic DNA
atggcgtaccagccaccccactggaagcgcaagaagaccatccagcaggtgcaggagcagacccggaccaaggcctggatcccccaggccggcagccaggtcctcttcctcacctgcccggtcttcgagaccctgtacgagggcacccgcggtccgggcaagaccgacgcgctcctggcggacttctgccaacacgtgggccagggctacggcgctgcctggcgtggcatcctgttccgcaccacctacaagcagctgtccgacgtggtggcgaagtccaaggtgtggttcaagctctggttccctggggccaagttcaacgagagcgattatacctggaccttcccggagggcgagcagctcctcctgcggtacatgtccaagcccgctgactacgacaactatcacggccacgcgtacccgtggataggctgggaagagctcaccaattgggccaccagcgaaatgtacctcaagatgttcagctgctgccgctcgacggtacctggcatgccccgcaaggtgcgcgctacgaccaacccgtacggcaagggtcacaactgggtcaagctgcggttcaggctgcccggcatgcggggcaaggtcatcaagaccgagggcgagcccgaccgcatcgccatccacgggcacatcagcgagaacaggatcctgctggatgccgacccggattacatccagcgcatcagggcagctgcatcgaacccctcccaggtcgcggcctggctggaaggcagctgggacatcacctctggcggtatgttcgacgacctctggcagacgaccacacacgtggtccgacccttccaggtcccgcgcacctggatcgtggaccggtccttcgactggggcagcagcaagcccttctccgtgggctggtgggctgagtccgatggtacggacctggtcttccctgacggcaggcgcatgcgcaccgtgcggggcgacatcttccgcatcgccgagtggtacggcatgaagaagggcaccgagaacgagggcctgaagatgctggcctccgacatagcggagggcatcaggctcagggaggtcggcctcggcctggccggacgtgtgaagcctggtcccgctgaccctgccatctggtcggaggagaacgggaactgcatcgagcgggacatgcgcgccaagggcatcaagtgggagaaggctgacaactcccgcgtccagggctgggaacagttccgcaagaagctgaagaactccctcaacctcgatgagatggacctgcccaggaacgtgccgcgtgaggcaccaggcatctacgtggtaggtgagcgctgccctgacttcgtgcggaccgtgccacccatgccgcgtgacgagaagaagcctgacgacgtggacaccgacgtcgaggaccacgctggcgatgattcacgctaccgcgtgatgcacaagaggaaggaggtccgccagggcaacttctaaagtgatggtgttcgagccatggatggcccggcatcattaacccatcctccgacacgctgaccgacgagacagcgctaggctggcaccaagtaagaggcgacgcccatgactcagcggtccaggggctgaccatccgaaaagtccacgcagtaggatcaccctctcgttcgccccgcccggaggtccacccgagggcggggcaccatggggtccaggtcgtctaacatggctaggacacctcccggttaggtttgaagccgccaggaggagaagcaggttcgatacctgcccagtgcccctccacaacagtcttcaccggcgagctcccttacgatgttcacaggagtgcacgcctgagcaggtcagccgacacggtcctatccccagggcacggtcgcagagcctgcgggaaccctagggagctccccggtgcagactggcaggacaggatcggcgggaccaccctaccatgggagagtggagcaaaccgttgtccagcctagcgggctataagcgcctccgacccctgccagcacctctcgaagcccccgccgatcgggggcttcgccttttgtggagttcgatggcgttcggccatggctgggcccggtaaactgagctccctaccaaggagtccatccatgaagatcttcgacccgaacgccatcgtgccctatgaggtagcacccctccctgaggacgaggccaatcaggccgtgacgtcccgcgaccaggggcgacgctccgcaggcctgctgtccatgctggccagtgagcaggagaagttcctccaccagctggctgtcgaccgagccgacaagacctggctggagaccaacaccccgatgggtactgtcttcgaggtcctgggcgtggcccacatggtggtcagcctgccgcactacatcaagacgccggagcgtcccggctggggcccgatgctggtgaatgtcatggcgcccgacggccggggcggcatcgaccgctccgtgctgagctgcacccagctgcgcgccatgctcgagcccgggttcgtccgcccatgagcgcggcgtactcttcggtccgcaagggtgtcagggcgtggctcgaggccaaccccggcgagcacgccatccagcacattgccacacagtccggcctcgaccggagcgccgtgacggacgtgctgggcaagatgcgtcgtgcaggggaagcccgctgtaccaaggtcggccatggtcgcctgtatgagctcgtgccgggcgcggccgacacctccaggaagatcggcaggcgggaccccgaggccaagcgtgagtacgccaggctctacttccagcgcaagagcgccgagatgaagagggagcgcatgtcgcgcctggcggacgagcaggcacctccgcccgaggagcccagggaggagcgggctgagaccgtggccgagttcaggcgtagaggagggcgggtggaagtgctggccagccattggaactgaacgacggcccgcagcgagccttccccgcggcatcatgcgtctaccgggtcttggacaccccggtcatggcgttccatcggttggaagggttgagagccccgatcccacaagggtcggggctttctttttcgccggctcgcgctacgagcacgcatgcgtcacgatgcgcgctctaccccgagccgtacccgaccacctggagcaccccatgatcgacccgaagacgggcattcgcctcgtcccagcccgcgactccctcctgacggagttcggcgccaccaccctgtccaaacagtactgcctgcccggcgaatcctaccagcaggcattcgcccgcgcagccaaggccttctccggtggcgacgacgccctggcgcagcgcctgtatgactacgcctccctgcagtggttcatgtttgccaccccgctgctctccaatggtggcaccaatcgcggcctgcccatcagctgcttcctcaacgacgtcgaggactccatcgacggcctggtcgccaacttcgccgagaacgccaagctctcgaccaacggtggcggcatcggcaccaactggagccgcatccggtcgatcggcgagacgacgaccaagggcgtcgacacccccggcgtgatggccttcatgcacgtgcaggactcccaggcgatcgcctaccaccaggggcgcaccaggcgaggtgcccacgcggtctacctggacgtctcccaccccgagatcgtcgagttcatcaacatgcgctcggccactggtggcgacgtccaccggaagaacgaaaacctccaccacggggtcaacatcacggatgacttcatgcgcgccgtggagtccaacggcacgtgggacctggttgacccgcactccggccgggtgaccgacacggtccaggcccgcgccctgtggatccagatgctccagcagcgcgcccgcctcggcgagccctacctcttcttcattgacgcggccaaccgcgacctgcaccccgccctgcgcgccaagggcctccgggtcaaccattcgaacctgtgcaccgagatcaccctgccgaccacgccggaccgcacagcggtctgctgcctgtcgtccaccaacgtcgccaaggccgacgagtggtgggaggtgcgggagcagttcattgccgacctggtgaccatgctggacaatgccctgacggtcttcgtcgagcaggcccccaaggccatgtggcgcgcggtcgcctccgtcatgggcgagcggtcgatcggcctgggcaccctgggcttccatacctattgccaggacaagggctgggcgctggactcccatgaggccgccaccttcaacatcaccctgtactccgagctgaaggcccacgccgtggccgcctccatgcagctggctgttgagcgcggcgaacctgaggacctggttggtaccggcctccgcaacgcccacctgctggccatcgccccgaacgccaccagctccatcatctgcggcggcgtcagcccgagcaccgagccgatggtggcgaatgccttctcccagaagacgatggctggcacggggatcatgaagaaccccgcgctgcagcgcaggttgatcgagatcggccaggacaacgacgacgtctggcgcagtgtcttcctcgaacgcggatcggtgcagcatctgccgttcctggacgctgcggacaaggctctgttcgcgaccgcctcggagaccgacccgggcgtcctgatcgagctggccgcgcagcgtcagcccttcatctgccaggcccaaagcctcaacatcttcttgccggccggtgtggacaccaagacgatgcaccaggtgcacatgcgtgcatggaaggtgggcctcaagtcgctgtactacctccgctccagctcggtcaaggccacctcggtcggcgtgatgcccgagatcatgcgcgagcccgcccccgtcgtagtcgaagaggtggttgacctccccgaggtgagcggcgcagtatgcaacctcggcggcgactgcgtcgcctgtgaaggctgaggaccacatgaccaacgtacccgtacccaccccgcaggccccttctctcttcgagaagcgggccgagtacaagcccttctggtacccctgggcgtaccaggccttcaccgagagcgagcagatgcactggctcgtgcgtgaggtgcccatgacggcggacgtcaagacctggcgggtcgacctgaccgaccgggagcgccacctgctgacccacatcttccggttcttcacccaggcggacgtcgacgtcgcctccgggtacatcgaccggtacctgccgacgttcaagcccaccgagatccgcatggcgatggcctccatcgccgcccgggagggcgtccacatacaggcttactccaccctgatcgacgagctcggcatccccgaggtcgagtactccgcgttcatggggtacaaggagatgctggacaagcacgagtacttgttccagcgccgggagggccttgaaggcctggccctggacatcgccgtcttctctgccttcggggaggggctgcagctcttctccagcttcgtcatgctgctcaacttcacccggttcggcaagatgacgggcatggggcaggtggtgagctggtccatccgggacgagaccctgcacgtcgagttcatgatgagggtgtaccaccagctgctagccgaacacccccacctccgcacggccgagcactccgagcgtatccgcgaggtggctcagaagatggtggagctcgagttcgccttcatcgacctggcctatgagaccggcgagaaccagggcctcaccccggaagacgtgaagcagtatatccgctataccgcagaccagcgtctccagcagctcggcgagcgcccgctgtttggcatcgacaagaacccgctcgcctgggtggatgccatcgtattcggcaaggagcacaccaacttcttcgagaaccgggcgaccgactactccaagggcgcggtgcagggcaactgggacgacgccttcgacaactgaccagcgccaagctgggaacgatggcttaacctcctgaggggcgacgatacactgtgatcgtcgcccctattcattatccgggcctggcggcacccggtcaggagataccaatgcaacagacctcagggtccatgacccgtcatgcaccggtcgcacaggtgaccatcatcccgcgcttcgcgcaccgcttcgacgacgtgccgcaggccctccatgccgccctcgagcgagcccagctgaacgtggtgcccaatgccttccgcgtcaacgcgggccgcgacctgttcgagctctacttggagcaattcgacccgcaggaccgccagtaccacaactgcaactgctgccgctcgttcatcgggcgctacggcagcctggtgaccctcacccccgacggcaagaccaagtccgtgctgtgggacgagaccctgctgggctcccgccacccctaccgcaaggtcatcaaggccctgcgtgaggccgtcgagcgcggccacgtggtggaccagttcttctgggatggcaagggcgactggggtgtgcgcgagcagggcggcttcacccacctgtggaccagcccgggcgtcgtgtcacattcatcaacgctgaagaacgctgaccagctggcagccgagcagcgtgagaaccgcaggcacctgcaccgcgccctgtcagagttcaccctgggcgacctggagcgggcccgcgacctgctgctgaccgggggcctcaaccagggcgacaagacggccaagatggcggagttcctgatcgaggccaagcgttcgatggcccacatctccggtggtgaggccgtgaaccgtcgcctctggttccgtgttgctctggcagccaaggggtggtgcacgccgcgctcctcggtgctcggcgccctgatcgatgacctccgctccggcgcctcggtcgagtccatccgccggaaccacaacaagcgagccgatcccttgacctaccagcgggcgcaggtcgcaccgaccgccggcaacgtggcgcgggccgagcgcctgttcgagcagatgggcctcgcccgctcgctcgagcggcgtccggcgcgggctgatgaggtcgtgttcgactggaccccgcaagtgacggatgccccgcagtcctcgggcggcatcttcagccacctcctggcccaggaccggctgaagaccgagcgggcgctgctcaatgtccaggcggagcgcatcacctacgcccgcttcgcccgcgacgtcctgccgcgcgccctggagatcgaggcagtggtgccccaccagggcaacttctgtgcgatcacgacggctgtccatcccgacgccccgccgatcctgcagtgggactccctggagtgccgcaacccgtttgcctggtacgtgtaccaccagggctcgccggcatccaactggggcctccgttcgggccgtgtaaaggtcgtcggcgtcacgaagcagccgtcgcagtggaacggggatcacttctcccgccatggccggtcggtgatcttcctgctcgagggcgcagctgaccagcgcaatgcttcgctggctctcttcccggagtgcctgcggagcgagctgcacgaggtgcgggccaccctggaggcgcactcccgcgccaccaagctggcacgactgcgtccgggtgtccagcatgctgcgggcctgcgcgtcgacgaccgcaccccgctcgaggtcctggtgcgcacctccggtggcgtggccaggtaccagctggatcgcatggattgatggtacgcggttaactggggaggagcctatcatggctcctcccctccttttacccctggagaacacaatggacttctcacctcccaacttctggctcaccctcgtgatagcactgttcgccgtgtccgcggcctggctggcacgctcgatccgcaggcccggcaacatgtaccgcgctggcattgagtatgcccttgctgagctctacctggcggaggacgccgaagagacggccgacgtgctctgggcgcgcagcgagccagcattcgacgagccggagtccgcgctggacttcgaccgtggcatccgtgagggcatccggctgtacgccaaggccgacgacaccggcatccgagagctggaggagctgcgatcccagctcacccgcatggtgggcgacggcgaggcaagcctgagcgaggtcggcgtcgccctcgacgtcatcgaccggcgcatcggcgtcggttaccccactgaacccgagctggagcagaccagtgagtactaagcccctctacatcttcgacctggacggcacgctggccaccatcaaccaccgccgtcacctggtggagtccgatcccaagcagtggcgtgagttctatgccgcctgcgaccgcgacaccccgtgccaggcggtgatccgcaccgccaacgcgctgtacctggcgggcgccgacgtgtgggtctggtccggccgctccgacgaggtggcggacaagacctccgcctggctgctgaagcacctgccgtggctgcgggagcacgaccccttcaatagcatggcgctgcgcatgcggtacgcccatgaccaccagccggacgtgaagctcaagcgcctgtggctctcccagctgaccccggacgatcgcgccaggctcgtggccgtgttcgacgacaggaagtcggtggtggacatgtggcgggccgagggcgttccctgcttccaagtcgcgccgggggacttctgatgagcttccgtcccatgctcgccgcgtcgatcgacgacgtcgctaagctgcgcttcccactgcagacctcgcccaagctcgacggcatccgctgcatcgtgcgggacagcgtggcggtcagccgcagcctcaagcccatccccaacccgtttgtgcaggccgtgctcggccacccgttgtacaacggcctcgacggggagcttatcgtaggcgacccgaccgatccgatggccttcaacaacacgacccgcggggtcatgtccaagagcggggagccggacttccggttccacgtgtttgacgacgtgacccacccggagatgggcttcaacaagcgccacgacgaggccagccgcagggtgatggccctcggccggccgtgcgtagtggtgccccactgggaagtgcacacaccggaggagctggtgacgatcgagacgtccgtactgggcgaggggtacgagggcctcatggcccgtgacgcctgctcgccttacaagttcggccgcggcacgctgcgcgcccaggacctgctgaagctcaagcgcttcgaggatggcgaggctttgctcctgggcatggaagagctgatgcacaatgccaacgaagcaaccaccagtgcactggggcttactgagcgcagccacagcaaagacaacctgctgggcatgaataccatgggcgcaatgacagtgcgcgcgttgaatggtatcttcgaaggcgtggagttttcgattggcactggctttacctctgaccagcggaaagacctgtggagtcgtcgccatcaaggcttgaacggccgggtggtgaagtacaagtggttccccggcggtagcaaggacgcgccgcgcttcccggtcttcctcggattccgggataagatcgacatgtgacgggacggaggtcgctggctcacaaccagcgacctcctgggctaccatcgcgagcatcagctcacaactagcccaaggaacccgcgatggccgacggacccagcaagaagccgacggtagccacgccgtccggcgcttacctgcgcatgcagccccggtggaagatgatcgacgccctcttgggcggcaccgagaccatgcgcgcggccgggaaggagtaccttccccagtacgacaacgagtcgaacaagaattacgagacccgcctggagcgggccgtgctgctcaacatgaccgagcagacgctggacaccctagccggcaagcccttccgcgagcagatcgtcctgggcgacgacgtggcggcggacttccaggacatgtccgaggacattgacatgcagggcagcaacctgcagtcgtttgccagggcgtggttccgggagggctgggccaagggcctgtcccacgtgctcgtcgagcaccccacaccggaggagcaggtcgacgaggccggcctgccggtggcccgaacgctggccgatgaccggagccagggcctgcgcccgtactgggtgcacatcaagcccgagtgcctgatcgctgcctatgccgcggtggtcaacggcaaggaggtccttacccacgtccggatcaaggagacctcggtcgagcgggtaggctgggaggagatgctcgtggagcgcgtccgcgtgctggagccaggcatctggcaggtctgggcgccggacgagaagggcgaagagtggcacatcgagtccgagggcaccacctccctggacttcatcccgctggtcaccttctacgcgggcaagcggtccgggttgatggagtgcaagccgcccctgatcgacctggcccacctgaacgtcgagcactggcagtccaagagcgaccagcgcaatgtgctgaccgtctcccgcttccccatcctggctgcggcaggcgttccctcggaccagaagatcaccgtggggcccaacaacttcctcaccaccgaggacgtgcagggtaagtggtactacgtcgagcacaccggcgcggcgatcgccgcaggccagaccgacctggagtccctcgaggaccagatggccacctacggcgccgagtacatgcgcaagcagccgggtgacgagacggcgaccgggcgagccctggactcggctgagagctcgtcctacctggcgtccacggtgcacgacttccaggactgcctcgagcaggccatgaagtacacggcaaactggctcggccagggcgatggcggctctgtacaggtcgactccgacgtggaccttggcgaggccgacgctgctgagctggataccctcaacaaggcccgcgcccagcgggacatctcccgcaagacctacctcggcgagctccagaagcgcggcatcctctcggacgacttcgacgaggagcaggacgccgagttcctcgaggaagaagccaagaacacgatgggtgacatgttcggcggcggcaacggcaccggcctgcccggtcagcagcccccgggcaaccagccgcccaacccccaggacccggcccaggccgaccacccccaggacccggcccaggccgacccgcccaccccggatgacgagtgatgcccaagaccgctaacgaggagatcctcgacgcgaccgtacgccaccagatcaagctgctgcgcttctcccagggggaggcccagatggcggcctccctgcttgcagagagcgacgccgagcttgtggccctgctgcagtcaaagctcaccgagacgtcggaggcccgcatcaggggcctcctggcggaggtgcgccggatgcgcaccgcggtagctgagcgcatccaggtggagcttgaagaggacatggagggtctctccaagaccgaggctgagtgggaggtctcgatgctccagggagcaacgccaatcgccctttccttcaatgcagtgcccgccacggtcgtcaaggccgtcgcgggctctccaataaacggtatcccgctccaagggtggctgggaaagatggcgaccaacgacgtcgcccgcatcgagcagcagatccggctgggtgtcctgcagggcgagaccatcgaccagatggtgcgccgcatccggggcaccaaggccgccggctacaaggacggcgtcctggagacgacccgccgcgaggcggagatgatcgcccgcacgtcgactaaccacgtgtccacggccgcccgtcaggctacgtgggatgccaacgccgacgtcatcagcggcgtccgctgggtcgcgaccctggacggccgcacctcccctgtctgccagagccgggacggcgaagtgtaccccattgacaagggcccgcgtccgccagcccaccccaactgtcgttcgacggtggcgccggtgctgcacggtgaggagatcatgggcgaccggcccacagtgaccgacacccgcacccgacgccagcgcgagatcgacttccgggcggaggccaaggaggcggcgggcgacaactggaagaacatgtcggcggctgagcgcaacgccgccatcaaggcgcgccgcgacaagtggggcgacgagaacatcgggcagacccccacctcgaccaactaccagtcatggctgaagggccagtccaaggagttccaggacgacgtgctaggcaagggcaaggcgcagctcttccgggacggcatgccgctggagaagttcgtcgacgagaagggcaagccctactccctggcgcagctgaaggccgagctggagggcgacaagcttaacgtcatccagccaggcgtaggcctgaaggccaagtcgctcctgcagcagggcatgtcacccacccaggtgctggagcagatcaagcaggagttcccggacgcgtccacctcggccgcgtcgattgcctcctacaagtctgagctcaacaaggccggggcgttgaacctcccgtctgcgggccaggtgcccactggcgccctcaagcaagccaaggcgatggccgacgtcgtctccgacctggacgcctccctgccatccaacctcaagcatgccattggtgaccagtggtccaccgtcgtggacgacctcgatgggtcgcccggtgcctacgggtactaccaggctggcaagggcgtcgtactgagcgggaaaaagctgtccgcgctgccggccgtacaggccaagcaggtcgcggcccacgagctcggccacttgctgcacaagcagcacgagctgctgctcgacccggacgtcctggcgaccgtgaaggcctcggcaaaggccctgtcgccggatgctcgaaagctctattcgtactacctgtcgagccctgacgagcttgtggctgagatctacggtcaggccctgagcccgagcgccatgacttcccagggcctgtcgtccctggagttcaacaaggccttcgggcccgccatacaggcggccaaggacgcgatggccaagaagttccctgctcccgcgttgtccgccaaggctcctctgcccggcgggcccgtgctgccctacgaggtagctggcaagcacacctcggtcgggtcgctcgccaaggcgctcctgcagcagggcatgccggacgagcaggtcctcaagtctgtcctggcggagttcccgggggcacagaccaagcaggcctcgatcgcttcgtacaagtcccagctgaagaaggatggtctgctgcctaacaaggcgtcgggccctgtcgttacggcaaagcccatccccgacgtcgtgccggtcccatcctctggcgcgtccgccgtcgtggcccccgaagctgcggccgcctccccgtcggccctgacgctcacctcggcccagctcaaggacgaggcgatcaagctcatgcagaagggcatgctcggcaaccaggacctggcggagacgctggctaagcagttccccgccaacgctaaggacatcaagaccaccaacattgccacctggaagtccaactggaagaaagacagccccaactcctacgcccacgcggtctcgctgtcggagaaggccacggtgaaggaggcactgtccggcccggtgcagaagcccaagctggaaggtcagaagctcggcgccacgtccatgaacgccctcaacaaggtgaagtcagtcctggcggccggcggcaagccccaggacgcctacgacgccatgaagtcggtgttcggcacgatccagcagcccggtgcggacgacctgctcgagctggcccagtaccaactggctaccgccaaggcggccggcaagccctacctgaacgcgaccttccaggcgcccaaggggtttgtgccggacgccaaggtcgaggcctaccttgcctcgctggacatcaagggccagctggcggtagaggcctacaagaaggccctgcaaactggcctcggtccggtcaacaccaacaagctggtgaagaagaccgcaggctacgagccgtcggcgtccgctaaggtgaagatgaaggaagctgcggcctacgagctgaagaagggtaccaccaaggcggccccgtccgcaccgtctgcagccaagccggcgccagctgcgaccgacatgaccccggtcaggccggcctcaacgccccgcgaaggtctacccccgccgccgcgctactcggcggagcagcgggcggcgggcatccgcaaatacgctggtggcgtgtcgaacagtgtgaccgagtccatcaacgcgaagcagcgggctgccgggctgccagagctaacgatggaggaagccgcggccattcgagcgtatactggaaacacgtaccgggcgctgaatggcgcgctccgtgggggcaagtactcctcggacccgcacctccaggcgtacgtggatgcggcccagcacggcatggccaagatgcccaagtacaagggcctcagctcgcgaggcatgtccttcaacgagacccagctgaaggcgatgctgtcgacttaccgcaagggggccgtcgtcgaggatgctgccttcgtctcgtcgtcctacggcgagcaggcagccttcggtggcaacgtgttcatgaagatcaacggaaaaacgggcgtgaacgtctcccagtactcacagtaccagggcgagcgagaggtgctgttcatgcccggcacccagttccgggtggacgacatccagcagatcaacggcaagtacatcatcagtatgacggaggtgtgatatggcagaccccctggaagcggggccggagtgggagggcaagatgtccttcgctccgggtgtaccggaggaccccgacgcaataccggagctgttctaccaggtcctgctcggccgggtgtataccctgacccggtggaaggacggctccacggcccgcggcgaggtgcagctggccgaccttgaggccgtcgcgggaggcacgataacccgggagggctggtatgatgcgctggggacataccttggcgcggagctcccgggctccctgtaaaacaggcccgccgcaatggcgggctttttacttctgcttgaacgctggctcgcgtggcccggcgccggtgataaggtgccagcctatacaccccgggcgcgacgcccacacagccagcgcgtgatgcgcagaaggagagtacaatggatttcgagttcctgaagaaccccaccgtcgattcgatcgacaaggtcccggaacagttccgcggcttctacggtgagggcgagggcggctacgtcctgcaggactcgttcaaggccaccgccaccgcggtcgacggcctgaacaagtcgctcaaggcggcacgccgtgacgccgacgaggccaagcgcaaccgcccggacctgtcgggcttcagcgccatcggccagctgctcggcgtcgagggcgacgatgcgacaaaccccgagaccctgcgcggcgcggtcgagaagctgatcggcgactcgaaggacggcaaggtcaactgggagaagatgaagcgcgacctggagggcggcttcaaccagaagctccagttgaaggacggcgagctgcagaccatgagcaagtccctccagaagtacctggtggactcggccgcggtccaggcgatcgccgcccacaagggcgtgccggacctgctgctgccgcacatcgccgcccgcaccaaggtggtgcgtgacggcgaggactacgtggtccgcgtggtagacgagtcgggcgacccgcgtggcaacgcctcgggcggcttcatgacggtcgaggacctggtcaaggagctcaagggtcaccagaccttcggccgggccttcgagagcgaggcgccgagcggcaacggcaagccgccgggctcgggcaaccagaagccggtccagcgccagggcgagatgaccgccaaccagaagatcgccgcgggcctggcaaagcgccagtccggtcgctgatccaactgttgtgcaataagaaagggcgcctacgtggcgccctttctctttacggcagaaccagcaggtcttcccgcaagtccgtcaggacctggccgagccagttggtaccgcgccactcactcgggtcgtggcagcggggatctcgctcgtccaggccgatgccccagatcacgtccgtcgggctggcctccacaagcagggtgccctccgtgagcagcagctgcgctcgcagcttggggtcgctggtgaactttgccaggctggcgcgcatgacgacgtcgcgagacaccgagtcccactgacgacggtcgaagcccttgacgcggcgaccgatcgccttctgctccgccgggttggacgatgccatgatctcgtcgagggccttctcgtccccgaagacccgggccttctgggccatcatgtactgctcggcgcacccgtactcgacaccgtcgatcaccatgggcgaggggtaccactggctgaacaccccgccgtagaacagggtgtagcggacgtattgctgtttcacgggaaaactccttacctatcagggggttacagtgtaccgtcagacgcgcttcgagactgcgggcggcgcgacgggcgcgggcaccttgtgcaccgacacggcctggagcacgaagaacggggtgccggggttctcgtgggccagcttcacggcttgcgcttcggcgtggtcattccggccctgcaccacccgcggcgggttcttcagcgtggggcgtccgtgtggcccgccttccttgtagacgtcaccgttggcgaccacgtagaagcggccgtcgtcgagctcggacgtctcgcgggccgggttccaggtcacggtggcagctttccggccggtcgagcggcccacgacgttgtcgacgacctgtcgacccttgggcgtcaggctcgggggcgtgcgcccgctcggatcgaagtcgatgaggtcgtcggccacgaggaaggtgatgtccggcggcggcaggcccttgacgtgctcggggctggaaaagcccattgccaccgtcaggagggtgcgcaggcgagactccggagacgacgaggtatagcggggcttcggcgggatcatgggattgggattgaccttgacggtgatggcgggaacgggctcgaagtccgaggccacgatgaggtcacggttcacgccgagctgctcgagacggcaggcgatggcatgctcggtgcgaccgtgcgccctcgacagcttggtgaggttgatcttgccggcggcggccaccaggaggtcgcgctcctcgacttcggtccacggggcaccgccgcgcggggccgcggtcgggtgggcggagttgccgaccagcgtcgaccagccgcgcttgacggcgatggcgtgggacggctgacggtagcgcgagaagatgagttcgaacacgccctcggcaaaagcgtcgaggtaatcgtcggggatcaggtacagttcttcgaagtccatgggactctccttggttggacaggttgatgggacatgggcatcatgacgcccaaataggcgacacgacgccactgtttaaggggtattacgaggcctgctgcatgagctccttcgcgcggtcccaagcggcattccacagcacgtggacgtcatcgggcatctcgaagtcgtcctcctcgggcgccgggtcgacgccaaactctttcaaagcggcgtccatcaccatgttggagtcgcaaaagtcgcccgagttgcagacgtcgggattcagctcagcggcattgagggctacgatctttgcgtaatcctcctcaccaacggtttcgcggaggatgcgaacaaaggcgattgccacctgttcgacagtggggagagcccttgaggcttcttcaggctgggagtcacaagagcagtcgccaaagtcgaagcccttcccacagatgttgcacgagtatgcagccatttcggcgctccttaatgaatgagaaagtaaacagtgttgaggacgcttttgcgctcctcttcggagaggttcggccactcgctcagtgaacggacagcatcgatggggccatacgagtcgtacggcaccatatccaacagtccgagcgcttcatgcgcaagacggttaatcttgatgagggagtccgtccacgtctgcgcctcttcgacagttttgaaccaccgaatgggcacattgccaaccccactcgggtgacaatggctaataacgacagcggacatgccgtacttgcgacgggcaagggtcacgacttcgaaaggcggcttcgtgtcagcggacatgggtattctccttattagagctttttcagctcaggggcttccgattgcgcatccgacatgcagtagcagtgggtacgcttgacacgaccgtcggccgtgatcgccatgatgggcgattcgtcaccgagggtaggatgctcgtacagatcgacgccggcgacagtgccgaagtacgtgggattctttgcgaggaaggcaatggccttctcggtggtgggcttgttcatgtctacctcagaggtggaacatcttgagttcgtcctcagacaggaggacggagtagggcgttgcatcgcccgcgatttggaaccacgctcggccctcgtcgacggacgtgagcccctcgagcggtttgccatgcaggcggcgggcctcttcgaacaggtcgcgccacagttcccggttcatcggttgccgagggcaggcctgtcggtatcgcggggccttgatcttggttgagggcttacggtccatctgtttaccaggttgccgtggtgtgagtccattatacggggtcttttgggacatgggagcccctttaagaactatttttattctttttattagatataaagaaataagggtatctaaggcagtcttaccctcttctaaggcagtctgaccatctaagtccttgtcgcagctaagccatctaggcttctaggccttctagggctgtttctcgagccgtggccggacctggccgacaggctgttttcctggtacaactgcgcgccgaaggctcgttcaggctcagaactgacctaagtccttggtccgtaaagctttttctcgtctgaggcggctcctggaaggcccgaaaggctcggattctcgcgctggaccagcgttcagggggttacgagctcgagacgtcacgacaaactcccgaaccatagcgcgcgagcacggtcataacacccggcccgcgctcgctgaccctgcaaaggcgtgatgccttggccaggggtcgaatcgtcgggcgatccggcacctcccaagcatcccaccacccgccttacaggagatccctaatggcatccgttaccctcgccgagtcggcgaagctggcccaggacgagctcgtcgctggcgtcatcgaaaacgtcatcaccgtcaacgagatcttcgagcagctgcccttcgacggcatcgacggcaacgccctcgcctacaatcgcgagaacgtgctgggcgacgtccagatggctggcgttggctcgaccatcaccgccaagaacccggctaccttcacccaggtgacctcgaccctgaccaccatcatcggcgacgccgaggtgaacggtctgatccaggccacccgctcgggcgacggcaacgaccagaccgcggtccaggtcgcctccaaggccaagtcggccggccgccagtaccagagccagatggtgaacggcgatggcaccggcaacaacatggccggcctgttcggcctggtcgcgggcagccagaccatcaccgccaacaacggcgcggccaacggtgccggcctgtccttcgaggacctggacgccctgatcgacctcgtcaccgacaaggacggccaggtcgactacctgatgatgcactcccgcacccgccgcaagtacctggcgctgctgcgtgcactgggcggcacctcgccgggtgacgtgtacgtcatggcctccggtcgttcggtcccggcctaccgcggcatcccgatcttccgcaacgactggatcccgatcaaccagacccagggcacctcggccaacgccacctcggtgttcgccggcacgttcgacgacggcagccgtacccacggtatcgccggtctgaccgccgagcgccaggcgggcatgcacgtcaagtacgtgggtgagaaggaggatgccgacgagagcatcacccgtatctcctggtactgcggtctcgcgctgttcagcgagaagggcctggccgtactgaagggcgtcaccccgggctgatcccagccagggtctcagccagcccgccggcctagtgccggcgggctactaataggagatcggaaacatgagtgcacatctcgtacgcctgagcgggtcccgcggcgggcagaccctgtacgacaaggccgacgcggtcatcgtctgggtcgaggacgactcggtgacccagcaggcggatgcgcgggctgcggctgcggccgcccggcctggcccggatggttactgggccgacgctgtcgtcctggagctgagcgaggcgaacctcgcgaccgccattccggtgaagagcatcacctgatccatgagcctcgccggtacgccggcggggcttcgtggtccatagagcaagagaaggagagcccagatgtcccacaagttcgtactggtcggcccgcatgcgggcaagaccatgaatgtcaacggtcaccagttcgaggacggcgagttcacgttcgtcggcggtgacgcccaggcggcagtgcttgcccgcgtgttcgagttctacggcgccctgccggccgacaaggctgagctggtccgcctcaagggccgtgagcgcgagccgggccgcggccgcaaggagctggaccaggccatcgccggcctgccgggcgagcacaccgacgccgactacgtggtcaactcgatgcgcagccactggggcgacctgttcaccgccggcgacgagctcatggtgcgcgaggtcgtggtcaagccggaaggcgacaagaccgatgccaccgtcggcgaccagaccaacacccagacccccgagccgcccaaggcgccggtcatgccgagcctggctgaagccatcggcctgctggacccgagcgacgaccaggactggacgtccaacaacctgccgaacctggagcgcctcgaagccctgaccggcaagaagccctcccgcgccgaggtcgaggcgatcgctgacggctacacccgcgccaaggcaaaggccgccaaggcctaagcaaccagagaggattgacaccatggcattcaatcagcaggacaacgacggcacgatcgacggcgccaacgcgtacaccgacccggcgaccgtcagggcttactggttggaccgcggtgtcgacctctccgccaagacggactccgagctccaggtagcaatcgtcgttgcgacgacctacctggatgctcggtactcctggactggctaccagctacgtcgactgcagggcacccagtggccccgtggcggcgtgacctcattcttgcgcggcctgccgccggccctcactacggccgtgtgcatggtcgccaaccgcgccctctcgggcaagccgctcatgccggatccgacgactgatccgagcggccaggcggtcacccagacgaccaagaaggtcggaccgatcgaggtatcgaagacgttcgccgagagctcctcgagcaacccggcggcgaccgtacctcagtttccggaggtcaccatgacgctgcagcaggccggcctgatcctgtcaggcaactctggctccctggcgcgaggctgacatggcaacctttgactatgctgacctcaagacggaagtcgacgagctgctggccgagttcgggcagagctgcatcctgcgtcgcccgggaggtccggttgtcgtcgatcccgtagagggcaccgtgacgccgggcagtggcccagtggacttcccggtgctcggggtcatcaccgactactccgaccgacagatcgacggcgacaatatccgtcggggcgaccgcctcatgtatatccagggcaacgaacgcccagagcagggcgacgtcttcctggaggcgaacggcacccagtgggctatcatcgattttgactcggttgacccggccgggttggccctggtgtttgccctgcagctccggaggtaacgtggcaaggttccagcagcagctcaaggggttcggcatcaagaccctggacaaggtggacaaggtccgccgggcctcggtgctcgagctgttcaagctggtcatcttctcgaccccggtagacacgggcaggctccgcggcaactggcagacgaccatcaactcgccggccggggcagcaattgaccggctcgacatgggcggcggggcggcaatggcggaagcggtcgccaacctggggtccctgacagacgtcatctggttcaccaacaacctgccgtatgccgagcgaatcgagtacgacgggtggagcaagcaggctccagagggcatggtgcgcaggcacctagcctcctggaaaaggatcgtggccgccaaggcccgcgcattttaacaggggaatgagatggcagttaacccgtacagcggactcaacaaggctctgatgcagggtgtcaaggactccccgctcgccctgccgtacgccgtcgagaatgcccccttcaacaagccgactgaccaaagcccctgggccaaggccttcgtgctgatgaaccagccttccgttgccaccctcggggcggaaggccaggatgcccatgacggcatcctgcagatcgacctgaactacccactcaacaccggcgaggcggccgtgacggccaaggcggacgagctgtcggacttcttcaaagcgggcaagcgacttgcccactcaggggtcgagctcacggtggcttcgtgcggccgctcacgcgggcgcgaagtcgatggctggtaccgcgtgagcatgaccgtcacctggttcgcccgggtctctcgtaactaatccacagtaggagcgtaccaccatggcaaacggcagccgccactccatgcgctacgtcgccgagaccgtctacggtcagactccggcgacccccgcgttcaagcccatccgccacacgggcaccaccctcggcctgtccaaggagtccctgcagtccgaggagatccgcgacgaccgtcagattgccgacttccgccacggcgcgcgccaggtcggtggggacatcaacttcgagctctccttcgagagcctggacgacctgctcgaggccgtcaccctgggctcctggcttgccgacggcgcgccgggcggtgacggcgatcgactgaaggccggcacccagcgccgctccttcaccgtcgagcgcttcttcggcgacatcgccaccatggacaagccctaccaccgcttcaccggcgtcgagatgaataccctggcgctggcgatcagtgccaacgcgatgattaccggcaccctcggcaccgtcggctcggacatgagcacggccaccgcgatcatcgccggggcgacctacgccgcgccgacgaccacctcgccgctggactcgttcaccggcaccctgaacgaggccggcgtgccgatcgccgtcatcaccgagatccagctgaacctggagaacggtctggaggcgcgcttcgtggtgggctccaagaagtcgatcctgccgtccatcggccggtccaacgtctcgggcaccatcaccgcgtacttcgagaactccctgctgctggacaagttcatcaacgagaccgagtcgtccatcgtcttcgagctcccggacggcgccggcaacaagtacgtcttcaccctcccgcgcatcaagtacaacggcggccagccggacgtcgagggcgaaggtcccatcaccctgagcatgccgttccaggccctcctggacagcacgacccagaccaacatcatcatcgaccgagtgccggcataaccatatgaacgagaacaacaccaccgcgggggcggcaggcatgaacgagttcttcacccgaggcaaggccaacgaggggatccaggtccccctgtggcgtcccgacggtacgaagagcgagcactgggtgcgcatcctgggcatcgactcggacatcttccgccaggcggatgccgagtcgcgccgcgaggccatcaagatcgcacagctggacagccaggccgagaaggtcgaggccatcgcccgtacgaagcgccgcctcatcgcgtcgctcgtgacggcctggtccttccctggcgaatgcacgaccgacgctgtcgagcagttcttcatcgaggcgccccagatcatggacgccatcgatacggccgcgagcaagcgatccctttttttcgcgatcgggtcgagcaactcgcagccttcgccgagtacgagttccgactcgacctgatccccaagggatcgaagcagaccctgcgtgactccctcatgcaggtctggaaaacgctgaagcgcaagccgcctcagctggcagacgccccggagctccccgaggagctccggtatgtctgggagtggttccgggaagtgttcgcggctgagccgctgacgtatgccgagctgcaagcttggtccagcatgacaggcaagagcctgaagggctgggaggccgagctcatcaagtccctcgaccgcattttctggaaggtgcagaatggcaaccgacgtagctagcctagcgatcaagatcgagtccctccaggtccagcaggcggactcccgcctgaagggcctggcctcgtccggcggcaccgccgagaaggccacctccggcctgatgggagcattcaccaaactgctggggccgcttgctgcggccgtcagcgttatgggcaccctcaacaagctgatggatgtccagcgccagttcgacgtactgaacgctggcctcatcaccgcgacgggctcctccgagaaggcggcaatcgccttcgacgccctgagggagttcgcccagaacaccccatacgacctgaaccaggccgttgagggcttcaccaagctggtgaacctcggtctcgacccgagcgagaaggccctcatgtcgtacggcaatactgccagtgcgatgggcaaggacctcaaccagatgatcgaggccgtggccgatgccgccaccggtgagttcgagcgtctgaaggagttcggcatcaaggccaagcagaacggggaccaggtgtccctcacgttccgcggggtcacgacctccatcggcaacaatgccgccgagatcgagaagtacctgaccgacctgggcgagaatgagtttgcaggcgccatggagacgcgcatggactcgctcgacggcgccgtggcgaacctgggcgacacctgggaccagctgtggctgaccatcagccagtccggcatcggggacgccatcgaagcctccgtgcgcacggcgaccgacgccctgcaggagctgaccgacatgatcgcgtcgggccagatggaggcgctgctcaagtcgcagactgtgcagtgggaggtatggggcaaagacattgaggagtccatcgacattgtcacccagttcatcaaggacaactttggtgaatgggaggacgagggccagtccgtggtggacttcctgatcgacgccttcaagcagctgccgaccaacctccgggccatggtccagatcctgaccgtcgagttcgcctcgggcttcgaccgcatcatcgctggcgccgagttctggcgcgacacgatgaaggcgatcttcagcgataccaccatcgctgatgccggcaggaagtgggtctccgagcagcagcggatctcccaggtgcggctcgattccatctcgggcatcatggacgagcgcgacgccacgctcaaggccagcgaggaccagctcgccgccgccaagaagcttcgcgaggagtacgacgccgcacaggaggccaagaagaaggccaatgctggcactgatcgactggcccagttccgcatcggcgccgacaaacccaagacggcgtcctcgggggtcgacaaggatgcggcccgcgcacagaagcagcgggagcaggagttccagcgggtcaaagatgccctgcagaccgaggaggaggccatccggtcgtcgtacgagaagcggaaggctatcatcgaggcgaacaccaaggtcggcaccgaggagcgcacgaagctcatgggtcgcctggatgccgagcgggacaacgagctgaagaagctcggtgcctacggcaactctgagctggagcaactgcggcagtcactgctgaagcaagaggacgcgatcaaggagtcctacgaccgccgcatggaaatgatccgtgcaaatacggaggagggctccaaggcgcgggcagagctggaagcgcaggtcctcagggatcgcgacaaggccctggccgacaccgagcggcagcgccagtccgagcgggacagcctgtacaactccctgcttaccgaggaggaggccctcaagcagtcgtacgagcggaagaagcagctcatcttggagagcgagtcggtcaccgagctggagcgccaggatctcctgcgccgcttgcagaagcagttccaggacgagcaggctcagatggaaaaccagcgcatccagacccagctccaaggcgctgccgccatgttcgacggcctggctgggctggcaaagggttacgctggcgagcagtccaaggcctacaaggtactattcgccgtgagcaaggcgttcagtgtcgcccaggctgccatgtccatctcgaccggcctcgccaaggcccaggagctgggcttcccggcgaaccttgccgagatggcccgggtcgccgcgaccggcgcgtccatcatctcccagatcaacggggcccagtttgcgggcgcctacgaccagggcggccagattccggccggcaaggtgggcatcgtcggtgagtacggcccggagctggtcaagggacctgcctcggtgcgcgggcgcgagctgtcttccaggtcctacccggacggtggcggccagcaggcatcggctgcgccccctgtcgtgaacgtcaggaacatcaacgtgctcgatccgaacctggtgggagactacctgggcacggacgagggcgagaagctcatcatgaatgtcgtcaaccgcaacaagagctcgctgggctactgactaggagaagattagatggccttcgtaacaggcacggccgccaaccacgtggacgcgctggacaagctgcgcctgttcctgaccagcgacgacgccctgtcgtcgcttggtcagacctgggcccagctgcggtgggtgcccgacaacgtggactcggtcgacaccaatatcccgttcggctcgggcgtccagctgccgcgcctgttccggccggactaccggacccagaactacacctcggagaccagcagccagtacctcagctcaacctcgttcacctccgggcagtacgtccgcctgaagatgcgcgccgccaaggcggtgaccaagttcaccctgaaggcaggcaccggctcgagcctgacgaactataccccgcgcaacttccggctggagtattccgacgacgggtcgacctggtcgaccgccgtcacgctgaccgatcagcgggcctgggtggccaacgaggaacgcaccttctcggtgccctctaccggcgagcatctgtggtggcgtttggtcaccttgcagaccggcgattaccagggcacgctgaccgggcagtactgggagctgcgctccatctggctgtatgacggcgacgtcctggtgtcctcctcggagtccaacctggtagtcaagggcccaggcctggcaggcgacgaggagatcttccttgccttccgtaccacctacaacaccggcaccggcgagtacgccatcctggtacaggggctcactggctatctgccggctgaacagtccctgcacaagcagcccggcctgcacccgagcggatggccggtggtgcccctctggtcggcggccatgccgtactggttcgtcggtagcggccggcgagtggtcttcgtgttcaaagtgtccaccgtcttcgagtcggggtacgccggattcttcctgccgtacgcctctccggagcagtacccctaccccctggctatcggcgggtccatgtcgcccgcgtcgtcaagctaccggtacgactacgtgtcggcggcgcacagctgcttcgtcatgcccggcggaaataccggcaccagctcaagcgtggacgtggtgtacaacaccaccctcaacgtcatgctgcccgacgggagctggttcgacttccagaaccggcccacgaccagcagcaacaactccgagagctacctgacctggaataactctccggccagtgtgctgccacacggcaccttcaacgacaccaccacctcgggctacggcttccgcgagaacattggcgggggtttctcggtcttccccgcgacgctgttccagcggcgcacggccggccggttcctcggcgagctggacggctgtttccagatctcggggttccagaacggttccgagaacaccggcaccatagcgggcgaggactacctcgtcttccagaacacctaccggaccgacgtacgagagtactgggccctcaaggcggagtaacagagatggcatacgaaactggcgccgccacgagcgtgaccgacctgctggacaagctccggctcttctgcattgccgcgggctggactgtcaaccggtgggatgatccggcaatcacccgccgtctcaacatgcagaagaacgggctgtttgccaacctctgcgcccaccagggcaccacggcgctgaacgacaacctcaacggcttcaccaaccagagctcaacgacctattttgccctggcggtcagcatgtccgacggctatgaccccgacgccaccggagcgttcaaccagcccggggctccgaagtacaacggatacccgcgcggggcactgctttcgcagctgaccgcagctatccccgcctaccacttcttctcttactccgactccgacgacatcctcgtggtggtggagtaccgtaccggccgcttccagatgttcggcttcggcagtttggccaagttcaacgtcaccgctccgggtggtgcatggtttggcggtggcagcccaagccccaactgggcctactacgagcagagcgggtacggccccgactcgagcaaccagaacgagctcatcccgttccgcatggcttaccagcgcggatccgattcgaccagcttcctgcgctgcaacgtggattccaacaatggctgggcagcttcccggtatattgcggatggttcgaccatgggcccgctggccgccatcggtcaggctttctacgacgaggagctccgccgatacacgccaagcgcactgggctggcagacctcgctgatgcgccagaccgtgtacgtcgggcgaggcaaccagtttgcctcgccatacggtgagatcaagcacatgcgccgcctggagatcacgaactacgtgcctggcgacgagttcaccctgggctccgacacctggaaggtcttcccctaccaccagaagggcggcccgaccgagcagcgcgggtacgccctcctgaaggagacctgatatggcagtcatcgagatgaccggcgtggtgcgctccgtgacgcccacgccagtggcctcggctctggacacttcgatcaccctggggggttggacctacccctggggctttcctattgtggaaccgggcagcaataaccccaagcagggctctttcgcaactccaccagccgtggccgtgtccgcccctccgtctttctcggtagccagccgcatcggcggcttcgtggacgacctgtactaccgggtccacgtccggccgggcgtgctcgagctgggcaacctgctgtccagccagacccgggccatcgaagtctggaatgcccacttcgagggcaagaccctggaggcaatcgacgctgaaggcctggacgggattgtgctcacccagccggaggtgccaccgaccacgttcggtgcactggagtcccgcatctaccaggtcagcatctcgaccaacggcgccccgacgatcgacggtcggtacgtctttgacttcggtgacgaggagcccaccctacgcatcaccggccggcgcgtcgtgctctggcccttcattccccagaccaagttcagggagtcgctggagtggcagactgacttgctgcaggcctactcgtccgagcagcgcctggcgctccgcacggcccccaggcagcgcttcctgtacgagttccagctcctgccgcagcagtactccagggccaaggccatcagcacccagtgggcgcaccgggtctacggcgtgccggtctggggcgagctcacccggctcggccagctcctggagggtcaggcatccctgaccttcgacgcaaccagcgcggactaccggaacaacgacattgccctggtgtggcaggacgacgagaccttcttgacgatcgagactgtaggtgccagtgcgaccggcctggagctgaaggtgcccctgggacggtcgttcgacaacgcctacgtgatgccgctccgctacgcgcgcaccctcaatgggaccgagttcacccgccgtccggacgacgtcacgatggcccgcctggagttcctggttaccaacaacattgacctgggcgcgtcggtggggctgccgcagtaccggggcaaagacgtcctcatggaccgctcggtcacactgtccgacctggcggagaagatcgtgaggcctgtcgatcagttcgacaacggctcaggccccatcacggctgacccgcagcgtggctaccccgaccggacggagaccctgggtctggacgccttgtccagggcggaggcgtggcggtaccgcacctggctgcacgcccggcgcggcaagcagaagggcttctggctgccgggctggaaccgggacctcctcatcctggcgaacgtcgactcagccgcaaccagcatcactgtgcgcccgatcggctacccgctgtactacggaatctccgacatcatgctcgtgctgaccgacggctcggtgttctacaaccgagtgctgtccggctcgaccgacacggacggtaacgaggttctgtcgctcggtggcggcttcggcagaagctttgctgcgtccgaggttgacctggtgtgcttcatgcgccacgtgcgcctggacaccgacagcgtcgagatcacccactcatacgcgggccgctgcagcagcacgatccccgtcatcgaaactcccgagggattctaatgagttacgcaacgatcgaggcatcgcgggagcagggcgctccggtagagctgtacgagtttacgcaggggctgcagcgctgggcctttgcctcgggggcctttgaagtggtgcgggacggcgtggtttacaagccgtccagcatccgccgtgaccgggtaaagcagtcgacggacatcttcaagaacgggatcaaggtcaccttcccccgggacgacgagttcgctagccagttcctcggcttctccccggaggaggtcacctcgcttaccatctaccgagggcactacggcgaccccgacagccagtttgtgatctactggaaaggccgcgtcctgagcgccaccggcggcgactcggccgtcgacctggagtgcgagccggtctacacctccatccgccggccggggctgcgcgccaagttcgagtacggctgccgccacgtgctgtacgggcgtggctgcggggttaaccgggaggcctacaggcatgacggcacagtcatcggcatgagccaggggctcaacgtcgtcgtgtcgggcgtcgagggccagtacgaagacgggtggtttgccggcgggatcatcgttgcccccaacggcgcgtctcgcttcattgtcagccacaccgggggcacgatcgtgatgtcccgaccgctggccggactcgctggcgaccaggcggtcaagctctacccgggctgcaaccacctcaagtccacctgtgccgccaagttcaacaacctgcccaacttcggcggcttcccgtggattcccacgcgcaacccgttcgacggaagctccatcgtctgagaggttactagcatgatctggtggtatatcgtagtcttcatcgtggccctcgtggcgtcctacgccatgatgccaaagcccgagaacgcccggcccgccgggctgggggacatcacggcgccgacggccgaggtcgggcgcgcgatccctgtgcttttcggggagcgagacctgaagggtcccaacgtctgctggtacggagacttccggaccgaggccatcaaggctaagggcggtaaaaagtgacagagccccgccaagcagtgcggatggaacacatgcgccggttgggctactgctcttccggcgttcgcacattcttccagcgcaatgggctggactacagcgccttcctccgggacggcatcgacgcagacaagctggcggagaccggggacgccatggccctggccgccgtagaggagtccaaaaatgggcggcggtaagaagcagaccatcgggtacaagtacttcctgggcatgcacatggtgctggcccacggtccgctggacaagctgaccgagattcgcgtcgatgacaagctggcttggaagggcacgtcgactggcgggcccatcatggtctgcgcacccaacttgtttggcggcaaagagcgggagggcggcgtaggcggcttcctcgatgagatattcaacaagctgtacggggaccgcatcgacccgcctctcaacccgggcaccctgcaggccatgagcgccggcaccattgacgtcatgatgggccgggacgaccaggcgccgaacgcctacctgtccggccagctcggcggcgccataccggccttccgccgtgtaatgggcgtcgtgctccgccgctgctacctgggtaacaacccgtacctcaagatgtggtccttccgggcctcgcgcatccacacccgccagaacggcattgagcagtggtacgatgccaaggcggagatcgcgggcgacatgaacccggcccatatcatccgcgaggtcctgaccgacccggactggggcatgggataccctgaaggcgacatggacgaaaccgcgttccgcctggccgccgaccagctgcactccgagaatatgggcatgtccctgctctgggacacccagcaggacctgagcgacttcctggccatcgtgctccgccatatcgacgggtccctgttcaccgaccgggccacgggccgattcgtgctcaagctggcgcgcggcggctacgacgagagcaccctgctactgctggacgagcaaaacgtcatccgtgtgtcggacttcaagcgccgcacggtggacgagctgactaaccaggtcagcgtgaagtactgggagaagtccaccggcaaggacggctccaccactgtgcaggacattgcgcttgccgccaaccagggcacgacggttggcacgaccatccagtacccgggtttcaccaacggcaccatcgccacgctggcagcgtcccgcgacttgaaggccctgtccatcccgctcgccaccgccacgctctacgttacccgcgcggcggcgctcctgaacattggcgacgtcttccgcttctcctgggaggagtacgggatcgagaacatcgttttccgggtaaccaacatcgagctgggcgaactgcagagcaaccagatcaagctctcagtcgtcgaggacgtcttctcgctcacctcggcgtcctatgcgcccccgccgccctctgaatggcagccgccgagcggcgacgcagccccgtccccgtaccgcctggtcatggactcgccctactacatgctcgtccgagagattggagacacctcggcccaagcgctgccgaagaccgcaggctacgcgctggccgcaggcgtctccccgggcgggacctcgatgaacatggcaatgcataccaacgctggcgcgggctatactgaccagaccgatctctccttctgcccgacggccgtcatccaggcagcctatagcgacgacccaaccgtcgagaccttctcgatcggcgtgactacagactggaacctcgtgcaggccggcgacctggcggtgatcgggtacggcccctccaacaaccgcgagattgtccagctcaccgtggtatccgacacggaggtcaccgtcaggcgtgctgtgctggactctatcccgcgtgagattgcctcaggtgcgcgcctgatggtcttgggcctcagcggcgagcataccggcatggactcgaccgagtatgcccccggcgagcaggtgtccgtcaagctgaccccttccgcagccaagggccagttgcctctggcgtcggcaccggtcgacgttgtgccgatcctggcccgccaagcccggccctatccgccaggcatggtgcgagtcgatggctccaggaagcccgcgaccgcgtctggtccggtggtcatctcgtgggcccaccgagaccgcacgcagcagaccggcgagaccctgatcggccaggacgcgtcctcggtcggccccgagaccggggtacgctacgggctgaggttcttggacgctggtggactcgtactggttgcgcgcgataacatcagcggcacctcggcgaccggccgcctggcctacaccggcaacgtgaccatggagctctactcgatctcggacgcgggcgaaagcatcaaccgccacgtcaggaccttcgcctacactccggaggtcggcacgaccgagagcacgatcacggcgggcacctggacgccggatgaggtcatcttcgacggaggcggggcctgatggcaaccatcgtaataccacagaggtttgcccagcgccgtgacaccacggccaactggaacagcaaggaccccgtcctctggagcggcgaggtcggcatcctcatggacccaggccaggccgtcaagctgaaggtcggtgacggcacgaagaagtggagccagctcgacttctttgcctctgacggcaagcctgtgcagctgcgtgcggccgatggattcatccagtggaactacgtgggcgatacttcctggatcaacctggtgtcgctggacagcctcaggggcgcagacggtgacgacggtgacgacggggctgacggtgagagcgcctatgagatcgccgtcgacggcggctttattggcaccgtgccggagtggctggcctcactgaaaggcgagcctggtgacaagggcgacaagggcgacgctggcaaccccggcacgccctatgcccgacggatccagcacgtgaccgacaccgacgcaggcacctttgagtgcgactggagtcagtacgacgagatccgtatctccctgaccgccactgtggtgctgagctttactggtgccatcgacggtcagggttgtgtactgaagctgcgccagccgccggcaggcgggtgccaggtcgggctgcctggcggcgtggtccggtttaactccctgatccaggcctacgtcgtgacccagaccgggtccagggcggacaaggttggtttcgtctttgacggcgaagacgcacgatacgacctggtctccattattcccgggatctaacccatggacgactaccagccgccacaggcgctgaacgtgcccttcctgttcgacggctcgtacgacccgccacaggccctcagtgtgggcttcgtgttcggggccgacgggggagggggcaccacagacccgctgccctgcaatttcatgatcctactcaccatctgaggaacacccatgaccgtccgtgtatactccagctccgactccggcgcgccggtgctgaacggcaccactgccggcgacctcatcaacctgctgaccaagtgccttgtcgacggctacggcgccaaggccggcgcgggctggaccaagccctactccggcggcaaccgcgccgcgttccgccagggcacgggcagccgcggtcgctacctgtacgtggacgacacccgcaccaccgtctcgggggccgcgcgggtgtacggcatggacaccatgactgccctcgacacgggcgagggcccgttcccgaccaacacccaggtccccggcggcctgtactggcatgtccactactacggcacggcgaacgtcggcagggcctggaccctcgtcgccgacgagaagatgatgtacctgacgatccacacctatccggacgccgcaacttcgaaccagtaccgggagacctactggttcggcgacctggccggcgcggcgtcgatcgacacgttcaacaccatcatccagggccagagctcgtcaagcgccaactcgtcccagcaccagcccaccgaatcggtcggcatcggcagcgcggtgtcggggctctacgcggtgcgctcgtacacaggcctcggcgggtcgatccagctcggccgccgccacgactataccctgtccggtgccaccgtgtggggaggcagcggcaacctcagctatccccacggcccggacggcgccctgatgctgtcaccggtctggatccacgagcctggcagcaccaacgccgctgcacagcgcggcacgatgccaggcttgtgggccccgctgcagtacgtgctgaacactggcgacactttccagggtgccggtcccctggcaggtaagaccttcctggccttccgccagtatgagtcgcgctactgcttcgagacctcgaacacctgggggacctaaccgtggccgaccttggcgccattggcgcgtcctacgcggtaggcagcctgcgcgccttgggatggcctcccgtaatccgggcctacccggggccgagccggcttccgaccaacatgcctgggtggcacgtgcagtctgccacccagttctatggcggcccgcaggtgcagcccggcactccctcgtggtacggcccgccgaggccgcccggtactgacccaatggccctgtacggcattggcggcacggtcaagcagcggctgaacggcgtggatagccccctcgttggctgcctggtccgcctgtatgccaggcagtccggggtacttgccggcaccgcaatttcaggccttgatgggtctttcgagatagacaacctgctgccaagcgttgccggtttctttgccgtcgcttttgatcccgagggcgcgccggtgcagaacgccctcatctttgacaggttgaaggccctgccgctggtgcccggcgagatcaaggacctggacctgtcgttcagcacgtccggcacggcgtcctaccacctgtcaaccgtctatatcgaaggggctgtgacctatgccgtcacctccggggctctgcctgatggcatcgtgctcaacacctccaccggtgccatcactggtaagcctctgacggctgggccctactccttcaccatcacggctgtgggatcggtgtacggcacgggccaccgggcctggtctggcgaagttacgtccggcctggcatacctgaagacactgcaggggtccgcaagcttggcgttggtgcgctccggtcaacaggacgaagggttcattgtactccccgccctgcctttccccttcagcctgttcggctcttcctaccagaacaacatatacgcctgtgccaacagtttcattaccttcggcttcggcgtctcggtctactccagcttgtcacccaccaaccctggacgaggtctgctgctagccgccgcagaccgttcctggcagacactgcatgccgggtcagtgttgtccgggcagggcttcctggtgcggttcgatggctcaaccggctacgccagttacgacggcggcaacctgtgggaggtgacgttctacgtggacggcaccatcggcgtagtcaccggcaatttccccaccggcggcgtaaccaatatatcggatggcaccagctggcgtagcgatggtgcggccccggtgttcatgtcgaacaaggcataccttggcacgcccaccggcgccggcggcaactacgtctgggaggagaacccgtgacggagcgcaacgagaactggaagtccagctggcgggtacggcgacgcttcatgtttgccgtgtcggccttctgcatgtgggtgatcggctatgtcctttaccgggacctgggctccagcccagcagacaccgcaatcaccatggcattcctgaccctcatcagtatcgtcggatcctacgtattcggcgctacctgggaggacgtcagcctggctaaggccaagctaaagatgccggcagggaataccggcaagcccgccccggcaccaggggcgtcaacgaagatggaggatataccatgagcttcgtactgggaaccaagtcgcgctccagcctgcgtggggtgcacccgcacctcatcaaggtggtggaacgcgccatccaggtcacgtcggtcgacttccaggtctacgagggcctgcgcaccagggagcgccaggcgtcccttgtggcgcgcggcgcaagccagaccatggactctcgccacctgcccggccgggacggtctcggccacgcggtcgacctggtgccgctgatcgatttcgacggggatggcaaggccgagctgcggtgggactggtccctctgctacaaggtcgcccaggccgtacggctggcaagcctcgagctccaggtgccgatccgctggggcggggtctgggaccgcgcgctggccgacctggccgacccggaagatgaggtggcggaatacgtggtccgtcgcaaggcccaggggaagaaggccttcctggacggcccccactttgagttgcccgtcggcaactacccctgaggacaagcacatgattccgttgggatacaagctcggcgctggcgcgcttatcggggtatgcctggtcacggccattgcgttatcataccgtcactactccggccttgtccaggacaaggtcgagctcacggcccaggtcgcaaccctggagcagggcaaagctgccgagaaggcccgggctgacgccctggacaaggccattgacaagtgggacgacgccgccaagatccaggcggacgccctcgaccgattctcaactgtccagcgtgacgctggcgaaaccacgaggaagctgacggatgtcctatccaagcacgacctcggcgcgctcgccaggagcaagccgggtctcatacagtctcgcgtcaatgctggcactgctgatgctttccgcctgctcgagcaatccaccggtggcgcagcccccggtcgaggccaagcagcccccgctgcccgtcctgcccaagccccagtccgtaaggactgagtcggtagagtggcgagtggtccaggtcgacggcgagtccctcttcgccgtcaccgcccgggggtacgaggctctctcccgaaacctggcggacaccatccgctgggccaaggaggcctcctggcagctcgacttctaccgtgactcccgccagccggcggacgatcccaagggggaatcgaagtgaccaacctgcccgggccggatcagcccctgaacaacctcacgagggaggaggcccagctcctcatccgagagtccgtccgggaggtgttcctgatgctcggcgtgaaggtcgacgaccccatcgaggtgcagaaggacttccagcacctgcgcgagtggcgtagcaccaccgagaccctcaagcggaagactctgctcaccatggtaggcatcgtgctctctggcatggtgggcgccgtggtggtgggcatcaaggagatcttcagtaagtgagccccgcggtgggcctggcggttactctccttcctgccaggctaccttccaccgccttcgggcggtggctttttcggaaaccaggtatataaggccgcctcgagcggccttacgcgtctaaggccctgggcctaggccacctcggaagctgcagccggcctggaatgtccagaaggcacgccgtggcagcctcgggcgagcaagaccgagccgactaccaggccccagaacagtacgctaagccccagggccagggtgatgccccgagccgcccgcaaatcgtcgccaccttcgtccagctcgcacatacgaaaatgcctcccaaggatagtccctgggaggcatcatgacgtgacgtctgcgccggtcgacgccgtcagtagacccacacccgctggtacttctcgggcatgcggctgcaactccactccgacttgcggccctcatgctccgccttcgggtcctcgacctggacgcactccttcgagtgccacgagacgtgcactatggggcggtccagcgcgtcggcgaaggacttgattaccagcacccccatcagcaggcaggcgagaacgcagagggcttgagcgaggtagtggcggggcatgtgggtctctccttgaaccgtggccgttactggcgggtggtgggcgctgcgtgggtgggatggggctggtcggcaggcggctcgcccgcagtgatgcggatgtcgccggtgtcggaatcctgggtgatcccaatgaacttgccgccgatctcggcgagctctgccgtcgagacggtcaggcctccgggcgtgcgactggccacgacgccgagcagggcagtcacctgctgcagcttgatttcgtgggggcagacgtcgcccgtcagaaggcgggccagcagttccagcgagtcgttacggttgctgctcatactgtttggtctcccaattgatctctacagaggtggtacccttgatgcggcacttggccacggcggacagcttgaggtcgagcaccttcgcgatcgcgggggcgtcctgcctcggaatgtagcccagcatctgtccgcaggcgtcgtacacggccacggcgttgctgtcaaacttgttggcgcgctcgcggcggagcgtcaggacctcgtcggtcctgagctccagcactgcttcgcgggcgcccttgtggtgcacggagcccacaatgtacgtcctcatctgtggcattacgcctccttcttgggctgggcgcgcgggcggttcggcaccttctcgccgcgctcgcgcatgtggacggcgtaccagcggaggcacgccacagtggtctttgcgccctcgaactgctgatggatgcggtcgagcacggtctcgtaggagtgaccgtaggggcgcttgtcttcgtcgtgggacacgacctcgagcagcaggccctcggcgacctgccgaattacgggccccttctccttcttctccttcggagccttgtccttcttcgccttcgtcttcggggccttgtccttcgtctccgtcatctgcttcagcagcatcgacaagccgttgggctcctccttcgccttctcgatcttctcggacagctcgggggtgggggtgccggcgagctccacgatggcggcttcggtctgcgaagcctccattgcggcgatctgctcgagcaacttgcccttacccctcttcgcaagggacttcgggtcagcttccttgccgctcagctcgttgtggcgggcagcgatttcagcgatattggattcgttggacagggtcatggcattctccgtggacggttggtggcacgacggacgcattgcgcaccgtcgatgggttccattatggcgggttgtgtgggcaatagccccaacatttgggctattgcgcttgaacgatgggattactgaacagtagacttcatgatggcgacgagctcaaggtcggacaggccgttgaggatcttcgcagtggggttcttcttggccaccagctcaaggaactgaggcgtcacgacgccgttggaggccttgatggtgtacagtttgccgtccttgaggatggcaaccttacccttcgtcagcttcgcggcatccttgaggaggaatgcgtcgttcacgaggtcatctacgaaggactcgacggcctcaaactcagggaccttaggcagagagtggacgtaggccttcatcagctcgtgctcaccctcgactttccattcgatattcaggcagccgcctgaagcgtcgtcgtaggcgaaggcgacaagcttgccatcacgatagatggaggcgttgtagccactgccttcgtttccaatgaaggacttgaggcccttaacagtgtaaccgtggccgctgacggcggcgactagcgccttctgcttgggggccggcttaggggcctttgatatgacctgtccgcccgctttcttcgctttgctcctatagtaggagacacatgcgggagaggtgttagcatttgggtgggcctgtttgaccagcgcgaggatttcctcgttggtcttgccatccgccaggccggcgcggatggtgtctgcgatggttgccatttttaggacctcacgtgtttgcgttggtgtgagtccattatatggggtcttttgggaaaagggagcccctcccagcaaattattttgctaaagttctgctagtgccagtttgggccttatacatataaaagaagggcctccggacgtctccggaggcccctcaggtcccctatcatgttttcgtcccccgggaacccggttagtgcacggtgggcttgccgggggcggtgcggccgtccttgacgttcacatcctcgccatcgcgacgcaggcgggaggcataccactggacggtcttgacagaggtgttggcttcggggtggcgggccttgatgatgtccaccatcgccgggtaggtcaaggcgcgcttgcggcggcccaggatgcggacctcttccttgatggtgcgggcggtgttcggcatgactgttctccttgctttatgagaggcggtccaggtcgtcgcccggttgccgcatgctccagtggtggagcacgaagtcagtatgcacttacgtccggacccaaaacaccatcgttcccagctaggtgagcgtaccgcggttgcccaatgaattagacgcaaactccagcagctccttggccccgtgggttggggccagcacagacatctcggccagccgggcctctgtgaccccgtcggccagctcctgggccttgaaccccggcaccaggtagcgcagcacgtcccggcccttaccgacgcgggcgtagatccaggtgttgccgccgcagcgccacctcttcctgtgccacacgacctgggcctgccttacctcgaagccgagtagcccgtcgcgcttcggccggtcgcagcccttcagctcgagctcgaagtacagtccattccagcacccatccacgtccggatcgccggagctgaccaggttctcgactcgccgcatgtgcaggccgggcgtgcccctcagctggtcgcgcagccactcccagagccttacctcccgggccacttcatgtcctcagtgaacacgcgcaccttgacgtcccccacggagatctgcaccggcgtgtcgccgttgttcggcaggtagctcgccagctcgccggcgtgcatgcccccgcgtagctccgtgggcacaacggtgatgaaggcccgggtcacgtagcctagcctcagtgcagcaagcgccagggtggggccgccgatgagccagccatcggggtggtccaggtgggcctgccccagggatttgcccaggcccaggttctcggcgtcgggctcccgggtgatgcgcaccatcgagcggttcggcagacggggcatctggtcaaaggtggtggacccggcgagcaggacgtcggtcgcattcgacatggtgagcagacggaagatggccttgtccgtcttgccagtccagcgcatgtcgtcgtcggccccgctggccaggtagccgtcaatagatgaggctagcagcagtcgcatgaaggattctccacaatgtaggtgataggtatgccggcagccgttaggatggcggtagagactgtccaggatttcccccaccgcgcgtggccgaggtcgggctttggggccacgatgcggtggacgcctgcaagcctgagcttactggcacaggtcaggcaggggaagcgggtaacatagatggtgcagccctccggggagaagggagactgccggaggcagttgtcctcagcatgcaccatgtttgcaagcttgaagtcgcggtcggccaggagcgatggcaagtcaggcaccccgggcggaaaaccgttgtacccgggggagacttgccgccggtcaggcgtcacgaggacggcgccgaccttgcgatccggatccttcgacatagaggccgccaggaccgccatgccatagaagaactcgtcccactcttcctgggtccgcttgatcggcgcctccatcactcgatgacctccggcttcggactgaacgccggccacgtgagctgctttgcctcctcggcatagcggaccacgtagtcgtcggggtgctgctcgatctgggaaagcttccagccgggcagctgcagctgcggcagcaccgggtcctggtggagcatctgccccgccatgtcccagtgagcgtcgtacaggtgggcatgggccagggagacgtgcatcacccccgggcgaatgcccagctcgtgcgcaacggcgtccatcaggagcgcgtggcccatgacgtcgtacggcaggccgacgaacaggtccgagctgcgcaggaacaggctggagtgcagctccccacccgtgatgctgaaggtgaagctggtcgggcagggcacgttcttctgtccctgtgcgcccaggccgtcttcagccgggtcccaggcggacacgtagacccttcggtcgctcgggtccttgcgcagcgcttcgattgccagcctgatctggtctcggtcgaagtgacgacgccaccggtaaccgtaagcggacttgaccccccggatgaactcggggccggcaaccttgcgatcgccctccatgtgggtacggtacatgacgttcggcaccggaccattgaacggccgtgcgtagtcgtgctcgtaggggatctcctcgacgaacttgtcccacagcggtgcatacttggtgatgaaggtcgcgtcctggctgcccagcacgtaccaggcaacctcggcggcggcggacttcgggaaggtcttgcggaagccgatcgtcggcaggaggccgtcgctcaggtcgaccctgaacgccacgcctccccggccgacacggacgcgcgttccggtgcgctcattcgcctcgatcgggctcgacagcgcccaggcgataagagctccgtacgtgtcgtagaacggcatcaggaccccggtcacttgtcaccgcccatgccattgagcttcagccactcggcgtagtaggtgccgtagttcaccaggtcgcgggcggtgtcgtacagaccctcgtagttgggctcgcgcccctggcgcatcgcggtgatgagcgactggatgcgcaggttcttggtgtggagcatatgggcgtacgactcgtggccgaacgggaagtaggcctcgcgcccgccgggcacgttgttgtagtcctggcccttggtctcccgcaggtgctgcagctccatccagaccgggctgatgctctcccgcaactgttcctgcttgcgcagttcctggagatcagacacgtccgacaggtcgaacgacagcagccaggcatggttgggcggctcccaaccctcaggcttgacggcatcacggccgttccaaccggggcgcttcgacaggtcgccgcgcacctttgccatgttggcggcctgcaccgcgtcgaatacggctagcggcggcacgcccatctcgacgagacggcccagcgcgaagtagatcaggtccaccagggcgtcagccgcctcgagcacgtcgccatcggagtgggcgtcctcgaactcctggatctcttccttcagggcgtcgaccgaagcgtccatgcgctcgcccgacagtaccgtgggtacccccggaatcggagtgtccaggatcttgacattgaactcctccgctttcaggagcatgcgcgccacaagggccgccacaagggcctgatgctggcccgtcttttcgatctcatccatctatgcagtactcggttggtgggtgaaagggtattttggcgtagcccgagaagcgggcataccgccaagtcaggtttagcggttacgggcttctcgtatgcctcgccgggcagcgcacaccagtgaatgcaggaatagaccggatgggctgccgctcagagtcaccttgcaggtcgacccgtctttgctgaccatgacgatgaggtggtcccctcgactgaaacgcactggcgtcacggtaaacccgtcctcctccagcgcagctatgccttctttatgcggtcgtagcaggatgcgcaggcccatgctcaggcctccgccgtcttcttgacccgcggctgcttgggggcaaagctctggtgcccgtcggggacgatcaggcgggcctgtgaactgtcctcgctcagctcgtagcccagcccgttctccttgttgatggtaaacaggtgggacagcacggctgaccggtcgaggtccagctgtgccatggcgtcggcgatcgggaagaaccctcctacgaacagcctggccaccgtggcccgcttgctcggctcggggatcggcttgagcgcgtcctggatgacgggcttgccgccggtccgcttcttcggctcgtagggcgtgccgtcctcgttgaggcgcaccggcttctccggcttgggctccctgacgggctcgacgtaggcaaacaggtcgaagccctcaggcaccagcaggcgggcgcagtcgctcaccagctcgtagcccacgccgtggtctcggttgagggtgaacaggtgggacagcacgccggagcgggacagcccgaggcgggccatcgcctcgtggagcgactgagggtcttcctgcaggaagaaggcagcgacctgaccgcgcttgctctcggggcggcagggcttgagggactcggtcacgatcggcttgccgccgcgctttgactcgtcagacttggacgggtccggcgggggcggcaggaacttgggcaccgggaagcccatctcggtgagcaccatggcggccacgccgtagtccttctggaacccaagctttacactcatctcccaggctttgtcgatgaagtgggccatcttggagggctccacgtcaaagcgctcggccgtctggagctcgccgcactggttgctgacctggaaggcctcgagcgagtgggggcagaggatggtggagcgcttctcacccttaatgatgaccacgtgggcgaagccgctggtgggcgggtcggtgatctcgaacctgcgcttccagaagttgggggccccgccccgaacgaagtagaccttggcgaagacaatgttgggaggaagcatggactggctccaaagagaaagggacctggtctgcaccaggtccctctatcttatggcaggagcttggccccttaaaccatcatttccaggcgaactgcccggccgcttcggtgattactcgaagatgcccttgtcgccggcggtctcgccgcgctgggcgtccgcttccttctgggccttggcttcggccttggccttgtcggcggcgtccttcttggcctgcttctcggcgtccttggcagccttcttgtcagccttggccttttcggcggcttccttcttggcctgcttctcggcgtccttcttggccttctgctcggccttggcgtcgcccttcagctcgcgagcggtcgggaccttctcgccgtccgaacgcagcttgttgcggtaccagttgatgctggccatcgaggtcttggcttccgggaactgctcgcggatggcagccaggacttcctcgttggtcttgccgccacggatcaggtccttggcgacgtcgccgacgcccggggccttcggagcctgctccttggtggtctcggtggtttcgccggtctgggtgttggtgtcttcgctcatgggtgctctccttcagagacttgggaatgatggggactgtcgccgcccgatcgggcggcttgcccggcgtgcgtcagtgggtgtagtgtatcgtcgggcgtctgatcgtggagccgtcgttcgcacgaccggccgggtgtatcacagctgctgtctgaacagagccaacagcctgtcgcgcagtcctcggccggcgagctcctccgacacggagcgcttgctgtccaggttggcgagtatgtactcgtccaccgagctcggggtgacgtagtccctgatggtgacggtcttgccgccgatctgggtggcacgctcgttcgcctggtcccgctcgatcaggtcaaacgtgtgggagtaccagaggatcacgtctgccgccgacaggtccaggcccgcgccgccggccttgggctggccgacgaagaccttcaccgaggggtcattgttgaaccggtcgatggcctcctggcgcttcgcctgggagtgcacgttcccgtggtactcgacgcagcctatgccagccttctccagggtgcgcaccacccggcggatgtcctctcggaacttgcaccacacgatggtcttgcggtctgactcccggacgtcctccagcatgccctgcaggcgtgggttctcctcgtccggcaccatgtcgcgcacgttgccttcggagtcgatgacccagccgctcagcagctgctggagctttatgacccggacgcctccctccacagcctcgacctccccaccgtcctccagctccaggatcatctccttcaggagcttcttgtactgcgcctgcatgtcgtcggacaggaggatggtcctcgggtccatcagcaggtcgggcatgtcgtcgacgtcctcgcgcagcacaacggacgcccactgggccatgcgggcctgcaggtcgtcgaggttcctgtagtggtccaggcggtcgtagctgcgcccgcccttggtcttctcctgcacgtagtaggcaaagtgggactcgaactccccgaaggtggcaaaccccagggcgtggtccgccaggagctcgaactggctgtaggcggccagcggactgttggacaccgaggtgcccgtcagggtgcgccgcacccggcagtaccgcttcagggcgcgggcacgtttggtgcgcttcgagcctggggaccggaagtcatgagattcgtccaccaccagcatgcacttgcccttgtggcgctgcaggaacttcttgatgagtgccgccggcttgtcgtggatgatggactcggagttgacggcgaacaccgccaggccgtccgtgtgggtcaggcacctgtccagggacgccgcgtggccgggcttgtgggcctcgctggcctgccaggcgtgggcgacgtactgtatgccctcccacatgtggatgggcagctggcggcgcacccagttcacgtgcacgccatttggcgccagtaccaggatgccggtgatgtcgcccttctcgtaccggtagcacgccaggtcgagcaccgccttcgtcttgcccgtgcgcatctgccagagcagggccctggcgtcgtcgtcccggtgacgatcccactcgtcctgctgatgcttatagtttggaagcctgaatcggggcgtcacttgcggtacctcatgccagtccatccttcggccttgaccgggcagccgtcggcccagtccagggtgtatgccatcgtggcctcaaagtccttcacgtccccggcgtccatgtcacactcggcgatcagttcatcgtgtacagacaggatgacgtcgtacagaccctccttgtggcaccggagcatggcgtcagccatcaggtcccgcgcggacgcctgggtgatgttctccacaagcatgccgccataggtgtcctggcgacgccacttcttcgtgtacggatctacgcccatgtaggtcagggcaggcttcttctccccccagggagtcggcttcatgacgatccgcggatcacagtagcccagcagcctgccggagggcagcttgcagtgcaggaagccgtcgaagcagcaccattgcaccctgccgcacttcacgatgcggcctggggtcctgacggcggcgatcgctgcggcctcctggtcccaccacatcttcttgacccgccagaacttggcgcggtaggcgtcgacgatcttctgtgcgaactcctcctcgatgaagatcccgtacttctcagccagcgtggcccggaacttcttggcccccatctggtagcccagacccaggactgcttgcttgcccatctggcgctcgtccgcctgggcttccttgtcgtagatatggcgcccgtagatctcggtcgccatcgccatgtagatgcactcgttacggcggaacacctccagggcctcgtcgtcgccggcaagccagagcacgacgcgtgcctcgatggcggcatagtcggccaccatcagccgtcggccgggggtcggtacgatcatcccgcgcagggcatacgacagcagctccatggcgtcgccgtaaagcatctccatcatgcccaggtcgcgggacttgatgatctcccacgccagctccatgttcttgatgttcccgcgcgggaagttgtgcggctgtacgcctgagccggaccaccggcctgtacctgcaccgtggtacagcagcccgccgtggatcctccaggtatccgggtcagcccagttctgagcagcaatgaacttggcagtgctagaccgcccgagcgccctgacgagctccagggctcgccgcagcttcggggcgatgtcctcccggcgaagccaggagtcgatggtgccgccctgggtattctcaatcggcagcccgttgtcgttgaaccactcgatcatgcgggcccgctgggttgccttctggacccggccgccggtgatctccaccagctccttgttcagctcggtgaagatgccgtcaacaatctccagtgccgcctcgatgccctccttgtcgagctggaacccgcgctggttgatcgcctggtccatcaggtacatctccgtctccttaggagacaggtccctcaggcggtgcgacacggcctcctcagccaggacgtcgatgcggcagtacgagcacaggcgtgccagcagctcggcgctctcgttccagaagacaggcaggcggaagacctcctcctcgacgtcggggtccgggtggtaggctactgcgttgtaggtgccgtcctcgttggggtacagctcgatcttgtacttcttggcgggcagggccaggctgccgttgtcgtcgatccaggcaaccacgtcccgcttgagcggcttgcgcggcttggccatcttcttcatgaccttggcgccctcggtgtctttctccaccttgagggccagggccggggccaggtctgccagcttgcgtggcagggaatacgccgccgctttggctgcggagcatcgccactgctcgtggccgatggcgggccagtttaggcgggggacgcagacgttggtccagatgccgcgctcgaaccaggcgttgtgggcctcgacaagacggccctcccggatccactcgaaaagctcggcgagctcggggcagtcggcttcctctacgtcgaactgcgggaaggcagggtgccacagagcggtgcggccctcctcccagtgcggcaggcggaacgccaggcacatgacctcggtcgtggggtcaagcgagtaccgccaggagccgcagtccttgatggagcagacggaccgggtctcgaagtcgatcgtggccttgggtggattgtcgtactggatgcccgctgtctcgtacaccgaggcggaggcgatcttgaacagctgagacttgaccgccgccgcgatctgggaccgctgcggcgtcggggccggtgacgagggcagcacgagcggggactggcggtactcactgcccccgatgagctggttctcgctacctccgtgattcacggtggccaccagctcaccgtcacggtaggtctgggttatggtcatggatcctcctggctagccgcatacattaccagggcggatcgtcgaagtcgaccgccgtctcccaggtcctgaacagttggttggcgcggagacactcctccctggacagctcgcctatgtggaaggttggggtgcccatcatcttggccatcatgctgtagacctcgccacggctcatggccggcgtgttccacagcgggtcaatcatggcgtgtagctgcctgcgcatctgcctggtctcgcggtccgccatacggccgagcgggaacaccgagtacgggtggcacccgacgaaggcttcgcaggacatacagaggtagatccaaggccagtcgccgcagggcctaccatagactaccgtgttgttgaccagcacgacgagtggctcgccgcagcagtcacaaacctggggcggatcgagccagtctttgtaccgcttcttgcggtggtagtctgtgaaggtcaccagtccacctcctcctggatgattgcacgcacgtaggcatccaccacggggtccgcgtcggccgttgcgcccttggctacagcaagagctgccttctccaagcgaccgacgtctatggcgcctatgcgggcctcacggaccagggcgtttttggtggcgtatatcggccttagggccgtcagcttgacacgctcgagttccgtccaccgcctgccgatcgattggactacctgggagagccgtatggtccgctccccgggcaccaggccggtatcatcgacggctttgccggcaaagtccgcgattgcgttcaggtctctcaggggccaggccgccagggcgcacagcgggcacggcagttcgtgcctgtggtcctcacacttcaagggcgcacctcgtaggcagggtccttgatgagctcgtgcggatagtagaagacacagctggaggccccgtcccgcttgacccatacccggccgtccggcgcatggaagttcacctcaccgcgggcccctttatggaagcctgcatgcggtgccacgatgatgcgctggccgaccccgaagtactccggctcgtcagggtccatctgggtggggatcggttccaccagcagcctgccgccggccttcaccacgcggaagggctggtgctccgggatggtcagcagcttcgagccgaagccgccagtcaggatataccacaggatcgttttgagccagctcatttgatatgctccagagcagcctgctgctcttccatgggacggtggagggtgaagtccgcagcagcgcgggcgccagcatggaatgcgccgccgtcaagttccttcttctcgaacttgtcctgctggacgacgccgtattcgtagatcttgttgcagtaccgctggatggcgcggtcctcagcttccgtcggggcgatggcggagatctgcttgtacaccgagttgagccagccgatatggaaggcttgccgcttgccactgtcgcccttcatatcagggcgacggatgaggaggtcgtcccacgaagcctgcatggcccgccacaccaccttgtgggcgtattcggccagcatcacgcggcccttgggaccaatgtaacggacgttgagacgggcggcggagccggggttccgctcgaagacggccttgacgccgaaggcgcgctccatcatggtggccaggttgctcatggtgcggcaccggccgaagccctcacgcgtcttgacgaccacgtcggccgtgtccaggccgtccagctcgtcctcggtgacgcccagctcagccatgatcttttgggcctgcctaagcgctgcggccgcctcgtgcggctcggggctcttcgagagggccatgcacttcttcagcttttcggtgagcctcttgcggcggtcagcgtccatccgtttctccttctttggtgaggccgagctccgaggctgcggcccatattgagttgccaagctgtggcgaccgtgttccccgcacctccgaccggtcgtcggcgtcgtacaaggcccagccgttgtcgtccttgaggaactggtaggcagcttcctcaatgaggcccatcatgcgcttcgtggggctcacttgaaccccagcaaacggatgccccgctggagcaaggactctttgtcagccgccagcttggcgcgggcccgctcgagggcctcacgctggccgggcttgaccgccagcttcacagccgcttcgtcacgccagcgctggtcttcgttgcgctggtccagcagctccaggtttgtccgccagtctttgctcacggcgattgctccgtaacagtgtgggatcatcatgcccgaggtttccgccctgggacgccattgaatgggcaaaaagaaggggacccgaaggtcccctcctggggcttacctgcctcgcggcggtgttccgaccggggcggtcgggtggactcgtcagtccaggaagcttccgctggcctgctcgccctcgccgacgaagtcgtcgaccgagtcgaagtcgttctcggcggcggtgcggccgctgaaggcctcgccgtcacccagcttctggacgttctgcaggccgaacgccacgcccttgttgccggccttgtcgtacccgtaggcagtcagggtggcacgggcgaagcagccggagtagaagccctccgggctcacctcatcggtgatgaggcggttcagggcgttgtcgacgcagcccggctgcatcttggtggtcgcagcaacgaaggtcatgccggcatagccttccagctccgacttctcggcgccgtcacggaaggggttgcgcaggccgtggtaccagccgttgccgtcgggcttcagcttgtcgccgaacttctccttggccgccgcgtgggccagcttcttcatggcttcgaactgggccgtcttgcgcgccgccgcgtcgaacagcatggtcacgccgtacttcggctcgccggtgctgccctccatcgggggctggggcttgaagatccaggcaaagctggcgcggaacttcggggaagtgaccttgcggtcgttggacttggctgctgccatgttgtacgctccttaataggcgatttagcgatttagcgatttaggtggagtctgccccgacgccgggtctgggtgccgccgtgacgcaacccgaagagggaggcggggacggcgacgtcggggcaggtgttcattattccgggacgtgcgtcgcgtcgacaccaccgagctgctcgtacagctcctcgtcggtgaacttgcccgtcgagacgttgaccagcccgatcttgtagttccaggactttgccgcctccaggttgtcgcgctgcaagtcggccttgtcggcttcaagcttgcccgacgccacggccttgtccagggtgcgccgccaggcggtcatcatctccgcgtcggtgcgggtgacccacttgtgcgtggcggtgtccggcaggtcgtacaccgggccggtcatggctcggatatggtgctcgtacgacttggcgccgatatggacgatgaagggggtcacgccgtcacggctattccacaccttcagcacgtcgggagcgtcgggcttttcggcgttggtctggatataggtcatcagccggaaggcttcagcgtggccgaagttgggctgggccggatcgacgctggccgtagcctgtttgatggtcttcaccagggcgcgcagccgcactacctcgcgggccaggtccttcttgccctgcgcggcgaggcccttgaccaggttggcctcctcgtcgatgaagtccagcatggcctcctgcagcgcctcgcgctggccagccttcaggtcttcaggggtccaggtgcccgcccgggcgcgctccaggcgctcttccagggaggggccgcggtgctcgttgctttcctggatcagctcgtgggcgcgctccagttccttcaggtcggctttggtcagttcctgcatgggtttatgttcgtgcatggcggtgccttagttgtggtggagccagttgggaaggttcttgcgcttttggtcggcgtgccgccggatagccagcacatccaggtcacccgcctcgaccatcatctcctggacggcgagcaggtcacccagctctttctccaggagatccttgttggtggtcatcgggaagtcggggtggtggctgtacagcccgtggcggaggatcttggtcacggactggccgacctcgcagccctcttccgccaagcaggcaagacgctcggcctggtcgtcggtgagtccgttgaagggattgttgctcatggtttctcccggttaaagaaaagggtggaagcacataatgcttccacccgggtcctgctcggggccgtcagtctgcgctttcggtcccgtcgtacacgtcgaagtcaccctcggcggcggccgtcgcatcgactgcctctctgggatcgtcgagcgcggccacggtggtgccaccttccggcttgaacgataccccggcgacgagcgctttgatatgcgccgccggagcgcgcacaccctcggctttcagcttggccatcagctcggcggggcgcacggcctcgatcttgctgggcgacttcggcttgggctcctcgtacatcagctcacgggggataccctcggccgccagcaggtcgaacgccgtcacgggctcgccagtcacttcgtccgtcaggtcggtcctgaaggcacgattcgacttcttgcggaccagcttgccaaagcaggcctgaccgccaggggtctccctgaggcggcgcagcacctcggtcttcgccgacttgatgaagatgtccagcagcggaactgcccgcatcctgagcatcaggtcttcgtcgctgtcctcgggcccgcttacgctcacgctgtcctccgtaaagccgtctccgaactccagggctgcctgggaaaaggcttcctcccgcaatgccgggcacaccgccgcggccttacagaaggtgcaccagtcgcccgccttgagcggtgcgtcccactcctcagtggcacgtgctgcctcgcgcagccgggcctcgaacgcccgcagggttgccttgtccgtggaccagcgccggaccttaccatcctggtgccgggcacgcggctgcacgatcaccaggtccagggtctcgaaggcccactggagctcgtgcgccttgcccagcgcgtagtacagctcctggtcattgtcctccacctcgacgacgacgccctggccgtgcttgtagtcgatgacggagacatgatcgaagggcagatacagcgagacgtcgttggtgccaaacatcgggccccagcacacccggccgtcggggtggaacaggtgccccagggggaagtcgtctgtggcggcatagtggatcccgctcgggctgacgtaggacgggtccttctcccaggcctcgaagtcgaagtcgaagccgatcagccagttgagactgaactgacgctccacctccatctcggcgtgctggcccatgcgctccatctcatcccgcactgcatccaggtagacctgtacagcgtctgccatgtcggcatcgatagggaagtcctcatggccttcaggaggcagaccgtcctgggtggcatggaccgggacagtcacatcggacgcctccaccatcagtacggagttggcgggccggtgtaccgtggcttgctcggtggggtcgaggcggacaaagcctcccatccactcccaggcctggctgccgtcaagcaggcaggcctcgccgagcgcgtgcgcggcagtccccagccttgcggccggggaagagttgttgggacgcccgtactccatgcggatggagcccaggcagttcatccaccgctttgcccccgacgcgtttcgtactgcgtgggcgctaggcatgtcagttcaccattgcgagctggatggtggggtactcgaaggtcacgccgcgcaggtcggcgcgggcgaagatcgactcggagcgcaggccgcggccgtccgggtaggagaggaacgtgacgtcctcgcccgccttgaaggcctgcacggccttgtctgcctcctcacggaggaccaggaaggcggtcggctgcggcaggcccttgaaccacaggaccagctgcgcggagtccttcgggagcttctggttgggctgctcgctcatgctgcgttcttcccggcagccttgtcgatcagcttctgcaggctgtccgggccctgctcggccaggtcgctgacgctcttggcgttcaggctggtcagcaggtccatggctgcgtcattgccttcgatggccgcgtaggccttcagggcggcgcgggcgtcgtcgatggtgaccttcttcttggtctcggcgggcttctccgtttcgacgggcttgtccttctcgacctcggcgggcttgtcctgcgtggcggcgacctgctcgaccggggctgcggcctcagcagcctgcttggtctcctgcacggcagccttgctagccgtttccttggtcacgacattgctgacggtgaccggctgggcaccgtgaatggctacctggatgggttcgccatcgacattcgccacgatgacgccgttgtcgttcatgtccttcagcgtctcgaggatggcctcgagcagggacgtctgacgggcctgttcccgcagactgttttccatgaaggtgttcacatccattgcgtgctccttgttgagcggttggtagggagtgacaatgtaccatccggagaccgggcgtgaagccaccgtccacggccgacggcgccctcagaccgagcgcagtgcgttcgtcggtttcgtaatgcactgcgtcatcgcactatgctcatcccggcctgtcgccggcccgatcaagatgcacccacggagtacaggggaatgagtttgaaccagcagatgtccctccgcgtatcggaggaccaccgcaggatcctgcggggtaagctcgaggagatgagggcacacagccccgagcccgagaaggtgactgaggccgatgcggcccgcgcaatcatcgaagaggctgccgccaggaaggtgacgcagtgaccgctattaagcgaccgcgcccgggtgacatgcgcgcgtacgtagagaacggtctgcagctcattccgctgcaccggtacgatgcggtggacagcaagggccgaccgcgcggcaagacccccagggacggtgcctggcaggcgaaggagtacgactcccgtgccgtgatcgagaatgccgatcgccagggcgtcaacgtgggtgtgcgtctgcccgccaacatcatggtgctggacgtcgacccgcgcaacttccctgaaggtcgcgactccctggccgagctcgtcgctgacatgagcctggacctgagcgtggcgccgcacaccgtgacgggctccggcgggcaccactactggttcaccaagccggtggacgtcgacctcctggactccctcgaggactaccagggcatcgagttcaagtcgcgcggccgccaggtcgttgcagcgggctcggtccacccgaacggcacccactatgagtgggacgacctggcccccggcctggacgagatgccggagatgcctgccaacctgatgcgcctttgccgccgacccacccgtgcccacggtgaggctgcaggcctgggcgagcttacccctgagatgctcgcctcgaccctggagcagctggaggccgaggatttcgccgaccacgacaggtggcgcgacctgatgatggcctgccaccacgccaccaacggtgagggccggcaggagttcatcgagtggtccacgcaggacgtgaagtaccaggacgacgcctggatcatcggccgtcgatgggactccctgcacgccacctccggtcgtggcggccgcccggtcaccatcaagttcctccacaaggtggtccaggagggcggtggtgaagtgacccgcgtcgacgcggcagacgactttgacgtgtgggaagaccccgacgacctcggccagggcgttgacgatgaggagctgcgtgcagagcccaagtccgagggcctgatgggcgtgctcgaggacatgaatgagacccactgcgtcgtgatggagggtggcaagttccgcatcttcaccgagaagatggatcccgtcctcaagcggccgttcttccagcgctccaccaaggaggacttcgagaacctctactgcaaccagctcgtggagatgcacgacaagctggtgaccaagtcctcgctgtggatcaggtcgccgcaccgccgacagtacgacggggtgatcttcgaccctgaggcaaaccatgaaggctggctgaacctgtggcgcggctgggccgtgcaacccaagaagggcgactggtccctgctccaggagctggtgcgcgacgtgctctgcgatggtgacaaggcatcctacgaatacgtgctcaactggcttgcctacatggtgcagcacccgtcgcaggccgctgaggtggcaatgtgcttcaagggtgagaagggtaccggtaagggcacgctaggacgcgcagcctcattcctggcgggctcgcatggcctccagatctcctcgcccgagcacctggtaggccggttcaactcgcacctgcagaactgcatctgcctgttcgccgacgaggccttctgggccggcgacaagtcgggtgaggcaaagctcaagcagctggtcaccgagccgaccatcgcctacgagggcaagggccgcgacgccgtgaccggcaagaacatgatccacatcatcatggctgccaacggtgactgggtggttcccgccggtctggacggtgagcgccgcttcgccgtgttccaggtcaacaactcgaggcgcggggacaaggccttcttctccaggctgaacaagcaaatgtaccgggacggcggtatcgagggcatgctcttcgacctcctggcgcggaacatcaacggctgggcgccgcgtgacgacgtgccctcgacctctgccctcgtggaccagaaggtcatgactatggatgacgtcgagcggtggtggtacaacaagctcctcgagggcatcctgccgaacgcccgcggcgattggcacgagggccctgtcaccgtcatcaaggagcacctccgtgcggactactcggacttcgccaaggaccagagggtgtacaggccggcagaccctgtgtcgttcggcatgcgcctcaacaagctggtgagcggcaagctggagaacacccaggtcaagccgggcgacgaggactacacggtcaaggtagaccggatgggtcgcgcgtccgcgtcgaagctgcccagcctggacgattgccggtccatgatggaagccaagctgggcagcaaggtgcagtggcccaaggacgccctcgactgatcgggggcgcgctcggccacggtcgggcgggagtacgagcctaacgaatcccttgaacgccaggctcagacgctcagacgagccgtctgaggcttacggatcaaggacttaggcccggaatctaaggcgtttaggtcgtacgaggctttggctcgatgttgtcccaggaaaaaccgatcgaccgaccatgacggcagcaacacacttcggtctagtcggcttagatgcttagattgtggttgaaaactgtataaggatcagtaatttaattaatctagatctttttaataaaggtttagattatctaagcctttaaccagactttctactaaatacaccaatctaggctttctgagtgacacggccgacacggccgacacggtccgccctgggcaacacgaccggcatgctgcataggcgcctccgctcatcgtgcccagcccgtggccgagcccggacggtggccgagaaggcggggcccctcagaccgctcacgcaaaatccgtccgatcgcagtcctggactcctcgtgcacgaggaaacaccgggaaggcctcccggagaccgttggcttaccgcccggcctgggcggcgataccatcggaccaatgtaccagcaccgcacacggagtacctagtgactgccaagaacctcaccgacgacgagcgcatgttcctgcatgagcgaggcccggtatccgagctcgagctcgtcgagtgggagctcgacggcctgaacacccaggagcgcatgtcctacgagcggcgtcgcctgttcctgcgcgccttcgctctccgaggcatcgtcctggacggctgccgcgctgcgggcgtgtcgcgtggtgctgtggagcactggagggagtcctccgagtggtttgacaccatgttccacatcgcacgggaggaggcggccgatcgcatcgagggcgaggccttccgccgcgcggtcgacgggtacgacgagccggtcatctaccagggcatgacgaccacggtcatcgaccctgtcaccggcgaggagaagcagctgatggtccgcaagttcagcgacgccctgatgcagaccttgctgaagggtgcacgccccgacaagtaccgggagaaccacaaggtcgagcattccggtcaggctggtggcgtcctggtgatccccgcggctgtcgacccgaccacctggtacaagaccgtgcaggagcagcaggccaagtacgccgggaacaacgaaggcggcgaggctcctcctaccgcgtaacaatcacagtgcaccagccagggcgtccacaagggcgccctttccacaaccgagagaacgccatgtcctacgaacccgtgcccacaggccggatgcgcctgcgcgagcagcaccgctccggcctcatcttcagcaagccctcgctcctcgtcctccaggtcgaggtcgacgtcccggacggtccgcccgactccaacggcatgccccagtggctcgcgacccgcacctggatcgacgcccaggtcgaacatctccccatcatcccgctcgaagtagcctgagaccccgccatggacatccaacccgctgagaacttccctgaccccgtcgatcgcgcatcggccgagtccctcgcccacgacgacgcctcggtcgacgcggccaagcgcgccgcggcagcccgccagaagcgctgggctccccgggaagatggtgactgcgcctgtgggtgcggcaacgaggtggacccgcgcaggctcgccctgggctacggcctgaccatcgagtgcgccaccaagatggagcgccgatgaacgcgacctgcgtacagcagctgggcaatatcctggcggccaacgcccgcgtcctgggcatgcaggccgagaaccagcagcgggcgatccagggtgagtccatggcctacacggcccaggacttcaacgtggaggccgaccagatggaggcggcagcacgcgaggtcgccaactggggacacctgccatgagtgagctacccactcagggacagatcaacgacctgaaggccggtcagctggacgaggtgcgcgctgcatggggccttcgcctcgcggccgaatcccagctgagccgcctcgccaagtacaagagcatgtcgcccggcatgaaggacgaccaaaagcgctggctcaagcagctggtatccgccaacgcggtcatcgaccgcatcctgggagcatgaaccgtggccgagatcaccgacattcgcagggtacgccagaacagggagcaggcccagctgtaccaccgcgaccctgacctcttcctggaggcctggctcaacgacaagggcgagatcgtggcaacccaggtcaagggcactttccgagcgccctccgagaccggcccccaggcccacgacctggcggacaacctcctgggcatggcctcccagggtgcatccatcctgggtgacgagcactggcaggcccagcccgtcttcacggcccacctcctgcgaggcggcttcatgatgacccgcgccaggcgcttctggcacgaagaggggaagcagcccctggcaaagcgcctccgctgtgcctggtgggtcgcacggagcgcctggggagccctggcgggcgtcctggcggcttgctactgcctggtcctccaccccggcaaggccttcccggctgaagaggaagactg

SEQ ID NO: 9 - DNA, 63771 bp, unidentified
  source 1..63771: mol_type = genomic DNA
ccacggacatgacgccggtgcggcccgcctctacgccccgcgagggcctgccaccgccgccgcgctactcggcggagcagcgggcggcgggcatccgcaaatacgctggcggcgtgccgaacagtgtgaccgagtccatcaacgcgaagcagcgggctgccgggctgccggagctaacgatggaggaagccgcggccattcgagcgtatactggaaacacgtaccgggcgctgaatggcgcgctccgcgggggcaagtactcctcggacccgcacctccaggcgtacgtggacgcggcccagcacggcatggccaagatgcccaagtacaagggcctcagctcgcgaggcatgtccttcaacgagacccagctgaaggcgatgctgtcgacctaccgtaagggggccgtcgtcgaggacgccgccttcgtctcgtcgtcctacggcgagcaggcggccttcggcggcaacgtgttcatgaagatcaacggtaagacgggcgtgaacgtctcccagtactcccagtaccagggcgagcgagaggtgctgttcatgcccggcacccagttccgggtggacgacatccagcagatcaacggcaagtacatcatcagtatgacggaggtgtgatatggcagaccccctggaagcggggccggagtgggagggcaagatgtccttcgctccgggcgtaccggaggatcccgacgcgataccggagctgttctatcaggtcctactcggccgggtgtacaccctgacccggtggaaggacggctccacggcccggggcgaggtgcagctggccgacctcgaggccgtcgcgggaggcacgataacccgggagggctggtacgatgcgctgggagcatacctcggcgcggagctcccgggctccctgtaaaacaggcccgccgcaatggcgggctttttacttctgcttgaacgctggctcgcgtggcccggcgccggtgataaggtgccagcctatacaccccgggcgcgacgcccacacagccagcgcgtgatgcgcagaaggagagtacaatggatttcgagttcctgaagaaccccaccgtcgattcgatcgacaaggtcccggaacagttccgcggcttctacggtgagggcgagggcggctacgtcctgcaggactcgttcaaggccaccgccaccgcggtcgacggcctgaacaagtcgctcaaggcggcacgacgcgacgccgacgaggccaagcgcaaccgcccggacctgtcgggcttcagcgccatcggccagctgctcggcgtcgagggcgaagacgcagccaaccccgagaccctgcgcggtgcggtcgagaagctgatcggcgactcgaaggacggcaaggtcaactgggagaagatgaagcgcgacctggagggcggcttcaaccagaagctccaggcgaaggacggcgagctgcagaccatgagcaagtccctccagaagtacctggtggactcggccgcggtccaggcgatcgccgcccacaagggcgtgccggacctgctgctgccgcacatcgccgcccgcaccaaggtggtgcgtgacggcgaggactacgtggttcgcgtggtcgacgagtcgggcgacccgcgcggcaacgcttcgggtggcttcatgactgtcgaggacctggtcaaggagctcaagggccaccagaccttcggccgggccttcgagagcgaggcgccgagcggcaacggcaagccgccgggctcgggcaaccagaagcccgtccagcgccagggcgagatgaccgccaaccagaagatcgccgcgggcctggcgaagcgccagtccggccgctgatccaactgttgtgcaacaagaaagggcgcctacgtggcgccctttctctttacggcagtaccgccaggttttcccgcaggtccgtcaggacctggccgagccagttggtgccgcgccactcactggggtcgtggcagcgggggtcccgctcgtccaggccgatgccccagatcacgtccgtcgggctggcctccaccagcagggtgccctcggtgagcagcagctgcgcccgcagcttggggtcgctggtgaactttgccaggctcgcccgcatgacgacgtcgcgggacaccgagtcccactggcggcggtcgaagcccttgacccggcggccgatcgccttctgctccgccgggttggaggtcgccatgatctcgtccagggcctgctcgtccccgaagaccctcgccttctgggccatcatgtactgctcggcacacccgtactccacgccgtcgatcaccatgggcgacgggtaccactggctgaacaccccgccgtagaacagggtgtagcgaacgtattggtctttcaagggaaactccttacctatcagggggttacagtgtaccgtcagacgcgcttcgagactgtgggcggcgtcacgggggcaggaaccttgtgcaccgacacagcctggagcacgaagaacggggtgccgggattctcgctggccagcttgacggcctgcgcctcggcgtggtcattcctgccctgcacgacgcgcggcgggttcttcagcgagggacgcccgtgcggaccgccctccttgtagacgtcgccgttggcaacgaggtagaagcggccgtcgtccagctcggacgtctcgcgggcctggttccaggtcacggtggcggctttccggccggtcgagcggcccacgacgttgtcgacgacttgtcgacccttgggcgtcaggctcggaggcgtgcgcccgctcggatcgaagtcgatgaggtcatcggccacgaggaaggtgatgtccggcggcggcaggcccttgacgtgctcggggcccgagaagcccatagccaccgtcaagagggtgcgcaggcgggactccggtgacgaggaggtgtagcggggcttcgccggcgtcggcgccggggtggcgctcggcacggcctcgaagtcggaggccacgatcaggtcgcggttcacgccgagctgctccagtcggcaggcgacggcgtgctcggtgcgaccgtgcgccctcgacagcttggtgaggttgatcttgccggcggcggccaccaggaggtcgcgctcctcgacgtcggtccacggggcaccgccgcgcggggccgcagtcgggtgggccgagttgccgaccagcgtcgaccagccgcgcttgacggcgatggcgtgggacggttggcggtagcgcgagaagatgaggtcgaacacgccctcggcgaaggcgtcgagatagtcgtcggggatcaggtacagttcttcaaagtccatgggactctccttggttggtggacatgggcatcattacacccaattgggtaaggcaataccactgtttagagggcacggccctcctgcatgatctccttggcacgatcccacgctgagttccacaggtcgcagacctcctgcgtcatgccgtcgtcctcgtcgacgcggccgtaggtcgaggggtcgatgccgaactccccgaaggcagcgtccatgaccatgttggagtcgcagaagtcgcccgagtggcagacgtcggggttcagctcgcgagagttgaggtctacgacggtgtcgtaggcgtcctgaccgagggtgtcgcgcaggaagcggacaaaggcgagagccaggtcttctttgttgggcagtcccatcacagttctcccatcaccttgaggaacgactgcgcgccctcgaagatcatgttgtgcatgtccatgtcctccgcctcgatcgtgcggttgtcgtggagcgcgacctcgacggtcgtgaaggacgcctctgccgtctcgacggcgtcgagcgccgtcgcgtaggccatgagggtgatgggcgcaacctcgaggtcgcgcaggagctgaagcacctgcgcgaggtcgtcgatgggcgtgtcctcgaggttcttgtacttgacttgggcgttcatggggcctccttagcggccgatgatcttgtggagcgacttgaggacagcctcgcggtcctccgccgacaggttctcgtactcgggcagagcccgcacggcgtcgatcggcccgaacgagtcgtacggcatcatctgcatcatgtcgatggcgcgatgtgcgagggactcgtggtccactgccttggcgatctccatcagagcttcctcagttcggtggcctcggaccgcgcgtccgacatgcaccagcagtgggtgcgcttgactcggccgtcggccgtgatggccatgatgggcgactcgtcccccatcgtcgggtgctcgtacagatcgacgccggcgacggtgccgaagtacgtggggttctttgcgaggaaggcgatggccttctcggtggtgggcttgttcatgtctacctcagaggtggaacatcttgagttcgtcctcagacaggaggacggagtagggcgtcgcatcgcccgcgatttggaaccatgctcggccctcgtcgacggacgtgagcccctcgagcggtttgccatgcaggcggcgggcctcctcgaacaggtcgcgccacagttcccggttcatcggttgccgagggcaggcctgtcggtatcgcggggccttgatcttggttgagggcttacggtccatctgtttaccaggttgccgtggtgtgagtccattatacggggtcttttgggatatgggagccccctttaagaactatttttattctttttattagatctaaagaaataagggtatctaaggcagtcttaccctcttctagggcagtctggccatctaagtccttgtcgcagctaggccatctaggcttctaggccttctgaggctgttcctcgagccgtggccggacctggccggcaggctgttttcctggtacaacgaggcgccgaaggctcgttcaggctcagaactgacctaagtccttggtccgtaaagctttttctcgtctgaggcggctcccggaaggtccgaaaggctcggattctcgcgctggaccagcgttcagggggttacgagctcgagacgtcacgacaaactcccgaaccatagcgcgcgagcacggtcataacacccggcccgcgctcgctgaccctgcaaaggcgtgatgccttggccaggggtcgaatcgtcgggcgatccggcacctcccaagcatcccaccaccccgccttacaggagatccctaatggcatccgttaccctcgccgagtcggcgaagctggcccaggacgagctcgtcgctggcgtcatcgaaaacgtcatcaccgtcaacgagatcttcgagcagctgcccttcgacggcatcgacggcaacgccctcgcctacaaccgcgagaacgtgctgggcgacgtccagatggctggcgtcggctcgaccatcaccgccaagaacccggccaccttcacccaggtgacctcgaccctgaccaccatcatcggcgacgccgaggtgaacggtctgatccaggccacccgctcgggtgacggcaacgaccagaccgcggtccaggtcgcctccaaggccaagtcggccggtcgccagtaccagagccagatggtgaacggcgacggcaccggcaacaacatggccggcctgttcggcctggtcgcgggcagccagaccatcaccgccaacaacggtgcggccaacggcgcggccctgtccttcgaggacctggatgccctgatcgacctcgtcaccgacaaggacggccaggtcgactacctgatgatgcactcccgcacccgccgcaagtacctggcgctgctgcgtgcactgggcggcacctcgccgggcgacgtgtacaccatggcctcgggtcgcaccgtgccggcgtaccgcggcatcccgatcttccgcaacgactggatcccgatcaaccagacccagggcacctcggccaacgccacctcggtgttcgccggcacgttcgacgacggcagccgtacccacggcatcgccggcctgaccgccgagcgccaggcgggcatgcacgtcaagtacgtgggcgagaaggaagatgccgatgaaagcatcacccgcatctcctggtactgcggtctcgcgctgttcagcgagaagggcctggccgtcctgaagggcgtcaccccgggctgatcccagccagggtctcagccagcccgccggcctagtgccggcgggctactaataggagatcggaaacatgagtgcacatctcgtacgcctgagcgggtcccgctgcggccagaccctgtacgacaaggccgacgcggtcatcgtctgggtcgaggacgactcggtcaccaagccggcggatgcgcgggctgcggctgcggctgcacggcccggcccggatggctactggaacgacgccgtcgtcctggagctgagcgaggcgaacctcgcgaccgccatcccggtcaagagcgtcacctgacccatgagcctcgccggtacgccggcggggcttcgtggtccatagagcaagagaaggagagcccagatgtcccacaagttcgtactggtcggcccgcacgcgggcaagaccatgaatgtcaacggtcaccagttcgaggacggcgagttcacgttcgtcggcggtgatgcccaggcggcagtactcgcccgcgtgttcgagttctacggtgccctgcccgccgacaaggccgagctggtccgcctcaagggccgtgagcgcgagccgggccgcggccgcaaggagctggaccaggccatcgccggcctgccgggcgaccacaccgaccccgactacgtggtcaactcgatgcgcaaccactggggtgacctgttcaccgctggcgacgagctcatggtgcgcgaggtcgtggtcaagccggaaggcgacaagaccgacgccaccgtcggcgaccagaccaacacccagaccccggagccgcccaaggcaccgatcatgccgagcctggctgaagccatcggcctgctggacccgagcgacgaccaggactggacgtcgaacaacctgccgaacctggagcgcctcgaagccctgaccggcaagaagccctcccgcgccgacgtcgaggcgatcgccgacggctacacccgcgccaaggcgaaggccgccaaggcctaagccaagaagaggaccgacaccatggcattcaatcagcaggacaacgacggcacgatcgacggcgccaacgcgtacaccgacccggcgaccgtcagggcttactggctggaccgtggtgtcgacctctccgccaagacggactccgagctccaggtggcaatcgtcctcgcgactacctacctggacgctcggtactcctggactggctaccagctccgccggctgcagggcacccagtggccccgcggcggcgtgacctcattcctgcgcggcctgccgccggccctcaccacggccgtgtgcatggtcgccaaccgcgccctctcgggcaagccgctcatgccggatccgacgaccgatccgagcggccaggcggtcacccagacgaccaagaaggtcggaccgatcgaggtgtcgaagacgttcgccgagagctcctcgagcaacccggcggcgaccgtgcctcagtttccggaggtcaccatgacgctgcagcaggccggcctgatcctgtcaggcaactccggctccctggcgcgaggctgacatggcgacctttgactacgccgagctcaagggggaagtcgacgagctgctggccgagttcgggcagagctgcatcctgcgccgcccgggaggcccggtagtcgtcgaccctgtcgagggcaccgtgaccccgggcagcggccccaccgacttcccggtgctcggcgtcatcaccgactactccgaccgacagatagacggcgacaatatccgccggggcgaccgcctcatgtacatacagggcaacgagcgtccgaagcagggcgacgtcttcctggaggcaaacggcacacagtgggcgatcatcgacttcgactcggtggaccccgcgggtctggccctggtgttcgccctgcagctccggaggtaacgtggcaaggttccagcagcagctcagggggttcggcatcaagaccctcgacaaggtggacaaggtccgccgggcctcggtgctcgagctgttcaagctggtgatcttctccaccccggtggacacgggcaggctcaggggcaactggcagacgaccatcaactcgcccgccggcgcggccatcgaccggctagatatgggcggcggtgcagcgatggcggaggcggtcgccaacctgggctccctgacggacgtaatctggtttaccaacaacctgccgtacgccgagcgaatcgagtacgacgggtggagcaagcaggctccggagggcatggtgcgcaggcacctcgcctcctggaaaaggatcgtggccgccaaggcccgcgcattttaacaggggaatgagatggcagttaacccgtacagcggactcagcaaggctctgatgcagggtgtcaaggactccccgctcgccctgccgtacgccgtcgagaacgcccccttcgagaagccgtcggaccagagcccctgggctaaggccttcgtgctgatgaaccagccttccgtcgccaccctcggggcggaaggccaggatgcccatgacggcatcctgcagatcgacctgaactacccactcaacaccggcgaggcggccgtgacggccaaggcggacgagctgtcggacttcttcaaggcgggcaagcgacttgcccactcaggagtcgagctcacggtggcttcgtgcggccgctcacgcgggcgcgaagtcgatggctggtaccgcgtgagcatgaccgtcacctggttcgcccgggtctctcgtaactaatccacagtaggagcgtaccaccatggcaaacggcagccgccactccatgcgctacgtcgccgagaccgtctacggtcagaccccggcgacccccgcgttcaagcccatccgtcacacgggcaccaccctcggcctgtccaaggagtccctgcagtccgaggagatccgcgacgaccgccagatcgccgacttccgtcacggcgcccgccaggtcggcggggacatcaacttcgagctctccttcgagagcctggacgacctgctcgaggccgtaaccctgggctcgtggctcgccgacggcgcgccgggcggtgagggcgatcgactgaaggctggcacccagcgtcgctccttcaccatcgagcgcttcttcggtgacatcgcgacggtggacaagccctaccaccgcttcaccggcgtcgagatgaacaccctggccctggccatcagcgccaacgccatgattaccggcaccctcggcaccgtgggctcggacatgagcacggccagcgcgatcatcgtcggggcgacctacgccgcgccgacgaccacctcgccgctggactcgttcaccggcaccctgaacgaggccggcgtgccgatcgccgtcatcaccgagatccagctgaacctggagaacggcctggaggctcgcttcgtggtgggctccaagaagtcgatcctgccgtccatcggccggtccaacgtctcgggcaccatcaccgcgtacttcgagaactccctgctgctggacaagttcatcaacgagaccgagtcgtccatcgtcttcgagctcccggacggcgccggcaacaagtacgtcttcaccctgccgcgcatcaagtacaacggcggccagccggacgtcgagggcgagggtcccatcaccctgagcatgccgttccaggccctcctggacagcacgacccagaccaacatcatcatcgaccgagtgccggcataaccatgaacgagaacaacaccaccgcgggggcggcagcaggcatggatgagttcttcacccggggcaaggccaacgaggggatccaggtccccctgtggcgccccgacggcacgaagagcgagcactgggtgcgcatcctgggcatcgactcggacgtcttccgccaggcggacgccgagtcgcgccgtgaggccatccggatcgcgcagctggacagccaggcggagaaggccgaggccattgcccgcacgaagcgccgcctcatcgcgtcgctcgtgacggcctggtccttccccggcgagtgcaccaccgacgccgtcgagcagttcttcatcgaggcgccccagatcatggacgccatcgacacggccgcgagcaagcgatccctttttttcgcgatagggtcgagcagctcgcagccttcgccgagcacgagttcaagctcgacctgatccccaagggatccaagcagaccctgcgtgagtccctcatgcaggtctggaagacgctgaagcgcaagccgcctcagctggcagacgccccggagctccccgaggagctccggtacgtctgggagtggttccgggaagtgttcgcggctgagccgctgacgtatgccgagctgcaagcttggtccagcatgacgggcaagcgcctgaagggctgggaggccgagctcatcaagtccctcgaccgcattttctggaaggtgcagaatggcaaccgacgtagctagcctagcgatcaagatcgagtccctccaggtccagcaggcggattcccgcctgaagggcctggcctcgtccggcggcaccgccgagaaggccacctccggcctgatgggagcattcaccaaactgctggggccgctcgctgcggccgtcagcgttatgggcaccctcaacaagctgatggatgtccagcgccagttcgacgtgctgaacgctggcctcatcaccgccacgggctcctccgagaaggcggcgatcgccttcgacgccctgagggacttcgcccagaacacgccctacgacctgaaccaggccgttgagggcttcaccaagctggtgaacctgggcctcgacccgagcgagaaggccctcatgtcgtatggcaatactgccagtgcgatgggcaaggacctcaaccagatgatcgaggcggtggccgatgccgccaccggtgagttcgagcgtctgaaggagttcggcatcaaggccaagcagaacggggaccaggtgtccctcacgttccgcggggtcacgacctccatcggcaacaatgccgccgagatcgagaagtacctgaccgacctgggcgagaacgagttcgcgggcgccatggagacgcgcatggactcgctcgacggcgccgtggcgaacctgggcgacacctgggaccagctgtggctgaccatcagccagtccggcatcggcgacgccatcgaagcctctgtgcgcacggcgaccgacgccctgcaggagctgaccgacatgatcgcgtcgggccagatggaggcgctgctcaagtcgcagaccgtccagtgggaggcgtggggcaaggacatcgaggagtccatcgacattgtcacccagttcatcaaggacaactttggtgagtgggaggatgagggccagtccgtggtggacttcctgatcgacgccttcaagcagctgccgaccaacctccgggccatggtccagatcctgactgtcgagttcgcctcgggcttcgaccgcatcatcgcgggcgccgagttctggcgcgacacgatgaaggcgatcttcagcgacaccaccatcgccgacgccggcaggaagtggatctccgagcagcagcgcatctcccaggtgcgcctcgactccatctcgggcatcctggacgagcgcgacgcgtcgctcaaggccagcgaggaccagctcgccgccgcaaagaagctccgcgaggagtacgacgccgcccaggaggccaagcggaaggccaacgccggcaccgaccgcctggcgcagttccgcatcggcgccgacaagcccaagacagcgtcctccggggtcgacaaggacgcggcccgcgcccagaagcagagggagcaggagttccagcgggtcaaggacgccctgcagaccgaggaggaggccatccggtcctcgtacgagaagcggaagtccatcatcgaggcgaacaccaaggccggcaccgaggagcgcacgaagctcatgggccgcctcgacgccgagcgggacaacgagctgaagaagctcggcgcgtacggcaactccgagctggagcagctgcggcagtcgctgctgaagcaggaggacgccatcagggagtcctacgaccgccgcatggagatgatccgtgcgaacacggaggagggctccaaggcccgcgccgagctggaggcccaggtcctcagggaccgcgacaaggcgctggccgatgccgagcggcagcgtcagtccgagcgggacagcctgtacaactccctgctcaccgaggaggaggcgctcaagcagtcgtacgagcggaagaagcagctcatcctggagagcgagtcggtcaccgagctggagcgccaggacctcctgcgccgcctgcagaagcagttccaggacgagcaggcgcagatggagaaccagcgcatccagacccagctccagggcgctgccgccatgttcgacggcctggctgggctggcaaagggttacgctggcgagcagtccaaggcctacaaggtactattcgccgtgagcaaggcgttcagcgtcgcccaggctgccatgtccatctcgaccggtctcgccaaggcccaggagctgggcttcccggcgaacctcgccgagatggcccgggtcgccgcgaccggtgcgtccatcatctcccagatcaacggcgcccagtttgcgggtgcctacgaccagggcggccagatcccggccggcaaggtgggcatcgtcggcgagtacggccccgagctggtcaagggtccggcctcggtgcgcgggcgcgagctgtcctccaggtcctacccggacggtggcggccagcaggcgccggcagcgcccccggtcgtgaacgtcaggaacatcaacgtgctcgacccgaacctggtgggcgactatctgggcacggacgagggcgagaagctcatcatgaacgtcgtcaaccgcaacaagagctcgctgggctactgactaggagaagattagatggccttcgtaacgggcacggccgccaaccacgtggacgcgctggacaagctgcgcctgttcctgaccagcaacgacaccctgtcgtcgctgggccagacctgggcgcagctccggtgggtgccggacaacgtggaggccgtcgacaccaacataccgttcggctcgggcacccagctgccgcgcctgttccggccggactaccggacccagaactacacctccgagaccaacgggcagtacctcagctcgacctcgttcacctccgggcagtacgtgcgcctgaagatgcgcgccgccagggcggtgaccaagttcaccctgaaggcgggcaccggctcgagcctgacgagctacaccccgcgcaacttccggctggagtactccgacgacgggtcgacctggacctccgccgccacccttacggaccagcgggcctgggtggccaacgaggagcgcacgttcgcggtgccctcgaccggcgagcacctctggtggcggctggtgaccctgcagaccggcgacttccagggcacgctgaccgggcagtactgggagctccgctccatctggctgtacgacggcgacgtgctggtgtcgtcctcggagtccagcctggtggtcaagggcccgggcctggcgggcgacgaggagatcttcctcgccttccgcaccacctacaacaccggcacgggcgagtatgccatcctggtgcagggcctcaccggctacctgccgaacgagcagtccctccacaagcagcctggcctgcacccgagcgggtggccggtggtgcccctgtggagcgcctccatgccctactggttcgtcggcagcggccgccgggtcgtcttcgtgttcaaggtgtccacggtgttcgagtcggggtacgccgggttcttcctgccctacgcctcgcccgagcagtacccgtacccgatggccatcggcgggtccatgtcgccgctctcgcccagctaccggtacgacttcgtgtcgggcgcccacagctgcttcgtcatgcccgggggcagcacaggcgccagctccagcgtggatgtggtgtacaacaccaccctcaacgtgatgctgcccgacggcagctggttcgacttccagaaccggcccaccaacagcagcaacaactccgagagctacctgacctggggcaactccccggccagcgtgctgccgcacgccaccttcagcgagtccgcctccgcgggctacggcttccgcgagaacatcggcgggggcttctcggtcttcccggccacgctgttccagcggcgcccggccggccggttccttggcgagctggacggctgcttccagatctcggggttccagaacggctcggagaacaccggcaccatagcgggcgaggactacctcgtcttccagaacacctaccggaccgacgtacgcgagtactgggccctcaaggcggagtgacagacatggcttacgagaccggcgccgctacgagcgtcaccgacctgctggacaagctccggctcttctgcatcgccgccggctggacggtcaaccggtgggacgctccgtctatcacccgccgactcaacatgcagaagaacgggctgttcgtgaacctgtgcgcccaccagggcaccacggcgctgaacgacaacctcaacggctacaccaatcagggctcgacgacctacttcgccctggcggtcagcatgtccgacggctacgacccggacgccaccggggcgttcagccagccgggcgcgccgaggtactccggctacccgcgcggggcaatgctggcgcagatgaccgctgccgtgcccgcgtaccacttcttctcgtactcggactccgacgacatactggtggtcgtggagtaccgcaccggccggttccagatgatcggcttcggcagcctggcgaagttcagcgccgcggacggcggcgcctggttcggtggcggcagcgccagcccgaactgggcctacttcgagcagagcggctacggccccgactccagcaaccagaacgagctgatcccgttccgcatggcctaccagggcggctcggagtctaccagcttcctgcgctgcaacgtcgactccaacaacggctgggcggcctcgaggtacgtcgccgacggctccaccatgggcccgctcgccgcgatcggccaggcgttctatgacgaaaacctgcgccgctacaccccgagcgcgctcggctggcagacctccctgatgcgccagaccgtgtacgtcgggcgcggcaaccagttcgcctcgccctacggcgagatcaagcacatgcgccgcctggagatcaccaactacgtgcccggcgacgagttcaccctcggctcggacacctggaaggtattcccgtaccaccagaagggcggcccgaccgagcagcgcgggtacgccatcctgaaggagacctgacatggcagtggtgcagatgaccggcgtggtgcgctcagttacgcccacgccggtggcctcggccctggacacttcgagcaccctggggggttggacctacccctggggctttcccattgtggagccccgtaacgggtcgccggcgaccggcaccttccaggcaccgcccaccgtggccgtgctcaccccgccgtccttctcggcgcagggccgcgtcggcggcttcgtggacgacctgtactaccgggtgcacgtccgcccgggcgtgctcgagctcggcaacctgctgtccagccagacccgcaacatcgaggtctggaacgcccactttgagggcaagaccctggaggccatcgactcgcagggcctggacggcgtcgtgctgacccagcccgaggtgcccccgacggtgttcggcgcgctcgagtcccgcatctaccaggtcagcatctcgaccaacggcgccccgaccatcgacggccggtacctcttcgacttcgtggacgagacgccctcgctgcgcatcacgggccgccgcgtcgtgctgtggccgttcatcccccagacgaagttcagggagtccctggagtggcagacggacctgctgcaggcctactcgtccgagcagcgcctcgcgctccgcacggcccccaggcagcgcttcctgtacgagttccagctgctgccgcagcagtactcccgggccaaggccatcagcacccagtgggcgcaccgcgtctacggcgtgccggtctggggcgagctcacccggctcggccggctcctggagggccagacctcgctgaccttcgacgcgaccggggccgactaccggaacaacgacattgccctggtgtggcaggacgacgagaccttcctgacgatcgagaccgtcagcgccagcgccaccggcctggagctgaaggtcccgctgggccggtccttcgagaacgcctacgtgatgcccctccgctacgcccgcaccctgaacggcaccgagttcacccgccggccggacgacgtcacgatggcccgcctggagttccttgtcaccaacaacgtggacctgggggcgtcgatcgggctgccgcagtaccggggcaaggacgtcctcatggaccgctcggtcacgctgtccgacctgtccgagaagatcgtgaggcccgtcgaccagttcgacaacggctccggcccgatcacggccgatccccagcgtggctaccccgaccgatcggagaccctcggcctcgacgcactgtcgagggcggaagcgtggcgccaccggacctggctgcacgcccggcgcggcaagcagaagggcttctggctgccgagctggaaccgggacctgctcatcctggcgccggtcgactcggccgccaccagcatcacggtgcgcccgatcggctaccccctctactacggcgtcaccgacatcatgctcgtgctgaccgacggctcggtgtactacaaccgcgtgctgtccggctcgaccgacacggacggtaacgaggttctgtcgctcggcagcggcttcggccgaggcttcgctgcgtccgaggttgacatgctgtgcttcatgcgccacgtgcgcctggacaccgacagcgtcgagatcacccactcatacgcgggccgctgcagcagcacgatccccgtcatcgaaacccccgagggactgtaatgagctacgcatctatcgaggcatcgcgggagcagggagctcccgtagagctgtacgagttcacccagggcctgcagcggtgggccttcgcctccggggccttcgaggtggtgcgggacggcgtggtctacaagccctccagcatccgccgcgaccgggtcaagcagtctacggacatcttcaagaacgggatcaaggtcaccttcccccgggacgacgagttcgccagccagttcctaggcttctcgccggaggaggtcacctcgctgaccatctaccgcgggcactacagcgacccggacgaccagttcgtgatctactggaagggccgcgtcctgagcgccactgccggcgactccgccattgacctggagtgcgagccggtctacacctccatccgccggcccgggctgcgcgccaagttcgagtacggctgccgccacgtgctgtacggccgaggctgcggggtcaaccgcgaggcctaccgccacgacggcaccgtcatcggcatgagccaggggctcaacgtcgtcgtgtccggcgtcgagggcaactttgaggacggctggttcgccggcgggatcatcgtcgcccccaacggcgcctcccgcttcatcgtcagccacacaggcggcaccatcgtgatgtcccggccgctggccgggctcgcaggcgaccaggcggtcaagctctacccgggctgcaaccacctcaagtccacctgtgccgccaagttcaacaacctgcccaacttcggcggcttcccgtggatccccacgcgcaacccgttcgacggaagctccatcgtctgagaggttactagcatgatctggtggtatatcgtagtcttcatcgtggccctggtggcgtcctacgccatgatgcccaagcccgagaacgccaagcccgccgggctcggggacatcacggcgccgacggccgaggtcgggcgcgccatcccggtactgttcggggagcgagacctgaaggggcccaacgtctgctggtacggggacttccggaccgaggccatcaaggccaagggcggcaagaagtgacggagccccgccaagcagtgcggatggaacacatgcgccggttgggctactgctcttccggcgttcgcacattcttccagcgcaacgggctggactacagcgccttcctacgggacggcatcgacgcagacaagctggcggagaccggggatgccatggccctggccgccgtagaggagtccaaaaatgggcggcggtaagaagcagaccatcgggtacaagtacttcctgggcatgcacatggtgctggcccacggtccgctggacaagctgaccgagatccgcgtcgacgacaagctggcctggaagggcacctcgaccggcgggcccatcatggtctgcgcgcccaacctgttcggcggcaaggagcgggagggcggcgtgggcggcttcctggtggagaccctcaacaagctgtacggggaccgcatcgacccgccgctcgacccgaacgcactgcagggcgtcagcgccggcaccatcgacgtcatgatgggcagggacgaccaggcgcccaacgcgtacctggccagccagctcggcggcgccatcccggccttccgccgcgtcatgggagtagtgctccgccgctgctacctgggcaacaacccctacctcaagctctggtccttccggggctcgcgcatacacacccgccagaacggcatcgaccagtggtacgacgccaaggcggagatcgcgggcgacatgaacccggcgcacatcatccgggaggtcctcaccgaccccgactggggcatgggctaccccgagggcgacatggacgagacggcgttccgcctggcggccgaccagctgcactccgagaacatgggcatgtccctgctctgggacacccagcaggacctgagcgacttcctggccattgtgctccgccacatcgacggctccctgttcaccgaccgggccaccggccggttcgtgctcaagctggctcgcggcggctacgacgagagcaccctgctcctgctggacgagcagaacgtcatccgcgtctcggacttcaagcgccgcacggtcgacgagctgacgaaccaggtcagcgtgaagtactgggagaagtcgaccggcaaggacggctccatcacggtgcaggacattgcgcttgccgccaaccagggcaccacggtcggcacgaccatccagtacccgggcttcaccaacggcgccatcgccaccgtggccgccgcccgcgacctgaaggccctgtcgatacccctcgccacggccaccctgtacgtgacccgcgccgccgcgctcctcaacatcggcgacgtcttccgcttctcctgggaggagtacgggatcgagaacatcgttttccgggtgaccaacatcgagctgggcgagctgcagagcaaccagatcaagctctccgtcgtcgaagacgtcttctcgctcacctcggcgtcctacgcgcccccgccgccctccgagtggcagccgccgagcggcgacgcggccccatccccgtaccgcctggtcatggactcgccgtactacctgctcgtccgggagatcggggacacctcagcccaggcgctgccgaagaccgcgggctacgccgtggccgcaggcgtgtcccccggcgggacctcgatgagcatggcgatgcacaccaacgccggcgcgggctacaccgaccagaccgacctgtccttctgcccgtcggccgtcatccaagccgcctacagcgacgacccgaccgtcgtgaccttctcgatcggcgtcaccacggactggaacctggtgcaggccggcgacctggcggtgatcgggtacggcccctcgaacagccgcgagatcgtccagctcgtcgtggtctccgacacggaggtcaccgtgaggcgcgccgtgctggactcagtgcccagggagatcgcctccggggcgcgcctgatggtcctgggcctcagcggcgagtacaccggcatggactccaccgagtacgcccccggcgagcaggtctccgtcaagctcaccccgaccgccgccaagggccagctgcccctggcctccgccccggtcgacgtgctgcctatcctggcccgccaggcgcgcccctaccatcccggtctggtgcgcgtcgacggcgccaggaagcccgcgaccgcgaccggcccggtggtcatcacgtgggcccaccgagaccgcacgcagcagaccggcgagaccctgatcggccaggacgagtcctccgtcggcccggagaccggggtgcgctacgggctgcggttcctggacgctggtggactcgtactggtcgcgcgcgataacatcagcggcacctcggcgaccggccgcctggcctacaccggcaacgtgaccatggagctctactcgatctccgacgcgggcgaaagcatcaaccgccacgtcaggaccttcgcctacaccccggaggtcggcgcgaccgagagcacgatcacggcgggcacctggacgccggacgaggtcatcttcgacggaggcggggcctgatggcaaccatcgtagtaccacagcgattcgcccagcgccgtgacaccacggccaactggaacagcaaggaccctgtcctctggagcggcgaggtcggcatcctcatggacccgggccaggccgtcaagctgaaggtcggcgacggcacgaagaagtggagcgagctcgacttcttcgcctccgacggcaagccggtgcagctgagggccgcggacgggtatatccagtggaactacgtcggcgacacgacctggatcaacctggtgtccctggacaacctcaggggcgcggacggcgaggacggtcaggacgggcaggacggcgagagcgcctacgagatcgccgtcagcgacggcggcttcgtcggcaccgtgccggagtggctggcctcgctgaagggcgacaagggtgacaccggcgacaagggcgacgccggcaaccccggcacgccctacgccaggcgcatccagcacgtggccgacaccgacgccgggaccttcgagtgcgactggagccagtacgacgagatccgcatctccctgacggcgactgttaccctgagcttcaccggggcgatcgacggccagggctgcgtgctgaagctgcgccagccgccggcgggcgggtgccaggtcgggctgcctgggggcgtcgtgcgcttcaactccctgatccaggcgtacgccgtgacccagaccgggtccagggcggacaaggttggtttcgtgtacgacggcgaagacgcacgatacgacctggtctccattattcccgggatatagcccatggacgactaccagccgccgcaggcgctatctgtgcccttcctgttcgacggctcgtacgacccgccccaggccctgagcctgggcttcgtcttcggcgccgacggcggcgggggcacgactgacccgctgccatgcaacttcatgatcctacttaccatctgaggtaacaccatgaccgtccgcgtatactccagctccgacgtaggggcgccggtgctgaccggctccaaccccggagacctgctcaacctgctcacgaagtgcctggtggacggctatggctccaagcctggtgccggctggaccaagccctacaccgccaccaaccgcggcgccttcaagaccggcacgggcagccgcggccggtacctctacgtggacgacacccgcacctcggccacctacgcggcgcgggtgtacggcatggacaccatgaccggcatcgacgcgggcgaggggcgcttcccggccgactccgtcgtctcgggcggtctgtactggcacgtgcactacacgggcagcacctcggcggcgcgcccctgggtcctcgtggccagcgagaagatgatgtacctgtacctgcagaactaccccgacgccgggtcgaccaacacccagtaccgggagttctactggttcggcgactacgacgccttctcctcggccaacaccttcaacacgtgcatccagggcaagtcgagcaacagcccgacgacctccgagcaggacccgttcacctcggccggcacgagcagcacctcgccgggcctctacgccccgaggtcgtacaccggcctgggcggcgcagtccagctcggccggcgccacgactacgccctctcgggcagctccaactggggaggcaacggtacgctcagctacccccacgggccggacggcgcgctgatgatgtccccggtgtggctccacgagcctggcagcaccaaccaggcggccctgctcggcaagatgcccggcctgtgggcgccgctgcagtacgtgctgaacacgggcgacacgttccagggtgccggcgacctggcgggcaagtccttcaccgcgttccgccagtacgagggacgtgccgtcatcgagacctcggacacctggagctaaccgtggccgacctgggcgccatcggcgcatcctacggggtggggtcagagcgcgcgaccaacccggtcgggcgcaccctcatatacccaggccccagcagcgtggcgaccgccgcgccaggcgccaacctggcgtccaggcaggcgcgcccgcgcccaggcccgtccaacatcacggtgccgggcaccccgtcctggtacggaagcccccgcccgatcggcgcggacccgcaggctgtgtacgcagtgggcggcaccgtgaagcagaggcttaacggcgtggactccccgctggtcgggtgcatgatccggctgtacgcccggcggaccggcatgcccgtgggtgcggccacgtctgccaccgacgggtccttcctggtgccgggcctgctgccggaggccaggggcttcttcgccatcgccttcgacccggacggcgagcccgtgcagaacgccctgatattcgaccggctgatggccctgcccgcggtgcccggcgagatccgcggcgagagcctcgtgctcacccagggcatcgccgtgtcgtacgccctgcgcgccgtgtacgtggaaggatccatcgcatggtccgtatcggccggggccctgccggccggcatgtcactgaacccgagcaccggcgtgctcagcgggacacccaccgagactggcgcctacagcttcacggtccaggccgtagggtcggtgtacaactcggcctcgcggtcctggtcgggcgaggtggccggcgggctggagtacaggaagaccctcaacggcacgatcggcctctccctggtgcgctccggtcagcaggacgaggggtacatcgtggtgcccgccctgcccttcccggtcagcctgttcggcaccgcctaccagaacaacatctacgtctgcgccaacagctacgtcaccttcggcttcggcgtctcggtgtactccagcctgtccccgaccaaccccgggcgcggcatcctgctcggggcgggcgaccggtcgtggcgggcgctgtacgcgggcccgatcctggacggtcagggctacctcatccggttcgagggctccaccacctacaccacggacgacggcacgaacatctgggagctcgccttctacgtcgacggcacgatcgggctcgtcaccgggcccttcccggccgacggcatcaccaacatgtccgacggctccgcctggcggaccaccggcggcatggcgatccagcccaacaaggcctacctcggcgcgccgaccggcgccggcggcaactacgtctgggaggagaacctgtgatggagcgtaacgagaactggaagtccagctggcgggtgcggcgacgcttcatgttcgccgtgtcggccttctgcatgtgggtgatcggctacgtcctgtaccgggacctgggctccagcccggcggacacggcgatcacaatggcattcctaaccctcatcagcatcgtcggatcctatgtgttcggcgctacctgggaggacgtcagcctggccaaggccaagctgaagatgccggcagggaataccggcaagcccgccccggcaccaggggcgtcaacgaagatggaggatataccatgagcttcgtactgggaaccaagtcgcgctccagcctgcgcggggtgcacccgcacctcgtcaaggtggtggagcgcgccatccaggtcacgtcagttgacttccaggtctacgagggcctgcgcaccagggagcgccaggcgtccctcgtggcgcgcggcgctagccagaccatggactctcgccacctgcccggccgggacggcctcggccacgcggtcgacctcgtgccactgatcgacttcgacggagacggcaaggccgagctgcggtgggactggtccctctgctacaaggtcgcccaggccgtacggctggcgagcctcgagctccaggtgccgatccgctggggcggggtctgggaccgagcgctggccgacctggccgaccccgaggaggacgtggcggagtacgtggtccgccgcaaggcccaggggaagaaggccttcctggacggcccccactttgagttgcccgtcggcaactacccctgaggacaagcgcatgattccgttgggatacaagctcggcgctggcgcgcttatcggggtatgcctggtcacggccattgcgttatcataccgtcactactccggccttgtccaggacaaggtcgaacttacggcccaggtggcgacactggagcagggcaaggctgccgagaaggcccgggctgacgccctggacaaggccattgacaagtgggacgacgccgccaagatccaggcggacgccctcgaccgattctcaactgtccagcgtgacgctggcgaaaccacgaggaagctgacggatgtcctatccaagcacgacctcggcgcgctcgccaggagcaagccgggtctcatacagtctcgcgtcaatgctggcactgctgatgctttccgcctgctcgagcaatccaccggtggcgcagcccccggtcgaggccaagcagcccccgctgcccgtcctgcccaagccccagcccgtaaggactgagtcggtcgagtggcgggtggtccaggtcgacggcgagtccttcttcgccgtcaccgcccgggggtacgaggcgctctcccgcaacctggcggacaccatccgctgggccaaggaggcctcctggcagctggacttttaccgtgattcccgccagccggcggagccccagggggactcgaagtgaccaacatgcccgggccggaccagcccctgaacaacctcacccgcgaggaagcgcagctcctcatccgggagtcggtacgggaggccttcctgatgctcggactgaaggtcgacgaccccatcgaggtgcagaaagattttcagcacctccgggaatggcggagcaccaccgagaccctcaagcgcaagaccctgttcacgatgatcggcatcgtgctgtcgggcatggcgggcgccatggtgatgggcgcaaaggaaatcttcagcaagtgagccccgcggtgggcctggcggtacctctccttcctgccaggtcgccttccaccgccttcgggcggtggctttttcggaaaccaggtacataaggccgcctcgagcggccttacgcgtctaaggccctggacctaggccgcctcgagcgctgcagccggcctggaatgcccagaaggcacgccgtggcagccccgggcgagcacgaccgagccgatgaccaggctccagaacagtatgctcaggcctaccgccagggtgatgccccgggccgcccgcaaatcatcgccaccttcgtccagctcgcacatacgaaaatgcctcccggggaccatccccgggaggcatcatggcgtgacggccgcgcggtcgacgccgtcagtagacccacaccctctggtacttctcgggcatgtgcccgcagctccactccgacttccggccctcgtgctccgccttcgggtcctcgacctggacgcactccttcgagtgccacgagacatgcacgatcggacggtccagcgcgtcggcgaaggacttgattaccagcatccccatcaacaggcaggcgagaacgcaaagagcttgggcgaggtagtggcggggggtgtggggttctcctttagacccggggcttttttggggggggggggggggggggggggggggggggggggctgctcggcgggtcgctcgccggcggtgacgcggatctcgagggtgtcagggtcctgctcgatgccgatgaaccggcccgacatgctaatgatctcactcatgctgatggtcagggaaccatcaggcgaacgggccgccacggcacccagcaaggcggtaacccgctgcagctgaatctcgtgggcacagacgttgccgccgagcaggtcggcgagcaggtcgagggcatccatatcacgggcgctgctcatactgtttggtctcccaattgatctctactgaggtggtgcccctcacgcggcacttggccacggcgggcagcttgaggtcgagcaccttcgcgactgcgggggcgtcctgcctcggaatgtagcccagcatctgcccgcaggcgtcgtacacggccacggcgttgcggtcgaacttgttggtgggctcgcggcggagcgtcaggacctcgtcggccctgagctccagcactgcttcgcgagcacccttgtggtgcacggagcccacaatgtaggtcctcatctgtggcatcacgcctccttcttgggctgtgcgcgcgggcggttcggcaccttctcgccgcgctcgcgcatgtggacggcataccagcggaggcatgccacggtggtctttgcgccctcgaactgctggtggatgcggtcgagcacggtctcgtaggagtgtccgtaggggcgcttgtcctcgtcgtgggacacgacctcgagcagcaggccctcagccacctgccgaatgacgggccccttttccttcttctccttcggggccttgtccttcttggccttcgccttcggggccttgtccttcgtctccgtcatctgcttcagcagcatcgacaggccgttgggctcgtccttcgccttctcgatcttctccgacagctcgggggtgggggtgccggcgagctcgacgatggcggcctcagtctgtgcggcctccatggcggcgatctgctcgagcagcttgcccttgcccctcttcgcgagggacttcgggtcggcatcctttccgctcagctcgttgtggcgggcggcaatgtcggcgatgttggattcgttggacaggttcatggcattctccgtggacggttggtggcacgacggacgcattgcgcaccgtcgatgggttccattatggcgggttgtgtgggcaatagccccaacatttgggctattgcgcttgaacgatgggattactgtgcggcctcgacggccgcgaggacttcgcggaactgcgccacagtcatcccattgatgatggtggcagtggggttcttcttacggacgagctccacagtggcgcccttcacagtgtacagcttggagtccttcatgaggcagaccttgcccttagtgaggcggtcgtactcccttttggcgagaatgtcggccgcgagctcgcggatctcagcgatgttgagggtcttgtacgcctcgaggttggagaactcgaagtgggagctgtccccatcgtcgcccatgtcgatgacgccgctgtagagcttgccgtcgacgtagaccttcgcggtgaagccctgccgccactccttcaccaggtagtcgacggtcttaagctccaccttggatgcggtggcgggcttcgtaggagccttgatggccttcgtagggctcgacttcttcattttcgagcggtagtaggacacgcaggcggcagacgtgttggactgtgggaagtgcttcttcacctcagcgagcaccgccccattatcgaggcccgtcgagatgccctcgcggatcacgtcggcgatggtgcgcttcgacgtggccgacttaggggcctcaatctgaggcggagtcggcggctcaatggtttggatcactgtgtcgaagatctcctcatggccctcttcgccgtaggtgcccctccacgtgcgtccgttgtaggacacgtagccgaagtgggtgcgaccgccgatcttgtagagccagccgtcagacttcttgaggtcggagcctccgaagtcgttggcgtcaatccacgcgcggaacagtttggatgcttcagcgagtgagccgacaggatggcgggtgccgccaaacttcacttcaaacatcatcatattgggcctcacgtgtttgcgttggtgtgagtccattatagggggtcttttgggaaaagggagcccctcccagcaaattattttgctaaagttccgctagcaccagtttgggccccatacatataaaagaagggcccccggacgtctccggaggcccctcaggtcccctatcatgtttttcgtcccccgggagcccggtcagtgcacggtgggcttgccgggggcggtgcggccgtccttgacgttcacgtcctcgccatcacggcgcaggcgggaagcgtaccactggacggtcttgacggaggtgttcgcctcggggtggcgggccttgatgatgtccaccatcgccgggtaggtcagggcgcgcttgcggcggcccaggatgcggacctcttctttgatggtgcgggcggtgttcggcatgactgttctccttgcttttatgagaggcggtccaggtcgtcgcctggttgccgcatgccccagtggtggagcacggagtcagtatgcacttacgtccggacccaaaacaccatcattcccagctaggtgagcgtatcgcgattgcccaatgaattagacgcaaactccagcagctcccgggccccatgtgttggggccagcactgacatctcggccagcctggcctcggtgaccccgtcggccagctcctgggccttgaaccccggcaccaggtagcgcagcacgtcccggcccttgccgacgcgggcgtagatccaggtgttgccgccgcagcgccacctcttcctgtgccacacgacctgggcctgccgcacctcgaagcccagcaggcccccgagcttgggccggtcgcagcccttcagctcgagctcgaagtaccggccgttccagcacccgtcgacgtccgggtcgcccgagctcaccaggttctcgacccggcgcatgtgcagcccgggcgtgcccctgagctggtcgcgcagccactcccagagccttacctcccgggccacttcatgtcctcggtgaagacgcgcacctcgatgtccccgacggcgatccgcacgggcgtgtccccgttgttgggaaggaactgggctagctcgctggcgtgcatgccgccgccgagctcggtgggcacgatggtgatgaacgccctggagacgtagccaaggcggagcgccgccagggccagggtcggcccgccgatgagccatccgtccgggtggcggaggttggcctcgccgaggctgatgcccagccccaggttctcggcgtcgggggctcgggtgatgcgcaccatcgagcggttcggcaggcgcggcatctggtcgaaggtcgtcgaccccgccaggagcacgtcgttggcgttagacatggtgagcaggcggaagacggccttgtccgtcttgccagtccagcgcatgtcgtcgtcggcgccccgggcgaggtagccgtcgatggaggaggctagcagcagccgcatgagtgattctccgcaatgtaggtgataggtataccggcagccgttaggatggcggtggagactgtccaggatttcccccaccgcgcgtggccgaggtcgggcttcggggccacgatgcggcggatgccggcgagcctgagcttgctggcacaggtcaggcaggggaagcgggtgacgtagacggtgcagccctccggcgagaagggggactgtcggagacagttgtcctcggcatgcaccatgtttgccagcttgaagtcgcgatcggccagcaacgacggcaggtcaggtaccccaggcggaaagccgttgtaccctggggagacctgccgccggtccggcgtcacgaggacggcgccgaccttgcggtccggatccttcgacatggaagccgccaggactgccatgccatagaagaactcgtcccactcttcctgggtccgcttgatcggcgcctccattactctacgacctccgggcgggggctgtacgtgggccattcgaactgcttggcatcgtcggcataccggaccacgtaatcgtcaggggccgcttcgatctgggagaggctccagcccggcagccacagcttcggcacgacgggctcctggcgcagcgcctctgccgccaaatcccagtggctctcgtacaggtgaacgtgcgccatcgtgacatgcatcacgccaggccggatcttcagctcatgggcgacagcgtccatcaggagtgcgtggcccatcacgtcgtacggcagaccgacgaacacgtccgagctgcgcaggaacaggctggagtgcagctcaccgccggtgatgctgaaggtgaagctggtggggcagggcacattcttctgcccctgttcacccaggccgtcttctgccgggtcccaggcagacacgtagacccttcggtcggtcgggtccttgcgcagcgcctcgactgccagcctgatctgatcccggtcgaagtggcgacgccaccggtagccataggcagacttgaccccaaggaagaacggcaggccatcaacaaccttacggtcaccctgcatacgcgtgcggaaccgcacattgggcgccggagcaagcggatcgtgcaggctcaagacgtcggaggagtacgggatctcctcaacgaacttgtcccacagcggcgcgtacttggtgatgaaggtggcgtcctgttcgcccctgatgtaccaggctacctcggcagcggcagacctcgggaaggtcttgcggtagccgattgtcgggagcatgccgtcgctcaggtcgacgcggaacgccgtgcctccccgaccaacacggacgcgcgttccggtacgctcatttgcctcgacaggcgcctggaagacccaggcaagcaaggcaccgtacacgtcgtagaacggcatgaggacgccgctcacttgccaccacccaggccattggtcttcagccactcggcgtaataggtgccgtagttcaccaggtcgcgggcggtgtcgtacaggccctcgtagttgggctcgcggccctggcgcatcgcagtgatgagcgactggatgcggaggttcttggtgtggagcatgtgggcgtacgactcgtggccgaacgggaagtaggcctcgcgcccgcccgggacattgttgtagtcctgacccttggtctcgcgcaggtgctggagctcgagccagacagggctgatggcctcgcggccctgcgcctgctggcgcagctcctggagctccgacacatcggacaggtcaaaggtcagcagccagtcgtggttgggcggctgccagccctcgggtttgacggcgtcgcggccgtgccagccggggcgcttggacaggtcgccacgcactttggccatgttggcagcctgcaccgcgtcgaacacggccagcggcggcacacccatctcgacgaggcggccgagggcgaagtagatcaggtccaccagggcgtcggcagcctcgagcacgtcgccgtcggagtgggcgtcctcgaactcctggatctcttctttcagggcgtcgaccgaggcgtccatgcgttcgccggacagtacggtcggggtgcccgggatgggcgtgtccaggatctggacgttaaactgctccgccttcaggagcatgcgcgacaccagggccgctacgagggcctggtgctggcccgtcttttcgatctcatccattgtgtatctcggttggtggtgaatgggtattttggcatggcgcagtaagtgagcacgccgccaagtcgggtttaacgggcagaagcttcccggatgcctcgccgggctgcgcataccagagaatgaaggaacaggccggacgggctaccgctgagggtcaccttgcaggcagccccgcccttgctcaccctaacgatgaggtggtcccctcggctgaagcggacgggctccacagtgaacccgtcttcctccagcgcggctatgccctccttgtgagggcggagcaggatgcgcaggcccatgctcaggcctccgccgtcttcttgacccgcggctgcttgggggcaaagctctggtgcccctcgggaacgatcaggcgggcctgctggctgtcctcgctcagctcgtagcccaggccgttctccttgttgatggtgaacaggtgggacagcacggccgatcggtcgagttctagctgagccatggcgtcggcgatcgggaagaacccgttgacgaacagcctggccaccgtggcgcgcttgcttggctcggggatcggcttgagcgcgtcctggatgacgggcttgccgccggtccgcttcttcggctcgtagggcgtgccgtcctcgttgaggcgcaccggcttctccggcttgggctccttgacaggctccacgtaggcgaacaggtcgaagccctcgggcaccagcaggcgggcgcagtcgctcaccagctcgtagccgacgccgtggtcccggttgagggtgaacaggtgggacagcacgccggagcgggacagcccgaggcgggccatcgcctcgtggagcgactgggggtcttcctgcaggaagaaggctgcgacctggccgcgcttgctctccgggcggcagggcttgagggcgtcgggcacgatcggcttgccgccgcgcttggactcgtcggacttggacgggtccggcgggggcggcaggaacttgggcaccgggaagcctatctcggtgagcaccatggcggccacgccgtagtccttctggaatcccagcttgacgctcatctcccaggccttgtcgatgtagtgcgccatcttggagggctctacgtcgaagcgctcggccgtctggagctcgccgcactggttgctgacctggaaggcctccagcgagtgggggcagaggatggtggagcgcttctcgcccttaatgattaccacgtgggcgaagccgctggtgggcgggtcggtgatctcgtaccggcgcttccagaagttgggggccccgccccgaacgaagtagaccttggcgaagacgatgttgggaggaagcatggactggctccatagagaaagggacctggtctgcaccaggtccctctatcttatggcaggagcttggccccttaaaccatcatttccaggcgaactgcccggccgcttcggtgattactcgaagatgcccttgtcgccggcggtctcgccgcgctgggcgtcggcttccttctgggccttggcttcggccttggccttgtccgcggcttccttcttggcggccttctcggcgtccttggcggccttcttctcggccttggccttctcggcggcttccttcttggcggccttctcggcgtccttcttggccttcagctcggccttggcgtcgcccttcagctcgcgggcggtcgggaccttctcgccgtccgagcgcagcttgttgcggtaccagttgatgctggccatcgaggtcttggcttccgggaactgctcgcggatggcagccaggacttcctcgttggtcttgccgccgcggatcaggtccttggcgacgtcgccgacgcccggggccttcggagcctgctccttggtggtctcggtggtttcgccggtctgggtgttggtgtcttcgctcatgggtgctctccttcagagacttgggaactggaatgatgggaactgtcgccgcccgatcgggcggcttgcccggcgtgcgtcagtgggtgtagtgtatcgtcgggcgcctgatcgtggagccgtcgttcgcacgaccggccgggcgtatcacagctgctgtctgaacagagccagcagcctgtcgcgcagtcctcgtccggcgagctcctccgacaccgagcgcttgctctccaggttggcgagaatgtactcgtccaccgagctcggggtgacgtagtccctgatggtgacggtcttgccgccgatctgggtggcccgctcgttcgcctggtcccgctcgatcaggtcgaacgtgtgggagtaccagaggatcacgtccgccgccgagaggtccaggcccgcgccgccggccttgggctggccgacgaagaccttcaccgaggggtcgttgttgaaccggtcaatggcctcctggcgcttcgcctgggagtgcacgttcccgtggtactcgacgcagcctatgccggccttctccagggtgcgcaccacccggcggatgtcctcccggaacttgcaccacacgatggtcttgcggtccgactcccggacgtcctccagcatgccctgcaggcgcgggttctcctcgtccggcaccatgtcgcgcacgttgccctcggagtcgatgacccacccgctgagcagctgctggagcttgatgacccggacgccgccctccaccgcctcgacctccccgccctcctcgagctccaggatcatctccttgaggagcttcttgtactgggcctgcatgtcgtcggacaggaggatggtcctcgggtccatcagcagctcgggcatgtcgtcgacgtcctcacggagcacgacggacgcccactgggccatcctggcttgcaggtcatcgaggttcctgtagtggtccagacggtcgtagctgcgcccgcccttggtcttctcctgcacgtagtaggcaaagtgggactcgaactctccgaaggtggcgaaccccagggcgtggtccgccaggagctcgaactggctgtaggcggccagcgggctgttggacaccgaggtgcccgtaagggtgcgcctcacccgacagtaccgcttcagggcccgggcgcgcttggtgcgcttcgagccgggggaccggaagtcgtgggactcgtcaaccaccagcatgcacttgcccttgtggcgctgcaggaacttcttgatgagcgccgcgggcttgtcgtggatgatggactcggagttgacggcgaacaccgccaggccctccgtatgggtgaggcacctgtccagggaccgagcgtggccgggcttgtgcgcctcgctagcctgccaggcgtgggcgacgtagggtatgccctcccacatgtggatcggcagctggcggcgcacccagttgacgtgcacgccgttcggcgccaggaccaggacgcccgtgatgtcgcccttctcgtaccggtagcacgccaggtcgagcacggacttggtcttaccggtgcgcatctgccagagcagggctctggcgtcgtcgtcccggtggcggtcccactcgtcctgctggtgcttgtagtttgggagcctgaatcggggcgtcacttgcggtacctcatgccggtccatccttcggccttgaccgggcagccgtcggcccagtccagggtgtatgccatcgtggcctcaaagtccttgacgtcgccggcgtcaatgtcgcactcggcgatcagctcatcgtgcacggagaggatgacgtcgtacaggccctccttgtggcacctgagcatggcgtccgccatcaggtcccgcgcggacgcctgggtgatgttctccacaagcatgccgccgtaggtgtcctggcgacgccacttcttcgtgtaggggtccacgcccatgtatgtcagggcgggcttcttctctccccagggggtcggcttcatgacgacccgcgggtcgcagtagcctagcagcctgccggagggcagcttgcagtgcaggaagccgtcgaagcagcaccactgcaccttgccgcacttgaccacccggcccggcgtgttgacggctgcgatcgccgcggcctcctggtcccaccacatcttcttgacccgccagaacttggcccggtaggcgtcgacgatcttctgggcgaactcctcctcgatgaagatgccgtacttctcagccagcgtggcccggaacttcttggcccccatctggtagcccaggcccaggactgcttgcttgcccatctggcgctcgtccgcctgggcctccttgtcgtagatatggcggccgtagatctcggtcgccatcgccatgtagatgcactcgttgcggcggaacacctcgagggcgtcgtcgtcgcccgccagccagagcaccacgcgcgcttcgatggcggcgtagtcggccaccatcagccggcggcccgggctcggcacgatcatcccgcgcagggcgtacgacagcagctccatggcgtcgccgtagagcatctccatcatgcccaggtcgcgggacttgatgatctcccacgccagctccatgttcttgatgttgccgcgcgggaagttgtggggctgcacgccggacccggaccaccggcccgtgcccgcaccgtggtacagcagcccgccgtggatcttccaggtctccgggtcggcccagttctgggccgcaatgaacttggcagtgctagaccgcccgagggccctgacgagctccagggctcgccgcagcttcgggtcgatgtcctcccggcggagccaggagtcgatggtgcctccctgagtgttctcgatcggcagcccgttgtcgttgaaccacgcgatcatgcgggcccgctgcgtcgccttctggacccggccctcggtgatctccaccagctccttgttcagctcggtgaagatgccgtcgacgatctccagcgctgcctcgatgccctcccggtcgagctggaacccgcgctggttgatcgcctggtccatcaggtacatctccgtctccttgggagacaggtcgcgcaggcggtgcgacacggcctcctcagccaggacgtcgacgcggcagtaggcgcacaggcgctccagcagctctgcgctctcgttccagaagactggcaggcggaagacctcctcctcgacgtcggggtccgggtggtaggccaccgcgttgtaggtcccgtcgtcgttcgggtacagctcgatcttgtacttcttggcgggcagggccaggctgccgttgtcgtcgatccaggctaccacgtcccgcttgagcggcttgcgcggcttggccatcttcttcatgatcttggcgccctcggtgtccttctccaccttgagggccagcgccggggccaggtccgccagcttgcgcggcagggagtacgccgccgccttggcagcggagcacctccactgctcgtggccgatcgcgggccagcccaggcgcgggacgcagacgttggtccagatgccccgctcgaaccaggcgttgtgggcctccacgaggcggccctccctgatccactcgaagagctcggcgagctcggggcagtcggcctcctcgacgtcgaactgggggaaggccgggtgccacagggccgtgcggcccgtctcccagtgcggcaggcggaacgccaggcacatgacctgggtcgtggggtcgagcgagtaccgccaggagccgcagtccttgatggagcacacggaccgggtctcgaagtcgatcgtcgccttgggcgggttgtcgtactggatgcccgccgtctcgtagaccgaggcggaggcgatcttgaacagggccgtcttgacggccgctgctacttgggagcgctcgggcaggcctgagacctgcactggctccttgttcggggcgattaccatggatcctcctggctagccgcatacattaccagggcggatcgtcgaagtcgaccgccgtctcccaggtcctgaacagttggttggccctgaggcactcctccctggagagctcgcctatgtggaaggtcggggtgcccatcatcttggccatcatcctgtagacctcggcccggctcatcgccggcgtgttccacagcgggtcgatcatggcgtgcagctgcctgcgcatctgcctggtctcccggtccgccatgcgcccgagcgggaacaccgagtacgggtggcacccgacgaaggcctcgcaggacatgcagaggtagacccatggccagtcgccgcagggcctgccgtagacgacggtgttgttcaccagcacgaccagtggctcgccgcagcagtcgcaggcctggggtgggtcgagccagtccttgtaccgcttcctgcggtggtagtcggtgaaggtcaccagtcggtctcctcctggatgatggcgcgcacataggcgtccaccaccgggtcattgtcggccgtggctcccctggcaacggccagtgctgcgcgctcaagccggcccacatcgatcgctcctatgcgggcctcgcggaccagggcgtttttggtggcgtatatcggcctcagggccgtcagcttgacacgctcgagttccgtccaccgcctgccgatcgaccggactacctgggagagccggatggtccgctcccccggcaccaggccggtgtcgtcgacggccttgccggcaaagtccgccacggcgttcaggtccctgaggggccacgccgccagggcgcacagcgggcacggcagctcgtgcctgtggtcctcacacttcaagggcgcacctcgtaggcagggtcctttatgagctcgtgcgggtagtagaagacgcagctgcccgcgccgtcccgcagcacccacacccggccgtcgggcgcgtggaagttgacgacgccccgggcgcccttgtggaagcccgcgtgcggcgccacgatgatgcgctggccgaccccgaagtgcacgggctcgtcggggtccatctgtgtggggatcggctccaccaggagcctgccgccggccttgaccacgcggaagggctggtgctccgggatggtcagcagcttcgagccgaagccgccagtcaggatataccacaggatcgtcttgagccagctcatttgatatgctccagagcagcctgctgctcttccattgggcggtgcagcgtgaagccggcggccgcgcgggccccggcgtggaaggcggtgccgtcgagctccttcttcttgtgcgcgtcctgcgtgacgatgccgtattcgtagatcttgtcgcagtagcgctggatcgcgcgctcctcggcctccgtcggggcgatggcggagatctgcttgtagaccgagttgagccagccgaggtggaaggcctggcgcttcccgccgtcgcccttcatgtcgggccgccgtacgagcaggtcgtcccacgaggactgcatggcgcgccacaccaccttgtgggcgtactcggccagcatcacgcggcccttggggccgatgtagcggacgttgaggcgggcggcggagccggggttccgctcgaagacgggcttgacgccgaaggcgcgctccatcatggtggccagcgagctcatggtgcggcaccggccgaagccctcgcgcgtcttgatgacgacgtcggcagtgtccaggccgtccagctcgtcctcggtgacgcccagttcggacatgatcttctgggcctgccgaagcgctgcggccgcctcgtgcggctccgggctcttcgagagggccatgcacttcttcagcttttcggtgagcctcttgcggcggtcagcgtccatccgtttctccttctttggtgaggccgagctccgaggctgcggcccatattgagttgccaagctgtggtgaccgcgttccccgcacctccgaccggtcgtcggcgtcgtacagggcccagccgttgtcgtccttgaggaactggtaggccgcctcctcaatgagacccatcatacgtttcgtagggctcactttaaccccagcaaacgagcgccccgctggaggagcgtcaggcgctctgcgtccagcttggcgcgggcccgctcgagggcctcgcgctggccgggcctcacagccagcttgaccgccgcctcatcacgccagcgctggtcttcgttgcgctggtccagcagctccaggtttgtccgccagtctttgctcacggcgattgctccgtaacagtgtgggatcatcatgcccggggtttccgccctgggacgccattaaacgggcaaaaagaaggggacccgaaggtcccctcctggggcttacctgcctcgcggcggtgttccgaccggggcggtcggctggactcgtcagtccaggaagctgccgctggcctgctcgccctcgccgacgaagtcgtcgaccgagtcgaagtcgttctcggcggcggtgcggccgctgaaggcctcgccgtcgcccagcttctggacgttctgcaggccgaacgccacgcccttgttgccggccttgtcgtacccgtaggcagtcagggtggcacgggcatagcagccggagtagaagccctccgggctcacctcatcggtgatgaggcggttcaggttgttgtcgacgcagcccggctgcatcttggtggtcgccgcaacgaacaccatgccggcgtagccttccagctccgacttctcggcgccgtcacggaaggggttgcgcaggccgtggtaccagccgttgccgtcgggcttcagcttgtcgccgaacttctccttggccgccgcgtgggccagcttcttcatggcctcgaactgggccgtcttgcgcgccgccgcgtcgaacagcatggtcacgccgtacttcggctcgccggtgctgccctccatcgggggctggggcttgaagatccaggcaaagctggcgcggaacttcggggaagtgaccttgcggtcgttggacttggctgctgccatgtgatgcgctccttaataggcgatttagcgatttagcgatttaggtggagtctgccccgacgccgggtctgtgtgccgccgtgacgcaacccgagagggaggcggggacggcgacgtcggggcaggtgctcattattccgggacgcgcgtcgcgtcgacaccaccgagctgctcgtacagctcctcgtcggtgaacttgcccgtcaagacgttgacgagcccgatcttgtagttccaggacttcgccgcctccaggttgtcgcgctgctggccggccttctcagcgtcgaggcgcccggaggccacggccttgtccagggtgcgccgccaggcggtcatcatctcggcgtcggtgcgggtgacccacttgtgcgtcgcggcgtccgggaggtcgtacaccgggccggtcatggccctgacgtggtgctcgtacttcttggtgccgatgtggacgatgaagggcgtcacgccgtcgcggctgttccacaccttgagcacctcgggggcgtcgggcttctcggcgttggtctggatgtaggtcatcagcctgaaggcctcggcgtggccgaagttgggctgggacgggtcgacgttctccgtggcctgcttgatggtcttcaccagcgcgcgcaggtggacgatctcgcgggccaggtccttcttgccctgtgcggcgaggcccttcacgatgccggactcctggcggatgaagtcgagcattgcgccgtggagcgcctcgcggtggtggacctgcaggtcctccttggtgtaggtgcccgcgcgggcgcgctccaggcgctcctccagggacgggccggagagctgccggctctcctggatcagctcgcgggcgcgctccatctcgctcaggtcggccttggtgagttcctgcatgggcttgtgttcgtgcatcgtggtgtcccttagttgtggtgcagccagttgggaaggttcttgcgcttctggtcggcgtgccgccggatggccagcacgtccaggtcgcccgcctcgaccatcatctcctggacggcgagcaggtcgcccagctccttctccaggaggtccttgttggtggtcatcgggaagtcggggtggtggctgtacagcccgtggcggaggatcttggtcacggactggccgacctcgcagccctcctcagccaggcaggcgaggcgctccgcctggtcgtcggtgaggccgttgaaagggttgttgctcatggtgtctcctggtaaagaaaagggcggtagcacatgatgctaccgccccgtcccggcttgaaccgctagtcggcgctctgctcgccgtcgtatacgtcgaagtcgccctcggcagctgcggtggcgtccacggcttcccgcgggtcgtcgagcgcggccacggtgatgccaccctccggcttgaacgacacccccgctacgagcgccttgatgtgcgccgccggagcgcgcacgccgtcggccttcagcttggccatcagctcgggcgggcgcacggcctcgatcttgctgggcgacttcggcttggggtcctcgtacatcagctcgcgggggatgccctcggcagccagcaggtcgaacgccgtcacgggctcgcccgtcacctcgtccaccaggtcctggcggaaggcgcggttcgacttcttgcgcaccagcttgccgaagcaggcctgtccgccgggggtctcccgcaggcgccgcagcacctcggtcttcgccgacttgatgaagatgtccagcagcgggacggcccgcatcctgagcatcaggtcctcgtcgctgtcctcgggtccgctcacgctcacgctgtcctccgtaaaaccgtctccgaactccagggccgcctgggagaatgcttcctccctcagtgccgggcacacggccgcggccttgcagaaggtgcaccagtcgcccgccttgagcggcgcgtcccactcctcggtggcgcgtgccgcctcgcgcagccgggcctcgaacgcccgcagggtggccttgtcggtggaccagcgccggaccttgccgtcctggtggcgcgccctgggctggacgatgaccaggtccagggtctcgaaggcccactggagctcgtgcgccttgcccagcgcgtagtacagctcctggtcgttgtcctccacctcgacgacgacgccctggccgtgcttgtagtcgatgacggagacgtggtcgaagggtaggtacagcgagacgtcgttggtgccgaacatcgggccccagcacacccggccgtctgcgtggaacaggtgccccagggggaagtcgtcggtggcggcgtagtggatcccgctcgggctgacataggacgggtcccgctcccaggcctcgaagtcgaagtcgaagccgatcagccagttgaggctgaaccggcgctccacctccatctcggcgtgctggcccatgcgctccatctcgtcgcgcacggcgtccaggtagacctgcaccgcgtcggccatgtcggcgtcgatcgggaagtcctcgtggccctccgggggcaggccgtcggccgaggcgtgcaccgggacggtgacgtcggacgcctccaccatgagtacggagttggcgggccggtgtacagtggcttgctcggtggggtcgaggcggacgaagcctcccatccactcccaggcctggctgccgtcaagcaggcaggcctcgccgagcgcgtgcgcggcggtccccagccttgcggccggggaggagttgttgggacgcccgtactccatgcggatggagcccaggcaattcatccaccgcttcgcccccgacgcgtttcgtactgcgtgggcgctgggcatgtcagttcaccattgcgagctggatggtggggtactcgaaggtcacgccgcgcaggtccgcacgggcgaagatcgactcggagcgcaggccccggccgtccgggtaggagaggaacgtgacgtcctcgcccgccttgaacgccgccacggccttgtctgcctcctcgcggaggaccaggaaggcggtcggctgcggcaggcccttgaaccacaggaccagctgcgcggcgtccttcgggagcttctggttgggctgctcgctcatgccgcgctcttcccgccggccttgtcgatcagctgctgcaggctgtccgggcccttctcggccaggtcgctgacgctcttggcgcccaggctggtcagcagctccatggccgcgtcgttgccctcgatggccgcgtaggccttcagggcggcgcgggcgtcgtcgatggtgaccttcttcttggtgtcggcgggcttctcggtctcggccggcttgtcctgcttctcgacagccgtctcggcgacctgggtggcggcttcctgggccggggcggcctcggcgaccttcttgacctcctgcacggcggccttgccggcagtctcctcggtggtcacgtggttgctgaccacgaccggcgcggcgccgatgatcgcgacctgcacgggctcgccgtccacgttagcgacgatcaccccgttgtcgttcatgtccttcagcgtctcgaggatcgcctcgagcagggccgtctggcgggcctgctcccgcagactgttttccatgaaggtgttcacatccattgcgtgctccttgttgagcggttggtagggagtgacaatgtaccacccggagaccgggcgtgaagccaccgtccacggctgacggcgccctcggaccgagcgcagtgcgttcgtcggtttcgtaatgcactgcgtcatcgcactatgctcatcccggcctgtcgccggcccgatcaagatgcacccacggagtacaggggaatgagtttgaaccagcagatgtccctccgcgtgtcggaggaccaccgcaggatactgcggggtaagctcgaggagatgagggcgcgcagccccgagcccgagaaggtcaccgaggccgacgcggcacgggcgatcatcgaagaggctgccgccaaggtggaggcccgagcatgaccgcaataaagcgaccgcgcccgggtgacatgcgcgcgtacgtagagaacggcctgcagctcatcccgctgcaccggtacgacgcggtggacggcaagggccgaccgcgcggcaagacccccagggacggcgcctggcaggccaaggagtacgactcccgcgccgtgatcgagaacgcagaccgccagggcgtcaatgtgggcgtgcgcctgcccgccaacatcatggtgctggacgtcgacccgcgcaacttccccgagggccgcgactccctggccgagctcgtcgccgacatgagcctggacctgagcgtggcgccccacaccgtgacgggctccggcgggcaccactactggttcaccaagccggtggacgtcgacctcctggactccctcgaggactaccagggcatcgagttcaagtcgcgcggccgccaggtcgtggcggcgggctcggtccacccgaacggcacccactacgagtgggacgacctggcccccggcctggacgagatgccggagatgcccgccaacctgatgcgcctctgccgccggcccacccgtgcgcacggcgaggcagcgggccttggcgagctcacccccgagatgctcgcctcgaccctggagcagctggaggccgaggacttcgccgaccacgacaggtggcgcgacctgatgatggcctgccaccacgccaccaacggtgagggccggcaggagttcatcgagtggtccacgcaggacgtgaagtaccaggacgatgcctggatcatcggccgccggtgggactccctgcacgccacctccggtcgcggcggtcgtcctgtcaccatcaagttcctccacaaggtggtccaggagggcggcggcgaggtgacccgcgtcgacgcggcggacgacttcgacgtgtgggaagaccccgacgacctcggccagggcgtcgacgacgaggagctgcgcgccgagccgaagtccgagggcgtgatgggcatcctcgaggacatgaacgagacccactgcgtcgtgatggagggtggcaagttccgcatcttcaccgagaagatggacccggtcctcaagcgcccgttcttccagcgctccaccaaggaggacttcgagaacctctactgcaaccagctcgtggagatgcacgacaagctggtgaccaagtcctcgctgtggatcaggtcgccgcatcgccggcagtacgacggggtgatcttcgatcctgaggcgaaccacgagggctggctgaacctgtggcgcggctgggccgtgcagcccaagaaaggcgactggtccctgctccaggagctggtgcgcgacgtgctctgcgacggcgacaaggcctcctacgagtacgtgctcaactggctcgcctacatggtccagcacccgtcgcaggccgccgaggtggcgatgtgcttcaagggcgagaagggcaccggcaagggcacgctcggccgcgcggcgtcattcctggcgggctcgcacggcctccagatctcctcgcccgagcacctggtaggccggttcaactcgcacctgcagaactgcatctgcctgttcgccgacgaggccttctgggccggcgacaagtcgggcgaggcgaagctcaagcagctggtgaccgagccgaccatcgcctacgagggcaagggccgcgacgccgtgaccggcaagaacatgatccacatcatcatggccgccaacggcgactgggtggtgcccgcgggcctggacggcgagcgccgcttcgccgtgttccaggtcaacaactcgaggcgcggggacaaggccttcttctccaggctgaacaagcagatgtaccgggacggcggtatcgagggcatgctcttcgacctcctggcgcggaacatcaacggctgggcgccgcgcgacgacgtaccctcgacctctgccctcgtggaccagaaggtcatgaccatggacgacgtcgagcggtggtggtacaacaagctcctcgagggcatcctcccgaacgcccgcggcgactggcacgagggcccggtgaccgtcatcaaggagcacctccgcgcggactactcggacttcgccaaggaccagagggtgtaccgccccgcggacccggtgtcgttcggcatgcgcctcaacaagctggtcagcggcaagctcgagaacacgcaggtcaagccgggcgacgaggactacacggtcaaggtggaccgcatgggccgcgcgtccgcgtcgaagcttcccagcctggacgactgccgtgccatgatggaggccaagctgggcagcaaggtgcagtggcccaaggacgccctcgactaatcgggggcgcgctcggccacggtcgggcgggagtacgagcctaacgaatccctcaaacaccaggctcagacgctcagacgagccgtctgaggcttacggatcaatgacttaggcccggaatctaaggcgtttgggtcgtacgaggcttcggctcgatgttgtcccaggaaaaaccgaccgaccgaccatgacggcagcatcacacttcggtctagtcggcttagatgctcagattgtggttgaaaactgtataaggatcagtaatttaattaatctagatctttttaataaaggtttagattatctaagcctttaaccagactttccaccgaagataccaatctaggcttcttgagtgacacggccgacacggtccgccctgggcagcacggccggtacgtctggcgggcggtcccgcttatcgtgcccaaccgtggccgagcccggacggtggccgaaacggcggggccccttggaccgtccacgaaaaatccgtccgatcgcagtcctggactcctcgtgcacgaggaaacaccgggacggcctcccggagaccgttggcttaccgcccggcctgggcagcgataccatcggaccaatgtaccagcaccgcacacggagtacccagtgactgccaagaacctcaccgacgacgagcgcatgttcctgcatgagcgcggcccggtatccgagctcgagctcgtcgagtgggagctcgagggcctgaacacccaggagcgcctctcctacgagcggcgtcgcctgttcctgcgcgccttcgctctccgcggcatcgtcctggacggctgccgtgcggcgggcgtgtcgcgcggcgccgtggagcactggagggagtcctccgagtggttcgacaccatgttccacatcgccagggaggaggcggcggaccgcatcgagggcgaggccttccggcgcgcggtcgacgggtacgacgagccggtcatctaccagggcatgacgaccacggtcatcgacccggtcaccggcgaggagaagcagctggtcgtcaggaagttcagcgacgccctgatgcagacgctgctcaagggcgcccgcccggacaagtaccgtgagaaccacaaggtcgagcactccggcgcgtccggcggcgtcctggtcatccccgcggccgttgacccggcgtcctggtacaagaccgtccaggagcagcaggccaagtacgcggggaataacgagggcggcgaagcgccaccctccgcgtgacaatcacacagcagtaaccggggcgtccgtcagggcgccctttccacaaccgagagaccgccatgtcctacgaacccgtacccaccggccgcatgcggctgcgtgcccagccccgcaagggcttcttcggcagccgtgagccgctgctcgtgctccaggccgaggtcgacgtgcccgacggcccgcccgactcgaacggcctgccccagtggctcgccacccgcacctgggtcgacgcccaggtcaagcacctccccatcatcccgctcgacctagcctgagacccagccatggacatccaaccagccgaacacttccccgatcctgtcgaccgcgccgcggccgaggcccttgcgcacgacgacgcctccgtcgacgcggccaggcgcgaggcggcggcccgccagaagcgctgggcaccccgggaggacggggactgcgcatgcgggtgcggcaacgaggtcgacccgcgccgcctggcgctgggctacggtctgaccatcgagtgcgccaccaagatggagcgccggtgacatggagacgccgacccaggggcagatcaacgacctgaaggcgggccagctggacgaggtgcgcgtcgcctgggccaagcgccgagaggccgagtcccagctggcccgcctcgccaagtacagggccctcaccccgggcatgaaggacgaccagaagcgctggctcaagcagctggtctccgcaaacgcagtcatcgaccgtatcctgggagcgtgaaccgtggccgaggtcaccaacatcaccaagctgtcgaagcgccggcttgagcgcgacgtcttctcccgcgaccccgacctctacctggaggcctggctcgacgacaagggggagatcctggcgacccaggtcaagggcaccttccgggcgccctccgagaccgggcgccaggcccacgacctggcggacaacctcctgggcatggcgtcccagggcgcgtccatcctgggcgacgagcactggcaggcgcagcccgtcttcgccgcccacctcctgcgtggcggcttcatgatgacccgcgccaggcgcttctggaacgaggaggggcagcagcccctgggcaagcgcctcctgtgcgcctggtgggtcgcacggagcgcctggggagccctggcgggcgtcctggcggcctgcgtgaccctcgtggtgcggcccggccggttcccgacggacgaggaggactgatggcgtaccagccccctcactggaagcgcaagaagacgccccagcaggtcgcctccgagggcccgaaggtccgggcctggatcccccaggccggcagccaggtcctcttcctcacgtgcccggtcttcgagaccctgtacgagggcacccgcggcccgggcaagaccgacgcgctcctggcggacttctgccagcacgtgggccagggctggggcgccaactggcgcggcatcctgttccgcaccacctacaagcagctctccgacgtcgtggcgaagtccaaggcgtggttcaagctctggttccccggggccaagttcaacgagagcgactacacctggaccttccccgacggcgagcagctgctgctgcggtacatgtccaagccaggggactacgacaactaccacggccacgcgtacccgtggatcggctgggaggagctcaccaactgggccaccagcgagatgtacctcaagatgttcagctgctgccgctcgacggtgccaggcatgccccgcaaggtgcgcgccaccaccaacccgtacggcaaggggcacaactgggtcaagctgcggttcaagctgcccggcatgcggggcaaggtcatccgcaccgagggcgagcccgaccgcatcgccatccacgggcacatcagcgagaacaggatcctcctggacgccgacccggactacatccagcgcatcagggcggcggcgtcgaacccctcccagatcgcggcgtggctcgagggcagctgggacatcacgtccggcggcatgttcgacgacctgtggaagacccaggtccacctggtgagccccttcccggtgccgcgctcctgggtcgtcgaccggtccttcgactggggcagcagcaagcccttctcggtcggctggtgggcggagtcggacggcacggacgtggtcttccccgacggcaggcgcatgcgcacggtgcggggcgacctcttccgcatcgccgagtggtacggcatgaagaagggcaccgagaacgagggcctgaagatgctggcctccgacatagcggagggcatcaggctcagggaggtcggcctcggcctggccggacgcgtgaagcccggcccggcggacccggccatctggtcggaggagaacgggaactgcatcgagcgggacatgcgcgccaagggcatcaagtgggagaaggccgacaactcccgcgtccagggctgggagcagttccgcaagaggctgaagaactccctcaacctggacgagatggacctccccagggccgtgccgcgcgaggccccaggcatctacgtggtgggcgagcgctgccccgacttcgtgcggaccgtgccgcccataccgcgcgacgagaagaagccggacgacgtggacaccgacgtcgaggaccacgccggcgacgactcgcgctaccgcgtgatgcacaagaggaaggaggtccgccagggcaacttctaagtgatggtgttcgagccatggatggcccggcatcattaacccatcctccgacacgctgaccgacgagacagcgctaggctggagctgaacgacgacctcccatgacttagcggtccaggggaattagactggaaggctccacgcagtaggatcaccatctcgttcgccccgcccggaggtccacccgagggcggggcaccatggggtcccggtcgtctaattggcgtaggacgccaccttgttaggtttgaagccgctcggtggatatgaaggttcgactccctcccagtgcccctccacaacagtcttcaccggcgagctcccttacgatgttcacaggagtgcacgcctgagcaggtcagccgacacggtcctatccccagggcacggtcgcagagcctgcgggaaccctagggagctccccggtgcagactggcaggacaggatcggcgggaccaccctaccatgggagagtggagcaaaccgttgtccagcctggcgggctataaacgcctccgacccctgccagcacctctcgaagcccccgccgatcgggggcttcgccttttgtggagttcgatggcgttcggccacggctgggcccggtaaactgagctccctaccaaggagtccatccatgaagatcttcgacccgaacgccattgcgccctatgaggtagtacccctccctgaggacgaggccaatcaggctgtgacgtcccgcgaccaggggcgacgctccgctggcatgctgtccatgctggccagtgagcaggagaagttcctccaccagctggctgtagaccgcgccgacaagacctggctggagaccaacaccccgatgggcactgtcttcgaggtcctgggcgtggcccacatggtggtcagcctgccgcactacatcaagacgccggagcgtcccggctggggcccgatgctggtgaatgtcatggcacccgacggccgaggcggcatcgaccgctccgtgctgagttgcacccagctgcgcgccatgctcgagcccgggttcgtccgcccatgagcgcggcgtactcttcggtccgcaagggtgtcagggcgtggctcgaggccaaccccggcgagcacgccatccagcacattgccacacagtccggcctcgaccggagcgccgtgacggacgtgctgggcaagatgcgtcgtgcaggggaagcccgctgtaccaaggtcggccatggtcgtctgtatgagctcgtgccgggcgcggccgacacctccaggaagatcggcaggcgggatcccgaggccaagcgtgagtacgccaggctctacttccagcgcaagagcgccgagatgaagagggagcgcatgtcgcgcctggcggacgagcaggcacctccgcccaaggagcccagggaggagcgggctgagaccgtggccgagttcaggcgcagaggagggcaggtggaagtgctggccagccattggaactgaacgacggcccgcagcgagccttccccgcggcatcatgcgtctaccgggtcttggacaccccggtcatggcgttccatcggttggaagggttgagagccccgatcccacaagggtcggggctttctttttcgccggctcgcgctacgagcacgcatgcgtcacgatgcgcgctctaccccgagccgtacccgaccacctggagcaccccatgatcgacccgaagacgggcatccgcctcgtcccagcccgcgactccctcctgacggagttcggcgccaccaccctgtccaaacagtactgcctgcccggcgaatcctaccagcaggcattcgcccgtgcagccaaggccttctccggtggcgacgacgccctggcgcagcgcctgtacgactacgcctccctgcagtggttcatgtttgccaccccgctgctctccaacggtggcaccaaccgcggcctgcccatcagctgcttcctcaacgacgtcgaggactccatcgacggcctggtcgccaacttcgccgagaacgccaagctctcgaccaacggcggtggcatcggcaccaactggagccgcatccggtcgatcggtgagaccacgaccaagggtgtcgacacccccggcgtgatggccttcatgcacgtgcaggactcccaggcgattgcctaccaccaggggcgcaccaggcgaggcgcccacgcggtctacctggacgtctcccaccccgagatcgtcgagttcatcaacatgcgctcggccaccggcggcgacgttcaccggaagaacgagaacctccaccacggggtcaacatcacggacgacttcatgcgcgccgtggaatccaacagcacgtgggacctggtcgacccgcactccggccgggtgaccgacacggtccaggcccgcgccctgtggatccagatgctccagcagcgcgcccgcctcggcgagccctacctcttcttcatcgacgcggccaaccgcgacctgcaccccgccctgcgcgccaagggcctccgggtcaaccactcgaacctgtgcaccgagatcaccctgccgaccacgccggaccgcacggcggtctgctgcctgtcgtcgaccaacgtcgccaaggctgacgagtggtgggaggtgcgggagcagttcatcgccgacctggtgaccatgctggacaatgccctgacggtcttcgtcgagcaggcccccaaggccatgtggcgcgcggtcgcctccgtcatgggcgagcggtcgatcggcctgggcaccctgggcttccacacctactgccaggacaagggctgggcactggactcccatgaggctgccaccttcaacatcaccctgtactccgagctgaaggcccacgccgtggccgcctccatgcagctggccgtagaacgtggcgaacccgaggacctggttggcaccggcctccgcaacgcccacctgctggccatcgccccgaacgccaccagctccatcatctgcggcggcgtcagcccgagcaccgagccgatggtggcgaatgctttctcccagaagacgatggctggcacggggatcatgaagaaccccgcgctgcagcgcaggttgatcgagatcggccaggacaacgacgacgtctggcgcagtgtcttcctcgagcgcggatcggtgcagcatctgccgttcctggacgctgcggacaaggctctgttcgcgaccgcctcggagaccgacccgggcgtcctgatcgagctggccgcgcagcgtcagcccttcatctgccaggcccaaagcctcaacatcttcttgccggccggtgtggacaccaagacgatgcaccaggtgcacatgcgcgcatggaaggtgggcctcaagtcgctgtactacctccgctccagctcggtcaaggccacctcggtcggtgtgatgcccgagatcatgcgcgagcccacccccgtcgtagccgaagaggtggttgacctccccgaggtgagcggcgcagtatgcaacctcggcggcgactgcgtcgcctgtgaaggctgaggaccacatgaccaacgtacccgtacccaccccgcaggccccttctctcttcgagaagcgggccgagtacaagcccttctggtacccctgggcgtaccaggcattcaccgagagcgagcagatgcactggctcgtgcgcgaggtgcctatgacggcggacgtcaagacctggcgggtcgacctgaccgaccgggagcgccacctgctgacccacatcttccgcttcttcacccaggcggacgtcgacgtggcgtcgggctacatcgaccggtacctgccgaccttcaagcccaccgagatccgcatggcgatggcctcgatcgccgcccgcgagggcgtgcacatacaggcctactccaccctgatcgacgagctcggcatcccggaggtggagtactccgccttcatggggtacaaggagatgctggacaagcacgagtacctgttccagcgccgggagggcctcgagggcctggccctggacatcgccgtcttctccgccttcggggaggggctgcagctcttctccagcttcgtcatgctgctcaacttcacccggttcggcaagatgacaggcatgggccaggtggtgagctggtccatccgggacgagaccctgcacgtcgagttcatgatgcgggtgtaccaccagctgctggccgagcatccccacctccgcacggccgagcactctgagcgcatccgcgaggtggctcagaagatggtggagctcgagttcgccttcatcgacctggcctacgagaccggcgagaaccagggcctcacccccgaggacgtgaagcagtatatccgctacacggccgaccagcgtctccagcagctcggcgagcgcccgctgttcggcatcgacaagaacccgctcgcctgggtggatgccatcgtattcggcaaggagcacaccaacttcttcgagaaccgggcaaccgactactccaagggcgcggtgcagggcaactgggacgacgccttcgacaactgaccagcgccaagctgggaacgatggcttaacctcctgaggggcgacgatacactgtgatcgtcgcccctattcattatccgggcctggcggcacccggtcaggagataccaatgcaacagacctcagggtccatgacccgccatgccccggtcgcacaggtgaccatcatcccgcgcttcgcgcaccgcttcgacgacgtgccgcaggccctccatgccgccctcgagcgagcccagctgaacgtagtgcccaacgccttccgcgtcaacgcaggccgcgacctgttcgagctctacctggagcagttcgacccgcaggaccgccagtaccacaactgcaactgctgccgctcgttcatcgggcgctacggcagcctggtgaccctcacccccgacggcaagaccaagtccgtgctgtgggacgagaccctgctgggctcccgccacccctaccgcaaggtcgtcaaggccctgcgcgaggcggtcgagcgcggccacgtggtggaccagttcttctgggacggcaagggcgactggggtgtgcgcgagcagggcggcttcacccacctgtggaccagcccgggcgtcgtgtcgcactcggcgtccaagggcgctgaccagctggcggccgagcagcgcgagaaccgcaggcacctgcaccgcgccctgtcggagttcaccctgggcgacctggagcgggcccgcgacctgctgctgaccggcggcctcaaccagggcgacaagacggccaagatggcggagttcctgatcgaggccaagcgctcgatggcccacatcgccggcggcgaggccatcaaccggcgcctctggttccgcgtcgccatggctgccaaggggtggtgcaccccgcgctcctcggtgctcggtgccctgatcgacgacatccgctccggcacctcggtcgagtccatccgccggaaccacaacaagcgcgccgatcccctgacctaccagcgggcgcaggccgcaccgaccgccggcaacgtggctcgggccgagcggctgttcgagcagatgggcctcgcccgctccctcgagcggcgcccggcgcgggctgacgaggtggtgttcgactggaccccgcaggtgacggatgccccgcagtcgaccggcggcatcttcagccacctcctggcgcaggaccggctgaagaccgagcgggccctgctcaacgtccaggcggagcgcatcacctacgcccgcttcgtccgcgacgtcctgccgcgcgccctggagatcgaggccgtggtgccccaccagggcaacttctgtgcgatcacgacggccgtccacccggatgccccgccgatcctgcagtgggactccctggagtgccgcaacccgttcgcctggtacgtgtaccaccaggggtcgccggcgtccaactggggcctccgctcgggccgcgtcaaggtggtcggcatcaccaagcagccgtcgcagtggggcggtgaccgcttcgcgcaccacggccggtcggtggtgttcctgctcgagggcgcggctgaccagcgcaatgcctcgctggctctcttcccggagtgcctgcggtccgagctgcacgaggtgcgggccaccctggaggcgcactcccgctccaccaagcttgcacgtctgcgtccgggcgtccagcatgctgcgggcctgcgcgtcgacgaccgcaccccgctcgagatcctggtacgcacctccggcggcgtggccaggtaccagctggaccgcatggattgatggtacgcgtctgactggggaggagccatgataggctcctcccctcttttcaacccctggagaacacaatggacttctcacccccaaacttctggctcaccctggccatcgtactgttcgccgtgtccctggcatggctcgcccgctccatccgccggcccggcaacatgttccgcgctggcatagagtacgcgctggctgagctctacctggcggcggaccccgaggaggcggccgatcgcctgtgggagcagagctcctccgccttcgaggagcccgagagcgcgctcgagttcgaccgcggcatccgcgagggcatccgcctgtacgtgcaggccgacgagagcggcgtccgtgagctggaggagctgcgctcccacctcaccaacatggtgggcaacggtgaggccagcctgtcggaggtcggcgtggccctggacgtcattgaccggcgcctcggtgtcggcggctaccgcaccaccgaggccggcgagcaggcactggagcaggcccatgcgtaagcccctctacatcttcgacctcgacggcaccctggcgacgatcgaccaccgtcgccacctggtggagtccgacccgaagcagtggcgggagttctacgccgcctgcgaccgcgacaccccgtgccaggcggtgatccgcacagcgaacgccctgtacctggcgggcgccgacgtgtgggtctggtcgggccgctccgacgaggtggcggacaagacctcggagtggctgctgcgccacctgtcgtggctgcgggagcacgaccccttcaacagcatggccctgcggatgcgcttccagcacgatcaccagccggacgtgaagctcaagcgcctatggctctcccagctgagcccggacgaccgtgccagactcgtggccgtgttcgacgaccgcaagtcggtggtggacatgtggcgcagcgagggcgtgccctgcttccaggtcgcaccgggggacttctgatgagcttccgtcccatgctggcagcgtccgtagccgaggtcgagaagctccgcttcccgctgcagacctcgcccaagctcgacggcatccgagccatcatccgcgactccgtcgtggtgagccggagcctgaagcccatccccaacctgcacgtgcaggccgtgctcggccacccgctgtacaacggcctggacggcgagctgatcgtgggcgatccctctgatcccatggccttcaacaacaccacccgaggcgtcatgtccatcaagggagagcccgacttccggttccacgtgttcgacgacgtgacccaccccgagatgggcttcaacaagcgccacgacgaggccagccgccgggcggtcgcgctcggcaggcccctggtggtggtgccacactgggaagtcaaaaacccggaggagctgctggcggtggagcgctccgtgctcggggagggctacgagggcctgatggcccgcgacgcctgcgccccgtacaagttcggtcgtggcaccctcagggcgcaggacctgctgaagctcaagcgcttcgaggacggcgaggccacgctgctgggcatggaagagctgatgcacaatgccaacgaggcaaccaccagcgcgctggggctcactgagcgcagtcacagcaaggacaacctgctgggcatggacaccatgggcgccatgacggtgcgcgcgctgaacggcatcttcgagggcgtcgagttctcgatcggcaccggcttcacctccgaccagcggaaggacctgtggagccgccgacacgacctgaacggccgggtggtgaagttcaagtggttccccggcgggagcaaggacgcgcctcgcttcccggtgttcctcgggttccgggaccgcatcgacatgtagcgggcggaggtcgctggctcacaaccagcgacctcctgggctaccatcgcgagcatcagctcacaactagcccaaggaacccgcgatggccgacggacccagcaagaagccgacggtagctacgccgtccggcgcttacctgcgcatgcagccccgatggaagatgatcgacgctctcctgggcggcaccgagaccatgcgcgcggccgggaaggagtaccttccccagtacgacaacgagtctaacaagaactacgacacccgcctggagcgggccgtcctgctcaacatgaccgagcagacgctcgacaccctggcgggcaagcccttccgcgagcagatcgtcctgggcgacgacgtggcggcggacttccaggagatgtccgaggacatcgacatgcagggcagcaacctgcagtcgttcgcccggtcgtggttccgggagggctgggccaagggcctgtcccacgtgctcgtcgagcaccccaccccgcaggagcaggtcgacgaggccggccagcccgtcgccaggacgctggccgatgaccggagccagggcctgcgcccgtactgggtgcacatcaagcccgagtgcctgatcgccgcgtacgccgcggtggtcaacggcaaggaggtcctcacccacgtccggatcaaggagacttctgtcgagcgggtcgactgggaggaggtgctggtggagcgcgtccgcgtgctcgagcccggcatctggcaggtctgggcgcccgacgagaagggcgaggagtggcacatcgagtccgagggcaccacctccctggacttcatcccgctggtcaccttctacgcgggcaagcggtccggcctgatggagtgcaagccgcccctgatcgacctggcccacctgaacgtcgagcactggcagtccaagagcgaccagcgcaacgtgctgaccgtctcccgcttcccgatcctggctgcggcgggcgtcccgtcggaccagaagatcacggtggggcccaacaacttcctcaccaccgacgacgtacagggcaagtggtactacgtcgagcacaccggcgcggcgatcgccgcgggccagaccgacctggagtccctcgaggaccagatggccacctacggcgccgagtacatgcgcaagcagccgggcgacgagacggcgaccgggcgggccctggactcggctgagagctcgtcctacctggcgtccacggtgcacgacttccaggactgcctcgagcaggccatgaagtacacggcgaactggctcggccagcccgacggcggctccgtgcaggtcgactcggacgtggacctcggcgaggccgacgcggccgagctggacaccctcaacaaggcccgcgcccagcgggacatctcccgcaagacctacctcggcgagctccagaagcgcggcatcctctcggacgacttcgacgaggagcaggaccaggagttcctggaggaggaggccaagaacagcctgggcgacatgttcggcggcggcaccggcacaggcctgccgggccagcagcctcccggcaaccagccgccacaggatccgccgcaggatccgcccgcttcggatgacgagtgatgcccaagaccgctaacgaggagatcctcgacgcgaccgtacgccaccagatcaagctgctgcgcttctcccagggggaggcccagatggcggcctccctgctcgccgagagcgacgccgagctggtggccctgctgcagtccaagctcaccgagacgtcggaggcccgcatcaggggcctcctggctgaggtgcgccggatgcgggcggcggtagccgagcgcatccaggtggagctggaggaggacatggagggcctctccaagaccgaggccgagtgggaggtgtcgatgctgcagggcgccacgcccatcgcgctgagcttcaaccaggtgcccgccacggtcgtcaaggccgtcgcgggctcccccataaatggcatcccgctgcagggctggctcggcaccatggcgtcgaacgacgtctcccgcatcgagcagcagatccgcctgggcgtgctgcagggcgagaccgtggaccagatggtgcgccgcatccggggcaccaaggccgctggctacaaggacggcgtcctggagacgacccgccgcgaggccgagatgatcgcccgcacagcgaccaaccacgtgtccacggccgcgcgccaggccacgtgggacgccaacgccgacgtcatcagcggtgtccgctgggttgccaccctggacggccgcacctcccccgtctgccagagtcgggacggcgaggtgtacccgatcgacaagggcccgcgcccgccggcgcacccgaactgccgttcgacggtggccccggtgctgcatggcgaggagatcatgggcgaccggcccaccgtcaccgacacccgcacccggcgccagcgcgagatcgacttccgtgaggaggccaaggaggcggccggcgacaactggaagaacatgtcggcggcagagcggaacgccgccatcaaggctcggcgcgacaagtggggcgacgagaacatcgggcagacccccacctcgaccaactaccagtcctggctgaagggccagtccaaggagttccaggacgacgtcctgggcaagggcaaggcccagctcttccgtgacggcatgcccctggagaagttcgtcgacgagaagggcaagccctactccctggcgcagctgaaggccgagctggagggtgacaagctgaacgtcatccagccgggcgtgggcctgaaggccaagtcgctcctgcagcagggcatgtcccccacccaggtgctggagcagatcaagcaggagttcccggacgcgtccacctcggccgcgtcgatcgcctcctacaagtccgagctcaacaaggccggcgcgctgaacctcccgtctgccgggcaggtgcccacgggcgccctcaagcaggccaaggccgtggccgacgtcgtctccgacctggacgcctccctgccgtccaacctcaagcacgccatcggggaccagtggtccaccgtggtcgacgacctcgacgggtcgccgggtgcctacgggtactaccaggccggcaagggggtgatgcttagcgggaagaagctgtccgccctgcctgccgtacaggccaagcaggtcgcggcccacgagctcggccacctgctgcacaagcagcacgagttgctgctcgacccggacgtcctggcgaccgtgaagtcctcggcgaaggccctgtcgccggacgctcgaaagctctattcgtactacctgtcgagccctgacgagctcgtggctgagatctacggccaggccctgagcccgagtgccctgacgtcccagggcctgtcgtccctggagttcaacaaggccttcgggcccgccatccaggccgccaaggacgcgatggcgaagaagttcccggcgccctcgctgtccgccaaggcccctctgcccggcgggcccgtgctgccctacgaggtcgcgggcaagcacacctcggtcggctcgctcgccaaggcgctcctgcagcagggcatgcccgacgagcaggtcctcaagtcggtcctggctgagttccccggggcccagaccaagcaggcctcgatcgcctcgtacaagtcccagctgaagaaggacggcctgctgcccaacaaggccgccggcccggtcgtgacggcaaagccgatccccgacgtcgtgccggtgccctcctccggtgcgtccgccgtcgtggcccccgaggctgcggccgcgaccccgtccgccctgacgctcacctcggcccagctcaaggacgaggccatcaagctgatgcaaaagggcatgctgtccaaccaggacctggcggagaccctggcgaagcagttcccggcgaacgcggccgacgtcaagattaccaacattgcgacctggaagtccaactggaaaaagtccagcccgaactcctacaaccacgccgtctcgctctccgagaaggccgcggtcaaggagtcgctgtcgggcccggtgcagaagcccaagctggacgggcagaagctcggtgccacctcgtccagcgccctggagaaggtgaagtcggtgctggctgccggcggcggcccgcaggacgcctacgaggccatgaagtcggtgttcggggtcatcaagcagccgggcgccgacgagctgctcgagctggcccagtaccagctggccacggccaaggctgccggcaagccctacctgaacgcgaccttccaggcgccgaaggggttcacctccaacggcctgaccgagaagtacattctcggcctggacgccaagggcaaggctgcactggacgcctacaagaaggcgaagcagcagggcctcgggccggtcaacaccaacaagctggtcaagaagatggcgggctacgagccctcggcctcagccaaggtgaagctgaaggaggccgcggactacgagctgaagaagtcggcggcaggcctggcgcccaagccggccgctgccgcaccgggcgtcaagccctcggcgcccgccacgg

SEQ ID NO: 10 - DNA, 61011 bp, unidentified
  source 1..61011: mol_type = genomic DNA
cgcggggtgcaccagcccgcgccggccatggcgacgttgaaccacaggcgccggttgcgggcctcgccgcggatgccgccgatggacttctgcacctgcaccaggaaggacgccatcggcagcagcttgtcggagcgggcgagcgagccgtgggtcagcatgccctgcaccttctcgagctcctgcagggtgaagtcctgcagcgcgtggttcaggtgcagccggttctggcgctgctcggcgatgagctggtccgcgtccttgtggcccgtgtgggagcgcacgcccgggttggtccacaggtgcgtccagccgcccgcctcgcggtggccccactgctgctcgtcccagaagaactggtcggtgaccgtgcccttctcgacggcctcgcgcatggccttgacgaccttgcggtacgggtggcgggagccgagcttggtctcgtcccagatggcggacttgatccggccgtcgctgtagatggtcaccagcgcgccgaagcggttgatgaacgagcggcagcagttgcagttgtggtactgacggtcctgcgggtcgaactgctggaggtagagctcgaacaggtcgcgccccgggttggagcggaacaggttgggcacgatctgcagttgggcgtcgtgcagggccgcgtggatggcctgggtgacgtcgtcgaagcgctgggcgtatcgcggcacgtggccgacgtgggccgcgtggccctggtgcgcggtggtcgccgcgccgagtgactgttgcatgggtatctccttggccgggtgccgccaggcccgggtaagaataaggggcgacgctcacagtgtagcgccgccccctgcccatctaaaccatcgttcccagctgggacgctggtcagtcgaacgcgctgccccagtccccggtcatggcgcccttcgagtagtccgtcgccctgttctcgaagaagttggtgtgctccttgccgaagacgatggcgtcgacccacgccagcgagttgcggtcgacgccgaacagcggcctctcgccgagctggccaagccgctggtccgccgtgtagcggatgtactgcttcacgtcctcggccgtgaggccctggttctcgcccatctcgtaggccaagtcgatgaaggcgaactcgagctccaccatacgctgggccacctcgcggatgcgctcagagtgctcggcggtgcggagctgggggtgctcggccaggagctggtggtacaccctcatcatgaactcgacgtggtgtgtctcgtcccggatggaccagctcaccacctggcccatgcccgtcatcttgccgaaccgcgtgaagttgagcagcatgacgaagctggagaagagctgcagcccctcgccgaaggccgagaagacggcgatgtcgagggcaaggccctccaggccctcgcggcgctggaagaggtactcgtgcttgtccagcatctccttgtagcccatgaaggcggagtactctacctcagggatgcccagctcgtcgatcagggtcgagtaggcctggatgtgtacgccctcgcgggcggcgatcgaggccatcgccatgcgcacctcgaccggcttgaacgtcggcaggtaccggtcgatgtaccccgaggccacgtccacgtccgcctgggtgaagaagcggaagatgtgggtcaggaggtggcgctccctgtccgtcaggtccgcgcgccaggtcttgacgtcctgggtcatgggcacctcgcgcaccagccagtgcatctgctccgaggccacgaaggcctcgtacgcccaggggtaccagaagggcttgtactccgccctcttcgagaagagggacgggctgttgtctaccatcatgtcggtctccgttatccttcgcacgaggtgcacgcctcgccgaggttgcatactgcgccgctcacctcaggcaggtcaaccgtctcttcctgctgcgcgggctgcggctcgcggaggatctcgggcatcacgccgaccgaggtcgccttgaccgagctggagcggaggtagtagagggacttgaggcccagcttccaggcgcgcatgtggacctggtgcatggtcttcgtgtcgacgtcggccggcaggaagaggttgaggctctgggcctggcagatgaagggctggcggtgcgcggccaggtcgaccaggacgcgcgggtcggtctccgaggcggttcggaacagggccttgtcctcggccgacaggaacggcaggtgctgcaccgagccgcgctcgaggaacacgctgcgccagacgtcgtccgtgtcgtggccgagctcgcgcagcctgcggatcagcgcggggttcttcatgatcccggtgccagccatcgtcttctgggagaaggcgttcgccaccatggactcggtgctcgggctgacgccgccgcagatgatggagctcgtggcgttcggggcgatcgccatcaggtgggcgttgcgcaggccggtcccgacgaggtcggtcggctcgccgcgttccttggccaggcgcatggacgccgctacggcgtgggccttcagctcggagtacagggtgacgttgaaggtcgccgcctcgtgggactccatggcccagcgcttgtcctggaggtaggtgtgcaggccgagggtgccgagaccgatcgaccgctcggcgcgcaccgactggaccgcacgccacatgcccgggggcgcccggtcgcagaacacctcgagcgcgttgtccagcatggtgacgaggtcggccacgaactgcttgcggtcgtcccaccactcgtcgagcgtggcgacgttgacggaggagaggcagcagacggccgtacgctcggggctcgtcggcagggtgatctcagtgcacaggttcgagtggcggacccggaggcccctcgccttcagggcggggtgcaggtcgcggttggcggcgtcgatgaagaagaggtagggctcgccgaggcgggcgcgctgctggagcatctggatccacagggaccgggccttcagcgtctggcgcacggcgccggagtgcgggtccaccaggtcccagtcggcgtcggcctcgacggcctgcatgaaggcgtcggtcacgttcacgccgtggtgcaggttctcgttcttgcggtggacgtcgccgccggtcggggaccgcatgttgatgaactcgacgatctcggggtgggagacgtccaggtagactgcgtgggcgccgcgcctggtggagccctggtggtaggcgatggcctgggagtcctggacgtgcatgaaggccatcacgccgggcgtgtcgacgcccttgctggtcacctcgccgatggagcgcacgtcgccccagtaggtgccgatgccgccgccgttggtagagagcagggcgttctcgccgaagttcgccaccaggccctcgatggagtccgcgacgtggttgaggaagcaggagatgggcaggccgcggttggtgccgccgttggcgagcagcggcgtggcgaacatgaaccactgcttgctggcgtagtcgtagaggcgctgggcgagggcctggtcccctccgctgaaggcatgcgccgcccgcgcgaacgcctgctggtgggactcgccgggcaggcagtactgcttggtcagggtggcgacgccgaactcggtgaggagggcgtcgcgtgcggggtcgaggacgatccccgtcttctggtcgatcatggtgtggctccgtgctgtcggttgttcgggagggttgcgaacgcgcatcgtgacgcgcgcgtacgcactgcgcgagccggcgaaaagaaagccccgaccctcgcgggccggggctctcaacccttccaaccgatggaaccgcatggccggggtgtccaggcccggcaggagcatgatgccgcggcggccgcggacgatgaagccgtcgtaaagcaacgaggcccgcttgcgcgggcctcgaggggccgtctggtgaccaggtggccgatcctgggctcaggccgcgatggcctgggcgtacacgctgtcgttggcaggtgtggtttttgcgctgctaggggcagtcgcctctccggctgtccactctgcatgctcgccccgtcgaaacctgggcaggcccatcagatgcgccccgctgtccgcggctaccgctggacatgccggcgtgcagccggagatgggctgcttgcctgggttcgcgaccccagccgacaagggcgaggcgcatctggtggacctggcgggaatcgaacccgcgtccgagacgcatccgcgtcgcttcatacagccatagcagggagccgtggggctggcatttgctcatcccccgatattgaactccgaagtcgttgccagtagcctcggggctagcgggctacctcacgactccctgctatggcggcactgaggagcgccctgagggctcccgccaggtcttacgggaggcggggagacctccctgggctgcctggctcaggcgtgcactcctgtgaacatcatacagggcgctcgtcagtaccgccgccccgtatagccggggccacgctcgacgacaacctacgctctcgcgctggtgtctggttggaggagatgggatcgaaccatcgaccgccggcttatcgggccggtgctctgccagctgagctatcccccagtttggtagcggaggtgggactcgaacccacgacctccgggttatgaacccagcgagctgccagctgctctactccgcggcattggtgccccgccctcgggtggacctccgggcggggcgtgatgagaggttgatcctgctgcgagagcccaggtcaggacggcgacctgcatcacccctgaactctgcctaacgccgtctcatcggtcgacgcgtcggaggatgggtgtatgatgcggggcggacccggccacgaacacgaacaccatcactttcgcagccggtgcgctgggttagaaggacccctggcgcacctccttcctcttgtgcatcacgcggtagcggctctcgtccgccgagtggtcctcgacgtcggagtcgacgtcgtccgggtccttctcgtcgcgcgggatgggcacaaaggtgcgcacgaagtcggggcaacgctcacccaccacgtacaggcccggcgcctcgcgcggcacgcccctgggctggtccatctcgtccaggttgagggagttcttcaggcgcttgcgcacctgctcccagccctgcttgcgggcgttgtcggcgcgctcccaccggatgcccttgttgcgcatgtcccgctcgatgcagttgccgttctcctcggaccagatggccgggtctgccgggccgggcttgaccctgcccgccaggccgaggcccacctcgcgcagcctgatgccctcggcgatgtcggccgccagcatcctcaggccctcgttctcggtgcccttcttgaggccgtaccactcggcgatgcggaacaggtcgcccttgacagtgcgcatgcgcctgccgtcggggaagaccaggtccgtgccgtccgactcggcccaccagccgaccgagaagggcttgctcgagccccagtcgaaggaccggtccaccgtccaggtgcgcggcacctggaagggcctcaccacatgcgtggtcgtctgccacaggtcgtcgaacatgccgccggacgtgatgtcccagctgccgtcgagccacgccgcgatctgggcggggttcgaggcagcagcgcggatgcgggagatgtactccgggtcggcgtccagcaggatccggttctcggagatgtgcccgtggatggcgatgcggtcgggctcgccctcggtcctgatgaccttgccgcgcatcccaggcaggcgccaccggttcttgacccagttgtgccccttgccgtacgggttggtcgtggcgcgcactttgcggggcatgccaggcaccgtcgagcggcagcaggagaacatcttgaggtacatctcgctggtggcccagttggtgagctcctcccagccgatccacgggtacgcgtggccgtggtagttgtcgtagtccgcgggcttggacatgtaccgcaggaggagctgctccccgtctgggaaggtccaggtgtactcctgctcgttgaacttggcgccggggaaccacagcttgaaccacgccttggacttcgccacgacgtcggacagctgcttgtaggtagagcggaagaggatgccgcgccaggccgcgccgtagccctgccccacgtgctggcagaagtcggccaggagcgcgtcggtcttgcccgggccgcgggtgccctcgtacaggcactcgaacacggggcacgtcaggaagaggacctgggagcccgcctgggggatccacgccttggtcgtggaccgcccctcctctacgcgcgcccggccgaccttcttcctccgccagtgcgggggctggtacgccatcactccacctctaggtccttgagcctgccgggccgcgcgaccaggtcgcgcacgttggccagcatggcgctgttgatgccccacagctggcggagcacccaccacgcgcacttcaggcgctgcctgagcggggtgtgggactcgccgcgccagaaggcgttgggccgcgtgcagtagaagccaccccgcatcagggcgacgtgcatgatgggttcagccatccaggcgtcgccctcctccatctcagagaggatgaccgcgccctgcctcgccgcggcgagcgccaggtacgcggcgtccagcttctggtccccggtgtccgtgggcacgcgcgacgtgcccttcaggcaggacgcgcagacttcgcccttcgagtcgacccagacctccaggatcatgtccgggctgcggaagtccgcctctcggctgtcacgcgcctcacgggcgcgccggatgtcggtgaccttgtccatgtcagcgacgctccatcctggtggcgcactcgatcgtgagcccgtaacccagggccaggcggcgcgggtccacctcattaccgcacccgcaggcgcactccccgtcctccctcggtgcccagcgcttgcgcgccgcctccgccttcctcctcgccgcgtcgaccgcggcctcgtcgtgggccaaggcctctgcggacgcgcggtccactggatccgggtggtgctcggctggctggacttccatcgctgttctcccctgttggtctgttggtaggtgctgcatgtgatgagggcgcccgaattgggcgccctgtgtgctagcgagtagtcattatcccgcggaggactcgctgtctccgccctcgttgttcccggcgtacttcgcctgctgctcctggacggtcttgtaccaggaggcggggtcgaccgcggcgggcaccaccaggacgccgccggcgccgccgacgtgctcgaccttgtggttgtcgcggtacttgtccggacgcgagcccttaagcagggtctgcatcagggcgtcgctgtacttccgcacgaagagctgcttgtcctcgccggtcacggcgtccttgacgactgtcggcatgccctggtagatcacgggctcgtcgtagccctcgaccgcgcgccggaaggcctcgccctcgatgcgatccgcggcctcctcgatcgcgatggcgtacatggtgtcgaaccactcggaggtctccctccagtgctcgacggcgccgcgggacacgcctgccgcgcggcagccgtccaggacgatgccacgcagggcgaacgcgcggaggaacaggcggcgccgctcgatgctcaggcgctcctgggtggtgaggccctcgagctcccactccaccagctcgagctccgacacggggccgcgctcgtggaggaagagccgctcctcgtcggtcatgttcttggcggtcactgggccgctccttgggtatgttggtgcgatggtccgatggtagcgccgcccggcctgggtcgtaagccagcacggctcggcgggccgctccctcggtccttcgtgcgcgaggcctcctgggccgcggtcggacgcttttcaacgtgaagcagtgaagggatgaggggaaacgcgcgggccccgggttcggccacggctgggccggacgagggaaaactcctatgcggcgtcgcatccgacacgcccagggcggactcgccggccggttccctcatttgccctagattgtcaactttactggataacttcaggataggattggtttaaaggcttagattatctaaacccttattaaaaaggtctagattaactaaactaatgattttcaaggcactttctccccgaatctgaggatctggggcatctgaggcagtaagccgtggtgccgtctctccggtggtgttgtttttcctgggacaacacggcgcaaaaggctcgtacggtccgtacgccttagacgaacgccgcaacgtcttgatccgtaaagaaaaagccagcctagatgcgatctaggccggctgttcgagggccttagacagcccagattccccgcgaccgtggccggccgcggcccctccgttagtcgagcgcgtcctttggccacggcaccttgctccccagcttggcctccatcatctcccggcagtccgccaggctcggcagcttcgatgccgacgcgcgtcccatgcggtcgaccttgaccgtgtagtccgcgtcgtccggcttgacctgcgtgttctcgagcctaccgcccaccagcttgttgaggcgcatcccaaaggcgaccgggtcggcgggccggtacacgcgctggtccttggcgaactccgcgtagtccgccctcaggtgctccttgatgaccgtgacgctggactcgtgccagtcgccccgcgcgttcggcaggatgccgtccagcagcttgttgtaccaccaccgctcgacgtcgtccatcgtcatgaccttctggtcgacgagcgcggaggtggtgggcacgtcgtcgcgcggcgcccagccctcgatgttccgcttgagcaggtcgtacagcatggcctcgatgccgccctcgcggtacatctggcggttgaggcgccggaagaactccttgtccccgcgccgcttgctgttcacctggaagaccgcgaagcgccgctcgccgtccaggcccgcggggaccacccagtcgccgttggcggccatgatgatgtggatcatgttcttgccggtgaccgcgtcccggcccttgccctcgtacgcgatggtgggctcggtgaccagctgcttcagcttcgcctcgcccgacttgtcgccggcccagaaggcctcgtcggcgaacaggcagatgcagttctggaggtgcgagttgaaccgtccgacgaggtgctccggcgagctgatctgcaggccatgcgagcccgccagggcggaggcggcgcgaccgagcgtgcccttgccggtgcccttctcgcccttgaagcagagcgctacctcggcggcgtgcgacggccgctggaccatgtaggcgagccagttcatcacgtactcgtaggaggcctcgtcaccgtccaccaggacctcgcggaccagctcctgcagcagggaccagtcgcccttcttgggctgcacggcccagccgcgccacaggttcagccagccctcgtggttgctctcggggtcgaagatgacgccgtcgtactgtcggcggtgcggcgacctgatccacagcgaggaccgcgtcaccagcttgtcgtggatctccacgagctggttgcagtacaggttctcgaagtcctccttggtggagcgctggaagaacggcctcttgaggaccgggtccatcttctccgtgaagatacggaacttgccgccctccatcacgacgcagtgggcttcgttcatctcctcgagcacacccatcacgccctcagacttgggctcttcacggagcaccgcatcatcgacgccctggccgagctcggaggggtcctcgtacacgtcgaagtcgtcggcggcatcggtgcgggtgacctcgccgcccgcctcctgcacgaccttgtggaggaacttgatggtgacggggcggccgcccttgccggaggtggcgtgcagcgagtcccaccggcggccgatgatccatgcgtcgtcctggtacttgacgtcctgcgtggaccactcgatgaactcctgccgtccttcgccgttcgtggcgtggtggcaggccatcatcaggtcgcgccacctgtcatggtcctggaagtcctcggcgtccagctgctcgagcgtcgtggcgagcatctcgggggtgagctcgccgagccctgcggcctcgccgtgcgccctggtcgggcggcgggtcaggcgcaggagcgcgccgggcatcggtggcatctcgtcgaggtgcggggcgaggtcgtcccactcgtagtgcttgccgttcgggtgcacggagcctgcggacacgacctgacgaccacgcgacttgaactcgatgccctggtagtcctcgagggagtccagcaggtcgacgtcggacggcttggtgaaccagtagtggtgcccgcccgagcccgtgatcgtgtggggcgccgtggacaggtcgagccccatgtcggcgacaagctcggccagggagtcgcggcccttggggaagttgcgcgggtcgacgtcgagcaccatgatgtttgacggcaggcgcacgcccacgttgatgccggtcttctcggagagctcaatgacctgccgggagtcgtagtccttcgcctgccaggcgccgtcgcggggcgtcttgccgcgctgccggcccttgccgtccacggcgtcgtacttgtggagcgggatgagctggagaccggcctctacgtacgcgcgcatgtcccccgtgcgcggtcgcttatttgcggcggtcatgcccgcacctcggccttcctggcggcggccgcttcctcgatgatcgcgcgggccgcgtccgcctccgtcaccttctcaggctcctggctgcgcgcccggagctcctctagtttctcccgcaggatcctgcggtggtcctccgaaacccggagggacatctgctggctcagtgccacgtgattcccctttgcttgttgcttgatcggctcgacccggaggtcgggatgagcatagtgcgacgacgcagtgcattgcgtagaccgccgaacgcactgcgtccgctttgcggggaccatcgcccgtgaacgaaggctccgcatccggggcccgggcggtacagtgacactccctaccaaccgctcaacaaggagcacgcaagatggatgtcaacgagttcatgagcaagagcctggagcaccaggcgaagcagaccgccctgctggaggcgatcctcgacgggatcaactccatcaacgagtccggcgtcgccgtggtgaaccaggtcagcatcgccctgccggagggcaccgacctcaaggccgtcggcaacgtggtgcacgcgcagcccgccgacaaggtcgagaagaaggccgagccgaagcaggtccaggccgacaagcccgccgagaccaagaaggccgacgccgagccggcggctgaggcacccaaggacgacaagcccgccgagaccaagaagaaggtcaccgtggacgacgcccgcgccgccctgaagaagtacgcggcgatcgagggcaacgacgcggcgatggagctgctgaccggcctgggcgcggcctccgtgtcggcgctcgccgagaagggccccgaggccctgcagcagctgatcgacaagtgcgaagggaagggtgagtaagtcatgagcgagcagcccaacatgaagatgcccaaggacgccgcgcaggtggtgttctggttcaagggcctcccgcagcccaccgccttcctcaccctgcgcgacgaggccgataaggccgtcgaggccttccgcaagcgggaggagaccatctccttcctttcgtacccggacggccgtggcgtgcgctcggagtcgaccttccgggtcgacgagctgcgcggcgtgacgatcgagtaccccaccatccaactcgcgacggtgaactgacatgcccagcgcccacgcagtacgaaacgcgtcgggggcgaagcggtggatgaactgcccgggctccatccgaatggagcacgggcggcccaacaactcctccgacgccgccaggctcggcaccgcggcgcacgcgcttggtgaggcctgtctgctcgacggcagcgaggcctgggagtggctgggcgggtacgtccgcctcgaccccaacgagcaggccacagtccacaagccagcccaggccttcctccccggcgacgaggagaagacggtcatggtgcccgtgcacgcctcggaggagggcctccctcccgccggccacgaggacttcccgatcgacgccgacatgacggacgccgtccaggtctacctggacgcggtcagggcggagatggagcgcctcgggccccacgccgagctcgaggtcgagcgccgcttcagcctcaactggctgatcggcttcgactacgacttcgacgaggaggaccgcatgcgcgaggcgggggactactacgtctccccttcgggcatccgccgcgacgacgagggcatgctcaggcacgccgacggccgcgtgtcgtggggcccgatgttcggcaccaacgacgcctcggtcggcctgatcttcgaccacatctccgtcttcgactacaagcacggccagggcgtcgtcgtcgaggtggaggacaacgagcaggagctgtactacgcgctcggcaaggcgcgcgaaatggactgggcgttcgagaccctcgacctcgtcatcgtccagccgcgcgcccggcaccaggacggcaaggtccggcgctggtccaccgacaaggccaccctgcgggcgtacgaggagcggctccgcgtggccgccatcgccaccgaggagccggacgcccctctcagggcgggcgactggtgcaagttctgcaaggcggccggcgtgtgcggggagctccgagaggaggccttccgccaggccggcctggagttcggcgacggctttacggaggacagtgcgatgacgagcgggcccgaggacagcgacgaggacctgatgctgcggatgcgggcgatcccgctgctggacgtgttcatcaagtccacgcagaccgaggcgctgcggcgcctgcgggagactcctggcggctcggcctgctacggcaagctggtccgcaagaagtcgaaccgcgccttcaggacggacctggtggacgaggtgacgggcgagcccgtgacggcgttcgacaggctggtcgaggcgggcatcccccgggagatgctgtacgaggagcccaagccgaagtcgcccagcaaggtcgagtcggtccggccgcccgagctgatggcgaggctgaaggccgagaaggtcagggcgcccgcggcgcacatcaaggcgctcgtcgccgaggtgtccttcaagcccgagggtggcatcaccgtcgcggcgccggacgatccccgcgaggcggtcgacccgacggcggcggcggagagcgacttcgacgcgttcgacggcgagcagagtgcggactgacggtccgcgcgggaacggggcgggagcatgattgtgctcccgcccttctttttcacaggagaccaacatgagcaagtccgaccgggccggcgagcacttcgagcagatccacgaccaggtgaatgaccagcacctcgcgtcgatcggcgtgggcgacggcagcggcaacctcttcgtcaaggggccctacgaggccgtcaagcgcgtgcagcacttcatcctcgagaacgagcagctgcgacgggacaggcagttcaacgggctgacggcggccgagcacgagcggctgtccatcctgatggaggagatggccgaggcccagcaggtcatcggcaaaatcctccgccacggcttcgagagctcccacccggacgcggtcgagaccaccaaccgcgacctgctcgagaacgagctgggtgacgtgacggcagccctcgagatgctcgtctcggccggtgacgtcaacaccctgcgcatcgccgaggcagcccgccgcaagcaccgcagcgtcaagcagtacctccaccacaactgacaggaaccagtccaacatggaaatgaaacccgcattcgacgacgtacaggcaggcccgacgccccagcagcaggccttcatggagcagcagcgccgggagcagtcccagctcaagcaggacctgctggacttcgtggcccaggagctcccgatggtcaagagcctggcgtcgcagagcaagaaggacctggcgcgtgaggtggtgcacctgcgcggcatggtcaagaccatcaagaaggccaccgaggccgtcacccccggtgcggccgcgttcggccacgccgaggcgttccggctgatggagtacacccagaccaacgccgccgagggcgaggagccggtcgtgccccacgtctggaacagccgcgacggcgtgacgcccttcatcgtccacatcggcgcccagacgttccagtgcacccgcccgatgggcgagatgctgttcgacctgccggcggcagcgacccacaagtgggtgacccgcaccgaccgcgaggtgctcgtggcctggcagcgcacgctctccaaggcggtcgagcagggcaagctcgaggcggacaaggccgagaccatgcgggacaacctggcggtcgcccggtcctggcactacggcatcgggctcgtcaacctcgccaccggcaagttcaccgacgaggaggtcctcgccgatgcgtgacgtcaaggtgttccatctctccggcctgcgccagcctatcgcaggcgacgtcggcccgggctcacgcattgcctccaccgccgacgtggtcgtggacctcgagacactgggccgcggtgcgggctgccaggtgctggaggtcgcggccgccgtgctccagcccgacggccaggtcggctacttccaggcgcacccgagcctcttcgaccagaaggccctgggcctgaccgtcgacccggccaccctgctgtggtggctcgaccacgcgctccgaggtcctcgcccaccacagggaggaggcctccaggcccgcccgctgcggtccgtgctgctgggctttggcgactggctgcacgagctgggtcagacccgcgaggtccgcctctggggcaatggcgccagcttcgacctcggcatcctgggcgccctgtacgacgcggcgaacctgccgcggccgtggaagttctgggcggagcgcgacctgcgcaccgtcttcgacctgaagggcaagatggtgctggaccgcgtcaccggcaccacccacatcggccgcttcgacgcggcgcacgagctggcgcagctctacatcgccctcgggcagaaggactgaacccatgaaccagatacccaccaagaccctcgtgctggtcccctacgaccagatggtccgcaacctcttcaagcccatgggcacgcaagcggccaccgtcctgcacgccgcggtcggcatcgccggggaggtcgcggagctcctcgtagccgggtccatcgagaacctcgtcgaggagatgggcgacatcgagttctacatcgaggccgcctaccagagcactggcgggcgcaacttccccgagctgatcgtcgagggacacgacatgtcccagcaccaggtcttcagcacggtcggcacggccctgtcggtcaccgccggcaggctgctcgacctggtcaagaaggcctgggtgtacgagcaggagctgaacctcgacggcgtgcgctacgagctgatgcgcctggagctgatgctcggcaccatgcgggagctcctgagcgtccgccgccccgacgtgctcggcgccaaccagaccaagctcggtaagcgctaccccgacggcgtctacaccgaccgcgacgcgcaacagcgcgccgacaagcagggcgtcgagttcgactgatctacccacccgccaactctgaaggagagaacaatggcaaccagcaagaaggcggcaaagcccgccaagaagcgcatctccaagccgtctgacccggcccgtgtacgcaccccgcagggcttcctgcgcatggcgatcgagctgcgcatcatgcgcatcaagggcttctacaccaagatcagcggcggcaacaaggccaagggcgagcgcggcctgtacgactactgcgtggaggtggctaccctctgctcccagaagcgctaccacgaggcccgcctcgccgtcagcaacctgccccagaagtcgtacaccggcctggacgtcggcctcgagcaggccatcatccgggaggaggtcgactcctacatccgcgactgcatgtcccgcgacaccaagttcggcatggaagcggacgtcgtgacgctcgacgacggcatcgccgtggagcacaccctgggataatgcgcatctgccccgacgtcgccgacaagccgctcccgctacccgcgggaatcttggcggcaaacagacccggcgtcggggcaggcttcaggctaactcgcctacatcgtcaactgtctcgaatcctactaaggagcaataccatggcaaacgccaagcccaacgaccgcaaggtcacgtcccccaagttccgtgccagcttcgcctgggtgttcaagccgcagcccccgatggagggcagcactggtgagccgaagtacggcgtcaccatgctgttcgacgcggcggcccgcaagaccccgcagttcgaggccatgaagaagctggcccacgccgcggcgaaggagaagttcggcgacaagctgaagccggacggcaacggctggtaccacggcctgcgcaaccccttccgcgacggcgccgagaagtcggagctggagggctacgccggcatggtgttcgtcgccgcgaccaccaagatgcagcccggctgcgtggacgcccagctgaaccggatcatctccgacgaggctggccccgagggcttctactcgggctgctacgcccgcgccaccctgaccgcctacggctacgacaaggcgggcaacaagggcgtcgcgttcggcctgcagaacctgcagaagatcgccgacggcgaggcgttctccggccgcgtggccgccgagaacgacttcgactcggtggacgacttcgtcggcggcgaggcctccggcgagggcaacttcctggactgacgggtccgggatcgaccgccccggtcgagcgcactgccgtgaggcggtaagccctggaaggggcccagcaatgggccccttctttttgcccattcaatggcgtcccagggcgaaacagtccggcaagatagccccatcaaccctgaggacacgacgatgtctgacaccaacgttcacatggagctcgtggaccagcgcaacgaagaagagcgctggcgcgaggaggccgcacggaggctcgcccccgttcccggccagcgcgaggcactcgaggcgttccgccagcgccagcaggcccagaagaagggcaagttcaagcgcgtgctgcgcttcctgaggggcggccggtgagccccaccgtcaagatgcgagacggcatcgaggcggcaggctaccagttcctgaaggacgataacggctgggccctgttcgacctcgacgacaggtccgaggtgcccggcacgaggacgaggcagtacggcaacacgatatgggccgcggcatccgcgctcggcctggacatagactggagcaaggtgtgatgtaagaggaacgcaggaagaagctgaccgagaagctcaagaagtgcatggccctgtcgaagagcccggagccgcatgaggcggccgcggcactccggcaggcgcagaagatcatgtccgagctgggcatcaccgaggacgacctcgacggcctggagatggcagacgcggtcgtcaagaccctcgagggcttcggccgctgccgcaccatgagcgcgctggccaacatgctggaggacgccttcggcgtgaaggccgtgttcgaggccaaccccggctccgccaaccggctgaacgtccgctacatcggcccgagggcgcgcgtcatgctcgccgagtacgcccacaaggtcgtgtggcgggcgatgcagtcagcttgggacgagctgctggtcacccgtccgtggatgaagtccgacggcggcaagcggcaggccttccacctcgggtggctgcgcggcgtgagggagaaggtcatggcgatcgccccgaccgaggccgaggagaaggccatccagcgctactgcgaccgactgtaccgcggcgggctcgtcacgcaggaggcccacaagcgcaagcaactggacgcctcggcgttcctggcgggcaacgcggccgccgccaacttcaacctccaccgcccggtggaggagcagcaactctcgctggagcataaggcatgagctggctcaagaccctgatgtggatcctcctgaccggcggcctcaagtcgaggctactgtccatccccgagcaccagccgttccgcgtcgtcaaggccggcggcaggctgctcgtcgagcccattcccacccagatggaccccgagcagccagtccacttcgacgtcggccagcgcgtgatcgtggcgccgcacgccggcttccaccgcggggcgcgcggggcggtcgagttccacgctccggacggccgcgtctgggtgctgcgcgacggggcgggctcggtctgcttctactacccgcacgagctcatcaaggacccgtcgtacgaggtgaccccgtgaggtgcgcccagcacggcgtcctcgagccgtgcccgctctgcgccctcggcgcctggccactccgcgacctcaacgccctggccgactttgcgggcaagcccgtcggcggcgaaggcaccctcccgccggagcagaggaccgttcgcctgtcccaggtcgtccggtcgataggcaggcgctggaccgagatagagcgggtcaagctgaccgccctgaagccactgtacgtcaccaagaacgccctggtgcgggaggcccgcatcggcgcgatcgacgtcggcaggctcgagagggcggcgctcgccgtggcgaagggcgcgacggccgacccggacccggtggtggacgcgtacgtgcgcgccatcatccaggacgaggtggagtggtagttggctcgcccagttcgggctccgcggcatcatggcagtccgactgaggaggcgcaatgaccataacccagacctaccgcgacggcgagctggtctccaccgtcaatcatggcggcagcgagaaccagcttatcggcgggcgggactacgatgaggccgtgaggcgtcgggagcccgaggtctcccgcgtggcaacggccgtcaagtccgccctgttcaagatcgcctcggcctccgtgtacgagacgacgggcatccactacgagaccaatgcccccaaggcgacgatcgacttcgagacccggtccgcgtgctccatcaaggactgtggctcctggcggtactcgctcgaccccacgacgcaggtcatgtgcctggccttccgcctcccgacctgggagaagggccgcaccgccctgtggcaccccgcgttcccgcacctcggcatcgaggaggccgactgccccgagctggtcgagctgttccagtggatcgccgagggccgcctcgtcgaggcgcacaacgcgtggttcgagcgcggcatctggaccaacatctgcgtgcccaagctaggctggcccgcggtcggccacgagcagtggcggtgctccgccgccaaggcggcggcgtactccctgccgcgcaacctggagaacctgaccgtcgcgctcgccctcaaggtcaagaaggacaccgagggcgccaaggtcatgaagaagatggccaagccgcgcaagccgctcaagcgggacgtgcaggcgtggctggacgacaacgcgaccctcccgctgcccgccaagaagtgcgtgaccacgctgtactcgaacgacgacggcacctaccgcgtcgtggcggagtgggacggtgggtccgaggagcacgacctcccgctcttctggaacgagagcgccgagctgctcgagcgcctgtgcgcctactgccgcgtcgacgtgctggccgaggaggccgcgtccaaccgcctgagggacctctcccccaaggagacggagatgtacctcatggaccagcacatcaaccagatgggcttccagctcgaccgcgagggcatcgagtgcgcgctggagatcgtcaacggcatctacgccgagctgaacaaggagctggtggagctgaccgagggccaggtccagaaggcgacgcagcgcgcccgcatgatggcgtggttccaggagaacggcctgccgctggaggacacgcagggcagcaccatcgactcgtggctgaagcgcgaggacgtggacccgaaggtgcggcgcggcctggagctcgtccgggcgctcggacggtcgagcactgccaagttcgttgcggcccagaactgggctcacccggacacctggcgggtgcacggcgggctgctataccacggcgcgggcacgggccggtggtccggctccggcgtgcagccccacaacttcccgcgcggcaacatcaagaacatggagctggcgtgggaggtcatcaagtcccgcgacctggctgccatcgagatgctctacggcgacgccatggagctgctgtcccacgcgctgcgcgggatgatcgtcccgacgccgggcaggcggctgatggtggcggactacgcggccatcgaggcccgagtggtgctctggctcgccggggacgacgaggccctcgaggtgttccggcggaacgagtgcatctacatggcgatggcgaccgagatctacggccgcctgatccacgacaaggaggcgcaggccgaggagcgccagatgggcaagcaggccgtcctcggcctgggctaccagatgggggccaagaagttccaggccacgctcgccgagaagtacgggatcttcatcgagctggagttcgcccagaagatcgtcgacgcctaccggaacaagttctggcgggtcaagaagatgtggtgggaccaggaggccgcggcgatcgccgccgtgcgcacaccgggccgtgtcgtcaagtgcggccgggtgcagtggtgctgcttcgacgggttcctgcactgcaagctgccctccggtcgcctgctgggctactgcgacccgcgcatcgtcgacaagccgacgccgtggggcgagaagaagcccgcgctcacctacatgggcgtggacccctacaccaagaagtggcgtcgccaggacacctacagtggcatgctagtggagaacatcacccaggcgaccgcccgggacctgatggccgacgcgatgctccgctgccacaaggagggcctgtacgacgtgatcctctcggtgcacgacgaactcatcgccgagtgcgacatggacaagggcgacgtgaaggacttcgaggccacgatggcgtacacgccggactgggccgagggatgccccgtgaaggcggagggctggaccggcctgaggtacaggaagtgagatacaagatccactggaaccgcgatgcgggcgggccgtacaagtcggcctcgacggtcatcacacgggacgagctcgtggtgtggaccacgcccgccctcaggtgggccgtgggctggcgcatagggcacctgctcgatgccctgtaccgcaagatgtcccgatgggagctcgtcgggcaggagtgccaaccgcgaccggagaacatcgagtgaccccgcagttccgactacccaactacaagcaccagcaggatgagtgggaccgccaccgcgacgacgacgcccgggccctgctctggcagatgcggacaggcaagaccaagtccgtcctggacctggcgtgctaccgccaccagaagggcgacatcacgggcgtgctcgtgctcgcccccaacggcgtgcacgtcaactgggtccgccgccagctgcccgtccacatgtgggagaccgtcccgtacgtcgcccacgcctggcaggccagcgaggcgcacaagcccggccacgcggcgtcgctcgaccggtgcctccagtaccgcggcgacggcctggccgtgctcgccgtcaactcggagtccatcatccacgacaagccggccgcggtcatcaagaagttcctgcagcggcacaagggcaaggtcatgctggtcgtcgacgagtcccatgactaccggtcgccgggctccaagcgcaccaagcgggcgagggcactcaagcggtactgccgggtccgccgcatcctgacgggcacctcggtgtccaacagcccgctcgcggcgtacagccagttcgagctgctcgaggaccatgccctgggcttcgctaccttcggggagttcgagtcccactacgcctactacgtgcaggagcggacgaagggcggcaggtcctacgagaagctcgaccactaccgcaacctcgacgacctgcaggagaggatgtccaggctggcgtccgtcgtgctccgtgaggacgtcgacgacatgcccgagctgctgatggacccgaggacggtcgtcctgccggaggccatgcaggcccagtacaccacgctgctcaaggagctgatactggagctcgaggagggcggcgaagtggaggcggtcgacggcggcgcgcggatcatcaagctccagcagctgctcggcggctgggtcatcgacgcggacggcaacgtgcgcgacctggtgacggacgaggagaacccgaggctgcagggcatgctcgaggacgtcggggagtccgaccggaagtgcatcgtgtggtgcaagttccgggaggacatccggcgggtagtgcgcgtgctgaccaaggcgggcgtgcggtgcgtcgagtaccacggtgccatccactcgcagtccaagcgtcaggcggccatcgacgccttcaacaacgacccctcggtgaaggtcttcgtcggccagcccaaggccggcggcgcgggccttgacctgtcggcggcggacgtcatcctctggtactcgcacaccttcgacctcatcgagcgcgaccaggccaacgagcgcgcgacccagatcggcggcaagaccgtcaccatcagggactacgtcacgcccaacacggtcgacgagtacatcctcgccaacctggaggcaaagcgctcggtgtccgagtcgctcgccgggcgaggcctgcgcgatcgactgctggctctattccgcacgcagctgtgatgcgcccgagctgacgcgcgaacgacggctccacagcctcaagcccggcgttacagtacacccactgacgcacgccgggccatccgcccgacagggcggtcggcagtcactacccacctagactctgaaggagagcaccatgagcgaagagaccaccaacaccggcgccgagtcgaccgagagcaaggagccgaagggcccgggcgtcggcgacgtcgccaagaccctgatccgcgagggcaagaccaacgagcaggtcctcgccgcgatcaaggagcagttcccggacgccaagacctcgatggccagcatcaactggtaccgcaacaagctgcgctcggacggcgaggacgtgccgaccgcccgttcgctgaaggcggacagcaaggccgaggccaaggccgcgaaggaagccgccgaggccgaggccaaggccgcgaaggaagccgagaaggccgccaaggccgaggccaaggccgccgagaaggccgagaagaagcgcctcgccgacgaggccaaggcgaaggccaaggccgagaaggaagccgccaaggcgaaggccgaggccaagggcgacgccccgaagggcgagggcatcttcgagtaaggcgccctgaagtgatggtttaaggggcactgctcctgacctagaatagagggacctggtgcgaaccaggtccctctttccattggagtccagccatgcagcttcctgccaacatcgtcttcgccaaggtctacttcgtccgcggcggtgcccccaatttttggcgccgccggttcgaggtgacggacccgccgaccagcggctacgccggctgcgtggtcatcaagggcgagaagcgctccaccatcctttgtccgcactcgctggaggccttccaggtcagcaaccagtgcggcgagatccagacggcgacccgcatggaggtcgagccggagaagatcgccttctacatcaacaaggcgtgggagaccagcgtcaagctgggattccagaaggactacggtgtggccgccatggtcctcaccgagatgggcttcccggtgcccaagttcctcccgcccccgccggacccctcgaagtcggaggactccaagcgcggcggcaagcccatcgtccacgaggccctgaagccgtgccggccgaccagcaagcgcggcgaggtggcggccttcttcatgcaggaggacccgcagtccctgcacgaggcgatggcccgcctcggcctcacccggtccggcgtcctctcccacctgttcaccctcaaccgcgaccacggcgtcggctacgagctggtcagcgactgcgcccgcctgctggtgcctgagggcttcgacctgttcgcctacgtcgagcccgtcaaggagccgaaggccgagaagccgcagcgcctcaacgaggacggcacggtctacgagccgaagaagaggaccagcggcaagccgatcaaccccgaggccctgcagccgatcccggagccgagcaagcgcgccacggccgccaggctgttcgtcggcggctggcacgacatagaggccgcgtgcgtcgccctcggcatcaaccgctccgccctgctctccatgctgttcaccatcaacaaggagaacggcctgggctacgagctgagcgaggacagcaagggcgcccgcctgctggtcccggacggccacgaggtgttcgcgcccaagcagccgcgcccgaagaaggacaagacgacggcggaggagtgatggccatccgcatagttctcaagccgcacaaggagggcatagccgccctccagcgggacgggttcgacgtcgagcccgtccgcttcggcaagggcgatcacctcgtggtgcgtgtctgccaggagggcgcctgcggtcaggtcacgatcagcggtagccccaggggcagcttcctcggctcgctcgtgtcgtcggctcgccgtgctgtccgtgaagcaatggccaaatagtaggacttggcggcttgctcgcctaaccggctatgccaagatgtattaccttcaacaacctgaggaagcaaacagatggaagagattgagaacctgggcaccaacgaggcgtttgccgctgcgcttgtagcccgcatgctcggcaaggtcgagcagttcaaccgcgaggtggtggacctgccgatccccggcacacccaccatcatctccgaggagcgccgccagtgggcagatgcggccctgcaggaggagctgaccgagttcaacgacgcctgctctaacggcgacgtgctcgaggccgcagatgctctgatcgacctggcgtacttcgccctcggccgcctcgtcgagatgggcgtgcccgcccaggctgtgttcgacggcgtgcagcaggccaacatggccaagcgcaagggcgagctctccaagcggccgggcagcctcggccacgacgcggtcaagcccgagggctggacgcctccggaccacggctggctgctgggcttcgacctgagcgacgtctccgagctggagcgcctgcgcaagcaggagtccgagcgcgaggccatcagtccggtgtggctggagctgcagcagctccgcgagtcgaagggccgcgactacaatgacgtcccaggcgggcgcgacgcgtacttccccttcgggcacttctcctacgcccacatgctccacaccaagaacctgcgactgcagtcgctgctgtccgccatgcagaagggtcgccccgtcaaccacgagggcctgtacgacacggtccgcgacctcgtgaactacggcacctactactgcgaggcgatccgcgacgggcgcctggccgatgtcgctgggggtgagtcgtgagcggcgtcctcatgccgttctacgacgtctacggcgcgctcctggcctggaccttccaggcccccgtcgaggcgaacgagcgcaccggaacgcgcgtccgcgtcggccgtggcggcacggccttccgcgtcgacctgggtgacggcctcctgccgaccatcggctaccgcaagaccttcccgaagtcggcggcagccgaggtggcgtggtacgtgcggggcgagcaggacgccacgttcatccgccagtacgccccgctgtgggacaagttcgtcgagcacctgccctacgacgtcgagactgccgacccgcgtgacgaggtgccggcgagcctgagcatcgagaccatcgacctccagccgatcgggtccagggacgtgcagcgtgtcgcgggccagtcctacttcgagggcgtcaagtccgcctacggctaccggtggcgccgccacttcggccgggaccagctgcggctcggagttgaggcgctgcgcaaggacccgagcgaccgaagggtctacgtgtccgcctgggacccggcggaggacggccttggcgcgcaggggcagaagaacgtgccctgcccggcgagcttcaccttcagcgtgactggcggcgagctccactcgagcctgttcctgcggagctcggacgtgttcgtcggcctgccgtacgacgtcatgggccacgcgctcctgatggacgccgtcgcccacgagctgcgcatccgcccgggcgtgatgcacgtgacgctggcccatgcccacctgtacgagtcgcactgggacctgacggccgaggcgctcaggcaggagccggtcgtcccgcagatgcagctgccgggctggagcctgacgcagatcgagcgggacccgcacgactacgtccagcgctacgccgaggaggccaagcagttcgcgtggccggcctacagcccgcggccggaggtcatcgagtgatggaggcgccgatcaagcggacccagcaggagtgggacgagttcttcatgggcatggcgcgcagcattggcgagctgtcgaaggacccggaccgcaaggtcggcgccgtcctcgtctcgccggaccggcggcagatgtccatcggcttcaacggcttcccgccggagaccgaggacctgccgtcgctcctggccgaccgcgacttcaagctggcgaacatggtgcacgccgaggacaactgtctgaggcaggcgccgttctccccggccgggtgcacggtctacgtcacccgatacccctgcctcacctgcgcgagcaagctcaaggccgccggcgtccgccgcgtggtcgcaccgaggcccgacctcggccacgcgcggtggggaaagtcctggaccgtcgccaccgccatcctggtggcggccggcgtgtccatcacccacatggaggcaaacccatgcgactgctgctagcaagctccgccgacggctacctggcccgaggccccaaggacgacatgaagtggaccggcccggtcgacaaggccgtcttccgcctgctcaccctctcgaacgggaacgacgtgctcctcgccggctcccgcacgttcgaccagatgcccaagctgcccggccgcacgatggagcgcctctcccgtaagggcgaggatggcacggcggactcctggaaggagggcacctccctggaagccgccgcagcctgctggcccgacgcctggctgatcggcgggccgaccgtggcgcgcgaggcgctccagttgggcctcgtgcgacgcgccttcatctgcgtctcgcccgtggagctcggctctggcatgcacgcccgggagctcgaacagttcctccccgccgagccggagttcaccatcaaggtggacgacgtccgcgtcctggtctacacggaggaccagcagtggcgcgggaggtaaggctctgggagtggctgcgcgacgggctcaagggcacgccgggcctccacatgcgccgcgtcgagaacctggtgagcgagggcgacccggacgtggacgggtgctggaacggcctgtacttcgagctcgagctgaagggctgcaaccggccgaaggctggaggcctgctggacttcgacgtccggcagtcgcaggtcatctggcacaggaagaggtggcgctgcggcggcaacgtctggctctacgccagggtgggcatcggccgagacgtcaagcgctacctggtgccgggctccaagacggcgctggtaaaggagggcgtcacggaggcccagctggccgccatgtcagtcctgcccccggatcacggggtgctggacctgctccgattcgcgactaattcgctgggcaatcgcgacacgctcacctaactggggaatgatggtgtttctccagcaacgggcgccgtacactgtctccgtgccaccactaatgggcaccggccgggatcgcccgggccgccaccaagaaggagacaccgccatgagcaccaccagcaaccgcacgatcaaggacgaggtccgcatcctgggccgccgcaagcgccccctgacctacccgggcatggtcgacgccatcaaggccaagcaccccgaggccaacaccagtgtcaagaccgtccagtggtacgcctcccgcctccgccgcgagggcgagaccgtgaacgtcaaggacggccggacctccgacacctgcagggcggcataaccgcccagcgggctagggggaaggatgagcaaggggccttaggagccgccagacgtctggcggctcctttcttatatgcgccctcgacagcccccccccccccccccccccccaatgagctagcgaaactttagcaaaaataatttgctggagggggctcccgtatcccaacggaccctgtataatgacctcacaccgcgacacactggaggtcatgagaaatgggtaccatcgctgacacgatccgctcggccatctcggccggcaagaccaacgaggaagtcctcgccgcagtcaaggcggcccacccggactccaacacctcgcccgcatgcgtctcctactataggagcaagatgaagaaggcgggcaccaaccttccggcggcccccaaggcgtcaaagcagacgcccatcgcaaaggccacggccgccgcagtcggccacggctacactgtcaagggcgtcaagaacttccgcggcaacgagggctatggcttcaacgcgaccctctaccgcgacggcaaggccatcgccttcgtcatcgacgacgcgaacggcggttgctacagctacgagtggaaggacaaggcggaggaggccatcctcgacgcctacgtcaagactctgccgacgcgccacgagtacggaatggacctcaccgtcgacgccgactggttcgtctccgaccttgtggacgacttcaacctcgagaaggacgccgccaagctgacgaagggcaaggtcgccatcctcaaggacggcaagatctacaccgtcaaggcccccaacggcaccgtgacgccgcagttcctcgagctcgttgccaagaagaacgctggtgctcgtgtcctcaacggcgcaccgaccactgagctcgtcgcgctgctcaagtccatgagcaactgatcccatcattcaagcgcaacggtccaaatgttgggtccgttgcacccacaacccgccataatggaacccacgacgaaacgcagtgcgttcgtctgagggtaagcccgaagtccaaccgtccaaggagccaacatgaacgtcaacgaacagtccaacatcgcagacattgccgcccgccacaacgagctgagcggcaaggggcttgaccccaagaacctcgccaagcgcggcaaggccaagctgctcgaacagatcgccaccatggaggccgaggcggccgagaagaaggccctcgagctcggcgccacccccgagaaggtcgaggaggcgaaggagcagcccaacggcatggcccacctgctgaagcagatgcaggatgcgcaggacaagaaggacgccaagcccgccaagccgaaggcgaaggacaagcccaagaaggagaagaaggagaagggtcccgtgattcgggtggtcgccgaggggctgctgctcgaggtcacccacaaggacgacgacggccgcccctacggtcactcctacgagacggtgctcgagaagatccgcgagcagttcgacggcgccaagaccaccgtggcatgcctccgctggtatgctgtccacatgcgcgagcgcggcgagaaggtcccgaaccgcccgcgcgcccagcccgccaagaagaccgaggaggcgtgatgccgcagatgctcaccttcatcgtgggctcccaatacagagtgggagcccgcgaggcgatcgccgagctcaggaccggagaggtcctgacgctccggcgggagccggacaacccgcacgaccgcaacgccgtggccgtgtatgacgcctgcgggcaacacctcggctacgtgccgaggcaggacgcgcccgcggtggcgaaggtcatggacctgcgcctgccgtacatcgcgaagtgccgctcccgcggcacgacctccatcgacatcagctgggagacgaagacctatgaacagcaaccgtgacgacgaagagcagggcctgagccccgacgagctgctcgccatcctgaccggcaagtgcctccacgaggtgcagctgacccgagccatggccatgctgggcgcgctggtgatccgcgcgggcggcaccgtgaccctcacccccgaggagatgctcgccctgtcggagcgcgccatctcgatcgacggcggccccgacggcttccgcctcgaggtcatcgcccggccgaccgagcagaagcagcccacccaccaagccccctcgacccggcagtaacggccactgccaaggagaatccgccatgcagcgccactacctgacctatgccctagccgtgctcgccctgctcctgatgggctgcgccctcatccactcctttgccaaggtcctcgacctgcccgaggtccgcgagtcgtggtccgagaagaagtgcgtcgaggtgctcgaccccgcagcggaggccgagggccggaagtcggagtggtcctgcgaccgcctgcccgagaagtaccggcacgtctgggtctactgacggcttcggtcgcggcagctccgcgccatgatgcctcccggggtcgacaatcttgggaggcattttcatgtgcgagtgcgacgacgagggtgatgggctgaacgcgttccgtggcctgatggtggcgtgcgggttcagcgtactgttctgggtggctgtggtagccgtggtctacgccgtgcgctcggctccggacgcgccgcctgagcgttccaggtcggctcaggcatccgaggcggcctaggcccagggccttagacgcgtcaggccgctcgcgcggcctgactgacacctggatcctgaaaaagccaccgccacgagggcggtggaaggcccggcacgagggaaggagagggacctcgtgccgggtgccgcggggctcatttgccgccgagcatctcccggatgcccatccatgcggctgcggcgaggcctgacaccacgatgccgatgatcgtgagcatgcccttccgcttgatcgagtcggtggtgctgcgccactcgcggaggtgctggaagtccttctgcacctcgatggggtcgtccaccttcaggccgagcatgaggaacgtttcccggaccgcctcgcggatcagggcgcgagcctcctcgggcgtgaggttctggagctgctgctccggtccgggcgtctgtccgctcacttctcttcccccttggtcttcggctgctccgtcggctggcgggtgtcgcggtagaagtcgagctgccagctggcctccttggcccagcggatcgtgtccgccaggttgcgcgccagggcctcgtagcccctggcggtgacggcgaacaggctctcgccgtcgacctgcaccacccgccactcgaccgactcagtccttacgggctggggctttggcaggacgggcagcgggggctgcttgtgctcctccggcgggtgccgcaccggtggattgctcgagcaggcggaaagcatcagcagtgccagcgttgatgcgagtctggatgagacccggcttgctcctggcgagcgcgccgaggtcgtgcttggataggacatccgtcagcttcctcgtggtttcgccagcctcacgctgggcattggagaatcggtccagtgcgtccgcctgcacggcggccgcctcgtcccacttgtcgatcgtcagcttgaacgcgtcggcccgggccttctcccgggcgacgtcctgctcgagagtcccgaccttggcggtcagctcggctttgtcgttgaccaggccggtgtaatggcggtatgatagcgcgatggcagtcaccaaggcaaccccgataagcgcgccagcgccgatcttgtaacccagcggaatcatgtttccctccttaggggtagatgctggcaggcagctcgaagtgaggcccgtccaggaacgccttcttgccctgcgccttgcggcgggccacgtactccgccacctcgtcctcgggatcggctaggtcggccagggtgcggtcccagacgccgccccacctgatggggacctggagctcgatgcttgcggcccgcatcgccagggcgacccggtagcacagggaccagtcccaccgcagctcggcgcggccgtccttgtcgaagtcgatcagcggcaccaggtcgacggcgtggccgagcccgtcgcggcccggcaggtggcgggagtccatcgtctggctggcgcccgcggcgaccagcttggcctgccgggcgcgcgtcctcagcccctcgaagacctggaagtccacccccgtcagctcgatcgcgcgctccaccacccggaccaggtccgggtgcacgccctgcaggttggtcctcgacttacttcccagcacgaacgtcatggttcgtcctccatcttagcggatgccccagggccaggggcgggcttcgccgtcacagtcgtcgtggtggtcgccgagacggcggcagctccacccttgcccagcttcgccttggcgatgctcacgtcctcccaggtcgcgccgaacacgtaggagcccacgatgctgatgagcgtcaggaacgccatcgtgatcgccgtgtcggccggcccggacgtcctgtccttgtagaggatgtagccgatggtccacatgcagaaggcggcgacggagaacatgaacctccgccgcacgcgccagctcgacttccagtccgggttgcgttccatggtctcacctcgtcgtggcgtagttgtgcttgaacaggctggtgagaccgtcacgcacagattccagctcaacgcgcacgaaggtattcagctgcggtgggctgggtgttagctcagatgcgggcggcgtgaagggagcgctgtacttacactccttagataccctcacctcgtcgatcttgccgttgaagtctaggctgaaaccatccacggcgcctatgaccacgttgctcgagctgacggctatggtctgtgcgaaggtcgcggaggtcagcactgccccgtctacgaatacacgcaccaccccggaagcatctcgtgttgcggcgaggtggtaccaggtgtcgacagcgggggtccacgtggcctcggtgtcgcggtaggccgagccgtcccagaacctgaagcagagcttgccggcgttcatccacaaggcgaaggacgtctggctgccggatacgccccactgcgacaccaggccgcagcttgagagggccacggcgaagttggcaaagcactccaccgtcagcgtgcccgcaccaaactggaagtcggcgtgagccggggtgtatacgtaatcgccggcaccatcaagcagcaggcacgccgaaccgaacttcggcccggtcactgtgagctgcgcgttgccggcggcagtccaggccttgccgctctcgtccgtgaagaccgtggacccggcggcaccgttgaagtgcagcagcgcggagtcgcctgccgccaggccgctgtcggcggactccgtagtccacgagtacgaggtgtcggtaaggccggtgacggtgcggcgcagtacgtccccgttcccgtacagcctcagcgtgtaggtagtgcccgcctcgggccccacgctcgcagctccctgatcgactaggacctgagccgtctgctgcagcctgtcgcggtgggcccacgttacaaccagcggcccggagatggagaccgggtaggatgccccgttgagcctcagctggccggggggatatggcttcgactgcctggcgaccatggtgagggtgtcggtcggggccgatgcaaggtcaagcgtgccctgcccggtggttggcagcatgcgcgcgctgacagcctcaccgagggcgtattctaccggcacgtcggtcaggtaatcgccctcgccgtagaacagcacccgggtgccggaggccagggacggcagcggcacggtgtcaagcatgcctcgcttgaccgtcaggacggtgtctgagacgctcacgacctggaaccattccctcgcattggaggcgcccacgccgaaggcgccaatatcccccggctccaccaggtcgaggtctgctccgccggcaatcgacagcacggtgtcgccagggccgtaggttgcctgcagtaccgccgtcggggcgaagtttaccacgccctgctgcacatagcctgcgccctcgtcgatgtacacctgcgcgctgatcgcaccgccgccgggcttcgcgccgcccaccaagacgtacgtcgcggtcggctcgagcgcggccgcctgtgaatcatcgagtccgcgtgctagcaggtagtaagggctctcggtcagcacgcggtgcgccatggccgtcggcgccccgaacgggttctcccactcgctcggcggcggcggggcgtagatagccgagcccagggcgaacacgtcttcgatcgccgacaccttgaccatgttgttggtgagctcgcctagctcgatgttggtgacacgcatcacaagctgggagacgccatactctgcccaggagaacttgaagacgtcgccgatgttgaaggtggcggccttgcgattcacgtacagcgtggccgaggccagcggcgtggatagggccttcaggtctcgcgaggccaccctggacgctatggcgcccttggtgaatcccgggtactggactgtggtgccgaccgtggcgccctgctgcgccgtaagcgcgatgtcctgcacggtgacggagttgttcttgcctgtcgtcttgtcccagtaggtcacgctgacctggttggtgagctcggccacggtggaccgcttgaagtcggtgacgcggtcgatggactgctcgtccagcacgggcagggtggagatgtcatagccgccacgagccagcttgagcacgaacttgccggtggtccggtccacgtacagggagccgtccacgtggcggagcaccgtggccaggaagtccgagagctgctgctgcttgtcccacagtagggacatgcccatgccctccgagtacaacgtatcggcggcagaggcgaaggaggtgtcgtccacgtccgactcgttgtagcccaggccccagtcgggatcggtcaggacctcgcggacgatgtgggcggggttcatgtcgcccccgatctcagccttggcgtcataccactgggcaaggccgtcctggcggacgtggatccgcgtggcccggatcgcccagcgcttgaggtaggggttgttgccgaggtagcactggcggagtacgagcccgagcacgcggcggaaggcgggtatcgcggtgcccagctgcgactgcaggtacgtgttgcgcccctggtcggtgcgtcccatctcgatgtcgacggtgccctggacgcccccctcgcgctcctctccgccaaacaggttgggggagttgacgtagatcgagccgccggtcgagttgcccgaccacgccaccttgttgtcgaccttgacctgggtcaccttgtctacggggccgtggcacataatcatgtgcatgcccaggtagtacttgtacccgacagtctgcttcttactgctgcccattgcgagcctcctcgattgccattatggccataccgtcgccggtctcggccagtgtgcgcccggagatgccgttggccagaaagtcagagtagtccaggccgtggcggttgaagaatgagcgaacgccgcttgagcagtagcccaagcggcgcaggtccgccatgcgtacgacgacttcgtcgtacttgtccaggtcgtcggtcacttcttgccacccttcttcttgatgggcacggcccggaagtcgccgtaccacgtcacattgggaccttccaggtcacgctccccgaacagtacggggatctcgcggccgacctcggcagtcggtgccgtcacgtcgcccaggccggcgggcttggcgttctccggcttcggcatcatcgagtaggacacgacgagcgcgacgatgaatactacgatgtaccaccacatgctgcaacctcctagacgatggaactgccgtcaaacggattccgggacgggatccagggaaaacccccgaagttgtcgaggttgttgaacttggtgtcgcacgtgctgcgcaggtggtcacacccggggtacaggcgcaccaattgagtgggcgccaggccgctgatcgggcgggacatggtgaccacggagcctgcgtgagataccaggaacctggacgatccgtccggggcgatgaggatgccgcccgagaagtagccgtccgggaatgtgccggcgccgaccacgtccacgttcagccccccggccaccgtcaccacaagcccctcgtgcttgtaggtctcgcggttgacgccgcagccgcgcccgtagagggcgtggcggcagctgtactcgaacttcgcccgcagccccggccgcttgatcgaggtgtagatgggctcgcactccagctcgatgcgcgactcggtggccttggcggacagaacgcggcccttccagtacgtcacgaactgggcgtccgggtcggtgtagtgcccgcgcagtatggtgaccgaggtgacgtcctcgggagcaaagccgaggaactgactggcgaactcgttgtcacgcgggaaggtgagcttgatggagttcttgaacacgtccgtcgactgcttgacgcgatcgcgctgcactgcgtacggggtgtacgtctgcccagagcgcactacctcctcggccccgctacagcacgcccaccgcttgagcccctgaacaaactcgtagagctcaacgggggctccctgctgtacggatgtctctagtgtcgcgtatgtcatgttatccctccggcacctcgattacgggaaccgagacgctgactcgcccgccgtagctgtggcccagctccaggcggtcgctgtcgaacctcacgtgcttcatcaggctgatgcgcacgacgtcggtcctggcgatgttgattccaaagctggactccaggtccagcacctcattgccgccggcgttcacgttacccgacaagatacgcttgaagatacgggtaccgtttaccaggtccaccatcacgtcggtcaccccgtagtagagcgagtagccgatgttgcgcacctcgatcgtcaggtccgatgccagcacatctgcgaccagcacgatgtcctcattccagctcggcacccagaaggtacgctggcgcccgcgacgtgcgtggagccacttacgcatggtccacgcatcgtggcggttcagcgggtcgaacgtcacggtctccgtccggtcggggtagcccctcagttggtccgtggtcatcgggccggagccattgtcgaacacatcgaccggcctcacgatgcgctccgacaggtcgccgagcacgacggacctgtccgtcagcacgtccttgccacggtactgcgggaacgtgctggccgcgcccaggtcgacgttgttggtcacctggaagctgagcttggccttagtcacgtcgtgggcatcgcgggagaactccgagccgctcagcgtgcgcccgaacctcaggggcatcacataggcattggagaacgagcgggtcaggggctgcttcagctcgatgccggtgggggtgactgttgtcgtctccgccgccacgaagttctcgtcgtcgtcccatagcaggattaggtcgtcgttccggtagtcggcgtccgcggtgttgaacaccacgagagtgatgccagaggctagcgcgcccagcctggttgcctccgcccataccggtgcgccgtagacccggtgagcccacgcggtgctcagtgccttggcccgggagaactgctgcgggtcgagctggaagtcgtactgcaggacctggcgcggggcctcgcgaagcgccagccgctgctctgccgagtaggcctgcatgacgtcggtcatccactccagggtctcgcggaacttggtctggggcacgaaaggccacaccactacgcgacgccccgtaacacgcagccgcggcgcttcgccggcgaagttgaacgtataagcagcatcgatggtcggtgggccgttggtggacacgctcagctcgtacagcctcgactcattgggcgcgaaggtggtcggaggggcggcgggctcggccagcgtgaggccctcggtgttggaccggtcgatggaggacaggagcttcgccgtgaggtgggcgttccacacctccacctcacggacctggctggacagcaggttgcctaggtcgatgagggacggcttcacgtggatccggtcgtagtagtcgtccctgtaggatgtcgggcgccacgaggccttgacgaccggcgtcgtgctgaccggcaggttcgacgtcacggcgaccgagaacgcgccgccaggcaccgacacatgcgcaggccagtagtccaggccgaactcccggagctcgtccgagagccgcgtgttcgcgaccggtacggccgggctcgccggcacgaaggaggtgacgaccgccataatcagggcccgtcgtagcgcacggcgaccgcgaaggtgccggagtggttgatgttgctgccgccgttgggcacgtccgcgttcttgcggagccacgggtacactttccacttgtccgggccaatctcgatgatgtcgccgggctcgtagttgctgatgcggcagtaccgcgcgtggccgagctcgcctacgaaggacagcttgcgctcggtgcggtgccacatggggcggatgggcaggagcaccgtctcggagttccacgcattgggctggtagctctgcagcggtgcaaggcaggaccacgcgtccgcggcgcactcggagcgcgggtacgagctgcctggatccatgaagacgatcagcggcgtgtagcccgaccagccgagactgtccaggccgtggtggatgtacgaccccacgcagtagccctggatccagccgccgtagttgcagaacaggatgccgctgccgcccggtgcgctgccggtccagcctccaccgaagtccgcgccaatgaccaggttaccgtaagaccggtccggatcccacgacgcgccgcaccagttcccagtgccgggcaggcccgcgcagggcgactgcccgaacgccatgtactggtagtacacggcgttgtagttcaagaagatgtagacctcgtcgggggcggtgccgatgtgcacgtgccaggtcgccggccaggttagggccgcggacggaatgttcccgatggccgggctgccgggtgacggggtcgtgggcgtggtgcctgacccgcccagcgcgccggtgatccgcagcgcgctgccggacacgtagatccggacgtagcaggtgcccttgtacaccatctcgccgtccaccgtccagccgttggcggacagcacgccgatgatgttggtgcgaaggtcggagatgctggtggcggagccggttgcgtagggcatgtcagtccatcctcagggcgtagtagtcgcggaagccggtgcggccgacgtcctggatgatgacggcgggctcgccgtcgatcgtggtggtgttctcgacgacgttgttgaagccggagaagtggtagatgccgtcgagctcgccgaagatggccccaggcgatggcgtgtcgctcatcagcagcacggggctggctgggtagctgcctccggtgtcgcgaacgtcgccccagtagctgccagtgtgggggacgtagttgccggacgcgacgatgccattcttccaggggtaggccatgacctgcttccacgagccgtccacgaaccgcatggcgaagttggcccgttcgcccttgtacggcatcgagtgcgaggtctcggagtagcggaccgccgccggcccgtccagcatgccgccgacgactagagggtacgggaactgtgccggcgtgccgtaaggccggaacagccccacgtacccggactcgtatacgggggtgccgaccttcaggccgaacgccaggcgctgaccgttgacggtcagccagtagtcgatccgcacattgtgggccgggatgccggactcgcggtagcccggctgggcggtgaacgcattggcgggcacgtagcccacgaagccggccacgctcaggttgtagtagtcggccgccacgttctggtaggaccgcagccccacgaagatctcctgggtgccagacaggcccggcgctcgcattatcagctcccgggtgtcggaagcggtgtcgtacctcagggtcgtccacccctcggtctcgcacgctgtcttgatgaaggcgagcatggcccggttggcgtacgtgccgccgctgttgtcgacgaagccggtgtacgacgtcatctctatcactcctgttagtagcccagcgactgctggttgcgctgcaccacgttcatgatgagcttctcgccctcgtcagtgccgaggaagtcgcccaccaagctcgggtccagcacgtttatgttccgcacgttgacctgcggggccggagccggggcctgctggccgtcggggtaggacctgccggtcagctcgcggccgcgcacggacgccgggcctcgcacgagctccggaccgtactcaccgacgatacccaccttaccagcggggatctgcccgcccttgtcgtaagcgcccgagaactgggagccgttgatctgggcgacgatggacgcgcccgtagcggcgacgcgtgccatctcggcgaggttggccgggaagccaagctcctgcgccttcgccaggccagtcgcgatcgacatagcggcctgggcgacgctgaacgccttgctcacggcgaatagtacgcggtaagccttggactgctcgccagcatagcccttcgccagcccagcgaggccgtcgaacagcgctgcggcggagccgagctggttctggatccgctcctgctccatctgggcctgctcgtcagcgaactgcttctgcagccggcgcagcaggtcctggcgctcgagctccgtgaccgcctcgctctcgaggatgagggtcttcttccgctcgtacgcctgcttgagcgcctcctcctcggtgagcagggagttatacaggctgtcccgctcggcctgccgctgcttttcgacctcggccagggccttgtcgcggtcggcggcgaccttgccctcgagctcggcgcgggccttggagccctcctccgtgttcgcccggatcatgtcgatccggcgctggtaggactccttgatcgcctcctcctgggtgagcagggactgccgcagctgctccagctcggagttgccgtagtcgcccagcttcttcagctgctccgaccgctcggcatcgaggcgcgccatcaggttgcggcgctcctcggagcccgccttggtgttctgctcgatgatggcgcggcgcttgtcgtaggacgcctggatggcctcctcctcggtctgcagcgactccttcagccgggcgaactccgtctccccgcgcttctgctcggcggccgcggccttgtcctggccggacgatgccctgctcggtcggtcgccgccgatgcggaactgggccagccggtcctggccctcgttggccttcttcttggcctcctgcgccttgtcgtactcctcgcgcaggcggcgggcggcggcgatctggtcctcgctggccttgacggtcgcgtcgcgctcctggagggccgcgtcgatggagtccagcctggcggcctggatggcctccatgcgctgcacgtaccgctggccggctgcgacgatggtgtcgtcggtgaacacggccttgatggagtcgcgccacagctcggcggacgcgatcatgcggtcaacgccggcggcgaactcgacggtgaggatctgcaccatcgcccgcaggttggacggcagctgcttgaacgcgtcgatgaggaagtccacgacggactcgccctcatcctcccactcgccgaagttgtccttgatgaactgggtgacgatgtcgatggtccgctcgatgtcggtgccccacgcctcccactgcacggtctgcgaagccagcagcgcctccatctgcccggaggcgatcatgtcagtcagctcctgcagggcgtcggtcgccatgcgcaccgcgtcctcgatcacgtcgccgatgccggactgggagatggtgaggaacagctggtcccaggtgtcgccgaggttcgccagggcgccgtcgagcgagtccatgcgctgctccatcgcgcctgcgaactcgttctcgccgagcttggtcaggtactcctcgatctcggcggcgttgttgccgatggaggtcgtgaccccgcggaacgtaagggacacctggtccccgttctgcttggccttgatgccgaactccttcaagcgctcgaactcgcccgtggcggcgtcggccacggcctcgatcatctggttgaggtccttgcccatcgcactggcggtgttgccatacgacctgagggcgcgctcgctcgggtcgaggcccaggttgacgagcttggtgaagccctcgacggcctggttcaggtcgtagggcgtctgctgggcgaactcgcgcagggcgtcgaaggcgacggcggccttctcggaggagcccgtggcggtgatgaggcccgcgttgagcacgtcgaactcgcgctggacgtcgaccagcttgttcagggtgcccataacgctgacggccgcggtgagcggcccgatcagcttggtgaatgctcccatgaggccggaggtggccttctcggccccgccgcccgccgaggccaggccccgcaggcgggtgtccgcctgctggacctggagggactcgatcttgatcgctaggctagctacgtcggtcgccatgctgcaccttccagaagattcggtcgagggactttatcagctcggcctcccaacccgtcaggcgcttgcccgtcatgttggaccaagcctgcagctcggcgtaagtcagcggctcacccgcgaacacctcccgataccactcccacacataccggagctcctcggggagctccggcgcgttctcaagctgaggcggcttccgcttcagcgtcttccacacctggttcagggaagcccgcagtgtctgcttactccccttcgggatcaggtcgagcttgaactcgtgctctgcgaaggctccgagctgctcgaccttgctgcgaaaaaaagggtgcgcttgctcgccgcaacgtcgatggcgtccatgatctgcggggcgttcacgaagaactgctccacgttgtcgacggtgcactcctggtcgaaggaccacgccacgaccaggtgcgcgatcagccggcgcttggagcgggcgatctcagccgcccgctccgagcccgagtccagctgcgcgatccggatcgcatcccggcgcgcctccgcgtccgcctggcggaagacgtcggagtcgatgccgatgatgcgcacccagtgctcgctcttcgtcccgtccggacgccacaggggcacctggatgccctcgttggccttctcgcgggtgaagaactcgtccatgcctgccgcccccgcggccttgttattttctgcgttcatgattatgcgggcactcgctcgatctggatgttggtctgggtcacgctgtccaggagggcctggaacggcatgctcagggtgatggggccctcgccctcgacgtccggctggccgccgttgtacttgatgcgcgggagcgtgaagacgtacttgttgccggcgccgtccgggagctcgaagacgatgttggactcggtctcgttgatgaacttgtccagcagggtcgagttctcgaagtaggccgtgatggtgcccgagcagttcgagcggccgatggacggcaggatcgactgcttggagccgaccacgaagcgcgcctccaggccgttctccaggttgagctggatctcggtgatgacggcgatcggcgtgccggcctcgttcagggtgccggtgaacgagtcgagcggcgaggtggtcgccgggttggcgtacgtcgcgcccgccagcgccgtggtgcccgtggtcatgttctggcccacggtgccgaaggtgccggtaatcatcgcgttggcgctgatcgccagggccatcgtgttgagctcgacgccggtgaagcggtggtagggcttgtccgccgtcaggatgtccccgaagaagcgctcgacggagaacgagcggcgggtcgtgccggccttcagcttcgcccggagggtgtccagggtgcgcccggccgccgcggcgtcgaccgccatggtctggccctcgagcggcgtcaccgtggccgacgttgccgtcagggcggtgatgcggaagcggccgttgttgcccgcggtggcgaagcccgacgagatgatgacgtcgtccacggccaggccgtcggtgatgaacgagcccgccgcgcgggcgaagctgcccaccgccgcgctcaggctctgcgcgccggtcgtggcgttggggacccaggtgccgagggtcaccgcctcgagcaggtcgtcgaagctcccgaaggagagctcgaagttgatgtcgccgccgacctggtaggcgccgtggcggaagtccgcgatctggcggtccgagcggatctcctcggactgcagcgactccttggacaggccgagggtcgtgccggtgtggcggatgggcttgaacgccggggccgcgggagtctgcccgtaggtggactcggcgacgtagcgcatggagtggcggctgccgtttgccatggtagtacgctcctagatggattagttacgggaaaccctggcgaaccaggtgacggtcatgctcacgcggtaccagccgtccacctcacgcccgcgtgagcggccgcatgaggctactgtgagctcgacccctgagtgggcaagtcgcttgcccgccttgaagaagtccgtcagctcgtccgccttggccgtcacggccgcctcgccggtgttgagcggatagttcaggtcgatctgcaggatgccgtcgtgggcgtcctggccctcgtcgcccagggtggcgacggagggctggttcatgaagatgtgcgccgcggcccaggggctctggtcggtcggcttgtcgaagggcgagttctcggcggcgtatggcaggtcgagcggggagtcctcgaccccctgcatcagcgccttgcgcagccccgtgaacgggttcacagccatgacctcttccccttatctgccgctgaaggctcgcgccttcgcctctacgatcctccgccaggaggccacgtgccttcgcaccatgccctccggcgcctgcttgctccacccgtcgtactcgatccgctcggcgtacggcaggttgttggtgaaccacacgacgtcggtcagcgatcccaggttggcgaccgcgtccgccatggccgccgcgccgcccaggtcgagccggtcgatcgcggcgccggccggactgttgagcgtcgtctgccagttgccgcgcagccgcccggtgtcgaccggtgtggagaagatgaccagcttgaacagttccagtaccgaggcgcgccgcaccttgtcgatgcggtccagcgtcttgatgccgaacccgcgcagcttcgcctcgaagggtcctgccatctacctcacctccggagctgcagcgagaagacgaccggggtccccgcggggtccaccgagtcgaagtccaccaccgcccacgtcgttccatttgcctcgacgaaggtgtcgccgcgcatgggccgctcggtcgcctggatgtagacgatccgatccccgcgcaggatgacctctccgtcgatctgcttgtccgtgtagtccgtgatgacgcccacgacagggaacacctggtcggggccgcccgtcacggtgcccgcgaccgggtcgacggtcacggggctgcccttcctgcggagctcgcagctctggccgaactcggccaggagcgcgtcgacgtccgccttgaggccaatatagtcgaaggtcgccatcgcttaacccctcacgacctgcccggagttgccggaggcgatcatgttcgcgttctggagcgtcagggtgacctcagggtactgcggcgtggacgacgccaggcctgccccgaagctctcggcgtacttcttcgagacctcgatcggcccgaccttcttcgtctcctcggtgaccttctggccgctcgcgtcgtacgtcgggtccggcatcaggtccttggtcagcgcgcgggtggtcagcatgcacgtcgccgcgatgagcgccgggggcaggccgcgcaggaaggagtagccgctgtcgttgggccagggcgtcgtggtcaggccgccgcggggccactgcgtgccctggaggcggcgcatctggtagcccacgaacttgtaccgcgcgtccaggtaggtcgtcgccttgacgatggcggccttgagctggtcgtcggtgctggcggagaggtcgacgccacggtccgcccagtacgcacggacggtggcagggtcggtgtacgcgttggcgttgtcgacggtgccgtcgtcgttctgctgggtgaatgccatggcgtcgttcctccgggtcgcttagttgccggccttggcctggcgggccttggcgcgggtgtagccggcggcgatcgcctcgacgtcggcgcgggacaccgacttgccggtcagcttggacaggtcgtccaggcccggcaggttgttcgaggtccagtgcgcgtcgttctcggggtcgagcatgccgatcgcttccgccagggtcgggagggccgggtccttcacgtccttgtcgttggtgtcgctgccgaccggtgcggcgggggcctgggtctgctcgccgcccttgcccgcgccggtgtcggccggggcctgggtctgctcgccctggctcttctcggcgcgcagctgctcgagctcggccttctcggccgggacagcgccatagaagccgaagacgttggcgagtatggcgatctgggcactggagccctggaacgtgaactcgccgtccacgaactcgtggccgttgaccgccatggacttgccggcgtgcgggccgacgaggacgaacttctgtgaggtggtgccggacatctggtctctccttctttctgttggctagaggccacgaagccccgccagtttcctggcgaggctcgcgggtcagtcggtggtggccaccaggatgggcgcggcgagcgtcgcgtccagctcgtccaggttgagggagttcttcaggcgcttgcgcacctgctcccagcccttcgcgcgggctggacgcagggcgggccggggtcatgtcgacctgtgcggacgccgcgaccgagggcttggcctgcttcgctgccgcctgggcctcggcgaaggtcatcgtcggggtcgcgcccttcttgagctcgtagtccgcggcctccttcagcttcaccttcatggtggccgagggctcgtagcccgccatcttcttgaccagcttgttggtgttgatcggtccgaggccctgctgcttggccttcttgtaggcctccagggccgccttgccgctcgccggcaggccggacacgaaggcctcgatcttctggttggcgacgaagcccttcggcgcctggaaggcggcgtcgaggtacgccttgccggccgccttggcggtgttcacctggtacatggcgagctccagcaggtcggacgcgcctggctgctggatcgtgccgaacaccgatttcatggcgtcgaaggcctgggagggcgtgccgccggccgcgacgaccgacttgaccttctcgagggccttgctagccgtcgggctgagcgtctggcccagcagcttcggcggcttgatggggccggacaccgccgccttcaccgtcgacttctcggcgaggctgaccgcgtggttgtaggaggccgggctggacttcttccagttggacttccaggtcgcgatgttggtgaccttgatgtcgcccgcgttgttcgggaactgcttggccagggtctccgccacggacttgttgtccagcacgcccttctgcatcagcttgatggcctcgtccttgagctgcgacgaggtcagcatgagggccgagggctgggcggctacgacctcgggcgcggcgatcgccgcctggctggaggccgggaccggcacgacgtccggcacgaccttggccgcgacggtcgggcccgcagccttgttgggcagcaggccctgcttcttcagctccgacttgtaggagctgatggacgccagcttggtcttggcgtcggggaactcagccaggacggacttcaggacctgctcgtccggcatgccctgctgcaggagcgccttggccagcgagccgaccgaggtgtgcttgccggcgacctcgaagggcgtgacggggccgcccgggagcggcgtcttggcggacgcggccgggacggggaacttcttcgccatcgcgtccttggcggactggatcgcggggccgaaggccttgttgaagtcgacggccgagaggccctgggacgtcagcgtgctcgggctcagggcctgcgcgtagatctcagccacgagctcgtctgggctcgacaggtagtacgagtagagctttcgggcatccggagacaggcccttcgccgaggccttcacggccgccaggacgtcgtcgccgagcagcaggtcgtgctgcttgtgcagcaggtggccgagctcatgggctgcaacctgcttggcctgcgccagcggcagggcggacagcttcttcccgcttagcacgacacccttgccggcctggtagtagccgtacgcaccgggcgacccgtccaggtcgtccaccacggtggaccactggttgccgatggcgtgcttcaggttcggtgccagcgagttgtccaggtcggcgacgacgtcggccacggccttggcctgcttgagggcgcccgcgggcacctgcgcggccgggccgaggttgagcgcgcctgccttgttgagctcggacttgtaggaggcgatggacgccatcgaggtcgacgcgtccgggtactcctgcttgatctggtcgagcacctcggccgggctgaggccctgctgcagcagcgacttggccttcaggcccacgcccggctggacgacgttcagcttgtcgccctccagctcggccttgagctccgccagggagtagggcttgcccttctcgtcgacgaacttctcgaggggcatgccgtcgcggaacagctgggccttgcccttgcccaggacctcgtcctggaactccttcgactgacccttcagccaggtctggtagttggtggagctcggcgcctgcccgatgttctcgtcggcccacttgtcccggcgcgccttgatggcggcgttgcgctcggcggcggtcatgcccttccaggcgtcgcccgcctcgtccttggcctcctggcggaagtcgatctcccgctgccggcgcgtgcgcgtgtcagtgatggtcgggcggtcgccgacgatctcctcgccgtgcagcacgggggcgacggtcgagcggcagttcgggtgcgcgggcgggcgcgggcccttgtcgatcgggtagacctcgccgtcccggctctggcagatgggcgaggtgcggccgtcgagggtggcgacccagcgcacgcccctgatgacgtcggcgttggcgtcccaggtcgcctggcgcgcggccgtcgacacgtggttggtcgccgtgcgggcgatcatctccgcctcgcggcgggtggtctccagcacgccgtccttgtagccgttggccttggtgccccggatgcgggacaccatctggtcgatggtctcgccctgcagcacccccagcctgatctgctgctcgatgcgggagacgtcgttcgcagccatcttgccgagccagccctcgagcgggatgccgttgatgggcgacgacgcgacggccttcagcacggtcggcgagacggtgttgaaggcgagggccaccggagtggccccctggagcatggacacctcccactccgcctcggtcttggagaggccctccatgtcctcctccagctcggcctggatgcgctccgcgaccgcggcgcgcatgcggcggacctcggcgagcagggacctgatgcgggcctcggccgtgtcggtgagctccgtctggaggagcttcacgagctcggcgtcgctctgcgccagcaggtcagccgccatctgtgcctccccctgggagaagcgcagcagcttgatctggtggcggaccgtggcgtccagcacttcctcgtttgcggtcttagccattgagcagggcccttgccattgtcctgacgacctcgtcgtcccaaggccccttggctaggttgtaagcccagcacacgagccgcacgttgccctgagtataacccaggtccgagtccacgcgatccactgacggcgcccagggattctggcgggctttgccgagacctccgtcggccgacagcttcacgccagtcaccgagcaggtcattggggcgaacagctcctgcaggaactcgactgtcaggtcgaactcgagcccccgcttgctggcccgcgtgctgagctccttgaaccagaacgccgcagggttctccctgcggcgcttggccatcgatacccgggcttgctccctagatcgctcagggttggcctcccggtaccgccggcaggcgtctaccctgctctggcggttcgcggtctttgccatcactcatcgtccgggttggggttggtgttgcccggcgcgggctgcggcgggtcctgcgggtcgttggggtcctgcggcggctggttgccgggctggcccggccgcgtcatcgtgccctgcccgccgccgaacatgtcgcccatggtgtccttggcctcctcggcgaggaactccgcgtcctgctcctcgtcgaagtcgtccgagaggatctggcgcttctggagctcgtccaggtaggtcttgcgggagatgtcacgccccgcgcgggccttgttgagcgtgtccagctcggccgcgtcggcctcactcaggtccacgttgtcgttgatctggaccgagccgccgtcgtccttgccgatccagtccgccgtgtactgcatggcgagctcgacgcagtcctggaagtcgcgcacggtggacgccaggtaggacgagctctccgccgagtccagggcgcggccggtcgccgtctcgtcgcccggcttcttgcgcatgtactcggcgccgtaggtcgccatctggtcctcgagggactccaggtcggtctggcccgcggcgatcgccgcgcccgtgtgctcgacgtagtaccacttgccctgcgggtcgtcggtcgtcaggaagttgttcgggccgatggtgaccttctggtccgcgggcacgccggccgccgccaggatggggaagcgggacacggtgagcacgttgcgctggtcgctcttggactgccagtgctccacgttgaggtaggcgaggtcggccagcggcggcttgcactccatcaggccggtgcgcttgccggcgtagaaggtcaccagggggatgtagtcgagggtcgtggtgccctcgtcctcgatgacccactcgtccttcttctcgtcctgcagcttccacagctgccagaggccaggctccagcacgcggatgcgctcgacctcgacctcctcccagcccaccttctcggtggtgatctccttgatgcggacgtgggtcagcacctcctggccgtgctggatcatcgcgtacgccgcaatcaggcactcgggcttgatgtggacccagtacgggcggaggccctcgttccggtcgtccgccagggtgcggacctggccctcggctgccggctcgggcgtggggtgctcgacgaggacgtgggagaagcccttggcccagccctcgcggaaccaggtccggcagaaggcctgcaggttgctgccctgcatgtcgatgtcctcggagaactcctcgagctcggacgggacgtcgtcgcccaggacgatcggctctcggaacggcttgcccgccagggtgtcgagggtctgctcggtcatgttgagcagcgtggcccgcgctaggcgggcctcgtagttcttgttggtctcgttgtcgtactggggcaggtactccctcgcctgtcgcatcgtctcggtgccgcccaggagggcgtccatcatcttccagcgcggaagcatgcgcaggtaggcgccggacggcgtcgccaccgtcggcttcttcttctgaccgtcggccatcgtcgggctccttgggctcggttaagcggatgctcgcgatggtacaccgggaggccgctggtcgtgagccagcgacctccgccccgtcacatgtctcccgggtgccgctcgccctggaagatggggaagcgcggcgcgtccttgctgcccgtcatgaagaacttgtacttgacggtcctgccgagccagcgggcctgcgtggaccagatgaggtctcgctgcgcctggttgaagcccgagccgatgttgaactgcacaccggcgaagggcccgttgatcgcccggaccaccagcgcgccgagcgtgccgccgccgtacttgccctccttgctcgtgctccgctcggtcagccctagcgcgctcgtggtcgcctcgttggcgttgcgcatcagctcctcgaagcccaccacctctgcctcgccgtcctcgaagcgcttgagcttcatgaggtcctgcgccctgagcgtgccccggccgtgcttgtagggcgacagggccgagcggagcatgatgccctcgtagccgaggcccagccgccactgctccagcttctccacgtcggccgcgctgtcgagctcgtgctggtagaccagctgcaggggcccgccgagtgccttgatcttcgccgcggccagcttgtaccggtggcggaactccagggccgggtcggtgcagtcgtcgaagacgtggaactggaagtccggctcgccctcgacggacatgacgccgcgcgtggtggcgttgaaggcgagctcggagcacgggtccccgacgatgagctcgccgtccaggccgtcgtaccgcgcgtggccgagcatggcctgcacgtgtcggttggggatgggcttcaggttgcggctcacgacgacgccgcccctgacgatagcccggatgccgtccagcttgtccgagccgagcagcgggtaggtcagcttgtccagcgactcgacggtcgcggcgagcatgggtctgaactgtcccatcagaagtcccccggcgcgacctggaaacacgtgacgccgtgctcccgccacatggtgaccacggaggagcggtcgtcgaagacggccacgagcctggcgcggtccgcggggtccatctgctcgagccacgagcgcttgagcttcacgtccggctggtggtcccgggcctcgcgcatccgcaggacggtgtgggtaggcaggtggaggcggagccactcctccgtctcggcgcgcacctcgtcggagcggccggaccagacctggacctcggcgccggcgagccacaggccctgggcggtgcgcacgaccgcctcgtttggcgtgtcgagcgggcaggcggcgtagaactcccgccagcgcttgggcgtggactcgacgaggtggcgccggtggtcgatcagcgccagggtgccgtccaggtcgaagatgtagaggggcctcacgacgccatctcctcgagcacgccgagggcaacgctaacctcgctggacgaggcctcgccctggtccaccatggacctcaggcgcatgatcgcctcggtcagcgcctcgtgccgggcgtcgcggacgctcaggtacgccccgactgcgtccaggatggcgtcgtcgaagggcgacgggtcgtgcagccggccctcgcgggcctcgttgaagaggcgctcggccgtctcctccttgtcgtcggagcggtggagctccaggagggcgtaggtcaggccgcgctcataggcgacctcgcggccggagcgggcaggcctggcgcgcagcgaggcccacacgatggcgaccgccagcagggcgacgcaggcgagcagccagaagttgggggttgagaagtccatgtcgtttcctctgtcggtgtatgagaagggggagacgcctatcatggcgcctcccccggtcagctcacgccatcattccatgcggtcgatgacgtagcgggcggtcccctgggcggtgcgcacccagacctcggccgggccgttgtccccgacgcgcagaccggcggcgttctgcgtgccgcgcggcagcttggccgtccaggccgtggtggatgtacgaccccacgcagtagccctggatccagccgccgtagttgcaggcgggcgtcaggaagtacgcgggcagcctgcccaccagcgagacggcggccataaaccgccagcagaaggcgcagggcctgccggagctaacggtggaggaggtcgcggccatcaaggcgtatactggatccacctaccggtcgctgaacaacgcactccgcgctggcaggtactcgtcggacccgcacctgcaggcctacgtggacgctgcccagcacggcctggcgaagatgcccaagtacaagggcctcagctcgcgcggcatgtcgttcaacgacgggcagctgaaggccatgctgtccacgtaccgcaagggcgcggtggtcgaggactccgccttcgtctcgtcgtcctacggcgagcgggcggcgttcggtggcaacgtgttcatgaggatcaacggcaagacgggcgtgaacgtgtcccagtactcgtactacaccggcgagcgcgaggtgctcttcatgcccggcacgcagttccgcgtggacgaggtggtccagcagaacggcaagtacatcatcacacttacggaggtttgacatggcagacgagttcgagccgggaccggactgggaggacaagacctccttcgccccgggcgtgcccgacgacccggacgcggtgccggagctgctctaccaggtcctcctgggccgggtctacacgctgaccaggtggaaggacgggtcgacggcccggggcgaggtggcgctggccgacctcgagggagtggccggcgggccggtcaccagggagggctggtacgacgccctcgggaagtacatcggcgccgagctccccggctccctgtaacaccagcaaggcccgctgcactggcgggccttctccttctgcttgaatgctggctcgcgcgggccgggcgccggcgttaaggtgccagcctgaacacaccccgggcgcgacgcccaaacaacccagcgcgtgacgcgcagaaggagagcaagatggacttcgagttcctgaagaaccccaccgtggacgacgtggccaaggtgccagaacagttccgcggcttctacgccgagggcgagggcggatacgtcctgcaggacagcttcaaggcgaccgccggcgcggtcgacggcctgaacaagtcgctcaaggcggcgcggcgagacgccgacgaggcccgcaagaatcgccccgacatctccggcttcgccgccatcggccagctgctcggcctggagggcgacgatgtcaccaacgccgacaccctgcgcgccgccgtcgagaagaccctgagcgagtcgaaggacggcaaggtcaactgggacaagatgaagaaggacctggagagcggcttcaaccagaagctccaggcgaaggacggcgagctgcaggccatgggcaagaccctgcagaagtacctggtcaccaccgccgcggtccaggcgatcgccgcgcacaagggcgtgccggacctcctgctgccgcacatccagtcgcgcaccaaggtcatcaaggacggcgaggactacgcggtccgcgtggtcgacgactccggcgacccgcgcggcaacgcctcgggcggcttcatgaccgtcgaggacctggtgaaggagctgaagtccagccccaccttcggccgggccttcgagagcgaggcgcccaacggtggcggcaagccgccgggctcgggcaacaagccgccggccaacaagcccggcgagatgacctcggtccagaagatcgcggccggcctggccaagcgccgctgatccagctggcggaaacgatgaagggcgccctagggcgccctttctcttttacaggtgcgacgtgcagctggagctcgacatggcctgcaggctgtcgcgcaggtcgttgaggacctgaccgagccagttggtgcctcgccactcgctccggtcgtgcacccgcgggtcgtcctcgtccaggcccacgccccagatgacgtcggtcgggctcgcctcgaccagggtggtgccctcggtcagcagcagcttggcccggagcacggggtcgctggtgaacttgtgcaggctggcccgcatcacgacgtcgcgggagaccacggcccagacgcgggcgtcgaagcccttgacctgccggccgatcgccttctgctccgacgggttccgggtcgccatgatggcgcggtgccggacgaggtcgccgaacagtagggccttctgcgccatcatgtactgctcggcgcagctgtactccacgctgtcgatgaccatgggcgacgggtaccactggctgaacacgcccccgtagaagggcgtgaacttctcttgctgcttcatggatctaccctcctcaggggaattgttggaaggaccaggcccggaggcctggtctgtcactgtgcgctcagacgcgcttggagtacgccggcgtcggctgcggcggcgggacctcgtggaccgagaccgcctgcagcacgaagaacttggcgccggggttctccttggcgagtcgcagggcctcggcctcggccgtctgcccgcggtcctggaccacgcgcggcgggttcttcagcgtcgggcggccgtgtgggcctccctccttgtagacgtcgccgctcgccacgaggaagaagcggccgtcctcgagcacggaggtgccgcgcgcggggtcccacgcgaccgtggccgactttctggtggtcgagcggccgacgagcgaatcgacgagctgcttgcccttgtccgtcaggcccggaggctcgcgtccgctcgggtcgaacgtgatgaggtcgtcgacgagcaggaaggtgaggtccggaggcgggagccccttgacgtgctcgggcgacgagaagcccatcgcgatcgtcagcagcgtccgcaggcgggactccggcgacgtcttcgagatgcgcggcttcggctgggcgtcgcggcggagctgctcgcgggcgaccgccgaggcctgctccgccgacgtgaggccgatgggctcgaagtcggacgcggcgatggtgccgcggtccacgccgagctgctcgaggcggcacgctatggcgttctccgtccggccgtgggccttcgccagcttggtcaggttgatcttgccggcagcggccacgaggaggtcgcgctcctccgcctcggtccacggggcaccgcctcggggcgtgtggcgcgggtcggcggagttgccgacgagggtggaccacccgcgcttgacggcgatggcgtgggaggggaccttgaagcgcgagaggatcagcgcgaacgcggcgtcctctagggcgtcgaggtagtcgtcgggcatgaagtcgcggaagtactcgccctcatcgaatgctggaaacatggacgttctccttggttgggtttcacggggtgcaaggcatcgtgccacccaactgggcggcgtgacgccactgtttgtggggttcagacggccatcagctccttcgcgcgattccacgccgcgttccagaggttgcagacctcctgcgacatgccgtcctcctcggtgtagccgtactccagcgggtccacgccgaaggtgtggaaggccgcgtccatcaccatgttggcgtcgcagaagtcgtgcgagtggcagacgtccgggttgagctcgacgccgttgagggtgacgacctcggcgaactgctcggcggtgagctgctcgcgcagttccttcacgaaggcctcggcgagggcgtcaacggtggggagggtgacggtggcgttcatggcttagccctttatcagcatgttgagggtgtggaggaccgcggcgcggtcgtccggggacagttgagggtactcctcgagcgaccgcacggcgtcgatcggcccgaaggagtcgaaggggatgagctccatccgcgcgagggcctctcgcgcgagacggtcgagctcgggagggtcgagtttagtgggcatggaccttccccatccgcacgaggatcagcctcgcgtcgctgtggaggtcgtccacgaggtcgccgtcgtccgactcggcctcgtggttcatctcgagggcctcctccacggagacgtcgttgtcctcggcgccatcgatggcgtcgagcgcgacggcgtacgagaggagggtcgtgggcgagacgcccacgtccttcatcagctgcatcagctgcgcgagctcctcgagctcgatgccctcgagctcgcggtacttgaagtcttcagcggccatggcttcgctccttagagggtcttgaggtcggcgccgtcctcagcggagggcacctcccaatggtcggtgtgcttgacgcggccgtccgccgtgatggccacgagggtcgtctcgtcgccgagcgtcgggtgctcgtagaggtcgacgccgtgaacgcggccgaggtgggtcgggttcttcgcgaggaaggccttcgccttatcagtggtgggcttgttcatgacagtctccttcagaggtggaacatcgcgagctcggcgtccgacaggacgatcgagtagggcgtggggtcgcccgtgacttggaaccacgcgcggtcgcccttgatactgacgaggccgagctgctccttaccgtgtgcctctcgggcggcgtcgaacagccccttccagaggtccttgttcatcgggcgcctcgggcatgcgccgcagtatcgcagggccttgatggcggtggagggcttgcggtccattacgtttaccagtttgcgttggtgtgaggtcattatactgggttcctttggataagggagcgccctggaagcactattttctatcttttttataggatctaaagaaataagggtaatctaaccctttcttagcctggtctgaggcagtccggccgatccggggcttgccgtggctgctccgtctaggcctctagggcatctaggccgattctcccgggccgtggccgaccccggggcaagccgttttcctgggacaacgaggccgaaaaggctcgtcgtggctcagatcgggcctaagtccttggtccgtaaggcttttctgcgtctgggcctggcccggataggcccagaaggctcagattctcgcgctggtccagcgtttagggggttacgagccctgaccgtcgcggcaaagtcccgaaccatggcgcgcgagcacggtctttcccggcccgcgctcgctgacccggccgaggcgtgacgcctggctaggggtcgaatcgtcgggcgatccggcacctaaccaagcatcccaacacactctgtcaggagatcacaccatgtcttccgttaccctcgccgagtcggcgaagctggcccaggacgagctcgtcgctggcgtcatcgagaacgtcatcaccgtcaacgagctgtacgagctgctgccgttcgacggcatcgacggcaacgcgttggcctacaaccgcgagaacgccctgggcgacgtccagatggcgggcgtcggttcgaccatcaccgccaagaacccggcgaccttcacccaggtcacctccaccctgaccacgatcatcggcgacgccgaggtcaacggcctgatccaggccacccggtcgggcgacggcaacgaccagaccgccgtccaggtcgcgtccaaggccaagagctgcggccgcaagtaccaggaccagatggtcaacggcgacggcaccggcaacaacatgaccggcatgttcggcctcgtcgccgcgggccagaccatcaccgccaacaacggcgccgcgaacggtgcggtcctgtccttcgaggacctggacgccctgatcgacctggtgaccgacaaggacggccaggtggactacctgatgatgcacggccgcacccgccgcaagtacctggcgctgctccgcagcctgggcggcacctccccggcggacgtgtacaccatggcctccggccgccaggtcccggcgtaccgcggcatcccgctgttccgcaacgactggatcccgatcaaccagacccagggcaccgcgacgaacgccacctcggtgttcgccggcaccttcgacgacggcagccgcacccacggcatcgcgggcctcaccgcggagcgccaggccggcatgcacatcaagtacgtcggcgagaaggaggatgcggacgagagcatcacccgcatcagctggtactgcggcctggccctcttcagcgagaagggcctcgcggtcctgaagggcgtgatcccgggctaatcccagccgcgggctaaccaactagcccgccggcctcgtgccggcgggcccatattgggagatcgagaaaatggccgatgcactgtactacgtgcgcctgtcgggctcgcgctgcgggcagaccctcaacaacaaggtgtcgcgtcgtacagggcgcccaggatgccgaggtcgaagctggcgccattgccccagaggcggacctcgcgggtc

SEQ ID NO: 11 - DNA, 56232 bp, unidentified
  source 1..56232: mol_type = genomic DNA
atggctgacggaggccacttcaatgatctaggcgagttgatccgcctgaccgccgaaagcgttctggttccgccggagcgcttgtctgtttctgacgccgcagcgaagtaccgctaccttgacaacgaaggctcgttcgtcgggcagtgggacaacaacgaaacgccgtacctcgtcgagccgatggacgtgctcacgagccgcgagttcgagtcgtgcatcttcgtaggcccggcgcagggcggcaagaccgaaatcatcctcaactggatcgcgtacacggcgaagtgcgacccggccgacttcttcctcatccagacagcgcgcgacactgcacgcgacttctcgtatcgccgcatcgacaagatgcaccgcgacagcaaggagctgggcgcgatgctgcggcccggcagcgacaacgacaacatcttcgacaagttctaccgcaacggcatgatgctgacgctgggctggccgacgatcaatcagctctccggcaagccggtgccgcgcgttgcgctgaccgactacgaccgcatgccgcaggacgtggagaagaacggcccgccgttcccgctcgcgcgcaagcgcacgacgacgttcggttcgttcggcatgacgctggccgagtcgtcgccgtcgttcgacgtgaaagacccgaagtggaagttgccgcacccggactcgcatatgttcccgccgaccgacggtatcggtggcctgtacaacgaaggcgaccgtcgctgcttctactggcagtgccctcactgcggcgagtggttcgagccgaagttcgcgctactgaagtgggacttcaagaatcccgatccgttcgaggctgctgcggcgacgatgatggcgtgcccgaagaacggatgcgtgatcgagccgaagcacaagtacgagatgaatcgtcgcggcgtgtggctgcgcgagggccagcgtctcgaccgcgacggcaaccgcctcggcgtcggtgtgcgttcgcgcagtgcgtcgttctggctgaaaggcccggcggcgcgcttcattacgtggcagacgcttgtcgagcgctacttgctcgcgcagcagacgctcgaacgcacaggcgaaacgaaggcgttgaaggctacggtcaacaccgatcaaggcgaagcgttctggccgctcaacgcgaaggactcgaaccgtctgccggaagacctgcaatcgaaagcgatccagtgggcggacaagaaggtgccgtacggcgcgcgcttcctgctcgcgaccgtcgacgtgcagaagagccgcttcgtcgtgcaggtcttcggcgtcggcccgagcgataacggcgtcaacttcgacctgtacctcgtcgaccgattcgacatccagaagtcgaagcggcaggacgatgccggtgatacgctgtgggtaaagccgtacgccgtgcaggaagattgggaactcatcaccgagcaggtcgtcgagcgcgagtacgagctggaagacggcagcggtttcatgtcgatcaagatggtcggcatcgactccggcggcaagtcaggctcgacgacgcgcgcgtacaactactggcgctcgatgcgcgacaaaggcgaaggcgctcgcgtgctgctcatcaagggcgagccgaagctcggtgcgccgcgtgccgaagtcgacttccccgattcggatcgtaaggatcgttcggccggtgctcgcggtgaaatcccggtgctgttcctcaactcgaacgtgctgaaggacatgctgctcggcatggtcgactacgacgagaagacgacgctcggcggtcgccacttcacgaacaagtggacgcctgaagttgtgtacgccgaactcactgtcgagttccgcgatgaccgtggccgctggcagaacccgggcaagcgacgcaacgaagcgtgggacttgggctactactgcctcggcctgtgcgtcatcttgaaggtcgaaggattcgattgggactcgcccgaatcgtggtacgcggagtggagtaacaactctcttgtgcgccgtgtggatcaggaaaaacggtttgcgtcaagccccatcacggattatggtttcgccaagttcgggaaatccttgggatgagagatggcgactctagagcagttgcaagcatggctggcggaagcacaaaccgcctaccatagcgtcatgatcggcggcggcgtgaccgtcgtcgtcgaccagaacggggagcgggtcgagtacagccgagccaacgcaaccggcctcgccaaatacatagccactttgcaggcacagatcaattccctattgggggtcgcagtaacgggcggcccccttcgtccgttcttctgagggtaaaacgacatggcccgagcactcactgtcgttcgctcccccgagggcgacgaagcattcaacagcaccggcaaagagtcggccttcggcggtgcgtacgaaggcgcgtcgcgtctcaaccgacagaccgcgatgtggagcgcgccgtcgctgcccgccgacatggaaatctcgccggacaaggttcggctcgacgcgcgcactcgcgaactcgttcgcaacgacggctacatccaaggcgcgctcgacacgagcaccgactccatcgtcggcggccagtacatcctcaacgcgcgccccgattgggagacgttgggcctgagcgaagcgtgggccgaagagttccagctcatcgccgaacgcaagttcatgctgtacgccgaatcgccgatgaactggatcgacgcctcgcgcaagaacggactcacgggcctcgtgcgcatggcgctcggtcagtccttcatgtcgggcgaagcgctcgccgctgcggagtggttgtcgaagtccggtcgtccgtacaagaccgcgatcaacatgatcgaccccgaccgcctgagcaacccgaacgacaacagcgataccgcctacatgcggcgcggcgttgaaatcgacaagttcggtgcggccgaggcgtaccacattcgtgacgcgcacccgatggagtcgtactacgaccgcttcggctcgaagtggacgcgcgtgccggcgttcaagccgtggggccgtccgcagatcatccacattgccgaagtgctgcgcccgggccagacgcgcggcgtgtcgaagatggtcgcggtgctgaaagaaatgcgcatgacgaaggtctacaaggacatcgttctgcaaaacgccgtcgtcaatgcgaccttcgctgctgcaatcgagtcggagctgccgcgcgagctggtgttctcgcagctcggtgccggcgacatgggttggttgcagaagtacatgggcgcgctggctgagtacgtcggttccgccgacaacctcgccatcgacggcgtgcgcattccgcacctgttcccgggcacgaagctcaacctgcaaaacgccggccaaccgggcggcgtcggcagcggcttcgaggactcgctgctgcgacacatctgcgctgcgctgggcctgtcgtacgagcagttctcgaaggactactcgaagacgaactactcgtccgcacgcgcgtcgatgatcgagacgtggaagtacatgcagacgcgcaagaagctcgtcaccgaccgcttcgccacgctcatctacatgctgtggctcgaagaggaaatcaatcggccggacaccgatcttccgctgccgaagggcgctgcgcacttctatcagggcatcaaccgcgaggcgtattgccgttgcgactggatcggcgcgtcgcgcggccagatcgacgagctgaaggaaacgcaggcggccgtgctgcgcatcgcgtcgggcctgtcgacctacgaagaagaactcggcaagctcggcaaggactaccgcgaagtgttcactcagcgcgctcgcgagatgggcctcatcgagaagaagaagctcaacttcacgctcagcaccagcaagccgggcacgcagaaagaaactgacagccgtgcgtcgaacaacgccgatgacacggacaccgataccgacaccgacacggagaacgacgatgaatgaactgctcgcaatgcgcatggcgcttgtcgagggattcaacggccgcccggcgttgatcgaccctcgcgatgtcgagaaggtcgcaacgctgtgcatgacgatggcgcaggcgaccgtcccgccgagcgccgagcagcgcgcgcaggcgcaggaaggcatcaccgcggcggtcgaatccgcgttcgacgtgtcgttcccgcgtgaccgcgccaagccgttcctcttcagcaacggcctcgccttcattccgatgcgcggcacgctcgtgcatcgcaacggcgacccgtggtacggcacgcgcggctacgacgacatccgccgcgagttcgacgccgcgcaggctgacccggacgtggcgggcatcgtgttcgacatccactcgggcggcggcatggtgtacggcaacttcgagctggccgagcacatccgcaagggccgcgacacgaagccgtcgctgtccgtcgtcaacgcaggcgcgatgtcgggcgcgtactcgctcggcagttccgcgcagcgcatggtgtcgacgccttcgggcgacagcggcagcatcggcgtgctgacgatgcacgtcgacatgagcaaggcgctggaaaagttcggcgtcgccatctccctcatccatgccggcgaacacaaggtcgacggcaatcccttcagcccgcttcccgacaacgtgcgtgcagacatgcaggcacgtctcgacggcatgtggcagaagttcatctccgtggttgcgatcaatcgcgggatgtccgaacaagcggttcgtgacacgcaagcccgtgtgtatcaggcggacgatgcggtcaaaatcggcttggtcgatgcggtgatgtctccacaggatgccatcgctaccttccgggccgaagtcttcggctcttccaccaacgataggagtgacaccatgagcgacacgaagaagaccgatgccaccgtcgagcagaagaaggccgacgagcaggtcgaaaacaagaccaccgacaccaccgtcgacgcgggcaagaagcaggacgagcaggtcgatgccggcgcggccatgcaggcgcgttgcgcggcgatcaccggctgcgaggaagccaagggccgcgaggcgctggcgaaccacatcgcgttcaagaccacgatgtcggtcgacgaagcgaagtcgatgctgtcggcctcgccgaagcaggccaatgcgtcgtccgcactggacgcggccatgtcgaactccggcggcggcgcggacatcgccaacaacggcggcgacgaagaagagcaggcgcgcggcaacgacgacggcggtctgttgggcgcgtacaccgctgccaccggcaacaagagcgtgcttcgcgtcgtcaagtaatatcggcacaccgtcgccagcctagacgggaaaaatccggctaaccgtcaatcacagaaggagtaacgaaatgaccaacttcggccccatcgctggctacgtggctcgtaccgacacgaacagcatccagctctatgccggcgaagccgacatcgtgagcacgcagggcgcactcgtcaccggcgtcgcgtacgtcggcggtcaggttctcggccgcgtcaccgcgtccggcctgttcgccaagcatgatccggccgcgaccgatggcagcgagaacgccatcgcgatcctcgcgtacgacgtggcgaccccgaccgccggcaagaaggaagcgatctatgtcggtggcgtgttcaacatggaagcgttgaccttcaacgccgcgaccaacaccgacgccctgaaggccgccgcgttcgacggcaccaacatcgtcgcgcagaagctctacggcaacccgccggccggttccggcccggtctaagccggcatcaccaacagcaagacgtttcgcaactacacaccgaaatagaaggagacaacgatggatttgttcagcactgcggaactgcgcaaggtgatcgtcgacagccgggcacccgtgcagtatttcctcaaccgtctgtacaaggagcagatcaacttcacgaccgaagaaatcatgttcgacgagctgaagctcggccggcgcatggctccgttcgtggctcccaacgtgcagggtcgagtcctgaagcgttccggcttctacaccaagtcgttccgtccggcctacgtcaagccgaaggacgccgttaccccgggccgcatgctgcgccgcctcgcgggtgaagcactgaccggcgacatgacgcccggccagcgctggcgtgccgtggtggccgcgtaccagctcgaccagcgcaaccagatttaccgccgctgggaatggctgggcgcgcaggctgcgctctacggtcaggtcacgatttcgggcgaggattacccgaccgtcaccatcgacttcggccgcgccgccaaccacaccgtcatcctgaccggcaccgcgctgtggacggaccagacgaacagcgacccggacgacgacctcgaagagtgggccgctcgtgtgcatgacgccgaaggtttcgtcgtcacgcgcgtcacgatgggccgcctcgcgtggaaggcgttcaagaagcacccggtcatcaaggagctgctggaaacccggcgcggctcgaagtccgaagccgaaaccggcccgggcctcggcgagtcggtggagttcaagggccagatcggctcgttcaacatctacgtctacaacgacgtgtacgaggacgagaccggcacgatgcagccgatgatggacccgcgcgacgtgctgctcgaagccgaggctggcttcgacggcgtgcgtgccttcggcgcgatcatggatgcggacgccgatcttcaggcgctcgacatcttcccgaagatgtggaagaacccggacccgtccgtgatctacctcatgtcgcagtcggctccgctcatgatcccgagccgtccgaactgcacgctgcgggctcgcgtcgtcgcgtaagcaacgtcgcacacggcaagcccggttcgccgggcttcgctgtagcaacacaactccccaaccgaaagaaggagcatcaagatggcgaagtacaagttcgtggcccgcgtggcgctgaagggcgatttcgacgccgaagacggcctcggcaccgcgttgcaggaagtgcaggcgggcaccaaggccggcaccgacgacaagaagctctacgactcgctgctggaacagggctacatcaagtccgcgaaggacgccgcgaaggaagaggacgaggctccggctgcgtcgtcgaacccgagcaccgcgccgaaggtcgagtcgaccgacagcacggccaagagcggcggcaagcagggcgcgggcaagtaagcccggcgcgctgaagggagaacggaatgggctggctcgaaaccaagcagaaggctcggcaaaccgtgcatagcacgtttggtctgccggcccaatttcgcccgaagtcgggcggtgctgtcgtcgacggcaccgctcggctgcactacaaggttcgcacgttcggcgacttggaccgcgaaggcttcgcgaccgtcaccgaagcggtggactacatcatcatcgacacccggattttcgtgggcgctgacgaaggcgaccgcgtgttcttcccgcagctcaaccgtgcgttcaagctcgatgtgcgcggtgaagcggaagacgacattttcatcaagtgggaagtgactgaggtagcaccgtgaccgtcgagattggcttccgtggattggacgacgtgcgcaagcgcgttgccggcataccggaaacggtagaccgggcttccgcgttcgcgatcaacgaagcagtcacgttcggtcaggccgagagcagccgccgcattcgcgagcaggtcgcgttcaaggcgagctacatcggcacgtccgacaatccgaacgctcgcctgcgcgtgtcgaagaaggcgcgtgtcggcgacctcgaaggcgtcatcgccggtcgcatgcgcccgacttcactcgcgcagttcatgaccggcgcgaagctcggcaagggcggctacgcgcgcgtcaaggtctcggcggccggcgcagcgcgacgcatcccgaatgcgttcccgatgaagctgcgtcgcggtactggcgtgtacgacccggagaacgcgaacgtcggcctcgccgtgcggttgcaggacgggaagctgccgggcggcatgaacaagaagcagatggtgcaggtcagcggcaatctctacctgctgtacggcccgtctgtcgatcaagtttttcgcgatgttcgattcgatgtgcaagggccagtcggcgacgtgctcgaatcgagcttcctgcgcaactacgggagactgagccgtggctgatacgaaacgactgctgctgctgaaggcaatctgcgatcacctgaagaccgaaatcacgacggcgaacggctacaacttcgacctcgcttcggtgtaccggggcaagaagaacttcggcaaggaagtgaagctgccagcgctcgtggtgttggagaacttcaacccggatcgtctgccggagaccatcggcggcgtcgtcggcaccaagcacaagtacgaccagatttacctcttgaacggatgggccgaaggcggcgatgtcgagcaggaagaagactcggcgcatctgctcatgggggacgtgaaaaaagcgctcggcaagctgctggtgccgcgcaaccaaagcgggttcttcgatggtctcgcaaacacgctgtccatcgagcccggggttgttcgccctcccgacgagcaatccgaaaaggcgtatttctggatgaggattcgtctggaagtcgtcgaaaaggtgggagacccgtactggattcgtgattaaccgttgtatcgacagaaggagaccgtaaatgggcagcgagaattacacccttggccgtggcgaactgcatttcgacaagttcgcaccgggcacgttcaacaagaccggcgagcgctacctcggcaacacgccggagttgaaccgcaccaccgagagcgaaaacctcgatcacttcaacagtgaccgtggcattcgcgtcaaggacaagagcatcgtgctcgaaaagaacgacagcggcacgttcatcgccgacgaaatcagcgacgagaacatcgcgctgtggttcctcggtacgcagaacgtggtcgcgcagtcggcgaccgccagcgtggtgcagaacatcccggccaaccgcgtcaagccgggcacctacatccagctcggcgagtcgcaggccaacccgaccggccatcgcaacgtgaccctgaccagcgtcaccagcgatccggtcggcacgaccttcgacaacctgaccgactacaccgtcgaccccgagctgggccggctgtacatcgtgccgggcggggccatcgacgggaccgagccgttgatcgtgacctacgccaccgccgcgtcgacccggacgcagatcgtggtgggcgagggcacgaccatcgaaggcgcgctgcgcttcatctcgtacaacccgaccgggccgcgccgcgactactactggccgtacgtgcagctccgggccgatggcgacttcgcgatgaagggcgacgaatggcagcagctttcgttcgcattcgacatcctgaagcgggacggctacgcttccgagtacatcgacggtcgcccgaccgccgcgtaaccggggatcgtcaaacgcggtcaaggccaacttagtcaagaccaagcgagccaagaccaacttgacaggccgcctcgggtatcccccggggcggcctgtctcataaccaccagaggaaaaacgcatgtcccttgccaacctgcaactccgcactgcaaccgttccgtatgtcggcgcgaacgacgagcagcacgacatcgtgctgcacggcctcagcgccaatgccatcgccggtctcatcctgtcgcagctcagtaacatcgaagaaatcttcaacatcgtcgaaggtgccggcgtcaagaaagccgaagacctcgcaaacgtcaacatcgtcgaagtcggccagcggcttctcgtgcagctccccgatttcatcgcgcacgtcatcgcgtactccgcgcacgagccggagcagtggagcaaggtgatgcacctgcctgcgcccgtgcaggtcgattgcttgaacaagctcgcgaagctcacgttccaagacgaggccggcttccgagaattcgtgggaaacgtggtcgcggcactgcgaagcgcaaaaggcgtagtgccgcagaacagcaaccgaaatctcgccgccagcggttcgccgaatggtggctcggcatccgcgccgcagtctctttcctgacggcggaaggtcactcgaacgctggcgaatatccactcgggtatttgatcgtcgaagccgaaatcgcacgcgagcgagtgaacaacaggatcagaacggaaatgacgctgacgcagagtgctatcgcctcggcgctcagcaagaaagcagcatcggcattcaaagaaaacatcgaaggactataggcgatggccgctcagaacgaagttgaactgattgtacgtgcgaagaacctcagcacgcgaaccatcaaccagctcaacgacgagctgagcaagatcgcagataaccaagagcaagtagccgatgcgaaccgactggcggagcggtcgttcgagagcctgaagtccgagcagcagcagttgctcgcgatcatgaagtctctcaacgaccgcgcttccaagctcgatgcgtactcgcggcaggagcagcaagtccgcagtctgcgcgacgagctgagccgcgcacgcgacaacctcaacacgctcgcgcaggagttctacaagacggagaagccgtcgaaggaattcacgcagcagttgaagacggccgccagcgaagtgacgaggttggaatcgtcgctgcgcaacaacgagcgccgtctggaaaccactggcacgaagctgcgcgacatgggcgtggatgtcacgcgcttctcgcagtcgcaggccgaagtcaatcaggcgctcaacagctcggtcgcgctgtacaagcgctcgaccgacaacgtggagcgctacgacgccgccgtcaaggaagtgcgcacgacgcagcagcaggcccgcgaggctgagcgcgccgccgcgcaggaagcccgcgactcggcggcgaagctggaacaggccgcccgcgagcgcgaagaccagatgcgccgcgagcagaagatggccgagctgacggccaacgtctaccgcacgctggcccgggagaaagaaaaggcggctcaggccggggcgcagttccgcgcgggcggcacgcaggcgctcgctgcggcccgcgcggcggctgtccctgccgtgggtagcgggtcggccgcgagcggggctgctgcgggcgtacaggcgcttctcgacccggccaaggatgcggtcgcgacgctcgaccggctggaagaggccgtcgaccagctcgacgaggaattcaaggcgctcacgccggacgccctgcaagccgctgacggcatcgacaagctggccgatcaaagccgccggctgcgcgctgccgccgatgcgctgaaggggcaggccgggctcgccgacgaattgaaccgccagaacaccgcgctgctcgcgagccaacagcggttcgaggaagcgcggcaagaagtgatccagtacgcgcaggcggtcgagcgcgccgacaagccgaacgacgaactggcggcgtcgttgcagcgcgcgcagaacgagatgaagcaggcgcacggcgaactgacgcgccagaccgaagcgttcaaccgtgtgcagcagcgcgccgctgccgccggcatcacgctcaacaacctgaccggcatcgagcagcgtctcgctcaggccgcgacgcgcgtgcgcaccgggcaggagcaggtcgcgcagacgatgacgcggttggagcagacgaccgcgaagaccaacacgcagttgaagctcttcaacgacggtcagcgtaccgcgctgtcgctgtatcagcgcacccgtggtcaggtgctctcgctggtctccgcgtatgtcggcgtgttcggtgcgctgaacctcgtcaacagcgcgatggatgcggcactggaacgcgagcgcgtcatgtcgcgtctgctcatcgcgaacaagggcaaccagactgcggcggcggaagaatacgactacctacgcaagaaggccgacgagctgggcgctgcgttcgggccgctgtccgagtcgtactcgcgcttcgccgtcgctgcacgcgacgcaggcatgagcaccgaggcgacgcgctacatcttcgaggcgttcaccgaagctgcgaccgcgatgcggttgagcggcgacgaaacggccggcgcgttccgtgcgttggagcaaatcttctcaaagggcttcatccaagcggaagagctgcgtggtcagttgggcgaccgcatgactggcgcgttcaacctgttcgcgaaggccatcggcgtcacgacgcaagagttgaacaacatgctcgaaaagggcggcgaagtgaaagcagagttcgtgctgctcgccgcacagactgcccgtggcatctacggcccgcaggcgaaggctgcgtcgaatagtttgctcggcgacctcaaccgcatgcagaacgcatggggcgatctgaagcgcgaaatcatcgacggcggcctcggcgatgcgctgcgtcgtttgttcgtcgacctgacgaagtacctgaagagcgacgacggcaagaagttcgcggagaacttgacgaaggtgttcgtcgctgcggccgacgctggcggcgaactgctgaaggtgctcgcggagaacgacgaaatcatcaagctggtggcggacaccgttgcgttcctcatcaagaacttcaaggcgctgctggcgatcatgctggcgattcagggcgcgcgcatcgcaatggtgttcacgtcgctcgcaacggaaatcctgaaggcgcgtgcggcgacgctcgcgctaaacactgctctcggtgccggcactgcggcgtcggcgggtcgcgcgggtgtcgcgctgggcggcctcatctccgggccgattgccgcgatcctcgccatcgcggctgcgggcatcatcatcccgatctatttccagatgaagggcgagctggaatcgaacaaggtcaaggtcgacgcgcagaagacgatcaacgacttgaaccgtgggttcgaggtctcgcagcgcagcctgtccgacacgtcgaagaccaacgccgaacaactcgaacgtcaggtcacggcggcgtcgcggctgctcgaaatctacgacaagcagaaggagtcgctgcaagcgcagattcgcgagaacacggccgtacgccgaaaccaagtggcggttcgcgttgcgcagggtacgcgcgagcacgacatgaatttcccggccaagcagctcgccgctgtgcgggaagtcgagaacgaaggcaaggcactggaagcacagctcgccgcactcgaacagcgtgccgctccgcttcgccagcaagtcgctgccgccagccggcagatcggcgagacgaaagcacgcgaggcggctgcggagaacgacgcgcttgcggctgagttcaagcgcattcaagcggcggccgatgccgctgctgcgcgtgctggcaccgacgcaaaggcggcgaaggcggctgaggctgcgcgcaagaaggccgaggctgaagagaagcgtctggccgcgctcgccgagcgccggctgcgtctggaagaggacgtagcggaaaagctgcgcgacatcgacaacgacatcgccaactcgcgcccggatacgctcgaagcgcggctggctgtgatcgacaacaagatcgcggatcgcaaggctgaactggaacgcatgctgcgcgaagccgacaagctcggtcagtcggatgcggccaagggcgagattcagcgcggcatcaattcgctgcctgagttgcagaaggcacagcagcaggcgacgacgcaggagttctacgagcagcggatcaacgacctgttgcaacagcggcagtcgtcgatggatgcgatcaacaccttgcaagaggccggactgctgacgaccaccgaagccgcaacccggatcgaggaagtcaacgcgcgtcttctgccgcagctcgaagcgttgcgcgcgaaggccgccgagttcatggcgacgctgggggacggcccgcaggcgcaggccgcgcgcgcaagcctcgaaaacctgagcgcgcagattcaggcgatgtcggtcgaactcagcgcgcagaagcgacaggtgatcgacgtgttcgtcaacggcttcggtcaggcgttcatggagaccgcgaccctcatctccgacacgctgaagggcgtgcaggatgccggcgacgcatggaaggcattcggcgacatcgtgctcaacaccatcgccgacatcctcatccagctcgcgcagatgattattcagcaggcgattttcaacgcgctgaaggcggcggccgagaacagcggcggcggctggggccagattatcagcgcggtcgcgagctacctgcacgttggcggcctcgctggttccggctccggccgtcgttcgtcggtgccggcgtacgtgttcgaggctgcgccgcgttaccacacgggcggcgtcgcgggcctcgctcccgacgaagtgccggcggtgctgaagcgcaacgaggaagtgctgaccgaagacgatccgcgccaccgctttaacggcggaatggcgggcggcgctcagcctgcgatggacgtgtccatcatcaacaccatcgacagcgagagcgtggtcgctgccggcgcgaacacccgcgcaggacgccagtccatcttcaacgcaatcaaggccgaccgcagctcgtacaagaaacttctcgcataaggaatcgacatgggacacgtaattgcaactgtgactggcggcagcggcgacgaggcgcactacaaggtgctcgctgcgatcaagacgctcgccgaggcgaacgggtggacgacgctgcgctacgtcaacaccggaaccgtgcgcgagttgatcctcaactcgtccggcctgtcgggtaccgaagacatctacatcggcttccgcacctacagcagcgtgagcggcgactactacaacatgctcgtcggcacgtttaccggctacgtctccgcgaactcgttcgactcgcaaccgggcgcgaagctgagtggtgtgccttgccacaacaacgcggtgacgtacttcatcactgcgaacgcgcaacgcatcgcgggctgcttcaaggtcggcactccggtctacacccacttctacgcaggcaagatgtttccctactcgcgtccgggcgagttcccgtcgccgctggtgtgtgccggcatgttcgacggtgcagcaccgaagcgtttcagcgacaccgactaccgcttcccgtatcacggccgcgagtcgggctatacgggcggctcttcgtcgaacgtgcgtccgtcgtacctgtggttgcgcgatcaagcaggtacgtggcgtcggctgtcgcacttcccgttctacaacggcccggccggcagcgatgcgtcgagcgcctacaacgcgctcgaaaactggaactacttgaccggcggcgatcaaagccgttcgctcgttccggccggcacgaattaccagccgcagccgatcatcctgtacaccacgagcgcgccggccggcgtgtgggaaggtgcggtgtacggcgagctggacggcgtgtacgccgtgtccggcttcaacaacaacgtcgagaacgtgttgcaggtcggcggcacctacgtcgacccggcgggcctgagcatcgccgatcacgtcgcggacattctcactgccggcgggcgtgcgttcgtcgtgttgcaggacgtgaatcaaaccgactggcgcagctttatcgcattggagatgacctaatggcttactacaccggcaacttttcctcgttcgcatcgctgaagaattcggtcgagaccgcacttcaggcaaacggctgggggctcaacggcgacggcgtgctggaaaagaacggcatgtacctgcgcctcactgcgactgctgcgcaactgctgttgcaggccggcaccggaagcgcaaccggcgcgctgcccggcgctgcgccgaacggcgtcaagatcatggacttcgagggttcgccgatgaatttcccggcgacttacgacctgcacgtcaacgtcggcccggacgaagtgttcctcgtggtcaactacaacgccgacaagtaccagcagctctcgtggggcaagtcgaacatccagcagatcggcggcaccggcatgtggttctcaggctcgttcaacgagaacgccgcgtcgaaccagaaccagctcgtgtataccagcgccgacgcgagctacttcggcttcggttggtcgggcatgggctgcggcctgttcgctgagtattacacgcaggcgctcggttgctcctacatccacaccggcctcgattcgactgcgtggcgtcgcgtctacagcggtgacggcaacctcgtcggttccggcgatgtcgttgcgggcctgctgcaagcgttgccgtcgatgttcaaccagaacacggtgctgctgccgctgctggtcacgcagcgtcgtctctcgcagggccagaccatcgtcgccgacatggtgaacgcacgcctgtgccgcaacgacaatcacctgtccggggaaatcgtcacctacggcaccgaccgctggaaggtgtacccgttccaccgcaagaacgccgacgtgcgcaacggcgtcccgtggtcgacgggcgcgaaccactccggcactttcgcctacgcgatccgctacacggggccgtaactcatggcaggcatcaccggacaattcagcagtgaagtcgagcgcggcatcaacaacgcgatgctgagcgaggacttggacgacaacaccgaagtcgtctcgatgttcgacttttacgaaatgcgcccgggccttcaaggcggctacgggcgctggcgcgtgcatgccgacaaccattggggcgtcatcggtcagcgcaagtcgaccagcttcttcgacgactactacaaccgcatctacatcgtgccggccgcactcgacgccggcaatttgctgtcgacgcaggtacgccacatcatcctgtggaatgcgtacgttacgccgcagaccttggaaaacgccgcgctcggcccgcaggcaggcatctcgatgtcgctgccggtcggcgtgagtctgccgtacgagatggagccgctgcgcgagctggacttcaccgtgcagatcgaactcagtggcccgccgactatcgacagctatgcgaacttcactgtcgagggcatcacctacaccgtgccgatcaccggccgacgcatcgtgctgttcccgttcgcgccgaattggggctcgcctgtcgacgagacggtcacgatgcgctcgtgggttctggccgccgaggatggcagcgagcagaccggcagcgagtcgggcgaagtgccgcgccgcacgctcgaatacaacatcaacctgcgcacggcgttgcaggcgcagcgatgcgagaacctgctgttcgcgtggcagtcgcgcttcttcggcgtgccgcattggggcgaggaagagcgcatcgacgcagacgtggcggccggcgctacgacgattccgttcgacaccttcggcctgtcgctcgaacccggctcgctggtcgcgctgtacctcgacgacgagacgaacgaaatccgcgaagtgcagacggtcggcgtcgacggcattacggtcacgaccgggttgcaatacgactggccggaaggctcgcgcatctatccgtgcttcgtcgggctcatgaacgatgcgatgagtggatcgcgcgaaacgtcgacggtgggccgcatgccggtcgcgttcgactgcgaaccgagcgtgaccccgggcaacgtcgcgctcaacatcgcgccgttgacataccggggcaaggagctgtttctcggtcgcatcaactggcagtcggctatgcccttcaccttcacgtcggatgtcaagcgcgtcgactcgaacaccggcaagttcgtcgcgttctcgtcggcaggcttctcgaagatgtcgcgccggcacaactggacgctgttcaaccgtggcgacatcttctcgttccggcagttcctcggccgccggcagggcgtcgcgcgttcggtgttcatgccgagcggcacggtcgacttcaacatggccgcgccgatcctcgacaccgaagacatcctcgtggtcgagaacaacgaatacggcgcgctggccggcgcacacccggcacgccgcgacatcatcatcgagctgcacgacggcacgtatttctgccgccgcattctcggcaccagcgacttcgacaacttcacccggctgcaactcgattcgtcgctgggcgtctcgctcgatgtcgacgacgtggcgcgtatcagcttcctcacgctgtaccgcttcgagtcgccgtccaccaccatccgccacctgaccgactcgaaggctacggtagaagccatcatggtcgcgaagacgaccgaggattgacatgagcctcttgcaatacgaaagcgacaaggaactcagctcccgcgtggagctgtacttgttcgagagcgacgatggccgctatcgctgggcctacacgaccgatgcgcgcgaaaaggtgctcggccccatcgtgtacaagcccgagtcgatcaagcgcggcgagctgaagcagacggccggcgacgcgaatatcgagaacctgcaagtcacgatgccgttcgacaacccggtggcactggcgcatgtgccgtacctgccggcgcggccgatcaagctgacgatctacgcctaccagcgcaacgaccctgctgcggaaatcgtgcaggcattcaccggccacatcaccagtttcaaccagaagggcgctgaggccacgctcgaatgctcgcagatcatcgacaacctctcgcagacggtcccgtgggcggtgttcaagagcggctgcatttggggcttgtaccaagtcggctgcggcgtcgacaagcagttgtggaagaacgatgcgctggtcacgaccgtcaacggtgcggtgctgggctcgcctgagttctcggccaagccgaccggctggtacaccaacggcttcgcctacaacccggcaaccggcgagcagcgcttcatcgttgcgcacgacgccgccgccggcacgatcacgctggtgtatccgttcctcgaaattaacgggagccagatcatcgaggtttacgccggctgcgcacgcacgaaggaagtgtgcgcggacaagttcaacaacaagctcaactacgtcgggttcgatcacttcccggcctacaacgtcttctcgcaggggatcacctaatggtttgggtagccatcgtagttgcgctcgtcatggctgtagttggtgagctgcttcggccgaagccgaaattcaacgacccgaagccttctgctgtcggcgacttctcgttcccgactgcggatgcctcgcgcgtcattccgatcttcttcggtacctgcaagatgcaaggcccgaacgtcgtgtggttcggcgacctgacgatcatcacgctgaagaagaaggtcaagaccggctggttctcgtcgaagcgcatcgtcaccgggtacaactattacctcggcgtgcagcttgtgttcgcctacgggccgtgcgacgagttcatcgagctgcgtatcgacgacaaggttgcgccgatcagcaacaagacgttcactggcgacgtgtgctcgttctacatcaacgcgccgacgattatcagcaacgacgacccgccgaacggcgtcaagggcaactgcaagctgtatcgcggcaccttcgagcagccgccgaatatgtacctgagcgagcagtgggacgagccggagatgaccgcgttccgtccgctgctgcacatggtcatggagaagtgctacctcggcaacaccgacacgccgccgcccatctcgatcatcacgcgccgctgcccgaaccagctcggcttgaccggcggccggcacaacgtcaacggcgactcgaacatcgcgtgcgcggtgtacgaggtcatgaccaacaatatgtggggcatgaaaatccccgaagacaagatcgacgtggattcgttcatcgcctgcggcaacacgctggccgacgagagcatcggcatctcgatgctggtgcagaccgccatgctcggccgcgacctcgtggcggaaatgctgcggcacgctgacggcgtggtgtacgccgacccggtgacgggcctgtacacgatgacgctggctcgcgagattcccgacgaagagcaagacgagctgctgattgtcgacgactcgaacatcctgccggatacgttcgagttctcgcgttcgtcgtgggaaatgacgaagaacacgatcatcgtgcagtacaccgaccgcaccacgttcgagacgacgccggtccaataccaagacctcgcgaatatcgacgtgcgcgggggcatgatcgactcggaagaattcagctacctcggcttcagcaactcgaccgccgcgatgaacaccgctgctcgcgtgtcgaagatgaaggcgtcgccgttggtgtcagcgaagatgtcgctcaaccgcatcggctaccagctccgtcccggttctgcgttctggctgcgcaagccgaaccgtggactggcgaacgtgctcatgcgcgtcatcgaaatcaactacggcacgctggacgacccggccgtcaagatcacggcgatggaagacatcttcgcggtcaatgccgtggcctacgttccgccggacccgagcgactggcaaccgccggttggcgcggtcgtgccgttcacgcagcagcgcatcatcgaagcgccggcattcggtgccgaggatatgtcgcggcgctacgtcatcacgatgggcgtgccgaacagcaacggcgtgatcggctacgacgtgtggaccgacaccagcggcggcacgaacttccagcagacgaacgccatcgacgcgctcacgccttcgggcgtgctggtgtcgggtttgtcgcgcaccgggccggaagtcgatgctgcgggcttcaccgtcacgtcggtcgtcggagtggctgacatcgaagcgggcactacgggctcgcgcgagtcgggcgaaaatctgctgctggtcggcaacgaactcatggcgtggcagaacatcgtcaacaacggcaacgacacctacacggttactggcgtgtatcgcggcgtgctcgacaccatgccgcaagaccacggctccggcgcgcgcgtttacttcatgtcggaaggtgcaggcacgaccaacgaagacggctacggcggcgacctgacgctcaacacgaagctgacgccgaagagcatcgtcgacacggtgccgctggacaacgctgcggcgatgtcggtcacgaccaacgctcgtgcgctgcgtccgctgccgccgggtcgtctgcgcatcgacggtgcagtcgtcggctccggcgcaacctacgacggcgacatgctgttctcgtgggcgcaccgcaaccgcctcgacgacagcatcgcatcgcaggccgatccaagccgtacgcccgaggaaggcacgacctacaacatccgggtctacaccagctcgaacgcgctgctggcatctgcgctggaagtgtcgagcgccgcatcgaccggcaccatgcggttcgcggtgtcaggcgatatgcgcattgaaatcgaggcggttcgggacggctatgtgtcgtggacgaagctggtcggctacttcagctatactccggcctcgggggctaccgccaacgaaatcatcgtcgacgagcctgagtacgtcttggacgggggtggcgcgtaatggcacaggtagtcgttgcacaacgcatgtggcagcgccgcgacactgcggcgaattgggctgcgaagaatccgatccttgcgggcggcgaaatcggcgtgcagctcggcgctacttcggacgagaccaagttcaagatcggcgacggcgtgaccccgtggaactcgttgtcgttcttcgagggtcggctcatcgaaatcggcacgggcggcggctacatccgctggcgctatgtcggtgatccgacgtggatcaatctggtctcgctcgaatcgctgcgcggcccgcagggtgcgcaaggcaacccgggcgcgaacggcctgagcgcgtatcaggtcgcggtcgccaacgggttcgccggcacgcaggccgaatggctcgcatcgctgaaaggcgagaagggcgatcaaggcgaccaagggccgcccggtattccgtcgcagcgtcgcatcctgcgtatcacgaacaccgacagcggctccatcgtgtgcgactggaatgcctacgacgaaattcgcgtgacgctgactgccgacacgctcgtcaatatgacgggcgcgctggacggtcaaggctgcgtgctgctgctgaagcaaggcggcgtcggcggtcacggcgtttcgttcggcagcaacgtgcgcttcaacaacctcatcccgatctacaacccgacaacgactgccggcaagtccgacaggctcggcttcgtttatgacgacgacgccggcttctacgacgtgcaggcaatcgtggatggaatctaacgatggcagacgactacatcccgccgttgtcgccgaacatcgtgtgggtcttcaagggcaacgactacacgcccccactgaccccgaacatcgaatggatattcggtgcagatgatgaaggcggcggaaacgagcttcgcaaatccacctacatgctaatcctgacaatgtgaggtattgaaatgactgttcgcacctactcttcttccgacgctggcgctccggttctgcgcggcaacacgccgggcgacctcatcaacctgctcgaaaagtgcctcgtcaccggctacggctcgaaggccggcgcaggctggacgaagccgtacaccggcacgaacgttgccgcgtttcagcagggcgcgggctcgaacggcatgttcctgcgcgtcgacgatacgagcacggcgaccagctaccgtgcagcgcgcatcgtgggctacgagtcgatgagcgatgtcaacaccggcacgccgacttcgttcccgacgccggcgcagcgcagcggcggtgcggcgtggttcacgcactacagcagcggctccgttgcgaatcctcgcccgtggcgcatcgttgccgacgagatgttcttctggttcttcctgtcgacctacccggaaaacaacgacagcggcttctactacaacgagagctatgcgttcggcgacatcatcccgttcaagccgggcgacacgacgcacaccatcttgctcgccagctactcggtcgattcgccgaattcttcggagacttacccgtgggatggcgttagcatttcgagcgcgatgggaggcaatcgctacggcctgtgggcggcgcgttcctacacgaacctcggcggcccgatctggctcggctggcacgccgatcacgtcaaggcttcttcggcttggggccaaggattcctgtcgtacccgcatggcccggacggtggcttgtacctgtcgcctgtgtgggttcacgagtaccacgtctcgccgtacaacgtgcgcgggatcatgccgggcctgtgggtgccgtgccactaccaaggaatcctgagccagtatcaggtgttcgatggtcagggcgaattggccggaaggcagttcatggctcgccgccactacgagcgcacggtctgcatcgaaatctcgaatacttgggataggtaacgcgcgatggcgctcatcttcaacctgccgatgacggggccgaacggctccacgacgatcaccgacaccacggggaatttctcgtggtcggtgacaggcaacgcgcagattcaatccaacgctctcgtccttgacgggagcggtgactacgtgagcaccactgctgacgttcgattgaacttcgggccgatcaacgatttccgtatcgcgttcgacatgaagatggcggctgcggacaagggcggctataagatcatcttcgaccagctcaacaagggtgcgtcgaatacgtggacgtggcagctctacacctatgaaggtgtgccgtacttcaacgtctataacaattactacggcaatccgacgccggttcaaggcacgaccgatcttgctgacggcaactggcacacggttgaagtcattcgcactggcggcgctctctcgatgtgggttgacggcgtgcaggttgcaactgctaccgacaatcgcgactacgtgttccagccgcctttcggtatcggttcgcgtatcggctacaacgcatcgtcggcctacgactacaagggcgagctgcgcaacctgtccatctcgatcacgacgccggtcatcctgacgaatcgcatcgcgtcttggactcggcacagcgacatcggctggaaccgtggccgccgcagcagcttcattcggcgcatggcgttctacccggtgcagccggtcacgaccaagaaggtgcagacggtcaaggtgacgcgcggcgtgccgccgtggtgggggccgagcgggtcgaccacgcagctcccgacgtacaagctgcgcggccgggtgatgcagcgcgatcctgacggcgtgttgcccgacgccccggtacagtacgcgcgcgtcgtgctgttcttccggcgcttgcatacgctcgtagacatccagctctccgatgtcgacggctacgtgcaattcgataacctcatgccgggcagtcaagcgtactacgcgattgcattcgacccggaaggcgcaccgttgcagaacgcggtgatttgggatcgactgtcgcccgagcccggcccgtaaggagaagtgccgtgagcccgaacaacaccaacgagcagaacaggaaccgacgagtgacggacaaagcagggggacttctggacgccgcgcaacaggccattcggcttgaacgcatcgaaggcgatatgcgtctgctcacgcagcgcgtcagctccggcatggagaacgtcagcaccacgctcgcggccgtgcaggtcgaagtgcgcggttgctcgacgaatgtgtcggagctgcgtgggctgcaaggcgcgcacgactcgaacaaggtagcaatcgacaaggtggagaaatcagtgtcggaacttggtgcgaggttggagtcgtggttcgatgagttcgaggccaagcaggaacaacggtggcgcgactactcgaacaaccgcgatcaatggcggcgcgagcacgaagccgagaacgaaaacgtcaagaaggatttggagaaggaaatccgcagcgtgcgcgagaccgtcatccgcttcgtcgggttcggttccgcaatcggcgcattggcgggcgtgatcgttggcggcttcctgtggaacatcaactaccgcttcaacgacaacaaagaggacacggatcgcgtcgagaagtcgtcggcctacaaccggcagctcatcgacgcgatgggtgtagaacacggcaaagagctggccgacatcaagctctatctcgctcgcgggggccgcatccccgaagagccctacgttccgcaatcacagaggaaagaaaatggacaccaacaacagcagcccggccaacccggaaagtaagatgccgttccgtcgtcgcgcgtgggagttctggcgccgcaaccagatcatcctcttccagctcccggtcatgctggtcttcctcatcggcagctacatcgtgctgaagtcggtcgactcgcgcatcggcgtcgaaggcttcggcgacatcttcggctacgcgctcaacgcggtgcgcatcacgctcatcatcttcaccgcatggtggatgaagaagtggtgctggttcgacctgcacgaccgcaccgaactcgaactgttcgacctgcgcaagcaaggcaaccgcgacgcgcactggatcgtctggaccgaccgcatcgagtggatgctggcgctggcgttcgcgaccttctggtacacccgatgagcgcccgggtcgtagtcctcgctgcggccctcctgctgggcgcgtgcgcccggccggcagcggtacccccggtcgaccagaccgtgctcccgccggccgtggagagcctgccagcggccacgccggagccggtcgtcgagcaggtcgtctcggcccaacccctgccccgggccgagcaggcggtttcggagaccgtcacggagccgcttctggctgcgcaggcggcgctcgcggaccttaccccgctactacccccgccgccggcccgggacgcggcttgccggcgcgctgcggcggccctgacgctacgctgggaagtgaccagcccggcgttctaccggaagcggctcgaactgccgatctggccgggcggggcgtccggggtgacgtgggggatcgggtacgacggcggccaccagccccgggcggtgatcctcgacgactggcacgaccacaggcaggtcgaccggctgggccagaccgccggcatcgtgggccaaccggccaaggtggcgctgccgcgcttccgcgacatcccgaccggcttcgaccacgccagtcgcgtgttcgaggaacgcagcctcgtcgagtacgagcgccgcaccgagcgcgcgttccgcaatggcttcacggagctgcggccgaacgcatgcggggcgctcatctcgctggtgtacaaccgtggcgcggcgatgaccggcgactcgcgacgggagatgcgcaacatccgcgacaactgcgtaccgaagcaggactatgcctgcatcgcttcggagattcgcagcatgaagcggttgtggcgcggcacggtcaatgagaacggattgtctgcgcgccgcgaggccgaagcgatcctcgtcgaaaccccgtaaggagatgagcatgtggacgaaagcaatcgcgtggctgttcggaacggcgatgggtcgcggtgtgctgcttggcggcagcatcgcgataggcatggcgctcggctggtatgcgttctcgacgcactactacaacgagggcgtcgcgtcttgccaagctggccgcgccaccgatacgaacgcggccaacgtcgcgcaaggtgaaaagaacatcgccgacaaccagaccgcttcggaaatcggcaaggtcgccgacgccgaagcagcgaaggtcgcagccgatgccgaagaagcgaagaacgactcgaaggagaccatccatgatgtgtacaaaaagccgcccgtcactgcgcctgttgctgttggttcttgtgttcaccctctcgatgagcgggtgcaagaccggatcggcaaagcgcgagctgccgcagttgaagcaagaggcaccgctcgttaactgcaagcagcctgcgtcgccggcagtgccgcgcgagccgaaggccgacgagtggatcgagtggaacccgccgcgcccgggcaagaccgaaggcgaagcgcggctcagcgagcgtgcggtgaactggatcatcgacgtgctgggcgtggtgcgagtgagcgaggggtaccgccgcgtcgagcatggatgcctcgacgacctcgaagcgaaagggctcatccggcagtagttgacaggcccgaggcgctgcattacggttgatcccgctggtggcacttcgcgttgcatcggcactcggcagagggacagcggcgcggtgaatcggcgctccgcaccgcagggaacgaggaaccccggactaaccatccggggtttctttttgcgtcaagaccaagtgcgtcgtgaccaagttcgtcaagacccaaaaagaaaccccgcaacgttgccggggcggggtctcgggtcgctgcggcgtcgcgccggagcagtgggtatcgaggcggtggttctgctgattccggtgtccgctcgtggagcgctgcgccggctggaagggcaatgtcgcgtcgatgagtcgaccctaatgcgatgcgctcagggtgtcaacaccttcgtcagtccttccacgtctcgaccagcttcatcatcttcttgcgcgccttctcgacgccggcactccatttgtcccacgccttcgtgtcgacgtgcgtcaggatttcgttgcgcgccatttcgctcagcacggtcggcggcagcgcgtccagctcccagctcttgtcgccgaagcgctggcggtatttcacgaagcgcgcgtcggtcgtcttggccgggttcggcggcggcttcagttcttcgatctggtcgaggttcaacgccatgcgcttcagcgtgaactcgccgttccagccgaacagctcgaagcgctcttcgaggtcgcgcgtcatgtcgatgccgctcgggtcatggtctccgaagtgcaggatcacgacatccttgccgtcgctctcttcgatttcccgcttcgcgaaatcgcgcacgaccgatgcgctcgggtagccgcgcgccgcgagcagcggcacgtcgaactcgtggcacacgcggctgaagacgccaaccagcgcttccttctcgacgacgaggaacaggcgcttttcctgcgtcgcccacgggtcggtgtggtactgccgcgccgacgccgtgagaatgtcctgcgggcgcgaccaacggctgcgctgctcgaacgagcgcgtgcggtcttcgatagcgtcccaatcaatcaggccggcgatgcgcgcgtcgttgacgatgctcgtggtctgcttgtacgacttctcgttgttcggaatgatgtcgcgactgaccaactgatagaacaactggcggacggtcagcgtgtagcctgcgtccagatactcttcgatgatcgcgttcatgcgatcaatctgtgcaagcgtcttcgtcttgaaggtgatttccttgtagcgttcacggctcatggctttttctctcggcagattggttgcgggttttcagcgagcgcagcttttcccaatattcgctgcggcgttgctctagttcggcgtcgacagcacttccgccgttcgcaccgccgcgtcgtgccggcggcagtcgcaggaagtcgagcgcgatcaacgcttcttcccgtttcgtcacgagccacggcagaacagcttcaatgacgagttccgcgtccgtcgcgttgcagaaccatgtgtacgcggacgagtagtgttgcttctggctatcttgcatgtgcagcgatccgagcccggtgatttcccggcaccgccgcacagttgcaagatggcacatcgagaccttcaggacgagccggtagttcgggctaacgcaccgattcttccgctgcgggcttcgacgggtcagacttatgcagccctcgccgtcgatcaaaccggcgagccacgcaagctgctcgcgtcgattcaccctgcctgctcctgcgcgcggatgtcggtcgcgcggatggcttcgacttccggcggcagctcgatgcgctcgaccgcatagcccacgtcgcgcccgtagtacacgccgcgcacgtcgggcaccgggtagatgtggtagcagccggcgtgcatgtgcagcgcgtggtggatgcgctgctcgatctgcgggtaggtgtgcggattgtccgggctcggctgcacggtgcgcacgccgatgccgacgtaaccgctgcgcgccagcgtctcgcggaacagcgcggtgtggcctgcatgccacggctggtagcggccgatcatcgcgccctgcggcgtgaggtagcgcaggcatgcggcgatgcgttcgagcgtgggctgcatcacttcgcccgtgacttgcaccgcgacctgctgcgggcgctcgaacatttcgtcggtgtccgggtactggctcttctgcaccgtgtccatgaagacgatgcagtcaggcgcgaacgcctcgcgcgtctcttcggtcgggcacacgaacgaggcgacgacaatgccctcgtggctgtcggcgacctcgcgcatgagctgcgcttggcggatgcggccgggcgtgctgaagtcccaatcgccatgttcttcgcgcactgcgtcgccgtcgatgtgcgtcgccggcaggatgcgcgcaagagctgcgccgagcgtggtcttgccgctgcccggcaggccgcagatgaggatgcgcttagccattggcggcctccttcgcagcgcgcagttcttcgcgcacttccatgaggatttcgccgaggcggttcttgcctttgccgtcgcacacgccccaatacgtgtcgccccaccaattgccctcgaccagcttcgacttgccggtcttcaacagcttcgacttcagcggctcggttccgaacttctggcgcagcaggttgcgcatcacgtcttccttcacttcctcccaatcctcgcggagagtgacggtcttgccccggcgcttcgcaccgcctgcgtcgggttcgttgcgaatgcgacggcgctcgtcctcgtcgaacgtcttggccgcttggaaggcgtgctcgaccgtgcggtacgagtggccctcgaaagcgatggcgacggaccagaaattcgagaggaagcgatgcggcccggtgaatgatccgatggtcttcatggcgtgtcctagtggaagttgatcttggcgcggctgaagagctggcgttgcttcgccatgtcagtgcgcgcgatctggtcttggatcggaacctgcacgttgcggttcatcatctggtgcaggtagcgcggctcgacggcgtgcccggtcgcgaacttcgcaatcgccatgaggatttgcggcgagtgcagctcgaagaacgtgcctgtcatcgaccaatggtgcgggcggatgtgcgcagcgatgtcgagcagttgccgctcggccttgcgcacgttgagcggcggctggatgccctgcttctgcatcgagtgctcgacctcgctcgccgcgcgatgcacgacgaggtactgagcgcccgggaagcgcagcagcagttggtcgaagaagaacagcccggccacgtccgacacgaacacgcggccggaaggttgcgcgtcgatcttttggcccagctccgcgatgctcgcgcactgctgcaatgggttgtgcagcgacgcagcgcacagcggccgaaggaactcggccatccatgcgctgcggctacgcggcaggctgagcatgatcgtcagatgctcgtaggccacgtcacccttccttctgctcgcgcttcgcctgtgcgttgtccgcgtacgtgtcgagcacgcggacgaaggcgtcgtgcagcagcgtgccggcgggcacgtagatcaccgtgccgccggtcaggtcgttgcgggtgtagatggtcgcaggcgcgctctcgatgagctgaccttgaccttcgggcgtggcctgcatgcgatccggcggacgtgagtcgaactcgcgcaccatgccgtcagccggcccgccgacgaagaagcctcgaacggttgcattcatcgcacgtctccgtcgccctgcaacgtgccgcgttccttgcgcccgttgagcttttcgcggttgtcgaacagcagcttctcgtagccgccctcgcaacccaccagcggccccgtgcgctcggcgtactcgaccgacacggcgatcaccgcagcgagcgcaccgcgcagctcggcgatcttctccgcacgcttctcggcgctccacgtcgcaccgtcgcgcatcatcttcttgatgacgcccagcacgcggccggcgtgcgcacacagggccgattgcaggtcgtagccgctgatacggacctcgcggtactcggcgtcggcgaggcgctgcatgccttcctgcaccagcacgtcgaagcgcggcagctccggcgtctcggcgcacaggcgcgcggcgtaccactgcacgtcgcccagctcgtgccacgccttctgatagcgctcgacgcggaactcttcgcgaatggcttcttggtcgaacagctcggccagctcgccgacttcgttcgccagtccgatgccggtgtacaacatgccggcgctgacgttgccggcgagctgcacaatgtcggtcgggtacttggccgtggtgacggtgaaggcgttgtacgtttcggcgaagacacgcaccggctcgatgcgcgcggcacgcgcttcgcgtgcggtatcgagagacaggatgctcatgcgcggcccccggcggccaacgcctcggcgaagtcgttgctgtagctggcgtcgaacttcgtcgccatgtcgtgaagcacgagcgtggggccgccgtgcgcagccgggatcatcgcgaagtcgacaccgcgcacgagcgggttgcgcgcaccgtcgtcggcgatggcgtggacgaccagtgcatcggggttctcgcgcgcggcgcgacgctcggccttcaggatgcggcgcatggtcttgccgccgaacgccttgcgcaacttctcctgcggcgagccgtggtcgcggatcgcgaggacgccggcaatgccgccctttgacgtgcgcacttggcgcttgttcttctgctgctcgttcgcgttgtcgcgggcttgcagcaggaaggcgtagttctcgtcgacggcgagcatgcgcttgcgccacgggctcagggtcttgcccttctcggcgtcgtacgaacggaagatgcgcttcaacaggttcatcgtgtgctccttggaaatgaaaaagcggcccggccaatgtcgacagggccgcttcgatgtactacgtcaacgccacgggctcagcggccggcgacgaacttggtctgcttctgcacccggccgcgcttggtctcgcggaacagcacgatggtcgtgttgtcgtcggccatgatgctcgcgtcgtcgagcgcattgccctcggtcgcgaacgggccgttcatggtgctggccttctgcgtgccgtcttcctgcgcggtcagcagcaggtacgcgaactgcttcgcgcccttcttgccgcgacgcacgccaaccttgcgggcagcggtcttcttgccggccgggcgaccgcgcttcttggcgggtgcagcgacctcggccttcttcgcgacgcgcttggccggagccttcttcgcggcggccttgcgtgcggtcttcttggcgggagtggccttcttggtggccttcttggcggggcgcttcttcgcgaccttcgcctcggtggcttcggcgttctcggacatctggtttctcctagcgttgttgtcgacaactcgcggaatgcgagcggggttcccttgcgggattcggttcagtccacgcagtacgcggggacttcggtgcggaacgtccgacactcggacggctgcgtgatgtacaggcccgccatgcaggccagcagcagcacgacgtagacgatcttctcgcggcggctcatcactcgcagcccacggtggcattcgcgcgggtcgggtgcgcggcggtgtactggctgaagtcgcgccagccttccgagccgccgcacgcgaagccccagcggcgcacgatggagccggtcatgaagagcgtccagcacggctcgtcgttgttgccgaacagttcgagcaggtgcatgtggtcggcgctcagacggcggaagtcgcccgtgtggaattgctgcgtgtagtcgaacttgtgctggcccgggaacttgcccttgttgcgcgcgacgctgccttcgacgtaggtgcggccgtcgcccggggtgaacagtcggtgcatgtacgagacgtgcgcgtccatgccggcggcgctctcgtcgaccgcgtgttcgtagcaccactcgctcgtgtgctcgatgtaacggccgtcgaggatgagcgatgcgctgacccacggatggtcgtgcagtgcgcggtcgtcgtcaccgtggacgaacttgtgcaggtacaggttgaaccagcggttgcgcgggatgatgtgccagcgagtcaggtacgggcgacgcgggccgccgtcgatgccgtcgagcatgatgaccttgctcggcttgacgatgcgtgcgtagagcttgaacgcgccgacgaagaccgaccacaggccgatcatcgtgagcacgtcgaagaagcgacgggaaactttgggagcgatcatggcggggaacatcctcgggatgacgggaaagttcatgcgtcgagcgccgtgtcggcggcgacgggcacggccggcgcgctgctcgaaccgagcacgcctgcattgacgttggccttggtgaagtcgatctggtagcgctgcgccagatgcttcatgccggcgtcgatgcgcgtctggaagacggtcagcagttcgtcccgggaaagttcaccggcatgcgtgccgccttcggacaccacgcggaactgctcgactccgctgctggtgatgttggagtggttgtgctggtcgacgatgagcttgtcgagcaggtcgcgaatcttcggcacttcggcgatgtcgattttcattggttctctcggcgtgagatgaagagcggcgtatcgtgccgcaagccgccgggttgacccttcaagcgctggggagtgcgccatccagttgaccgggggtatcgcctcggcgaccccgtgcagttcgtgatttaccccgtagggggacgaagtaaattcgttactgcggggccactctagcgccagcttttcggcttgtcaacacccttcctcgtgtccggcggccggctcagccgggccatcttgcgctcgccccggaagagcctgtcgcgcagcatcttctcgctgacgtgcgggcagtgtcgcttgatctgctcgaacgtcatttcgtcgccgtcgatggtgtacagccgaacgcgcgcaacctctttcactgcgtaatcctcgtcgtcgaatttctgcctgctcatagcgcccgcccgtgggtctggatgtaaacgtcgtgcagcatctcgtgagcgactgccttgcgaaacgcttcctgctgcacaagcgcatgcgcgaagtcgcgagcgctcggctccttcatgccgagatgcgcggtcatgcgcagcgcctcgtcgatgatggcctgcggttcgccctcggcgtagccctcatcggcgagcagcgcatggatagcctcgcggtacttcgcgtgccgcgcgcgctgccgcagcatcgcaatgccagcgatgacgttggggccgatcaccagcagcaaccaatcgaaccagctcatacagacctcgcgtgtggacgctcttcgccttccttcggcgcaggaacgtggtggagtgtttcgagtcccttcttgatcttcgccgccatcgctttgccgaactccgacgcatcgccgtacatgaggtcgaggtcagggtcagcgcattcggcggcgacgttgcgcagcgtgtcgagcagcatcgggagctggtgctgcgcgctgtagttctggtggatcatcggccacgcgccctgcgccttccaccactgcttgcgctcgtgctcggtcagcgcgacgtattggtcgatcatcgccatcgcgaggaacggcgaccaaaagcacgtatcgaccggcgtgatcggctcgcccagctcatcgagcgcgaagtacaccgcgaatacgggcgtcgtgccgatgagatacacgggctcgtcgagcgggtctttgtacgtggcgatggtgtagccccggtacgcggccatgtgtgcgtagcggcgcttgctggcgtcagggagtggcatgcgaaaactctcgttgaagtacgggtcaagggacgctgaggcgtacaagcacgcctgcttgggctcaggttgcgcggctctcatggcgatgaagctgcgctcgctcacgcgccgcccgcgtcacgcacgagcacgacaggctcgccatcggcgtctccgtcaggcaggcacgaagcgagcacgtcggccgcgccctgcgtgtcgccgagcacgagcagttggatcgcggcgcggatcgcggtctcggtctcgaccgctttgcgctcggcggcgagcacgtagcccgcaccgtcgcacagctcttcgagcagatggcgcaaccactgcgcggtcgtaaggtctttgcgatccagcgtcacgccgtacttcttcaggccggcgtccgcgcgctgacggatgatcgcgatgaggtcgttcgtggtctgcatgtcgctcatggtcaaaagtccttggcaaaatcacgttcaacgcgcagcaaggccgaaacctttgcgtcgaactttttcggggtgtcgatgaggatgtccgccgcagcgcacgcgatgacgggagacgtgaagtaggcttggatcgggtgcagcacttcgccgaagtcgtcgacgatgtagtaggcaacgtggacgccaatgccgccgtcgagcacgaccagcgggccgccgtcgctgcgcacttggtcgctgtgcagctcggcgatgaacacgtcgcggtagggttggatgcgcttgaacttcatgcggctttttccttcaggtggtcgagctgccagccggcctcgattgcagcgaacaaccgcagctcgctcgcgtcgtcgacatcgaggcgcaggtactcgatgaagctgtcgatcatctgcggcgtcatcgggcgcttgtcgtagaaacggcggtatgcactttgcggaatcatgtcccacaccgggcacaggtcgacgatacgcttgccttcttcgcgaaggtggcggcgcatgatgtcgcgcaccgtcttcgggttcttcttgaccgtgatctttcggccagtcgacggacggaaactcatagcccgatgtcctgtccttcctcgcgcttcagcagccacatcggcttgcgcgagagcatcggcagcgggccgatccagccatcgacggagccgtggtgccggttccatccgtagttgtcccaccatcgcccgcgcatctggccgtactccggcaaccacacggcaatttccatctccgcgtgctgcggcagcgcgtgcgggtacgggtggtgccagatggcgtagaagccgaactccggcgggtcttcgagcacttcgatgtcttcgtagcgcatcggcccggcccagccgagcaccatgccggtgaagggcacgaacggcgtcttcaggctcggcctgcgctcccaccaatggccgttcgcccagcgcatcaccgcgtacatgcgcgggtcgtggacgattgtcgggttgcgcgtcaactcgacggcgtacagcccttcgactgccggatcgtcgagcacttcgagatgttcaatcttcgtcatgcggtgcctcaacgtgcgcgcgtagtggccgcaggcgcggcagcgggccgatccagccgtggacttctcccctgaagtattggtcgctgttgaggtagcaccagcggcccccgaaccacatgaggaagatgtcgacgacgagcccgcgaccgtgcgggtcgtctacgcggcaagcgtagacgcccgtgtcctgcggcagtccgatttcttcgtactgcaccttcatgctcactcgcccttcggtagcggcagcgcgtagaacagcacttcgccgctcatgcgctgcacggcgacgaccgcgtgaccgagcttgcgcgcggtcttgatcgaggtcgtcgtgtcggtgctgacgccggtctcgctggcgatatgcacgccgcccgggtactcgtgcgtccagctcgcgcgctgtgcatcgagcacgctttccagctcttcgacgcgccgcttgtagcgacgcgcgtcggcctgcgagatggtcttggacatggctcagacctcttcgcgagcggagtgggcctcgcacttggtcacgagcagcatgaagtgctcatgcggcaggcccagcagcgtgtcggcatcgagcgacgcgagcgcttccttcagcgcggccttgccgtggtgccgggcgaacagcagggcgtagtggcgaatcatctcgcgcatggtgtcctgctctcggcgcacgcgcgctgcgtcccacgcaccgccgcgctcctgcttcagcttgtcgacctcgcgcgtgcgcacgcccagcagggacgacagctcgcggttcttgtccgacagcttggcgacctcgttggtgctggtctcggcgatctgctggtagttgcgcatgtgcttgttgatcgagcggatggcacgcagcgcgagacccacgtcgtcgatgttctcgtagtgcgcgcccatgttgcgccagcccggcaccttgcgatccagctcgcggtagatgacgttgagctgccgttcggcgttggcttcgcggaagtccatcatcgcctcggccgcagcgtgcgcctgctcgccgacgttgcgcagcgcttcgctggcgtccttcgtgtccagccgcagctcgacctcgacgacctcgcgcgcttcgccttcgtcgtctgccggccgccacgttgcgagccacgtcgcatggtcccggtaggtgaacttggtgcggtggccgtcgccgtcgcgctccatcgtcacgtagtagtccgtgctgtccggcttgcgacgcgcgtcgatcacggtgtaggtgccgcccgagatgacggagaagtagcgctcgccagcggccggcggctgctcggtgccgtcgaactccacgttctcgatgaagtcgcggaacagcgactcgatgaggccgtagcccatgccgagttcgggcggcatgccgacgcggcgcgagcgtgcaggcttgaacgacacgtcatgcagctcggcggccatctgcgcgtacgggttgcccgggacagcgccggcagtcgtcggcgcgaacaggtcgttccatgcgctcgccgtggtgaatatccactcgtactcgccgccgcgaccgttgtcgacgcgcagcatgcggacgtggctgtggccctcgcactcgtgcgtgctgacgaccatgaagaagcgtgccgggcggttgcgatcctgccagtaggtgccgaccttcggcgcgaactcgtagcccgggtggccgaccgtcaccgcacgcgcttccttgcggtcgctcgctgcgcccttggtcgtctgcgtcttgctgaagtcgcggcgcatgatgcgctcgatgaggctcggcgtgcccttcatcgcatcggcgatagcgtccgggctgaagtcgatggtgttgatgatgtggatttccggctgcttcgagaacgggtactcgcggcggtgcggcttctcggccgagaacacggtgccgtcgtgcgcgttgaagaagaagctgtgctgaccgatgaaggtctcgcgaatccacttgtgcatgcgctgcgcttccgcgcgctggtcatcgctggtgccgacgacgccgccggtcgcatggatttcgcgcacgatgccctgctcgtcgacgcacgcagcgacggacacgatcatgggggtggtagcggtattgcggaactgcttttcgatgtgatgagacatttcggcgtttcctcgggttgggttaggtggtgctgacgtgaccggcggcctcgcggtcgagttgaaggtctgcgatgtcacgcagcgacgagggccagtcgtcgagcggcacgagtccgtcctcgtgcatggtgatctggtcaggcgtcatgccgcacaggtagtacgccttcgcgagcgagaagcctgcattgaggcgatagcgcttcgctgctgcgccccacttcaccgactcgcgctcgcgccagccgatccagccgcgtgcgttgcacagccggcacggccgcatctcgtactcgtcgtggatgatgtgcgtgagctggtgcttgtggccttcgcacttcgggcagacggtgcggtcgaacagttgaagccatgcagcgcgcaccttcatccgcagggcgagaattactgcgcgggtcagcagggtggtagcgctgcgcaggcgagacaaagggggtaccggagcgttccgaagagccgcaagcctacggcccaacattttcgcctctgcgatttcgcggtgcgtgtggcgcatggttgcggtcactccatccgggtgacagtgaggaacgcgaacatggcgtcgttgctggcgctcatgtaggtgccgcgctccatcttgaatcgcttcgacttgtgctcggccacgccgcgcaccttggcgatgccgccgctcaggatcgagttctgctgcttgaagtatttctgtgcctcgttgttgatcgcggcgatgttgccgttgtcgagcgggatgcgctggcagcgcgcgtgcgactcgccgatgtcgagcttgctgagctggtcgttgagcgagcccggcaggaagatgagccggggcttctcggtgatgcgcacgcgcgggttggcgatgtgcttcttcaatgcggccttcgaccccggcttcttgcgggtcttctgcgcagcgttggtgctgctgttcgtgctggcggatgccattgggttgtgcctcctgttccggggaagtaagcggacaggaaacatactactgcgcggccccgggtcggtgtcaagcccggcgttctcggtcacgacccattgggcactgctcgccgcactgaaaaacgatccggctgggttgccgaagcgggcgcatttttggaaccggctgggtcggcaaagcgagagcgcaatcggaaccggctggctttgcgaagcgggccgaattttggaacgggctgggtatccgaagcggggacgttttcggaattgcatcctcatatgtacgtgcgtgcggatgtgcgcgcgggcacgcatgcacgctcgcctgcgcacgcgctcacgttctatgtcacgcgggcgcgcggcgcgtgcgggcgcgtcaaggttccgcgcgctgcgcgttgcgcgcggttcgtttgtgcggcgatgcgttgcacgtcgcgcggttgccgttcgtcggctcgcaaaaataattgcgcggagtagttgcactactgcgcgggacgtgttctaattttctcgccggcacttccgccggcatcgcaaagggaagacaacatgcgcgccaatcgttccgaattcgccgcccatgccgcgctcgccgcgtcgcgtggcgcttccgctgttcgcaccatgcgcaacgctcgcaaggtgcagacgttgcgcgacgtgatcgcgcggcttcccttcctgttcgccgttgccgttgccgcgttcgtcgcggttgcggccgtcgccgtttccatcgtctgagggttccgcaatgcgccgttatctcttcgtttccgccgatacgctgcccgttgtcgcctatgccgacagcaaagacgcaatgcgcgcctatgtgcgcgacttgctcgggattccctacgggttcccgctgccccgtcacgctgtcgtttccatcgcctaatcactcacacacaaagggaaaacacacaatgaaaaccgtctttgatcgcgatatggtcgcgcacctttgggcgaataagtcgcaagataccgcgcgcgtttcgtccggcaatttttggttcactggcccgacgttgtatagctatggccggcacttcgtctgcgcgcaccacatgccggaagagtacaaccgcgacggccgcgcgctggcgctgttcaatgactcgcgttattccatgacgacgggccgccacatggatgcagcgtggcgcgcgctgccgggccgcgttgtgcgcgttgacgtgccgggcttggatgaaaacatggtgcgcgagttctcgcgattcggcacgggcgcagcggtcgcggccatcctcgcgaagatgcgccgcacggccgacaaggcggcgaatcctcgcattaagcccgacacgcgcggcgcgctgttctctgagttgcgcgatatgcgcgccgatgcgttgcaccttgcaaccgttgacgctgcgcggcgcgacctgagcgcggaacgtcgcaaggcggcccgggcgcaagttgccgaattgaaggcggccgacgttgacgcattcgcgacggaaggcaacgcggacaaggccggcgcggcggcctacgctttcgcgctgaaccgtggcgaatggatgcagaaaatgcgcgaagccgcagcgagcgcggaacgtctggcaaatcgtgcaatcggcgagtgcgacgcgggcaacgtcggcggcgcgctggactgcgcgcaacaggcggaacgctatgcggccggcgcgcgtgagctggcggaaaaggccgccgcgaaactgccgcgcgcgacgctgcgcgcactggccgcaatcaaggccggcacgaaatggcgcgcagacgtggaagcccgcgtgcgcgtgtcggaagtcgcggcggcccggatcgaatgggcggaaggcgaagcgctcgcgcgcgaagcgctcgccggccgtgagttctatttgattgaccgcgcgttgtctggcgacctgcgccgcgcgtttgaaaccttgcacggcgaagacggcgacagcgagcggcgcgcgttcgtggcgatgctggaaagcgagcgcaacgcatggcgcgagaaaaacgaagtgcaacaggcgcacgcgcagctagacgcggcgcgcgagctgttcgccgccggtaagttctcgcaagcgtgtgacgttgcgcgcagcgccgcgcacaagatgcgccgcaacttcgccggccgttccgacatggcggccaatgacgcactagacgcggcggaagcgctggcgaatgacgcggaagcccgcaagcccgaacagttcgccgccatgctggccgattggcgcgacgcgaagcccggcgcgcgcttcccgtctgagttgcacaacagcgaccgcgccgcgttcctgcgcctgagcccggacggccgccgcgtggaaacgtcgcaaggcgcggaagttcccgtgcgcgtgtgctcgcttatgtggcatttgatcggcgaacagcgcgcagcgggcgagccgcgcacgttcgcggccggttccgtcacgctcgggcatttctcactggacagcattgacgcggaaggcaacgtgcgcgccggctgtcatttcatccgctatagcgaattggccgacatcgccggccgcctttccttcaatccgcacaactaagggagcacacgccgtgcaactgcattcaatcaacacggaacagcggctttatgtcatgccggccggcgatggtttttcctgctacgggtttgacgtgttagaccgcaaggcgcgcgcggtcgccgcatggataagccgcgaagggttccagccgcgcattaacgacatttacgattttaagcgcgtcgccggcttcaatccgggcgagcccggaaccgctgagcacttcgccgcctgcgcggccatgatggaacgcggccggcaattcgcggcgcagaccggcaagcgctgcccggcggaacttgtgccggccttgatcggcttggaaggaaagcgcgtggagtgcgagcactacggcgagcgcgtgcggttctacgtcggccgttctaccggatggatgccgggccatctcatgattaagacgcgccgcagcactggcggcgagatgctgagcgcggacagcgtgcgcaatgtgcgggtgatcgcatgaacgcgcgcaagggtaagacgaagacgcgcgccgacttgctgcgcgaaaatctggaattgcgcgcgcagttggcgcatgtgtatcacttcgcaagcgcggagattcacaaggccggcgattctctcatgggctcgggtgtcctgttgcagttgcacgcgcttggcggccgtgagctgattaacccggtagtgatccgcgacgggctgagcgcggacacaatcgaagcgctgcgccgcgactttgtgcgcagctatcaaggcgcaacgctgttcaagcccaagggggcgacgccgtgaacgcgcgcacgatcctgcgccgccttgacgcgctcgcgcttgtgcaactggcggaacatgccgcgcggctcgccgtcgcgctggaacaggcggaagcgcgcgcatatgcggcggaagacgcggccgaatcgtggcgcgatgacttcctgagactatgcgaagagaccggacagcggccgggcatcacgcaagccggcgcgcttgtcgcgctgccgggcgacgtgcaaggcatcgcgcgcgagatgcgcgccactgccgcaaagcatcgcgcccgccatcgtcacggccgcgccgtggagctggaacaattcgccgcacggattgagggggcgcagtcatgacggaaccgtcattgcgggaaaagcgcgaaaccctgcgcgctaacatcctggccgacaccgtggcgcgcgtcgtgcgatggatcgcgtttgcggccatcgtgtgcggccttgtgttgccgctcgcatggggcgcactgcgcgcgcatggtttcgtgtctggcgctgtcgtgctggcgctatgcctcgccctatgctggcacgtcaagccgcaaggccgcagcgccgcagcgcaagcgcgggacatagcggcccggtatccaaggggcgattaaaccgcgcgcccccgcgcccccacgttctgccaactgcccggcctttgcgccgggctttttattgcgcgtgatcctgccgcgctaggccgcctgcccggccttcccttgtgcgcaccttgtcgcatggtgccgcgcgtgctcgcgcgccccttgccctagcgctgcgcgttttccttttgttcatggtcgccgcctgcccgctcgcccgggctcgggcgcgcttgcgtgtgcgccttgcatgggcggccgacctgcgcgcatggccgcatgggcgcatgggcgcatggccggattgctcgggcttttattcgtgcgcaccttgcctagcgcacgctgcgccgttctgcgcgcattgcatttatttccttttattcgcatggccgcatgcctgcgcgccccgtgtgcgtttattcgtgcgcccgtggacgggttaaagggatagccgctcggcgagtaaaaaggtacttccggcctgcgcgcgggcgtcgcggggggcgccgcccgtggacgggttaaagggatagccgctcggcgagtaaaaaggtacttccggcctgcgcgcgggcgtcgcggggcgctgacctcggtgctcgcgtaattttcggaattttcgcggtttcgtctcctttggacccccggacggcaggaaattcccgaattaattccccggaattgatttatttctttgtgacagtagtgacagtgacgtttttgggtactgtcacaggtcggccccccgtgcgaaagggctaaaaacaaggcgtttttgcgcgcgaatttactgcgaatttcggctcagtgacagtgtgacagtgacttcttttccttatacggagaaagagaaagcgtgccttccaagaaaactttctcgcgtatgaggaaatgtactgtcactactgtcactactgtcacaaattagggaaaaggtaggtagaacaagaagttaggttgtgacactgaagctgtgacagtaccttgccgacccgccgattgggccgatttaattggtagtgtcacaagatcgcgcaaaatttttgcgttcgtccatacggtctgaattttttccgtatgtgacagtaccaaaaaataggcaatttttaattcgagtgccgtgttgacttggacgcggcccgggttcaacatggcactgcggaaattcctccgcgcacgccgaattaaaggagcccgacatgggtagctacaagcacgtcgcctgccagtccaatgtgtccgcaatttccgacgcaatttcctcgctcgaagagctggggagcgagtgccgggaaatcgtcgacaacgccagcgagaatttgcagcagacctcgcgcatccagaccttcgaggaaacggcctcgacgctcgaaggaatttccgagccggatattcccgactgcatcgctgatttgccgatcaactacaacgagcagcgttcgacgaggaaggggcgcggcgagtcacgggccgttcggcgcgacaatgcgctcgctgtaatttccgccgctcgcgaggcggctgacgagtggatcaacactcgcaccggagagcacgaggacgccggcagcagcatcgacgatgacgaggaagcgcaggctgtcgtcgaattcgtcggcgaactggaaaacctcgaatcggacatcgagggctgcgaattcccgggcatgtacggatgactcggcggccgtacaccaagccgaagaaagatcgcgcgctgcggccgagtgaagtgcaggcgctcgcgcggtacgacggatggaacgacgcggcgctggttgcacggcagcaggagttgaagaagcggttgctcgatgacgcgcacgagctgcacatcatcaaactggcacgcaagcaactggcgttgcagcagaatccgatgacggtactcgctgaagcgctgcgcaaggaagggcacgaactcgatgcaccgagcttcgagcgagcgcgactcgaactagaccgcaaagactgaaagccgcgcaatgaaaaacccccgggtcgccccgggggtttctttttgcctgcaactcgcgacgtgttacagcgtgcccttcggtccttcgccgacacgcacgtcctcgacgttcgagccgttgtcgccggcaccggccggcaggtcgccgctctcgtagcgattggcgtcggtgttgctctcgtcgaccgtggcgttcgcttccatgccttgctgcttcgtcgcaccgtggaagtcgccggtctcgcgcacgaggaactgcgcgtcgccgtggatgttctgctcgaacacgtcgccgggcgaggtcagtgtcgcggcggtgctgccgtcccgctggtcgacgacttcgatgtccttgttgccgtgcatgtactcgactttgattcgggtggtcattgcggttctcctgctgcccgggattgggcgtttgtaggttataccttcagggatgtcagctcgatgaagtcgtcgatccacgcctgaaggttcggcttgacgacgacatccgggtgccgggaccaataccgcgcctgcttgccgttcgcgccgcgcgcccggccgacgtacacgaagcctttcgacgacaggaagttcgacagcttgggtccgtacggcacaccgatgctgctgtccatcgagatgtcgcggagccgaccgacgttgagcagcatcgagttgacttccgggtctttcgagtcggtgatgatttcttccagctcgtcctcgtcgtcgttgcgcgccatgtcgatcatgcgggccttggcgtcggtcatcggcgcatggccgtccgggtcgaactccgggtgcagcgggtaatcttccagccactcgcgaatcgcgcccgggtggttggcgatggcgttgaagatgtcgtcgtagtgatccgggtgcgcggcgcggaacttctcgatcatctgcttcgtctggaagtgggtcgagatgacgaagtagcgacggtcggcgtcgtagaccggcaacgcatcgctgtggttggtcaggatgatggtcgacgtgacgttcggcacgttgtacgagtcgcggtgcatgcgtcgaatcgaaaccacatcgttcgtgatgaagggcttcagcttgtccatcactgcgtagcgcgacgtgccgtggatgcgcgcttcttccagcaccacgaccttgcgcgactcgaagaacgctgtgtacttctcttcgagcgcctgagcgttgacggtctcgacgttgttgcgcgacatgatcgccatgagcatttcgcccacgaagcctttacctgcgccgtcgacgccctgcatcacgaccgcccaacggattttgcgatccatgcgcttgatcgtgtacgccagccacgagagcaggatttcgcgctcgcgttcgaccgggtacgaaatctcgaagtgccgcttcactgcttcgaccgcgcgcttggctttgccgctcagtttctccggtacgggaacgatgtcgtcagggttgaacttgttggcgtgcttttggccgtcccattcgacgattcgatccgcgccgggcaagtagacgtagccgctgacaacgggaatctggtacacgttcaacgcgagtgcggcggcctgctgctccggcaccgcttccatgttcgagcggtctttcttcgacagcagatggcggttgttgcgtgcgttgaagccgcgttcgctcagcgcgaggcggttgtccatgtagtagaactcttcctcggcgtcaacgtacaccacgtcgttgcaccaatgcggcatttccttgtagttgaagtccgagttcttgtagccttcattgatagccttgcgtacgaggtcgacacgcaccttgcgaccgctcagctccttgacgcgctcgatgatcgcaccagccagcaggtcgacttggtagtcgtgttccaacatccggccccacttcgtcgcaagcgaaccgagcagttcgacttcgctgccggtctccttgaccttgcgctggattttctcgaactgttctttcgagtgctcctgcctgtgttccttcgccattttgataagcgaagcggccgtggtgatgttgcggcccatgtcgtcatggaacgagttccacttgcgttcgagcacgtctgcatcgtagttgtgcgcgttctcggaccactcgtgccagagctgcaagccttcttcgttgccgtcgaattggtgatgcagcgccatgccgaccttcaaccactgttcgtagtcgtcggaacccggcacccattgcagcacttcgcgaagttgatcttcggtcaggttttccagcgggcgcttgtattccagcagcgcgttgtcgttctcgtcctcgttgttgctggactcgcgcggcgcgttgtgcttcttcaacgtccagccgcgacgctgcgcttcgagcttgaacaccgagaacaactcgtcgatgtgctccggcgtgatttccggcaggaagtccgcctcgactgtcagcggcgtcatgtccttgccggaagtccagcggtacggcttcttcgtgtccgggtgcgtgccgatgccgacgaactgttggccgtctgcgagcacttcaattgcttgctcgtggccgtccgcgtcgaggaacgtgatcttgcgcttctggaaaggcactgtcgtgcggtacacgagcaacgtcttgggcgcacgacctacgcgcgtcatcgtcttgccgatgatttcctgcgcgtgttccgacatgagagaggccatctcgtcgtcggtgatgtcgatgtcgacagcaggcgtgtgcttcgtatggaagccgatgttgccctgcttgtagttgccgttcgcccacttgcgaatcagcttttcgtccgcttggattttttgccacgccggctcagtcggacctttgcggccggctggaattggcagaattgagtatccgttttctagcagtcgcgcgccgtactttcgtagcacgctggtgatgggtcggccagccatgcgtcactccgaaatgtcgtcgccaacaaggtcatcgagattgaacccgatgctgcgattgaagtccttatgcagaatcgtcgccttgtcgcgcggcacaccaccgagtcgctgccaacgcgaaacagttgtttcgtgccagccgtacttcgtgcatagggcgttgagttgaccagtcggcggatcgaggatgagagcaatgcgtcgaagaaggtagcggacgcgcgcttcggcgctatccagtgaatcaagagtcgggtctcggcgcataaatcctcgcgaaagtaggtgttttcaaggggccgctaagtggctttgcgtgcctattgacttagcatggggacgggcgcatagtgcgctcgccgggcaggaattgcaatccacccgtcaatcccaaccaaccaacctagctaggagtaacccgatgtcgaaactcaacgcgaagtccctcgccgaagcaatcgccgctgcgctcgcccccgttctggtcgccgcgttcggcggtgccgccagcaacgacgccgacgatggcgacggcgaagaagaagctgcaccgaagaagggtcgcggccgtccggccggcagcaccaagaccaagaccgaaaccaagccggccgcgaagggcaagggcaaggcgaaggacgaggaagaggaagaagaggacgacgacggcctcggcgacgacggcgacgacgacctcggcctcggcgacgaggaagaagaagtcacgcaggaagatgtcgtcaacgccttcaaggcgctgaaggccagcaagggcatcgacaagtgccgcgaagtgctcgcgaagctcgacgagtccaacgtgctgaacatcccgccgaagaagtacgccgaagcgctgaaggaaatcaaccgcgccggctcgaagaagtaattcggccagcacgtcactcgaaacgcccgggttcgctcgggcgtttctttccgagagagcccatgaagccacgccgcaacaaactcgcaaaggcagtcgaagaaacggtgcgcgcacacgcccgattcgcgccttcatctgcgcaccgaattcacgattgcccggcgagcctgctgctcaacgagcaagagcccgaccgcgagatttgggaagccgcagagggtactgttgcacaccacgttgcggaaatttgcgcacgcgagcgccgtgatccagaagagtttctaggaatgacgttcgatagcggcgacctcgacgccgactacgacgaagagcttcattcctcgaaaggcttcgccatcaccgtcgacgacgagatggtgcaaggcgtcggggaatacctcgaccgcatcatgaccctgcccggcgaccactacgtcgaaacgcgagtcaacatctccccgtggtgcccgatccccgatcaattcggcacatgcgaccacgcggcagcaacgcacaagaagctcatcatcaccgacttgaaatacggccgagtgcaagtcgacgcaccgcagaacaagcagctcgtgatgtacgcactcggcttcatcaacgaatacgattggatgtacgacttcgatgaagtcatcatccgcatcgcgcaaccacgactcgatcacttcgatgtgtggatcaccagcaaggccgaactgcttgctatcggcgagaagatcaaggaacgctttgcgctggcactgaagcccaatccgccgttcggtccgagcgagaaggcgtgccgtttctgcaaggtcaactacaagtgcaaggcgaaccacgacttcctgtaccacgagcggattatgctgctcgacgaggacgatgagttcgttgaacccgacctcatgctcatgagcgacgaagaactggcggccctgtggctgcgcaagggcatgtacgaaagccgcatgcgcgccgttgaggactatctgcacaagaaggtcgccgatggtgacttcgtgccgggcttgaaaaccgttgcaggccgcagctcgcgctacttcaccagcgaactcgacgcggagctgctgctcgcggaagccggcgtgcctgagtcgaagatgtactccaaacccgaattcgtttcgcctgcgcaggctgaaaagctggtgcgcggcgaggcgaaaaagaaattgcaggacttcatcaaatcgaagcccggcaaaccgtgtctggtctccgcagacgacaagcggaaagacctgactgtgcagtcgctcgaattgctcgacgactgattccctgttgtacgaatgcgcgaaagcgaactacgaacgtcgaatgacgaaggagaaatcgaaatggcgaagaagaaagttggtgatctggtcgacaagggcaacggccgctacttgctgaagaacgtgcggctcagcttcccgtacttgttcgagcccgacgagcaggagaacgacgacggacagaagaagaagtcctatcgcgtcacgctcctgctgccgaaggccacgcacaagctggtggcgcagaagctcaaccgactcatctccgagatgtgcgaggaagagtacggcaacgccaagctggcggctgaccgcaagttcttgcgcgacggcgacgagtcggatgtcgacgaccatcacggctgctggacggtgacggtgcgcgagactcgcaagccgatcctcgtcgaccgcgaccgtcaacccacggaagaggacgacgagctgctgtacagcggcgcgtgggccaacgtggtgatccggccgtgggcgcagaacggcaagtcgatgaagaagaagaacaagtacggcaagcgtatcaatgccggcttcgacatcgtgcagttcgtcgatcacgacgacaacctcgcgggcaatgctcgcccggatgtcgacgaggttctggacgagttggacgacgacttcagcgacgacgataccgagaccagctcccgcagcagcaagtcgtcgaagagcaagagcaagccgaagggccgctcgcgcgacgatgacgacgatgacgacggcgacgatgacgacgacgacatcggcctgtaagccccgggccatcgtgtagtaccttcggtcgcccgggcactccccggtcggccgtttttcagggaaacggtatggacaagctgcatcacgacttcgagaccttcagcaagtgcgacctgaagaagcacggtctggcgcgatacgctcgcgacaagtcgaccgaagtgctgttcctgtggttcgcgttcaacgacgaagagcccgaagtgtggttccccgcgactgagccgatgccgaagcgcttgcgtcgcgcgctcacagacccgaacgtgcagaagtgcgcgcacaacgctcagttcgagcgcgccatctggaagcacgtcatcggcgtcgacattcccgtggagcagttctattgctcgatggcacacgccttctggctgtcgttgcccggcaacctcgacgaactctccggcgtgctgcgcctcggcgaaaacgcgaagatgaaagagggcaagtcccttgtgaagttcttctgcggcccgcgcaagccgaccaagaccaagcagtatctccgcaataccgaaaagaccgacccggcgaagtgggcgacgttcgtcgagtacggtcgccgcgacgtaatcgcagagcgtgcagccgggcgcaagctgtcgttgttcccgatgagcccgttcgagcaaaacctctggtacatcgaccagcacatcaacgagcgcggtattccgttcgacaaggaattcgtgttgaccgcgctgcgcgtcatcgcgaaggagaaaaagcgtctggtcggcgagatggcgcgcatcactggcctgagcaacccgagcagtggcacgcagttgctcccgtggctgcgcgaacgaggctacccgttcaccaatctcaaatccgcttcgatcaagaaggcgcgcgaggattgggactggaacatgactgacgatgcgaacgatgtactcgcattgcatgccgaagcggcgcgttcgtccgtcacgaagttgcagaagatgctcgacatcgaagtcgacggcgttctctgctacacgatgcagttcgcaggcgcagggcgtacggcacgttgggccgggcgcgcagtgcaggtgcaaaatttgccccgccccctgcgcgaactagaagaacaaggggcgctgctggctgtgcgcgatgcgattgcccgggaggacatcgagttcattcgcctgctcgtgtcgtcgccgatgggtgcgattgcatcgtgtatccgcaccgcgatcaaagcaccgcccggctacgaatatgcaacttgcgacttggcctcaattgagtccgtcgtcattgcatggctgtcaggctgcgacaagctcattgaggtctttcagaaaaacctcgacgtgtacaaagtgttcgcgtcgaagatgtacaaggtcgattacgagaaggtcgagaagtggatgcgtcaacacgcgaaacccggcgtgctcggtgcaggcttccgcctcagcggcggcatggaactcggcgagtacccggaagtcatcaagaccggcttgtggggctacgcggagaacatgggtatcgagatgtcgcagaaggacgcctcggctgtcgtgaagttcttccgcgaggaatacaccgaaatcgttgagctgtggtacgagctggaacgcgccgtcgcaaaggtgatgaacacgaaggagccggtgcgcgttggaccgatcctcatggacgtgaaggggccattcctgcgcatgcgtctgccgtccggccgtcacctgcactacctgcgcccgcagatggtctggaagaagatcaaggtcggcatcgacaagaaaaccggcaagccgaagtacaagtcgaagaagggcttcacgtacgaaggctacaacacgaagaagaagtggacgcgcatcgactcgcacggcggcaagatcgtcgagaacttggtgcaggctatcgcccgcgagctattggccgccggtctcgtcaaggcatggaaggctgggctcgatgtgcgcatgcacgttcacgacgaaatcgttgcactcgtcaagcgtaagctcgctgacatctcggcgtcgacgctcgaagagcagatgatcgagaagccgaagtggtggggtcacgacgttccgattcgcgcaaaggctgacgtggtggagtgctatcagaaatgacgttcatctcagactggacagatgtcattctcggcaagccgatgcgcggcgatattttgtcgaccgacaagcatcgcctcgaaaaagaagtcgagaagaagtggtgcgacacggcgaagcgtttcggctggaaggcgtacaagttctcgtcgccgggtaacagcagcgttcccgaccgcatgttcatccgcaacggctttgtgttcttcatcgagttcaagcgccccggcggcgcggctacgccgaatcaggtcgaagagcacaaggagatgcgagaaaaaggcatgctggtgtgggtgatcgactacttcgataaagaattcgcggagtggatttttgaatgaaagaactcctgaagcgttccgacctcgatgagtttcaagtagctgccggcctgttcctcgaacaagtcggcagttgcgcgttgtggatcgacatgggcctcggcaaaaccatcgtcgtgctcacgcacgtttcggacaaggtgttttccggggaatggagccgcgtgctggtgatcgggccgccgttggttatctccgatacttggtcgactgaagtgaagagctgggagcacacccgctggctcgactatcaggaactcgacggcgacagcgagcatatgcgcatgcagttgcagcgtccgtgcgaagtagacggcatctcggtacataagctgggccgcctcgctgctctgttcaagcggggggacaccgtgccgtgggacgcgattgtgttcgacgagtcgagtatgttccgcaacaagacctcgaagcgctggaagtacggcgttcgcttgacgtggggccagccgaacgacgtaatccagctcacaggtacgccgagcccgaatggcttgcatcaagtctggtcgcagattgcaatgatcgacggcggcgaacggttggagctgacgtacaagaaattcctgttccgctacttcaaacaggagttcatgggccgcaaggtactgccgaaagcgaacacgcttgcgcgcatcacgaagcgcctgagcgacatcgtgtacacgttgcgcgaagaggattacgtcaagttgccgccgctgcgctctacgcctgtgccgatcatcctgccgccggatgtgatggctcgctatcaggaattcgagcgtacgtctgtgctgcattggggcaaggaaaacgatccgaaaattcgcgcactgtcggaaggcgcgctgtacggcaaactgttgcagttcgcgtgcggtcgcgtttacacgggcgagttggacaagagctttgtcgacgtgcatgacaagaagatcgagcgcctgaaagaaatcgttgagttcagcgacggctctccgatcctcgttgctcggacgtggcagcactctcgtgaccgactacgcgatgagttcccgggcatccgttcgatcaagaccaagcgcgacatcgacgcatggaatgccggcgacattctgcttgccgagacgcatccggcaagcatcggtcacggcacgaacatccagaagggcggcaacaacttcatctggtacgaccacacacctgacctcgaactctacatgcagttgcgaaaacgactgcaccgacgcggacaaacgcgaagccacgtcaacatgatgcacctgactgcaataggcactatcgaagaggatttgacacgagagctggtcaagaaagaaattacccaagacgccctgagagaacccatgcggcgacgagtcgcagacgtacagagagaactagccaatggccgcacctaagatcgactacgaagaagagtttttcgacggcatgaccgtgccgcgtctggcgcagttgtttcgcctcgaccgccgcaccgtcaccgagaagttgcgcccgctgcgcccgactggcgaccgtcgcggcgcaccgacgtactacatcgtcgacgctgcaccctaccttgtggagcccatcgtcgacatcgccaagtaccttgcggaagtcggtcccggcgacctgcctgcaccgctgcaagcgcaatactggaatgcgcagaacagcaagttgaagtacaaggagcagtcgggcgatttgtggcgcacgcagcaggttctcgaagtgctcgtgggcgtatttcgttcgctcacgcaatcgctgcgcctgctcgccgaccgcatcgaggcgcagacgggcctcacatcggagcagcgcgcgatcatcgaaaaggaaatctccgacaaggccatcgacatgctgcgcaagcggctcgtcgacgacttcgagatttacgtcggcatcaaggataaggaacagctcgccgacatcaaactcgacgacatcggtctggacgaagaggacgacgaca

SEQ ID NO: 12 - DNA, 55251 bp, unidentified
  source 1..55251: mol_type = genomic DNA
gctaacgacatgacgacgattaccgcatacgcatacaatgccgcgcttcattgcccgcgctgcgcgttccgatatttccgcgtcgatcctgcgaaggtgccgccgggcgcggatgcaatggaaggcgcacgcgaccgcgaagggaacgcgcccgcgccgctgttttcgacagacgcgaacgcggatggatattgcgacacttgcggcatggcgtacggcgacgctgagcccgtggcgcaattgctgagcgtggaagcatggcgcgagcccgaaggctggacgtggaataactggcacaagcgcggcatggtgccgcttgcatggtgcgacctgaagccgcgcgcgctgctgcgcaaactgcgcgagcatggcggcgcgtaccctgcgccgggcttgtgcgcggtcgaggatgacgggcataacgtcgttatcgtcatgcgtggtacgcgcgaacctatcgcggccattgcctacggcgaggcttgcgcatgacggaaccgacactaaacgaaaaggcgcaaatcctgcgcgctggcattctcgccgatagcgtgacgcgcgcggttcgctggtgctgtttcgctgccattgtttgcgcgggcgcgttgccgctggcatggggagcgttccgggcgcatggcatcgttagcgggctcgccgtgctggcgctggtgctggcgctatgctggcacgtcaagccgcacgggcgcagcctagcggcgcaagcgcgcgagattgaagcccggttcaagccgcacgattaaaaacgcgctaggcgcgttccctgcatcgcctaccctgagcccggccgcgtgccgggctttttattgcctgcgcgtctaggcgcgttctagtggcattgccgggcgcacgtctgcccggccttccgtatccctgccctgagcccgtgcccgcatcgcctgcgcccgggctttttctttttcccgctgcccggccttgcccgggctcgcatgcgtgccggcctgcccgctgcccggccttgcatggtggcgggcttatccgctgcccggccttgcatgcgtgcggcatggctgcccggatgcggcaacgtggaattaatgcagcgctgcgccgcataggtgcgcgcgtgcggcctttccgaatttatttattgcatcgcatgcccgcatgcgtgcgcgccgcgctgcgcgcgttgtggcgcggcaggaagggataaagggatagcggctaggcgagtaaaaaggtacttccggccctgctgcgagcgtcgcggggggcgctgacctcggtgctcgcgcatttttcggaattttcgcggtttcgtctcctttggacccccgggcggccccgaatttccgaatttattccccgaataaacgcgaatttcctgtgacagtagtgacagtgacgtttttgggtactgtcacaaattcggccccccaagaaatccgctcaaatcaacgatttacgggcgcgaatttactgcgagtttaggctcagtgacactgtgacagtgacttccaatcctttacggcggaaagaaaagttctgcctgccaagaaaaaattctcgcgtatgagagaaggtactgtcactactgtcactactgtcacaagatagggaaaaaggtatgtagatcaagcacttgaatttgtgacagtaccttgtgacagtgaccgatttgcgcctcggagagcatggaaaaccgggtactgtcacaagaatcggcctttttccgaatttccgcccatacggttgcaattttttccgtatgtgacagtgaaaagaattcggaattaatttaatcggagccgctgcggggcgtcgtgcggaaattcggaaattccgggcaataaaaagccccgggggatgagcccggggccggcactgcggaaattccgccgaattaaatcgcgctcttcggcgctccatcgcctacacgcacgtcctcgacgttcgagccgttgtcgcccgcgcccggcggaagcggatcgctctcgtagcggttcgcgtcggtgttgttttcgtcgacggtcgcgttcggcaccatgccctgcggcttcgacgcgccgaagaagtcgccggtctcgcgcgctgtgacctgcaagtcaccgtgcatcgtgatttcgaccgagcggccgggtgcatcgagcactgcatgcaccacgccgttgccgtcgaccaactcgaccgccttgttgccgttgacgtgcgtgaacttcacggtagtcgtcatgtcgtttctcctgtgctcgggattgagcgtcttcgatcatacgctcgcaggcatgaaaaagcccggttgcccgggcttcttcgatcacaccttcagcgacgtgatttctatgtagtcgtcgatccacgcttgaaggttcggccgcaccaccacgtcaggcgagcgtgaccaataccgggcctgctttccgttcgcgccgcgcgcgcggcccacgtacacgaagcccttcgaggtcaggaagttcgacagcttcggcccgtacggcacaccgacgctgttgtccatcgccatgtcgcgcagcttgccgacgttgagcagcaggtggctcacttccgggtcgcgcgactccgcgatcatctcttcgatttcgtcttcgtcgtcgccgcgcgcgaggtcgatcatgcgcgacttcgcatcggtcatgggcgcatggccgtccgggtcgaactcgggatgcagcgggtagtcttccagccactcgcggatcgcacccgggtgataggcgattgcgttgaagatgtcgtcgtagtgatccgggtggcgctcgcggaacttctcgatcatctgcttcgtctggaagtgcgtcgagatgacgaagtagcggcggtcagcgtcgtagaccggcagcgcgtcgctgtggttggtcaggatgatggtcgaggtcacattcggcacgttgtacgagtcgcggtgcatgcggcgaatcgaaaccacgtcgttcgtgatgaagggcttcagcttatccatcaccgcgtagcgcgacgtgccgtggatgcgcgcttcttccagcaccacgaccttgcgcgactcgaagaacgacgtgtacttctcttcgagcgcctgtgcgttcacggtctcgacgttgttgcgcgacatgatcgccatgagcatttcgccgacgaagcccttgcctgcgccgtccacgccctgcatcacgaccgcccaacggattttcctgtccatgcgcttgatcgtgtacgccagccacgacagcaggatttcgcgctcgcgttcgaccgggtacgaaatctcgaagtggcgcttcaccgcctcgaccgcgcgccgggccttgctggtcaacttgtccggcaccggcacgatgtcctcggcgttgaacttgttcgcgtgcttctggccgtcccactcgacgatgcggtctgcgcccggcaggtagacgtagccgctgacgacgggaatctggtacacgttcaacgcgagcgcggcggcctgctgctcaggcacggcttccatgttcgcgcggtccttcttcgtcagcaggaagcggttgttgcgtgcgttgaatgcgcgctcgctcagtgcgagacggctgtccatgtagtagaactcttcctcggcgtcgacgtacaccacgtcgttgcaccaatgcggcagctccttgtagttgaagtcggaattgcggaagccttcgttgatcgccttgcggatcatcgcgatgggaaccttcttccccagctccgcaacgcgctccttgatcgcgccggccaacagctcgacttggaactcgttctccaacatgcggccccacttcgccgcgagcgggccaagcagctccatctccgaagtcgtctcggcgaccttgcgcttgatcttctcgaactgctcctgcgagtgctcctgccgatgctccttcgccatcttgataagcgaggcggcggtcgtcaggttgcgacccatgtcgtcgtggaacgagttccacttgaactccaactcgtccgggtcgtagttgtgcgcgggctcggaccactcgtgccaaagctgcaagccttcttcgttgccgtcgaattggtgatgcagcgccatgccgaccttcaaccactgctcgtagtcgtcggcacccggcacccattgcagcacttcgcggagctggtcttcggtcaggttttccagcgggcgcttgtattccagcagcgcgttgtcgttctcgtcgtcgctgctgcgcgattcggtcggcgcgttgtgcttcttcaacgtccagccgcgacgctgcgcttcgagcttgaacaccgagaacagttcgtcgatgtgctcggtcgtgatttccggcagcatgtcggccggcacgctcagcgggttcagctccttgcccgaagtccacttgtacggcttcttggtgtcggggtggatgccgatgccgacgaactgttggccgtccgcgagcacttcgatggcctgctcatgaccttcggtgtcgaggaacgtgatcttgcgcttctggaacggaatgtcggtgcgatatacgagcaacgtcttcggcgcacggccgactcgcgtcatcgtcttgccgatgatttcttccgtgtgctcagccatgagcgcggccatttcgtcatcggtgatgtcgatgtcgaccgcaggcgtgtgcttcgtgtggaagccgatgttgccctgcttgtagttgccattcgcccacttgcgaatctgcttctcgtccgcgcggattttctgccactgcggttcgattgggcctttccttcctgccgggatcggcaagatggagtacccgttttccagcaattgcgcgccgtacttacggagcacgctggtgatcggtcgtccagcagccataggtcactccgcgatgtcgtcgctaacaaggtcttcgaggttgaagccgatcttgcggttgaaatccttgtgcaagatggtcgccttgtcgcgcggcacaccgccgaggcgctgccaacgcgagacagtggtctcgtgccagttgtacttctcgcaaattgcgttgagccgaccgtacggcgggtcgagcatgagggcgatgcgccgaagcagatagcgcactcgcgcgtctgcgctgtccagtgaatcaagagtagggtctcggcgcatgaattcctcgcagacgttgggatttaaggggtctgctaagtcggtgagcacgcctattgacttagcatcgggacaggcgcatagtgcgctcgccgggcaggaattgcaatccacccgtcactcccgaaaccaacctagctaggagatacaaccgatgtcgaagatcaacgcgaagaagctcgccgaagccatcaccctcatcatcgaagcagtcggcggcggtgccgccaacgagtccgaggatgcgggcggcgaagaggaagcgccgaagaagggtcgcggccgtccggccggcagcaccaacaaggccaaggccgagaccaagcccgccgccaagggcaaggccaaggcgaaggacgaggacgaggacgaggacgacggtctcggcgacgacgacgatgccggcgacgacgatgacgacctcggtctcggcggcgacgacgaagaagtgacgcaggaagatgtcgtcaatgcgttcaaggcgctgaaggcgagcaagggcatcgacaagtgccgcgaagtgctcgccaagctggacgagagcaacgtgctcaacatcccgccgaagaagtacgccgaggcgctgaaggaaatcaaccgcgccgcgtcgaagaagtaactcggcctgcacgtcacacgaaacgcccgggttcgctcgggcgtttctttcggagaggaacacatgcccggttcgcacgcccgcttcgcaccatcgtcggcgcatcgcatctacgattgcccggcgagcctgttgctcaacgagaacgagcccgaccgcgaaatctacgaagcggccgagggcaccgttgcacaccacatcgcggaaatctgcgcacgcgcgcgccgcgagccggaagagtttctaggaatgacgttcgacagcggcgacctcgacgccgactacgacgaagagcagcattcctcgaaaggcttcgcaatcaccgtcgacgacgagatggtgcagggagtcggggcgtacctcgaccgcatcatgggcctgccgggcgaccactacgtcgagacgcgcgtcaacatctccccgtggtgcccgatccccgatcaattcggcacctgcgaccacgcagccgcgtcgcacaagaagctcatcatcaccgacctgaagtacggccgcgtgcaggtcgatgcgccgcagaacaagcagctcgtgatgtacgcgctcggcttcatcaacgagtacgactggctgtacgacttcgatgaggtcatcatccgcattgcgcaaccgcgcctcgatcacttcgacgtgtggatcaccagcaaggccgaactgctcgctatcggcgagaagatcaaagagcgcttcgcgcttgcgttgaagccgaatccgccgttcggcccgagcgagaaggcgtgccgcttctgcaaggtcaacttcaagtgccgcgcgaaccacgacttcctgtaccacgagcgcatcatgctgctcgatgacgacgacgagttcgtcgagcctgacctcatgctcatgagcgacgacgaaatcgctgcgctgtggctgcgcaagggcatgtacgagaaccgcatgcgcgcggtcgaagactacctgcacaagaaggtcgcggacggcgacttcgtgccgggcctgaagaccgtggcgggccgcagctcgcgctacttcaccagcgaaatcgacgccgagctgctgctgctggaagccggcgtgcccgagtctaagctgtactccaaacccgaattcgtgtcgcctgcgcaggctgaaaagctggtgcgcggcgaggcgaagaagaaattgcaggacttcatcaagtcgaagcccggcaaaccctgtctggtctcttccgacgacaaacggaaagacctgaccgtccagtcgctcgaactgctcgacgactgacgcaaccgttgtacgaatgcgcgaaagcgaactacgaacgtcgaatgacgaaggagaaatcgaaatggcgaagaagaaagttggtgatctggtcgacaagggcaatgggcgttttctgctgaagaacgtgcgcctgagcttcccgtacttgttcgagcccgacgagcaggaagacgacaacggcaacaagaagaagtcgtaccgcgtcaccctgctgctcccgaaggcgacgcacaagcccgtcgcgcagaagctctcccgtctcatctccgagatgtgcgaggaagagtacggcaacccgaagctggcggccgaccgcaagttcctgcgcgatggtgacgagtcggatgtcgaagatcatcacggctgctggacggtgacggttcgcgagacccggaagccgatcctcgtcgaccgtgatcgtcagcccaccgaggaagacgacgagctgctgtacagcggcgcgtgggccaacgtggtgatccgcccgtgggctcagaacggcaagtccatgaagaagaagaacaagtacggcaagcgcatcaatgccggcttcgacatcgtgcagttcgtcgaccacgacgacaacctcgcgggcaacgctcgcccggatgtcgacgaggttctggatgagctggacgacgacttcgcggatgacgacgacaacagcaccagccgcagcaagtccaagagcaagtcgaagggtcgttctcgcgacgaggacgatgacgacgacgggctcggcgacgacgatgacgacgaccgcagctcgcgccgcagccgtccgtcgaagagcaagaccagcagcaagagccgtcgctcgcgcgacgacgatgacgatgacggcgacgaggacgatgacgacctcggcatctaaaatcgggcatcggtaagcggtacctacggtcgcccgggcactccccgggcggctgtttttcagggatacggtatggacaagctgcatcacgacttcgagaccttcagcaagtgcgacctgaagaagcacggcttggcgcgctatgctcgcgacaagtcgaccgaagtgctgttcctgtggtacgcattcaacgacgaggaacccgaagtgtggttccccgcgacggagccgatgccgaagcgcctgcgccgcgcgctcaaagacccgaacgtgcagaagtgcgcgcacaacgctcagttcgagcgcgcgatttggctgcacgtcctcggcatcgacatcccggtcgagcagttctattgctcgatggcgcacgcattctggctctcgctgcccggcaacctcgacgaactctcgggcgtgcttcgcctcggcgagaacgcgaagatgaaggaaggcaagtcgctcgtgaagttcttctgcgggccgcgcaagccgacgaagaccaagcagtacacgcgcaacaccgcgcagaccgatccggcgaagtggaagacgttcgtcgagtacggccgccgcgacgtgatcgccgagcgcgcggcaggtcgcaagctctcgctcttcccgatgagcgatttcgagcgcaacctgtggtacatcgaccagcacatcaacgaacgcggcattccgttcgacaaggaattcgtcgagaccgcgctgcgcgtcatcgcgaaggagaagaagcgcctgctgggcgagatgagccgcatcaccggcctgagcaatcccggcagcggcgcacagttgctcccgtggctgcgcgagcgcggctacccgttcaccaacctcaaatccgcctcgatcaagaaggcacgcgaggattgggactggaacatgaccgatgaggcgaacgcggttctcgccttgcacgcggaagcggcgcgttcgtctgtcacgaagttgcagaagatgctcgacatcgaagtcgacggagtgctgtgctacacgatgcagttcgcaggcgcggggcgcacggcgcgctgggccggtcgcgcagtgcaggtgcaaaatttgccccgccccctccgcgaactagaagagcaaggggcactgctcatggcgcgcgatgcgatcatgcgcgaagacatcgagttccttcgcctgctggtgtcgtcgccgatgggcgcgattgcatcgtgcatccgcaccgcgatcaaagcgccgcccggctacgagtatgcaacgtgcgacttggcctcgattgagtccgtcgtcattgcatggctgtcgggctgcgacaagttgatcgaggtctttcagaagaacctcgacgtgtacaaggtgttcgcgtcgaagatgtacaaggtcgactacgagcaggtcgagaagtggatgcgtcaacacgcgaagcccggcgtgctcggcgcaggcttccgcctcagcggcggcatggagttgggcgagtacccggaagtcatcaagaccggcctgtggggctacgcggagaacatgggcatcgagatgtcgcagaaggatgctgcggccgtcgtgaaattcttccgcgaggaatacaccgaaatcgtcgagctgtggtacgagctggaacgcgccgtcgcgaaggtgatgaacacgaaggagccggtgcgcgttggtccgatcctcatggacgtgaagggaccgttcctgcgcatgcgtctgccgtccggtcgctacctgcactacctgcggccgaagatgatctggaagaagatcaaggtcggcatcgacaagaagaccggcaagccgaaatacaagtcgaagaagggcttcacctacgaaggctacaacacgaagaagaagtggacgcgcatcgactcgcacggcggcaagatcgtcgagaacttggtgcaggcaatcgcacgcgagctgctggccgccggtctgctgcgcgcttggaaggccgggctcgatgtgcgcatgcacgttcacgacgaaatcgttgcgctggtcaagcgcaagctgtcggacatctcggccgcgacgctcgaagagcagatggtcaagaagccgaagtggtggggcgaagacgttccgatccgtgcgaaggctgacgtagtggagtgctatcagaaatgagctggctgaccgattggcgcaacgtaatcaacggcaagccgccgcgcggcgacatcctgccgaccgacaagcatcgcgtcgaaaaggacgtggagcagaagtggtgcgccgttgcgaagcggcacggatggaaggcatacaagttctcgtcgcccggcaacagcagcgttcccgaccgcatgttcatccgcaacggcttcgtcttcttcatcgagttcaagcgccccggcggcaaggcaaccgacaatcaactcgaagagcacaaggagctgcggcgcaagggcatgatcgtgtgggtcatcgactacttcgataaagaattcgccgagtggatttttgagtgaaacaactactgaagcgctccgacctcgacgagtttcaaatcgctgccggcctgttcctcgaacgggtcggcagttgcgcgttgtggatcgacatgggcctcggcaagaccgtggtcgtgctcacgcatgtttcggacaaggtgttctccggcgagtggagccgcgtgctggtcgtaggcccgccgctggtcatctccgatacgtggtcgaccgaggtcaagaattgggagcacacccgcttcctcgactatcaggaactcgacggcgacagcgagcacatgcgcatgcagttgcagcggccgtgcgaggtcgacggcatctcggtgcataaactcgggcgtctcgcggcgctgttcaagcgaggcgacacggtgccgtgggacgcggttgtgttcgacgagtcgagcatgttccgcaacaagtcgtcgaagcgctggaagtacggcgtgcgcctgacgtggggccagccgaacgacgtgatcgagctgacaggtacgccgagcccgaacggcctgcatcaagtctggtcgcagattgcgatgatcgacggcggcgagcggctgggcttgacgtacaagaagttcctgtcccgctggttcaagcaggagttcatgggccgcaaagtgattccgaagtcgcacgcgatggcgtcgatcacgaagaagctgagcgacatcgtgtacaccttgcgcgaagaggattacgtcaagttgccgccgctccgctctacgcctgtgccgatcatcctgccgccggatgtgatggctcgctatcaggaattcgagcgcacgtctgtgctgaagtggggcgaagagcaagacccggcagtgcgtgctctatcggaaggcgcgctgtacggaaagctgttgcaatttgcgtgcggtcgcatctatacggattcagagacgaaagagttcgtcgacatacacgacaagaagatcgagcgcctgaaggaaatcgtcgagttcagcgacggctcgccgatcctcgtggcacgtacgtggcagcactcgcgtgatcggctgcgcgatgagttcccgggcatccgctcgttgaagacgaagcgcgacctcgacgcatggaacgcgggcgacatcgagatagccgagacacaccctgcgagcatcggtcacggcacgaacatccagaagggcggcaacaacctcatctggtacgaccacacgcccgacctcgaactctacatgcagttgcgcaaacgactgcaccgacgcggccagacccgaagccacgtcaacatgatgcacctgacagcagtaggcactatcgaagaggatttgacacgcgagctggtcaagaaagaaattacccaagacgccctgagagaacccatgcggcgacgagtcgcagacgtacagagagaactagccaatggccgcacctaagatcgactacgaagaagagtttttcgacggcatgaccgtgccgcgtctggcgcagttgttccgcctcgaccgccgcactgttaccgagaagctgcgtccgctgcgaccgaccggcgaccggcgcggcgcaccgacgtatcacatcgtcgacgctgcaccgtacctcgtggagcccatcgtcgacatcgccaagtacctcgcggaagtcggccccggcgacctgcccgcaccgctgcaagcgcagtattggaacgcgcagaacagcaagttgaagtacaaggaacagtcgggcgacttgtggcgcacgcaacaggtgctcgaagtgctgaccggcgtgttccgctcgctcacgcaatcgcttcgcctgctggccgaccgcatcgaagcgcagaccgggctcacgccggagcagcgcgcgatcatcgagcgcgaagtgtcagacaaggccatcgacatgctgcgcaagcgccttgtcgaagacttcgagatttacgtcggcatcaaggacaaggaacagctcgccgacatcaagctcgacgacatcggcctcgacgaagaggacgaagaagatgtctgacggcagctttttcaacgacctcggcgagctggtcacgttcgttgccgatagcgttctggttccgccggagcgcttgaccgtttctcaggccgcagcaaagtaccgctacctcgacaacgaaggctcgttcgtcggcgagtgggacaacaacgaaacgccgtacctcgtcgagccgatggacgtgctcacgagtcgcgagttcgagtcgtgcatcttcatcggcccggcgcagggcggcaagaccgaaatcatcctcaattggatcgcatacaccgcgaagtgcgacccggccgacttcttcctcatccagaccgcgcgcgacaccgcacgcgacttctcgtatcgccgcatcgacaagatgcaccgcgacagcaaggagctgggcgcgatgctgcgtccgggcagcgacaacgacaacatcttcgacaagttctaccgcaacggcatgatgctgacgctgggctggccgacgatcaaccagctctcaggcaagccggtgccgcgcgtcgcgctgaccgactatgaccgcatgccgcaggacgtggagaagaacggcccgccgttcccgctcgctcgtaagcgtacgacgaccttcggctcgttcggcatgacgctggccgagtcgtcgccgtcgttcgacgtgaaagacccgaaatggaaggcaccgcacccggactcgcatatgttcccgccgtgcgatgggatcggcggcctgtacaacgaaggcgaccgccgttgcttctactggcagtgccctcactgcggcgagtggtttgagccgaagttctcgctgctgaagtgggacatcaagaaccccgacccgttcgaggctgcgatgtcgacgatgatggcgtgcccgcgtaacggttgcgtcatcgagccgaagcacaagtacgagatgaatcgacgcggcgtgtggctgcgagaaggccagcgtattgatcgcgacggcaacaagctcggcgtcggcgttcgctcacgtagcgcatcgttctggctgaaaggcccggcggcgcgcttcattacatggcagaccctcgtcgagcgattcctgcttgcgcaccagacgctcgaacgcacgggcgaaaccaaggcgctgaaggccacgatcaacaccgatcaaggcgaagcgttctggccgctcaacgcgaaggactcgaaccgcctgccggaagacctgcaatcgaaggcgatccagtgggccgacaagaaggtgccgtacggcgtgcgcttcctgctcgggactgtcgacgtgcagaagagccgcttcgtcgtgcaggtcttcggcgtcggcccgagcgataacggcgtcaacttcgacctgtacctaatcgaccgattcgacattcagaagtcgaagcgcaaggacgaggctggcgacacactatgggtcaagccgtatgccgtgcaggaagattgggacttgattaccgagcaggtcgtcgagaaggaatacgagctggaagacggcagtggcttcatgtcgatcaagatgaccggcatcgactccggcggtaagtcaggctcgacgacgcgcgcatacaactactggcgctcgatgcgcgacaacggcaacggcggtcgcgtgctgctcatcaagggcgagccgaagctcggtgcgccgcgtgccgaaatcgacttccccgactcggatcgcaaggatcgttcggccggtgcgcgcggtgaaatcccggtgctgttcctcaactcgaacgtgctgaaggacatgctgctcggcatggtcgactacgacgagaagacgacgctcggcggcaggcacttcacgaacaagtggacgccggaagttgtgtacgccgaactcactgtcgagttccgcgacgaccgtggtcgttggcagaatccggctaagcgacgcaacgaagcgtgggacttgggctactactgcctcggcctgtgcgtgatcttgaaggtcgaaggattcgattgggacgcgcctgagtcgtggttcgcggagtggagtaacaactctcttgtgcgccgtgtggatcaggaaaaacggtttgcgtcaagccccactacggattatggtttcgccaagttcgggaaatccttgggatgacaaatggcgaccctagagcagttgcaagcatggctggcggaagcgcaaaccgcctaccatagcgtcatgatcggcggcggcgtgaccgtcgtcgtcgaccagaacggggagcgggtcgagtacagccgggccaacgcaaccggcctcgccaaatacatagccactttgcaagcgcagatcaattccctattgggggtcgcagtaaccggcggcccccttcgtccgttcttctgagggtaaaacgacatggcaaaagcactcactgtcgtgcgctctcccgagggcgacgaagcgttcaacagcaccggcaaagagtcggcgttcggcggtgcgtacgaaggtgcgtcgcgactcaatcggcagaccgcgttgtggagcgcgccgtcgctgccggccgacatggagatttcgccggacaaggttcggctcgatgcgcgcactcgcgaactcattcgcaacgatggctacatccaaggtgctctcgacacgagttcggactccatcgtcggcggtcagtaccttctcaacgcgcgccccgattgggagacgctgggcctgagcgaagagtgggctgaagagttccagctcatcgccgagcgcaagttcatgctgtacgccgagtctccgatgaactggatcgacgcctcgcgcaagaacggtctgaccggcctcgtgcgcatggcgctcgcgcagtctttcatgtcgggcgaagcgctcgccgctgcggagtggctgtcgaaggcaggccgtccgtacaagaccgcgatcaacatgatcgaccccgaccgcctgagcaacccgaacgacaacagcgatacggcgtacatgcgtcgcggcgtcgaaatcgacaagttcggcgcggccgaggcgtaccacatccgcgacgcgcacccgatggagtcgtactacgaccgcttcggcgcgaagtggacgcgcgtgccggcgttcaagccgtggggccgtccgcagatcatccacatcgccgaagtgctgcgcccgggccagacgcgcggcgtatcgaagatggtcgcggtgctgaaagaaatgcgcatgacgaaggtctacaaggacatcgttctgcaaaacgccgtcgtcaatgcgaccttcgctgctgcaatcgaatcggagctgccgcgcgagctggtgttctcgcagctcggtgccggcgacatgggttggttgcagaagtacatgggcgcgctggctgagtatgtcggttcggccgacaatctcgccatcgacggcgtgcgcattccgcacctgtttccgggcacgaagctcaacctgcaaaacgccggccagcccggcggcgtcggcagcggcttcgaggactcgctgctgcgccacatctgcgctgcgctgggcctgtcgtacgagcagttctcgaaggactactcgaagacgaactactcgtctgctcgcgcgtcgatgatcgagacgtggaagtacatgcagacgcgcaagaagctcgtcaccgaccgcttcgcaacgctggtctacatgctgtggctggaagaggaaatcaaccgtccgaataccgacctgccgctgccgaagggcgcggcgcacttctacgaagggatcaaccgcgaggcgtactgccgctgcgactggatcggcgcttcgcgcggccagatcgacgagctgaaggaaacgcaggctgcggtgctgcgcatcgcgtcgggcctgtcgacctacgaggaagaactcggcaagctcggcaaggattaccgcgaagtgttcacgcagcgcgctcgcgaaatgaacctcatcgaaaagaagaaactcaacttcacgctcagcaccagcaagccgggcacgcagaaagaaaccgacagccgcgcatcgaacaacgaagacgcggacgccaccgacgataccgacacggagaacgacgatgaatgaactgctcgcgatgcgcatggcgctcatcgagggattcaacggccgcccggcgttgatcgaccctcgtgatgtcgagaaggtcgcaacgctgtgcatgacgatggcgcaggcatctttcccgccgaccgccgagcagcgcgcgcaggcggatgaaagcatcaccgccgctgtcgagaaggcgttcgacgtttccttcccgcgcgaccgtgccaagccgttccttttcagcaacggccttgccttcatcccgatgcgcggcacgctcgtacatcgcaacggcgacccgtggtacggcacgcgcggctacgacgacatccgccgcgagttcgacgccgcgatggccgacccggacgtggcgggcgtcgtgttcgacatccactccggcggcggcatggtctacggcaacttcgagctggccgagcacattcgcaagggtcgcgacacgaagccgtcgctgtctgtcgtcaacgcgggtgcgatgtcgggcgcgtattcgctcggcagttccgcgaagcgcatggtctcgacgccttcgggcgacagtggcagcattggcgtgctgaccatgcacgtcgacatgagcaaggcgctcgaaaagttcggcgtcgccatctccctcatccatgccggcgagcacaaggtcgacggcaatcccttcaacccgctgcccgacaacgtgcgtgccgacatgcaggcacgtctcgacggcatgtggcagaagttcatctccgtggttgctgttaatcgcgggatgtccgaacaagcgattcgcgacacgcaagcccgtgtgtatcaggcggacgatgcggtcaagatcggcttggtcgatgcggtgatgtctccgcaagacgccatcgctaccttccgggccgaagtcttcggctctaccaccaacgataggagtgcaaccatgagcgacacgaagaagaccgacgccaccgtcgagcagaagaaggacgacgcgcaggtcgagaacaagaccgccgacaccaccgtcgacgcgggcaacaagaacgagcaggtcgatgccggcgcggcgatgcaggcgcgttgcgccgccatcaccggctgcgaggaagccaagggccgcgaaggtctggcgaaccacatcgcgttcaagaccacgatgtcggtcgacgaagcgaagtcgatgctggccgcctcgccgaagcagtcggccgccaccggcaagtcgccgctcgattccgcgatggacaacagcggcggcggtgccgacatcgccaacaacggcggcgacgaagaagagcaggcgcgcggcaacgacgacggcggcctgctgggcgcgtacaccgctgccaccggcaacaaggccgtgctgaaggtcgtcaagtaaaccgaacaccgtcgccagcctagacggaaaaaaccggctaaaccgtcaatcacagaaggagtaacgaaatgaccaacttcggccccatcgctggctacgtggctcgtaccgacacgaacagcatccagctctacgccggggaagcggacatcgtgagcacgcagggcgcgctcgtcaccggcaccgcctacgtcggcggtcaggtgctcggccgcgtcaccgcttccggcctgttcgccaagcacgacccggccgcgaccgatggcagcgagaacgccatcgcgatcctcgcgtacgacgtggcgaccccgactgccgacaagaaggaagcgatctacgtcggcggcgtgttcaacatggaagcgctgaccttcaacgctgccaccaacaccgacgccctgaaggccgctgcgttcgatggcaccaacatcgtcgcgcagaagctctacggtgcgccgcccgccggctccggcccggtctaaccggcatcaccaacagcaagacgtttcgcaattcaactcagaaatagaaggagacaacgatggatttgttcagcactgcggaactgcgcaaggtgatcgtcgacagccggccccccgtgcagtatttcctcgaccgtctgtacaaggagcagatcaacttcacgaccgaagaaatcatgttcgacgagctgaagctcggccggcgcatggctccgttcgtggctccgaacgtgcagggtcgtgtcctgaagcgttccggcttctacaccaagtccttccgcccggcgtacgtcaagccgaaggacgcggtgactccgggccgcatgctgcgtcgcctcgcgggcgaagcactgaccggcgacatgacgcccggccagcgctggcgcgcagtggtcgccgcgtaccagctcgaccagcggaaccagattttccgccgctgggaatggctgggcgcgcaggctgcgctctacggtcaggtcacgatttcgggcgaggactacccgaccgtcaccatcgacttcggtcgcgccgccaaccacacggtcatcctgaccggcaccgcgcggtggaccgaccagaccaacagcgatcccgacgacgacctcgaagagtgggccgctcgtgtgcatgacgccgaaggtttcgtcgtcacccgcgtcacgatgggccgcctcgcgtggaaggcgttcaagaagcacccggtcatcaaggagctgctggaaacccggcgcggctcgaagtccgaagccgaaaccggcccgggcctcggcgagtcggtggagttcaagggccagatcggttcgttcaacatctacgtctacaacgacgtgtacgaggacgagaccggcacgatgcagccgatgatggacccgcgcgacgtgctgctcgaagccgaggctggcttcgacggcgtgcgggccttcggtgcgatcatggatgcggacgccgaccttcaggcgctcgacatcttcccgaagatgtggaagaacccggacccgtccgtgatctacctcatgtcgcagtcggctccgctcatgatcccgagccgtccgaactgcacgctgcgggcgcgcgtcgtcgcgtaagcgtcgtcgcacacggcaagcccggttcgccgggcttcgctgtggcaacacaactccccaaccgaaagaaggagcatcaagatggcgaagtacaagttcgtggcccgcgtggcgctgaagggcgatttcgacgccgaagacggtctcggcaccgcgttgcaggaagtgcaggcgggcaccaaggccggcaccgacgacaagaagctctacgactcgctgctggaacagggctacatcaagtccgcgaaggacgccgcgaaggaagaggacgaggctccggctgcgtcgtcgaacccgagcaccgcgccgaaggtcgagtcgaccgacgccggcaagtccagcggcggcaagcagggcgcgggcaagtaagcccggcgcgctgaagggagaacgaaatgggctggctcgaaaccaagcagaaggctcggcaaaccgtgcatagcacgtttggtctgccggcccaatttcgcccgaggtcgggcggtgctgtcgtcgacggcaccgctcggctgcactacaaggtccgcacgttcggcgacttggaccgcgaaggcttcgcgaccgtcaccgaggcagtggactacatcatcatcgacactcggattttcgtgggcgctgacgaaggcgaccgcgtgttcttcccgcaactcaaccgcgcgttcaagctcgatgtgcgcggcgaagcggaagacgacattttcatcaagtgggaagtgagcgaggtagcgccgtgacggtcgaggttggcttccgtggattggatgacgtgcgcaagcgcgtcgccggcataccggaaacggtagaccgggcatccgcgtttgcgatcaacgaagcggtcacgttcggtcaggccgagagcagccgccgcatccgcgagcaggttgcgttcaaggccagctacatcggcagctcggacgatccgaacgctcgcctgcgtgtgtcgaagaaggcgcgcgtcggcgacctcgaaggcgtcatcgccggccgcatgcgcccgacctcactcgcacagttcatgactggcgcgaagctcggcaaaggcggctacgctcgcgtcaaggtgtcggcgcacggtgcagcgcgtcgaatcccgaatgcgttcccgatgaagctgcgtcgcggtaccggcgtctacgacccggagaacgcgaacgtcggcctcgctgttcggttgcaggacgggaagctgccgggcggcatgaacaagaagcagatggtgcaggtcagcggcaatctctatctgctgtacggcccgtctgtcgatcaagtgtttcgcgatgttcgagtcgatgtgcaagcgccggtcggcgacgtgctcgaatcgagcttcctgcgcaatttcgggagattgaaccgtggctgatacgaagcgcctgctgctgctgaagagcctgtgcaactacctgctgaccgaaatcacgacggcgaacggctacaacttcgacctcgccgccgcgtatcgcggcaagaagaatttcggcaaggaagtgaagctgccggcaatcgtggtgttggagaacttcaacccggatcgtctgccggagaccatcggcggcgtcgtcggcaccaagcacaagtacgaccagatttacctcatcaacggatgggccgaaggcggcgatgtcgagcaggaagaggactcggctcatctactcatgggggacgtgaagcaagcgctcggcaagctgctggtgccgcgcaatcaaagcgggtttttcgatggtctcgcaaacacgctgtccatcgagcccggggttgttcgccctcccgacgagcaatccgagaaggcgtatttctggatgaggattcgtctggaagtcgtcgaaaaggtgggagacccgtactggattcgtgattaaccgttgtatcgacagaaggagaccgtaaatgggcagcgagaattacacccttggccgtggcgaactgcacttcgacaagttcgtcgccggcacgttcaacaagaccggcgagcgttacctcggtaacacgccggagttgaaccgcaccaccgagagcgaaaacctcgatcacttcaacagcgaccgtggtatccgcgtcaaggacaagagcatcgtgctcgaaaagaacgacagcggtacgttcatcgccgacgaaatcagcgacgagaacatcgccctgtggttcctcggcacgcagaacgtcgtggcgcagtcggcgtccgcgagcgtggtgcagaacatcccggccaaccgcgtcaagccgggcacctacatccagctcggcgagtcgaccgccaacccgaccggccatcgcaacgtgacgctgaccagcgtgaccagcgatccggttggcacgaccttcgacaacctgaccgactacacggtcgacgccgagctgggccgcctgtacatcgtgccgggcggggccatcgacgggaccgccccgctgatcgtgacctacgccacggcggcctcgacccgcacgcagatcgtggtcggcgagggcaccaccatcgagggcgcgctgcgcttcatctcgtacaacccgaccggcccgcgccgcgactactactggccctacgtgcagctccgggccgatggcgacttcgcgatgaagggcgacgaatggcagcagctttcgttcgcattcgacatcctgaagcgggacggctacgcttccgagtacatcgacggtcgtccgaccgtggcgtaaccggggtacgtcaaacgcggtcaaggccaacttagtcaagatcaagcgagccaagaccaacttcgacaggccgcctcggaacccccggggcggcctgtttcgcatcaccagccagaagaggaaagtccatgtcccttgccaacctgcaactccgcaccgcaaccgttccgtatgtcggcgcgaacgacgagtcgcacgacatcgtgctgcacggtctgagtgcgaacgccatcgccggcctcatcctgtcgcagctcagcaacatcgaagaaatcttcaacatcgtcgaggcggccggcgtcaagaagaccgaagacctcgccaacgtcaacatcgccgaagtcggccaacggcttctcgtgcagctccccgacttcatcgcgcacgtcatcgcgtactccgcacacgagcccgagcagtggagcaaggtcatgcacctgccggcacccgtgcaggtcgagtgcctgacgaaactcgcgaagctcacgttcaacgacgaagccggcttccgagaattcgtgggaaacgtggtcgcggcgctgcgaagcgcaaaaggcgtagtgccgcagactctcaaccgaaatcccgccgtcaacgcttcgccgaatggtggcttggcatccgagcagccgtctctttcctgacggctgaaggtcactcgaacgctggcgaatatccgctgggatatttgatcgtcgaatcggaaatcgcacgcgagcgggtgaacaacagaatcagaaccgaaatgacgctgacgcagagtgcaatcgcttcggcgctcagcaagaaagcagcatcggcattcaaagaaaacatcgaaggactataggcgatggccgctcagaacgaagttgaactgattgtacgtgcgaagaacctcagcacgcgaaccatcaaccagctcaacgacgagctgagcaagatcgcagataaccaagagcaagtcgccgatgcgaaccgcttggcggagcggtcgttcgagagcctgaagtctgagcagcagcagttgctcgcgatcatgaagtctctcaacgaccgcgcttccaagctggacgcatactcgcgtcaagagcaacaggtgcgcagtctgcgcgacgagctgagtcgcgcccgcgacaacctcaacacgctcgcgcagcagttctacaacaccgaaaagccgacgaaggaattccagcagcagttgaagtcggctgcgagcgaagtcacgcggctggaatcgtcgctgcgcaataacgagcgccggctcgacacgaccggcaacaagctgcgcgacatgggcgtggatgtcacccgcttctcgcagtcgcagcaggaagtcaatcaggcgctcaacagctcggtggcgctgtacaagcgctcgaccgacaacgtggagcgctacgacgcggccgtcaaggaagtgcgcacgacgcagcagcaggctcgcgaggccgagcgcgccgcagcgcaggaagccaaggactcggcggcgaagctggaacaggccgcccgcgagcgcgaagaccagatgcgccgcgaacagaaaatggccgaactgacggccaacgtctaccgcacgctggcccgggagaaggaaaaggcggcccgggcgggggtggacttccgcgccaccggcacgcaggcgctcgccacggcccgcgcgaccgctgcccctgccgtgggtagcgggtcgtctgccggcgcggctgcggcgggcgtacaggcgcttctcgacccggccaaggatgccgtcgcgacgctcgaccggctggaaaaggccgtcgaacagctcgacgaggaattcaaggcgctcacgccggacgctttgcaggccgccgatggcatggacaagctggccgatcaaagccgccggctgcgcgctgcgtcggatgcgctgaaggggcaggccgggctcgcggacgaattgaaccgccagaacaccgcgctgctcgccagccagcagcggttcgaggaagcgcggcaagaagtgatccagtacgcgcaggcggtcgagcgtgcagacaagccgaacgacgagctggcgcagtcgttgcagcgcgcgcagaacgagatgaagcaggcgcacggcgagctgacgcgccagaccgaggcgttcaaccgcgtgcagcagcgcgccgctgccgccggcatcacgctcaacaacctgaccggcatcgagcagcgtctcgctcaggccgccgcgcgcgtgcgcaccgggcaggagcaggttgcgcagacgatgacgcggttggagcagacgaccgcgaagaccaacacgcagttgaagctcttcaacgacggacagcgcaccgcgctctcgttgtatcagcgcacccgtggtcaggtgctctcgctggtgtcggcgtacgtcggcgtgttcggtgcgatcaacctcgtcaacagcgcgatggacgcagcaatcgagaaagagcgcgtcatgtcgcgcctgctcattgcgaataaggggaaccagactgcggcagcggaagagtacgactacctgcgcaagaaggctgacgagctaggcgctgcattcggcccgctcgccgagtcgtactcgcgcttcgccgttgctgcacgcgatgcggggatgagcaccgaggcgacgcgctacatcttcgaggcgttcaccgaggctgcgaccgcaatgcggttgagcggcgacgagacggccggcgcgttccgtgcgctggaacagattttctcgaagggcttcatccaagcggaagaactgcgcggccagttgggcgaccgcatgaccggcgcgttcaatctgttcgcgaaggctatcggcgccacgacgcaagagctgaacgacatgctcgaaaagggcggcgaagtgaaagcagagttcgtgctgctcgctgcgcagacggcccggggcatctatggcccgcaagcgaaggctgcatcgaacagcctgctcggcgacctcaaccgcatgcagaacgcatggggcgacctgaagcgcgaaatcatcgacggcggtctcggtgatgcgctgcgccgcctgttcgtcgacttgacgaagtacctgaagagtgacgacggccagaagttcgccgagaacttgacgaaggtgtttgtcgctgcggccgacgctggcggcgagctgctgaaggtgcttgctgagaacgatgaaatcatcaagctactggcggacaccgttgcgttcctcatcaagaacttcaaggcgctgctcgcgattatgctcgcgatccaaggtgcgcgcatcgcgttggtgttcacgcagcttgcaggcgaaatcctgaaggcgcgtgcggcaacgctcgcgttgaacactgcgcttggtgccggcaccgccgcgtcggcgggccgtgccggtgctgccttgggcggcctcatctccgggccgattgccgcgatcctcgccatcgctgctgcgggcatcgtcatcccgatctacttccagattaagggcgagctggaatcgaacaaggtcaaggtcgacgcgcagaagacgatcaacgacctcaaccggggcttcgaggtttcgcagcgcagcctcagcgacacgtcgaagaccaacgccgaacagctcgaacgtcaggtcacggccgcacagcggttgctcgacatctacgacaagcagaaggagtcgttgcaggcgcagattcgcgagaacactgctgtgcgccgcaaccaagtggcggtacgtgttgcgcagggcacgcgcgagcacgacatgaatttcccggccaagcagctcgccgccgttcgagaagtcgagaacgaaggcaaggcgctggaagcgcagctcgccgcactcgaacagcgtgccgcaccgttgcgccagcaggtcgccgccgccggtcgccagatcggtgaagtgaaagcgcgcgaggcggctgcggagaacgacgcgctcgcggccgagttcaggcgcatccaagctgcggccgatgcggctgcggcgcgtgccggtaccgacgccaaggcggcgaaggcggccgaggctgcacgcaagaaggcggaagccgaagagaagcgtctggccgcgctcgccgagcgccgcctgcgtctggaagaggacgtggcggaaaagctgcgcgacatcgacaacgacattgcggcgtcgcgcccggatacgctcgaagcgcgtctggccgtgatcgacaacaagatcgcggatcgcaaagccgaactggaacgcatgctgcgtgaagtcgacaagctcggtcagtcggatgcagccaagggcgaaattcagcgcggcctcgacgcactgccggcgttgcagcaagcgcaggcgcaggcgaccacacaggagttctacgagcagcggattaatgacttgttgcagcagcgacaggcgtcgatggatgcgatcaacacgttgcaggaagccggtttgctgactagcagcgaagccgccgcgcgtatcgaggaagtcaacgctcgcctgctgccgcagctcgaagcgttgcgtgcgaaggcggctgagttcatggcgacgctgggcgatggtccgcaggcgcaggccgcgcgcgccagcctcgaaaacctcagcgcgcagattcaggcgatgtcggtcgagctgtcggcgcagaagcgtcaggtcatcgacgtgttcgtcaacggcttcggtcaggcgttcatggagaccgcaacgctcatctccgacacgttgaagggcgtgcaggatgccggcgacgcatggaaggcattcggcgacatcgtgctcaacaccatcgccgacatcctcatccagctcgcgcagatgattattcagcaggcgattttcaacgcgctgaaggcggcggccgagaacagcggtggcggttggggccagattatcagcgcggtcgcgagctacctgcacgttggcggcgtggcgggctccggttctggccgtcgttcgtcggtgccggcgtacgtgttcgaggcagcgccgcgctaccacacgggcggcgtcgcgggcctcgcgccggacgaagtgccggcggtgctgaagcgcaacgaggaagtgctgaccgaagatgatccgcgtcaccgcttcaacggcggcatggcgggcggcgctcagcctgcgatggacgtgtccatcatcaacaccatcgacagcgagagcgtggtcgctgccggcgcgaacacccgcgcaggacgccagtccatctttaacgcaatcaaggctgaccgcagctcgtacaagaaacttctcgcataaggaatcgacatgggacacgcaattgcaactgtgactggcggtagcggcgacgaggcacactacaaggtgcttgctgcaatcaagacgctcgctgaagcgaacggctggacgacgctgcgctacgtcaacaccggaaccgtgcgcgagttgatcctcaactccgccggcctgtcgggcaccgaggacatctatatcgggttccgtacctacagcagcgtgagcggcgactactacaacatgctcgtcggtacgttcaccggctacgtctccgcgaactcgttcgactcgcagcccggcgcgaagctgagcggcgtgccttgccacaacaacgcggtgacgtatttcatcactgcgaacgcgcagcgcatcgccggctgcttcaaggtcggcactccggtctacacccacttctacgcgggcaagatgttcccgtattcgcgcccgggcgagttcccgtcgccgctggtgtgcgccggcatgttcgatggtgctgcaccgaagcgtttcagcgacaccgactaccgcttcccgtatcacggccgcgagtcgggctacacgggcggctcgtcgtcgaatgtccgaccgtcgtacctgtggctgcgcgatcaagccggtacgtggcgtcgactctcgcatttcccgttctacaacggccccgccggcagcgatgcgtcgagcgcttacaacgcactcgaaaactggaactacctgactggcggcgaccaatcgcgctcgcttgttccggcgggcacgaattaccagccgcagccgatcatcctgtacacgaccagcgcgccggctggtgcgtgggaaggtgcggtgtacggcgagctggatggcgtgtatgcggtgtcgggcttcaacaacaacgtcgagaacgtgttgcaggtcggcggcacctacgtcgacccggcgggcctgagcatcgtcgatcacgtcgctgcgatcctcgccgctggcggccgtgcattcgtcgtgctgcaagacgtgaatcaaaccgactggcgcagctttatcgctttggagatgacctaatggcttattacaccggcaacttttcctcgttcgctacgctgaagaactcggtcgagaccgcgcttcaggcaaacggctgggggctcaacggcgacggcgtgctggaaaagaacggcatgtatctgcgcctcactgcgacggctgcgcaactgttgttgcaggccggcacgggcagcgcgaccggcgcgcttccgggcgcagctccgaacggcgtcaagatcatggacttcgagggctcgccgatgaatttcccggcgacctacgacctgcacgtcaacactggcccggacgaagtgttcctcgtcgtcaactacaacgccgacaagtaccagcagctctcgtggggcaagtcgaacgtgcagcagatcggcggcaccggcatgtggttctcgggttcattccacgagaacgctgcgtcgaatcagaaccatctcgtctacacgtcggcggatgcgagctacttcggcttcggttggtcgggcatgggctgcggtctgttcgccgagtattacacgcaggcgctcggctgctcctacgtccacacggggctcgacacgaccgcgtggcggcgcgtgtacagcggcgacggcaacctcattggctcgggcgatcctgtcgccggcctgctgcaagcgctgccttcgatgttcaaccaaaacaccgtgctgctgccgctgctggtctcgcagcgtcgactctcgcagggccagaccatcgtcgtcgacatggcgaacgcgcgactgtgccgcaacgataatcacctgtccggcgaaatcgtcgagtacggcgaggacaagtggaaggtttatccgttccaccgcaagaacgccgatgtgcgcaacggcgtctcgtggtcgacgggcgcgaaccactccggcaccttcgcatacgccatccgctacacggggccgtaactcatggcaggcatcaccggacaattcggcagtgaggttgagcgcggcatcgccaacgtgatgctgagcgaagacttggacgacaacaccgaagtcgtctcgcagttcgactcttacgaaatgcgcccgggccttcaaggcggctacgggcgctggcgcgtgcatgccgacaatcattgggcgatcaccggccagcgcaagtcgaccagcttcttcgacgattactacaaccgcatctatatcgtgccggccgcgctcgacgccggcaatttgctgtccacgcaggtgcgccacatcatcctgtggaacgcctacgtcacgccgcagacgttggagaatgccgcgctcggcccgcagtccggcatctcgatgtcgctgcctgtcggcgtgagcctgccgtacgagatggagccgctgcgcgagctggacttcacagtgcagatcgaactcagcggcccgccaaccatcgacagctatgcgaacttcaccgttgaaggcgtcacctacaccgtgccgatcaccggccgacgcatcgtgctgttcccgttctcgccgaattggggctcgcctgtcgacgaaacggtcacgatgcgttcgtgggtgctggccgccgaggatggcagcgagcagaccggcagcgagtcgggcgaggttccgcgtcgtacgctcgaatacaacatcaacctgcgcaccgcgttgcaagcgcaacgctgcgagaatctgctgttcgcgtggcagtcgcgcttcttcggcgtgccgcattggggcgaggaagaacgcatcgctgccgacgtggcggcgggctcgctgacgattccgttcaacaccttcggtctgtcgctcgaacccggctcgctggtggcgctctaccgcgacgacgagaagaacgaaatccgcgaagtgcaggctgtcgccgtcgactgcgttacggtcacgaccgggttggagtacgactggccggaaggctcgcgcgtctacccgtgcttcgtcggcctcatgaacgatgcgatgagcggcacgcgcgaaacgtcgacggtcggccgcatgcctatcgcgttcgactgcgagccgagcgtgaccccgggcaacgtggcgctcaatgcgccgccgctgacctaccgaggcaaggagctgtttctcggccgcaccaactggcagtcggcaatgccttttaccttcacgtcggatgtcaagcgcgtcgactcgaacaccggcaagtttgtcgcgttctcgtcggccggcttctcgaagatggctcgccggcacaactggacgttgtacgaccgcgccgacatcttcgcgttccgtcagttcctcggccgccggcagggcgtcgcgcgctcggtgttcatgccgagcggtacggtcgacttcaacatggctgcgccgatcctcgacactgaagacatcctcgttgtcgagaacaacgagtacggcgcgctggccggcgcacacccggctcgccgcgacatcatcatcgagctggtcgacggcacgtacttctgccggcgcattgtcggcacgagcgacttcgacagcttcacccgtctgcaactcgattcgtcgctgggcgtgtcgctcgacatcgacgacgttgcgcgtatcagcttcctcacgctgtaccgcttcgagtcgccgtcgaccaccatccgccacctgaccgactcgaaggctacggttgaagccatcatggtcgccaagaccaccgaggattgaaatgagcctgctgcaatacgaacaagacaaggaactcagctcccgcgtggagctgtacctgttcgagagcgatgacggccgctaccgctgggcctacacaactgacgcgcgcgaaaaggtgctcggccctatcgtctacaagcccgagtcgatcaagcgcggcgagctgaagcagacggccggcgacgcgaacgtcgagaaccttcaggtcacgatgccgttcgataacccggtggcgctggcgcatgtgccgtacctgccggcgcggccgatcaagctgacgatctacgcctaccagcgcaacgatcctgctgcggaaatcgtgcaggcgttcaccggcttcatcaccagcttcaaccagaagggcgcggaagcgacgctcgaatgctcgcagatcatcgacaacctctcgcagacggtgccgtgggcggtgttcaagagcggctgcatttgggcgctgtatcaggtcggttgcggcgtcgacaagcagttgtggaagaacgatgcgctggtcacgaccgtcaacggctcggtgctgggctcgcctgagttttcggccaagccgaccggctggtacaccaacggattcgcctacaacccgcagacgggcgagcagcgattcatcgtcgcgcacgatgccgctgccggcacgatcacgctggtatacccgttcctcgaaatcaacggaagccagaccatcgaggtctacgcgggctgcgcgcgcacgaaggaagtgtgcgctgacaagttcaacaacaagctcaattacgtcgggttcgaccacttcccggcctacaacgtcttctcgcaggggatcacctaatggtttgggtagccatcgtagttgcgctcgtcatggcagtagttggcgagctgcttcggccgaagccgaaattcaacgacccgaagccttccgctgtcggcgatttttcgttcccgactgcggacgcatcgcgcgtcattccgatcttcttcggtacctgcaagatgcaaggcccgaacgtcgtgtggttcggcgacctgacgatcatcacgctgaagaagaaggtcaagaccggctggttctcgtcgaagcgcatcgtcaccgggtacaactactacctcggtgtgcagctcgtgttcgcctacgggccgtgcgacgagttcatcgagctgcgtatcgacgacaaggttgcgccgatcaccagcaagaccttcaccggcgacgtgtgctcgttcacgatcaacgcgccgacgattatcagcaacgacgacccgccgaatggcgtcaaagggccgtgcaagctgtatcgcggcactttcgagcagccgccgaatatgtacctcagcgcacaatggaacgagccggagatgaccgcgttccgtccgctgctgcacatggtcatggagaagtgctacctcggcaacaccgacacgccgccgcccatctcgatcatcgcgcgccgctgcccgaaccagctcggtttgaccggcggccggcacaacgtcaacggcgactcgaatatcgcgtgcgcggtgtacgaggtcatgaccaacaatatgtggggcatgaaaatccccgaagacaagatcgacgtggactcgttcatcgcctgcggcaacacgctggctgacgagagcatcggcatctcgatgctggttcagaccgccatgctcggccgcgacctcgtggcggaaatgctgcggcacgctgacggtgtggtgtacgccgacccggtgacgggcctgtacacgatgacgctggcgcgcgagattccgtccgacgagcaagacgagctgttgatcgtcgacgactcgaacatcctgcccgacactttcgagttctcgcgttcgtcgtgggagatgacgaagaacacgatcatcgtgcagtacaccgaccgcaccacgttcgagacgacgccggttcagtaccaagacctcgcgaacatcgacgtgcgcggcggcatggtggattccgaagaattcagctacctcggcttcagcaactcgaccgccgcgatgaacaccgccgcgcgcgtgtcgaagatgaaggcgtcgccgttggtgtcggcgaagatgtcgctcaaccgcatcggctaccaactgcgtccgggctccgcgttctggctgcgcaagccgaaccgtggtctggcgaacgtgctcatgcgcgtcatcgaaatcaactacggcacgctggacgacccggctatcaaaatcacggcaatggaagacatcttcgcggtcaacgccgtggcctatgtgccgcccgatccgagcgactggacgccgccggtcggtgccgtcgtgccgttctcgcagcagcgcctcatcgaagcgccggccttcggtgccgaggatatgtcgcgccgctacgtcatcacgatgggagtgccgtcgagtaacggcgtgatcgcgtacgacgtgtggacggataccagcggcggcaccaacttccagcagaccaactccatcgacgcgctcacgccttcgggcgtgctggtgtcgggtctgtcgcgcactggcccggaagtcgatgttgcgggcttcaccgtcacgtcggtcgtcggcgtcagcgacatcgaatccggcactacgggctcgcgcgagtcgggcgaaaacctgctgctggtcggcaacgaactcatggcatggcaaaacatcgtcgacaacggcaacggcacctacacggtcactggcgtgtatcgcggcgtgctcgacacgatgccgcaagaccacggctccggcgcgcgcgtttacttcatgtcggaaggtgcgggcacgaccaacgaagacggctacggcggcgacctgacgctcaacacgaagctgacgccgaagagcatcgtcgacacggtgccgctggacaacgctgcggcgatgtcggtcacgaccaacgctcgtgcgctgcgtccgctgccgccgggtcgtctgcgcatcgacggtgcagtcgtcggctccggcgcaacctacgacggcgacatgctgttctcgtgggcgcaccgcaaccgcctcgacgacagcatcgcatcgcaggccgatccgagccgtacgcccgaggaaggcacgacctacaacatccgggtctacaccagctcgaacgcgctgctggcatctgcgctggaagtgtcgagcgccgcgtcgaccggcaccatgcggttcgcggtgtcaggcgatatgcgcattgaaatcgaggcggttcgggacggctatgtgtcgtggacgaaactggtcggctacttcagctatactccggcctcgggggctaccgccaacgaaatcatcgtcgacgagcctgagtacgtcttggacgggggtggcgcgtaatggcacaggtagtcgttgcacaacgcatgtggcagcgccgcgacactgcggcgaattgggctgcgaagaatccgatcctcgcgggcggcgaaatcggcgtgcagctcggcgctacttcggacgagaccaagttcaagatcggcgacggcgtgaccccgtggaactcgttgtctttcttcgagggccggctcatcgaaatcggcacgggcggcggctacatccgctggcgctacgtcggtgacgagacgtggatcaatctggtctcgcttgaatcgctgcgcggcccgcagggtgcgcaaggcaacccgggcgcgaacggcctgagcgcgtatcaggtcgcggtcgccaacgggttcgccggcacgcaggccgaatggctcgcatcgctgaaaggcgagaagggcgatcaaggcgaccaagggccgcccggtattccgtcgcagcgtcgcatcctgcgtatcacgaacaccgacagcggctccatcgtgtgcgactggaatgcctacgacgaaattcgcgtgacgctgactgccgacacgctcgtaaacatgacgggcgcgctggacggtcaaggctgcgtgctgctgctgaagcaaggcggcgttggcggtcacggcgtttcgttcggcagcaacgtgcgcttcaacaacctaatcccgatttacaacccgacaacgactgccggcaagtccgacaggctcggtttcgtttatgacgacgacgccggcttctacgacgtgcaggcaatcgtggatggaatctaacgatggcagacgactacatcccgccgttgtcgccgaacatcgtgtgggtcttcaagggcaacgactacacgcccccgctgaccccgaacatcgaatggatattcggtgcagatgatgaaggcggcggaaacgagcttcgcaaatccacctacatgctaatcctgacaatgtgaggtattgaaatgactgttcgcacctactcttcttccgacgctggcgctccggttctgcgcggtaacacgccgggcgacctcatcaacctgctcgaaaagtgcctcgtcaccggctacgggtcgaaggccggcgcaggttggacgaagccgtacgccggcacgaacgtcgccgcgtttcagcagggcgcaggctcgaacggcatgttcctgcgtgtcgacgacacgagcactgcgaccagctatcgcgcagcgcgcatcgttggctatgagtcgatgagcggtgtcaacaccggcacaccgacttcgttcccgacgccgacgcagcgcagcggtggcgcagcatggttcacgcactacagcagcggctcggttgcgaacccgcgcccgtggaaaatcatcgctgacgaaatgttcttctggttcttcctgtcgacctacccggaaaacaacgacagcggcttttactacaacgagagctatgcgttcggcgacatcattccgtttaagccgggcgacacgacgcataccgttttgctcgccagctactcggtcgactcgccgaattcctcggagccttacccgtgggatggcgtcagcatttcgagcgcgatgggaagcaatcgctacggcctgtgggcggcgcgttcgtacacgaacctcggcggcccgatctggctcggctggcacgccgatcacgtcaaggcttcttcgagctggggccaagggttcctgtcgtatccgcacggcccggacggcggcctttacctatcgcctgtgtgggttcacgagtaccacgtctcgccgtacaacgtgcgcgggatcatgccgggcctgtgggtgccgtgtcattaccaaggaatcctgagtcagtatcaggagttcgacggacagggcgagctggcaggcaggcggttcatggcgcgccgccactatgagcgcacggtctgcatcgaaatctcgaatacttgggataggtaacgcgcgatggcgctcatcttcaacctgccgatgacggggccgaacggctccacgacgatcaccgacaccacggggaatttctcgtggtcggtgacaggcaacgcgcagattcaatccaacgctctcgtccttgacgggagcggtgactacgtgagcaccactgctgacgttcgattgaacttcgggccgatcaacgatttccgtatcgcgttcgacatgaagatggcggctgcggacaagggcggctataaaatcatcttcgaccagctcaacacgggtgcgtcgaatacgtggacgtggcagctctacacctatgaaggtgtgccgtacttcaacgtctataacaattactacggcaatccgacgccggttcaaggcacgaccgatcttgctgacggcaactggcacacggttgaagtcattcgcactggcggcgctctctcgatgtgggttgacggcgtgcaggttgcaactgctaccgacaatcgcgactacgtgttccagccgcctttcggtatcggttcgcgtatcggctacaacgcatcgtcggcctacgactacaagggcgagctgcgcaacctgtccatctcgatcacgacgccggtcatcctgacgaatcgcatcgcgtcttggactcggcacagcgacatcggctggaaccgtggccgccgcagcagcttcattcggcgcatggcgttctacccggtgcagccggtcacgaccaagaaggtgcagacggtcaaggtgacgcgcggcgtaccgccgtggtgggggccaagcgggtcgaccacgcagctcccgacctacaagctgcgcggccgggtgatgcagcgcgatcctgacggcgtgttgcccgacgccccggtacagtacgcgcgcgtcgtgctgttcttccggcgcttgcatacgctcgtagacatccagctctccgatgtcgacgggtacgtgcaattcgataacctcatgccgggcggtcaggcgtactacgcgattgcattcgacccggaaggcgcaccgttgcagaacgcggtgatttgggatcggctgtcacccgagcccggcccgtaaggagaagtgccgtgagccagaacaacacccacgagcggaacaggaaccgacgagtgacggacaaggcagggggacttttggacgccgcgcagcaggccatccggcttgaacgcatcgaaggcgatatgcgtctgctcacgcagcgcgtcagctccggcatggagaacgtcagcgccacgctcgcggctgtacaggtcgaagtgcgtggctgctcgacgaacgtgtccgagctgcgcggcctgcaaggtgcgcacgactcgaacaaggtggcaatcgacaaggtggagaaatcagtgaccgacctcggtgcgcgcttggagtcgtggttcgatgagttcgaggcaaagcaggaacagcggtggcgcgactatcaagccaaccgcgaccaatggcgacgcgagcacgaggccgagaacgagaacgtcaagaaggacttggaaaaggaaatccgcagcgttcgcgagaccgtcatccgcttcatcggtttcggttccgccataggcgcactcgcgggcgtcatcgttgctggatttttgtggaatatcaactaccgcttcaccgacaacaaagaggacaccgaccgcgtagaaaaatcgtcggcctacaaccgccagctcatcgacgcgatgggcgtggagcacggcagggagttgtccgacatcaagctgtacctcgcccgtggtgggcgaatccccgaagagccctacgttccgcaatcacagaggaaggaaaatggacacgaacaatccgcagcaagcagccaacccgcaaagtgaagtgccgatgcgcacgcgactgtgggagttctggcggcgcaaccaaatcatcctgttccagctcccggtcatgctggtgttcctcatcggcagctacatcgtgctgaagtcggtcgactcgcgcatcggcgtggaaggcttcggcgacatcttcggctacgcgctcaacgcggtgcgcatcacactcatcatcttcaccgcatggtggatgaagaagtggtgctggttcgacctgcacgaccgcaccgaactcgaactgttcgacctgcgcaagcaaggcaaccgcgacgcgcactggatcgtgtggaccgaccgcatcgagtggatgctggcgctcgcgctcgcgaccttctggtacacgcgatgaggggccgggtcgtagttctcgctgcggccctgctgctggccgggtgcgcccggcctgcggccgtgccggcggtcgaccagaccgtgctcccggcggccgtcgacgagctgccggcggccaccccggagcccgtggtcgaacaggtcgtttcggagcaaccgctgccgaccgccgtcgaggcggcttcaggcaccgtcgcggagccgcttctggctgcgcaggcggcgctcgaagacctgaccccgctactacccccgccgccggcccgggacgcggcttgccggcgcgctgcggcggccctgacgctacgctgggaagtgaccagcccggccttctaccggaagcggctcgaactgccgatctggccgggcggggcgtccggggtgacgtgggggatcgggtacgacggcggccaccagacccgcaccgtgattgtcgacgactggcatgaccacgggcaggtcgaccggctgggccagaccgccggcatcctcggccagcaggcccgggcggcgctgccgcgcttccgcgacatcccgaccggcttcgaccatgccagtcgcgtgttcgaggaacgcagcctcgtcgagtacgaacggcgcaccgagcgcgcgttccgcaacggcttcaccgagctgcgaccgaacgcatgcggtgcgctcatctcgctggtgtacaaccgtggcgcggcgatgaccggcgactcgcgacgggagatgcgcaacatccgcgacaactgcgtgccgaagcaggactacgcctgcatcgctgcggagattcgctcgatgaagcgcctgtggcgtggcacggtcaacgagaacggattgtctgcgcgccgcgaggccgaagcgatcctcactgaaaccccgtagggagaagagcatgtggacgaaagcaatcgcgtggctgttcggaacggcaatgggtcgcggtgtgctgctgggcggcagcatcgcgataggcatggcgctcggctggtatgcgttctcgacgcactactacaacgagggcgtcgcgtcgtgccaagctggccgcgccaccgatacgaacgcggccaacgtcgcgcaaggtgaaaagaacatcgccgacaaccagaccagctccgacatcggcaaggccgccgacgccgaagcagcgaaggtcgcagccgatgccgaagaagcgaagaacgactcgaaggagaccatccatgacgtgtacaagaagccccctgtcactgcgcctgttgctgttggttcttgcgtgcatcctctcgatgagcgggtgcaagaccggatcggcaaagcgcgagctgccgcagttgaagcaagaagccccgctcgttaactgcaagcagcctgcgtcgccggcagtgccgcgcgagccgaaggccgacgagtggatcgagtggaacccgccgcgcccgggcaagaccgaaggcgaagcgcggctcagcgagcgtgcggtgaactggatcatcgacgtgctgggcgtggtgcgagtgggcgagggctatcgccgcgtcgagcacaagtgcctcgacgagctggaagcgaaagggctcatccggcagtagttgacaggcccgaggcgctgcattacggttgatcccgctggcggcacttcgcgttgcatcggcactcggcagagggacagcggcgcggagaatcggcgctccgcaccgcagggaacgaggaaccccggactaacactccggggtttctttttgcgtcaagaccaagtgcgtcgtgaccaagttcgtcaagaccggaaaagagaaaagccccggtgctgaggccggggcttttcgggttgcgcgactcacgtcgggcggtgggtatcgaggcggtggttctgctgattccggtgtccgctctatgagcgctgcgccggctggaagggcatgtgtcgcgtcgatggatcgaacctaatgcggcacgcggcgcgtgtcaacaccctcgtcagtccttccactgctcgaccagcttcagcatcttcttgcgcgccttctcgacgccgctcgcccacttgtcccacgcacgcgcgtcgacgtgcgtcaggatttcgttgcgcgccatctcgctcagcacggtcggcggcagcgcgtccagctcccagctcttgtcgccgaagcgctggcggtatttcacgaagcgcgcgtcggtcgtcttggccgggttcggcggcggcttcagctcttcgatctggtcgaggttgagtgccatgcgcttcagcgtgaactcgccgttccagccgaacagctcgaagcgctcttcgaggtcgcgcgtcatgtcgatgccgctcgggtcgtgatccccgaagtgcaggatcaccacatccttgccgtcgctctcttcgatttcccgcttggcgaaatcgcgcacgaccgatgcgctcgggtagccgcgcgctgcgagcagcggcacgtcgaactcatggcacacgcgcgaaaacacgccgaccagcgcttccttctcgacgacgaggaacaggcgcttctcctgcgtcgcccacgggtcggtgtggtactgccgcgccgacgccgtgagaatgtcctgcgggcgcgaccagcggctccgctgctcgaacgagcgcgtgcggtcttcgatggcgtcccaatcaatcaggcccgcgatgcgtgcgtcgttgacgatgctcgtggtctgcttgtacgacttctcgttgttcggaatgatgtcgcgcgcaacgagctggtagtagagctggcgcacggtcagcgtgtaccccgcatcgagatattcttcgatgatcgcgttgatcctgtcgatctgttgcagggtcttcgtcttgaaggtgatttctttgtagcgttcgagactcatggcactcggctcctgttagcggctggcgggctgttcggcggcccggatgtcagtggcgcggatggattcgatttcaggcggcagctcgatgcgctcgaccgcgtagccaacatcgcggccgtagtacacgccgcgcacgtcgggcaccgggtagacgtggtagctgccggcgtgcatgtgcagcgcgtggtggatgcgctgctcgatctgcgggtaggtgtacgggttgtccgggctcggctgcacagtgcgcacgccgatgccgacgtagccgctgcgcgccagcgtctcgcggaacagcgcggtgtgtcccgcatgccacggctgatagcggccgatcatcgtgccctgcggcgtcaggtagcgcaggcacgcagcgatgcgttcgagcgtgggctgcatcacttcggccgtgacctgcaccgcgacttgctgcgggcgctcgaacatttcgtcggtgtccgggtagcggctcttctgcaccgtgtccatgaagacgatgaggtcaggcgcgaacgcctcgcgcgtctcttcggtcgggcacacgaacgacgcgacgacgatgccgtcgtggctgtccgcgacctcacgcatgagctgcgcttggcggatgcggcccggcgtactgaagtcccaatcgccgtgctcttcgcgcactgcgtcgccgtcgatgtgcgttgccggcaacacgcgcgcgagtgctgcgccgagcgtggtcttgccgctgcccggcagaccgcagatgagaattcgcttagccattgttcgattccttctgtgcgcgaagttcttcgcggatttccatgagcagcaggccgagatgattctcgcccttgccgtcgcacacgccccaaaaacggtcgccccaccaattcccttcgacgagcttcgacttcccggtcttcagcaggcgcgaccgaagcgggtcggtgccgaacttctggcgcagcaggtcgcgcatgacgccgaccttgatctgctcccaatcctcgcgcagcgttgcgtgcttgccgcgctgcttcgcgccagcggcactcggctcgttacgaatgcgacggcgctcgtcctcgtcgagcgtcttggctgcttggaaggcgtgctccacggtgcggtacgagtgcccctcgaaggcgatgcagcatgaccagaaattagagaggaagcggtacgggccgttgaagctgtcgatggtcttcatagtgtcccctagtggaagtcgatcttcgccttgctgaagagctggcgctgcttctgcatgtcggtgcgagtgatctggtcttggatgggaacctgcacgttgcgattcatcatctggtgcaggtagcgcggctcgaccgcgtgcccggttgcgaacttcgcaatcgccatgagaatttgcggcgagtgcagctcgaagaacgtgccggtcatcgaccacggttgcggtcgaatgtgcgccgcgatgtcgagcagttgccgctcggccttgcgcacgttgagcggcggctggatgccttgcttcttcatcgagtgctcgacctcgctggccgcgcgatgcacgacgaggtactgcgcgcccgggaaccggacgagcagttggtcgaagaagaacagcgcggccacgtccgacacgaacacgcggccgggcggctgcgcgtcgatcttctggcccagctcggcgatgctcgcgcactgctgaagcgggttgtgcatcgacgagacgcacagcggccgaaggaactcggccatccatgcgctgcggctgcgcggcaggctgagcatgatcgtcaggtgctcgtacgccatgtcagccctccttctgctcgcgcgcgttctttgcgttgtcagcgtacgtgtcgagcacgcgaacgaacgcatcgtgcagcagcgtgccggcgggcacgtagatcaccgtgccgccggtcaggtcgttgcgggtgtagatggtcggagccgcgcccgggatgagctggccttgaccttctggcgtcgcctgcatgcgatccggtgggcgcgagtcgaactcgcgcaccagaccgtccgcagggccaccgacgaagaagccacggacggacgtgttcatcgcacgtctccgtcgccctgcaacgtgccacgctccttgcggccgttgagcttttcgcggttgtcgaacagcagcttttcgtagccgccctcgcaaccgaccagcggccccgtgcgctcggcgtactcgactgagaccgcgatgacggaagccagcgcgccgcgcagctcggcgatcttctccgcacgcttctcgccgctccacgtcgcgccgtcgcgcatcatcttcttgatgacgcccagcacgcggcccgcgtgcgcgcacagcgccgattgcaggtcgtagccgctgatacgaacctcgcggtactcggcgtcggcaaggcgctgcatgccttcctgcaccagcacgtcgaagcgcggcagctccggcgtctcggcgcacaggcgcgcggcgtaccactgcacgtcgcccagctcgtgccacgccttctggtagcgctcgacacgaaactcttccttgacggcttcttggtcgaacagttcggccagctcgccgacttcgttcgccagaccgatgccggtgtacagcatgcccgcgctcacgttgccggcgagctgcacgatgtcggtcgggtacttggccgtggtgacggtgaaggcgttgtacgcctcggcgaagatgcgcgtgggctcgacgcgcgcggcacgcgactcgcgtgcggtatcgagggacaggatgctcatgcgcggcccccggcggcgagcgcgtcagcgaagtcgttgctgtagctggcctcgaacttcgtcgccatgtcgtgcaggacgagcgtggggccgccgtgcgctgccggggtcatggcgaagtcgacgccgcgcaccagcgggttgcgctcgccgtcctgaccgatggcatgcacgaccaacgcttcggggttctcgcgcgcggcgcggcgctcggccttcaggatgcgccgcatggtcttgccgccgaacgccttgcgcagcttttcctcgggcgagccgtggtcgcggatggcgagcacgccggcaatgccgcccttcgacgtgcgcacctgacgcttgttcttgcgctgctcgttttcgaggtcgcgctgctggacgaggaaggcgtagttctcgtcgacggcgagcatgcgcttgcgccagtcgctcagggtcttgcccttctcggcattgtaggaacggaaaatgcgcttcaacaggttcatcgtgtggctccttcaggtgtgaaaaaaaagcggcccggccgatgtcgacggggccgcttcgatgtactacttcaacgccaccgggctcagcggccggcgacgaacttggtctgcttctgcacccggccgcgcttggtctcgcggaacagcacgatggtcgtgttgtcgtcggccatgatgctcgcgtcgtcgagcgcgttgctctcggtcgcgaacgggccgttcatggtgctggccttctgcgaaccgtcttcctgcgcggtcagcagcaggtacgcgaactgcttcgcgcccttcttgccgcgacgcacgccgaccttgcgggcggcggtcttcttgccagcgggacggccgcgcttcttggcgggcgcggcggcctcggtcttcttcgcagcgcgcttggccggagccttcttcgcggcggccttgcgtgcggtcttggcgggagccttcttggtggccttcttggcagcggcgcgcttcttcgcgaccttgccttcggtggcttcggcgttctcggacatctggtttctcctagcgttgttgtcgacaactcgcggaatgcgagcggggttccctcgcgggattcggttcagtccacgcagtacgcggggacttcggtgcggaacgtccggcactcggacggctgcgtgatgtacaggccggcgatggcggccagcagcaacacgccgtagacgatcttctcgcggcggctcatcactcgcagcccacggtggcgttcgggcgggtcggatgcgcggcggtgtactggctgaagtcgcgccagccttccgagccgccgcacgcgaagccccagcggcgcacgatggagccggtcatgaagagcgtccagcacggctcgtcgttgttgccgaacagttcgagcaggtgcatgtggtcggcgctcaggcggcggaagtcgcccgtgtggaagtgctgcgtgtagtcgaacttgtgctggcccgggaacttgcccttgttgcgcaacacgctgccttcgacgaacgtgcggccatcgttcggagtgaacagtcggtgcatgtacgagacgtgcgcgtccatgccttcggggctctcgtcgatggcgtgctcgtagcaccactcgctcgtgtgctcgatgtagcgaccgtcgaggatgagcgacgcactagcccacgggtgatcgtgcagtgcgcggtcgtcgtcgccatgcacgaacttgtgcaggtacaggttgaaccagcggttgcgcgggatgatgtgccagcgcgtcaggtacgggcggcgcgggccgccgtcgatgccgtcgagcatgatgaccttggacggcgagacgatgcgcgcgtacagcttgaacgcaccgacgaagagcggccacaggccgatcatcgagagcgcgttgtagaagcggcgggagaccttgggggcggtcatggcggggaacatcctcggtatggtggggtagttcatgcgtcgagcgtcgcgtcggcggtggccgggccatccgcgttggtcgtgtcgacctgcgggcgaacgagcgggagcggctgcgagccatcgagattcttgaactcgatgtagtagcgcgtgttgagcgtcttcagtccggtgtcgacacggttctggaagacggtcagcagttcggccttcgtcagctctccggcgtgcatgccgccttcggagacgacgcggaagttctcggtgtcgccgctcgtgagcacggcgaggttgtggcggtcgaggatgagtttgtcgagcaagtcgcggatattcggcagttcggcgaagtcgattttcatgttgtctctcggcgtgagatgaagagcggcgtatcgtgccgcaagccgccgggttgacccttcaagcgctggggagtgcgccatccagttgaccgggggtatcgcctcggcgaccccgtgcagttcgtgatttaccccgtagggggacgaagtaaattcgttactgcggggcaactctagcgccagcttttcggcttgtcaacacccttcctcgtgtcgggcgggcggctcagccgggccatcttccgctcgccccggaacagcctgtcgcgcagcatcttctcgctgacgtgcgggcagtggcgcttgatctgctcgaacgtcatctcgtccccgtcgatggtgtacagccgcacacgcgcaacctctttcactgcgtagtcctcgtcgtcgaatttctgcttgctcatagcgcccgtccgtgcgtctcgatgtagatgtcgtgcagcatctcatgcgcgaccgccttacggaacgcgggctgctgcacgagtgcgtgtgcgaagtcgcgcgctgtcggctccttcatgccgagatgcgcggtcatgcgcagcgcttcgtcgatgatggcctgcggctcgccctcggcgtaaccgtcgtccgcaagcagcgcatggatggcctcgcgatacttcgcgtgtcgcgcgcgctgccgcagcatcgcgatgccggcgatgacattggggccaatgactagaagcaaccagtcgaaccagctcatacagacctcgcatacggacgctcttcgccttccttgggcttcggaacgtcatggagagtggacagtcctttcttgatcttggcggccatcgccttgccgaacttcgacgcatcgccgtacatgaggtcgaggtcgggatcggcgcactcggcagcgacgttgcgcagcgtgtcgagcaacatcgggagctggtgctgcgcgctgtagttctcgtggatcatcgtccacgcgccctgcgccttccaccactgcttgcgctcgtgctcgttgagcgcgacgtattggtcgatcatcgccatcgcaaggaacggcgaccagaagcacgtatcgaccggcgtgatcgagtcgcccagctcgtcgagcgcgaagtacaccgcgaacacgggcgtggtgccgatgaggtagaccggctcgtcgagcgggtctttgtaggtggcgatggtgcagccccggtacgcggccatgtgtgcgtagcggcgcttgctggcgtcagggagcggcatgcggaaactctcgttgaagtacgggtcaagggacgctgaggcgtacaagcacgcctgtttgggctcaggttgtgcagctctcatggcagtgaagttgcgctcactcatgcgccgccggcatcgcgcacgagcacgacttcgccgtcctcgccgtcaggcagacatgcagccagtacgtcggccgcgccctgcgtgtcgccgagcacgagcaactggatggcggcgcggatcgcggtctcggtctcgatggccttgcgctcggcggcgagcacgtagccagcaccgtcgcacagctcttcgagcagatgccgcaaccactgtgcagtcgtgaggtctttgcggtcgagcgtcacgccgtacttcttcaggccggcgtcggcgcgctgacggatgatcgagatgaggtcgttcgtggtctgcatgtcgctcatggtgttctccttaccagcggcgggccggggtttcttcgacgcacatgatcgtgtctgccgggaacgaatgcgtcttgccgtactcgtcggtaacggcgatccagccctcggagcgttcgcagtgcttgtagtggttgaacgtcatcgtctggccgtcgcgaaacttgatcgtgcatgtcgccatgtcagaactccttgtggaaatctttctcggcccggatgagagccgaaaccttggggccgaactttttcggcgtgtcgagcaggatgtcggctgcgcccatcgcgatctgcggcgacacgaaatagccttggatcggatgcagcacttcgccgaagtcgtcgacgatgtagtacgcgagatggatgccgacgccatcgagcacgattagcgggccgccgtcgctgcgcacgtcttcgctgtgcagctcggcgatgaacacgtcgcggtacggttggatgcgcttgaacttcatgcggttttgtccttcaggtggtcgagctgccagccggcttcgattgcagcgaacagccgcagctcgctcgcgtcttcggtgtcgagccgcaggaactcgatgaaactgtcgatcatctgcggcgtcatcggtcgcttgtcgtagaacctgcggtacgcgctttgcggaatcatgtcccacaccgggcacaggtcgacgatgcgcttgccttcctcgcgaagatggcggcgcatgatgtcgcgcaccgtcttcgggttcttcttgaccgtgatctttcggccggtcgacggacggaaactcatagcccgatgtcctccgcttcttccttctcgtgcatgcgcagccacggcagctcgacgcgcagcatcgggaacggcccgatccagccgagcacgttgccgtactgttgcgcccagccgtattggtcgtaccacgcgccgcgccgccagatgcacacgcgcatctccttgaagtgcggcgactggcccggccacggttgcagccacaccgcgtagtagccgacctgcgtcggatcgtcgagcgattccatgtcggcgagcgcgagagggccgtgccagccgtacacgatcatctcctttcgcgcagggtggcgctgctcgtgccattgcgccttgtcgtcgaggcggaagagctggtacgcgcgcctgtccgcgttcgccgccgggtactcgcacacttcgacgacgtagaagcccggctcgacgggatcgtcgagcacttcgagttggatggtcattcttccggtgcctcgacgttcgagcgcaaggggcgcaggcgcggcagcgggccgatccagccgtggacttctcccctgaagtattggtcgctgttgaggtagcaccagcggccgttgaaccacatgaggaagatgtcgacgaccagcccgcgaccgtgcgggtcgtctacgcgacatgcgtagacgcccgtgtcctgcggcagtccgatttcttcgtattgaaccttcatccgaacagcagccttgcgacaccgatcactgcgccgatggcgagcagcgctgcgcatgtccagatgacgacgatgacgaccgtcaggaaccgcttcatcggctcagccctcttcgttggcggagtgagcctcgcacttcgtcacgagcagcatgaagtgctcctgcgggagcccgagcaggttgtgcgaatcgagcgtggcgagcagttccttcagcttggccttgccgtggtgccgggcgaacagcagcgtgtagtggcgcagcagctcgcgcatggtgtcctgctcgcgacgcacgcgcgccgcgtcccacgcaccgccgcgttcctgcttcagcgcgtcgacctcgcgtgtgcgcacgcctagcagcgacgacagctcgcggttcttgtccgacagcttcgagacttcggtcgtcgcggtattggcgatctgctggtagttcagcatgtgcttgttgatcgagcggatcgcacgcagcgcgaggcccacgtcgtcgatgtgctcgtagtgcgcgcccatgttgcgccagccgggcaccttgcgatccagctcgcggtagatgacgttgagctgccgctcggcgttggcttcgcggaaatccatcatcgcctcggccgcagcgtgcgcctgctcgccgacactacgcagcgcctcgctcgcgtccttcgtgtccagccgcagctcgacctcgacggtcttgcgcgcattgccttcgtcgtctgccggccgccacgttgcgagccacgtcgcatggtcgcggtaggtgaacttggtgcggtggccgtcgccgtcgcgctccatcgtcacgtagtagtccgtgctgtcctgcttgcggcgcgcgtcgatcacggtgtaggtgccgcccgagatgacggagaagtagcgctcgccagcggccggcggctgctcactgccgtcgaacggcacgttctcgatgaagtcgcggaacagcgattcgatgaggccgtagcccatgccgagttcgggcggcatgccgacgcgacgctcgcgcgcaggcttgaacgacacgtcatgcagctcggcggccatctgcgcatacggactgcccggcacagcgccggcagtcgtcggtgcgaacaggtcgttccacgcgctcgccgtggtgaacatccattcgtactcgccgccgcgcccgttgtcgacgcgcagcatgcgcacatgcgagtggccctcgcactcgtgcgtgctcacgaccatgaagaagcgcgccgggcggttgcgatcctgccagtaggtgccgaccttcggcgcgaactcgtagtccgggtggccgaccgtcactgcacgcgcttccttgcggtcgctcgcagcgcccttggtcgtctgcgtgctgcccttcgagaagtcgcgacgcatgatgcgctcgatgaggctcggcgtgcccttcattgcctcggcgatggcgtccgggctgaagtcgatggtgttgatgatgtggatttcgggcgcgctcgggctctcggcgaacgacggcgcaggcaccttgccgttgtgcgcattgaagaagaactcgtgctggccgacgaacgtgttgcgaatccagcggtgcatgcgctgcgcttccgcgcgctggatgtcgttctggccgacgatgccgccggtagcgtgcatgtcgcgcactatgccgttgtcgtcgatgcacgcggcgaccgacacgatcatcggggtggtagcgtcgttggtgaactgcttttcggtacgacgagacattttcggcgtttcctcggttgggttaggtggtgctgacgtgaccggcggcctcgcggtcaagttgtaggtctgcgatgtcacgcagcgacgagggccagtcgtcgagcggcacgagtccttcctcgtgcatgatgatctggtcgggcgtcaggccgcacaggtagtacgccttcgcgagcgacatgccggcgatgagccggtagcgcatagcagcgcggccgtgcttgaaggattcgacttgcgcccgcgtcacttcgcctgtgcctcggcacaaccggcacttcgtccccggcaagttgtcgtcgtgtcctgcgtcggggccgaacatctcgttgaactcgatcatgtcgtgccgcccttcgcagcgcgggcagacggtcttgtcgcggagccaacgccacgccgcgcgcaccttcatccgcagggcggtacttactgcgcgaccgagcagggcggtagcggtgcgcagacgagacaaagggggtaccggagcattccgagaagccgcaagcctgcggcccaacattttcgcttcttcgatttcgcggcgcgtgtgtcgcatggcgtcggtcactccatccgggtgacagtgagaaacgcgaacatggcgtcgttgctggcgctcatgtaggtgccgcgctccatcttgaaccgcttcgacttgtgctcggccacaccgcgcaccttggcgatgccgccgctcaggatcgagttctgctgcttgaagtatttctgcgcctcgttgttgatcgcggcgatgttgccgttgtcgagcgggatgcgctggcagcgcgcgtgcgactcgccgatgtcgagcttgctgagctggtcgttgagcgagcccggcaggaagaccaaccgaggcttctcggcgatgcgcacgcgcgggttggcgatgtcgctcttcttgatcttcgagcccgacttcttgcggctcttcttcgcaggcgcggcgctgctgttcgtggtggcggatgccattaggtgatgcctcctgttccggggaagtaagcggacaagaaacatactactgcgcgcacccggggtcgtgtcaacccgggcgttctcggtcatgaccagctcgcgcgccgggccagcgccgcacaacgatccggctgggttgccgaagcgggcgcaatttcggaaccggctaggtcggcgaagcgagagcgcaaacggaaccggctggctttgcgaagcgggccgaattttggaacgggctgggtatccgaagcggggacgtttttggaattgcacccttacatgcacgcgcacacagatatgcacgcgggcacgtatgcgcgctcgcctgcgaacgcgctcgcgttctaagtcacgcgggcgcgcggcgcgtgcgggcgcgtcaaggttccgcgcgctgcgcgttgcgcgcggttccttcatccgggcgcgcttgccgccttccgcgcttcctgaatgcaaagtaaacggactactgcgcgcagtaaaaaacatcttgcgcggcgcgcgaaaccgtgtagcctacgcataccggcaacgtcgccggcatcgcaaagggtcgcaaacatggcacgcatgaaccgttccgaattttccgcccatgccgcgcttgccgcgtcgcgtggcgcgtccgctgcgcgcaaggtcgaaaccgcgcgcaaggtccagacgttgcacgatttgctcgcgcgtcttcccttccttttcgccgtcgccgttgccgcctttgtcgcggtcgcggccgtcgccgtttccatcgtctaagggaatcacacaatgcgccgctatcttttcgtttcatccgctacgcttcccgtcgtcgcctacgcggaaagcaaagacgcgatgcgcgcatacgtgcgcgacctgctagggattccgtacggtttcccgctgccgcgccatgccgtttgcagcatcgcttaacaattcactagacaaaggagattcaccatgcaacgcattagcctttcgcaagccttcgcacagtggcaagagctggccgcagacattccgcaagacgatgcgcccatgctggcggaatcgtggaacgattacacggattcgctttgcaaggatggcgcattgtgcgacctgcaataccactacgcgcccgcatacgatgaagagatgcccggcgacggttcgcgcttcgacccgctgagcgatgatcgcgaattcatcctagacgcgctaggcgtcaccatgcgcgcaacgcgcaaggatggaccgcgcgaaggatgggacgcgagcgcgtcacactggcgcgtcacgctgcgccgcgaccgcgcgagcatgacaacggattacagcatgggcgcggcgcatacgggctcgcctgagctggcggacgtgctgaattgtctaatgcgcgatgcggaatgcggcgcgcagtctttcgaggatttttgcgcggaccttggatatgacacggattcgcgcagcgcggaaaagacgtggcgcgcgtgcaaggtgacggccgtcgggctcgcgcggcttttcagcgatggcatgctgcgcgacctgcgcgaattgttcgaggatttttgaccatgagcgagctagacattagcgcggttgtcgccggcatgcgcgacccttggaattactcggcgagcgttgcggaacgcgggcaggatgccggccgcatgacgtgggaagccgcatgcgaggatgcgcgcggcttgttcggcgagcatttcgaccgcgccgcgttcgatgagtatttttcgcatttcggcgcgtgggatgatgaagagctggccgcgcatacggatgaagaatgcgccgcgcttatgctgcaattcatcgccggcgacatgcgcgaggctgatttttccagctatgcggacatcgaaggcggcgcggaaccgttcacggatgaatggtggccgcagtatgaaaaagcgagcgaggccggaaccgtcgccggccgtttctttcgcgacgctggcggcgttttttactacattggagaatgaaacatgcaaagcaaatgggcaaagacaaccgcgcagcgcatcgcatccggcgagctggcggaatccatcatccgcaaggcgcgcgcgttgctgcgcgatgccgtgaatgctgaagagtatttcaagcgcgaaccgtcgccgtctgctaccgctgcggaagcgtgggagctggtggagatgattagcacgcatgcgccgcgcgtcacggatgcgcaagcgcgcaagggcgcggaatggctgcgccgccttgtctacacgtcgcgcggcacggtgcgccgcacggaagccgcgcagcaattcagcgatgcggacctgcgcgttttgcaggcttgcatcgcgcgcccggccttccgtctggtggagctggaaccgcacagcgacggccgatacctgcgcgaccttgcgcccgtctatcgctgcatcggcgacaacggcgaatccttcgattacacggcgagcgcgtggcagtctggcggcgcgttcgcaatcctgcgccacgcttaacccttcccatccgtgacaagcccggagaatctgaaaatgtacagcatcgcaaacaacgcaaagcccgccattctgacgcgcacggaatcgcgcatccaatcgcagcgcgacaagcgaacgcgcgacacggaagcgcgccgcgcaaagtatcggcgcaacgctgcgcgctatctggccgcgtctttctggcgcggctcgcgcgacatcgccgatttttttaagggtcgcggattcgaccatgcgacgttgcaggatgcggaaaacgattgcatggataacgtcgatttttcttatctgtattcccgcgactatgcgcgcgagctggaaaaggaatacggcgacgacgcgcgcgaattgttcgcgtacctttgcccggatgcgccgctgagcgtgtaccgtgagcaaatcgccgacgacgtgacgcgcgcggtcgcagactcgcggcgcgcggattatgcgttgcagtttttcgactggtgccgcgatgcggtcgaggatgcggccgattcttccgggcttgtctggtgctggctggacaaggccggcaagcctacggatcaggaatacgatgcgcacgcggtaggcttcgcatgctcgcgccgcatgtacctttcgcgcaatgcggaatggtggccggaaaaatggtgggcgaaaggtgaaagcgtttggagcgattacgcgagcaatcgcgaacgcatggacgcggccgatgacgtgctgaacgaatttctcggtgagcatctggaaagcgaaggcgcggaccttgaatcgttcgatgagcgcggttcgcgctatgcggatgatgattattggccggaatacttcagcgactacagcgaagcgcgcgagcaatgggaaaacgacaaagcaaagatgcgcgcgcgtctgcgcgagatgatcgcgaaccgtgcgccgctggaattgcgcgccgcgcttgtcgcgagcgtgtacggcgagcccggccgcgcggccgatgaatccgaagattgaaaggga

SEQ ID NO: 13 - DNA, 55087 bp, unidentified
  source 1..55087: mol_type = genomic DNA
gggggcgctgacctcggtgctcgcgcatttttcggaattttcgcggtttcgtctcctttggacccccggagctgcccgaatttccgaatttattccccgaataaacgcgaatttcctgtgacagtagtgacagtgacgtttttgggtactgtcacaaattcggccccccaagaaatccgctcaaatcaacgatttacaggcgcgaatttactgcgagtttaggctcagtgacactgtgacagtgacttccaatcctttacggcggaaagaaaagttctgcctgccaagaaaattttctcgcgtatgagagaaggtactgtcactactgtcactactgtcacaagttagggaaaaaggtaggcagatcaagcacttgaatttgtgacagtaccttgtgacagtgaccgctttgcgcctcgaagagcatggaaaatagggtactgtcacaagaatcggcctttttccgaatttccgtccatacggttggaattttttccgtatgtgacagtgaaaagaattcggaattaatttaatcggaaccgctgcgaggcgtcgtgcggaaattcggaaattccgggcaataaaaaagccccgggggatgagcccggggccggcactgcggaaattccgccgaattaaattgcgttcttcggcgctccgtcgcctacgcgcacgtcctcgacgttcgagccgttgtcacccgcgcccggcgggagcggatcgctctcgtagcggttcgcgtcggtgttgcccggatcgacgctcgcgttcggcaccgcaccttgctgcttcggtgcgccgaagaactcgccggtctcgcgcgctgtgacctgcaagtcaccgtgcatcgtgatttcgaccgaacggccgggcgcatcgagcactgcatgcacaacgccattgccgtcgaccaactcgactgccttgttgccgatgacgtgcgtgaacttcacggtagatgtcatgtcgtttctcctgtgctcgggattgagcgtcttcgatcatacgcttgcaggcatgaaaaagcccggttgcccgggcttcttcgatcacaccttcagcgacgtgatttctatgtagtcgtcgatccactgctgaaggttcggccgcaccaccacgtcgggcgagcgcgaccaataccgggcctgctttccattcgcgccgcgcgcgcggcccacgtacacgaagcccttcgaggtcaggaagttcgacagcttcggcccgtacggcacgccgacactgttgtccatcgcgaggtcacgcagcttcccgacgttgagcagcaggctcgtcacttccgggtcgcgcgactccgcgatcatctcttcgatttcgtcttcgtcgtcgccgcgcgcgaggtcgatcatgcgcgccttcgcgtcggtcatgggcgcatggccgtccgggtcgaactcaggatgcagcgggtagtcttccagccactcgcggatcgcgcccgggtgataggcgattgcgttgaagatgtcgtcgtagtgatccgggttgcgcgcgcggaacttctcgatcatctgcttcgtctggaagtgggtcgagatgacgaagtagcggcggtcggcgtcgtacaccggcagcgcatcgctgtggttggtcaagatgatcgtcgaggtcacgttcggcacgttgtacgagtcgcggtgcatgcggcgaatcgaaaccacgtcgttcgtgatgaagggcttcagcttgtccatcaccgcgtagcgcgacgtaccgtggatgcgtgcctcttcgagcaccacgaccttgcgcgactcgaagaacgacgtgtacttctcttcgagcgcctgagcgttgacggtctcgacgttgttgcgcgacatgatcgccatgagcatttcaccgacgaagcccttgcctgcgccgtccacgccctgcatcacaaccgcccaacggattttcttgtccatgcgcttgatcgtgtaagccagccacgagagcaggatttcgcgctcgcgctcgatggggtacgaaatctcgaagtgacgcttcacggcttcgactgcgcgccgggccttgctgctcagcttgtcgggcaccggcacgatgtcttccgggttgaacttgttcgcgtgcttctggccgtcccactcgacgatgcggtctgcgccgggcaggtaaacgtagccgctgacgaccgggacttggtacacgttgagcgcgagtgcggcggcctgttgctcaggcacggcttccatgttcgagcggtctttcttcgacagcaggaaacggttgttgcgcgcattgaacgcacgctcgctcagcgcgaggcggttgtccatgtagtagaactcttcctcggcgtcgacgtacaccacgtcgttgcaccaatgtggcagttccttgtagttgaagtcggagttgcggtagccctcgttgatcgccttgcggatcatcgcgatgggaaccttcttccccagctccgcgacgcgctccttgatcgcgccggccaacagctcgacttggaagtcgctttcgagcatgcggccccacttcgcagcgagcgggccaagcaactccatctcgctcgtcgtctcggcgaccttgcgcttgatcttctcgaactgttcctgcgagtgctcctgccgatgctccttcgccatcttgataagcgaggcggccgtcgtcaggttgcggcccatgtcgtcgtggaacgagttccacttgaactccaattcgtcggggtcgtagttgtgcgctggctccgaccactcgtgccacaacgtcaagccttcttcgttgccgtcgaattggtgatgcagcgccatgccgaccttcaaccactgctcgtagtcgtcggcaccgggaacccattgcagcacttcgcggagctggtcttcggtcaggttttccagcgggcgcttgtattccagcagtgcgttgtcgttctcgtcgtcgctgctgcgcgactcgctcggtgcgttgtgcttcttcaacgtccatccgcgacgctgcgcttcgagcttgaacaccgagaagagttcgtcgatgtgctcggttgtgatttccggcagcatgtcggccggcacgctcagcgggttgagttccttgcccgaagtccacttgtacggcttcttggtatcgggatggatgccgatgccgacgaactgctggccgtctgcgagcacttcgatggactgctcgtggccctcggtgtcgaggaacgtgatcttccgcttcgagaacggaatgtcagtgcgatacacgagcaacgtcttcggcgcacggccgacgcgcgtcatcgtcttgccgatgatttcctcggtgtgctcggccatgagcgccgccatctcgtcatcggtgatgtcgatgtcgaccgcaggcgtgtgcttcgtgtggaagccgatgttgccctgcttgtagttgccgctcgcccacttgcgaacgagcttttcggtggcttggattttctgccactgcggttcaatcgggcctttccttcctgccgggatcggcaagatggagtacccgttttccagcaattgcgcgccgtacttacggagcacgctggtgatcggtcgtccagcagccataggtcactccgcgatgtcgtcgctaacaaggtcttcgaggttgaagccgatcttgcggttgaaatccttgtgcaagatggtcgccttgtcgcgcggcacaccgccgaggcgctgccaacgcgagacagtggtctcgtgccagttgtacttctcgcaaattgcgttgagccgaccgtacggcgggtcgagcatgagggcgatgcgccgaagcagatagcgcactcgcgcgtctgcgctgtccagtgaatcaagagtagggtctcggcgcatgaattcctcgcagacgttgggatttaaggggtctgctaagtcggtgagcatgcctattgacttagcatcgggacaggcgcatagtgcgctcgccgggcaggaattgcaatccacccgtcactcccgaaaccaacctagctaggagatacaaccgatgtcgaagatcaacgcgaagaagctcgccgaagccatcaccctcatcatcgaagcagtcggcggcggtgccgccaacgagtccgaggatgcgggcggcgaagaggaagcgccgaagaagggtcgcggccgtccggccggcagcaccaacaaggccaaggccgagaccaagcccgccgccaagggcaaggccaaggcgaaggacgaggacgaggacgaggacgacggtctcggcgacgacgacgatgccggcgacgacgatgacgacctcggtctcggcggcgacgacgaagaagtgacgcaggaagatgtcgtcaatgcgttcaaggcgctgaaggcgagcaagggcatcgacaagtgccgcgaagtgctcgccaagctggacgagagcaacgtgctcaacatcccgccgaagaagtacgccgaggcgctgaaggaaatcaaccgcgccgcgtcgaagaagtaactcggcctgcacgtcacacgaaacgcccgggttcgctcgggcgtttctttcggagaggaacacatgcccggttcgcacgcccgcttcgcaccatcgtcggcgcatcgcatctacgattgcccggcgagcctgttgctcaacgagaacgagcccgaccgcgaaatctacgaagcggccgagggcaccgttgcacaccacatcgcggaaatctgcgcacgcgcgcgccgcgagccggaagagtttctaggaatgacgttcgacagcggcgacctcgacgccgactacgacgaagagcagcattcctcgaaaggcttcgcaatcaccgtcgacgacgagatggtgcagggagtcggggcgtacctcgaccgcatcatgggcctgccgggcgaccactacgtcgagacgcgcgtcaacatctccccgtggtgcccgatccccgatcaattcggcacctgcgaccacgcagccgcgtcgcacaagaagctcatcatcaccgacctgaagtacggccgcgtgcaggtcgatgcgccgcagaacaagcagctcgtgatgtacgcgctcggcttcatcaacgagtacgactggctgtacgacttcgatgaggtcatcatccgcattgcgcaaccgcgcctcgatcacttcgacgtgtggatcaccagcaaggccgaactgctcgctatcggcgagaagatcaaagagcgcttcgcgcttgcgttgaagccgaatccgccgttcggcccgagcgagaaggcgtgccgcttctgcaaggtcaacttcaagtgccgcgcgaaccacgacttcctgtaccacgagcgcatcatgctgctcgatgacgacgacgagttcgtcgagcctgacctcatgctcatgagcgacgacgaaatcgctgcgctgtggctgcgcaagggcatgtacgagaaccgcatgcgcgcggtcgaagactacctgcacaagaaggtcgcggacggcgacttcgtgccgggcctgaagaccgtggcgggccgcagctcgcgctacttcaccagcgaaatcgacgccgagctgctgctgctggaagccggcgtgcccgagtctaagctgtactccaaacccgaattcgtgtcgcctgcgcaggctgaaaagctggtgcgcggcgaggcgaagaagaaattgcaggacttcatcaagtcgaagcccggcaaaccctgtctggtctcttccgacgacaaacggaaagacctgaccgtccagtcgctcgaactgctcgacgactgacgcaaccgttgtacgaatgcgcgaaagcgaactacgaacgtcgaatgacgaaggagaaatcgaaatggcgaagaagaaagttggtgatctggtcgacaagggcaatgggcgttttctgctgaagaacgtgcgcctgagcttcccgtacttgttcgagcccgacgagcaggaagacgacaacggcaacaagaagaagtcgtaccgcgtcaccctgctgctcccgaaggcgacgcacaagcccgtcgcgcagaagctctcccgtctcatctccgagatgtgcgaggaagagtacggcaacccgaagctggcggccgaccgcaagttcctgcgcgatggtgacgagtcggatgtcgaagatcatcacggctgctggacggtgacggttcgcgagacccggaagccgatcctcgtcgaccgtgatcgtcagcccaccgaggaagacgacgagctgctgtacagcggcgcgtgggccaacgtggtgatccgcccgtgggctcagaacggcaagtccatgaagaagaagaacaagtacggcaagcgcatcaatgccggcttcgacatcgtgcagttcgtcgaccacgacgacaacctcgcgggcaacgctcgcccggatgtcgacgaggttctggatgagctggacgacgacttcgcggatgacgacgacaacagcaccagccgcagcaagtccaagagcaagtcgaagggtcgttctcgcgacgaggacgatgacgacgacgggctcggcgacgacgatgacgacgaccgcagctcgcgccgcagccgtccgtcgaagagcaagaccagcagcaagagccgtcgctcgcgcgacgacgatgacgatgacggcgacgaggacgatgacgacctcggcatctaaaatcgggcatcggtaagcggtacctacggtcgcccgggcactccccgggcggctgtttttcagggatacggtatggacaagctgcatcacgacttcgagaccttcagcaagtgcgacctgaagaagcacggcttggcgcgctatgctcgcgacaagtcgaccgaagtgctgttcctgtggtacgcattcaacgacgaggaacccgaagtgtggttccccgcgacggagccgatgccgaagcgcctgcgccgcgcgctcaaagacccgaacgtgcagaagtgcgcgcacaacgctcagttcgagcgcgcgatttggctgcacgtcctcggcatcgacatcccggtcgagcagttctattgctcgatggcgcacgcattctggctctcgctgcccggcaacctcgacgaactctcgggcgtgcttcgcctcggcgagaacgcgaagatgaaggaaggcaagtcgctcgtgaagttcttctgcgggccgcgcaagccgacgaagaccaagcagtacacgcgcaacaccgcgcagaccgatccggcgaagtggaagacgttcgtcgagtacggccgccgcgacgtgatcgccgagcgcgcggcaggtcgcaagctctcgctcttcccgatgagcgatttcgagcgcaacctgtggtacatcgaccagcacatcaacgaacgcggcattccgttcgacaaggaattcgtcgagaccgcgctgcgcgtcatcgcgaaggagaagaagcgcctgctgggcgagatgagccgcatcaccggcctgagcaatcccggcagcggtgcacagttgctcccgtggctgcgcgagcgcggctacccgttcaccaacctcaaatccgcctcgatcaagaaggcacgcgaggattgggactggaacatgaccgatgaggcgaacgcggttctcgccttgcacgcggaagcggcgcgttcgtctgtcacgaagttgcagaagatgctcgacatcgaagtcgacggagtgctgtgctacacgatgcagttcgcaggcgcggggcgcacggcgcgctgggccggtcgcgcagtgcaggtgcaaaatttgccccgccccctccgcgaactagaagagcaaggggcactgctcatggcgcgcgatgcgatcatgcgcgaagacatcgagttccttcgcctgctggtgtcgtcgccgatgggcgcgattgcatcgtgcatccgcaccgcgatcaaagcgccgcccggctacgagtatgcaacgtgcgacttggcctcgattgagtccgtcgtcattgcatggctgtcgggctgcgacaagttgatcgaggtctttcagaagaacctcgacgtgtacaaggtgttcgcgtcgaagatgtacaaggtcgactacgagcaggtcgagaagtggatgcgtcaacacgcaaagcccggcgtgctcggcgcaggcttccgcctcagcggcggcatggagttgggcgagtacccggaagtcatcaagaccggcctgtggggctacgcggagaacatgggcatcgagatgtcgcagaaggatgctgcggccgtcgtgaaattcttccgcgaggaatacaccgaaatcgtcgagctgtggtacgagctggaacgcgccgtcgcgaaggtgatgaacacgaaggagccggtgcgcgttggtccgatcctcatggacgtgaagggaccgttcctgcgcatgcgtctgccgtccggtcgctacctgcactacctgcggccgaagatgatctggaagaagatcaaggtcggcatcgacaagaagaccggcaagccgaaatacaagtcgaagaagggcttcacctacgaaggctacaacacgaagaagaagtggacgcgcatcgactcgcacggcggcaagatcgtcgagaacttggtgcaggcaatcgcacgcgagctgctggccgccggtctgctgcgcgcttggaaggccgggctcgatgtgcgcatgcacgttcacgacgaaatcgttgcgctggtcaagcgcaagctgtcggacatctcggccgcgacgctcgaagagcagatggtcaagaagccgaagtggtggggcgaagacgttccgatccgtgcgaaggctgacgtagtggagtgctatcagaaatgagctggctgaccgattggcgcaacgtaatcaacggcaagccgccgcgcggcgacatcctgccgaccgacaagcatcgcgtcgaaaaggacgtggagcagaagtggtgcgccgttgcgaagcggcacggatggaaggcatacaagttctcgtcgcccggcaacagcagcgttcccgaccgcatgttcatccgcaacggcttcgtcttcttcatcgagttcaagcgccccggcggcaaggcaaccgacaatcaactcgaagagcacaaggagctgcggcgcaagggcatgatcgtgtgggtcatcgactacttcgataaagaattcgccgagtggatttttgaatgaaacaactactgaagcgctccgacctcgacgagtttcaaatcgctgccggcctgttcctcgaacgggtcggcagttgcgcgttgtggatcgacatgggcctcggcaagaccgtggtcgtgctcacgcatgtttcggacaaggtgttctccggcgagtggagccgcgtgctggtcgtaggcccgccgctggtcatctccgatacgtggtcgaccgaggtcaagaattgggagcacacccgcttcctcgactatcaggaactcgacggcgacagcgagcacatgcgcatgcagttgcagcggccgtgcgaggtcgacggcatctcggtgcataaactcgggcgtctcgcggcgctgttcaagcgaggcgacacggtgccgtgggacgcggttgtgttcgacgagtcgagcatgttccgcaacaagtcgtcgaagcgctggaagtacggcgtgcgcctgacgtggggccagccgaacgacgtgatcgagctgacaggtacgccgagcccgaacggcctgcatcaagtctggtcgcagattgcgatgatcgacggcggcgagcggctgggcttgacgtacaagaagttcctgttccgctggttcaagcaggagttcatgggccgcaaagtgattccgaagtcgcacgcgatggcgtcgatcacgaagaagctgagcgacatcgtgtacaccttgcgcgaagaggattacgtcaagttgccgccgctccgctctacgcctgtgccgatcatcctgccgccggatgtgatggctcgctatcaggaattcgagcgcacgtctgtgctgaagtggggcgaagagcaagacccggcagtgcgtgctctatcggaaggcgcgctgtacggaaagctgttgcaatttgcgtgcggtcgcatctatacggattcagagacgaaagagttcgtcgacatacacgacaagaagatcgagcgcctgaaggaaatcgtcgagttcagcgacggctcgccgatcctcgtggcacgtacgtggcagcactcgcgtgatcggctgcgcgatgagttcccgggcatccgctcgttgaagacgaagcgcgacctcgacgcatggaacgcgggcgacatcgagatagccgagacacaccctgcgagcatcggtcacggcacgaacatccagaagggcggcaacaacctcatctggtacgaccacacgcccgacctcgaactctacatgcagttgcgcaaacgactgcaccgacgcggccagacccgaagccacgtcaacatgatgcacctgacagcagtaggcactatcgaagaggatttgacacgcgagctggtcaagaaagaaattacccaagacgccctgagagaacccatgcggcgacgagtcgcagacgtacagagagaactagccaatggccgcacctaagatcgactacgaagaagagtttttcgacggcatgaccgtgccgcgtctggcgcagttgttccgcctcgaccgccgcactgttaccgagaagctgcgtccgctgcgaccgaccggcgaccggcgcggcgcaccgacgcatcacatcgtcgacgctgcaccgtacctcgtggagcccatcgtcgacatcgccaagtacctcgcggaagtcggccccggcgacctgcccgcaccgctgcaagcgcagtattggaacgcgcagaacagcaagttgaagtacaaggaacagtcgggcgacttgtggcgcacgcaacaggtgctcgaagtgctgaccggcgtgttccgctcgctcacgcaatcgcttcgcctgctggccgaccgcatcgaagcgcagaccgggctcacgccggagcagcgcgcgatcatcgagcgcgaagtgtcagacaaggccatcgacatgctgcgcaagcgccttgtcgaagacttcgagatttacgtcggcatcaaggacaaggaacagctcgccgacatcaagctcgacgacatcggcctcgacgaagaggacgaagaagatgtctgacggcagctttttcaacgacctcggcgagctggtcacgttcgttgccgatagcgttctggttccgccggagcgcttgaccgtttctcaggccgcagcaaagtaccgctacctcgacaacgaaggctcgttcgtcggcgagtgggacaacaacgaaacgccgtacctcgtcgagccgatggacgtgctcacgagtcgcgagttcgagtcgtgcatcttcatcggcccggcgcagggcggcaagaccgaaatcatcctcaattggatcgcatacaccgcgaagtgcgacccggccgacttcttcctcatccagaccgcgcgcgacaccgcacgcgacttctcgtatcgccgcatcgacaagatgcaccgcgacagcaaggagctgggcgcgatgctgcgtccgggcagcgacaacgacaacatcttcgacaagttctaccgcaacggcatgatgctgacgctgggctggccgacgatcaaccagctctcaggcaagccggtgccgcgcgtcgcgctgaccgactatgaccgcatgccgcaggacgtggagaagaacggcccgccgttcccgctcgctcgtaagcgtacgacgaccttcggctcgttcggcatgacgctggccgagtcgtcgccgtcgttcgacgtgaaagacccgaaatggaaggcaccgcacccggactcgcatatgttcccgccgtgcgatgggatcggcggcctgtacaacgaaggcgaccgccgttgcttctactggcagtgccctcactgcggcgagtggtttgagccgaagttctcgctgctgaagtgggacatcaagaaccccgacccgttcgaggctgcgatgtcgacgatgatggcgtgcccgcgtaacggttgcgtcatcgagccgaagcacaagtacgagatgaatcgacgcggcgtgtggctgcgagaaggccagcgtattgatcgcgacggcaacaagctcggcgtcggcgttcgctcacgtagcgcatcgttctggctgaaaggcccggcggcgcgcttcattacatggcagaccctcgtcgagcgattcctgcttgcgcaccagacgctcgaacgcacgggcgaaaccaaggcgctgaaggccacgatcaacaccgatcaaggcgaagcgttctggccgctcaacgcgaaggactcgaaccgcctgccggaagacctgcaatcgaaggcgatccagtgggccgacaagaaggtgccgtacggcgtgcgcttcctgctcgggactgtcgacgtgcagaagagccgcttcgtcgtgcaggtcttcggcgtcggcccgagcgataacggcgtcaacttcgacctgtacctaatcgaccgattcgacattcagaagtcgaagcgcaaggacgaggctggcgacacactatgggtcaagccgtatgccgtgcaggaagattgggacttgattaccgagcaggtcgtcgagaaggaatacgagctggaagacggcagtggcttcatgtcgatcaagatgaccggcatcgactccggcggtaagtcaggctcgacgacgcgcgcatacaactactggcgctcgatgcgcgacaacggcaacggcggtcgcgtgctgctcatcaagggcgagccgaagctcggtgcgccgcgtgccgaaatcgacttccccgactcggatcgcaaggatcgttcggccggtgcgcgcggtgaaatcccggtgctgttcctcaactcgaacgtgctgaaggacatgctgctcggcatggtcgactacgacgagaagacgacgctcggcggcaggcacttcacgaacaagtggacgccggaagttgtgtacgccgaactcactgtcgagttccgcgacgaccgtggtcgttggcagaatccggctaagcgacgcaacgaagcgtgggacttgggctactactgcctcggcctgtgcgtgatcttgaaggtcgaaggattcgattgggacgcgcctgagtcgtggttcgcggagtggagtaacaactctcttgtgcgccgtgtggatcaggaaaaacggtttgcgtcaagccccactacggattatggtttcgccaagttcgggaaatccttgggatgacaaatggcgaccctagagcagttgcaagcatggctggcggaagcgcaaaccgcctaccatagcgtcatgatcggcggcggcgtgaccgtcgtcgtcgaccagaacggggagcgggtcgagtacagccgggccaacgcaaccggcctcgccaaatacatagccactttgcaagcgcagatcaattccctattgggggtcgcagtaacaggcggcccccttcgtccgttcttctgagggtaaaacgacatggcaaaagcactcactgtcgtgcgctctcccgagggcgacgaagcgttcaacagcaccggcaaagagtcggcgttcggcggtgcgtacgaaggtgcgtcgcgactcaatcggcagaccgcgttgtggagcgcgccgtcgctgccggccgacatggagatttcgccggacaaggttcggctcgatgcgcgcactcgcgaactcattcgcaacgatggctacatccaaggtgctctcgacacgagttcggactccatcgtcggcggtcagtaccttctcaacgcgcgccccgattgggagacgctgggcctgagcgaagagtgggctgaagagttccagctcatcgccgagcgcaagttcatgctgtacgccgagtctccgatgaactggatcgacgcctcgcgcaagaacggtctgaccggcctcgtgcgcatggcgctcgcgcagtctttcatgtcgggcgaagcgctcgccgctgcggagtggctgtcgaaggcaggccgtccgtacaagaccgcgatcaacatgatcgaccccgaccgcctgagcaacccgaacgacaacagcgatacggcgtacatgcgtcgcggcgtcgaaatcgacaagttcggcgcggccgaggcgtaccacatccgcgacgcgcacccgatggagtcgtactacgaccgcttcggcgcgaagtggacgcgcgtgccggcgttcaagccgtggggccgtccgcagatcatccacatcgccgaagtgctgcgcccgggccagacgcgcggcgtatcgaagatggtcgcggtgctgaaagaaatgcgcatgacgaaggtctacaaggacatcgttctgcaaaacgccgtcgtcaatgcgaccttcgctgctgcaatcgaatcggagctgccgcgcgagctggtgttctcgcagctcggtgccggcgacatgggttggttgcagaagtacatgggcgcgctggctgagtatgtcggttcggccgacaatctcgccatcgacggcgtgcgcattccgcacctgtttccgggcacgaagctcaacctgcaaaacgccggccagcccggcggcgtcggcagcggcttcgaggactcgctgctgcgccacatctgcgctgcgctgggcctgtcgtacgagcagttctcgaaggactactcgaagacgaactactcgtctgctcgcgcgtcgatgatcgagacgtggaagtacatgcagacgcgcaagaagctcgtcaccgaccgcttcgcaacgctggtctacatgctgtggctggaagaggaaatcaaccgtccgaataccgacctgccgctgccgaagggcgcggcgcacttctacgaagggatcaaccgcgaggcgtactgccgctgcgactggatcggcgcttcgcgcggccagatcgacgagctgaaggaaacgcaggctgcggtgctgcgcatcgcgtcgggcctgtcgacctacgaggaagaactcggcaagctcggcaaggattaccgcgaagtgttcacgcagcgcgctcgcgaaatgaacctcatcgaaaagaagaaactcaacttcacgctcagcaccagcaagccgggcacgcagaaagaaaccgacagccgcgcatcgaacaacgaagacgcggacgccaccgacgataccgacacggagaacgacgatgaatgaactgctcgcgatgcgcatggcgctcatcgagggattcaacggccgcccggcgttgatcgaccctcgtgatgtcgagaaggtcgcaacgctgtgcatgacgatggcgcaggcatctttcccgccgaccgccgagcagcgcgcgcaggcggatgaaagcatcaccgccgctgtcgagaaggcgttcgacgtttccttcccgcgcgaccgtgccaagccgttccttttcagcaacggccttgccttcatcccgatgcgcggcacgctcgtacatcgcaacggcgacccgtggtacggcacgcgcggctacgacgacatccgccgcgagttcgacgccgcgatggccgacccggacgtggcgggcgtcgtgttcgacatccactccggcggcggcatggtctacggcaacttcgagctggccgagcacattcgcaagggtcgcgacacgaagccgtcgctgtctgtcgtcaacgcgggtgcgatgtcgggcgcgtattcgctcggcagttccgcgaagcgcatggtctcgacgccttcgggcgacagtggcagcattggcgtgctgaccatgcacgtcgacatgagcaaggcgctcgaaaagttcggcgtcgccatctccctcatccatgccggcgagcacaaggtcgacggcaatcccttcaacccgctgcccgacaacgtgcgtgccgacatgcaggcacgtctcgacggcatgtggcagaagttcatctccgtggttgctgttaatcgcgggatgtccgaacaagcgattcgcgacacgcaagcccgtgtgtatcaggcggacgatgcggtcaagatcggcttggtcgatgcggtgatgtctccgcaagacgccatcgctaccttccgggccgaagtcttcggctctaccaccaacgataggagtgcaaccatgagcgacacgaagaagaccgacgccaccgtcgagcagaagaaggacgacgcgcaggtcgagaacaagaccaccgacgccaccgtcgacgcgggcaagaagaaggacgagcaggtcgatgccggcgcggcgatgcaggcgcgttgcgccgccatcaccggctgcgaggaagccaagggccgcgaaggtctggcgaaccacatcgcgttcaagaccacgatgtcggtcgacgaagcgaagtcgatgctggccgcctcgccgaagcagtcggccgccaccggcaagtcgccgctcgattccgcgatggacaacagcggcggcggtgccgacatcgccaacaacggcggcgacgaagaagagcaggcgcgcggcaacgacgacggcggcctgctgggcgcgtacaccgctgccaccggcaacaaggccgtgctgaaggtcgtcaagtaaaccgaacaccgtcgccagcctagacggaaaaaaccggctaaaccgtcaatcacagaaggagtaacgaaatgaccaacttcggccccatcgctggctacgtggctcgtaccgacacgaacagcatccagctctacgccggggaagcggacatcgtgagcacgcagggcgcgctcgtcaccggcaccgcctacgtcggcggtcaggtgctcggccgcgtcaccgcttccggcctgttcgccaagcacgacccggccgcgaccgatggcagcgagaacgccatcgcgatcctcgcgtacgacgtggcgaccccgactgccgacaagaaggaagcgatctacgtcggcggcgtgttcaacatggaagcgctgaccttcaacgctgccaccaacaccgacgccctgaaggccgctgcgttcgatggcaccaacatcgtcgcgcagaagctctacggtgcgccgcccgccggctccggcccggtctaaccggcatcaccaacagcaagacgtttcgcaattcaactcagaaatagaaggagacaacgatggatttgttcagcactgcggaactgcgcaaggtgatcgtcgacagccggccccccgtgcagtatttcctcgaccgtctgtacaaggagcagatcaacttcacgaccgaagaaatcatgttcgacgagctgaagctcggccggcgcatggctccgttcgtggctccgaacgtgcagggtcgtgtcctgaagcgttccggcttctacaccaagtccttccgcccggcgtacgtcaagccgaaggacgcggtgactccgggccgcatgctgcgtcgcctcgcgggcgaagcactgaccggcgacatgacgcccggccagcgctggcgcgcagtggtcgccgcgtaccagctcgaccagcggaaccagattttccgccgctgggaatggctgggcgcgcaggctgcgctctacggtcaggtcacgatttcgggcgaggactacccgaccgtcaccatcgacttcggtcgcgccgccaaccacacggtcatcctgaccggcaccgcgctgtggaccgaccagaccaacagcgatcccgacgacgacctcgaagagtgggccgctcgtgtgcatgacgccgaaggtttcgtcgtcacccgcgtcacgatgggccgcctcgcgtggaaggcgttcaagaagcacccggtcatcaaggagctgctggaaacccggcgcggctcgaagtccgaagccgaaaccggcccgggcctcggcgagtcggtggagttcaagggccagatcggttcgttcaacatctacgtctacaacgacgtgtacgaggacgagaccggcacgatgcagccgatgatggacccgcgcgacgtgctgctcgaagccgaggctggcttcgacggcgtgcgggccttcggtgcgatcatggatgcggacgccgaccttcaggcgctcgacatcttcccgaagatgtggaagaacccggacccgtccgtgatctacctcatgtcgcagtcggctccgctcatgatcccgagccgtccgaactgcacgctgcgggcgcgcgtcgtcgcgtaagcgtcgtcgcacacggcaagcccggttcgccgggcttcgctgtggcaacacaactccccaaccgaaagaaggagcatcaagatggcgaagtacaagttcgtggcccgcgtggcgctgaagggcgatttcgacgccgaagacggtctcggcaccgcgttgcaggaagtgcaggcgggcaccaaggccggcaccgacgacaagaagctctacgactcgctgctggaacagggctacatcaagtccgcgaaggacgccgcgaaggaagaggacgaggctccggctgcgtcgtcgaacccgagcaccgcgccgaaggtcgagtcgaccgacgccggcaagtccagcggcggcaagcagggcgcgggcaagtaagcccggcgcgctgaagggagaacgaaatgggctggctcgaaaccaagcagaaggctcggcaaaccgtgcatagcacgtttggtctgccggcccaatttcgcccgaggtcgggcggtgctgtcgtcgacggcaccgctcggctgcactacaaggtccgcacgttcggcgacttggaccgcgaaggcttcgcgaccgtcaccgaggcagtggactacatcatcatcgacactcggattttcgtgggcgctgacgaaggcgaccgcgtgttcttcccgcaactcaaccgcgcgttcaagctcgatgtgcgcggcgaagcggaagacgacattttcatcaagtgggaagtgagcgaggtagcgccgtgacggtcgaggttggcttccgtggattggatgacgtgcgcaagcgcgtcgccggcataccggaaacggtagaccgggcatccgcgtttgcgatcaacgaagcggtcacgttcggtcaggccgagagcagccgccgcatccgcgagcaggttgcgttcaaggccagctacatcggcagctcggacgatccgaacgctcgcctgcgtgtgtcgaagaaggcgcgcgtcggcgacctcgaaggcgtcatcgccggccgcatgcgcccgacctcactcgcacagttcatgactggcgcgaagctcggcaaaggcggctacgctcgcgtcaaggtgtcggcgcacggtgcagcgcgtcgaatcccgaatgcgttcccgatgaagctgcgtcgcggtaccggcgtctacgacccggagaacgcgaacgtcggcctcgctgttcggttgcaggacgggaagctgccgggcggcatgaacaagaagcagatggtgcaggtcagcggcaatctctatctgctgtacggcccgtctgtcgatcaagtgtttcgcgatgttcgagtcgatgtgcaagcgccggtcggcgacgtgctcgaatcgagcttcctgcgcaatttcgggagattgaaccgtggctgatacgaagcgcctgctgctgctgaagagcctgtgcaactacctgctgaccgaaatcacgacggcgaacggctacaacttcgacctcgccgccgcgtatcgcggcaagaagaatttcggcaaggaagtgaagctgccggcaatcgtggtgttggagaacttcaacccggatcgtctgccggagaccatcggcggcgtcgtcggcaccaagcacaagtacgaccagatttacctcatcaacggatgggccgaaggcggcgatgtcgagcaggaagaggactcggctcatctactcatgggggacgtgaagcaagcgctcggcaagctgctggtgccgcgcaatcaaagcgggtttttcgatggtctcgcaaacacgctgtccatcgagcccggggttgttcgccctcccgacgagcaatccgagaaggcgtatttctggatgaggattcgtctggaagtcgtcgaaaaggtgggagacccgtactggattcgtgattaaccgttgtatcgacagaaggagaccgtaaatgggcagcgagaattacacccttggccgtggcgaactgcacttcgacaagttcgtcgccggcacgttcaacaagaccggcgagcgttacctcggtaacacgccggagttgaaccgcaccaccgagagcgaaaacctcgatcacttcaacagcgaccgtggtatccgcgtcaaggacaagagcatcgtgctcgaaaagaacgacagcggtacgttcatcgccgacgaaatcagcgacgagaacatcgccctgtggttcctcggcacgcagaacgtcgtggcgcagtcggcgtccgcgagcgtggtgcagaacatcccggccaaccgcgtcaagccgggcacctacatccagctcggcgagtcgaccgccaacccgaccggccatcgcaacgtgacgctgaccagcgtgaccagcgatccggttggcacgaccttcgacaacctgaccgactacacggtcgacgccgagctgggccgcctgcacatcgtgccgggcggggccatcgacgggaccgccccgctgatcgtgacctacgccacggcggcctcgacccgcacgcagatcgtggtcggcgagggcaccaccatcgagggcgcgctgcgcttcatctcgtacaacccgaccggcccgcgccgcgactactactggccctacgtgcagctccgggccgatggcgacttcgcgatgaagggcgacgaatggcagcagctttcgttcgcattcgacatcctgaagcgggacggctacgcttccgagtacatcgacggtcgtccgaccgtggcgtaaccggggtacgtcaaacgcggtcaaggccaacttagtcaagatcaagcgagccaagaccaacttcgacaggccgcctcggaacccccggggcggcctgtttcgcatcaccagccagaagaggaaagtccatgtcccttgccaacctgcaactccgcactgcaaccgttccgtatgtcggcgcgaacgatgagccgcacgacatcgtgctgcacggcctgagtgcgaacgccatcgccggtctcatcctgtcgcagctcaacaacatcgaagaaatcttcaacatcgtcgaggcggccggcgtcaagaagaccgaagacctcgcgaacgtcaacatcgccgaagtcggccagcggcttctcgtgcagctccccgacttcatcgcgcatgtcatcgcgtactccgcgcacgagcccgagcagtggagcaaggtcatgcacctgcctgcgcctgtgcaggtcgattgcctgaccaagctcgccaagctcacgttcaacgacgaggccggcttccgagaattcgtgggaaacgtggtcgcggcactgcgaagcgcaaaaggcgtagtgccgcagactctcaaccgaaatctcgccgccagcgtttcgctgagtggtggctcggaatccgcgcagccgtctctttcctgacggcggaaggtcactcgaacgctggcgaatatccgctcgggtatttgatcgtcgaatcggaaatcgcacgcgagcgggtgaacaacagaatcagaaccgagatgacgctgacgcagagtgcgattgcctcggcgctcagcaagaaagcagcatcggcattcaaagaaaacatcgaaggactataggcgatggccgctcagaacgaagttgaactgattgtacgtgcgaagaatctcagcacgcgaaccatcaaccagctcaacgacgagctgagcaagatcgcagataaccaagagcaagtcgccgatgcgaaccgactggcggagcggtcgttcgagagcctgaagtccgagcagcagcagttgctcgcgatcatgaagtctctcaatgaccgcgcttccaagctggacgcatactcgcgtcaagagcaacaggtgcgtagcctgcgcgacgagctgagtcgcgctcgcgacaacctcaacacgctcgcgcagcagttctacaacaccgagaagccgacgaaggaatttcagcagcagttgaagtcggctgcgagcgaagtcacccggctggaatcgtcgctgcgcaacaacgagcgccgactcgacaccaccggcaacaagctgcgcgacatgggcgtggatgtcacacgcttctcgcagtcgcagcaggaagtcaatcaggcgctcaacagctcggtggcgctgtacaagcgctcgaccgacaacgtggagcgctacgacgcggccatcaaggaagtgcgcacgacgcagcagcaggcccgtgaggccgagcgcgccgcagcgcaggaagccaaggactcggcggcgaagctggaacaggccgcccgcgagcgcgaagaccagatgcgccgcgaacagaaaatggccgagctgacggccaacgtctaccgcacgctggcccgggagaaggaaaaggcggctcgggccggagcggacttccgcgccaccggcacgcaggcgctcgccacggcccgcgcgaccgccggccctgccgtgggtagcgggtcgtctgccggcgcggctgctgcgggcgtacaggcgcttctcgacccggccaaggatgccgtcgcgacgctcgaccggctggaaaaggccgtcgaacagctcgacgaggaattcaaggcgctcacgccggacgctttgcaggccgccgatggcatggacaagctggccgaccaaagccgccggctgcgcgctgcgtcggatgcgctgaaggggcaggccgggctcgcggatgaattgaaccgccagaacaccgtgctgctcgccagccagcagcggttcgaggaagcgcggcaagaagtgatccagtacgcgcaggcggtcgagcgcgcggacaagccgaacgacgaactggcgcagtcgttgcagcgcgcgcagaacgagatgaagcaggcgcacggcgagctgacgcgccagaccgaagcgttcaatcgcgtgcagcagcgcgccgctgccgctggcatcacgctcaacaacctgaccggcatcgagcagcgtctcgctcaggccgccgggcgcgtgcgcaccgggcaggagcaagtcgcgaagacgatgacgcggttggagcagacgaccgcgaagaccaacacgcagttgaagctcttcaacgacgggcagcgcaccgcgctctcgctgtatcagcgcacccgtggtcaggtgctctcgctagtgtcggcgtacgtcggcgtgttcggcgcgatcaacctcgtcaacagcgcgatggacgcagcaatcgagaaagagcgcgtcatgtcgcgcctgctcatcgcgaacaagggaaaccagactgcggcggcggaagagtacgactacctgcgcaagaaggctgacgagctgggcgctgcgttcggccctctcgccgagtcgtactcgcgattcgctgtcgctgcacgcgacgcgggcatgagcaccgaggcgacgcgctacatcttcgaggcgttcaccgaggctgcgaccgcgatgcggttgagcggcgacgaaacggccggcgcgttccgtgcgttggaacaaatcttctcgaagggcttcatccaagcggaagagctgcgcggccagttgggcgaccgcatgaccggcgcgttcaatctgttcgcgaaggctatcggcgtcacgacgcaagaactgaacaacatgctcgaaaagggcggcgaagtgaaagcagagttcgtgctgctcgctgcgcagacggcccgtggtatctatggcccgcaagcgaaggctgcatcgaacagcctgctcggcgacctcaaccgcatgcagaacgcatggggcgacctgaagcgcgaaatcatcgacggcggtctcggtgatgcgctgcgccgcctgttcgtcgacttgacgaagtacctgaagagtgacgacggcaagaagttcgccgagaacttgacgaaggtgtttgtcgctgcggccgacgctggcggcgagctgctgaaggtgcttgctgagaacgatgaagtcatcaagctgctggcggacaccgttgcgttcctcatcaagaacttcaaggcgctgctcgcgatcatgctcgcgatccaaggcgcgcgcatcgcgctggtgttcacgcagctcgcaggcgaaattctgaaggcgcgtgcagcgacactcgcgttgaacactgcgctcggtgcaggcaccgccgcgtcggcgggccgtgccggtgctgcattgggcggcctcatctccgggccgattgccgcgatcctcgccatcgctgctgcgggcatcatcatcccgatctacttccagatgaagggcgagctggaatcgaacagggtcaaggtcgacgcgcagaagacgatcaacgacctcaaccggggcttcgaggtttcgcagcgcagcctcagcgacacgtcgaagaccaacgccgaacagctcgaacgtcaggtcacggccgcacagcggttgctcgacatctacgacaagcagaaggaatcgttgcaggcgcagattcgcgagaacactgctgtgcgccgcaaccaagtggcggtacgtgttgcgcagggcacgcgcgagcacgacatgaatttcccggccaagcagctcgccgccgttcgagaagtcgagaacgaaggcaaggcactggaagcgcagctcgccgcgctcgaacagcgtgccgcaccgctgcgccagcaggtcgccgccgccagtcgtcagatcggcgaagcgaaagcgcgcgaggcggctgcggagaacgatgcgctcgcagccgagtttaggcgcatccaagcagcggccgatgcggctgcggcgcgtgccggcaccgacgcaaaggcagcgaaggcggccgaggctgcacgcaagaaggcagaagccgaagagaagcgtctggccgcgctcgccgagcgccgcctgcgcctggaagaggacgtggcggaaaagctgcgcgacatcgacaacgacattgcggcgtcgcgcccggatacgctcgaagcgcgtctggccgtgatcgacaacaagatcgcggatcgcaaagccgaactggaacgcatgctgcgcgaagccgacaagctcggtcagtcggatgcagccaagggcgaaattcagcgcggcctcgacgcactgccggcgttgcagcaagcgcaggcgcaggcgaccacacaggagttctacgagcagcggattaatgacttgttgcagcagcgacaggcgtcgatggatgcgatcaacacgttgcaggaagccggcttgctgactagcagcgaagccgccgcgcgtatcgaggaagtcaacgctcgcctgctgccgcagctcgaagcgttgcgtgcgaaggcggccgagttcatggcgacgctgggcgatggtccgcaggcgcaggccgcgcgcgccagcctcgaaaacctcagcgcgcaaattcaggcgatgtcggtcgagctgtcggcacagaagcgtcaggtcatcgacgtgttcgtcaacggcttcggtcaggcgttcatggagaccgcgacgctcatctccgacacgctgaagggcgtgcaggatgccggtgacgcatggaaggcattcggcgacatcgtgctcaacaccatcgccgacatcctcatccagctcgcgcagatgattattcagcaggcgattttcaacgcgctgaaggcggcggccgagaacagcggcggcggctggggcgcgatcatctcgcaagtcgccgggtacctgcacgttggcggcgtcgtcggttccggcgctggccgtcgttcgtcggtgccgtcgtacgtgttcgatgcagcgccgcgctatcacaacggcggcatcgcgggcctcgccccggatgaagtgccgaccgtgctgaagcgcaacgaggaagtgctgaccgagaacgatccgcgccaccgcttcaacggcgggctggaaggcggggcgcaaccggcgatggacgtgtccatcatcaacaccatcgacagcgagagcgtggtcgctgccggcgcgaacacccgcgcaggacgccagtccatcttcaacgcaatcaaggctgaccgcagctcgtacaagaaacttctcgcataaggaatcaacatgggacacgcaattgcaactgtgactggcggtagcggcgacgaggcgcactacaaggtgctcgctgcgatcaagacgctcgccgaagcgaacgggtggacgacgctgcgctacgtcaacaccggcaccgttcgcgagttgatcctcaactccgctggcctgtcgggaaccgaggacatctacatcgggttccgtacctacagcagcgtgagcggcgactactacaacatgctcgtcggtacgttcaccggctacgtctccgcgaactcgttcgactcgcagcccggcgcgaagctgagcggcgtgccttgccacaacaacgcggtgacgtatttcatcactgcgaacgcgcagcgcatcgctggctgcttcaaggtcggaactccggtctacacccacttctacgcgggcaagatgttcccctactcgcgtccgggcgagttcccgtcgccgctggtgtgcgccggcatgttcgacggtgccgcgccgaagcgtttcagcgacaccgactatcgctttccgtaccacggtcgcgagtcgggctacacgggcggctcttcgtcgaacgtgcgcccgtcgtacctgtggctgcgcgatcaagccggcgcgtggcgtcggctctcgcacttcccgttctacaacggcccggccggcagcgattcgtcgagtgcctacaacgcgctcgaaaactggaattatttgaccggcggcgatcaatcgcgctcactcgttccggccggcacgaactatcagccgcagcctatcatcctgtacacgaccagcgcaccggccggcgtatggcaaggcgcggtgtacggcgagctggacggcgtgtacgcggtgtcgggcttcaacaacaacgtcgagaacgtgttgcaggtcggcggcacctacgtcgatccggcgggcctgagcgtcgtcgatcacgttgccgcgatcctcgctgccggcggtcgcgcgttcgtcgtgctgcaagacgtgaatcaaaccgactggcgcagctttatcgctttggagatgacctaatggcttactacaccggcaacttttcctcgttcgctacgctgaagaactcggtcgagaccgcgcttcaggcaaacggctgggggctcaacggcgacggcgtgctggaaaagaacggcatgtacctgcgcctcactgcgaccgctgcgcaactgctgttgcaggcaggcacgggcactgcgactggcgcgctgccgggcgcagctccgaacggcgtcaagatcatggacttcgagggctcgccgatgaatttcccggcgacttacgacctgcacgtcaacactggcccggacgaagtgttcctcgtcgtcaactacaacgccgacaagtaccagcagctctcgtggggcaagtcgaacatgcagcagatcggcggcaccggcatgtggttctcgggttcgttccacgagaacgctgcgtcgaatcagaaccatctcgtctacacgaacgccgatgcgagctacttcggcttcggttggtcgggcatgggctgcggcctgttcgccgagtattacacgcaggcgctcggctgctcctacgtccacacggggctcgactcgaccgcgtggcgtcgtgtgtacagcggcgacggcaacctcgtcggctcgggcgatcctgttgccggtctgctgcaagcgctgccgtcgatgttcaaccaaaacaccgtgctgctgccgctgctggtctcgcagcgtcgactctcgcagggccagaccatcgtcgtcgacatggcgaacgcgcgcctgtgccgcaacgacaaccacctgtccggcgaaatcgtcgagtacggcgcggacaagtggaaggtgtacccgttccaccgcaagaacgccgacgtgcgcaacggcgtctcgtggtcgacgggcgcaaaccactccggcactttcgcatacgccattcgctacacggggccgtaactcatggcaggcatcaccggacaattcggcagtgaggtcgagcgcggcatcgctaacgtgatgctgagcgaagacttggacgacaacaccgaagtcgtctcgcggttcgactcttacgaaatgcgcccgggccttcaaggcggctacgggcgctggcgcgtgcatgccgacaaccattgggcgatcaccggccagcgcaagtcgaccagcttcttcgacgactactacaaccgcatctacatcgtgccggccgcgctcgatgccggcaacctgctgtccacgcaggtgcgccacatcatcctgtggaacgcctacgtcacgccgcagacattggagaacgccgcgctcggcccgcagtccggcatctcgatgtcgttgccggtcggcgtcagcctgccgtacgagatggaaccgctgcgcgagctggacttcaccgtgcagatcgaactcagcggcccgccgactatcgacagctacgcaaacttcaccgttgaaggcgtcacctacaccgtgccgatcaccggccggcgcatcgtgctgttcccgttctcgccgaattggggctcgcctgttgacgagacggtcacgatgcgttcgtgggtgttggccgccgaggatggcagcgagcagaccggcagcgagtcaggcgaggttccgcgccgtacgctcgaatacaacatcaacctgcgcactgcgttgcaggcgcagcgctgcgagaatctgctgttcgcgtggcagtcgcgcttcttcggtgtgccgcattggggcgaggaagagcgcatcgcagccgacgtggcagcgggctcgctgacgattccgttcgacaccttcggcctgtctctcgaacccggctcgttggtggcgctctaccgcgacgacgagaagaacgagattcgcgaagtgcagtctgtcgctgtcgacggcgttacggtcacgaccgggttggagtacgactggccggaaggctcgcgcgtctacccgtgcttcgtcggcctcatgaacgatgcgatgagcggcacgcgcgaaacgtcgaaggtcggccgcatgcctatcgcgttcgactgcgagccgagcgtgaccccgggcaacgtagcgctcaacgcgccgccgctgacctaccggggcaaggagctgtttctcggccgtaccaactggcaatcggcgatgcccttcaccttcacgtcggatgtcaagcgcgtcgactcgaacaccggcaagttcgtcgcgttctcgtcggccgggttctcgaagatgtctcgccggcacaactggacgctgtacaaccgcgccgacattttcgagttccggcagttcctcggtcgccggcaaggcgtcgcgcgctcggtgttcatgccgagcggcacggtcgacttcaacatggccgcgccgatcctcgacaccgaagacatcctcgtggtcgagaacaacgagtacggcgcactggctggcgcacacccggcccgccgagacatcatcatcgagctggtcgacggcacgtacttctgccggcgcattgtcggcacgagcaacttcgacagcttcacccgactgcaactcgattcgtcgctgggcgtgtcgctcgacatcgacgacgttgcgcgtatcagcttcctcacgctgtaccgtttcgagtcgccgtcgaccaccatccgccacctgaccgactcgaaggctacggttgaagccatcatggtcgccaagaccaccgaggattgaaatgagcctgttgcaatacgagcaagacaaggaactcagctcccgtgtggagctgtacctgttcgagagcgacgacggccgctaccgctgggcctacaccaccgacgcgcgcgaaaaggtgctcggccccatcgtctacaagcccgagtcgatcaagcgcggcgagctgaagcagacggccggcgacgcgaacgtcgagaaccttcaggtcacgatgccgttcgataacccggtggcgctggcgcatgtgccgtacctgccggcgcggccgatcaagctgacgatctacgcctaccagcgcaacgatcctgctgcggaaatcgtgcaggcgttcaccggcttcatcaccagcttcaaccagaagggcgcggaagcgacgctcgaatgctcgcagatcatcgacaacctctcgcagacggtaccgtgggcggtgttcaagagcggctgcatttgggcgctgtatcaagtcggctgcggcgtcgacaagcagttgtggaagaacgacgcgctggtcacgaccgtcaacggctcggtgctgggctcgcctgagttctcggccaagccgaccggctggtacaccaacgggttcgcctacaacccgcagacgggcgagcagcgcttcatcgtcgcgcacgacgccgctgccggcacgatcacgctggtgtacccgttcctcgaaatcaacggaagccagatcatcgaggtctacgccggctgcgcgcgcacgaaggaagtgtgcgccgacaagttcaacaacaagctcaattatgtcgggttcgatcacttcccggcctacaacgtcttctcgcaggggatcacctaatggtttgggtagccatcgtagttgcgctcgtcatggcggtagttggcgagctgcttcggccgaagccgaaattcaacgacccgaagccttccgctgtcggcgatttttcgttcccgactgcggacgcatcgcgcgtcattccgatcttcttcggtacctgcaagatgcaaggcccgaacgtcgtgtggttcggcgacctgacgatcatcacgctgaagaagaaggtcaagaccggctggttctcgtcgaagcgcatcgtcaccggatacaactactacctcggcgtgcagctcgtgttcgcctacgggccgtgcgacgagttcatcgagctgcgtatcgacgacaaggttgcgccgatcaccagcaagaccttcactggcgacgtgtgctcgttcacgatcaacgcgccgacgattatcagcaacgacgacccgccgaacggcgtcaagggtccgtgcaagctgtatcgcggcactttcgagcagccgccgaatatgtacctcagcacacaatggaacgagccggagatgaccgcgttccgtccgttgctgcacatggtcatggagaagtgctacctcggcaacaccgacacgccgccgcccatctcgatcatcgcgcgccgctgcccgaaccagctcggcttgaccggcggccggcacaacgtcaacggcgactcgaatatcgcgtgcgcggtgtacgaggtcatgaccaacaatatgtggggcatgaaaatccctgaagacaagatcgacgtggactcgttcatcgcctgcggcaacacgctggccgacgagagcatcggcatctcgatgctggttcagaccgccatgctcggccgcgacctcgtggcggaaatgcttcggcacgctgacggcgtggtgtacgccgacccggttacgggtctgtacacgatgacgctggcgcgcgagattccgtccgacgagcaagacgagctgttgatcgtcgacgactcgaacatcctgcccgacaccttcgagttctcgcgttcgtcgtgggagatgacgaagaatacgatcatcgtgcagtacaccgaccgcactacgttcgagacgacgccggtccagtaccaagacctcgcgaacatcgacgtgcgcggcggcatgatcgactccgaggaattcagctatctcggcttcagcaattcgaccgccgcgatgaacaccgccgcgcgcgtgtcgaagatgaaagcgtcgccgctggtgtcggcgaagatgtcgctcaatcgcatcggctaccaactgcgcccgggctccgcgttctggctgcgcaagccgaaccgtggtctagcgaacgtgctcatgcgcgtcatcgaaatcaactacggcacgctggacgacccggccatcaagatcacggcgatggaagacatcttcgcggtcaacgccgtggcgtacgtgccgcccgacccgagcgactggacgccgccggtcagcgctgtcgtgccgttctcgcagcagcgtctcatcgaagcaccagccttcggtgccgaggatatgtcgcgccgctatgtcatcacgatgggcgtgccgtcgagcaacggcgtgatcgcgtacgacgtgtggacggataccagcggcggcacgaacttccagcagaccaactctatcgacgcgctcacgccttcgggcgtgttggtgtcgggtctgtcgcgtactggcccggaagtcgatgctgcgggcttcaccgtcacgtcggtcgtcggcgtcagcgacatcgaagccggcactgcgggctcgcgcgagtcgggcgaaaacctgctgctggtcggcaacgaactcatggcatggcagaacatcgtcaacaacggcaacggcacctacacgatcactggcgtgtatcgcggcgtgctcgacaccatgccgcaggatcacggctccggcgcgcgcgtctacttcatgtcggaaggcgcgggcacgaccaacgaggacggctatggcggcgacctgacgctcaacacgaagctgaccccgaagagcattgtcgacacggtgccgctggacaacgctgcggcgatgtcggtcacgaccaacgctcgtgcgctgcgtccgctgccgccgggccgcctgcgcatcaatggcgcggtcgtgggctccggcgcggcttactcgaacgacatgctgttctcgtgggcgcatcgcaatcgtctcgacgacagcatcgcatcgcaggccgacccgagccgcacgcccgaggaaggcacgacctacaacatccgggtctacaccagctcgaatgcgctgctggcgtctgcactggaagtgtcgagcgcggcgtcgaccggcaccatgcggttcgcggtgtcgggcgatatgcgcattgaaatcgaggcggttcgggacggctacgtgtcgtggacgaagctggtcggctacttcagctatactccggccgccggggctaccgccaacgaaatcatcgtcgacgaacccgagtacgttctggacgggggtggcgcgtaatggcacaggtagtcgttgcacaacgcatgtggcagcgccgcgacactgcggcgaattggtctgccaagaatccgatccttgcgggcggcgaaatcggcgtgcagctcggcgctacttcggacgagaccaagttcaagatcggcgacggtgtgaccccgtggaactcgctctcgttcttcgagggacgactcatcgaaatcggcacgggcggcggctacatccgctggcgctatgtcggcgacgagacgtggatcaatctggtttcgctcgaatcgctgcgcggccctgccggcgcgaacggtgcgcaagggccgcaagggttgagcgcatatcaggtcgcggtcgccaacggattcgccggcacgcaggccgaatggctcgcgtcgctgaagggcgagaagggcgaccaaggcgatcaagggccgcccggcattccgtcgcagcgtcgcattctgcgcatcgctaacaccgacaccggctccatcgtgtgcgactggaatgcctacgacgaaattcgcgtgacactgactgccgacacgctcgtcaacatgacgggcgcgctggacggtcaaggctgcgtgctgctgctgaagcagggcggcgtcggcggtcatggcgtttcgttcggcagcaacgtgcgcttcaacaacctcatcccgatctataacccgacaacgactgccggcaagtccgacaggcttggcttcgtctatgacgacgacgccggcttctacgacgtgcaggcaatcgtggatggaatctgacgatggcagacgactacatcccgccgttgtcgccgaacatcgtgtgggtcttcaagggcaatgactacacgcccccgttgaccccgaacatcgaatggatattcggtgcagatgatgaaggcggcggaaacgagcttcgcaaatccacctacatgctaatcctgacaatgtgaggtattgaaatgactgttcgcatctactcttcttccgacgctggcgctccggttcttcgcggcaacacgccgggcgacctcatcaacctgctcgaaaagtgcctcgtcaccggctacggctcgaaggccggtgcaggctggacgaagccgtacaccggcacgaacgtcgctgcgttccagcaaggcgcaggatcgaacggcatgttccttcgcatcgacgacaccagcaccgcgaccagctatcgctcggccaaggtgaagggctacgaagcgatgaccgatgtcaacaccggcaccccgaccccgttcccgactccggcgcaaaaagcggacggcgcgtattggttcacgcactacagcagcggctccgtcgcgaacccgcgcccgtggcgactcatcgcggacgagatgttcttctacttcatgctgtcgacttacccggaaaacaacgacagcggttactactacaacgagtgctatgcgttcggcgacatcatcccgtacaagccgggcgacacgacgcacaccgtactgctcggctcgtggcaggaaacgagtccgaacacttcggaaggctacccgtggtacggcgtcgacatcgcgagctacatgggctcgaatcgctacgtgcttttggctgcacgttcgttcactaacctcggcggcccgatctacctcggatggcatagcgaccacacgaaggggagttcgagctggggttctggcaggctctcgtacccgcatggcccggacggcggcctgtacctcgctccggtgtgggtgcatgaagcgcacgtctcgccgtacaacgtgcgcgggatcatgccgggcctgtgggtgccttgccacaactcgggcacgttcagtcaattccagacgttcaacggccaaggcgagttggcgggcaagcagttcatggcgcgcaggcactacgaccagaccgtgtgcttcgagatttccgacacttgggataggtaacgcgcgatggcgctcatcttcaacctgccgatgacggggccgaatggctccacgacaatcaccgacaccacggggaacttctcgtggtcggtgacaggcaatgcgcagattcaatcgaacgctctcgtccttgacgggagcggagattatgtgagcacgactgctgacgaccgcatgcggctcggagcgatcaacaatttccgcctcgctttcgacatgaagatggcgtcggcggacagcagcggctacaagatcgttttcgatcaactcaatactggcgtcagcgcatggacatggcaggtctacatctacaacggcgtgccgtatttcaacgtctaccatccgagcttcggcaacccgacagtcgtacaggggagcgcaagcatagcggacggcaactggcacacggtcgagttcatccgagctaacgggtcgatgcagttgtgggtcgacggcgttgtggtgtcgtcggctgcggataaccgcgactacatcatccaatcggcgttcggcatcggttctcgcatcggctacaacgcatcgtctgcttatgactacaaaggcgaactgcgcaatctcagtttggaaatcaccgagccggtagtgctgaccggacgcatcgctgcgtggatcaagcgcaacatcatcggctgggatcgagcgcgtactcgcagttatattcggcgcagcgtcttctacagcttcccgccgctcgaaacgaagatgcgctcgtacgtccgcatcacgcgcggcgtgccgccgtggtgggggccgagcggatcgaccacgcagctcccgacctacaagctacgcggccgggtgatgcagcgcgatcctgacggcgtgttgcccgacgccccggtacagtacgcgcgcgtcgtgctgttcttccggcgcttgcatacgctcgtagacatccagctctccgatgtcgacgggtacgtgcaattcgataacctcatgccgggcggtcaggcgtactacgcgattgcattcgacccggaaggcgcaccgttgcagaacgcggtgatttgggatcgactgtcacccgagcccggcccgtaaggagaagtgccgtgagccagaacaacacccacgagcggaacaggaaccgacgagtgacggacaaggcagggggacttttggacgccgcgcagcaggccatccggcttgaacgcatcgaaggcgatatgcgtctgctcacgcagcgcgtcagctccggcatggagaacgtcagcgccacgctcgcggctgtgcaggtcgaagtgcgcggttgctcgacgaacgtgtcagagctgcgcgggctgcaaggtgcgcacgactcgaacaaggtagcaatcgacaaggtggagaaatcagtgaccgacctcggtgcgcgcttggagtcgtggttcgatgagttcgaggcgaagcaagaacagcggtggcgcgactattcgagcaatcgcgatcaatggcggcgcgagcacgaggccgagaacgagaacgtcaagaaggacttggaaaaggaaatccgcagcgttcgcgaaaccgtcattcgcttcatcgggttcggttccgccatcggtgcgcttgcgggcgtgatcgtcggcggcttcctgtggaatatcaactaccgcttcaacgaccaaaaagaggacgtgacccgagtcgaacaaacgtcatcgcgcaaccgacaactcatcgaccagatgggtgtcgatcacggcaaagagctggccgacatcaagctctacctcgcgcgcggcgggcgaatccccgctgagccctatgtccctcaatcgcaaaggaaccacaatggaaacgaacaagactccggccaacccggaaagtgaaatgcccttccgccgccgcgcgtgggagttctggcggcgcaatcaaatcctgctgctgcaactgccgctcatgctggtcttcctcatcggcagctacgtcgtgctgaagtcggtcgactcgcgaatcggcgtcgagggtttcggcgacatcttcggctacgcgctcaacggcgtgcgcatcacgctcatcatcttcaccgcatggtggatcaagaagtggtgctggttcgacctgcacgacaagaccgagctggcgatgttcgaggcgatgaaggccggcgactggatggcgttctggatcgtggtgcgcgaccgggccgagtggctggcggcgctggcgttcgcgaccttctggtacacccgatgagcgcccgggtcgtagtcctcgctgcggccctcctgctgggcgcatgcgcccggccggcagcggtacccccggtcgaccagaccacgctcccgccggccgtggagagcctgcctgcggccacgccggagccggtcgtcgagcaggtcgtcgcggctcagcccctaccccgggccgagcaggctgtttcggagaccgtcacggagccgcttctggccgcgcaggcggcgctcgaagaccttaccccgctactacccccgccgccggcccgggacgcggcttgccggcgcgctgcggcggccctgacgctacgctgggaagtgaccagcccggccttctaccggaagcggctcgaactgccgatctggccgggcggggcgtccggggtgacgtgggggatcgggtacgacgggggccaccagacccgcaccgtgatcgtcgacgactggcacgaccacgggcaggtcgaccggctaggccagaccgccggcatcatcggccagcaggcccgggcggcgctgccgcgcttccgcgacatcccgaccggcttcgaccatgctagtcgcgtgttcgaggaacgcagcctcgtcgaatacgaacggcgaaccgagcgcgcgttccgcaacggcttcactgagctgcggccgaacgcatgcggtgcgcttatctcgctggtgtacaaccgtggcgcggcgatgaccggcgactcgcgacgggagatgcgcaacatccgcgacaactgcgtgccgaagcaggactacgcctgcatcgctgcggagattcgctcgatgaagcgcctgtggcgtggcacggtcaacgagaacggattgtctgcgcgccgcgaggccgaagcgatcctcactgaaaccccgtagggagaagagcatgtggacgaaagcaatcgcgtggctgttcggaacggcaatgggtcgcggtgtgctgcttggcggcagcatcgcgataggcatggcgctcggctggtatgcgttctcgacgcactactacaacgagggcgtcgcgtcgtgccaagctggccgcgccaccgatacgaacgcggccaacgtcgcgcaaggtgaaaagaacatcgccgacaaccagaccagctccgacatcggcaaggccgccgacgccgaagcagcgaaggtcgcagccgatgccgaagaagcgaagaacgactcgaaggagaccatccatgacgtgtacaagaagccccctgtcactgcgcctgttgctgttggttcttgcgtgcatcctctcgatgagcgggtgcaagaccggatcggcaaagcgcgagctgccgcagttgaagcaagaagccccgctcgttaactgcaagcagcctgcgtcgccggcagtgccgcgcgagccgaaggccgacgagtggatcgagtggaacccaccgcgtccgggcaagaccgaaggcgaggcccggctgagcgaacgtgcggtgaactggatcatcgacgtgctgggcgtggtgcgagtgagcgagggctaccgccgggtcgagcacggatgcctcgacgagctggaagcgaaagggctcatccggcagtagttgacaggcccgaggcgctgcattacggttggtctcgctggtggcacttcgcgttgcatcggcactcggcagagggacagcggcgcggagaatcggcgctccgcaccgcagggaacgaggaaccccggactaacactccggggtttcttttttgcgtcaagaccaagtgcgtcgtgaccaagttcgtcaagaccggaaaagagaaaagccccggtgctgaggccggggcttttcgggttgcgcgactcacgtcgggcggtgggtatcgaggcgggggttctgctgattccggtgtccgctctatgagcgctgcgccggctggaagggcatgtgtcgcgtcgatggatcgaacctaatgcggcacgccgcgcgtgtcaacaccttcgtcagtccttccacgtctcgacgagcttcagcatcttcttgcgcgccttctcgacgccggccgcccacttgtcccatgcgcgcgggtcgacgtgcgtcaggatttcgttgcgcgccatctcgctcagcacggtcggcggcagcgcgtccagctcccagctcttgtcgccgaagcgctggcggtatttcacgaagcgcgcgtcggtcgtcttggccgggttcggcggcggcttcagctcttcgatctggtcgaggttgagcgccatgcgcttcagcgtgaactcgccgttccaaccgaacagctcgaagcgctcttcgaggtcgcgcgtcatgtcgatgccgctcggatcgtggtctccgaagtgcaggatcacgacatccttgccgtcgctctgttcgatttcccgcttggcgaagtcgcgcacgacggaagcactcgggtagccgcgcgctgcgagcagcggcacatcgaactcgtggcatacacgctggaacacgccgaccagcgcttctttctcgacgacgaggaaaatgcgtgcgtcctgcgtcgcccacgggtcggtgtggtactgccgcgccgacgccgtgagaatgtcctgcggcttgttccaacggctgcgctgctcgaacgagcgcgtgcggtcctcgatggcgtcccaatcaatcaggccggcgatgcgcgcgtcgttgacgatgctcgtcgtctgcttgtaggacttctcgttgttcggaatgatgtcgcgcgcgacaagctggtagtagagctggcgcacggtcagcgtgtacccggcgtcgagatattcttcgatgatcgcgttgatcctgtcgatctgttgcagggtcttggtcttgaaggtgatttctttgtagcgttcgaggctcatggcagagggttcctgttatcggcgggtcttggtttgttcgagcagtcggtcaatcttgcgggtcagcctgtcgaactcttcgtcggttggcggcggcccgacatcggagcagtcgtagtgcgaatggtgcagtccgttgcgcgcctcgccgtcgagaatcggcttgcagcacaccgagcacgtatccgtgtcctcggcatgctcgatccgctcgcggcgctcatcgcggctgagccgccaaaattcaccggcagttagcggtttcatgcgcgcgggcaccgttcgggctgaccgtgtgctgcggcgtagcaaactccggcttcgtcgcagccaacacccatgtcgcagtgcgtgcttttagccttgccttccttctgtgcgcgaagttcttcgcggatttccatgagcagcaggccgagatggttctcgcccttgccgtcgcacacgccccaaaacttgtcgccccaccagttgccttcgaccagcttcgccttgccggttttcagcagcttcgacttcagcggatcggtgccgaacttctggcgaagcaggttgcgcatcacgtcgatcttgaccgcttcccaatcctcgcgcagcgtgacgtgcttgcctcggcgcttcgccccggcggcgtcaccttcgttgcggatgcgccgccgctcgtcctcgtcgaacgtcttggcggcttggaaggcgtgctcgaccgtgcggtacgagtggccctcgaaagcgatgcagcacgaccagaaattcgagaggaagcgatacggcccggaaaatgcagcgatggttttcatggtcatcccctagtggtacatcttcgccttgccgaacaactcgcgttgcttcgtcatgtcggtgcgggcgatctgctcttggatgggaacctgcacgttgcgattcatcatctggtgcaggtagcgcggctcgaccgcgtgcccggtcgcgaacttcgcaatcgccatgagaatttgcggcgagtgcagctcgaagaacgtgccggtcatcgcccaatggtgcgggcggatgtgcgcagcgatgtcgagcagttggcgctcgaccttgcgcacgttgatcggcggcgcgatgccttgcctctgcatcgagtgttcgacttcgctcgccgcacgatgcacgacgaggtactgcgcgcccgggaagcggagcagcagttggtcgaagaagaacagcgccgcgacatccgatacgaacacgcggcccggcggcagcttgtcgatcttctggcccagctcggcgatgctcgcgcattgctgcaacggattgtgcagcgacgcagcgcacagcggccgaaggaactcggccatccatgcgctgcggctgcgcggaagcgacagcatgaaggtcaagtgctcgtagctcatctcaatcctccaacgccacgagcagcaacgagcacttcagccccatgcactcgccgcagatgcacgccgtcttctcgtccgacagtgagcgcgcgaggtcgttgtccggccccatgacctgcgccagtgcagcgtgtccgccgagctgcaattcgagcccgtgctgctgcatgatcgcgttgtggtctaggccgaattgctcgaccttgacgcggtagaaaacgatgccgccagcggcgacaccacgttcgcacaggacgcacttcgagatgtccttgcgcttcagcccgggcctgtcagccatgtccgctctccttctgttcgcgcttcgcctgtgcggtctcgacgtagttgtcgagcaccttgacgaacgcatcgtggagcagcgacccggccggcacgtagatcaccacgccgccggtcaagtcgctgcggttgtatgtcgtcggcttggcgtcgagcagttgcccttggccttccggtgtcgcctgcatgcggtccggcgggcgcacgtcgaactcgcgcaccatgccgtccgccgggccgccgatgaagaacgccctcatcgcacttcaccgtcgccttgcagcgtgccgcgttccagccggccgttgagcttttcgcgattgccgaagagcaactgctcgtagccatcgtcgaagcccaccagaggcccggtacgctcggcgaactcgaccgacacgttgaccagcgcttgcaagtggaagcgcatctcgtcgagcttggcggcgcgcttgtcggcgttccacgttgcgccgtcgcgcatcatcttcttgacgacgcccagcacgtagcccgagtgcatgcacagcgctgattgcaggtcgtagccgctgatacgaacttcgcggtactcggcgtcggcgagacgctggaaagcgacctgcaccatcgcgtcgaatcgcggcagctccgggctctcggcgcacagccgcgcgatgtaccactgcacgtcgcccagctcgctccatccttttgcgtagcgttcggcacgcaggtcttcgcggacggcttcttggtcgaacagctcggccagctcgccgacttcgttcgcgatgccgatgctggtgtacagcatgccggcagtgacgttgccggcgagctgcgcgatgtcggtcgggtacttggccgtggtgatggtgaacgccgcatacgcttcggcgaagatgcgcgtgggctcgacgcgcgcggcacgcgactcgcgtgcggtatcgagggacaggatgctcatgcgcggcccccggcggcgagcgcgtcagcgaagtcgttgctgtagctggcctcgaacttcgtcgccatgtcgtgcaggacgagcgtggggccgccgtgcgctgccgggatcatggcgaagtcgacgccgcgcaccagcgggttgcgctcgccgtcctgaccgatggcatgcacgaccaacgcttcggggttctcgcgcgcggcgcggcgctcggccttcaggatgcgccgcatggtcttgccgccgaacgccttgcgcagcttttcctcgggcgagccgtggtcgcggatggcgagcacgccggcaatgccgcccttcgacgtgcgcacctgacgcttgttcttgcgctgctcgttttcgaggtcgcgctgctggacgaggaaggcgtagttctcgtcgacggcgagcatgcgcttacgccagtcgctcagggtcttgtccttctcggcattgtaggaacggaaaatgcgcttcaacaggttcatcgtgtggctccttcaggtgtgaaaaaagcggcccggccgatgtcgacagggccgcttcgatgtactacgtcaacgccaccggactcagcggccggcgacgaacttggtctgcttctgcacccggccgcgcttggtctcgcggaacagcacgatggtcgtgttgtcgtcggccatgatgctcgcgtcgtcgagcgcgttgctctcggtcgcgaacgggccgttcatggtgctggccttctgcgagccgtcttcctgcgcggtcagcagcaggtacgcgaactgcttcgcgcccttcttgccgcgacgcacgccgaccttgcgggcagcggtcttcttgccggccgggcgaccgcgcttcttggcgggcgcggcggcctcggtcttcttcgcagcgcgcttggccggagccttcttcgcggcggccttgcgtgcggtcttggcgggagccttcttggtggccttcttggcagcggcgcgcttcttcgcgaccttgccttcggtggcttcggcgttctcggacatctggtttctcctagcgttgttgtcgacaactcgcggaatgcgagcggggttcccttgcgggattcggttcagtccacgcagtacgcggggacttcggtgcggaacgtccggcactcggacggctgcgtgatgtacaggccggcgatggcggccagcagcaacacgccgtaggcgatcttctcgcggcggctcatcactcgcagcccacggtggcgttcgggcgggtcggatgcgcggcggtgtactggctgaagtcgcgccagccttccgagccgccgcacgcgaagccccagcggcgcacgatggagccggtcatgaagagcgtccagcacggctcgtcgttgttgccgaacagttcgagcaggtgcatgtggtcggcgctcaggcggcggaagtcgcccgtgtggaagtgctgcgtgtagtcgaacttgtgctggcccgggaacttgcccttgttgcgcaacacgctgccttcgacgaacgtgcggccgtcgttcggagtgaacagtcggtgcatgtacgagacgtgcgcgtccatgccttcagggctctcgtcgatggcgtgctcgtagcaccactcgctcgtgtgctcgatgtagcgaccgtcgaggatgagcgacgcactagcccacgggtgatcgtgcagtgcgcggtcgtcgtcgccatgcacgaacttgtgcaggtacaggttgaaccagcggttgcgcgggatgatgtgccagcgcgtcaggtacgggcggcgcgggccgccgtcgatgccgtcgagcatgatgaccttggacggcgagacgatgcgcgcgtacagcttgaacgcgccgacgaagagcgaccacaggccgatcatcgagagcacgttgtagaagcggcgggagacctcgggggcgttcatggcggggaacatcctcggtatggtggggtaattcatgcgtcgagcgtcgcgtcggcggtggccgggccatccgcgttggtcgtgtcgacctgcgggcgaacgagcgggagcggctgcgagccatcgagattcttgaactcgatgtagtagcgcgtgttgagcgtcttcagtccggtgtcgacacggttctggaagacggtcagcagttcggccttcgtcagctctccggcgtgcatgccgccttcggagacgacgcggaagttctcgatgtcgccgctcgtcagtacggcgaggttgtggcggtcgaggatgagcttgtccagcaagtcgcgaatgttcggcagttcggcgaagtcgattttcattgggttctctcggcgtgagatgaagagcggcgtatcgtgccgcaagccgccgggttgacccttcaagcgctggggagtgcgccatccagttgaccgggggtatcgcctcagcgaccccgtgcagttcggtgatttaccccgtagggggacgaagtaaattcgttactgcggggccactctagcgccagcttttcggcttgtcaacacccttccttgtgtccggcggccggctcagccgggccattttccgctcgccccggaagagcctgtcgcgcagcatcttctcgctgacgtgcgggcagtgccgcttgatctgctcgaaggtcatctcgtccccgtcgatggtgtacagccgcacgcgcgcaacctctttcactgcgtagtcctcgtcgtcgaatttctgcctgctcatagcgcccgcccgtgagtctggatgtagatgtcgtgcagcatctcgtgcgcgattgctttgcgaaacgcttcctgctgcacgagtgcatgtgcgaagtcgcgcgcgctcggttccttcatgccgagatgcgcggtcatgcgcagcgcctcgtcaatgatggcctgcggttcgccctcggcgtagccctcgtcggcgagcagcgcatggatggcttcgcggtacttcgcgtgtcgcgcgcgctgccgcagcatcgcgatgccagcgatgacgttggggccgatcaccagcagcaaccaatcgaaccagctcatacagacctcgcgtgtggacgctcttcgccttccttcggcgcgggaacgtggtggagtgtttcgagtcccttcttgatcttcgccgccatcgccttgccgaactccgacgcatcgccgtacatgaggtcgaggtcgggatcagcgcattcggcggcgacgttgcgcagcgtgtcgaccagcatcgggagttggtgctgcgcgctgtagttctggtggatcatcggccacgcgccctgcgccttccaccactgcttgcgctcgtgctcggtcagcgcgacgtactggtcgatcatcgccatcgcgaggaacggcgaccagaagcacgtatcgagcggcgtgatcggctcgcccagctcatcgagcgcgaagtacaccgcgaagacaggcgtggtgccgatgaggtagaccggctcatcgagcgggtctttgtaggtggcgatggtgcagccccggtacgcggccatgtgtgcgtagcggcgcttgctggcgtcagggagtggcatgcggaaactctcgttgaagtacgggtcaagggacgctgaggcgtacaagcacgcctgcttgggctcaggctgtgcagctctcatggcgacgaagctgcgctcgctcatgcgccgccggcatcgcgcacgagcacgacttcgccgccctcgccgtcaggcaggcatgcagccagtacgtcggccgcgccctgcgtgtcgccgagcacgagcagttggatcgcggcgcggatcgcggtctcggtctcgatggccttgcgctcagcggcgagcacgtagccagcaccgtcgcacagctcttcgagcagatgccgcaaccactgagcagtcgtgaggtctttgcggtcgagcgtcacgccgtacttcttcaggccggcgtcggcgcgctgacggatgatcgagatgaggtcgttcgtggtctgcatgtcgctcatgtcacagctccgaagttttcttgccggggttgcggcggtgccattccagtttcgcgttcgcttctatctgctggcgcgacaggcgggggctcttggctgcgagttcttcgcacagcgcatgaaaacccgggcggcggtcttcctgcatctgctggaactcggacagggtgttcttcttcagcatggctagaactccttgtggaaatctttctcggcccggatgagagccgaaaccttggggccgaactttttcggcgtgtcgagcaggatgtcggctgcgcccatcgcgatctgcggcgacacgaaatagccttggatcggatgcagcacttcgccgaagtcgtcgacgatgtagtacgcgagatggatgccgacgccatcgagcacgatgagcgggccgccgtcgctgcgcacgtcttcgctgtgcagctcggcgatgaacacgtcgcggtacggttggatgcgcttgaacttcatgcggctttgtccttcaggtggtcgagctgccagccggcttcgattgccgcgaacagccgcagctcgctcgcgtcttcggtgtcgagccgcaggaactcgatgaagctgtcgatcatctgcggcgtcatcgggcgcttgtcgtagaacctgcggtacgcgctttgcggaatcatgtcccacaccgggcacaggtcgacgatgcgcttgccttcctcgcgaagatggcgacgcatgatgtcgcgcaccgtcttcgggttcttcttgaccgtgatcttgcggccggtcgacggacggaaactcatagcccgatgtcctcgccagcctcgcgcttcagcaaccacatcggcttgcgcgaaagcatcggcagcgggccgatccatccgtcgacgagaccgtggtggcgattccagccgtagttgtcccaccagcgtccgcgcttctggcccagctcaggaacccacacagcaatctccatctccttgtgcgccggcagcgcggtcgggaacgggcggtgccagatggcgtagaagccgaattccggcgggtcttcgagcacttcgatgtcgttgtactgcatcggcccggcccagccgagcacgagcccgttgaagggcacgaacggcttttgcaggctcggtcgacgctcccaccacatgccgttcgcccagcgcatcaccgagtacatgcgcgggtcatgcacgatggtcgggttgcgcgtcagctcgacggcgtacagcccttcgactgtcgggtcgtcgagcacttcgagttgttcaatcttcatcgtgcggagcctcaacgtgcgcgcgtagtggccgcaggcgcggcagcgggccgatccagccgtggacttctcccctgaagtattggtcgctgttgagatagcaccagcggccgttgaaccacatgaggaagatgtcgacgacgagcccgcgaccgtgcgggtcgtctacgcggcaagcgtagacgcccgtgtcctgcggcagtccgatttcttcgtactgcaccttcacggcatgcacttctcggcgtaggtgcggcagtcgcgcatgaagtcgatgtagacctcgggcggcaggtcacgcatcgtcgtcacgccgaacgcctgcatgtgggccttcagcctgtcggtgccgtggatgatgcggaacagccgcgcgtactcgtacaccatctcgcgcatgcgatcctgctcggtacgaatgcgctccggtccccacgagccgccgcgttccttcttcagcgcgtcgacttcgcgcgtacgcgattcgagcgtggcggccaacttcttgttctgctcgcgcaggtcgtcgttctccttgcggccgtgcatgcgcaccagcgtgcggatagcacgaatcgcgaggtcggtctggttgagcgtgggtccgctggtcggctgcttgtcccagcccggcagacggcgatgcagttcatcgaacacgcgcacgaggtcgaacaccgctgcatcgtcgatggcctcgaacgcctcgtgcagcttgcgcccggcctcggccgccgctgcgctcgcttcactgacctgacgcatagcgtcgccagcgtcgacacgcagttcgacctcgacggtcttgcgtgcgttgccttcgtcgtctgccggccgccatgttgcgagccacgtcgcatggtcgcggtaggtgaacttggtgcggtggccgtcgccgtcgcgctccatcgtcacgtagtagtccgtgctgtcctgcttgcggcgcgcgtcgatcacggtgtaggtgccgcccgagatgacggagaagtagcgctcgccagcggccggcggttgctcgctgccgtcgaacggcacgttctcgatgaagtcgcggaacagcgattcgatgaggccgtagcccatgccgagttcgggcggcatgccgacgcgacgctcgcgcgcaggcttgaacgacacgtcatgcagctcggcggccatctgcgcatacggactgcccggcacagcgccggcagtcgtcggtgcgaacaggtcgttccacgcgctcgccgtggtgaacatccattcgtactcgccgccgcgcccgttgtcgacgcgcagcatgcgcacatgcgagtggccctcgcactcgtgcgtgctcacgaccatgaagaagcgcgccgggcggttgcgatcctgccagtaggtgccgaccttcggcgcgaactcgtagtccgggtggccgaccgtcactgcacgcgcttccttgcggtcgctcgcagcacccttggtcgtctgcgtgctgcccttcgagaagtcgcgacgcatgatgcgctcgatgaggctcggcgtgcccttcatcgcctcggcgatggcgtccgggctgaagtcgatggtgttgatgatgtggatttcgggcgcgctcgggttctcggcgaacgacggcgcaggcaccttgccgttgtgcgcattgaagaagaactcgtgctggccgacgaacgtgttgcgaatccagcggtgcatgcgctgcgcttccgcgcgctggatgtcgttctggccgacgatgccgccggcagcgtgcatgtcgcgcacgatgccgttgtcgtcgatgcacgcggcgaccgacacgatcatcggggtggtagcgtcgttggtgaactgcttttcggtatgacgagacattttcggcgtttcctcggttgggttaggtggtgctgacgtgaccggcggcctcgcggtcgagttgtaggtctgcgatgtcacgcagcgacgagggccagtcgtcgagcggcacgagtccttcctcgtgcatggtgatctggtcgggcgtcaggccgcacaggtaatacgccttcgcgagcgacatgccggcgatgagtcgatagcgcatagcggcgcggccatgcttgaaggattcgacttgtgcccgtgtcacttcgcccgtgcctcggcacagccggcacttcgtccccggcaagttgtcgtcgtgtcctgcgtcggggccgaacatctcgttgaactcgatcatgtcgtgccgcccttcgcagcgcgggcagacagtcttgtcacggagccaacgccacgccgcgcgcaccttcatccgcagggcggtacttactgcgcgaccgagcagggcggtagcggtgcgcagacgagacaaagggggtaccggagcattccgagaagccgcaagcctgcggcccaacattttcgcttcttcgatttcgcggcgtgtgtggcgcatggtgttggtcactccatccgggtgacagtgaggaaggcgaacatggcgtcgttgctggcgctcatgtaggtgccgcgttccatcttgaagcgcttgtgcttgtggtcgcccgctgcgcgcaccttcgcgatgccgccgctcaggatcgagttctgctgcttgaagtatttctgcgcctcgttgttgatcgcggcgatgttcccgttgtcgagcgggatgcgctggcagcgcgcgtgcgactcgccgatgtcgagcttgctgagctggtcgttgagcgagcccggcaggaagaccaaccggggcttctcgacgatgcgcacgcgcgggttggcgatgtcgctcttcttgatcttcgagcccgacttcttgcggctcttcttcgcaggcgcggcgctgctgttcgtggtggcggatgccattaggtgatgcctcctgttccggggaagtaagcggacaagaaacatactactgcgcgcacccggggtcgtgtcaacccgggcgttctcggtcgtgaccaactcgcgcgccgggccagcgccgcacaacgatccggctgggttgccgaagcgggcgcaatttcggaaccggctaggtcggcgaagcgagagcgcaaacggaaccggctggctttgcgaagcgggccgaattttggaacgggctgggtatccgaagcggggacgtttttggaattgctctcttacatgcacgcgcacacagatatgcacgcgggcacgtatgcgcgctcgcctgcgcacgcgctcgcgttctaagtcacgcgggcgcgcggcgcgtgcgggcgcgtcaaggttccgcgcgctgcgcgttgcgcgcggttccttcatccgggcgcgcttgccgccttccgcgcttcctgaatgcaaagtaaacggactactgcgcgcagtaaaaaacatcttgcgcagcgcgcgaaaccgtgtagcctacgcataccggcaacgtcgccggcatcgcaaagggtcgcaaacatggcacgcatgaaccgttccgaattttccgcccatgccgcgcttgccgcgtcgcgtggcgcgtccgctgcgcgcaaggtcgaaaccgcgcgcaaggtccagacgttgcgcgatttgctcgcgcgtcttcccttccttttcgccgtcgccgttgccgcctttgtcgcggtcgcggccgtcgccgtttccatcgtctaagggaatcacacaatgcgccgctatcttttcgtttcatccgctacgcttcccgtcgtcgcctacgcggaaagcaaagacgcgatgcgcgcatacgtgcgcgacctgctagggattccgtacggtttcccgctgccgcgtcatgccgtttgcagcatcgcttaacaattcactagacaaaggagattcaccatgcaacgcattagcctttcgcaagccttcgcacagtggcaagagctggccgcagacattccgcaagacgacgcgcccatgctggcggaatcgtggaacgattacacggattcgctttgcgaagatggcgcattgtgcgacctgcaataccactacgcgcccgcatacgatgaagagatgcccggcgacggttcgcgcttcgatccgctgagcgatgaccgcgaattcatcctagacgcaatgggcgtcaccatgcgcgcaacgcgcaaggatggaccgcgcgaaggatgggacgcgagcgcgtcacactggcgcgtcacgctgcgccgcgaccgcgcgagcatgacaacggattacagcatgggcgcggcgcatacgggctcgcctgagctggcggacgtgctgaattgcctaatgcgtgacgcggaatgcggcgcgcagtctttcgaggatttttgcgcggaccttggatacgacacggattcgcgcagcgcggaaaagacgtggcgcgcgtgcaaggtagcggccgtcgggctcgcgcggcttttcagcggtggcatgctgcgcgacctgcgcgaattgttcgaggatttttgaccatgagcgagctagacattagcgcggttgtcgccggcatgcgcgacccttggaattactcggcgagcgttgcggaacgcgggcaagatgccggccgcatgacgtgggaagccgcatgcgaggatgcgcgcggtttgttcggcgagcatttcgaccgcgccgcgttcgatgagtatttttcgcatttcggcgcatgggacgcggaagaattggccgcgcatacggatgaagaatgcgccgcgcttatgctgcaattcatcgccggcgacatgcgcgaggctgatttttccagctatgcggacatcgaaggcggcgcggaaccgttcacggatgaatggtggccgcagtatgaaaaagcgagcgaggccggaaccgtcgccggccgtttctttcgcgacgctggcggcgttttttactacctcggagaatgaccatgcaaagcaaatgggcaaagacaaccgcgcagcgcatcgcatccggcgagctggcggaatccatcatccgcaaggcgcgcgcgttgctgcgcgatgccgtgaacgctgaagagtatttcaagcgcgaaccgtcgccgtctgctaccgctgcggaagcgtgggagctggtggagatgattagcacgcatgcgccgcgcgtcacggatgcgcaagcgcgcaagggcgcggaatggctgcgccgccttgtctacacgtcgcgcggcacggtgcgccgcacggaagccgcgcagcaattcagcgatgcggacctgcgcgttttgcaggcttgcatcgcgcgcccggccttccgtctggtggagctggaaccgcacagcgacggccgatacctgcgcgaccttgcgcccgtctatcgctgcatcggcgacaacggcgaatccttcgattacacggcgagcgcgtggcagtctggcggcgcgttcgcaatcctgcgccacgcttaacccttcccatccgtgacaagcccggagaatctgaaaatgtacagcatcgcaaacaacgcaaagcccgccattctgacgcgcacggaatcgcgcatccaatcgcagcgcgacaagcgaacgcgcgacacggaagcgcgccgcgcaaagtatcggcgcaacgctgcgcgctatctggccgcgtctttctggcaagggtcgcgcgacatcgccgattttttcaagggtcgcggattcgatcatgcgacgttgcaggatgcggaaaacgattgcatggataacgtcgatttttcttatctgtattcccgcgactatgcgcgtgagctggaaaaggaatacggcgacgacgcgcgcgaattgttcgcgtacctttgcccggatgcgccgctgagcgtgtaccgtgagcaaatcgccgacgacatgacgcgcgcggttgcagactcgcgccgcgcggattatgcgttgcagtttttcgactggtgccgcgatgcggtcgaggatgcggccgattcttccgggcttgtctggtgctatctggacaaggccggcaagcctacggatcaggaatacgacgcgcacgcggtaggcttcgcatgctcgcgccgcatgtacctttcgcgcgacgcggaatggtggccggaaaaatggtgggcgaaaggcgaaacgacgtggaacgattacgcgagcaatcgcgaacgcatggacgcggccgacgacgtgctgagcgaatttctcggcgagcatctggaaagcgaaggcgcggaccctgaatcgttcgatgagcgcggttcgcgttatgcggacgatgattactggccggaatacttcagcgattacagcgaagcgcgcgaagaatgggaaggcgacaaagcaaagatgcgcgcgcgtctgcgcgagatgatcgcgaaccgtgcgccgctggaattgcgcgccgcgcttgtcgcgagcgtgtacggcgagcctgaccgcgcggccgatgaatccgaagattgaaagggagctaacgacatgacgacgattaccgcatacgcatacaatgccgcgcttcattgcccgcgctgcgccttccgttatttccgcgtcgatcctgcgaaggtgccgccgggcgcggatgcgctggacggttgcaaggatcgcgaagggaacgcgcccgcgccgctgttttcgacagacgcgaacgcggacggatattgcgacacttgcgacatggcatacggcgacgcggaaccgcgcgcgcacgtcctgagcgttgacgcatggcgcgacggcgaaggctggacatggaataactggcacaagcgcggcacggtgccggttgcatggtgcgacctgagcccgcgcgcgttgctgcggaacctgcgcgcgcacgggctcgacctgccgccgggcgcggtatgcgtcgaggatgacggatacaacgtcgagattcaggcgcgcggcacgcgggaaccgttgtatgccatcgcctacggcgaggcgcagcgatgagcgctaagcccggcctagcagaaaagcgcgaaattctgcgcgctggcattctggcggatcgcatcgaacgcggcgcgcgctggctttgtttcgctgccatcgtatgcgcgggcgcgttgccgctggcatggggagcgttccgggcgcatggcatcgttagcgggctcgccgtgctggcgctggtgctggcgctatgctggcacgtcaagccgcacgggcgcagcctagcggcgcaagcgcgcgagattgaagcccgattcaagccgcacgattaaaagcgcgctgcggcgcgttccctgcattgcctaccctgagcccggccgcgtgccgggctttttattgcctgcgcgcctaagcgcgttctagcggcttgccgggcgcacgtctgcccggccttccgtatcccttcgcttgagcccgtggccgcatcgcctgcggccgggctttttctttttcccgctgcccggccctgcccgggctcgcatgcgtgccggcctgcccgctgcccggccttgcatggtggcgggcttatccgctgcccggccttgcatgcgtgcggcatagctgcccggatgcggcaacgtggaattaatgcagcgctgcgccgcataggtgcgcgcgtgcggcctttccgaatttatttattgcatcgcatgcccgcatgcgtgcgcgccgcgctgcgcgcgttctagcgcggcaggaagggataaagggatagccgctaggcgagtaaaaaggtacttccggccttgctgcgagcgtcgcggggggcgctgacagatcggaataacgtcgggtaggtaaagagcgtagttat

SEQ ID NO: 14 - DNA, 55335 bp, unidentified
  source 1..55335: mol_type = genomic DNA
gggggcgctgacctcggtgctcgcgcatttttcggaattttcgcggtttcgtctcctttggacccccgggcggccccgaatttccgaatttattccccgaataaacgcgaatttcctgtgacagtagtgacagtgacgtttttgggtactgtcacaaattcggccccccaagaaatccgctcaaatcaacgatttacgggcgcgaatttactgcgagtttaggctcagtgacactgtgacagtgacttccaatcctttacggcggaaagaaaagttctgcctgccaagaaaaaattctcgcgtatgagagaaggtactgtcactactgtcactactgtcacaagatagggaaaaaggtatgtagatcaagcacttgaatttgtgacagtaccttgtgacagtgaccgatttgcgcctcggagagcatggaaaaccgggtactgtcacaagaatcggcctttttccgaatttccgcccatacggttgcaattttttccgtatgtgacagtgaaaagaattcggaattaatttaatcggagccgctgcggggcgtcgtgcggaaattcggaaattccgggcaataaaaagccccgggggatgagcccggggccggcactgcggaaattccgccgaattaaatcgcgctcttcggcgctccatcgcctacacgcacgtcctcgacgttcgagccgttgtcgcccgcgcccggcggaagcggatcgctctcgtagcggttcgcgtcggtgttgttttcgtcgacggtcgcgttcggcaccatgccctgcggcttcgacgcgccgaagaagtcgccggtctcgcgcgctgtgacctgcaagtcaccgtgcatcgtgatttcgaccgagcggccgggtgcatcgagcactgcatgcaccacgccgttgccgtcgaccaactcgaccgccttgttgccgttgacgtgcgtgaacttcacggtagtcgtcatgtcgtttctcctgtgctcgggattgagcgtcttcgatcatacgctcgcaggcatgaaaaagcccggttgcccgggcttcttcgatcacaccttcagcgacgtgatttctatgtagtcgtcgatccacgcttgaaggttcggccgcaccaccacgtcaggcgagcgtgaccaataccgggcctgctttccgttcgcgccgcgcgcgcggcccacgtacacgaagcccttcgaggtcaggaagttcgacagcttcggcccgtacggcacaccgacgctgttgtccatcgccatgtcgcgcagcttgccgacgttgagcagcaggtggctcacttccgggtcgcgcgactccgcgatcatctcttcgatttcgtcttcgtcgtcgccgcgcgcgaggtcgatcatgcgcgacttcgcatcggtcatgggcgcatggccgtccgggtcgaactcgggatgcagcgggtagtcttccagccactcgcggatcgcacccgggtgataggcgattgcgttgaagatgtcgtcgtagtgatccgggtggcgctcgcggaacttctcgatcatctgcttcgtctggaagtgcgtcgagatgacgaagtagcggcggtcagcgtcgtagaccggcagcgcgtcgctgtggttggtcaggatgatggtcgaggtcacattcggcacgttgtacgagtcgcggtgcatgcggcgaatcgaaaccacgtcgttcgtgatgaagggcttcagcttatccatcaccgcgtagcgcgacgtgccgtggatgcgcgcttcttccagcaccacgaccttgcgcgactcgaagaacgacgtgtacttctcttcgagcgcctgtgcgttcacggtctcgacgttgttgcgcgacatgatcgccatgagcatttcgccgacgaagcccttgcctgcgccgtccacgccctgcatcacgaccgcccaacggattttcctgtccatgcgcttgatcgtgtacgccagccacgacagcaggatttcgcgctcgcgttcgaccgggtacgaaatctcgaagtggcgcttcaccgcctcgaccgcgcgccgggccttgctggtcaacttgtccggcaccggcacgatgtcctcggcgttgaacttgttcgcgtgcttctggccgtcccactcgacgatgcggtctgcgcccggcaggtagacgtagccgctgacgacgggaatctggtacacgttcaacgcgagcgcggcggcctgctgctcaggcacggcttccatgttcgcgcggtccttcttcgtcagcaggaagcggttgttgcgtgcgttgaatgcgcgctcgctcagtgcgagacggctgtccatgtagtagaactcttcctcggcgtcgacgtacaccacgtcgttgcaccaatgcggcagctccttgtagttgaagtcggaattgcggaagccttcgttgatcgccttgcggatcatcgcgatgggaaccttcttccccagctccgcaacgcgctccttgatcgcgccggccaacagctcgacttggaactcgttctccaacatgcggccccacttcgccgcgagcgggccaagcagctccatctccgaagtcgtctcggcgaccttgcgcttgatcttctcgaactgctcctgcgagtgctcctgccgatgctccttcgccatcttgataagcgaggcggcggtcgtcaggttgcgacccatgtcgtcgtggaacgagttccacttgaactccaactcgtccgggtcgtagttgtgcgcgggctcggaccactcgtgccaaagctgcaagccttcttcgttgccgtcgaattggtgatgcagcgccatgccgaccttcaaccactgctcgtagtcgtcggcacccggcacccattgcagcacttcgcggagctggtcttcggtcaggttttccagcgggcgcttgtattccagcagcgcgttgtcgttctcgtcgtcgctgctgcgcgattcggtcggcgcgttgtgcttcttcaacgtccagccgcgacgctgcgcttcgagcttgaacaccgagaacagttcgtcgatgtgctcggtcgtgatttccggcagcatgtcggccggcacgctcagcgggtttagctccttgcccgaagtccacttgtacggcttcttggtgtcggggtggatgccgatgccgacgaactgttggccgtccgcgagcacttcgatggcctgctcatgaccttcggtgtcgaggaacgtgatcttacgcttctggaacggaatgtcggtgcgatatacgagcaacgtcttcggcgcacggccgactcgcgtcatcgtcttgccgatgatttcttccgtgtgctcagccatgagcgcggccatttcgtcatcggtgatgtcgatgtcgaccgcaggcgtgtgcttcgtgtggaagccgatgttgccctgcttgtagttgccattcgcccacttgcgaatctgcttctcgtccgcgcggattttctgccactgcggttcgattgggcctttccttcctgccgggatcggcaagatggagtacccgttttccagcaattgcgcgccgtacttacggagcacgctggtgatcggtcgtccagcagccataggtcactccgcgatgtcgtcgctaacaaggtcttcgaggttgaagccgatcttgcggttgaaatccttgtgcaagatggtcgccttgtcgcgcggcacaccgccgaggcgctgccaacgcgagacagtggtctcgtgccagttgtacttctcgcaaattgcgttgagccgaccgtacggcgggtcgagcatgagggcgatgcgccgaagcagatagcgcactcgcgcgtctgcgctgtccagtgaatcaagagtagggtctcggcgcatgaattcctcgcagacgttgggatttaaggggtctgctaagtcggtgagcatgcctattgacttagcatcgggacaggcgcatagtgcgctcgccgggcaggaattgcaatccacccgtcactcccgaaaccaacctagctaggagatacaaccgatgtcgaagatcaacgcgaagaagctcgccgaagccatcaccctcatcatcgaagcagtcggcggcggtgccgccaacgagtccgaggatgcgggcggcgaagaggaagcgccgaagaagggtcgcggccgtccggccggcagcaccaacaaggccaaggccgagaccaagcccgccgccaagggcaaggccaaggcgaaggacgaggacgaggacgaggacgacggtctcggcgacgacgacgatgccggcgacgacgatgacgacctcggtctcggcggcgacgacgaagaagtgacgcaggaagatgtcgtcaatgcgttcaaggcgctgaaggcgagcaagggcatcgacaagtgccgcgaagtgctcgccaagctggacgagagcaacgtgctcaacatcccgccgaagaagtacgccgaggcgctgaaggaaatcaaccgcgccgcgtcgaagaagtaactcggcctgcacgtcacacgaaacgcccgggttcgctcgggcgtttctttcggagaggaacacatgcccggttcgcacgcccgcttcgcaccatcgtcggcgcatcgcatctacgattgcccggcgagcctgttgctcaacgagaacgagcccgaccgcgaaatctacgaagcggccgagggcaccgttgcacaccacatcgcggaaatctgcgcacgcgcgcgccgcgagccggaagagtttctaggaatgacgttcgacagcggcgacctcgacgccgactacgacgaagagcagcattcctcgaaaggcttcgcaatcaccgtcgacgacgagatggtgcagggagtcggggcgtacctcgaccgcatcatgggcctgccgggcgaccactacgtcgagacgcgcgtcaacatctccccgtggtgcccgatccccgatcaattcggcacctgcgaccacgcagccgcgtcgcacaagaagctcatcatcaccgacctgaagtacggccgcgtgcaggtcgatgcgccgcagaacaagcagctcgtgatgtacgcgctcggcttcatcaacgagtacgactggctgtacgacttcgatgaggtcatcatccgcattgcgcaaccgcgcctcgatcacttcgacgtgtggatcaccagcaaggccgaactgctcgctatcggcgagaagatcaaagagcgcttcgcgcttgcgttgaagccgaatccgccgttcggcccgagcgagaaggcgtgccgcttctgcaaggtcaacttcaagtgccgcgcgaaccacgacttcctgtaccacgagcgcatcatgctgctcgatgacgacgacgagttcgtcgagcctgacctcatgctcatgagcgacgacgaaatcgctgcgctgtggctgcgcaagggcatgtacgagaaccgcatgcgcgcggtcgaagactacctgcacaagaaggtcgcggacggcgacttcgtgccgggcctgaagaccgtggcgggccgcagctcgcgctacttcaccagcgaaatcgacgccgagctgctgctgctggaagccggcgtgcccgagtctaagctgtactccaaacccgaattcgtgtcgcctgcgcaggctgaaaagctggtgcgcggcgaggcgaagaagaaattgcaggacttcatcaagtcgaagcccggcaaaccctgtctggtctcttccgacgacaaacggaaagacctgaccgtccagtcgctcgaactgctcgacgactgacgcaaccgttgtacgaatgcgcgaaagcgaactacgaacgtcgaatgacgaaggagaaatcgaaatggcgaagaagaaagttggtgatctggtcgacaagggcaatgggcgttttctgctgaagaacgtgcgcctgagcttcccgtacttgttcgagcccgacgagcaggaagacgacaacggcaacaagaagaagtcgtaccgcgtcaccctgctgctcccgaaggcgacgcacaagcccgtcgcgcagaagctctcccgtctcatctccgagatgtgcgaggaagagtacggcagcccgaagctggcggccgaccgcaagttcctgcgcgatggtgacgagtcggatgtcgaagatcatcacggctgctggacggtgacggttcgcgagacccggaagccgatcctcgtcgaccgtgatcgtcagcccaccgaggaagacgacgagctgctgtacagcggcgcgtgggccaacgtggtgatccgcccgtgggctcagaacggcaagtccatgaagaagaagaacaagtacggcaagcgcatcaatgccggcttcgacatcgtgcagttcgtcgaccacgacgacaacctcgcgggcaacgctcgcccggatgtcgacgaggttctggatgagctggacgacgacttcgcggatgacgacgacaacagcaccagccgcagcaagtccaagagcaagtcgaagggtcgttctcgcgacgaggacgatgacgacgacgggctcggcgacgacgatgacgacgaccgcagctcgcgccgcagccgtccgtcgaagagcaagaccagcagcaagagccgtcgctcgcgcgacgacgatgacgatgacggcgacgaggacgatgacgacctcggcatctaaaatcgggcatcggtaagcggtacctacggtcgcccgggcactccccgggcggctgtttttcagggatacggtatggacaagctgcatcacgacttcgagaccttcagcaagtgcgacctgaagaagcacggcttggcgcgctatgctcgcgacaagtcgaccgaagtgctgttcctgtggtacgcattcaacgacgaggaacccgaagtgtggttccccgcgacggagccgatgccgaagcgcctgcgccgcgcgctcaaagacccgaacgtgcagaagtgcgcgcacaacgctcagttcgagcgcgcgatttggctgcacgtcctcggcatcgacatcccggtcgagcagttctattgctcgatggcgcacgcattctggctctcgctgcccggcaacctcgacgaactctcgggcgtgcttcgcctcggcgagaacgcgaagatgaaggaaggcaagtcgctcgtgaagttcttctgcgggccgcgcaagccgacgaagaccaagcagtacacgcgcaacaccgcgcagaccgatccggcgaagtggaagacgttcgtcgagtacggccgccgcgacgtgatcgccgagcgcgcggcaggtcgcaagctctcgctcttcccgatgagcgatttcgagcgcaacctgtggtacatcgaccagcacatcaacgaacgcggcattccgttcgacaaggaattcgtcgagaccgcgctgcgcgtcatcgcgaaggagaagaagcgcctgctgggcgagatgagccgcatcaccggcctgagcaatcccggcagcggcgcacagttgctcccgtggctgcgcgagcgcggctacccgttcaccaacctcaaatccgcctcgatcaagaaggcacgcgaggattgggactggaacatgaccgatgaggcgaacgcggttctcgccttgcacgcggaagcggcgcgttcgtctgtcacgaagttgcagaagatgctcgacatcgaagtcgacggagtgctgtgctacacgatgcagttcgcaggcgcggggcgcacggcgcgctgggccggtcgcgcagtgcaggtgcaaaatttgccccgccccctccgcgaactagaagagcaaggggcactgctcatggcgcgcgatgcgatcatgcgcgaagacatcgagttccttcgcctgctggtgtcgtcgccgatgggcgcgattgcatcgtgcatccgcaccgcgatcaaagcgccgcccggctacgagtatgcaacgtgcgacttggcctcgattgagtccgtcgtcattgcatggctgtcgggctgcgacaagttgatcgaggtctttcagaagaacctcgacgtgtacaaggtgttcgcgtcgaagatgtacaaggtcgactacgagcaggtcgagaagtggatgcgtcaacacgcgaagcccggcgtgctcggcgcaggcttccgcctcagcggcggcatggagttgggcgagtacccggaagtcatcaagaccggcctgtggggctacgcggagaacatgggcatcgagatgtcgcagaaggatgctgcggccgtcgtgaaattcttccgcgaggaatacaccgaaatcgtcgagctgtggtacgagctggaacgcgccgtcgcgaaggtgatgaacacgaaggagccggtgcgcgttggtccgatcctcatggacgtgaagggaccgttcctgcgcatgcgtctgccgtccggtcgctacctgcactacctgcggccgaagatgatctggaagaagatcaaggtcggcatcgacaagaagaccggcaagccgaaatacaagtcgaagaagggcttcacctacgaaggctacaacacgaagaagaagtggacgcgcatcgactcgcacggcggcaagatcgtcgagaacttggtgcaggcaatcgcacgcgagctgctggccgccggtctgctgcgcgcttggaaggccgggctcgatgtgcgcatgcacgttcacgacgaaatcgttgcgctggtcaagcgcaagctgtcggacatctcggccgcgacgctcgaagagcagatggtcaagaagccgaagtggtggggcgaagacgttccgatccgtgcgaaggctgacgtagtggagtgctatcagaaatgagctggctgaccgattggcgcaacgtaatcaacggcaagccgccgcgcggcgacatcctgccgaccgacaagcatcgcgtcgaaaaggacgtggagcagaagtggtgcgccgttgcgaagcggcacggatggaaggcatacaagttctcgtcgcccggcaacagcagcgttcccgaccgcatgttcatccgcaacggcttcgtcttcttcatcgagttcaagcgccccggcagcaaggcaaccgacaatcaactcgaagagcacaaggagctgcggcgcaagggcatgatcgtgtgggtcatcgactacttcgataaagaattcgccgagtggatttttgaatgaaacaactactgaagcgctccgacctcgacgagtttcaaatcgctgccggcctgttcctcgaacgggtcggcagttgcgcgttgtggatcgacatgggcctcggcaagaccgtggtcgtgctcacgcatgtttcggacaaggtgttctccggcgagtggagccgcgtgctggtcgtaggcccgccgctggtcatctccgatacgtggtcgaccgaggtcaagaattgggagcacacccgcttcctcgactatcaggaactcgacggcgacagcgagcacatgcgcatgcagttgcagcggccgtgcgaggtcgacggcatctcggtgcataaactcgggcgtctcgcggcgctgttcaagcgaggcgacacggtgccgtgggacgcggttgtgttcgacgagtcgagcatgttccgcaacaagtcgtcgaagcgctggaagtacggcgtgcgcctgacgtggggccagccgaacgacgtgatcgagctgacaggtacgccgagcccgaacggcctgcatcaagtctggtcgcagattgcgatgatcgacggcggcgagcggctgggcttgacgtacaagaagttcctgttccgctggttcaagcaggagttcatgggccgcaaagtgattccgaagtcgcacgcgatggcgtcgatcacgaagaagctgagcgacatcgtgtacaccttgcgcgaagaggattacgtcaagttgccgccgctccgctctacgcctgtgccgatcatcctgccgccggatgtgatggctcgctatcaggaattcgagcgcacgtctgtgctgaagtggggcgaagagcaagacccggcagtgcgtgctctatcggaaggcgcgctgtacggaaagctgttgcaatttgcgtgcggtcgcatctatacggattcagagacgaaagagttcgtcgacatacacgacaagaagatcgagcgcctgaaggaaatcgtcgagttcagcgacggctcgccgatcctcgtggcacgtacgtggcagcactcgcgtgatcggctgcgcgatgagttcccgggcatccgctcgttgaagacgaagcgcgacctcgacgcatggaacgcgggcgacatcgagatagccgagacacaccctgcgagcatcggtcacggcacgaacatccagaagggcggcaacaacctcatctggtacgaccacacgcccgacctcgaactctacatgcagttgcgcaaacgactgcaccgacgcggccagacccgaagccacgtcaacatgatgcacctgacagcagtaggcactatcgaagaggatttgacacgcgagctggtcaagaaagaaattacccaagacgccctgagagaacccatgcggcgacgagtcgcagacgtacagagagaactagccaatggccgcacctaagatcgactacgaagaagagtttttcgacggcatgaccgtgccgcgtctggcgcagttgttccgcctcgaccgccgcactgttaccgagaagctgcgtccgctgcgaccgaccggcgaccggcgcggcgcaccgacgtatcacatcgtcgacgctgcaccgtacctcgtggagcccatcgtcgacatcgccaagtacctcgcggaagtcggccccggcgacctgcccgcaccgctgcaagcgcagtattggaacgcgcagaacagcaagttgaagtacaaggaacagtcgggcgacttgtggcgcacgcaacaggtgctcgaagtgctgaccggcgtgttccgctcgctcacgcaatcgcttcgcctgctggccgaccgcatcgaagcgcagaccgggctcacgccggagcagcgcgcgatcatcgagcgcgaagtgtcagacaaggccatcgacatgctgcgcaagcgccttgtcgaagacttcgagatttacgtcggcatcaaggacaaggaacagctcgccgacatcaagctcgacgacatcggcctcgacgaagaggacgaagaagatgtctgacggcagctttttcaacgacctcggcgagctggtcacgttcgttgccgatagcgttctggttccgccggagcgcttgaccgtttctcaggccgcagcaaagtaccgctacctcgacaacgaaggctcgttcgtcggcgagtgggacaacaacgaaacgccgtacctcgtcgagccgatggacgtgctcacgagtcgcgagttcgagtcgtgcatcttcatcggcccggcgcagggcggcaagaccgaaatcatcctcaattggatcgcatacaccgcgaagtgcgacccggccgacttcttcctcatccagaccgcgcgcgacaccgcacgcgacttctcgtatcgccgcatcgacaagatgcaccgcgacagcaaggagctgggcgcgatgctgcgtccgggcagcgacaacgacaacatcttcgacaagttctaccgcaacggcatgatgctgacgctgggctggccgacgatcaaccagctctcaggcaagccggtgccgcgcgtcgcgctgaccgactatgaccgcatgccgcaggacgtggagaagaacggcccgccgttcccgctcgctcgtaagcgtacgacgaccttcggctcgttcggcatgacgctggccgagtcgtcgccgtcgttcgacgtgaaagacccgaaatggaaggcaccgcacccggactcgcatatgttcccgccgtgcgatgggatcggcggcctgtacaacgaaggcgaccgccgttgcttctactggcagtgccctcactgcggcgagtggtttgagccgaagttctcgctgctgaagtgggacatcaagaaccccgacccgttcgaggctgcgatgtcgacgatgatggcgtgcccgcgtaacggttgcgtcatcgagccgaagcacaagtacgagatgaatcgacgcggcgtgtggctgcgagaaggccagcgtattgatcgcgacggcaacaagctcggcgtcggcgttcgctcacgtagcgcatcgttctggctgaaaggcccggcggcgcgcttcattacatggcagaccctcgtcgagcgattcctgcttgcgcaccagacgctcgaacgcacgggcgaaaccaaggcgctgaaggccacgatcaacaccgatcaaggcgaagcgttctggccgctcaacgcgaaggactcgaaccgcctgccggaagacctgcaatcgaaggcgatccagtgggccgacaagaaggtgccgtacggcgtgcgcttcctgctcgggactgtcgacgtgcagaagagccgcttcgtcgtgcaggtcttcggcgtcggcccgagcgataacggcgtcaacttcgacctgtacctaatcgaccgattcgacattcagaagtcgaagcgcaaggacgaggctggcgacacactatgggtcaagccgtatgccgtgcaggaagattgggacttgattaccgagcaggtcgtcgagaaggaatacgagctggaagacggcagtggcttcatgtcgatcaagatgaccggcatcgactccggcggtaagtcaggctcgacgacgcgcgcatacaactactggcgctcgatgcgcgacaacggcaacggcggtcgcgtgctgctcatcaagggcgagccgaagctcggtgcgccgcgtgccgaaatcgacttccccgactcggatcgcaaggatcgttcggccggtgcgcgcggtgaaatcccggtgctgttcctcaactcgaacgtgctgaaggacatgctgctcggcatggtcgactacgacgagaagacgacgctcggcggcaggcacttcacgaacaagtggacgccggaagttgtgtacgccgaactcactgtcgagttccgcgacgaccgtggtcgttggcagaatccggctaagcgacgcaacgaagcgtgggacttgggctactactgcctcggcctgtgcgtgatcttgaaggtcgaaggattcgattgggacgcgcctgagtcgtggttcgcggagtggagtaacaactctcttgtgcgccgtgtggatcaggaaaaacggtttgcgtcaagccccactacggattatggtttcgccaagttcgggaaatccttgggatgacaaatggcgaccctagagcagttgcaagcatggctggcggaagcgcaaaccgcctaccatagcgtcatgatcggcggcggcgtgaccgtcgtcgtcgaccagaacggggagcgggtcgagtacagccgggccaacgcaaccggcctcgccaaatacatagccactttgcaagcgcagatcaattccctattgggggtcgcagtaaccggcggcccccttcgtccgttcttctgagggtaaaacgacatggcaaaagcactcactgtcgtgcgctctcccgagggcgacgaagcgttcaacagcaccggcaaagagtcggcgttcggcggtgcgtacgaaggtgcgtcgcgactcaatcggcagaccgcgttgtggagcgcgccgtcgctgccggccgacatggagatttcgccggacaaggttcggctcgatgcgcgcactcgcgaactcattcgcaacgatggctacatccaaggtgctctcgacacgagttcggactccatcgtcggcggtcagtaccttctcaacgcgcgccccgattgggagacgctgggcctgagcgaagagtgggctgaagagttccagctcatcgccgagcgcaagttcatgctgtacgccgagtctccgatgaactggatcgacgcctcgcgcaagaacggtctgaccggcctcgtgcgcatggcgctcgcgcagtctttcatgtcgggcgaagcgctcgccgctgcggagtggctgtcgaaggcaggccgtccgtacaagaccgcgatcaacatgatcgaccccgaccgcctgagcaacccgaacgacaacagcgatacggcgtacatgcgtcgcggcgtcgaaatcgacaagttcggcgcggccgaggcgtaccacatccgcgacgcgcacccgatggagtcgtactacgaccgcttcggcgcgaagtggacgcgcgtgccggcgttcaagccgtggggccgtccgcagatcatccacatcgccgaagtgctgcgcccgggccagacgcgcggcgtatcgaagatggtcgcggtgctgaaagaaatgcgcatgacgaaggtctacaaggacatcgttctgcaaaacgccgtcgtcaatgcgaccttcgctgctgcaatcgaatcggagctgccgcgcgagctggtgttctcgcagctcggtgccggcgacatgggttggttgcagaagtacatgggcgcgctggctgagtatgtcggttcggccgacaatctcgccatcgacggcgtgcgcattccgcacctgtttccgggcacgaagctcaacctgcaaaacgccggccagcccggcggcgtcggcagcggcttcgaggactcgctgctgcgccacatctgcgctgcgctgggcctgtcgtacgagcagttctcgaaggactactcgaagacgaactactcgtctgctcgcgcgtcgatgatcgagacgtggaagtacatgcagacgcgcaagaagctcgtcaccgaccgcttcgcaacgctggtctacatgctgtggctggaagaggaaatcaaccgtccgaataccgacctgccgctgccgaagggcgcggcgcacttctacgaagggatcaaccgcgaggcgtactgccgctgcgactggatcggcgcttcgcgcggccagatcgacgagctgaaggaaacgcaggctgcggtgctgcgcatcgcgtcgggcctgtcgacctacgaggaagaactcggcaagctcggcaaggattaccgcgaagtgttcacgcagcgcgctcgcgaaatgaacctcatcgaaaagaagaaactcaacttcacgctcagcaccagcaagccgggcacgcagaaagaaaccgacagccgcgcatcgaacaacgaagacgcggacgccaccgacgataccgacacggagaacgacgatgaatgaactgctcgcgatgcgcatggcgctcatcgagggattcaacggccgcccggcgttgatcgaccctcgtgatgtcgagaaggtcgcaacgctgtgcatgacgatggcgcaggcatctttcccgccgaccgccgagcagcgcgcgcaggcggatgaaagcatcaccgccgctgtcgagaaggcgttcgacgtttccttcccgcgcgaccgtgccaagccgttccttttcagcaacggccttgccttcatcccgatgcgcggcacgctcgtacatcgcaacggcgacccgtggtacggcacgcgcggctacgacgacatccgccgcgagttcgacgccgcgatggccgacccggacgtggcgggcgtcgtgttcgacatccactccggcggcggcatggtctacggcaacttcgagctggccgagcacattcgcaagggtcgcgacacgaagccgtcgctgtctgtcgtcaacgcgggtgcgatgtcgggcgcgtattcgctcggcagttccgcgaagcgcatggtctcgacgccttcgggcgacagtggcagcattggcgtgctgaccatgcacgtcgacatgagcaaggcgctcgaaaagttcggcgtcgccatctccctcatccatgccggcgagcacaaggtcgacggcaatcccttcaacccgctgcccgacaacgtgcgtgccgacatgcaggcacgtctcgacggcatgtggcagaagttcatctccgtggttgctgttaatcgcgggatgtccgaacaagcgattcgcgacacgcaagcccgtgtgtatcaggcggacgatgcggtcaagatcggcttggtcgatgcggtgatgtctccgcaagacgccatcgctaccttccgggccgaagtcttcggctctaccaccaacgataggagtgcaaccatgagcgacacgaagaagaccgacgccaccgtcgagcagaagaaggacgacgcgcaggtcgagaacaagaccgccgacaccaccgtcgacgcgggcaacaagaacgagcaggtcgatgccggcgcggcgatgcaggcgcgttgcgccgccatcaccggctgcgaggaagccaagggccgcgaaggtctggcgaaccacatcgcgttcaagaccacgatgtcggtcgacgaagcgaagtcgatgctggccgcctcgccgaagcagtcggccgccaccggcaagtcgccgctcgattccgcgatggacaacagcggcggcggtgccgacatcgccaacaacggcggcgacgaagaagagcaggcgcgcggcaacgacgacggcggcctgctgggcgcgtacaccgctgccaccggcaacaaggccgtgctgaaggtcgtcaagtaaaccgaacaccgtcgccagcctagacggaaaaaaaccggctaaaccgtcaatcacagaaggagtaacgaaatgaccaacttcggccccatcgctggctacgtggctcgtaccgacacgaacagcatccagctctacgccggggaagcggacatcgtgagcacgcagggcgcgctcgtcaccggcaccgcctacgtcggcggtcaggtgctcggccgcgtcaccgcttccggcctgttcgccaagcacgacccggccgcgaccgatggcagcgagaacgccatcgcgatcctcgcgtacgacgtggcgaccccgactgccgacaagaaggaagcgatctacgtcggcggcgtgttcaacatggaagcgctgaccttcaacgctgccaccaacaccgacgccctgaaggccgctgcgttcgatggcaccaacatcgtcgcgcagaagctctacggtgcgccgcccgccggctccggcccggtctaaccggcatcaccaacagcaagacgtttcgcaattcaactcagaaatagaaggagacaacgatggatttgttcagcactgcggaactgcgcaaggtgatcgtcgacagccggccccccgtgcagtatttcctcgaccgtctgtacaaggagcagatcaacttcacgaccgaagaaatcatgttcgacgagctgaagctcggccggcgcatggctccgttcgtggctccgaacgtgcagggtcgtgtcctgaagcgttccggcttctacaccaagtccttccgcccggcgtacgtcaagccgaaggacgcggtgactccgggccgcatgctgcgtcgcctcgcgggcgaagcactgaccggcgacatgacgcccggccagcgctggcgcgcagtggtcgccgcgtaccagctcgaccagcggaaccagattttccgccgctgggaatggctgggcgcgcaggctgcgctctacggtcaggtcacgatttcgggcgaggactacccgaccgtcaccatcgacttcggtcgcgccgccaaccacacggtcatcctgaccggcaccgcgctgtggaccgaccagaccaacagcgatcccgacgacgacctcgaagagtgggccgctcgtgtgcatgacgccgaaggtttcgtcgtcacccgcgtcacgatgggccgcctcgcgtggaaggcgttcaagaagcacccggtcatcaaggagctgctggaaacccggcgcggctcgaagtccgaagccgaaaccggcccgggcctcggcgagtcggtggagttcaagggccagatcggttcgttcaacatctacgtctacaacgacgtgtacgaggacgagaccggcacgatgcagccgatgatggacccgcgcgacgtgctgctcgaagccgaggctggcttcgacggcgtgcgggccttcggtgcgatcatggatgcggacgccgaccttcaggcgctcgacatcttcccgaagatgtggaagaacccggacccgtccgtgatctacctcatgtcgcagtcggctccgctcatgatcccgagccgtccgaactgcacgctgcgggcgcgcgtcgtcgcgtaagcgtcgtcgcacacggcaagcccggttcgccgggcttcgctgtggcaacacaactccccaaccgaaagaaggagcatcaagatggcgaagtacaagttcgtggcccgcgtggcgctgaagggcgatttcgacgccgaagacggtctcggcaccgcgttgcaggaagtgcaggcgggcaccaaggccggcaccgacgacaagaagctctacgactcgctgctggaacagggctacatcaagtccgcgaaggacgccgcgaaggaagaggacgaggctccggctgcgtcgtcgaacccgagcaccgcgccgaaggtcgagtcgaccgacgccggcaagtccagcggcggcaagcagggcgcgggcaagtaagcccggcgcgctgaagggagaacgaaatgggctggctcgaaaccaagcagaaggctcggcaaaccgtgcatagcacgtttggtctgccggcccaatttcgcccgaggtcgggcggtgctgtcgtcgacggcaccgctcggctgcactacaaggtccgcacgttcggcgacttggaccgcgaaggcttcgcgaccgtcaccgaggcagtggactacatcatcatcgacactcggattttcgtgggcgctgacgaaggcgaccgcgtgttcttcccgcaactcaaccgcgcgttcaagctcgatgtgcgcggcgaagcggaagacgacattttcatcaagtgggaagtgagcgaggtagcgccgtgacggtcgaggttggcttccgtggattggatgacgtgcgcaagcgcgtcgccggcataccggaaacggtagaccgggcatccgcgtttgcgatcaacgaagcggtcacgttcggtcaggccgagagcagccgccgcatccgcgagcaggttgcgttcaaggccagctacatcggcagctcggacgatccgaacgctcgcctgcgtgtgtcgaagaaggcgcgcgtcggcgacctcgaaggcgtcatcgccggccgcatgcgcccgacctcactcgcacagttcatgactggcgcgaagctcggcaaaggcggctacgctcgcgtcaaggtgtcggcgcacggtgcagcgcgtcgaatcccgaatgcgttcccgatgaagctgcgtcgcggtaccggcgtctacgacccggagaacgcgaacgtcggcctcgctgttcggttgcaggacgggaagctgccgggcggcatgaacaagaagcagatggtgcaggtcagcggcaatctctatctgctgtacggcccgtctgtcgatcaagtgtttcgcgatgttcgagtcgatgtgcaagcgccggtcggcgacgtgctcgaatcgagcttcctgcgcaatttcgggagattgaaccgtggctgatacgaagcgcctgctgctgctgaagagcctgtgcaactacctgctgaccgaaatcacgacggcgaacggctacaacttcgacctcgccgccgcgtatcgcggcaagaagaatttcggcaaggaagtgaagctgccggcaatcgtggtgttggagaacttcaacccggatcgtctgccggagaccatcggcggcgtcgtcggcaccaagcacaagtacgaccagatttacctcatcaacggatgggccgaaggcggcgatgtcgagcaggaagaggactcggctcatctactcatgggggacgtgaagcaagcgctcggcaagctgctggtgccgcgcaatcaaagcgggtttttcgatggtctcgcaaacacgctgtccatcgagcccggggttgttcgccctcccgacgagcaatccgagaaggcgtatttctggatgaggattcgtctggaagtcgtcgaaaaggtgggagacccgtactggattcgtgattaaccgttgtatcgacagaaggagaccgtaaatgggcagcgagaattacacccttggccgtggcgaactgcacttcgacaagttcgtcgccggcacgttcaacaagaccggcgagcgttacctcggtaacacgccggagttgaaccgcaccaccgagagcgaaaacctcgatcacttcaacagcgaccgtggtatccgcgtcaaggacaagagcatcgtgctcgaaaagaacgacagcggtacgttcatcgccgacgaaatcagcgacgagaacatcgccctgtggttcctcggcacgcagaacgtcgtggcgcagtcggcgtccgcgagcgtggtgcagaacatcccggccaaccgcgtcaagccgggcacctacatccagctcggcgagtcgaccgccaacccgaccggccatcgcaacgtgacgctgaccagcgtgaccagcgatccggttggcacgaccttcgacaacctgaccgactacacggtcgacgccgagctgggccgcctgtacatcgtgccgggcggggccatcgacgggaccgccccgctgatcgtgacctacgccacggcggcctcgacccgcacgcagatcgtggtcggcgagggcaccaccatcgagggcgcgctgcgcttcatctcgtacaacccgaccggcccgcgccgcgactactactggccctacgtgcagctccgggccgatggcgacttcgcgatgaagggcgacgaatggcagcagctttcgttcgcattcgacatcctgaagcgggacggctacgcttccgagtacatcgacggtcgtccgaccgtggcgtaaccggggtacgtcaaacgcggtcaaggccaacttagtcaagatcaagcgagccaagaccaacttcgacaggccgcctcggaacccccggggcggcctgtttcgcatcaccagccagaagaggaaagtccatgtcccttgccaacctgcaactccgcaccgcaaccgttccgtatgtcggcgcgaacgacgagtcgcacgacatcgtgctgcacggtctgagtgcgaacgccatcgccggcctcatcctgtcgcagctcagcaacatcgaagaaatcttcaacatcgtcgaggcggccggcgtcaagaagaccgaagacctcgccaacgtcaacatcgccgaagtcggccaacggcttctcgtgcagctccccgacttcatcgcgcacgtcatcgcgtactccgcacacgagcccgagcagtggagcaaggtcatgcacctgccggcacccgtgcaggtcgagtgcctgacgaaactcgcgaagctcacgttcaacgacgaagccggcttccgagaattcgtgggaaacgtggtcgcggcgctgcgaagcgcaaaaggcgtagtgccgcagactctcaaccgaaatcccgccgtcaacgcttcgccgaatggtggcttggcatccgagcagccgtctctttcctgacggctgaaggtcactcgaacgctggcgaatatccgctgggatatttgatcgtcgaatcggaaatcgcacgcgagcgggtgaacaacagaatcagaaccgaaatgacgctgacgcagagtgcaatcgcttcggcgctcagcaagaaagcagcatcggcattcaaagaaaacatcgaaggactataggcgatggccgctcagaacgaagttgaactgattgtacgtgcgaagaacctcagcacgcgaaccatcaaccagctcaacgacgagctgagcaagatcgcagataaccaagagcaagtcgccgatgcgaaccgcttggcggagcggtcgttcgagagcctgaagtctgagcagcagcagttgctcgcgatcatgaagtctctcaacgaccgcgcttccaagctggacgcatactcgcgtcaagagcaacaggtgcgcagtctgcgcgacgagctgagtcgcgcccgcgacaacctcaacacgctcgcgcagcagttctacaacaccgaaaagccgacgaaggaattccagcagcagttgaagtcggctgcgagcgaagtcacgcggctggaatcgtcgctgcgcaataacgagcgccggctcgacacgaccggcaacaagctgcgcgacatgggcgtggatgtcacccgcttctcgcagtcgcagcaggaagtcaatcaggcgctcaacagctcggtggcgctgtacaagcgctcgaccgacaacgtggagcgctacgacgcggccgtcaaggaagtgcgcacgacgcagcagcaggctcgcgaggccgagcgcgccgcagcgcaggaagccaaggactcggcggcgaagctggaacaggccgcccgcgagcgcgaagaccagatgcgccgcgaacagaaaatggccgaactgacggccaacgtctaccgcacgctggcccgggagaaggaaaaggcggcccgggcgggggtggacttccgcgccaccggcacgcaggcgctcgccacggcccgcgcgaccgctgcccctgccgtgggtagcgggtcgtctgccggcgcggctgcggcgggcgtacaggcgcttctcgacccggccaaggatgccgtcgcgacgctcgaccggctggaaaaggccgtcgaacagctcgacgaggaattcaaggcgctcacgccggacgctttgcaggccgccgatggcatggacaagctggccgatcaaagccgccggctgcgcgctgcgtcggatgcgctgaaggggcaggccgggctcgcggacgaattgaaccgccagaacaccgcgctgctcgccagccagcagcggttcgaggaagcgcggcaagaagtgatccagtacgcgcaggcggtcgagcgtgcagacaagccgaacgacgagctggcgcagtcgttgcagcgcgcgcagaacgagatgaagcaggcgcacggcgagctgacgcgccagaccgaggcgttcaaccgcgtgcagcagcgcgccgctgccgccggcatcacgctcaacaacctgaccggcatcgagcagcgtctcgctcaggccgccgcgcgcgtgcgcaccgggcaggagcaggttgcgcagacgatgacgcggttggagcagacgaccgcgaagaccaacacgcagttgaagctcttcaacgacggacagcgcaccgcgctctcgttgtatcagcgcacccgtggtcaggtgctctcgctggtgtcggcgtacgtcggcgtgttcggtgcgatcaacctcgtcaacagcgcgatggacgcagcaatcgagaaagagcgcgtcatgtcgcgcctgctcattgcgaataaggggaaccagactgcggcagcggaagagtacgactacctgcgcaagaaggctgacgagctaggcgctgcattcggcccgctcgccgagtcgtactcgcgcttcgccgttgctgcacgcgatgcggggatgagcaccgaggcgacgcgctacatcttcgaggcgttcaccgaggctgcgaccgcaatgcggttgagcggcgacgagacggccggcgcgttccgtgcgctggaacagattttctcgaagggcttcatccaagcggaagaactgcgcggccagttgggcgaccgcatgaccggcgcgttcaatctgttcgcgaaggctatcggcgtcacgacgcaagagctgaacaacatgctcgaaaagggcggcgaagtgaaagcagagttcgtgctgctcgctgcgcagacggcccggggcatctatggcccgcaagcgaaggctgcatcgaacagcctgctcggcgacctcaaccgcatgcagaacgcatggggcgacctgaagcgcgaaatcatcgacggcggtctcggtgatgcgctgcgccgcctgttcgtcgacttgacgaagtacctgaagagtgacgacggccagaagttcgccgagaacttgacgaaggtgtttgtcgctgcggccgacgctggcggcgagctgctgaaggtgcttgctgagaacgatgaaatcatcaagctactggcggacaccgttgcgttcctcatcaagaacttcaaggcgctgctcgcgattatgctcgcgatccaaggtgcgcgcatcgcgttggtgttcacgcagcttgcaggcgaaatcctgaaggcgcgtgcggcaacgctcgcgttgaacactgcgcttggtgccggcaccgccgcgtcggcgggccgtgccggtgctgccttgggcggcctcatctccgggccgattgccgcgatcctcgccatcgctgctgcgggcatcatcatcccgatctacttccagattaagggcgagctggaatcgaacaaggtcaaggtcgacgcgcagaagacgatcaacgacctcaaccggggcttcgaggtttcgcagcgcagcctcagcgacacgtcgaagaccaacgccgaacagctcgaacgtcaggtcacggccgcacagcggttgctcgacatctacgacaagcagaaggagtcgttgcaggcgcagattcgcgagaacactgctgtgcgccgcaaccaagtggcggtacgtgttgcgcagggcacgcgcgagcacgacatgaatttcccggccaagcagctcgccgccgttcgagaagtcgagaacgaaggcaaggcactggaagcgcagctcgccgcgctcgaacagcgtgccgcaccgctgcgccagcaggtcgccgccgccagtcgtcagatcggcgaagtgaaagcgcgcgaggcggctgcggagaacgatgcgctcgcagccgagtttaagcgcatccaagcagcggccgatgcggctgcggcgcgtgccggcaccgacgcaaaggcagcgaaggcggccgaggctgcacgcaagaaggcagaagccgaagagaagcgtctggccgcgctcgccgagcgccgcctgcgtctggaagaggacgtggcggaaaagctgcgcgacatcgacaacgacattgcggcgtcgcgcccggatacgctcgaagcgcgtctggctgtgatcgacaacaagatcgcggatcgcaaagccgaactggaacgcatgctgcgtgaagccgacaagctcggtcagtcggatgcagccaagggcgaaattcagcgcggcctcgacgcactgccggcgttgcagcaagcgcaggcgcaggcgaccacacaggagttctacgagcagcggattaatgacttgttgcagcagcgacaggcgtcgatggacgcgatcaacacgttgcaggaagccggtttgctgactagcagcgaagccgccgcgcgtatcgaggaagtcaacgctcgcctgctgccgcagctcgaagcgttgcgtgcgaaggcggctgagttcatggcgacgctgggcgatggtccgcaggcgcaggccgcgcgcgccagcctcgaaaacctcagcgcgcaaattcaggcgatgtcggtcgagctgtcggcacagaagcgtcaggtcatcgacgtgttcgtcaacggcttcggtcaggcgttcatggagaccgcaacgctcatctccgacacgctgaagggcgtgcaggatgccggtgacgcatggaaggcattcggcgacatcgtgctcaataccatcgctgacatcctcatccagctcgcgcagatgattattcagcaggcgattttcaacgcgctgaaggcagcggccgagaacagcggcggcggctggggcgcgatcatctcgcaagtcgccgggtacctgcacgttggcggcgtcgtcggttccggcgctggccgtcgttcgtcggtgccgtcgtacgtgttcgatgcagcgccgcgctatcacaacggcggcatcgcgggcctcgccccggatgaagtgccgaccgtgctgaagcgcaacgaggaagtgctgaccgagaacgatccgcgccaccgcttcaacggcgggctggaaggcggggcgcaaccggcaatggacgtgtccatcatcaacaccatcgacagcgagagcgtggtcgctgccggcgcgaacacccgcgcaggacgccagtccatcttcaacgcaatcaaggctgaccgcagctcgtacaagaaacttctcgcataaggaatcgacatgggacacgcaattgcaactgtaactggcggtagcggcgacgaggcgcactacaaggtgctcgctgcgatcaagacgctcgccgaggcgaacgggtggacgacgctgcgctacgtcaacaccggcaccgtgcgcgagttgatcctcaactccgctggcctgtcgggcaccgaggacatctacatcgggttccgcacctacagcagcgtgagcggcgactactacaacctgctcgtcggcacgttcaccggctacgtctccgcgaactcgttcgacgcgcagcccggcgcgaagctgagtggcgtgccttgccacaacaacgcggtgacgtatttcatcactgcgaacgcgcagcgcatcgccggctgcttcaaggtcggcactccggtctacacccacttctacgcgggcaagatgttcccgtactcgcgcccgggcgagttcccgtcgccgctggtgtgcgccggcatgttcgatggtgctgcgccgaagcgtttcagcgacaccgactatcgctttccgtaccacggtcgcgagtcgggctacacgggcggctcgtcgtcgaatgtccgtccgtcgtacctgtggctgcgcgatcaagccggtacgtggcgtcgactctcgcacttcccgttctacaacggcccggccggcagcgatgcgtcgagtgcctacaacgccctcgaaaactggaactacttgaccggcggcgatcaatcgcgttcgctcgtcccggccggcacgaactatcagccgcagccgatcatcctgtacacgaccagcgctccggctggcgtgtgggaaggtgcggtgtacggcgagctggatggtgtgtatgcggtgtcgggcttcaacaacaacgtcgagaacgtgttgcaggtcggcggtacctacgtcgacccggcgggcctgagcatcgtcgatcacgtcgctgcgatcctcgccgctggcggccgtgcattcgtcgtgctgcaagacgtgaatcaaaccgactggcgcagctttatcgctttggagatgacctaatggcttactacaccggcaacttttcctcgttcgctacgctgaagaactcggtcgagaccgcgcttcaggcaaacggctgggggctcaacggcgacggcgtgctggaaaagaacggcatgtacctgcgcctcactgcgacggctgcgcaactgctgttgcaggccggcaccggcagcgcgaccggcgcgcttccgggcgcagctccgaacggcgtcaagatcatggacttcgagggctcgccgatgaatttcccggcgacctacgacctgcacgtcaacactggcccggacgaagtgtttctcgtcgtcaactacaacgccgacaagtaccagcagctctcgtggggcaagtcgaacgtgcagcagatcggcggcaccggcatgtggttctcgggttcgttccacgagaacgctgcgtcgaaccagaaccatctcgtctacacgtcggcggatgcgagctacttcggcttcggttggtcgggcatgggctgcggcctgttcgccgagtattacacgcaggcgctcggctgctcctacgtccacacggggctcgacacgaccgcatggcggcgcgtgtatagcggcgacggcaacctcatcggctcgggcgatcctgtcgccggcctgctgcaagcgctgccttcgatgttcaaccagaacaccgtgctgctgccgttgctggtctcgcagcgccgactctcgcagggccagactatcgtcgtcgacatggcgaacgcgcgcctgtgccgcaacgacaaccatctgtccggcgaaatcgtcgaatacggcagcgacaagtggaaggtgtatccgttccaccgcaagaacgccgacgtgcgcaacggcgtctcgtggtcgacgggcgcgaaccactccggcactttcgcatacgccattcgctacacggggccgtaactcatggcaggcatcaccggacaattcggcagtgaggtcgagcgcggcatcgctaacgtgatgctgagcgaagacttggacgacaacaccgaagtcgtctcgcggttcgactcttacgaaatgcgcccgggccttcaaggcggctacgggcgctggcgtgtgcatgccgacaaccattgggcgatcaccggccagcgcaagtcgaccagcttcttcgacgactactacaaccgcatctacatcgtgccggccgcgctcgatgccggcaacctgctgtccacgcaggtgcgccacatcatcttgtggaacgcctacgtcacgccgcagacattggagaacgccgcgctcggcccgcagtccggcatctcgatgtcgttgcctgtcggcgtgagcctgccgtacgagatggagccgctgcgcgagctggacttcaccgtgcagatcgaactcagcggcccgccgaccatcgacagctatgcgaacttcaccgtcgagggcgtcacctacaccgtgccgatcaccggccggcgcatcgtgctgttccccttctcgccgaattggggctcgcctgtcgacgagacggtcacgatgcgttcgtgggtgttggccgccgaagacggcagcgagcagaccggcagcgagtcaggcgaggttccgcgccgcacgctcgaatacaacatcaacctgcgcaccgcgttgcaggcgcagcgctgcgagaacctgctgttcgcgtggcagtcgcgcttcttcggtgtgccgcattggggcgaggaagagcgcatcgcagccgacgtggcagcgggctcgctgacgattccgttcgacaccttcggcctgtctctcgaacccggctcgttggtggcgctctaccgcgacgacgagaagaacgagattcgcgaagtgcagtctgtcgctgtcgacggcgttacggtcacgaccgggttggagtacgactggccggaaggctcgcgcgtctacccgtgcttcgtcggcctcatgaacgatgcgatgagcggcacgcgcgaaacgtcgacggttggccgcatgcctatcgcgttcgactgcgagccgagcgtgaccccgggcaacgtagcgctcaacgcgccgccgctgacctaccggggcaaggagctgtttctcggccgtaccaactggcaatcggcgatgcccttcaccttcacgtcggatgtcaagcgcgtcgactcgaacaccggcaagttcgtcgcgttctcgtcggccgggttctcgaagatgtctcgccggcacaactggacgctgtacaaccgcgccgacattttcgagttccggcagttcctcggtcgccggcaaggcgtcgcgcgctcggtgttcatgccgagcggcacggtcgacttcaacatggccgcgccgattctcgacaccgaagacatcctcgtggtcgagaacaacgagtacggcgcactggctggcgcacacccggcccgccgagacatcatcatcgagctggtcgacggcacgtacttctgccggcgcattgtcggcacgagcgacttcgacagcttcacccgactgcaactcgattcgtcgctgggcgtgtcgctcgacatcgacgacgttgcgcgtatcagcttcctcacgctgtaccgtttcgagtcgccgtcgaccaccatccgccacctgaccgactcgaaggctacggttgaagccatcatggtcgctaagaccaccgaggattgaaatgagcctgctgcaatacgagcaagacaaggaactcagctcccgcgtggagctgtacctgttcgagagcgacgacggccgctaccgctgggcctacaccaccgacgcgcgcgaaaaggtgcttggccccatcgtctacaagcccgagtcgatcaagcgcggcgagctgaagcagacggccggcgacgcgaacgtcgagaaccttcaggtcacgatgccgttcgataacccggtggcgctggcgcatgtgccgtacctgccggcgcggccgatcaagctgacgatctacgcctaccagcgcaacgatcctgctgcggaaatcgtgcaggcgttcaccggcttcatcaccagcttcaaccagaagggcgcggaagcgacgctcgaatgctcgcagatcatcgacaacctctcgcagacggtgccgtgggcggtgttcaagagcggctgcatttgggcgctgtatcaggtcggttgcggcgtcgacaagcagttgtggaagaacgatgcgctggtcacgaccgtcaacggctcggtgctgggctcgcctgagttctcggccaagccgaccggctggtacaccaacggattcgcctacaacccgcagacgggcgagcagcgattcatcgtcgcgcacgatgccgttgccggcacgatcacgctggtgtacccgtttctcgaaatcaacggaagccagaccatcgaggtctacgccggctgcgcgcgcacgaaggaagtgtgcgccgacaagttcaacaacaaactcaattacgtcgggttcgatcacttcccggcctacaacgtcttctcgcaggggatcacctaatggtttgggtagccatcgtagttgcgctcgtcatggcagtagttggcgagctgcttcggccgaagccgaaattcaacgatccgaagccttccgctgtcggcgatttttcgttcccgactgcggacgcatcgcgcgtcattccgatcttcttcggtacctgcaagatgcaaggtccgaacgtcgtgtggttcggcgacctgacgatcatcacgctgaagaagaaggtcaagaccggctggttctcgtcgaagcgcatcgtcaccgggtacaactactacctcggcgtgcagctcgtgttcgcttatgggccgtgcgacgagttcatcgagctgcgtatcgacgacaaggttgcgccgatcaccagcaagaccttcactggcgacgtgtgctcgttcacgatcaacgcgccgacgattatcagcaacgacgacccgccgaacggcgtcaagggaccgtgcaagctgtatcgcggcaccttcgagcagccgccgaatatgtacctcagcacgcaatggaacgagccggagatgaccgcgtttcgtccgctgctgcacatggtcatggagaagtgctacctcggcaacaccgacacgccgccgcccatctcgatcatcgcgcgtcgctgcccgaaccagctcggcttgaccggcggccggcacaacgtcaacggcgactcgaatatcgcgtgcgcggtgtacgaggtcatgaccaacaatatgtggggcatgaaaatccccgaagacaagatcgacgtggactcgttcatcgcctgcggcaacacgttggctgacgagagcatcggcatctcgatgctggttcagaccgccatgctcggccgcgacctcgtggcggaaatgctgcggcacgctgacggcgtggtgtacgccgatccggtgactggcctgtacacgatgacgctggcgcgcgagattccgtctgacgagcaggacgagttgttgatcgtcgacgactcgaacatcctgcccgacaccttcgagttctcgcgttcgtcgtgggagatgacgaagaacacgatcatcgtgcagtacaccgaccgcaccacgttcgagacgacgccggttcagtaccaagacctcgcgaacatcgacgtgcgcggcggcatggtcgactccgaagaattcagctacctcggcttcagcaactcgaccgctgcgatgaacaccgccgcgcgcgtatcgaagatgaaggcgtcgccgctggtgtcggcgaagatgtcgctcaaccgcatcggctaccaactgcgtccgggctccgcgttctggctgcgcaagccgaaccggggtctggcgaacgtgctcatgcgcgtcatcgaaatcaactacggcacgctggacgacccggccatcaagatcacggcgatggaagacatcttcgcagtcaacgccgtggcctacgtgccgcccgatccgagcgactggacgccgccggtcggtgccgtcgtgccgttctcgcagcagcgcctcatcgaagcgccggccttcggtgccgaggatatgtcgcgccgctacgtcatcacgatgggagtgccgtcgagcaacggcgtgatcgcgtacgacgtttggacggacgccagcggcggcacgaatttccagcagaccaactccatcgacgcgctcacgccttcgggcgtgctggtgtcgggtctgtctcgtactggcccggaagtcgatgctgctggcttcaccgtcacgtcggtcgtcggcgtcagcgacatcgaatctggcactgcgggctcgcgcgagtcgggcgaaaacctgctgctggtcggcaacgaactcatggcatggcagaacatcgtcgacaacggcaacggcacgtacacgatcactggcgtgtatcgcggcgtgctcgacaccatgccgcaagaccacggctccggtgcgcgcgtttatttcatgtcggaaggtgcgggcacgaccaacgaggacggctacggcggcgacctgacgctcaacacgaagctgacgccgaagagcatcgtcgacacggtgccgctggacaatgctgcggcaatgtcgatcacgaccaacgctcgtgcgctgcgcccgctgccgccgggtcgcctgcgcatcgacggtgcagtcgtcggctccggcgcaacctacgatggcgacatgctgttctcgtgggcgcatcgcaatcgcttcgacgacagcatcgcatcgcaggccgatccgagtcgcacgcccgaggaaggcacgacctacaacatccgggtctacaccagctcgaacgcactactggcgtctgcactggaagtatcgagcgccgcgtcgaccggcaccatgcggttcgcggtgtcgggcgatatgcgcattgaaatcgaggcggttcgggacggctacgtgtcgtggtcgaagctggtcggctacttcagctatactccggccgccggggctaccgccaacgaaatcatcgtcgacgagcctgagtacgtcttggacgggggtggcgcgtaatggcacaggtagtcgttgcacaacgcatgtggcagcgccgcgacactgcggcgaattggtctgccaagaacccgatccttgcgggcggcgaaatcggcgtgcaactcggcgctacttcggacgagaccaagttcaagatcggtgacggcgtgaccccgtggaactcgttgtcgttcttcgagggccggctcatcgaaatcggcacgggcagcggctacatccgctggcgctatgtcggtgatccgacgtggatcaatctggtctcgctcgaatcgctgcgcggcccggccggcgcgaacggcgcgcaaggcccgcaagggctgagcgcgtatcaggtcgcggtcgccaatgggttcgccggcacgcaggccgaatggctcgcatcgcttaaaggcgagaagggcgatcaaggcgaccaagggccgcccggcattccgtcgcagcgtcgcatcctgcgcatcacgaacaccgacagcggctccatcgtgtgcgactggaatgcctacgacgaaattcgcgtgacgctgactgccgacacgctcgtcaatatgacgggcgcgctggacggtcaaggctgcgtgctgctgctgaagcaaggcggcgtcggcggtcacggcgtttcgttcggcagcaacgtgcgcttcaacaacctcatcccgatctacaacccgacaacgactgccggcaagtccgacaggctcggcttcgtttatgacgacgacgccggcttctacgacgtgcaggcaatcgtggatggaatctaacgatggcagacgactacatcccgccgttgtcgccgaacatcgtgtgggtcttcaagggcaacgactacacgcccccgctgaccccgaacatcgaatggatattcggtgcagatgatgaaggcggcggaaacgagcttcgcaaatccacctatatgctaatcctgacaatgtgaggtattgaaatgactgttcgcatctactcttcttccgacgctggcgctccggttctgcgcggcaacacgccgggcgacctcatcaacctgctcgaaaagtgtctcgtcaccggctacgggtcgaaggtcggcgcaggttggacgaagccatacaccggcacgaacgtcgctgcattccagcaaggcgcaggctcgaacggcatgttcctgcgcgtcgacgacacgagcacggcgaccagctaccgtgcagcgcgcatcgtgggctacgagtcgatgagcgatgtcaacaccggcacgccgacttcgttcccgacgccgacgcagcgcagcggtggcgcagcatggttcacgcactacagcagcggctcggtcgcgaacccgcgcccgtggcgcatcatcgctgacgagatgttcttctggttcttcctgtcgacctacccggaaaacaacgacagcggtttctactacaacgagagttatgcgttcggcgacatcattccgttcaagccgggcgacacgacgcataccgttctgctcgccagctactcggtcgactcgccgaattcctcggagccttacccgtgggatggcgtcagcatttcgagcgcgatgggaagcaatcgctacggcctgtgggcggcgcgttcgtacacgaatctcggcggcccgatctggctcggctggcacgccgatcacgttaaggcttcttcgagttggggccaagggttcctgtcgtacccgcatggcccggacggcggcctgtacctgtcgcctgtgtgggttcacgagtaccacgtctcgccgtacaacgtacgagggatcatgccgggcctgtgggtgccgtgccactaccaaggaatcctgagccagtatcaggtgttcgatggtcagggcgaattggccggaaggcagttcatggctcgccgccactacgagcgcacggtctgcatcgaaatctcgaatacttgggataggtaacgcgcgatggcgctcatcttcaacctgccgatgacggggccgaacggctccacgacgatcaccgacaccacggggaatttctcgtggtcggtgacaggcaacgcgcagattcaatccaacgctctcgtccttgacgggagcggtgactacgtgagcaccactgctgacgttcgattgaacttcgggccgatcaacgatttccgtatcgcgttcgacatgaagatggcggctgcggacaagggcggctataagatcatcttcgaccagctcaacacgggtgcgtcgaatacgtggacgtggcagctctacacctatgaaggtgtgccgtacttcaacgtctataacaattactacggcaatccgacgccggttcaaggcacgaccgatcttgctgacggcaactggcacacggttgaagtcattcgcactggcggcgctctctcgatgtgggttgacggcgtgcaggttgcaactgctaccgacaatcgcgactacgtgttccagccgcctttcggcatcggttcgcgtatcggctacaacgcatcgtcggcctacgactacaagggcgagctgcgcaacttgtccatttcgatcacgacgccggtcatcctgacgaatcgcatcgcgtcgtggactcggcacagcgacatcggctggaaccgtggccgccgaagcagcttcattcggcgcatggcgttctacccggtgcagccggtcacgaccaagaaggtgcagacggtcaaggtgacgcgcggcgtaccgccgtggtgggggccaagcggatcgaccacgcagctcccgacgtacaagctgcgcggccgagtgatgcagcgcgatcctgacggcgtgttgcccgacgccccggtacagtacgcgcgcgtcgtgctgttcttccggcgcttgcatacgctcgtagacatccagctctccgatgtcgacggctacgtgcaattcgataacctcatgccgggcagtcaagcgtactacgcgattgcattcgacccggaaggcgcaccgttgcagaacgcggtgatttgggatcgactgtcgcccgagcccggcccgtaaggagaagtgccgtgagcccgaacaacaccaacgagcagaacaggaaccgacgagtgacggacaaagcaggggggcttctggacgccgcgcaacaggccatccggcttgaacgcatcgaaggcgatatgcgtctgctcacgcagcgcgtcagctccggcatggagaacgtcagcgccacgctcgcggccgtgcaggtcgaagtgcgtggttgctcgacgaacgtgtcggagctgcgcgggctgcaaggtgcgcacgactcgaacaaggtagcaatcgacaaggtggagaaatcagtgaccgacctcggtgcgcgcttggagtcgtggttcgatgagttcgaggcaaagcaggaacagcggtggcgcgactatcaaaccaaccgcgatcaatggcggcgcgagcacgaggccgagaacgagaacgtcaagaaggacttggaaaaggaaatccgcagcgttcgcgaaaccgtcattcgtttcgtcgggttcggttccgccatcggtgcgctcgcgggcgtgatcgtcggcggcttcctgtggaatatcaactaccgcttcaacgaccataaagaggacgtgacccgagtcgaacaaacgtcattgcgcaaccgacaactcatcgaccagatgggtgtcgatcacggcaaagagctggccgacatcaagctctacctcgcgcgcggcgggcgaatccccgctgagccctatgtccctcaatcgcaaaggaacaacaatggaaacgaacaagactccggccaacccggaaagtgaaatgcccttccgccgccgcgcgtgggagttctggcggcgcaatcaaatcctgttgctgcaactaccgctcatgctggcgttcctcatcggcagctacgtcgtgctgaagtcggtcgactcgcgcatcggcgtcgagggtttcggcgacatcttcggctacgcgctcaacggcgtgcgcatcacgctcatcatcttcaccgcatggtggatcaagaagtggtgctggttcgacctgcacgacaagaccgagctggcgatgttcgaggcgatgaaggccggcgactggatggcgttctggatcgtggtgcgcgaccgggccgagtggctggctgcgctggcgttcgcgaccttctggtacacccgatgagcgcccgggtcgtagtcctcgctgcggccctcctgctgagcgcggcgtgcgctcggccggcagcggtacccccggtcgaccagaccacgctcccgccggccgtggagagcctgcctgcggccacgccggagccggtcgtcgagcaggtcgtcgcggctcagcccctaccccgggccgagcaggctgtttcggagaccgtcacggagccgcttctggccgcgcaggcggcgctcgaagaccttaccccgctactacccccgccgccggcccgggacgcggcttgccggcgcgctgcggcggccctgacgctacgctgggaagtgaccagcccggccttctaccggaagcggctcgaactgccgatctggccgggcggggcgtccggggtgacgtgggggatcgggtacgacgggggccaccagacccgcaccgtgatcgtcgacgactggcacgaccacgggcaggttgaccggctgggccagaccgccggcatcctcggccggcaggcccgggcggcgctgccgcgcttccgcgacatcccgaccggcttcgaccatgccagtcgtgtgttcgaggaacgcagcctcgtcgagtacgagcggcgcaccgagcgcgcgttccgcaacggcttcaccgagctgcggccgaacgcatgcggcgcgctcatctcgctggtgtacaaccgtggcgcggcgatgaccggcgactcgcgacgggagatgcgcaacatccgcgacaactgcgtgccgaagcaggactacgcctgcatcgctgcggagattcgctcgatgaagcgcctgtggcgtggcacggtcaacgagaacggattgtctgcgcgccgcgaggccgaagcgatcctcactgaaaccccgtagggagaagagcatgtggacgaaagcaatcgcgtggctgttcggaacggcaatgggtcgcggtgtgctgctgggcggcagcatcgcgataggcacggcgctcggctggtatgcgttctcgacgcactactacaacgagggcgtcgcgtcgtgccaagctggccgcgccaccgatacgaacgcggccaacgtcgcgcaaggtgaaaagaacatcgccgacaaccagaccagctccgacatcggcaaggccgccgacgccgaagcagcgaaggtcgcagccgatgccgaagaagcgaagaacgactcgaaggagaccatccatgacgtgtacaagcaaccccctgtcactgcgcctgttgctgttggttcttgcgtgcatcctctcgatgagcgggtgcaagaccggatcggcaaagcgcgagctgccgcagttgaagcaagaagccccgctcgttaactgcaagcagcctgcgtcgccggcagtgccgcgcgagccgaaggccgacgagtggatcgagtggaacccgccgcgccccggcaaggccgaaggagaagcacggcttagcgagcgtgccgtgaactggatcatcgacgtgctggccgtggtgcgagtgggcgagggctaccgccgcgtcgagcacaagtgcctcgacgagctggaagcgaaagggctcatccggcagtagttgacaggcccgaggcgctgcattacggttgatcccgctggtggcacttcgcgttgcatcggcactcggcagagggacagcggcgcggagaatcggcgctccgcaccgcagggaacgaggaaccccggactaacactccggggtttctttttgcgtcaagaccaagtgcgtcgtgaccaagttcgtcaagaccggaaaagagaaaagccccggtgctgaggccggggcttttcgggttgcgcgactcacgtcgggcggtgggtatcgaggcgggggttctgctgattccggtgtccgctctatgagcgctgcgccggctggaagggcatgtgtcgcgtcgatggatcgaacctaatgcggcacgccgcgcgtgtcaacaccttcgtcagtccttccacgtctcgacgagcttcagcatcttcttgcgcgccttctcgacgccggccgcccacttgtcccatgcgcgcggatcgacgtgcgtcaggatttcgttgcgcgccatctcgctcagcacggtcggcggcagcgcgtccagctcccagctcttgtcgccgaagcgctggcggtatttcacgaagcgcgcgtcggtcgtcttggccgggttcggtggcggcttcagctcttcgatctggtcgaggttgagcgccatgcgcttcagcgtgaactcgccgttccaaccgaacagctcgaagcgctcttcgaggtcgcgcgtcatgtcgatgccgctcgggtcgtgatccccgaagtgcaggatcaccacatccttgccgtcgctctcttcgatttcccgcttggcgaaatcgcgcacgaccgatgcgctcgggtagccgcgcgctgcgagcagcggcacgtcgaactcgtggcacacgcgcgaaaacacgccgaccagcgcttccttctcgacgacgaggaacaggcgcttctcctgcgtcgcccacgggtcggtgtggtactgccgcgccgacgccgtgagaatgtcctgcgggcgcgaccagcggctccgctgctcgaacgagcgcgtgcggtcttcgatggcatcccaatcaatcaggcccgcgatgcgtgcgtcgttgacgatgctcgtggtctgcttgtacgacttctcgttgttcggaatgatgtcgcgcgcaacgagctggtagtagagctggcgcacggtcagcgtgtaccccgcatcgagatattcttcgatgatcgcgttgatcctgtcgatctgttgcagggtcttcgtcttgaaggtgatttctttgtagcgttcgagactcatggcactcggctcctgttagcggctggcgggctgttcggcggcccggatgtcagtggcgcggatggattcgatttcaggcggcagttcgatgcgctcgaccgcgtagccaacatcgcggccgtagtacacgccgcgcacgtcgggcaccgggtagacgtggtagctgccggcgtgcatgtgcagcgcgtggtggatgcgctgctcgatctgcgggtaggtgtacgggttgtccgggctcggctgcacggtgcgcacgccgatgccgacgtagccgctgcgcgccagcgtctcgcggaacagcgcggtgtgtcccgcatgccacggctgatagcggccgatcatcgtgccctgcggcgtcaggtagcgcaggcacgcagcgatgcgttcgagcgtgggctgcatcacttcggccgtgacctgcaccgcgacttgctgcgggcgctcgaacatttcgtcggtgtccgggtagcggctcttctgcaccgtgtccatgaagacgatgaggtcaggcgcgaacgcctcgcgcgtctcttcggtcgggcacacgaacgacgcgacgacgatgccgtcgtggctgtccgcgacctcacgcatgagctgcgcttggcggatgcggcccggcgcactgaagtcccaatcgccgtgctcttcgcgcactgcgtcgccgtcgatgtgcgttgccggcaacacgcgcgcgagtgctgcgccgagcgtggtcttgccgctgcccggcagaccgcagatgagaattcgcttagccattgttcgattccttctgtgcgcgaagttcttcgcggatttccatgagcagcaggccgagatgattctcgcccttgccgtcgcacacgccccaaaaacggtcgccccaccaattcccttcgacgagcttcgacttcccggtcttcagcaggcgcgaccgaagcgggtcggtgccgaacttctggcgcagcaggtcgcgcatgacgccgaccttgatctgctcccaatcctcgcgcagcgttgcgtgcttgccgcgctgcttcgcgccagcggcgctcggctcgttgcgaatgcgacggcgctcgtcctcgtcgagcgtcttggctgcttggaaggcgtgctccacggtgcggtacgagtgcccctcgaaggcgatgcagcatgaccagaaattcgagaggaagcggtacgggccgttgaagctgtcgatggtcttcatggtgtcccctagtggaagtcgatcttcgccttgctgaagagctggcgctgcttctgcatgtcggtgcgagtgatctggtcttggatgggaacctgcacgttgcgattcatcatctggtgcaggtagcgcggctcgaccgcgtgcccggtcgcgaacttcgcaatcgccatgagaatttgcggcgagtgcagctcgaagaacgtgccggtcatcgaccacggttgcggtcgaatgtgcgccgcgatgtcgagcagttgccgctcggccttgcgcacgttgagcggcggctggatgccttgcttcttcatcgagtgctcgacctcgctggccgcgcgatgcacgacgaggtactgcgcgcccgggaaccggacgagcagttggtcgaagaagaacagcgcggccacgtccgacacgaacacgcggccgggcggctgcgcgtcgatcttctggcccagctcagcgatgctcgcgcactgctgaagcgggttgtgcatcgacgagacgcacagcggccgaaggaactcggccatccatgcgctgcggctgcgcggcaggctgagcatgatcgtcaggtgctcgtacgccatgtcagccctccttctgctcgcgcgcgttcttcgcgttgtcagcgtacgtgtcgagcacgcggacgaacgcatcgtgcagcagcgtgccggcgggcacgtagatcaccgtgccgccggtcaggtcgttgcgggtgtagatggtcggagccgcgcccgggatgagctggccctgaccttctggcgtcgcctgcatgcgatccggtgggcgcgagtcgaactcgcgcaccagaccgtccgcagggccaccgacgaagaagccacggacggacgtgttcatcgcacgtctccgtcgccctgcaacgtgccgcgctccctgcgcccgttgagcttttcgcggttgtcgaacagcagcttttcatagccgccctcgcagccgaccagcggccccgtgcgctcggcatattcgaccgagaccgcgatgacggaagccagcgcgccgcgcagctcggcgatcttttccgcgcgcttctcgccgctccacgttgcgccgtcgcgcatcatcttcttgatgacgcccaacacgcggcccgcgtgcgcgcacagcgccgattgcaggtcgtagccgctgatacgaacctcgcggtgctcggcgtcggcaaggcgctgcatgccttcctgcaccagcacgtcgaagcgcggcagctccggcgtctcggcgcacaggcgcgcggcgtaccactgcacgtcgcccagctcgtgccacgccttctggtagcgctcgacacgaaactcttccttgatggcttcttggtcgaacagctcggccagctcgccgacttcgttcgccagaccgatgccggtgtacagcatgcccgcgctcacgttgccggcgagctgcacgatgtcggtcgggtacttggccgtggtgacggtgaaggcgttgtacgcctcagcgaagatgcgcgtgggttcgacgcgcgcggcacgcgactcgcgtgcggtatcgagggacaggatgctcatgcgcggcccccggcggcgagcgcgtcagcgaagtcgttgctgtagctggcctcgaacttcgtcgccatgtcgtgcaggacgagcgtggggccgccgtgcgctgccgggatcatggcgaagtcgacgccgcgcaccagcgggttgcgctcgccgtcctgaccgatggcatgcacgaccaacgcttcggggttctcgcgcgcggcgcggcgctcggccttcaggatgcgccgcatggtcttgccgccgaacgccttgcgcagcttttcctcgggcgagccgtggtcgcggatggcgagcacgccggcaatgccgcccttcgacgtgcgcacctgacgcttgttcttgcgctgctcgttttcgaggtcgcgctgctggacgaggaaggcgtagttctcgtcgacggcgagcatgcgcttgcgccagtcgctcagggtcttgcccttctcggcattgtaggaacggaaaatgcgcttcaacaggttcatcgtgtggctccttcaggtgtgaaaaaagcggcccggccgatgtcgacggggccgcttcgatgtactacttcaacgccaccgggctcagcggccggcgacgaacttggtctgcttctgcacccggccgcgcttggtctcgcggaacagcacgatggtcgtgttgtcgtcggccatgatgctcgcgtcgtcgagcgcgttgctctcggtcgcgaacgggccgttcatggtgctggccttctgcgaaccgtcttcctgcgcggtcagcagcaggtacgcgaactgcttcgcgcccttcttgccgcgacgcacgccgaccttgcgggcggcggtcttcttgccggcgggacggccgcgcttcttggcgggcgcggcggcctcggtcttcttcgcagcgcgcttggccggagccttcttcgcggcggccttgcgtgcggtcttggcgggagccttcttggtggccttcttggcagcggcgcgcttcttcgcgaccttgccttcggtggcttcggcgttctcggacatctggtttctcctagcgttgttgtcgacaactcgcggaatgcgagcggggttcccttgcgggattcggttcagtccacgcagtacgcggggacttcggtgcggaacgtccggcactcggacggctgcgtgatgtacaggccggcgatggcggccagcagcaacacgccgtagacgatcttctcgcggcggctcatcactcgcagcccacggtggcgttcgggcgggtcggatgcgcggcggtgtactggctgaagtcgcgccagccttccgagccgccgcacgcgaagccccagcggcgcacgatggagccggtcatgaagagcgtccagcacggctcgtcgttgttgccgaacagttcgagcaggtgcatgtggtcggcgctcaggcggcggaagtcgcccgtgtggaagtgctgcgtgtagtcgaacttgtgctggcccgggaacttgcccttgtttcgcaacacgctgccttcgacgaacgtgcggccatcgttcggagtgaacagtcggtgcatgtacgagacgtgcgcgtccatgccttcggggctctcgtcgatggcgtgctcgtagcaccactcgctcgtgtgctcgatgtagcgaccgtcgaggatgagcgacgcactagcccacgggtgatcgtgcagtgcgcggtcgtcgtcgccatgcacgaacttgtgcaggtacaggttgaaccagcggttgcgcgggatgatgtgccagcgcgtcaggtacgggcggcgcgggccgccgtcgatgccgtcgagcatgatgaccttggacggcgagacgatgcgcgcgtacagcttgaacgcaccgacgaagagcggccacaggccgatcatcgagagcacgttgtagaaccggcgggagaccttgggggcgttcatggcggggaacatcctcggtatggtggggtaattcatgcgtcgggcgtcgtgtcggcggtggccgggccatccgcgttggtcgtgtcgacctgcgggcgaacgagcgggagcggctgcgagccatcgagattcttgaactcgatgtagtagcgcgtgttgagcgtcttcagtccggtgtcgacacggttctggaagacggtcagcagttcggccttcgtcagctctccggcgtgcatgccgccttcggagacgacgcggaagttttcggtgtcgccgctcgtgagcacggcgaggttgtggcggtcgaggatgagcttgtcgagcaagtcgcggatattcggcagttcggcgaagtcgattttcattggttctctcggcgtgagatgaagagcggcgtatcgtgccgcaagccgccgggttgacccttcaagcgctggggagtgcgccatccagttgaccgggggtatcgcctcggcgaccccgtgcagttcgtgatttaccccgtagggggacgaagtaaattcgttactgcggggccactctaacgccagcttttcggcttgtcaacacccttcctcgtgtcgggcgggcggctcagccgggccatcttccgctcgccccggaacagcctgtcgcgcagcatcttctcgctgacgtgcgggcagtgacgcctgatctgctcgaacgtcatctcatccccgtcgatggtgtacagcttcactcgtgcaactgccttcacttcgtagtcctcgtcgtcgaatttctgcctgctcatagcgcccgcccgtgtgtctcgatgtagatgtcgtgcagcatctcgtgcgcaatcgcttttcggaacgccggctgctgcacgagtgcgtgtgcgaagtcgcgcgctgtcggctccttcatgccgagatgcgccgtcatgcgcagcgcctcgtcgatgatggcctgcgcttcgccctcggcgtagccgtcgtccgcgagcagcgcgtggatggcctcgcggtacttcgcgtgtcgcgcgcgctgccgcagcatcgcaatgccggcgatgacgttggggccgataaccagaagcaaccaatcgaaccagctcatacagacctcgcgtacggacgctcttcgccttccttgggcttcggaacgtcatggagagtggacagtcctttcttgatcttggcagccatcgccttgccgaactccgacgcatcgccgtacatgaggtcgaggtcgggatcggcgcactcggccgcgacgttgcgcagcgtgtcgagcagcatcgggagctggtgctgcgcgctgtagttctcgtggatcatcgtccacgctccctgcgccttccaccactgctttcgctcgtgctcgttgagcgcgacgtactggtcgatcatcgccatcgcgaggaacggcgaccagaagcatgtgtcgaccggggtgatcgagtcgcccagctcgtcgagcgcgaagtacaccgcgaagacaggcgtggtgccgatgaggtagaccggctcgtcgagcgggtctttgtaggtggcgatggtgcagccccggtacgcggccatgtgtgcgtagcggcgcttgctggcgtcagggagtggcatgcggaaactctcgttgaagtacgggtcaagggacgctgaggcgtacaagcacgcctgcttgggctcaggttgtgcagctctcatggcggtgaagctgcgctcgctcatgcgccgccggcatcgcgcacgagcacgacttcgccgtcctcgccgtcaggcaggcacgcagccagcacgtcggccgcgccctgcgtgtcgccgagcacgagcagttggatcgcggcgcggatcgcggtctcggtctcgacggccttgcgctcggcggcgagcacgtagcccgcaccgtcgcacagctcttcgagcagatggcgcaaccactgcgcggtcgtgaggtctttccggtcgagcgtcacgccgtacttcttcaagccggcgtcggcgcgctgacggatgatcgagatgaggtcgttcgtggtctgcatgtcactcatggtcagaactccttggcgaaatctttctcggcgcgcagcaaggtcgaaaccttcgcgtcgaactttttggggttgtcgagcaggatgtcggcggcggcttgcgcgatgatcggcgagatgaaataggcgttgatcgggtgcagcacttcgccgaagtcgtcgacgatgtagtacgcaacgtgtaccgcgatgccgccgccgatcttgccgtcgcggtcatcgagaacgcgcagcggccggtccatatgcagctcggcgatgaacacgtcgcggtacggttggatgcgcttgaacttcatgcggctttgtccttcaggtggtcgagttgccagcccgcttcgattgcagcgaacagccgcagctcgctcgcgtcttcggtgtcgagccgcaggaactcgatgaagctgtcgatcatctgcggcgtcatcggtcgcttgtcgtagaacctgcggtacgcgctttgcggaatcatgtcccacaccgggcacaggtcgacgatgcgcttgccttcctcgcgaagatggcggcgcatgatgtcgcgcaccgtcttcgggttcttcttgaccgtgatctttcggccggtcgacggacggaaactcatagcccgatgtcctcgccttcttcacgcttcaacagccacatcggcttgcgcgagagcatcggcagcgggccgatccatccatcgacgagaccgtggtgtcggttccagccgtagttgtcccaccagcgtccgcgcttctggcccagctcgggtagccacacggcaatttccatttccttgtgcgcgggcagtgcggtcgggaacgggtggtgccagatggcgtagaagccgaactccggcgggtcttcaagcacttcgatgtcgttgtactgcatcggcccggcccagccgagcacgagcccgttgaacggcacgaacggcttttgcaggctcggtcgacgctcccaccacatgccgttcgcccagcgcatcaccgagtacatgcgcgggtcatgcacgatggtcgggttgcgcgtcagctcgacggcgtacatgccttcgatggtcggatcgtcgagcacttcgagttgttcaatcttcatcgcgtggagcctcgacgtgagtgcgcagtggccgcaggcgcggcagcgggccgatccagccgtggacttctcccctgaagtattggtcgctgttgaggtagcaccagcggccgttgaaccacatgaggaagatgtcgacgacgagcccgcgaccgtgcgggtcgtctacgcggcaagcgtagacgcccgtgtcctgcggcagtccgatttcttcgtactgcaccttcacggcatgcacttctcggcgtaggtgcggcagtcgcgcatgaagtcgatgtagacctcgggcggcaggtcacgcatcgtcgtcacgccgaacgcctgcatgtgggccttcagcctgtcggtgccgtggatgatgcggaacagccgcgcgtactcgtacaccatctcgcgcatgcgatcctgctcggtacgaatgcgctccggcccccacgagccgccgcgttccttcttcagcgcgtcgacttcgcgcgtacgcgattcgagcgtggcggccagcttcttgttctgctcgcgcaggtcgtcgttctccttgcggccgtgcatgcgcaccagcgtgcggatagcacgaatcgcgaggtcggtctggttgagcgtgggtccgctggtcggccgcttgtcccagcccggcagacggcgatgcagttcatcgaacacgcgcacgaggtcgaacaccgctgcgtcgtcgatggcctcgaacgcctcgtgcagcttgcgcccggcctcggccgcagcgtgcgcctgctcgccgacactacgcagcgcctcgctcgcgtccttcgtgtccagccgcagctcgacctcgacggtcttgcgcgcattgccctcgtcgtccgccggccgccacgttgcgagccacgtcgcatggtcgcggtaggtgaacttggtgcggtgcttgtcgccgtcgcgctccatcgtcacgtagtagtccgtgctgtcctgcttgcggcgcgcgtcgactacggtgtaggtgctgcccgagatgacggagaagtagcgctcgccagcggccggcggttgctcgctgccgtcgaacggcacgttctcgatgaagtcgcggaacagcgattcgataaggccgtagcccatgccgagttcgggcggcatcccgacgcgacgctcgcgcgcaggcttgaacgacacgtcgtacagctcggcggccatctgcgcatagggtgtcaggcccggcactttgtccgaagtcgtcggcgcgaacatttcgttccatgcgctcggcgtcgtgaacgtccactcgtactcgccgccgcgctggttgtcgacgcgcagcatgcggacatgcgagtggccctcgcactcgtgcgtgctcacgaccatgaagaagcgcgccgggcgattgcggtcctgccagtaggtgccgaccttcggcgcgaactcgtagcccgggtggccgaccgtcactgcacgcgcttccttgcggtcgctcgcagcccccgtggtcgtctgcgtgctgcccttcgagaagtcgcgacgcatgatgcgctcgatgaggctcggcgtgcccttcattgcctcggcgatggcgtccgggctgaagtcgatggtgttgatgatgtggatttcgggcgcgctcgggctctcggcgaacgacggcgcgggcaccttgccgttgtgcgcattgaagaagaactcgtgctggccgacgaacgtgttgcgaacccagcggtggatgcgctgcgcttccgcgcgctggatgtcgttctggccgacgatgccgccggcagcgtgcatgtcgcgcacgatgccgttgtcgtcgatgcacgcggcgaccgacacgatcatcggggtggtagcgtcgttggtgaactgcttttcggtatgacgagacattttcggcgtttcctcggttgggttaggtggtgctgacgtgaccggcggcctcgcggtcaagttgtaggtctgcgatgtcacgcagcgacgaaggccagtcgtcgagcggcacgagtccttcctcgtgcatggtgatctggtcgggcgtcaggccgcacaggtagtacgccttcgcgagcgacatgccggcgataagtcgatagcgcatagcggcgcggccatgcttgaaggattcgacttgcgcccgtgtcacttcgcccgtgcctcggcacagccggcacttcgtccccggcaagttgtcgtcgtgtcctgcgtcggggccgaacatctcgttgaactcgatcatgtcgtgccgcccttcgcagcgcgggcagacagtcttgtcacggagccaacgccacgccgcgcgcaccttcatccgcagggcggtacttactgcgcgaccgagcagggcggtagcggtgcgcagacgagacaaagggggtaccggagcattccgagaagccgcaagcctgcggcccaacattttcgcttcttcgatttcgcggcgtgtgtggcgcatggtgttggtcactccatccgggtgacagtgaggaaggcgaacatggcgtcgttgctggcgctcatgtaggtgccgcgctccatcttgaagcgcttgtgcttgtggtcgcccgctgcgcgcaccttcgcgatgccgccgctcaggatcgagttctgctgcttgaagtatttctgcgcctcgttgttgatcgcggcgatgttcccgttgtcgagcgggatgcgctggcagcgcgcgtgcgactcgccgatgtcgagcttgctgagctggtcgttgagcgagcccggcaggaagatcaaccggggcttctcgacgatgcgcacgcgcgggttggcgatgtcgctcttcttgatcttcgagcccggctttttgcggctcttcttcgcaggcgcggcgctgctgttcgtggtggcggatgccattaggtgatgcctcctgttccggggaagtaagcggacaagaaacatactactgcgcgcacccggggtcgtgtcaacccgggcgttctcggtcgtgaccaactcgcgcgccgggccagcgccgcacaacgatccggctaggttgtcgaagcgggcgcaatttcggaaccggctaggtcggcgaagcgagagcgcaaacggaaccggctggctttgcgaagcgggccgaattttggaacgggctaggttggcgaagcggggaggtttttggaattgctctcttacatgtacgtgcgtgcgagcatgcgcatgtgcgcacgacgcgcgctcgctcgcgcgcatcacgcggttcctttatgtcgccggatcgcatcgccggcacgtcgcagcgcatgcgacgcgatgcgcgcagcgtgcaagggagcgcggcgcgttgcgcggttcccttcatccgggcgcgcttgccgccttccgcgcttcctgaatgcaaagtaaacggactactgcgcgcagtaaaaaaatacttgcacgcggcgcggaaccgtgtagcctacgcataccggcaacgtcgccggcatcgcaaagggtcgcaaacatggcacgcatgaaccgttccgaattttccgccaatgccgcgcttgccgcgtcgcgtggcgcgtccgctgcgcgcaaggtcgaaaccgcgcgcaaggtccagacgttgcgcgatttgctcgcgcgtctcccctttctgttttccgtcgccgttgccgcctttgtcgcggtcgcggccgtcgccgtttccgtcatctaagggaatcaattcaccatgaacaagactcgccgaaacatgctcgacgcgctgcaaaatcgcattagcgcgctgccgctggaaaatcttttcgatgaaatgcgcgccattgcggaagagctggaaagcctgcgcgatgaagagcaagacgcattcgacaacctgccgcagtctttgcaggacggcgagcgcgggcaggacatgcaagccgcaatcgacgcgatggatacggccggcgaattgctgcgcgcattcgaggatatttgcgacaacgcatccgaagcgttcgcagcgattgaagatgcaaaggggatcgcgtaatgcgccgctatcttttcatttcatccgctacgctgccggttgtcgcctacgcggaaagcaaagacgcaatgcgcgcatacgtgcgcgacctgctagggattccgtacggtttcccgctgccgcgtcataccgtttgcagcatcgcctaacaattcaccagacaaggaaaattcaccatgcaacgtattagcctttcgcaagccttcgcacagtggcaagagctggcggccgacctgccgcaagatgacgcgcccatgctggcggaatcgtggaacgattacacggattcgctttgcaaggatggcgcattgtgcgacctgcaataccgctacgcgcccgcatacgatgaagagatgcccggcgacggttcgcgcttcgatccgctgagcgatgaccgcgaattcatcctagacgcgctaggcgtcaccatgcgcgcaacgcgcaaggatggaccgcgcgaaggatgggacgcgagcgcgtcacactggcgcgtcacgctgcgccgcgaccgcgcgagcatgacaacggattacagcatgggcgcggcgcatacgggctcgcctgagctggcggacgtgctgaattgcctgatgcgcgatgcggaatgcggcgcgcagtctttcgaggatttttgcgcggaccttggatacgacacggattcgcgcagcgcggaaaagacgtggcgcgcgtgcaaggtaacggccgtcgggctcgcgcggcttttcagcgatggcattctgcgcgacctgcgcgaattgttcgaggatttttgaccatgagcgagctagacattagcgcggttgtcgccggcatgcgcgacccttggaattactcggcgagcgttgcggaacgcgggcaggatgccggccgcatgacgtgggaagccgcatgcgaggatgcgcgcggcttgttcggcgagcatttcgaccgcgccgcgttcgatgagtatttttcgcatttcggcgcatgggacgcggaagaattggccgcgcatacggatgaagaatgcgccgcgcttatgctgcaattcatcgccggcgaaatgcgcgaggctgatttttccagctatgccgacatcgaaggcggcgcggaaccgttcacggatgaatggtggccgcagtatgaaaaagcgagcgaggccggaaccgtcgccggccgtttctgccgcgacgctggcggcgttttttactacattggagaatgaaacatgcaaagcaaatgggcaaagacaaccgcgcagcgcatcgcatccggcgagctggcggaatccatcatccgcaaggcgcgcgcgttgctgcgcgatgccgtgaatgctgaagagtatttcaagcgcgaaccgtcgccgtctgctaccgctgcggaagcgtgggagctggtggagatgattagcacgcatgcgccgcgcgtcacggatgcgcaagcgcgcaaaggcgcggaatggctgcgccgccttgtctacacgtcgcgcggcacggtgcgccgcacggaagccgcgcagcaattcagcgatgcggacctgcgcgttttgcaggcttgcatcgcgcgcccggccttccgtctggtggagctggaaccgcacagcgacggccgatacctgcgcgaccttgcgcccgtctatcgctgcatcggcgacaacggcgaatccttcgattacacggcgaccgcgtggcagtctggcggcgcgttcgcaatcctgcgccacgcttaacccttcccatccgtgacaagcccggagaatctgaaaatgtacagcatcgcaaacaacgcaaagcccgccattctgacgcgcacggaatcgcgcatccaatcgcagcgcgacaagcgaacgcgcgacacggaagcgcgccgcgcaaagtatcggcgcaacgctgcgcgctatctggccgcgtctttctggcgcggctcgcgcgacatcgccgatttttttaagggtcgcggattcgaccatgcgacgttgcaggatgcggaaaacgattgcatggataacgtcgatttttcttatctgtattcccgcgactatgcgcgcgagctggaaaaggaatacggcgacgacgcgcgcgaattgttcgcgtacctttgcccggatgcgccgctgagcgtgtaccgtgagcaaatcgccgacgacgtgacgcgcgcggtcgcagactcgcggcgcgcggattatgcgttgcagtttttcgactggtgccgcgatgcggtcgaggatgcggccgattcttccgggcttgtctggtgctggctggacaaggccggcaagcctacggatcaggaatacgatgcgcacgcggtaggcttcgcatgctcgcgccgcatgtacctttcgcgcaatgcggaatggtggccggaaaaatggtgggcgaaaggtgaaagcgtttggagcgattacgcgagcaatcgcgaacgcatggacgcggccgatgacgtgctgaacgaatttctcggtgagcatctggaaagcgaaggcgcggaccttgaatcgttcgatgagcgcggttcgcgctatgcggatgatgattattggccggaatacttcagcgactacagcgaagcgcgcgagcaatgggaaaacgacaaagcaaagatgcgcgcgcgtctgcgcgagatgatcgcgaaccgtgcgccgctggaattgcgcgccgcgcttgtcgcgagcgtgtacggcgagcccggccgcgcggccgatgaatccgaagattgaaagggagctaacgacatgacgacgattaccgcatacgcatacaatgccgcgcttcattgcccgcgctgcgccttccgttatttccgcgtcgatcctgcgaaggtgccgccgggcgcggatgcgctggacggttgcaaggatcgcgaagggaacgcgcccgcgccgctgttttccacagacgcgaacgcggacggatattgcgacacttgcgacatggcatacggcgacgcggaaccgcgcgcgcacgtcctgagcattgacgcatggcgcgagcccgaaggctggacgtggaataactggcacaagcgcggcacggtgccggttgcatggtgcgacctgagcccgcgcgcgttgctgcggaacctgcgcgcgcacgggctcgacctgccgccgggcgcggtatgcgtcgaggatgacggatacaacgtcgagattcaggcgcgcggcacgcgggaaccgttgtacgccatcgcctacggcgaggcgcagcgatgagcgctaagcccgacctagcagaaaagcgcgaagccttgcgcgctggcattctggcggatcgcatcgaacgcggcgcgcgctggctttgtttcgctgccatcgtatgcgcgggcgcgttgccgctggcctggggagcgttccgggcgcatggcatcgttagcgggctcgccgtgctggcgctggtgctggcgctatgctggcacgttaagccgcacgggcgcagcctagcggcgcaagcgcgcgagattgaagcccgattcaagccgcacgattaaaagcgcgctgcggcgcgttccctgcatcgcctaccctgagcccggccgcgtgccgggctttttattgcctgcgcgtctaggcgcgacctagcagccttgccggccgcacgtctgcccggccttccgtatcccttcgcctgagcccgtgcccgcatcgcttgcggccgggcttttctttttcccgctgcccggccttgctcgggctcgcatgcgtgccggcctgcccgctgcccggccttacatggtcgcgggcttatccgctgcccggccttgcatgcgtgcggcatagctgcccggatgcggcattgtggaattaacgcattgcctgagcgcataggcgcgcgcgtgcggcctttccgaatttatttattgcatcgcatgcccgcatgcgtgcgcgccgcgctgcgcgcgttgtggcgcggcaggaagggataaagggatagccgctaggcgactaaaaaggtacttccggcctgcgcgaaggcgtcgcggggggcgctgaccgatcgga

SEQ ID NO: 15 - DNA, 42307 bp, unidentified
  source 1..42307: mol_type = genomic DNA
atggcccgcgaaagcggggaggcagcagccctgcgatggaagaagctcgggctgctgcaacgtcactacgtctccttcaacaagttcatggatgacatgatgagggagcttggtttctcgcctacgtggatgcagcacgacatcgcgtcgtacttgcagtacgggccgaggaacctcatgatccaagcgcagcgtggtgaggcgaagtccaccatcactgcgatgtttgctgtgtggtctctgatccagaatccgaaatgccgtgtggtcatcgtgtccgcaggcgaaggcactgccaacgagattgccacgctggtgaagaacctgatcctcacagtggacacgcttgagtgtctgcggcctgacaagtcctcgggtgatcgtacgtcaacggaagcgttcgacgtgcaccactcactcaagggcatcgacaagtcgccgtccgtggcgtgcgtgggtatcggcgcgaaccttccgggtaagcgtgcagacctcgtgatcgcggacgacgttgagtccccgaagaactcgctgaccgcgaccatgcgcgaaacgctggcgcggctcatcaaggagttctccgcgtggtgttcgacagactgggcacgcatcgtgtacctcggcacaccgcagagtacagagagcatctacaacgctctaccgcagcaaggctttgacgttcgcatctggccgggtcgttacccgaccgtggaagaaatgaagaactacggtgcgtaccttgcgccttcgctacgtgagcgcatcgaagctgatccgtcgttgcagatgggtggcggtgtcactggcgacaagggcaagcctaccgatcctgacctgttcggcgaggacaagctgaatgagaagtggcgcatttgggcagagtccgggttccagctgcaatacatgctgaacacgcggctgctcgatgcactacgcttcccactcaagctgaccaaccttgtcgtgatgaagggtggcgatggcaagaacttcccgctcgtggtgacgcgcggcttcggcccgcaagcgttgcaggcgtactcgtcgtcgggcttcaacttccagctgtctgcaccgcacaccgtctcgcaagagacagctgcgctgcaaggcatctacatgcacgttgaccctgcgggtggtggtgtgaatggagacgagaccggctatgccgtgaccggcttcctcaacggcaccgtgtacctgctggctgctggtggtatccccggtggctacgaactcgaacccttgactactctcgcacagatcgctgaacggtggaagcccaacagcatcggcgtcgagaagaacatgggctacggcgcattcgtcaaggtgtggctcccgatcctgcgcaagcattggcaggggaacattgaggaggagttcgtccacggtcagaaggaagtccgcatcatcagcacgcttgagcctgtcctcggacgtggtgcactcgtggtgatggaggacgtgatcgagcaggacaacgtagcaactgagaagtacgaagcgaccaagcgtcagacgttcagcctgttctaccagctggcgaagatgactcgctcgcgtaacgcactcaagcacgacgaccgggctgacgccctcgaaggtgccgtgcgcaagtggcttgctcagatcgccatcgaccaagagaagcagatcgagaagatcgagaacgccaagtggaagaagtggatcagtgacccgctcggccacaaccgttaccgccagtccaagactggtggccccaacatgctcaacaagtaccggaggtaacatgcaacgcattcagttcaaggactacctgcgcagcaaccagctgcaccgcgaggtgtccgtggccgtgcgctatgcgaaggatactccgcgcaagacgcaactcctgcgcgactacttcgcatcggctgtggccgagatcgacgcagcactccctcagcctgaaaccaaggagacgaaatgaacgtcgttgaaccccgcctgcgtccgcaggaatatggccgtgccaactacctcaagcgggaggtcgagcatgcccgtcgctatctcgtagctgccaagctgcgtggtgaaaccgacaaggccgaactgttggccgactacttcgagaccgtcgcggctgagttccgcgtcgataccagcaaccccgtcgatgacgcgggtggacagggcgacgcctaatggcctcgaccaaggtacgcatcgcggcagctgtcctcggtgcgtccttggtgtccgcagcgggtgtcgctatcatcaagtcccatgaggggctgcggtacaccgcctatcccgatccgggcacgggcggtgcgccgtggacgatctgctacggtcacaccaagggcgtccgccccggcatgaccgcaacccaagcccagtgcgatcagtggctccgcgaggacatcgctgaggcagagaaggtcgtgcaggcaaccgtacgtgtccagctgacgcagggggagtacgactcgtacgtgtcgttcgtgttcaacgctggcgcgaacaactggcgcaacagcaccatgctccgtctgctcaaccgaggtgagcgcgttgctgcttgcaaccagttccctcgctggatttacgccaacaagcgcgagcttcgtggcctgaaaatccggcgctacgaggagcaacaccagtgtctctctttcgggaggatggtctatgatccctctaagcactgatccaatcaagtccgcccagcgatgggcggcagtctgtggcatcctactgggtctcgtcatcattgcgtgtaccggcctctacatttggggcatgcaacgcaaggtcgagaaactggaagctgcaaacactaccgcagtggcaacaggtgcagctgacgaagcatggcgtcaaggccacatcacctacaccaaagaccgcgaggaggctaagaatgcgactgagcaagtgcttgagcgcaaccgcgactgggctgaccagcctgtgcctagcgacgttgctgaccggctgcgtaagcatcccgacgccgcgcgctgagtatctggccgactgctccatcagctacccgcctgaccgtaccctgaccaacggggatgtcgtccggctggccgaggagcgggagttcgacgtgcgccgctgcaatctggacaaggctgcgctgcgtgcgtggttcgaggcccagtgcgctggctggcgcaagcggtgcgtggcacccaaggactgaccgtggcaaccctaccggcccaatcaaccgggccgtgtagggccacacaggcagtctccgaggtgtactggtgaggtataacacccgcgcagctaggctgtcccattgggacaggcaccgtacgcatgcaggcataggagtacgggccgaaatttggtggagttccgcgagagggtcactccaacagaagctcccgcgcacgtccccgtgtgccctcgcgtacgcgcccacacgcgcgccgggaaccttgccgcgcacgcacacccatgcgcgcccgcgacatcgctcacgcgcacgcacaggccgttcagctacggttcagggctgccgtgggaggctgtgtctcgtggtcggcaccgctggtcacatggtacggtagcgtgggggtgtgctggtaaggtagcacacccgagcggtatctgtatcgttcgccgagtttcggcaccctacatacacagaccaaaccgacaggccgcgccgggtatctgttgccagcttaacaccagctgaacggacacacacagacacgggttgacagacgggaacggatcgggtagagtgacggacaagctagacggacggactacggacagggacaacctgaacggacactgaacggatagcaggacagggattgacaacccgcaacggatgcggtagagtacgcaacaggtaacagagacaacggaaccgagggccagcagagggaagccgctagagatagcgccgactgctaacagagcctagctaggaagcatcggaaccgctggcatagcatacgccataggcgagccgctagacctaacctgaacctaagctgaacggtaacagacgcaacgcttgacaacagctgcaaagtgtgagaggatacaatcatgcgaggcaaggcaatctatcgctggaacgtggtggacaagcatacgggttcaatcgtaggcgcgtactccacagaatcgggagccgcaagggcagctgtcaagctggccgaaaggttcaacagtccgggccggtacatcgcccgccatcgctgaacacaagctgaacgccagcatgtagcgcaacggttgcgacctagcgcgctggtatggccttgattccacgcttgcatggcgctgtgtggatgatcgggagagttacgcccagcagacgggagggcggtgcacactggcaatgtgcacgcgaagtcgaggcatcctcggcgagcgtcaagggactacggaataacgccggagaaaggtgcgcacgcattcacaagcgcacgctatagctccaatggcgtgacctgcccgagaactaggaaggctagggattgttgcgcactgtgcacccgagctttgccttacccgtttgcaacgggactggcatagcttcagtggtgcgacactgctagaccacttcgcacgtgagtctatggtggtgcacagtgcgcagcatttccgctgcatctatcctattcggagcaagatagtcatgaccaagaccaacaagatcatggacaaggcgcagatcgagaaggccatcgacagcattgccaagcaaggcaagaagctggatggtgacattcaggctgctgccgtgggttgcatcaatcacatcgaagcatgtggtgacgtgcgcctgttcaatcgcctgttcctcgccatgcccaagggtgcacgcaagtctgcgctgacgcagtgggcgctggcattcggcaaggtggaagcgaacacgggagacaacaagaaagagcagccgttcacctatgcgaaggacaagaccaccgatctggccggtgccatcggcaatccgtggtatgacttcgctcccgaaaaagcgcccgatgaaatgttcgacgtgcgcaaggcgctgaccgccctgctgaatcgtgcaggcaaggcgcagaatgtgaacgatgccgaactgctggcgaagctccgcaccttggagccgaccgagtaagtcaacactccgcaagctaatacccactggtgcaaaccggtgggtattgtcgtgcgtgtgcactgacgaggtgagatatggacgggctggcattcagcgtgaccgtgatcctgccgctgcttatggtggcgtgcaagctgggcatcatgttctccacgtggggactggtgatggcaggcattcgacttgtgaacgcactcactcgatacatccacgtgagggcagacaatgaagccacgcatccacgctgacaacatcagcgacaagatcattgcattgcagcacccgagcgagacgttgccgcagttcattgcaaggtgtgatgccttgcgggctgcgcaaggtgcgccggttgaggcggtgcaagaggaacaacccacgtactgcgacgactgcggaggattcggccacgtgctggatggtgcgcagaagttcaagtgcatcacttgcaaaggcacaggagttaaggcatgaacacgcaacaccatcggggcacggcacccaagccgttccaatccgcgcttgcaccgtggcagaacagccagcgcgcgctgtatcaggtcatcgacaccagtgatggtgatgcggtggtcggtacgttccgcaatcgtgtgcttgccgagaggcaggccgagacctcgcccgcttaccgggtgcgtgactacctgatcggagggtaataccatgtggcatgtatgggaggaagatcagactggcacgggtgtgtcctacctgtacgccactcgtcgtgaggcacggcagcacatgcgccgtgtccgtaacaacctgttcctgtccggttggttggtgcgaggcacgcatctgctgactggtgcggaggtggtgtgatgcgcgccttcatccaacgcatcaagttcctgctcactcgcaagcgtgagcggaggtacaaggtggaggaatcgtggtcaggtcagcggtggttcccgctgctcgacagcgccaccgaggaacaagcattcttcctgcacttcgtcaagccgaggaagtatccgggcttgcaggtgcgggtcactcgcatcaagtaaccaaccatcagggcatagcccgtcgaggagtacaccatgtatcagcgtaccaccactgcatcccgtcgtcgtgaccggatgatgaacaccaactggttgcacgtgagccagtggttcaagcccaccaagatcaaggatgcactcgggatcgagaccgtgcacatgatcccgcagatgacgcgcacccagccggacgccaagggcaacccggtgcaggttgcgcatggtagcacgtacaacgtgggccgcaatcgcttcaagcgtgcgtgccgtacgctgggcctgtcccgtgtcaaggtggagcgcaacctgcgtgccggtcagagtgccgagtacgtgatggcgcaggctggtgtactgtgagtgggcagcgttacgttcctgtcaagctgatcgctggcaaggagtacgtgctgcgcaatggcaggcatgtgaccgtgcgggagaacccgcactggcagtgccgtgtcaactacccgttcgctgtcatccaaggcccggacttcgtggtgtactacgatgaggaagggaacacgggtggcggtactgcacacgagcatgacatcatgcgccctgtgtacaaggacggcgaggtgtaccttgatcgcaacggcaagcgccgagtcattgacctcgatgacaatagcagtacctatccgctggaagatgacgagcgcgatgagtcgtggacacgtgatggcagggtgagtcactgcgcaacgagcgaccgtgagaatgatctcatggactacgaacagccgaagcgcagggcgctggatgttctgcttggtcagcctatcttcaagttcccgtcgaagccgatcttcccgcctccgatcttcaatcccatcggtaacatcccgatcccgccgcccgaacctgctgacccttgggttggtaagcgcgtgtacttccgtgaagatgggcgtgaaggttacggtgtggtgcacaagcgcatgtccggtggcagcgactattacaccatcaaggtggatgagccgtgcgactggggtcacagcggtgatggcgatctcggacaacgtggttgggctgtacacaagggcaacctgactctagccgagttgcaaggcaagcgtgccgatcttgtcatcgttgacgaggtgttcgccgtgcctgaacttgcacctgtcgaagcgtcaccctcgctcgttggtctgcgcgtcgaagttaatctcgactgcgccaccactgcccgaggtgtggtcaagttcgaggacaccgatggttacgtcgctgtcgagatcgacgccgacgtgcagtggcaagggttgcacagttgcaacggtcactgcaatgacgagcgtggttggtggacgctgcgtgattcgctgcgcgcagtgagcgaggccgagacaccagtcgaggccgagcgtagcgaggccgagacaccagtcgaggccgagcgtagcgaggcgctgaccgaggtggatgttgagcgaggccgagacaccagtcgaggccgagcgtagcgaggccgagacaccagtcgaggccgagcgtagcgaggcgctgaccgaggtggatgttgccgaagtgtgggctgcataccgcatcaacccgagcatcgacatcgactcgtggatcgaagcacgacgcaagctcaaggctgctgccaagtaacagggactaggccggtgcccatccatagtggtgggcactcacgtattccctgcgcaatgtgcgctaactcaggagtcagaaccatgaggttcgcagacaagacgacgatctccatcccgaaccacttcatcagcatgcttactggtgagattgccgagatcatcaagaccatcacgcaacagatcggtggagttaccatcgagtctgcacgtggtggatacgtgattgacgacggctccctctgcatcgagggcatcagcaaggtgtcgtggtggcacgcaccgcaagagcctgctctcattcacgtgtgtaagattgcacgtgcattgatcgagcgcggcgaggaagcggtactcgttgagtaccagcgtgaggcgggcaccgttgcccgtctgctgaccaaggtggacgtggaggaacaggacgatgagtgctaaggacaacgccgtcaagctggctaacttcctgcttgacctcgccgaccgtgagaaccctgattgcactgcgtacgacacgtgcaccactcgattcgagtacgctgcacaagagcacggcttcaacctgctcggctgcggttacttcgccgatgtgttctcacatccgagtgcaccgggctacgccatcaaggtgtgcgtacgtgatggtgactcgtctcctgcgtacatggcatgggcgcgtgccaaccctggcccgcatgtgccacgcatccaccacctcaagcggcacggtcagtacgtagtggctgtgctggatcagttgcaggaaatgaactacgatgcgcggtgtgagtacgaggaatacctcgaccgctacctgtccaagaccaacgatcacccggccaacctcgtagcgcagcgcatccgtcggttctttgacggtgcatgcaccttcgatctgcatcctgcgaactgcatgatggacaagaacaatcagctggtgctgaccgacccggtgtcgttcagtgacagcgagaaatcccgtgcgctgcgcacagggatcgagcgcgcgtttgacatcgcggcttgagaacagcagcatgatccaacttcaacaaggagaaagtgcatggcactcgtagcaccccccgctgtccgtcgataccctcaccgctggcaagcgcgtcgtctattacgatcccactgccgacaaggccggtgagaagtacggcaccgtcgtgtccgtggctcgtggtgtgtcgggcaccgacgttccgtacaccgtgaccgtcgcacccgaagcgggtggcgcgaacatcaccggctcgtcccagttcttccgggtggtcgatgacttcgtgcagccgccgctgcgtgacccgaacgtctgatccatcttggcagtgctgcgcttgcggcactgcctttctccttcaccaccgtagtaccaccatcaccaacgaggatacaccatgagcgagaacaccaacgagcagccgaccgtcaccaccctgctggacgagcgtatcaaggacgcacgtgaggacgtggcgaaggcgcaggccaagctcgacaagctgctgatcgagaaggcgaaccgcgaccgcatcgagaaccttgccgctggcactgccatcaagttcgagtatggccgtggcgagaagcgccgtgtgctggacggcaccgtcgttgccatcggcgatgacccgaagctgggtcgcctgctggccgtgcagtcgggcgaaggtctcgacgtgcagacctacaagattcgtgcggctgacgtgctgttcgatgacgcgcaggaggcgagcgagtaatgcgcacctacgactacctgcatcaaggtctgacggagggtggctcggccactgcgggcaagacctacaccgtaatccgtaccaagcagaacctcaagggtctgaccgatggctggatcgcaagcaagttcgtgaccgaggatggtctgcgtctgttcgtgcgtgaaggcacgggcagcgtggcgtgcttcggacgcgacgacatcctgcggtaatcacaacgaggtgaagcaatggaagttcgcatcgaacacgacgagttcctgccacatgcagagcagcttgctgtcggtgggtcggtgcgagtgaagcattgcaaccacaaccgcaccatgatagtgagccgtgatgttggtaaggtcacggctcactgtttccggtgtggtggcaggggatacaagcaagagcaggagaacttgcaggacaaactcaatcgcatcgcagccgaacaccacgctgaacgcgaggtggtggcaagcctcagcttgcctgagccacgggtctatgaccttaaactgtggccgagagacgcggctctgtggttgtactcgtcagggttctctccttccatgatcgcacgactcggtgcatactggtgcccggagatcgggcgggtagtattgccggtcatggaggacggccatgcagttttctggcaggcgcgcgctacgaaccgcaagcccaagatactctcgccgcgcatgcgacggggtggactggttgcgaagtacggcgtaggcgacactgttgtactgtgcgaggacatgctctcggcgtacaaggtaggccagatcacggaggcatggtcgctgctcggcacggcattgaatcctgcaccactcgcagagattctgtaccgtggatgtgatgtgatcgtgtggctcgacggcgacaagccggggcaagatgccgcagcaaaaattctaaagacgttgcgcgcgcatggcattgcagtgcgcaacatcgtgacagagaaagacccgaagaaatacaatcgtgcattcattaaggagcaactatgtctctcgacctgacgctactgcgtctgatgaaacatcgcaccaagttcgaccggctcatcggtggactgccggacgctggtcttgaggagacaacgaccgtactcctcaacgacttcaaggcatacttcaaggagtttcccgaagtcaaggtcatcgactactccacgttcatgctgtggttcgagcagttcaagcacacacagtttgcacctgaacgcacgggcatgttcgatgcgatcatgaaacgtgcagccgaggacatcacgcctgacgtagaggaaggattgatggagcggctggtgtctgccgaggccagctacaaactgattggcgtggtcgagcagtggaacagcggagcagagttcgatctgctcactcgattgcaagaggtggtagaggacttcgagaagaacatggatcgcaaggtgcgcactccattcgtggaggatgcaatcgaggacatgctcaaggaagatgaggacgacagtggtttccattggagactcaactgcttgaatggaagcacgcgtccgctgcgtggtggtgacttcggcatcgttgctgcccgtcctgacaagggcaagaccacgttcctcaccagcgaactgtccttcatggtgccgcagattccgcgcgctgccgatggtagtgtgaagccaatcctttggttcaacaacgaggggccgggcaagcgcatcaagcagcggtactatcaatcgttgcttggctgctccatccctgaaatggtggagaagctgcgtgctggtacgctgaccaaggaactattggaagtgacaggtggcatcgacccgaacctgttgctgcgtatcgtggacgtgcatgacgcgcgcagtcatgagatcgagaacatcatccgcaaccatccacctgcgttggtggtgctggacatgatcgacaacatccagttcagtgggctggctgcgaacaacgggcagcgcacggatcagatgctcgaagcaatgtaccaatgggcgcgcaaccttgccgtcaagtacgacgccccgttccttgccacctcgcagatcagtgcggatggtgacggcttgacgtatcccacgttgccgatgctcaaggattccaagacaggtaagcagggtgctgccgacttcatcatcactctcggtgcactcaacgatcctgcgatggatgggttccgatacatcggcatgaccaagaacaaactgcatcgtagtggtggacgtaaagacccacgcactgaggtgctgttcgacatggagcgcgcgaggtatgagaaccccgacgactaaaccgcacatcgtaaagagcggagcctactggtctgtgtatctggacggtaggctcatcagcagttggcctacaatcgaagcagcttggctgcgcttcaaggagaacacagaatgaaagctggcatcctcgtgagaggaggtagcgcgtgggttggtgtgcattggtcgtcgttcaatcgacgcttctgcatcaacctcgtacccttcgtcacgatctggatcacactcaagggaggcaatgtgccatgaacagcaacggcatccacatcacagtgtaccgataccaagacaacaagcgcatcgaacagacggtggtcatacctgaccacgacctgacggacttgcgctacccttgcgagttcatcgcaacgagagttgtcgagactatcaacaacgtgcaccagcatgtgcgtaataaaggaggcacggcacccgccgcgctcagtgtgcgcgcatgacgtacgttgtgtgggacgtagagaccacgatcaaaacctacaacaagaggaaggcgtcgcccttccatcccgagaatcacatcgtcgcctccggcttcaagcgtaaggggatgacgaaagcggtagccgattacttcggacgcaagcgtcccgagggtgattggttccgcaagctgctggctggcacgaagatgctggtcggcttcaacatcaagttcgatctgctgcatgcgctgcgtgacgaggacaactacacggcatgggtcgagtacgttgcgaacggcgggcgcgtgtgggactgccagcttgccgagtatctgctgcatggtatggaacgtgagcatcacatgctgtcgctcgatgaggtggcaccgaggtacggcggtcacttgaagaacgatgcagtcaaggcgctgtgggaagcaggcatcgacaccacggagatcgaccccgatctgctgctcgaatacctgatcggtgcacccaacgaggacaaagaccttggtgacatcggcaacaccgaggctgtgttccttggtcaagtcgatgcgctgcgtgcacgcaagggtctgaactctgtgctgctcaacatggacagcctgctgtgcaccacggaaatggaacgcaacggcatgttcatcaacaagaagctgggccttgagttggccgagcaacttgagattgagttgcagaaattgcgtgccgagttgcacaagtcgttgcccgaggacttgccattcgagttcaactggggcagcaggttccacctgtctgcgttggtgttcggtggcaagatcaagtacgtggcgaaggagaccatcactgacgacgagggcaacctcgtgtactaccagttgaaggagaagcactatgtccttaatgatggatcgaccactgcaactccgccttcgggaactgatgcgctcaactacgcgacgttcactggtggcaagaacaagggcgagtacaagaccaagcaggtcaccgtgcctgacattgcacgagggccgaagcaacgcaacgctgacttctacttcgagttccccggctacaccgagccgtctcccgaatgggagagcagcacgccgggtgtgtactcagtagcgagcgaggtgatcgaggcgctaggtaacagggacatcccgttcctcaagtcgctggcagaaatggcgtcgctcgtcaaggacttgggcacgtactacatcaccaccgatcccgagactggtgagagtaagggcatgctgacgctcgtcggtgacgacagcatcatccaccactcgctcaatcacaccagcacagtgacaggtcgcttctcgtccagcaatcccaacttgcagaatgtgccgaaggaaggcaagtcgcaagtcaagagtgttttcgtgtcgcggttcagcatgggcaagatcattcagtcggacttcacggcgctggaaatctatgtgcagggcaacctcactggtgacaagcgactgatccaagacttgatcgacggtctcgacatgcactgcctgcgtgcagctaccacgttcggtgcggactatgacttcgtgctgcttgcatcgaaggacgagaaccatcccgagcataagctgtggaagaagcggcgcacgaacagcaaggtgttcagcttccagcgtgcgtatggtgcaggcgcagcgaagatcgcggcgactaccggcatgcctatcgaggaagtcgaggcgctgatagcggcggaggagaagctgtaccctgcggtgactgcgtactacgaacgagtcacacagaagatcgcagagaatcgtgtgccaacgcagcgattcgtgcaacacccggagattgcaggcatcacgtgccagctggggcgctcgcacttcaccacaccagatggtaaggtgtacagctacagcgagcaaccatcgccgggttggttggtgcgacagaagaagatcacgcagtccttctctccgaccgagatcaagaactatgtggtgcaaggaacaggcggcgagtgggcgaaggcagcgatggcgctggctgttcgtgcattctacgcacacaagaactttggcggcaggtcgctgctcgtgaatcaggtgcatgacgcactctatctcgatagctcacccgaagtcgaagtgcaaagcgcggccctactgcatgcttgcatggaggaagccagtgcctatatgtccaagctgttcaactggaacattgcggtgcctgtgcctactgaaaccaagagcggtgccagcatgatcgaggaacatgatctgccggaagggttcaagctgcaagtcaagagctaccgcacatgggtgcgggacaactacatgccgggattcgtcccatcattcgagaaaggagagtaacacatggcattcaatctgcgtgctgctatcgacgctgcaaagaacaaaggcccggacatgacgcaagcgtctgccggtggtggtgacttcgagttgcccgccgagggtttcgttcgactgcgcttcgtcggttacttcgagactggcaagaaggaatcggagtggcagggcaagaagaaagtcaacgacaccgccgagttggtgttcgagttgagtggcccgaagcatcagccgcgtgacgtggacggtacgaagtacccgatgcgtgtgaccgagcgcgtcaagctctcgctcaacgagaagtccaacttcttcaagctgttcaccgcgctgaactgggaaggcaaggccacccacatcgccgagttgctgggcaacgattacgttggccgcatcgagcacaacaagaagaagatcgacggcaaggacttcacgttcgtgaacctgcgcgatatccgcaagccgttcgccaccaacccggagacgggcgacgagtaccgcatcagtgtggatgccccgctcacggaactcaagctgttcctgtgggatttcgccacgccggaaatgtgggacagcatcttcatcgacggccagtacgacgaacgcaagaacgacaagggtgaagtgacctcgcctgctcgcagcaagaacgtgctgcaagagaagatcatgaaggcgctgaactggaaggcgtgcccgatctacgactacgccaccaagacggtgacgaaggacgacagtgctgcgctggatgcagcggtcggtgatgtcgaggaagcgcacgcacccgaagaaggtgaggatgcgatggagggtatcgcctaatggacatcgcagcctatgcagcgaaggctgcggctgcgaatcctatgcccctcgtcaatgtgcccagccccacggaggggctggttgcacacgtggacggtgacttctgcgcgtacaactgtgcgggcagcgacgacaccgaccccggtcaagctcgacgcaacttgctgtcgaagctggactcgatcaagtttgcatcaggtgccacggcagtggtcgtgcatctcactgaccgggccagcacgaagggcgagagattcctcgccgcaactgtcaagccgtatcagggtcaacgcaacagcgggcgcaagccaaagaactgggaagttctgcgtgagtacatggagacgtacgagggtgacaagttccgcgtcaagaactggatgacgcgcgaggccgatgacggcatcgcttacgtcacacaccacgcagctgaccacggcaagctgtccgttatctgcaccgcagacaaggacatgcgtatgctgcccggtcgtcacgtcatctggaaaaccaagcagctgatcgacgttccattcgggacgtacgaaatgattggccccgatgatgagacgtacggacacaagtggttctggctacagatgctcatgggagacacggcagacttcatccccggcttgcccaagtacatcacgccatcagggaaggaggcgcagctaggcaagcagacagcgtacaagctgctcgcaggtacagagaacaacgccgaggcttacgccgtggtgtccggtctatatcgagggtactacgaggacgagtgggccgaccgattcgttgaacaagccacgttgttgtggctgcgcaccgacaggttcgccggactgctggacttcatgacgctcattccgtttgcacgcagtctcgatgaggctggtcaacgtctgtgtgatcgtgtggctacagcgcgcgctgaggtggaggccatactatgcggagactgaaacatgcagaggttgcgactgtgcgtgccacgatgcttgctgaccaacggaatctgtgcggtgtgtgcggaacccccgtcaccgcgaggcccgtcttggatcacgatcacagcactggcgctgtgcgcggtgtgctgcacgctgggtgcaactcactactgggcaagctagagaacaacgctgcacgctacggcgtgcgcaacatcggcgtgttcaccaacggtgtggctgcgtatctgcgcaagcacatggtcaatgtaactgggttacttcatccgacccacaagtctgaggatgagaagcgcgagttgcgcaacaagcgtgcacgtgcttcgcgtgcgaagaagaaggagactcaatgaagatcacccgagtcaagagtctcgacaagttcatccgtgtgtctgatcgaatgattgggccgaaggtgcttgtcgctgacatcgagacgttccctatcctcgcttatgtgtggggattgttcaagcagaacatcagcctcgaacagatcgccgaggactggtcgatgatgtcgttcgcgtgtaagtggctgggccaccccgaggtgtactacctcgacaaccgcgaccgtgatgatccgaaggatgactcgatccagctgcatgcactgcatgccatcctgtcggagtgcgacatggtggtagctcacaacggtgcacgcttcgatctgccaaagatcagggcgaggctggcgttgaacggacacaagccgctgccgccgatcaaggtcatcgacacgctgctgctgaatcgtacagcctttggcttcacgagtcagaagttgcagtacgtcagcgacagattcgcagtcgatgcgaagtccgaccacaagaagtatccgggttggaagctgtggctgggctgcatggcccatgacattggcgcatggcgtgagtgtcaggcgtacaacatcacggacatcacggcgctggaagaagtgtacctgtccactcgtggctggcatagcggtggcccgaactacggcccgtatatccacaacgaggaaggcgaacacaactgcccgaactgtggcagcagcaacgtcagcaagcaaggaactcgcaagacgcaggtgggcatctaccagcggtacagttgcgatgactgcggtgcttggagtcgtggccgtgtgttgatcgcgtcgaagaagcagcgcgcgcacatcctgatgaactaagaggaacgatgatggccgacgtattcattgcgggcgaccgagtgcagtacgtcggtcagcatcacagccgcagaggcaggaacaaccgtggtagggttgctgcacaacaaggcaacctctaccgaattaactacaacgacggcagtgtcggactcgccagcgcggcgaaccttcgattcacttccgcacaaatgtacgccgacgaggaggcacgattggatacacagaacgagcggggcttgggcctcaagtacgatgcaggcaagccgcaggcacgactggtgttcgagggtttccctctcaccttcctcgccttggccgacgtgctgacgatgggtgcacgcaagtacagtgcacactcgtggcagcatgtcgagaacggcatcgaccgttacagtgacgcagctgcacgtcacatgctggctcgcctgagtggcgagacgcacgacccggagtcgggtctgatccatgaagcgcatgaactcatcaacaggatgttcgtgctggaactcaagctgcgacaggagaaatcacgtggcgcagagtaagagtcgttccgtcaaggaagcgtgggtcaacatagccatcggctattccatcaactacagttgtaacatcgcgctgctgcctctgctgtggcacccggaacacccgttcctgtcggcgcatgccatcggcatcgcgttcacgctcatcagctttgtgcggcagtacatcatcaggcgttggttcgccaagggagattgacaatgagtcaggcatacgaaaagacaatgtttctgttcgaggaatacagcgaccgtatcgtgtacggttccgagcaggaagatgaggcgttgcagaacgcggtggactgggtgttccgtgatcgcacggatgacttccgctccgacctgtacgctcgcatcaaggaaacttgggacgcatgcaccatcgaaggtcggttcgtttacacgcagcagatcatcgagcaggaggtggtgaatggctgagtacatcgtgcacaaagctgtggagttgtcgaaggtcaaggcgaagcggaaggctgaactcagcgtccagaattaccttgaagaaaatttcatcgcacaacccaagtacgacggctgcaacatggttgcgctgttcgatggtgcaacggtggacttcttctctcgcactggtgagccggtgctgagcgtgcctcacattgaaatggcaatggctacgttcccgaacatgacgcccggtgcgtacttcggtgaatgctgggcacctgatctcccgttcaacgagatcagtggtttgttccgcaggcagactgcggacgaggacacgtgccgattgcagttcgccatcttcgacttcatcacgcccgaggagtgggacgacggcgtgagtaccgttgcctatggcaaccgcgttgctcgcatgacgccgcagctgtctgctattccgcaggcattgaatcccatctggctcgccggtagcttcggccacatcgcagagacgtgggcgaacaccactgcgcaggacgtgtgcaacaaactggtcgaggcaggtggctatgacggcctgatcctgcgtgatccatatggacactggcgcaagggcgaccgtggtactggtggtgagatcatcaagatcaagcgcaagctgtcgttcgatctgcgtgtggtcggcttcgagccgggtaagggcaagcatgcaggcaagatcggctcgctcatcgtggagttccgtggtcagcgcatgggtgctggcactggtctgcgcgacgacgagcgtgacgtggcgcagttcgagaacaactggctcggcaagatcgtggagatcgaggctatggactacagcgccgatggtctcctgcgcgagccgcgcttgaagggtatccggctggacaagttggagcctgacgcatgactgtgatcgcatgggacggaacaaacttggcgtgggattcccgcgccacgtcggatgaccgcaagcatacagtgaagaaggcgcgcgcgttgaaggacgggcgcgtcatcgttgtcgctgggctgctgtcgaatctcgtgcaggcacggaagctgctcgacggccacggctatcccgaattgccgcagtcgttggtggatgcgagcgacatcatcgtgtacgacaacggcgtggtgtatgcctacgacgacgcgaaggaagtgcggaaggtgaaggcacccgaagcatggggttccggtgaagcatacgctctcggtgcgctggcctgcggtgtgtccgcagcacagtcgtgcaagatcgcatgcaagtacagcgccacgtgtggcggaaagatcaactcaatctgaggtaacgatgcagacacaagtggaactcgaactggaagcctaccaatttggtaaggctcgcatggccgcagctatgcggggcaacgaggagaagggccgcgcccacaacaacccgtatgcccaagctgtctatcgccggttcgtccttccgctcgcggagatcatccgcgaggacttggctgcgaagcgggtggggaggcggcaggcgcatgtgcgtctgctatctcccatcgacccggaggcgacagcgtacattgtagtgcgctccgcactcatcgcactccttgcaggcaagggcgacaatctcgccgagggcgcagggcgcagcgtggttgctgaggttgggcgtagcgtgtatcacgagtacgtgttggaacacttcgcggagatcgagccggacttgttctaccacttggtcaatgacttcgagcggcgcatgtcgcacaatgaacgtcaccgcatgaccgtgttcaagatgcaggcacgcaaggctggtgtccacttcaacgagtggagcagtggcgaccgcgatcaagttggcgcgtatctgatggagcagctgtctaagctgggcatggtgcataccaagcagatcacgatcccgcatgtacacaagaacaacatccgaaccaagatcatcgttacgctctctgaggagtgtgctgcgttgatcgagcagatcaagggattcgcagtagagtccacaccgtacttcctgccgtgcgttgaaccgccgaaggattggacaggtgtgaccgagggtggattccacaccaaggaaatgcggcgcatgatgccgtggatggtcaagacccatccgtcgcagcgggacaacttccgtgaggcggacatgagtcaggagcttgcaacgatcaacgcattgcagcgagtcgagtggcgagtcaatcgcaagctgctcaatgccgtgcgccagatcagcaagcacttcgacatggacgagatcatcagtcaggccgaggttccgaaaccgcacaagcccgagtggctggtcggtgacatgaccaaggacgacatggacgagacgcagcttgaagaattcgtacgatggaagcgcagcgtagccgagtggcacaccgagcgcaaggttcgaggtacgaagtggggcaggttctacaacgctatgcgcatcgccaacaagttcgaggagtacgagaagctgtggttcgtttacttcgaggacttccgtggccgcaagtacgtgcagaccacgggcatcagtccgcagggaagcgacttgcagaaggcgctgctcgaattcgcaaacggcaagccgctggattctgaggaggcagtacaatggttcaagatcacaggagcgaaccgctggggttacgacaaggtgaccttgcaggatcgagtgaagtgggtggacgaacgatccgacttactcctcgcctttgcggacgatccgatctcgcatcccgagtggcaggaagcggacagtccgctctgtttccttgcatggtgcatggagtacgcggagtggttccgcagtccttcaacattcgcctcgcgggtggctgttgggatggacgggagttgcaatggcttgcagaatttctctgcaatgctacgcgattcgctcggaggcaaggcgacgaacttgctgccttccgagttaccgaacgacatctaccagatggtagcggatgttacgttgcgtttgctactcgctggggaggaggacgagcgtggctttcgtcgccgctggcttgcgcacgggatgaatcgaacgctggtgaagcgcagcgtgatgactctcccgtatgggtctacccggtattcatgcgcggagttcatcgtcgctgactacttgcgcggtggcaaggtgcctgagttcgagaagggcgagtacgagaaggctgcgaattacctgtcgcatttcgtgtgggctgcaatcggtgaggttgtggtcaaggcacgtgaggctatgacgtggttgcagcaaggcgctaggcagttggtgcgcgagggcaacaccgagatcaagtgggtcacgccatccggtttccctgcgatccaagcgtactgggagtccgacgtgcaccaaatccacaccaagctgtgcggtggtgcgcgcctcaagattcaccacgacaccgataccccggacatcaaccggcacaagaacgggatcgccccgaacttcgtgcacagcctcgacgcatcccacctcacgctcactgtgaacgccgctgtggccgagggcatcacgtcccttgccatgatccatgacgactacgggacgcacgctgcggacgcgccacggctgttccgcatcatccgcgagcagttcgtcggcatgtaccagcggcacgacatgctcgccgagttccgggcgcgctaccccggcctgcccgatccgcccgagcaaggcgacctcgacatcacgcaagtgcttgaatctccgtactttttcgcctgacggagtttcggcaccctacatagacgagacccacctctgaatccctcgggtaactcaagtgggtttcggcaccctacatacacaggagaaaccatgctccgcaacctcatcaatcgcctgctgcgtccgctgctggcccagcgatacatcgtccggcttgagccgttcgttctcgctgacctgcgccgcaaggtaggaggcacgtgtatcgtgacctcgcagaccaccgaacacatggctggctaccaacttggaatcgcccatgtcctcaacgtactgcaagaaggttacaccgtgtcgcgttcgtaaggtagatgcaagggatcgttcccgcatctattgccagatagagaaggcaagacagcgagtgaaagactccgacatcaccaagctctcgtacaccgggtacgctacggaaatgattgtactgggtggagtcgatgcactgatcctagatgaagccttcctagtagtgtacggcgtaggttcaccgtggtactctgaccgagtattccttgaggagaagatggtacttcgcattggcgaaggttccagctttgcctcggtgtgtgatctgctggacgacttggctgttgaacatgacgccaacgacatcatcgttggtggcgcactagccaagtatccacgggcactcattcggatgtacaaagctcgtgggtatgaactgatggacatcccctcactaatcaaacggaggtaatcatgggttcgattttcggcggaggttccgccaagcgagccgcgaaggaacaggcagctgccactcgtgaagccgctcgccgcgctgcggttgcatccaactaccaagccgagtctgctgcacagcagatgacgctggctcaggaacagcgcgcgcagcagcagtacgcgaacgacttgctgtccaccccgatggaatccgcgacggtcgatctcgccgcacctgccgacgaaggcggtgacgatgatctgctgacccgacgccgcaccacgcggcagacctatcaggcagaccgacgctccggcctcgccgtctaaggagtaggcatgcacgctgataccgcatccgggcggtggagcgaactggactcggatcgacagactttcatcactcgatgcgaaaagtacagcgcgttcaccatcccgaagatttgccttcccgaaggctacaaccaaaacaacgacgagttgcagcacgactaccagtcggtaggcgcgcaggcagtgaaccatctgagcaacaagctcatgctggcgctgttcgcaccgagccgcccgttcttccgccttgacccgtccgacaagctgctcgcacagatgagcgagttgggcatgtcgcgcgatgacttgaacaaccagctgtccactgcggaacagtcggcgatcaaggaactggatcggcgctcgattcgtccgaagatgtatgacgcgatgaagcacatcatcatcacaggcaacgccctgctggtgatgggcaaggacagcatgcgagtgctgggcttgaagaactacgtcgtgaagcgcgacaccgatggcatggtcttggagatcgtgaccaaagagtgcgttgacaagcaaggtctcgatccgaaggtggttgcagaactcggcgagaagctgacgtgcagtcccgatggcaaggttgatctctacaagtggatcaagcggcgcgaagatggcgactacgaactgacgacttgggtgggagcagacaagctctctgacaagttcgatggtaagtggcctgccaacaagatgccgtaccgcgcgatcacgtgggacttggcaagtggcgacgactacggcaccggactcgtggaggactacgctggcgacttcgcctccttgtccatcatgtcgaaggcaaccgtgcaagccgcgatccttgcgtctgagttccgctggctggtcaacccggctggcatgacgcagcccgaggacttggagaaatccgagaacggcgcagcacttcccggtgtgcaaggcgacatcagcctcgtgcagtccgacaagtccgctgacctgcaagtcaacgtcaacatcgcgcaggaatacatccaacgcatcggcatgggcttcttgctcgcgtccgccacgacccgcaatgcggagcgcgtgacggcggaggagattcgccgcaacgccgaggagttggagaactcgctcggtggtgcgtactcacgcatcgctgtcgatgtgcagatgccaatggcgtactggctcatggatatgtccggcaagaagattgccggtacggacatcgagccgaccatcgttactggtctcgctgcactctcgcgttctggcgaccgcgacaacttggtcttgttcttgcaggacgtgaccatgctcagttcgttgccgcctgatctccgcaaccggatgcgcattggcgcaatccaatctgcattcgcgtcagcccgtgggctgaacgtgtcgcagtacctactaaccgaagctgaattccaacagcaacaggctgctcagattcgtgaacagatggcgatggagcttgctaaccgcatgcccattgcaaacccggacggcatcgacgcctcgcaagctctcattgcgagccgcgctgcacaaacggctgagtctgctcgcgcagaacaagtagcacgacaggagtaaagaatgactgacatcctgaacccgaccggcgcacctgctgctccggcccaaccggctgcacctgcggcccccgctgctccggctatcgacccggcaactggtcagcccgtcgcggctgcacctgcggctcctgccgcaccagctgctccggcacagcccgcagcacccgctgctccggttgcggaaccggcatccacgaaggacgacaagactggcgtggtcacctacgagccgactggcgacgtgggcctcgacctcgctctcgaattcttcggcaagctcggactggacttcgcgtcccccgaaatgcaggaagctggcaagggcaacttcgcttacctcgaagccaagctcgccgctctcggcgacaaggcgcagggtggcgaccgctacctcgctctggcgaaggacgcctatggccgtctgcaagccaacgacaagagtgcatacgaaagccgcaaggctatcgcgcatgaagctgtcggtggcgaggagacgtggaattcgattcaggagttcgtgaaggcgaacgctgaaccggaagaactggaacaggtcaaggccgcgatgttgcagggcggtgtcgttgcgaaagcaatggccgagcatctgcatcgtctgtaccttgcctcgtccggcaccgtcgcggaaccggcatcgccgacgcgacatcaagccaccgcacctgctggtggtgcaccgctgacccgacagggatacctcgaagaactgaatggactggtcgctaagatcggttcccatcgactcgacgggtcacctgaatatgcggctctgcgtaagaagtacgcaaacatcaagtgatccaaaccaaggagtaatacatgcctctgtttaccgttaccccggtgcgcccgaatcagcagaatcagtcgggtgcgctcgacgcactgaacatcacggagttcaccggcatcgtggagggcaccctagcccgtacctcgaagctcgacccgtacatccagcgtcgccgcgttgtcggcaccaactcgctgaccaactacgctgtcggtgagacgcagctgcaaaccttgcagccgggtgtcgcgccggatggttcgctggtctcgttcagcaagctgaacctcgtgatcgacacggtggttctggctcgcaacatcttcccgctgctggaaaccttccagaacaactttgacgtgcgcaagcaggtcggtcaggagcagggcaagaagatcggcaagttcaccgatcaggcgttcatgatcgctggcatcaaggttgcccgactggcgaactccgcctacgcgaacgtcgctggcgacaagccggaaggccacgctggtggtcacatccagaccctcgcttccgctgcggacgcgaccgatccggctgctctgtatcaggccatcgctgacgcgctggttgcgatggaggagaaggacgtttcgccgcagaccgaggacgtgatgctgatcgtccgtcccgagcagttctacgtcttgcagcaggccgagcagatcatcaacggtgaatacctcaccagcgatggcaacaagctgaccggcgtgccgatcttcaaggcgtggggcatcccggtgatctcgtccaacaacctgccgaacaccaacatcacggctcacccgctgtcgaacgcgaacaacggcaatgcctacgatgtggatgcgaccaaggttgtcggtctgctgatctcgccgcgcgctctgctggctggtgagaccatcccgctgaccagcaacgtgttcttcgatgacctgtcgaagcagtggttcgtggacagctggctgtccttcggcgtgaccggcaaccgtgccgagttcgctgcgaccatcgaaattccgtaatgccaacgaccgggagtggagcaatccgctcccggtttctttcgtcttaggaggactgaatgttcatcacgcagcttgacgtagtgaatgcgtgcctcgctacgatgggcgagaccccgctcaatacgttggaggacgaccacagctacaaggctgcggccctgtcctacctgacgcaaaccaaccgcatcgaacagaagcgcggctggtggttcaacagcgagtacatcgaactcgtacccgatgtcagcaagttcatctacattccgcttgacgccatcgcggtaaagactgtggatcgttggtacacgccgccctatgcgcagcgtggtaagcgactctacaacatcgagaagaacaactacgaatgggaacagaaccttgtcgttgacatcgttcgcttgctctcgttcgatgatctgccgttccatgcagccgacgttgttggctacggcacggtgatgcgtttccagcgggagttcgatggtgacaccactcgatacaaccagctgacgcaggactacgcacgtgcgcgcgctgaactgagcgccgagaacacgcgcaacaaacggcccaatctgctggcaacgcccagcaatcgctataagatgggactgatcggtggcttcggtacgcgcggtgcgcgaatcccgtggactccgggctacccacgataactgaggagttcccatgagtaaggttggaggctcgtacgattctgttgtcctcggcgtgtccgagcaggttgcacatgaccgccgaccgggacagcatgaggaacagatcaacatgatctctgatcctgtgcatggactcgcgcgtcgtcgcgggtctgtgtacaaggacgagttccttgttggcgcaggcaccctcgcagaattcggaacagaggcaggcgcaatgcgcgagtacacgttcgtcatcgacggcgtggaatactgcctgctgtttaggacgaaggcaagcacgaaaggcaagccgacgttcatgtatctctacaacaagaccaccgacaagttcatgcccatcgtctatgagaatagcacgtgggtcgatcagctggtcagtggtggcgctacctgcatggcaagtgtagggcgctacgtgtacatcgctggccgcaccaccatcccacagctgactgtgacggatgtgtgggacgttaccagcaatctgtcgaagctggtggcgtggattcgtggcggcgcatactcgcgtacgttcagcatcacgctcactcgcaccgatggcacgaagctcacggtctcgtacaagacgaagccgagcgcgtatcccgaattgctggacaccagcgacatcccgttctacgagcctgacggtacgactccacgtgaggactatcagaaggacatcaacgaccgcgtgtacgcctacaactccgcagtgaacgcctacatcggcgaggctgctgaggacatcactggcgagaacatcgcgcagaagttggtggacgagttgctgcttgaaggtgtggctgcttcacggcaggacagcacggtcatcattgacgacgctgacttcgtggacatcagttccgatgacggtggcgacaacacgctgatccgcgcagtcggtaaggaagtgagtgcacctacgctcatgaccacgatccactacgtcggcaaggtggtgcgcattcgtccgcaaggcgcgagtgacagcgagtcctactacctgaccgcgtacgccaaggacgacgtgagtaccggctggacagaagtgatctggcgcgaaggcgttggtgtgttgcagcagccgacgcgcatgttcgcgcaggctgtgattcatgcgggcacgatgtacgttgcgcagaatggtgcgggtctcgaaactctggctcctgccagtggcgagcatcccgactacaagcccaacgctgtcggtgatgcagtgagcagcccgacgccggagttcttcggtcggcccatcacgatgatgacggtgttccaagatcgtcttctgctcggcagtggcggtacggtgaactgctctcgtccgggtgactacctcaacttcttccggcagacggtgttgacgattcaggacaacgaccccatcgaaatgttcagctacggcgctgagggtgacacgttgcgcagtgcagtgatgtacgaccgcgacctcatcatcttcggcgacctcaagcagtacggtatcacgggccgcagcgtgctgtcggcgaagtctccgaacatcacgacggtatccgcacacgaggacgcaacaactgcgttccccgttgcaagtggcaacttcgtgttctacggcaagaacgcagacggtgacgaaggcgatctgcgcacgacgctgcaccagttgcagatcggccagctgattgaatccccggtgtcgtacgaagtctcgcagcagcttgaccagtacatcaagggcacgccatgtcagctgatcgcaatcaccgcaccgaacatgatcctgtaccggactgaggaagtgcctaacgacatctacgtgtacgcatacgtggacgatcagggcggcggtcaacgcttgctcgattcgtggtcgaagtggcattaccacccaacgctgggtcgcatctgcggcgtgagcgcgcacaacggtacggctctgatcttcaccatgcgcgagcgtggagcgaatatcgtcatcgtggcagacaagcagagcgtcaacaccgagcttggctctctgccgtacatggacagcatgaagcgtggcgacttggttggcaccggctggcacagcgttgtcgatcacggtctgctcgcagtgtccattgacagcacgtccaactacttcctgctcggcacacaagctgacgaagttgcggacttgctcgaccagttggacggtgtgaccaacacgcagttgtggtacggtgtggtgtccgatgcaacagtgacgccgacgaatccgtacttccgcgacagcaacggtaaggcagtcctcagtgggcgcttgaccttgaaccaagttaaacccagcgtcaccaagaccagtggactgatcgctaccgtcacgactgtgaacggcagcatcacaaccaccgagttcaacgggcgcgtcctcggactgagcagcaacctcatcgctcgccagcccacgccgaccacgcagctgaccgtgggtgttggccgcgaggtacgagagtgcagctacacgttcacgtcgaaagactggttgccgatgacggtgaccgcaatcgagtggacaggtcaatacttcaaccgagtgcggagggctggttaatgggtagcgtaaatacgatcatccaagccaacaacatcactcgaatccagaagggcgagtacgatgcgaaggtgatgatccagcaggcgaacaacaagcgcgaggccgcaaaggtttcgctcgcggagttcagccgctcgctgggcaataccttgcgcattgaagccgcaggcaaggagttcaacgaagcgaccagcaatcttgctgcgtctctggaaggtcgcacgaccaaccggctgaactcctcgctggctgctgctgaacgcatgggtgcactggccgcgcaggctggtgcactcggagttggtggttctagcgttgagcttctgagcgacacgatcaagctacagcgcaatgtggagcaggacttgcaacagcaggcaaccactcgacttgctgcacaaggtagtcgtgcgaacgcgcagatcatggacaacgcctacaatcagattgacttgcagcagacgttcggctcgttcgatcatacggtgtacatcgcaccaaagcggatgaagcgccgtctcggtaagctgattggcgtggcggtagcaacatacttcggtggcccgcgagctggtgaagccgtggctgacttcgcagtcggtacgtggcaagctgacaacgcgaacttccaaggcatgtcgcagtctttcgactctggcttccagaacgcgatcaagggctatcagacgtggagttcgctgcaaggtggcgatggcccgaagtcgtggttcggtgcggtaacgcagaagcagaaccaacaggctgacgccgctgcggcgaagaatcagaacatcaactggggtggcttcactccgggcgaggactcgacgttcggctctggattcggcaacaactgggattggctgttcggtggcacgggcagcgatcaataactaggagacaacaatggcagagatcaacgcagcaatgcctgtgttccagttccaaccggaaacggtgcggagcagcggggcaggggcatccggtgcggcaccgcgcctcggtgtctccggtggcgaaggttcacgcgcaggcgtggagatcatcgccgacacacgcgacttgggtgcgggcagttcgctgcccgccttccttgaggaagcgtttgctccgaagctgaaagctgtgcagcagcagaagttttggagtggcttcaccgcagcgcgcgctggtaagagcgcggctgacatacacgcagagcagccgtggtacgcgcacatcttcggccccaccagctacgagcttggtgccgagacgttcgcggtgcagaaagcagcgagcgacatggagacacagttcatcgagcgtctgcccgagttgcgcaagatgtctcccgaagaagtcggcgtcgaactcaacacgatggcgacgaacatgcagacgggcaacctgtacacggacgcactgattcagaagtccatgatggaacgtgcaggcccgatgatggacacgcacatgaaggcccgctatgcgtggcagcaagaggaactggcccgtggtcagaactcggcgtggttgtcggcaagctctgcattccaagctgcggctgtcgatgacgccaagcgcgggcgcgaacatcctgcggaggctccgactgtggagcagctgcgcgagcgtggtcagttgttcttgcagacgttccaatcccccgagggacagaaccccgagagctacctgaacaacctcctgacgactgtcgatcagatggccgatcaaggtgactggtacagcatccgtgcactcgaagcgagtgggctgcttgggcagctgccgcccgaggacagggacaagttggacggtcgcattgatcgtgcacgctcgaagtacaagcgcaaccttgcaagcggcccgctgatgaagcccatcgcacagttgttcacgcaagcgaaggccggtgctatcagcgccgagtctgcggtcaacggtatgttcgagatcaacgcgcagtacgctgcactgactggtgacgacaccggcttgttcgatcaggacgatgcaatccgcattgcggagagcgcgggtggtgcgtactacagcatgtgggaacgcatgatgaacaagcgtgacgctgccatcgagaaggctcagacggctgcggagaaggaagcagccgaggctcgcggtgacgcgcagctggtggctgctgtcacgaccaatagcatcggcaccgtgtcgcacatgaagggtgtgacgacggacgacgccgaccgtgcgttcaattccgtcatcgaccaaaaccctgcgatgctgccagaggttgctgttggcaactacgcagtgtccacgagcggcaaggagccatacgtctccgcacgactcaagacccggttgcagaatcaggttgcgctgtcggcgggtgaggaatacacggacgggttcgagcaggcgtatcaagcgtggcgcagtattcgctatcacgagatcgacaatggcaacggcgtgactgatcggacttccggtctgtccacggccatcgaatactacgggccgttccagacgcagatgcaggcgtatgacgatcaggtgcgtgcgggtactccgcgcgagatcgcttatcgtcgtgcgttcggcaacgaggccagctacgctggtggcaacttgcgaggcgtcgatgccgacgcgaccaaggccgcacgcgagcagctgaccaccgtggtacagcggatcaatccgtcgtggtggcagctgggttctgagtcgatgggttcgagtgcgaccaacgtggtgaccaacgccgcgtctcgctacttcgagcagatcaagcgcaacgatcctgcgatcaatgatcaggaagctgcgaaccaagctatccagatggcacaggccaatggcttggagatcagtggtcgctacgcatggcagaacgtgcgtggtcagaaaccgctgtacgctgaggctggtatgcagaaggacgtgttcgaggattacttcgagcaagccctgaccaaccgcttccgtgcgcagggcatgcgcatcgctaaggacaccagcgtctcgatcatccgcatcggcaacgacacgaacggcccgcgcctcatggctacggcgtatcgtgatggtgagcgcaagacgatctggatcactggcgacgacatcaagaagctacgcaatcagcgagccgagtacgaagtgcaacgcaacaacaccatgatccccggccagcgtgtcggtgacatgatccgcatgcctgatggtagcctgcaaagggacatcagcattcaacccaaactctaaggagcctacatggcgctggaaaatctcaaaggcttgtctcaggacgaacagttcgaggctgctgcgaagttcgctggtgttccggcgtctgtcctccgcggcatttggcgcacagagtcggcggagggcaagaacatgctctccgccgccggggcggaaggacacttccaaatcatgccgaccacgcgcaagacgtgggaggatcgcgtgggtcgcaagctcgacccgtacgacttcgcggatgggctgacgctcgccgcattgacgatgcgcgagaacttgcaggcgacgaagggcaacgtgcccgacgcactgcgcatgtacaacgctgggcctgaccgctcgcgttggaacaatgcagagacacgagcgtacgctgccaaggtgctgggcaccgacgcagatacggcaacgtccacgagcgagtacgacattcgtccgtctagcttcgagcgccccgatgcgcaggaagcgtggacgacgagtgcgtacgacatcatgggcatggcgaacaaagacgcgagtggttccgcctcgaaggaatacttgtccgacgtggagaagggagtcatcgcgcaggctggtgtggagtcggctactgccgctgccatcactggtcaagaccctgcacaggctgcactggccggtcggcagaacgtccgcagtgacgtgactgctgttactggtcaggtcatcgacaagctcggtgaagctccggttggtactggtggagacagtggcggctgggaagcgatcctcgatcaagcagtgaccgaggagcagcggcagaaagagatcgacgccattacctttggcgacaagttcggtgcagcgtttgacaacaacacgttaaccgcaggtatcctgcacttcatagaacgacagaacggcccggtgtctcgtcccgatccgaactggaattacatggatcacattgacgaggtggagaaagatcgtagtgcagatgagattgacgagttgcgtgaagcacgcagccaaggggaagtgggtctcatcaaatctcgacaggataaggagcgcgagaacaaccgcatcatcgctgctggtagctctgacggagccatcatcggatacaacctcgctgctggtgttgcagacccagtgggctggttggctggctttggtgtgggtaaggcgtttcagattgtgggcgttggctcgcgcgctgcatttgctgctggcaacacggggcgtggcttcctgttggctggtgcagaaggtgcggcgggtaacttgctgaccacctccgcgctcgacgcgatgggtgagcatcagtccacgagtgactacgcgatgagcgccggcttcggtatgctgatcggcagtggcttcggtgcgttggcatggcgcggccaagctcgcgtccgagcgcagcaggagttcaccgacatggccgaacgattccagcagagcgcggcagagcagaatgccaagctgtatcagcaggctgttgctgaggcaggcccggatgcaacgtccgagcagatcgctgctgctgcaacgcgcatcaacgcgcagcaagagagccgcatcctcgacaccgtgttcggtgacatccccgacaacatgcggctgttcccacgccctgacgtggatggccctgtgttcgccacgccggaggctccggctggtgttgtggtgcccgagcgcgttgcaagcacggagcggttgcctgttgagttcacacaggaagtgggtggtgacggtacgacctacacgttcacgttcggtggcaaggaagtaggttcgattgaagtcaacgaagcaggcggcgtgatgtcgtccaaggttgacgaagctgtgcgtggacagggcattggtaagtcgatgtacatggagttggctgatcgccagctgcggcttggccgtccgttcacgagcgatggttcggtgacggaggatgcagcgcgcgtgtgggaatcgcttgggcgtgactacacggtgacgaagaatccgactgcggtgttcgagtcgggtgcgtggctcacggaagatggtggcccggtgttctcgctgactgcgaaggaagctgcacctccggctgctgcgcccacgcgcaacgattcgctgcccggtgctatcctgaacactcgtcgcaagcgccaagctgcctacaagcggtacggactggatgtgagtatcgccgatgatgcggagcgcaagatggttgcggaagtgttcgcacgcgctgaacgtgtcctcggtgagaacccggtcgatgtagagcggctgcgccccatcctgtcaaagatcggttgggaagcaacctcgacgcgcatgctactgtcggacaacccggtgatgcgtgcgttcgctgtcgtggcgttggagaacccggaaggtgcagctggccgcaaggtcacggctgcaatgaccaagagcatgcgtgagcgcgtgtatctcggcaacactttgcgtgactacgagaacgcctacgctgtgtggcgcaaccgcaatggtggttccgcactccgagacttctacgatgacacgctgcgtcgccgcttcgacaaggaagtgtacgcagagcgtgaccgccgttggaacggtaaggaaggccagcccatcgaccgcgaggttggtgcggcgagcgatgcactcgacctcggctatcagcgcatgggtcgggatcaggcatacgttggcaccatcggtgcagcgcgactcgactacgagaagcgcggttaccagccgcgtcgcatggctcccggtatggtggcacagctgaacgacgcgcaacgtcgcgcgttcactgaggcgctgtcgtccgagttccagatcagtgcaggcttcgacaaggagttcgctgaccgcttcgccatcaagtacattgagcgtgcgcagacccgtgcgaagggtgcatacgatgtgcctgcgaacctgcacagcgatgacgctgcggacatcatccgcgactcgctacgcgcaatgtccatgaacgaggagcagatcgctcaggtcatgggccggttctctcgtggtggcgcatcgcacacgaaggcgcgtatcgacgctgacctgacgacgatgtacgacgacggtgctggtggcaacgtgcagctgatggacttgatgaacaccaacaacctcgacctgttccgccagtacgctcgccgcgtgagtggcgaagtgtcccttgccaagtacggcatcatgggcgagcagggcatgaaggaactgcgcatggcaatgacggtcggtgctgacggcatgcgtgcgactgcaaaggagttggaagcgttcgatcaggttgcggctgagttccttggccgtccgttcggttcacagctgggcaagtgggcagacaatgcccgctcgttcaccagtgcactgcgactcggtggcatggggttcaaccagttcaacgagtacgcgaacggtgtggcaagcatcggtgtgttgcgtagcttcaaggcaatgactgcgctgccgcgactgatgggcgaagtgcgtgagttgaagtcgggacgaccggccaagaactcgctgctcggctcgatggagttgtacggtggtgagttcggcatggatgactaccgcatgcagggcatgtacgatgtgaacgaaggcttcgaggtgtacggcactgaggcgctaggtgtgttcgacaaggctatccgcgctggcgcacacgccaaccgggtgttgtcgggtcaccgcgcaatcaccgctgtgcagattcgtggcatggctgaacagatcgtgcagaaatctctgcgctatatccgtgagggtgtagaagatgcggcgctcgatgacatgggcatcaacgcagcagtgcgggatgctatgcgtgctgacttgaacaaggtcgctacgttcggtgccgatggtgaagtgcgttcattcgacatcaccaagatgcaggacaacgctgcggctcacgcctacatggtggccgtgcatcgcggcgcgaatcagatcatccaagcgacctacatcggcgagaccggcaagtgggcgcacgatgggtggctcaagctgctgacgcagttccgcacctacggcatcaccgcgacgcagaagcaatggcgtcggcaggcgttcacgcacggcacagcccgcgcgctgggcttcctgctgggcgcgatgagcgtggcgctgccgatccacttggcacgtgtccagctacgcgctgcgggccgcaatgaccgcgaggagttcttggacagggaactgtcgcccgtggcgctgggacgcgctacgatgaactacgtgtcgtctgtgggcctgttgcctgacgtgctggacatcggttccagcgtggtcggtgcagacatcacgggcggtcgcgcaggcaatacctcgcccttcgtgggcggacagatcgttccagcagcgggcgtagtgaatgacgtgtggcgcgcggctcaaaccaaagacccgcaccgcatggtgaagctgctccccggctctaacctgccgtacctgcaaggggcgatcaaccagctagacgaatgaccgaccgggccacaaggacgtggccctatttcggcaccctacatacacagattcaaggagaccgccaatggcgatcaacgatccgaactaccgctatgccactcagacgtgggaagcggacggcgtgcgtacccagtacgacatcgccttcgatggcggctacattcggcaatcggatgtcgttgccttctccgtgctggttgacgaggacactggccttacgaccgaccggcagattcatcctgtggttttcctcagtgaatccgttgacccggagactgaatggaaaactgcacaagtccagatcacaccagccgtcccggctgggcgtcgggtggttatctttcggagtaccgagaaaagtgctgcgcttgttaactatacgaacggctcgatcttgactgagaagaacctcgaccttgccaatgaccaaagcgtgttcggtatcgctgagatcatggatggcttgaacgctgcgcgtatcgacatcaactcgcaggtgcaagaagtcatcgacatgaaccagctgattcaagaactctatgagcagatcatagagttgcttgccgctggtggtatcgtctccgtcgcacctcgcgtgtggtttgggacgggcaatggcgaggacacagatttcccgttggtgggagcggacgtggacggctccgggttctacgatacctacattggtggtgtgggtatggagccggacacggactacgctatcatcatgggcgagaccatcgcagacacgctgatccgtttcacggttccacctgctgatggtgttcgctggttcactgtgctgcgcggctacgccaagccctacaccgggccgcagcctgtcgtgtctctgtcgatgccagtcatcgacgtacccgacccgcaatacttcatcggcaaggagagcgagtacgcattgctgcgcgcgctcaacgacaccgaggcaaccttcttcgtcaaggagattccgatctctggcgatccggccaacaagctgggcgatggcagctacgtctccatcacgcagcgtggcgctgctcaagtcgtactcgaacccgacactgccgaagtgcagctgatcgtgcctgcgggctacttgcccgcaacgcgcgcgctgaactcggtgatctcgatcacgtgtgagtatggtgacggcaacgcatggatcgtcagcggtgatctcgccaaggagtaaaccatgacctcagtatttcagttgtacgggcgaccgctagcagagaatgagccgctaccgccgctgaggatcactggcgagttggagggctacacctccggcgaagcctatgaaggccgcttgcagatcatcgacagtatcggcaagtgtgtagtggagattgtggaaagcagtctccctcccggctcgtacgccttcgttgacaacttcaccaaggagatcgtgctacgctggcctgcctacgcaccgcctgatgcaatggcatcgggtgtgccgaacggagacttcgagcaaggcaacgacggctcgtggcgcttcggtgctggctggtctatcgaagctggtggtgccgagacaggcacctactctgcggtgtatcagaatcaacgcggcattcagtccatcgaatccaaccgtgtgccttacactcccggccaatccatcactgctgcatgtcgcttccagcaaggcgcgtcgtcctcgggtaatctcgtagggcgcatcctcctgatttggtgtgacgcgaacggtaatatggttccgggtggtgaaggtatctcgtggacaggtggcacgctcattcgctctggctccaacggagaatggcgcacgtcggacgtgactggcgcaagcagtcatcctaatgtagcgaccgtcgcagtgggattcagtgcaaatcgcaagaaacaaaacaagctctgtcgcgttgacaacttcacgtggaatcacgagtacaccactgggacaaacagtgatctcgactttactgttacttttaaggtaacggattctgcaaaccgcattgcttactggactggtactgttggtaaatactcgctgttctttacaagccagccgtatcctcatttcgtatttgagtccgttacagcacagatgcctgacgttgctaacgcacggttggatattccaccaaacctgtttgactccgctacggcagaaatggctcctctatctggcgatctgcgtagcatccaagggtcttacgatcaccctgctgaggacttcaccacaggtgaaatgagtccgttgtctggcgcgatccgtgacatcatgcgggcatacgacattggtgtggagtctgttgactgtaccatgtctccaacttcgggaacactcctagcgatcctaatcactcagagcaacatggaagcggtgactggcaccatgtctccaacttcgggaacactcctatgaacaacattcacatcggcgtagccggttacttcaagatcgaggccatcaaagtcgatggcgaaggtaacgagatcagccgccgcgtggctgctgactggtttccgaacttgatcctcaatcaaggtctcgaccgcatggcggataacaatgacttcatgtcgtccgttcaggttggttcaggatcgactgcacctgctgacacagacacgcagttgcaatcccacattgcaggagttggaagtataacttccaacacttatggtgcacagtcgtctgcaccgtactacggttggcgtcgtaacacttggcgcttcactgccggtactgcaactggcaacctgtcggagatcggcgtgggttggtctgctactggcgcaactctgttctctcgttctctcatcaaggatgaagaaggcaatcccaccaccatcactgtgctggctgacgagattcttgatgtcacttatgaactccgcaattatccgttcttgaccgatcttccggggtcgttcgacatcggagccacgacgtacacaacgtcgatgcgggcggcgaacgtgaccagtgagtacggaatcttcacaggtgggtggggtgttaacaccagaggcccaatgtcccaaaatccagcctatctaccttgcgtgctgtatgcaggcgctacgatgggtgcgatcactgatatgcctacgggagcaacctcaaccctgtcgggtctttgggattcgcagtccacctatgttccgggaacctacactcgcactgctacttgcaagtggccggtgtcatctgcaatcaccaatgttagtcacatcagcttcgcactgggtggctgcactacgcagatgagcttgtctcctgcgacgctgagtaagacgactgcacaggaactcaagatcactgtgactctgacgtgggggaggtacacaccctaatgctgcccaataacacgctgtcctctgaaccgatccgtagtagttttacggagcaacagaaccggcgtacgcttccgctcatcgactacgaaatgggcggcgtggcggtcaacgatgcctcgggtggtttgctatatcgcctttggcaagctgaacttgtaggcgacaccgtgatgctttcctcggaaggcattgcggcagtccccttgttcactcgatcaggtatcacacagatcgggcttgccttcgatcagaacatgcgaccctttgtgtgcttcgtgcaaaacggacaagcacgctactggtggttcgacaccgaagctggtgcaccagtattcacagacttgcctgttgacgctgttacgccgcgcgctgcaatagatgaaaagcgggcagtgtacatcaacaactctgacatcatcctagcgtatatgcgcgggacgaatctctgctacaggcagcagcgcgaccgcttcctaaccgaaagaatcctagcctcagacgtacatggtacgctgacagctatcgggatgaacaaggtgggtcggtttcaattccggctgttgcctacgccataacaggagacaccatgaacgacgcgccttcggcagcgacggagtttgcacgtaacgtgccgctgactggcggcgcgttgtacctcagcttcatcagtcagtatggcgcagccatcgtcaccacgcttgccatcgtgtacggcgtgatgcaggtaacgctgcgcatactggaacatcgcgcaatcatgcgcaagaacaagatcgacaaggagcagcctgaatgagcagggctagtgagggtgagcttggtggcctgcacggcatcgttgcgcgatacctcgctgagaagattgcttccggcaaggcaaccgcatcggatgtctccaacgccatcaagctcctgaaagacaacaacattacctgcgacgtgaatgaggacaacgacctcgggaagttgcagcgcgcgttggacgagaagtccgcaggcaagccggtggacgacaccgaccttgcagctgctcttgagcagatcgacttctcccaaggcacgagtgtgaacta

SEQ ID NO: 16 - DNA, 44415 bp, unidentified
  source 1..44415: mol_type = genomic DNA
cgtccggtcccaccagcgtgagcatgcccttctgctctccggtcttctcgtccgtcgtgatgtagtacgtggacaagtccttgtggatgtcgtcgcgtctggcaagcgccttggtgaacggcaggttgcggtagcccagcgcctcgatcacgtcggcagcggtggagtacacgccgggatcgctcttgctttcccatgcagcatcaggctcggtgtagccagggaactcgaacagcatgtcctcgttgcggaacttctgcttggtcaagtcatcgaccttcaccttcttggtcttgtactctcccttgttcttgccgctgccgtacgtggtgtagcgccagaggttgtcgaagtcctcggccggtggcgtcgccgtcgtggtaccatcgaccagcacgtagtgcacctcgtccttctgcacgtaagtcggcccaccctcggtggacatgatcggaaccttggccgtgtacttcaccttgccgccgaagatcagcgcgctcttgtggaagcggctgttccagttgaaggtcaggccctcgggcagctcggggatgaagccgttgagttcggcggtcgccgttgcaagctcgacctccaactccttcgccttcgtaagcgcccagtccttgtccacgtacatgccgttgtactcggcttcgatggtgaagcacagcgcacccatgttgaggagcgccgagcgcagaccaccacgtgcacggaaggcggcgagctgtccgaggaacatcttctcggtgttaccgatgtcgcccacgtcgtcggtgtcgttggtgccgaggaggtaatccatcagcagcgtcttgtcgatgtcgcaggtgtccacgcccgcagcccacagggacttgactgcatcgtccttcaagttgccgccgtagcgtggagccgtctcgtccatgctcgccatgtggaactcttgcgtcatgccgtgcagcaggtactccgcaagctggcagtcccacaccatgccgccgccgtcgatgaactcgatccatgcctgccggttgagtgggccttggcagatggcgtgcaggatgtcgaacttgatgttgaacccgacgaggaactgctgcccgtaacacagctcacgcagccacccatcgggtgcgccgcccatgtactggttgtctatcccgactcgggtgtcgtagtacaggccggtgttccgtgcgtcacccttccgcttgtagccaatcgccacgatcttgttcatgtcgtagaacggattggccttgcgcttcaggatggaacggatcgtggtttcgaggtcgaaggaagtgaagctcacagcggccaccgttgcagggccagctggtacatttcatccgacgcatcgccatccaagtccagcccgtcgcgcacccaacgtaacacgatgatgcggtcctgcttgtccttgatgttgcggcgcttgcagatggtggtggcctcgaccgcgcgctgataccagccggagtcggcggtcaccatgacgttgaacacgccgttgcgcagcgcataccacgtggtgctgtagtcctcgtcctcctcgtagtgtccatcggcaccggagcacagggtccatccctgatcgaccagcttttcgatggcctcgtggaagtcctgcaccagcacgaggaagtcgatgtccgtgtcggtcacgggcggctcgactgtgtagctgctgccggtgcggctggacgtgatgacgcccacgttgcgcggcaggtagatgttcggttcggtactcacggtgtgttacctccgggcttggtgatccagaacgtgaagcacgggatcagattgatgcaccagcgcttgttgtgcggcgagtagtgcacgccgatccaagtgctgtgtttgttccgcagccatccccacttccactgcggcgcgtcgttgcggccttcgatgtagcctgcgtcgtgcaccttgcgcagcagcttggcaaggtggattgcttgcgcgttgctcacgcagttgaaggtcttcgcctcggtggattcaccggggaagctgaccgacaccgtgaacccggtggctacgatgtgaattggcttgctcatgctgcctcctgatagaagcgggcacgctctgcatccatcatcacttcttcccgaacgtcacgcttgccgcctgcgcggtgcagcttgttcttcggggtgccgatgtagcggaagcgttccatcgctgggtcattgagcttgccgcccatgatgatgaagtcgcacgcaccctgcttgccggtcttgctgtccttcagtgcggactgcggcgggtactggattccctcaccctcggcgctgatctgcgaagtcgccacgcccacggcgtcgtacttcacacaccagttgcgagcggcctgatacatcgcctccaacatctgatcggtacgctgcccgccgttggtcatgccaccggtgaacgtgatgttgtcgatcatgtcgaagatgatgaagccggggttggtctgcttgatgatggcctcgacttcaccggagttgaacccgtggatgtcgtagaactgcatgcggtggatgtccccgcccatcgcatcttcgatgcgcttgcggatgctaccatccttcgcccactccaccatctcagggatggtagcgccgagcagcgactgataccaccgctgcttgatgcgcttgcccggcccctcgttgttgagccagatgccggtgcgcttctggtccggccaaacgttgtcgagctgcgtgatccagtggctggactcgctggtcaggaacgtggtcttgcctgcgtcgggacgcatggcgtagatgccgaagtcaccaccacgcagagcgcgcaggttcttcgccaacgtgggcagtcggaagtggatgccgatgtcgtgctcgtccatctgcatcagttcctcgggcgtctcctgcaccagcgggagccgcgccttgcgatccattcggtcggtgatcgtctcggccaagccgtacagctcgtcgcgcaggctgaactcagcgccgccattccactgcacgatcttgctgaccgcagtggtggcaagctccaactccaacagcttctcgatcatgccctgctctgcctcgggcgggaccggctcgcgcatctgcttcagcagaactttgagcagggacttcttgtcgtcgggctgcgtcttccacttgaactccatggcccagccatcgaacacatcgaacggcaagtccttcgtgtccgggaactccttgtagtacgcacgcaacgcatcgagcatcagcacggtcagctcgtccagcccatcacgtggtgcgctgggtaccagccggtcgaacttgccacggttggtgcacaaccgcagcagcgtggtgtcaagactcatcaggttctccttcgggttcgtacttggaatcgagctggtgataccgggtgttgcgcgtctcgaacttgcgcccgccgtccgccacatacagcaccgtcgaggtgtgcacgatgtcgcagtcgccgaggttcggatgcgcaagcacgccgccgagcgtggcacggaagccaacgacgggcgggatgatagcgcgccggtagcgcacgatgggtttgctcattgcagcttctccttgatgtagtcggtcgtgtaatacttcgggtcacgtggtgacgtgatgttcctgtagtccagaccaaacgcacgtagacgcgcagcgattactcgcgcactgtcttggccgggattgctaccgttgcttctacctctgtcgtcatcgagccacgtcgctacacgttggcctcgatcagtcagctgcttcaacactttgttgtgcagcttggtgccgagcaacgaccacgcttcggttaccagtcccaccttgtatgcactgagcgggtcttcgcacagtacgatggtgtcacctgtgcccacgccgtagcgtgcgacaagtccgtctttcggaacgtcaggtgttagccacttcggctgtctcgttgccgaccgggctgtccagtataccacgttgtcgccttcagtgatcggtagtaccacccgcccgatgcttgggcaccagtacagccgcagcttctcgatcatctgaagcgagagtcccatcttgaagaaccacaccttagcgtcgagcggccactcgcgggtgtcgtatacccgtggctctggcaactcaacagtcgcacgcactctgcgttcgctcgtctgctcggcgtggattcgtgcaagcttggcctcgatactctcgtgctcacgcttgaatcctgtgccaccgcacctgaaacagaatgcggtggacttgtcgtgctctcgtgagataagcaagggcgtaccctccccgcactcatgggccacacgtgtgcggccaccaacaggcaggcgctcggcatgtggtagccagtcgttgtcgggaagggtatcgctcatgctatcctcgcttggttattcccagacctcgaagatgtcgtggctggtggcgtacaggacggagccgttgccgtccgtgctgacgatcagacgggagccgtcttcactggtcagcttggacacgacgaacccggtgcccttcggcagcttgttggtctgccgcgtgtcgatcaggtacgcattctggccgggcttcagctcgtcgccacgcttgacgacggccacgctgggtgacggcggggcgaggctcacgactgcccgccttcgccacccgcagccttggcggcagcggcttcggcggcgaggcgctgggcctcggcaacggcggcgtcgatttcttcctgcgccttcagcacttcctcggccgacatcagcagggcgctgctgtcgatcaggttcagctcggcatccagaccttcgccggtctgcaccttcagttgcagcacgcccttgtcgttcttgccggtggcgacgatcacgccggacaggacgcgcttgttcagggcacgaccgaacaggtaggacacggcgtcgcccgccttcagcgcttcgatggcggcgctgttggcctcgacggcatccagcttggcgagcttctcgttcaggccatcgaccttggcctgcgccttggcgatgtcttccagcagctcggcgcgcttggcttcgtagtggctgacggtggtctgctcggtggtgttttcgttcgacatgtagatggttcctcttgacggttgataggatggcccgtacgtgggccagtcgtagcctacccggctcgggttactgaaagatcagctcgctgttgtacccaccgccgccattgtagaagcggcgacgcagcacgctctcctcacccagcaccagcagacggtccacgatggcgcggatggcgctcatgtactggtccaccagctcgctgtgcaagttcaggtcgaagcggatcacggtcaccgcctcgtcgtccagtgcgccggtgtccttgcggacgtacaggccacggccattggtcatggtcgcaccgccgatcagcttcacggcggcggcaatctccggctgcacgttgagcagtcggctgtcgggcacagtcacctcgacccagcttcccatgcgcaggctcatgctgcacctgccagtgcggactgcacgttgggctgcaacgatgcaccggaacgcagctcggcagcacgacgcttcatgcgggagcgcagcttgcgacgctgcttgttgttcccgccgaggctatcggccacgcgcttcagctggttgttgccgacgatgcgggtctgaccctgccccttctgcacggggaagtagtcctgccccagcatcttgcgcaggatcgggttgtcgatgggaatcagcggcacgctgacgtgcaggtgccggctggtgtccggcgcaggcggcggcgtgtcgtcgtcatcgtggcgcggcttcaccgctgcgaccaccttgtccttgacgtacttggccgcagccttgatcttgtccatgaaacccatggttacttcctcctcgttccgaagtgattgaactccaactcatgccacacgtagtacgtggtgccgagcgggtcagtgtctgccttccagttgcgctggtcgcagtagtcgttggctgcgccgaggtcatcgaacgtcagcgagaacccagtggaagccgggccggtgcggaaccggcacagcttgccgtcgtcgtcatggtactggccgacgacaacccacgggccacgacccacgatccagtacagcaggatcaggatgcgcagccagagcttacgcatagtacggctcgacacggtagcccatgttctcgccgcccagcgactcggcattgaacacggcgcgcgctgcatcgcgggtcgggaacagcacgttgtactcgctcttgttgtactcgttgccgtcgatgcgcacggtggcgctcgggtgctggttgtagcagctgacatcggagtcgctgcggtcttcggcgaaggcgtaggtgatacgccaacccagcggcttgcgcaccggcttgcggatgctctcgcccacttcgaggatgtgccagttgaagaacgacccgccgtagctgttgagcacatccgcctcggcacgcacggcggcgcggcggtcgaagatggcgagctggttcgggtacgtgccgtcacgcagcgagtccagcaggctggtggtggcacccttggtgcgcagctcggcgatcaccgcatccagttcctcttgggtcggggtgcggccggtgccattggcgacgacgccagtgatgacgccatcgttgctgttcttggggatcgagacgatgaagtataccttacgcatggtggttctcctgattgacgggtgggatttcgatttcctctatcgagtagagggtgggcaccttctcgtggtgcttgcggtggtgttcgatggcttgctcgcacgcctcgtggctggtgtgatgtccgccgaggatgtaatccccgacagccacacccttcacggtaacgagcggcagcgccttcaccacaaggcgcaggctgacctcacgcataccagcgctccacgctgtgctcatgggtcacgaactctttccactggcgcggctgctcgcacagctggatcggcttgcgctccccactacggatgcgcttgtaagttacggggatcatgcaatgtgccctcctgttgggcgtggttccaaagctacgccctcgttagaaggcgcagcggtagatcacgcgcggctcgggtgccacttcacgcggtagcggcggagacggttcggatcgttgccgacgtgcgaggcgatggcgttgcgtgcagcctgcgcagtggtgaacgtgccgctgagtccgatcacagtggacgtattccaacccagctggtgagggcgccgcgcatgcttggtgaagaactcggcggtgtagaagccgcgatccttctccgggccatcgggagtgccttcgggcaccacacggtacgcatcctcgctgatgccctgcaccttggcccgcgccttcagcatgcggtacgcagcattgcggctgcgctgcggcaggcccagctcacgcacctgcgcccagttggcgagggcgatgctgccgtggcgcagattgaactgcacgatccagcccttggtcttcgtcttgttgaccagcccggtctgcgatgcagtcagggcgacgtggcgtgcgctctggtcgtccatcaggacatccggcagcttacgcggcaggttgtcgggcattgccaggccgggcaacaccatgcggccggtcacgctgccgaggaagtccagctgcgaggcatccaacaccaccggaggcaacggagacagcaggcacgccatcacccgcgcctcgatagcagcgaagtcaagttcacgcatgccgtagcccacggtgaacgtcggcggtgcgatcaggtcgcgcagcagctgtgcctcgacatcgctgtcacggcaggccgcaatcacgtcgtcctcgaattgcaggatggcgtcacgctcgaagctctcgacaccgaagtcgcgcagctcaccgtgcagcacggcgaactcattggacagcttgcggttggagtacgggtctgcctttgcggtcagtgcacaggcgatgtgaagggccgagcgcagcagggatgcttcgcgctgggtcactcgaaggttgatcttgggttccatgttacacgttctccttcttcttggtgggcttcggcacagcgcgggcagcgttgatgacggcctgttcctcctcggtcggcacgtagccttcctcggtcgccttttccagacggcccagcagcttgtgcaggtcggcggcgaacgagaacgcctctgcgggcttctcggtcttgaagtcgtaccacgccttcgcggcggcacgttccagcacgtcggccagagcttcgccctcgactcgcttgctcttggcaaacttcatgggcgcgctcgccttggtttccttgtcgtcgttcggagccatcgggccgaactcggacaggtacaggcgcagggcttcatgcttcatgccgttgcccacggcgagacacagatcggaagcgagcgtaacgtcgccgtggatgtgtgcgtggttgatgaccgcaatcgcggcctgctgaatctggtccaccagcttggtgcgggcggtgttgatcgacttgatggcgcgcttgatgtcagcgcttccggtgatgatgtccatggtggttcccttcaggttgggtccgtgccgattgcacgacactaggccctcttgcgaaggcccagtagcttgcatttaagcgagtcggatgtcgaatgaacgcccaccgcacggcaggacgtagagcgccgacacagagccggccggatgcttcatgatggcccgattgtaggaatcgcgggcagcttccacgtagtggcgagagaacttgaaccggatcacaggtaagccctcctgtcagcggcgtggttcgcccggttcgtcccgctgttaccctcgacaacaaacacagatcgctttccggcggttccgtggcgggcttcgtagcgctcggcttggcgcttgcgctcggcaagcttgcggtcatgctccgtggtgcgcaggtccatcacgcttgccgtccgggtgaactggcagaagcggcgcttacgctgggtgcggtcgagattggcattgatcgagccttgcatgttgtgcctccattggcactggtgggaaaactaacagattgatgcgccctcagaaagccgtcgagtcggtcaatccctcattctcgattagagccgttgcatcgcctatcgtgggcgcacactgaccaccggatttgcctgcatggtcatcgcaaagggagggcgcatcaatctgctagcccttcgggctgtcaaccctactccggctagcagtgccattgtcaccgtgtggcccgtagagccttttcacgaaacgcacagtattccatgcgataggaggctcaccacctccttatgaccggcttcccaccttggcagtgggttacttcccgtggccgactctcacggcagatgggaagccctaagcgttaggcttaggtaaagcggcaccagtgttgcaagtctggtggattctatgggcctttgaaatcccagttcatccggttatccgctagtgctacgttgcagcttggcggtccacgtcaactctcggccactattggctgtggttggcacgcttcccgttacaccctacccgttagcggtagtcctacgccatccaatgtggctgctcctcagagcgtggtgccatactagcacccttgttgcatcctgtcaagcccttggctcgctcgggtctctaacccgttgggcgtcctgtcgccaccatcccaccatgtacgtcggtggtccacgtgttgcaaggcctcaaagggctatctgtgccgccttgtcaagctatccgttagaggaccatgtgcgctcctgttagtgtcttgaccggtgtcccggtctcacctcagcctcaacacccgtaatctctcacgtctagccttaccgctaggtcgctccgctgttccggtggctaccacttgccgcctatcatagctaactgctagcttagtgtcaagcgtggttcggtagctcctcgcatcccttaccagtgactcccgtgtacccttagcccacttgttggcggcgccactacggatcacgtcactcgacttgcgttgcagcttactaccattgcggccgtgtgtctactactgcttgcatcgcaagcgtcaaccgttggcctagcgggtagctaactaatcagctcgacagagtaccgatagacggtgattcaggttgagccgactgtgtgctataggtgtaccaaaaggccgaaacgatacagatggccctcgcacgcctacagctgcggttcgcatggtagcaggtagggtagcccctgtcaagccccttgcggccctcctgaagccctgtcgctgccccagtgacgccattgaaccacaccgcaccggccacgtcaacacctttcgccaagagatttattaacgattcagccaaggcagcgcggtccagccatacaggcagcaggcgcacgcccacccgcacgcccacccgcaggcacccacgcacggccacgcacacgcacgctcaggcccacgcaggcaggcacacgggtacacccacgcggaaccttgacgcgggcgcacagacgcgcacacaggcgcacacgcgggcacgcacccacgcacacccgcaggcgcgtaacgcgagggcgtacgggggcacgcgcgggagcttctattggagtgacccccgcgcatttccgaagcaaattttggtccggctacccacgtggccttactcctaagcctcgcgaactggtgcctttagcttgacgataggcccggagctgtagacatcgtgagctatcgcagcagccatggccttagccacagacttgctcgcatgataggcccctagagctagcgccttgccactgccatcgaagtacggagcctcctcgacccactgctgcttaccagtagtgaccgtgagtacgccgtccttaaccacaagcaccgtcgcggacttgccaacgtgctcctcgtagccttcgcccgctttaagcgcagcgagaaccgggcgaagcactgtgaaatccccggtgacacccagcagcacagggccggtgggtgtcgatacgggcatgatcttacgcacggtgtgcttgtggtcgccctgcgtggcctgactatcggcccacaggtgcttgccgtcccatgcgatggtggtcatttgtcacccgtacaccggcgcttaccggtaccgcacacctcggccttccacgcacgcagcgcagccttgtccttgttgcacagaacggtgtccatgcggcggtcctgcgcgagcttgaccaccttgtcctgcgaggaggtggtgcccttctccccaccgaggtaggtgatgtggcagtctgcaagcagggagtcgtcagggaccggcaggttcgcgcaggaggtcagcgacatcagcaggaacagtgccatcccggtactccggggcagcgtcaagaacttcttcagtgcgaacacgcacgtcctccttctctttgatgtaggtcgcgtacccggtagcctgcgtctgcgccgccttggcggtagcggtcgtgccgacttgggcagtttccagcttctccaccttgcgttgcaggccgtagacgtacagaccgaagcacacgaacatggtcacgaccagcagcaagccaaccagcttgccgccgagccgcgcgatcacttcacttggggtttccacggttggatcacctcgttgttggggcgcaagcacagagcaaactctgcgtcgcggcgcttggggatgccggagcaacggctgctggacagtcggcagtcgagcttaccgacgtagacccagcgcaggaactccttgcagctaccttcacgatcccctgcgttcgctttgcgcagcatggtgctgtcggcgaacgccttctcacctacgttgaacacgaagtctgtgtaggcgtcgatctggttgcggttaacgggggccttcaggtgcttgcgcacgccctgctgggcgatctgtaggtcttcgatcagccacttgtcgcactgtgccttcgttgccgtcatgcccatcgctacgcccttggtgtggccgtagcagatggtcggcacccggccggtgtcgaggtacgcagcgtagcgtaccccttcgtggccttgggtgaatgacagcagcgttgccgaaatgccgatgaagatgccgccgatcaggccgaacagccccttgttgctggtatcttggttctgctgctggttcatggttgctccttacggggtcagtgggtcgtcatccgggtccagatcgaccggagtgtgcgggccggagttcggacccgaggacgcggtgcgtgcgcccgcagcgatcagggcgtccagcacgagggtggcgtccttctggaactgcgcgagcagctgcgctgcggttgcgggatgctgctctgcgtgctccatgagggcgagcagttcgcggtgcaggtagttgccacggccgaacagacccgtgtagttgctggtgaagtcggacttctgcattggttacctccggtaacggtcgagtagggatggacggccacgttgcagcggactcttgcgggtcgctgccttcatgccggtcggatcgttgatccagtcttggaactctcgctgctgctgcttggcgatggccttgttctggtccagtgcaagctgcgcaacccagtgacgcacgctaccttccagtgcatcgagccggtcatcgtgtgcgatgctgcccttctgctgcgtgatcttcgccatctggtggaacaggctgtagacctgacgcttgccgctggtggcgtagcgctgggtgtactcgtgatccatttcaaccacggattccagcatgaccagcgagccgcgagccatgacaggttcgagagtgccgatgatacgggcttccttgttgccggtcacgaactcctcgcggatgtcgcccttgtatcccttctccgtgccgcgatcttctcgcaggacaggcaggaacaccttggcgaacgcgccgtagcccatgttcttttcgatgctgatgacgttcggcttgtacttcaccgcaatgcggcgcagttctagcaagccatcaccgtcgtagccaccgggcacagctcccacggccaacacgtacacggtggagttgaggaaggcggtcacggcgaaggccgtctcgtctccgttggcaccaccaccggccgggtcgatctgcatgtgcacgccctgcacgggggcagtctcggtgctcatgtcgtgcggcatcatcatcacgaagccgtacccactggactggaagctgcgctggtgagcgttgctcaggccacgggtgatcgtcagcgggaagcggtcgccaccaccggggatcacgatcaggttatcggtcttcagcgggaagcgcagcgcatccatcagccgcgtgttgagcatgtagttcagctgatagctggacggtccacgctgacgcagctcggactggtgcttctgctcaccggccaacagctcgtcggtgcactggccctcgtcgcccatcgggccaccaccgaacgccaacatcgggtcggcttctaggcgctgcacgatagacggtgccagatgcgggccgtagtgctcgcgctgtgccggggtcgggtagcgaccgggccagatgcgaacgtcgtagccacgtccgggcagggtgttgtagatggagtcgccggtctgcggcgtgccgaggtacaggatgcgacccggagtaccgggcttgccggtgcagatggccgagaactccaacgtgatggtcagcagcagctcacggttcgcggcagtgcggctgttcttgttggactccacgtcgtcggcgatcagcaggtccgcacgcttacccggcaggttgccggtgacgccgatgcacgccacgctcggggacttgtcgattcccttcagcgagtggtgcacgtcgaacgcatccacggaggtacggtcgcccgcgttcttgtccgggcggatgcactccaacgtcggcaccgtgaggatgatgcgctgaatcagcgtagcaatctcggatgcctgcgtgccgcctgccgatacgatcagcacacggtgagtgggatcgtggatcaggcagaagacggcgtagatggcagcgatggtggacttcgcctcgcctcgctgcgcctgcaccattgcgaggtgcgggccatactgcatgtagttggcgatgtcgtactgcatccacgtcggctcgaaccccagcaccttcataatgtcgcgcatgaaggtggcgaagtgccggtagtggttctgcaacagctccaacttcttgcggcgcacgtcggccgcttcagctgattcacgcattgttggctacgctccccggaaagtgaacgatgttgtcgagtgcacgctgcaactcgtcgtcgtcagccggaggcagcgagtgcttgcccagctcgtcttccagctcgccgagtgccttgttggcctcgcgcgtcgccgtgatgttgttgtccttcaggaacttgatcgccgcattgatgtcggctgcggtgcacagctcgccatcttggatgcgctgcatcagcgcacgcgcgaccagttcgtgcagcgcaccgagtgcgccctcacttgccggattcgacatccttgcctcccatgatctttcggtgctcgcgtgcccgccagtagaactgagcgacggcgtacagaatggcgagcgtagttacgatggcagcaccgtacgtgctgatgaagttgaggtagaccgcgccgagcgtaagcggcgaggttcggacgacctcattgaccacactcggcggggtcatgctgttctcctgtaggttagggccagtcgtcgggattgccgacgagcttccattgcaggcggttgacgttgttcatgcccaccgcaatcaggtcgccggggattcccgaggcgatcacatgttcggttgcgaagcgctcacgctgcgcgcgtacgcacaggttgctgccgttcttgtacgacaggagcacgtcgctctgcgtggcgaagacagcccgcttctcgtccatgcacaggcgcggagtggtagcaccggggatcaccatggtctgcatcgaagcagccaccgtgtcgtaccagtagaacttgcacacaccgcccgccatgtacgccacgtgcgggcgcatggtctggtcgaaggccagtgcgatctgcgtgatcccggagtcggtcagcacggtgaccggggcaacgccgtcgcggtaaacgacgacgctgctgccgtcactctcggcagtccacagcgcagcttggaggtcgtccactgctgcgttgagagtcagcccgccctgctcgaagtcaatgagcgggcgggtgcgccgattctgctgctccacccagtcaccgcgttggatgctttgggagacagtggggatcatggcgtgtaccggctccaagaaacccgcatgcgcaagttcgccgtctccgatccggtcttggtgatacccggattgaagccgacttggaaggtcacgcacgcggagagtcccattgcagccgtgatcggaccaccgggcacgttgttgatcgacatccggcaaacgcagtcacggtagtaagtacccggaacataggctacctgctgaagctgcaagtcagagaagctggcaatcgtccccggcggatactggtcggtgatagctccggtgccgtcgccagtaccgccgtagaagtagtagcacccccacacgtagtccgaccaagcgactgccgactgaccgttcataccgccgctgcggcccattgcaataggcttacaggtaacagtggtgctaacacccttgatcgtctcagtagtgacaaccggcgtggtatctgcgtacatgcgcagctcgtaagtaaccacgaggatttcatccgacagcaccgtgatggtggtcgggttacctgcggagtccttgataagcgcacgggtggtcaggatgtacgcgccggtattgttgttgtatgctttggcaccaagctccgacagaacgccagtagcggtaccagccgggaactggtactggcagcgggagtaggcgtagtacggggcagtggtagtcccaccgctgtccgaggacgtacgaccaacctgcgccacctgtgcaccaagagcggtatcggtgaatgccggggtggcgctgccactaccgactgccaagtaagcaatgaggtcgtacatgctgcgaggatagccgctgccggtatcacccagtgcgtccataccaccgtccgtgataaggttgctctgccagtcggctacaacttcgagagtatcgagggacttacccttgctgatggtgaacacgccagcaatgccgaggtgattgtggatcatgcgaagctccatgatacgaagccagaccggagtcgtgcagtcgcgtcgagcggctggttgactacagggtgctgcttcagggtgaaggaatggaaagaactcgacagcttcgccgtctccgggtcaggcgtgtagtccttacggatggatcggatgtcgaacgaaacgaaagcgctcccgtacaacgtgctctccgggtcggcggcataatcctgcctagagcttcggagttcccagcttacgaaggaggaacccagcgacgcagtatccaaaggctggagcatgtcgatgttgctgtacccagcaaagctgctggtcagcatcgcggcatcgaactggtagaagctgtagagcttggacgtaacgtagatgccctgctcctcgatacgaccggaccagtaggccacacggttcaacccgtccgtgaccttgatgctaaggaagtaggagctgtcgtcgttctgacccagtacgtacttgtggttccacttaacggtgtccacccacagcggtttgttctgcttgctgcggaacgccgacagtacaacctgcacgtacttcgtgtccttgggcgcagcgccttcggcaacggactggtgccacgcaccgttgctgccggaggaaaccatgttgccccagttgcgttgcagctcggtcccatcctccttgcggtagatgatcgacacacgagcaccggccttgcccttggagcttgcgccctgctggacctcggcggtgcatcggatgtagtcgttgaccttggcagggatcagcgggttgagcaggtcgctgccgcccgtcttgatgttggcgaagcgcgcgctgtacacgccgctgtcggtgtcgtagtctgagccagtgccaatcgaccagccttcgccattcgatccaccgcccggcaaccacgtgccgtcgtcgcctgcctcgaagtcgccgttgggcacgagggtttcctcgtccacgacttcagtgaaagccgcccacttgacgacgacttccttggtgatgttgtccacccgtaccgcagcgcccgaagggagcgtcgattcgatgacctccacggtgcagcggccgactgggttgttgatggacaggcgagactcgtaagcctcgcccgccgtgtacccttccagcacgcccgtcaccgacaggccatctgcaacctcgtccgccatgagcggtcggccgtacagcctgaagtgattagccatgcttactccttagccaagtcgcccgagagcaaccacgtgttggtgtcgccgtcgatgcacgttgcagtgatgacggagttggtgccgcgagttgcggcggtgcagccgaccgggacttcgagcgtcacgcccacgtcgccagtgatgaccacagggcctgccttctgctgcacgctgaagtagctgcccgaggcgagcttggtttcaccgtcgcccacttcggggatcaggttgatgttgacggcgcaacctccggcgtacgtgcagcgcacgagtccgtactcggtagccttggcggcgtagtaagtcggaccctctgccgtgatgatcggcacccgcaggctcgcagcggtgatcggcgcaggcccggtgtagggcttggcgtaaccacgcagcacggcgaaccagatgctgccctcggcaggaaccgtggcgaagcggatgaagctgggatcggtgccgtcagcgagcgtgacctgatagtccacgtccggctgcatgccgatgccgttgacgtacacgtcgtagaagcccgcgccggatacgtccgcgcccaccatgtcgaagtcggtgtcacccacctgatcgccagtccaagcaccggaccagacgcgcggggcgacggacacgataccaccagctgccagcaactcggtgacctgcttgtagatgttctggataatctcgttcaggtccacgatcacaccgacctgctggtcgatgctaagggtggcgatgttgagtgagtcgaacatttcctgaatgatcttcaggagctggtcgttgctgaggttaaggtttgtcttgctgatgatgctaccgttaacgtagtcaacgagcatctgctgcaccggagtgctgcggtagatgtagagcttgcgcccagcggcgacggcaggcgagactcggacggtactagcgtcatcgtcttcgctcaggacttccacggtgtgcggagtccggtcggtcagcagctgagtctcctcgtccagcagtccgctcatggcgtacacgtgggacgggttgatgtagccaccggtaaagctgatctgccagtcagtggtcacgccatcggcgtcgaacacgtctgtcgcgtagcgcagctgcgggtctggaactgccatgctgcctcctgtttgctataggtgtaccaaaagggtgggccgtccttggccctgatcttactcctccttccactggctggctgcgcccttcagcagcgggatcaccatcggcagtcgcccgcccggaatcacgtcggccagattctccggcttgccagcaatgccctgagcgaagtcgttgatgactcccagcgacggcgcgaactgcccgcccaccacttccttgcggttgccgaactgcccaccggccagctgcttcagccacgtcggaccctgcgtatcggtggcgtactcgtaccagccgcccgccacgccagtgcccacgtccagcacatcgttgagcatacccgtcgccgacacgtagttcagcgtggccttgcccagcgccagaggcgacaggatgttctggtcgatggcctcgtcgcgctcctgatcgttcatcagggccacgcgggacagcacccgcagggcttgcagcggagccgccacagccatcgcagcagcgatcaggcccgccgtctgccatgcaccgtagttgcccacgtaccggcccagctgcttctgctgcgcgaccagcgagaacgtgcggtgctggaacagcagcttcagccagccgttgtgcgcccacttgccagtctcgccgatgaaggtgtcctgaagaatctgcgaggtgccacggttgatcgcgttgtagaacgccaaccatgcctgccgatccgccagcccctcgacgttgcgcgggtctactgcttccagcttaccatccgcgccccagcgcacgacctgatcctgcgtagcccgcaggcggttcagcaggttgtcgtcaatgcccatgtccttcagggcggtgtcagcttcagcaccatcacgcaggaacttcacgcccttggcgatcagcacttccgcgaagccacgctgctgcacagcaagcacggcccgctgccccgagaggatgcggttcgcatgcgctgccttctgcaccagcgaggtcaggaagcctgcgcgctcgctaccatacatcgacgcctgcgtgtccagcgagttgaacatgtgtaggtcgtaaccggcgagaccgaagccgcgaccgctgatgaactcgaagccgtcgaggatttggttgccgctgtcctcgcccttcaggatgcgcatgatttcgctgcgcatgcggggagcgatacggattgcgtcagccacaccagcagcaccaacagcggcgaggccgttgctgtactccgctgcctgattgatgcccgcgccgcccagctggatggccgaggtcagcagacgcgcattcgccagaacagtcggatcgccggtaccgaccgggcgaccaaggaactcggacatcacctgctcgaacgccttcagctccacatcgttggcaccggtcaggcgcattgcttcgcgcgccacgttgatgcctgcgtcgccgaggatgccgtgcttcgccagagcgatgtcaccagcaacacgtcccgcgtacttgcggtagttgtccatcacgcggttgtcgagatagtccatcagacggaacttaccgtcagcgtcctcgtactgcttggtcacgtcgaggtcgatacgcgccttggtgtgcttcgcaccgccacggctgtacttgcccatgaccttctgaatctcctcctcgttgagcgacatcgcccgcagagtgtcgcgcagcgtgtccgcctgcgactccgagaagacctgacccggcgcttcgatgacacccgcagccttgcgctcgatgcgttccagatacttggtagcgaacttatcgaggaagtcgtccccatacagctcgcccatcacctcgaactgatcgcgcatcgcctgacggataccctcgcgtcgcaccggaccagcagcagcgatgctgccgcccagccacgtacgggactcgtagccctccacgtcctcctccggcagacgctgtgcgcccaccgtaccggccgcgcgctgctctgctgccatgcggttgtagccacggtccaactcacgggccattgccttcactgcctcgtgcgcatccgggatgtccccgccgttgaagcgagtctcgcggtacagcttcactgcgtactcgaagtccgcgcgagccttccagcccgtggcgaagtccttgatcgcaccgataccgcgcacgtccgcacgccacaggcgataggccgcttcccactgacgcgggcgggtgcccatgaacgactcaaaccgaccatgccgatccatcgctgcggtgctgtgtcggcctgctgcaccctcgggattctccaacagggtgatcgcaagcatgcgggcaactggcgacttggacgacattagagtcgtgctcgtagcttccagcccgaagcgctgcatgatggtggacagcttcgccgcgtcgatgccgtactgcgcactgaagcgttcggagcgtgccatcacttcggcgacctgcacacgcatcgcgtcatcactgacggacttgtccagaccggtgcgctggtagaaagccttgcgctcgcggttcgacttgaagatcgagttggcgagcatgccacgcgtctgccgggtaccggcctgcgtgtcgcgcacttccgcgccgaggttgtcaccgacgaccgacatcaggcgttcgagcgcggactcctgattcttcagacccatcactcgcgcgatcttatccttcagccactcccacgcattcgggcgggtgttgcccggcgcgggcatctgacgcagcaccgcctgcacagcgcggttcgtcaggccgtaggaaatcagctcgtcagtgttggcgaggaagcctgcctgcggctggttgatgcgcgtctccatcgcagcggtggtcagcgtggagtccacactgccgatgctgttgttgatatgggtcagcagttcttccatttcctgcccgaacaccgagttgctgcgcagctcacgcagcgtggcagcgtgcagcatttcgtgcaccaccacttccggcgtgtagttccgcatcgccatcgcgtccagtccggcgttgtagccaccggccacacgcatacccggacccatgttggcaccggcgaaccacttgtcgagttccgattccggcacgatcttcaccgtgctcagccgcccgccacgcttcagcgcgttggcgatagcacgcacgtcctccgggatagaggcgttggattccagatacttcagcacgccatcgacgttaccgcccttgatacctgcggtcttccatgcgcgttccagcagcgggtcatgctgatcgacccggccacccacgctgtcgttgtaccgcccggtcgttgcgtccacgttgcccgcgtcccgtgcgagtgcaccagtggtgcctgcggtggtggtcgtctcctgcacgtcgggacgggcgaagatacggaagtcgtcaggcacgtcggccataccagcgcgcagccaatccacagcctcctgcttggcaagctggtggatgcggttgttcaccagcaccgggttggcgtcctcgcccagctcggccacagcgcgcgccttcaggtcggccgaccacgcttcgccgtaagcggcagcgttgcctgcggacaggtcgatggttgccttgtcacgaatctgcgcagccgagcgcacgcccggaatgtgcatcgcggtgcctatggtggtagcgaatgcagcgtcggtcatgaagtccgcgaagttgcggcgctcgcccatgccaaccagcgcggcgtccgtgatgacggaaccgaccgcgttctccgcagcagccgacgcgagcgacgcgcccacgcgcccttcggcaacgagtgcagccgagccgatgcccagcgccttagcgcctgcggcagtgacgccgccgatagcccagttgcccggatcggtgaagcctgccaccatgtcgtaaccgaagctaccccagccagtctgctgatccttgatgcgcatggagtggcggcgcaggaactgtcggtcgctgacgtacttcagctcgttcggcgagtacgctgcatcgcggatgtcttcgagttcgtcggcagtcatccacggcttctcccattccttcgggtcgtacttccaaccttccggaacgttctcgtcctcgcgcgcaaactggttgctgatcgcagcaccgatgccgctgtcgaacgcagcgccccacttgtcgaggaaggtcagcgagttgcgcagctcctcgtccgcgcggtcctgcgcgagcgcctgttcggtctgatccagcagcgccttgcgagcgccggtgttcagcacgtccacttcctgacgcacccaccacggcacaacctgatccgatgcacggacagcctgagccttgcctacggcctgcgcggcggtgccaccttcctgtgctacctgacccatcgacagctcggcgatgcccgcacgaatcttgccgatgtgttccttcgctgccgacgccagagcgttgcggccttcgatgggcgcacccgtccacgcatccgggatggacgcaccggaccacgtacggtcgcgcatgttcgggttgccctgccatgcggcgttgaggtctgcctgcgtggtggtcaggctgcgcggctgcgccgacactgcgggagcggacgcaccgcccagcacgctcggtgcataggctgcgttctcctgcccccagttcttcggattggtgccgccttggtagatgcgcagcgccttcgtcacgtcgcccttggcaagctgcatgttctcgcgcatgatgtcggcatacagctcgatgctgtcttggaagttgcgcatgtcgtacttgcgaccgttgcgcgcttcccacgttgcctgcgtggtgggcatgacttggaagtcgccctgtgctcctgccttgctgcggatcacaccgtcagcgtccttggcggcacgcccgttgccggactctactcgccactgaccgcgcacgatggactccggcactcccgcataagcggcagccttggcaatctgctggtcttgggtcagccccgaaagatcgagtgccattgtctatctccttacagtttgggttggatggaaatgctctgctgaatcgtaccgtcgttcatgcgaacgtagccctgcggtaccggggcctgcaactgacgctgctgcttggtgtgcttctcgtactcgtccttgatgtcgcgcccgtacaccggcacaaccttccagcccttctcgccaacagcgttgacgtacagcaccggctcgccgttctcgctgtccttcatgcggaacacgtcagccttcagcccggtgctcggctcgatgttgacccggcgcagtgctgcgtcgatggccttctcgatggcgggtccggtttccttcgtgtccatgaagcccagccatgcaccgacgctgccgatcactcggccttcgtcgtcgcgtccgttttcccatgcgtacttgcctgcgtcttccagaccgtaggccagcttggcgtgagtagccgcagcctgcaagccttccgcagaagtgtccagcagaccaccggtgtcagtgaccgagcggacgatggcgcgagcatacgcagcgcggccagagtcgcccagcttgttgccgaacatgccgaggtacttggggttgagcttggcgatagcttccgtaacacgagcctgagtagcctcggattccttacggctgttcgcgtcgaactgcgtcggatcgtcggtggtgatttctccacgggccacctcgtaagcaagctcgaagttcacgccaccattctccaacgcttgcagcttgttgaagaacgtgttgacgctatctccgaagtacagcgcagcggtagtcgcgccagtcagtcggccctgcacgggctgaccgttcgtgtcgatgcgtgcggcggtggtctgcttcagttccttccactgctggtacagtgcagccgctgccgtgttcggctgatcgcggagcacagcgcgcgccgtggtctggaactggtcggccacacccttcagcacagcgcctcgcccggtgttggcgttccacaccagctgcgacatggcgaccttggggttcgcggccatcgtggcattccatgcctgcaccgtgttcgcctcgatcagctccttgtccacgccggggatgttgatcgtctgcgcgtacgtgccgcgcttgaacgcttcgatgccaccacggatgtcctcctcctgcgcggccagcttctgctggtcggtcagcgcggccttggccgcagcgttacgctggttgatgacggcttcctgtgcgcggatgtgcgcgcctgcggactgtgccatgatcgaagccaactgcgtaccggagtacagcggtgcgtcgcttccagtctcggcggcgtaggtcgagttcatttcctcgatcatcgcctgcgacggcttggcaccaatgccctccgatgcgtacatggagacgagcgccatcttctcggcctgctccgggttggcatcgagccagtcggaacggtaacgatcctgcgcctgcttcacgtactgctggattcccagctgcccgtccgggtcgatggcgttcagaacgcccttgctgttgaggaacttcagcgtgtggaactcgccgcgatccgcagcgccacgatagaacgcagtgatcgcggacttgtacgactcgtccgtctggtagcgcgagggcgacagtccgtccagcagggacagctgcgcctgcgtcagcgcctcggtggccttctcgtccatgggacggttggtaccgagcatcgccgtgcgcttcgccagttcgttgaagccggtggacgccgacgagttcgcagcgtactgcgccttcaccagctcctgctgctgccatgccgtgcgctccttggtgtgcaggtccatgagggaacccgcgcgatccatgaaggtcttctgcaacaccgtgtccgcgaaaccgttgccggtcatgcgggcagtggcgaggtcgttgaactccttcgccatcgcctcgggaggaagctgacgcaactccggcatacgccgaagcaagtcgctctccatttcgttgacctgcgagagcgtgttatacatgctcgcgccaatctcgtagttggtgtctccgaagattttcttgtaccacggttcggtcgcagcaatctcgtccatggtcttaccagcgcgggcggcaacgaagccgtcccacatctgctgctgcttcagcttggcggtgttcggcgctgccagctcctgcaagaactctggcaggttgctgtccggcatcgtcataccaccagtgcttgcgaaccagtcgttgccggattgaaccggcccgacctgattcacaccagcgccttgaatgctggtgttgcccgacagtgctggggtggcgttgatgccaccctgcaatgcggactgcgtgttgaaggtaaccgtgccgatgtcagccattaccatgcacctcctgagttgcctccgctgccgctatcgaaccagccgaggccggacgtagtggtggagaagttgtcgtagttgttgccgaagttgccggtgaccttcgccccagtcacggactgcttgccggtgccgtcgttgtacccgaaggtagtggacgcccacgacttgccgccgcgatcattggactgctgccacgcctgcataccgttctgcgctgcgttgctgaaggactgagaggcaccagtgaagttgccgttgtccgcctgccacgtgccgaccgcgaagtctgccacggcctcgcctgccatcggcccaccgaagtaggtagccacggccacgccgatcagcttgcccaagcgacgcttcattgcctgcggctcgatgtgctgcgagtagtcgaactgcccgaacgaacggctcatgtccatcccgttccacgcgcgcgacatgatctgcgcagtctgcgatgcgccccgcgaggcgaggagcgagacagcgttggcctgcgtctcctgatccatttccgcctgcaaccgcaccatcgaatccatcaggtctgcggacgagccgccgacaccgacagcaccagcctgcgcctgaagtgcgccacgcgcgttcgccagttggagctgggagttaagcccagccccttggcgcgcacgcagctcctcggacagcgcttccatgttggagttgtactccttcgcggcggcgtccagttgggcgttgttcttcagggaccgcatgaaatcagcgaagccggtcttggcgacctcgctgcggttctggttgtcggtctgcgcaacggctgcacggtagttcgcacgggcaacgcgggtggtgttgttcgcttgcaggatcgtattaaccgaacccattagctaaccctccgtacattgttgaaagtctgacccgtccagctcaggccggtcacccggagcgggagccaatccttgctgcgaatctcgtaggtgcactcgcgcacttcgcgcccgacgctgatgttgagctgcccccggtacaccggttgccgcgcgatcagattgtcggagtcgccgaggatgcggccctcgaagtccgtagtggtcacattgctgttgcgggttgccaccgtggcgatcatgcctgccgtgttctccacgtccaccgtcaccttgttgagggacatgcgtccatcgagtacggcctgaccgttctggtcccgagggaacggattggtcgggatcaccagagcttcggacaccacgccgtattccagcgcaccagcagcgaggtcatcgaactggttaaggaagtcagacgcctgcgcgtagggacaacccagcaggaagtacgggctagtgctattgacggcgatgcttgcgctcgcagtctgtacgcccgtaggtgtaccaaaactcgcccagctgtcgaggcacgcatgcgagtccggctcgcccttcgggtcgaacacgtcgcacgccaccagcgacccgcgcgcagtgaacacgaggccgttcttcttgtagctgctcacgccgatgatttcgcccagcgccgggtggtaccggaacttcgaccacgcatccacgatgcgctgcccgttgttcttgttgtcctcgtaccggtacaggtagaagtcctgcgggtgctcgcgagtgcggaacatgacgaggttcggcgcagtgagcggggtgatctgcaacggagtgcccgacagccacgagtccagctcgttggacatttcgtccgtcaccgtctgctgcccgttgagcgcgcccactcgcatctggtgcaggctcgtgccttcgctgccgtactgcgcataaaagatgtagttgcccgaggtctgcgccttcgcgtcaaccgaatccttgttggcactgaacgctttaatcagcggattcttcggactgaacaccgagtcgccgctgatgccgtactgctgacggtcaccgaagatcacgaggttgccgttgtagagcgtcgcgtgccggagcacatcgccctcgctgccgtgcgcgaagatttcgatggggtcgctgtcttcgatggtgacggccgagccgcgccagaagttcaggtagtccgccgagcgtgaggcgttgacgtagttctgtgcgccgatgaccagccggtcttggaagacggacagcatcgtgatcggcttgtcgatgaaccacgggatcggcgaggtcagaccatcgcctgccactcgcgcaccgtaggccggatgctcgccgctgctcggagccagagacgtgaggcccgcaccgttgcgtgcgatgtagcctacaccgttgtagatgtagagctgcgacacgaggttgtcgatggtgcactccacgccgggcgcttcgtaccagtccaccgacccgtagccggaagtctcgccgttctccaactcagcgcgcaggtagtacgactcgtccgcgcctgcaccactcggccgcacgcgaatgaccttgccgtgccagtggaacttgacggcgtaggtcgcgtctgtaatttcctgccctgcggcgtagaaggtcgtgccgtctccctcgtcgtcaaccgtgatgtccttgaactggtcatcgtcaatgatgatcccgcccttgatgtacgttgccgacacgcctgcatcgaccagcaaatccgacagctgctccgcgatgtactccgggcgcgtctgctcagcgctcgtcacgatccactcgttgaccgcagagttgtactcgttcactcggtcgttgacgtacttctggtacgccgcgtccggctccgtgccaccgggaaggtagaacgggatgtcgctggtgtcgagcgttccggggtacgatgcggtaaccgtcttgaacgttaccgtcagcaccgtgttgtccgtccgcgtcaggttcaccgtgtacgtggtgttgtacttcccggtgcgcacccatgctgcgaggcgctggatgttcgtctgctcctgccacacgttcgtgctggtggccgaggggatcgtggtgttgcccgcgatgtagacgtagctgccgatggccgtgagcgacgatgcgcctccgctgaccagcgtgttgacccacgtgctgttctcgtacaccagagggatgaacgactcgtccgtcttgttgtagaggaacgcgaaggactcgctgcccaaggtcgaggcgtcgcgccggtacagcagcgcgtactccttgccctcctgcatgaagtcgaacacgtccatgttgcgcagctcggccgaggtgacaacggcttgggaagcagcgaaccgcgtaccacgacggcgcacgaggccgttcaccggatcggacagcacgttgatctgctcgtgcgtctgtcccggccgacgacgatgcgccggtttctgactgacaccctgaaggatgtcgggataggttccgcctgcctttgccatgttgtctccttagccggggaatgtgacgtggctgtgccacgggtgaccgctgtagttccagtaacgggaacgcagcacgtccacggatgcgcgagcgaacagcgggttcgccttgatctggcggatgtgctcggccttcaagttgatgtaactgtcatcgcgctgctgcttgatcttggcgtacttggtgttgtcgccgtcgaagtcagactggaaccgcagcaccgagtcgtcgcgcacgaacatctgcacctcgtaggggaggtcatcgaagtccagcagccgcaccagcttggcctgcacgttgtggtcgaactcgtaggtgttgcgcttgcggtcgtacagtcggcgtccgcgctgcaccacgtggccgaaccggctcgggttgcagtccagcttcagcacgtccgtggggaccatgatgtacttgctcgttgcctgcggcttcagctccacccattcggtgttgaaccacagcgagagtgaggacacgtcacggtgcacgcggtcgatcaagtcaacggcgtcgtccttgtatacgtggtcatcttccagcgtgttgagcttcgtctcgcccatcgtcttcaagcaggcgttcacgatgtcgagcttggtgatgaatgccatggtgtctcctgagaggaacaaggcagagacgccggagcgcccctgccgggatgttgcttagtccgcagccagagccagagcggccggtgcgtactcgatgtcctgcgagccgatttcgtcgtccacgaaacggacacggacgacccagcctgcggtgccacgggtgtcgtagtggacgccgacgacggtaccaacggagttggcgggcagaccggccacgccagttgcggcgacgacgcggttggaaatctcgaacggtcggtcaaagaccatgatgttgctcctgtgttggtggaagaagggcgcggtttgagttacccgaaggattcagggaccgcgcccagcggattaggcaaccttgtcgatgcggcccgcgttctcgacgcgatccagaccaacggcgaaggacatccacgagtccacgaagtagcacttcgaggcatcgctccaccacaccgaggactgcaacggcagcgcttcggcgatcagcagggccttcggcgacacggccacggcgatcagggtgctgaagtcgccgtcgtagaagtcgtcgttgtcgtcgttcgacagcaggtgaccttcgatcacggtgttcggcaggttctcgctcgacagcaccgggacgccccagccgtggaaggtcgggatgccggtcagcttgttgccgtccgaggtcaggtactcgccgttgctgatctgctcggcctgctgcaacaggtagaagatcgccgggcgcacgatcaggaccacgccatcgcgctgcggcttgaccttcttctcctcctccatgcgggagaacagtttgccgatggcggcgtacaccttggccggatcgttctcgtcaccagcggcggacagcacgacctgcgtggcaccgaagtggccctcgggcgcgcggccgttgcgggtgaagatcgactgcgtggcagcagcggccttcgcggcggcgatgctgatggtcaggtccacgaactcggcgatttcctgaccctgctcgatggcgatttccttgcgggtgtcgatgtcggtgaagatttcgtccagctgccagatgctgtgacgcgacagcagcatggtatcgacggtcaccgacgccttgctgaagtccaccggggtgccgtccggcgcgtcaccgcgcttcagcttctgaagcttggtacggccgatggccttcttggtcagggtgttggtgcccttgacctgcttgcgcgggaagaacttttccagcaccgagctggacacgtaggtgtgctcgacatcgccggtgaactgttcgaggatcagggcgttctcgttgccggactggttgacctgattcggcagaaccgggacagtcgggaagatggtgctcatgctttgtgttgctccttggtcttagtggatgacgcgcgcgttgagtgcacgcagttcttcggagtgggccgcaccacggatgcccttctcggcaaccagcttgcggtactcagcgcggtactgctccttcgtgataggagcgacgccgttgatcgacgcggcgggggcggcggcgttggtagccggtgcgcccttgacggtcgtcgcgggattggcctgtgccagagccatcaggtaacgcgcggtcgcctgagcgccgaagccaccagccgacagcgattcgcttgcctgcttcagttggtcggcgggcaggttggcccgtgcgaactgctggatcgcagcccagttctctgcgccacccacggcttcgtggacagcagcaacgttcgcggcgtgcgctgcggttgcagcggcggtgacacgagcgatgctctccttcgccagagcgaggatcggtgcggaacccttggccttgtcgccgaggacttccagcttggcttccagcagggcgaagttgcccttcgctgcttcggtcagttcgcggctgtcgatgtcgaggcccacggtgttgacgaagtattcggccgcgatgttcaggccgttgtcgccgtagtccgggatcgacaccgcagtcggcgcagcgttcgccggggcggcgggctgtgcgggagcggcaggttcgagactcagcgcgtcagcagccggaggtgcagcaggagctgcgggctgtgccggtgcggccggagcgggctggccgttgggcaacagcttgtcgtctgcgggagccggagctgccggtgcgggctggttgccgttcgaggttgcgatcacggttgcgccgggaccaccgcccggaggtgcgttggaactcattgtgtctgtgtctccatgttgttggcgttgtcgatctgctgggatgcgttctgcatggcgagctgctgctgtgcacgctgctgcatcatctggccgtactcggcctcagtcagcacgtagacgttcgggtccaagccaccagcggcggcgaggtctgcgatccacgcggacagcttcagtcgttcgagaatctgcggcggcagtgcgaggacgttggcgaggttgctgccgaactccaacagccggtcacggtcacccgtacgggagagcgcggccaagccggtgatgatgacaggctccaagtccttgcctcggatgtcgcggcccgtcaggttcatcacccaaaaggcgactggtacctgcacgtccgcagcgatccgggagtagccgccacccagcccgccttccagttcttcggcgaccatgcggatttcctgcgcggtcacacgttccgcctgacgagtcaccgccgtctgcaacaggaagcctgcgccgatgcggttgatgtaggtggactggattgcttggttggtttgcagcacgccatcgacgcctgcgttaatcagctcgatgtcacccttcatgccgggaatggccgcgccattgggcgacgccatgaagtcctcgacggaggtctgacctgcggggttaaccagccaccggaactcggaggcgaggatcgcgccctgcactgcggcctcggacagcatcgagagcgactggaagtcggcctcgtagtcttcgaccaagccggagccgtagtcatcgcctgcggccaagtcccagctaaccgcccggtagggcagcttgtctgcggtgtaggtcgaggagaagttggcgggcagcttgcagttgcaaatccacacgtcttcgttgtacttgccggtcttgtggtccagcttgacccacttgtactcccacaccatgccgtcgtcatcgggcttgaagtccgggtgcgcgacaatggcagcgagcgctgcgggttccagctgggtcttgtgcaccttctcccgaaggatcagttcgtagacctcgccggtgcgggtgcgcttgaccacgtagtgccgcatgttgagcacgcggatcgtgtccttctccaacaccatgagggcgttgcccagcacgatcagcatcttcagcaggtcgtacagccgggagcggatggagcgcttgtccagttcgagactggcatcctgctcggccttcgcaagcatcgcctgcatggcctgcaagtcagcgccttgctcctgcgcagcctgcttcgccttgcgcttcagctccaaccggaagaacgggcgggacggtgcgaacagcgacatcatcagcttgttcgccagatggttcactgcctgcgcgccgagagactggaacccgtgggtcagcggctcggtgtcctgatcgcggttcttgcgagggaacagcttgggcacggtccagctcgaatagcgttcgagtcggtacatgatgccctgtcgcttgttgtcgtaagcctcgaactggcggtgagcggtttggatcggatggtccatgctcacctcacaacaggtctgacccggccacggtcgtcagccgggaagctgcggtcgtggtcacgggtcgggtgtaagtggagcgggcggtcttgcgtcggccgatcaggtcggcagtctgcaagtcgaggtcggaagttcccagccgcacatcgacggtatcgacgggggcactcagcaacttctcggcgtactcagatgcggcctgctgtgcagctgcctgtgccatctgatcggccatcgcctgaatctggtagttcgtggattgagtttggaggttggtctgcttgtcgatagcagcagcttgcttcagcgctgctcgcttggcggacccaccaccaacgatgctacccataggttaactccttcgcttggtgaattggggagcatgccgttccagcaggtagccgtagcgtgcatacatccgtgtgagtgctcgggagttccgagctagtgcaccgcctgcgctcagtgagtcgcagtggttgatgtcagccagatgttccatcacggctatgtaccggtcgaaggaactgcccggcccaattcgcagcaccatgttctcaacgaacgtagtacggttcttggagtaccacggtgtgacaatggcaaagcacagcaggtaggcttcatcaatgattactgcatccactagaccctgtgttatcagggccactgtgtaatcagggtcatcacagttgtagctcacagaagattctctgttgtctaccttactatcttctctagatgacagatacaaagcggccgttaaagccgccttgatctgctcactatcacccgtcgttggtgttcggtacggaggaatcaacggtgaaaccctcctgtaagatgttcaggacgcgggccatccccaactgcatacctgcctccaagggcgtggtattcgagttgacggacagcgacagcccggacagcttccgcacggcggccagctggttcgggtggagcgtcatcaggactttcactttggcgtcttcggccatggtgtctcctctgtgctataggtgtaccaaaaggtccggcaccggttccgcttaccttcgcggccgctccaaccggacctcagttgcctcgtgctataggtgtactgaaactccgtcagctgaagaagtacggagaatcaaggacttgccgaaggtccagctcgcccatcggcggcggctccggcaggaacgggtaggccgagtggaaggccgacagcacgtcgtgccgctcgtacatcgacacgaacacctcccggatgatccggtacagtgccgcgctgtcggcggcgtgggtgccgaagtcgtcgtgaatcatggcgaaggcgtcgatgccttcggccttggccgcgttgaccaccagcgtcaggtggcttgcgtcgaggctgtgcacgaagttcggggcgatgccgttgcggtgccgggacttcttcaccgcgtccgtgctcttgcgcagggacagcttggcgttgccgcacagcttggtgttgatgcggtgctcctcggactcccagtagacctgcaccaccgggaacccggacggcgtgatccaccggatgcggtcgtacccttggttgaggatcgacccggagccgcgctgcaaccactccatcgcgcccgctgcggcgaccacggtgtcggcgatggcctcacccatgcgcttgctcaggaagcgcgctgcggggccgtacagggccttgtcgagcgaggggaacttcccacacttcaggtagtcttcgatgatgaagtccgcccacgaggactgccgcgagccgtacggcagggtcatcacgctgcgcttcaccagcgagcgtgtgaggccgtggtcgagccacagcgtgcggtacccttcggcatcctcgtcctcgcctagcaggacggcagtcacgcggtctgccaccatctggtagatgtcattcggcagcggtgctgggatcaggttcgtcgccacgccgcctgctgcgtcgcgcagcatcgccgagaagttctgaagcccattgcacgaaccgtccatgccgactgcgatgcggctcaggaagcgatccccgaacacttgccactgctcgtactccatgcaccagctcagaaattgcagcggcttgtcggcggtcttccactcgtcgttgttcaccgggtccgcagcgaacgccatgatctggtcgtgatgctccgctacccacttcacacgatccggcagagacgccttgtcgtatccccatcggtttgctcctgtgatgcagaaccaatccttcgcgtccttagtcagcagcggcttgccatcggcgaactccaagagcgccttctgcaagtccgaaccctgcggcgacacgccggtggtctgaacgtacttgcggccacggaagtcagcgaagtacacgaagtagatgctcgggtactcggcgaacttgcgcgccaccttcattgcgttgtagaaacgattgcccttgttctgtcgcaggcgctcgtcggtgtgccagttggacatgtcgcgcttccactgcttgaactccaactcctgattgtgggacatggtttccttggtcatgtccttcgtcagccactccggcttgcgcggcttcggcagctcgccctgagaaatgatttcctccatgtcgtgcaccttggcgatggccgacacagcttccatcagtcgcttgttgatgcgccacggcacgcgctgcaatgcgttgatcgcagccatctcgttgcgcagctcggcagcgcggtactcgtcgcgggtctgagcgtaggtcttcaccatccacggattgagtcggcgcatttccttcgtgtggaatccaccgttgtcgatgtccacccagtccatcggcggctcgacgcacggcaggtagaacggcgtggcctcgatcacgaagtcgctgatctgagtaatcagcttgcgcacctcgtcggtcagcacgatcttgacgtgcgtcttggtctggaacttgcggtacgctgcgcctgcactggcagcagtctcggtgaccacgccaatctccaacatgcccagctgcgcaagctgatcgcacaggtacgcgccgacctgatcgcgctgtgcctgtccccactccacgaactcgatgccgttcttgcgtccttgcatcttcatcaccgtcatgcggtggttctcgttgacagagagcttgcggtccatgtcgttcatcaggtggtagaacagagtcggctccgcgtcggcgaactgcgtcagcaggtactcatggtacacgttgatgccaacgttcttcaacacgtcgcggtcgctgccttcgccgtgcttgtctcgcatgcaggaggtaagggcaccgcgaacggcgacgaaggccacagcctcgtaccactcgcgtgcctgttcctcggcgctgacgggctgtccacgcttgttctgacgctcgggatcgtacttggcgcgcagaagtggcacgtgcgcttgcgcacggccgattcgcggagagtcgatgtccgcacggatgcgctccgcaagcggaagcacgaaccggcgatacactgcttgggcgtaggggttgttgtccgcgccgcccttctcctcgttgcgggcgatggacttctccatgcgctccttaccgaaggcgtaggtttccagttcgagttccacttgcgagagcattgttacctccgttgctgccgcacggtgtagtcgcgcggcgggtagcgtttcaggataccgcgcatgatttccatgtgcaggtcgtggatgatgtgcggccacgcctcaccgccgatatcctcggccatgcacgtggcagcagcgccgaacaagtcggcaccgtaccgggcgcgcaccgaaacctcgacgcggcccatccatgccgaggactggctgaagtccagctccggcttctcgaaagtgatcgcgtccatcagcccctccgctcgtcaaggaacttggcgaacgcttcctgcaccttgtcgcgcagcgtctcgttcggccacagggaaccggcgtactcgccgaaaggaacgctgatgcgcagctccaccgtgtcgcgctccatgttgtgccatgcttgcacctcgacgctcacaggtctgcctccttcttgtcgtgacggatgcccttgtatcgcggctcgcgcagcaggccgtacttgctgaaggacatcgcctcgatttccacgatgcctcccacgctaggcagctcgctctcgctgtgcggcacgccgctgccaacctcctgcgtcttgccttctccgaggtcaacgacgaccgtgtacacggcgcggccggtcttctcgccgactgcttcgttgatgccgagcacacgcaggtccagcgtcagggtcggcttgatcttgacgacttcgccgttggttcccttgtcgcccttcacccacttgccgctcggcttgcgcaggatcagcccgtcgtacgcgccgccctcgcacagcagcttcgccgcttccatgctgcccagctcttggtcgatcaggaagccctgcgactcggcgtagaacaccggcgcggtgccctcggcgatggcgtggcccatgctcggcaggcggctgacgcgctcctgatacacgaggtcgctgaaaccctgctcccattcttccagcgtcacgaagtcgaacaccacgaacatcggctcggtgtactgcgtgccgtccttcttgcggaacatgccgctgacggtgggctggtcgatctgcgggtgccagtattcgccgaagtacacgccgaccgggaagaacggcgcggatgcgagagcgttctcgatgtggtgtgcgctgacgacctgctcaccggtgcgggagaacaggtcaaccacgccacgatccaccggctgcatctgcacgtcgcccaccttgatggcatgcaggcccttgttcaccgtgggcacccagtggccgcgcttgatggcgaccatgttgcagccgtcgtacttcggctgtgcgatgtactcggtgcgaagctgctcctcggtgggccgcagcttcttcttgatcttgtcctgctcgactgccttgtggacgatgtagctcatgcgtagtccctccaaatctggaacatggcgagcggcacttcgtaccacggaacgtagcgctcccagtacgtggccttgccgtcgtaccactgcacgcggaagttgcccttggtgaaggcgcggttgatcttgaagccgcgcttgcgcttcttgtagccgggagcaacccggacattctggcgaggcacatcaaacatcggcgctgtcctccttcttggtgccgtcacccagcgcggcgttgaaccgtgcgatgcgggacgacatgaactggttgacgatggtgccgatccacagcttgcgcggagcgagcgaaccacggtagccttcccacgcatcggcgatgcgggtatacagctcggcctgatcttcgtcgggcaggttcgggaacccggccttgaccgcattctgcaatgcctcctcgtggtcggcactctcgccccacgcaacggcgttctcgtaggacttgatgagcatggcggtctggttcttgtagagcattcagttctccttcgacgggaatggaacgaaacctgcgaggcccctcatcacgaggatgcagaatgcgtcgtcagggtatgtacgatgccagagtgagttggcccactcgacatcgaactgcttgcgggtacggtgctcctctaggaagcgcgcccactcggcctcatgtgggacgtaccgatgcacttggccgcagcgggcgcaggccatcagtcacccttgctgaaccagcggcggatgatgtactggcggatgaagctgatcgctgtgaacgcaatgccgatggcgtgcgccgacagcagcggatgctcgggatgccacagcaccggaagcagcgcgatgttcgctgcgtagttgatgctgtagccgatgccgatgttcacccaagcctctttgatggagcgcgccttactctgcgccactggccttctcctcctcgcgcagttccagctccaacaggaacagctcgttgatgatgtggtgcgcccggtggtggatgcccgtctccgggtccagcttctcgccgaggcagcgcttgttgtcgtgtcggtagctcgcgtcctgataccgttcgagcgccttctcgacatgctgccacgagtgcgctttgtacttctgcgcgccgaaggtcagggtgtcgatgactcgggccagtgcacgcggcacgccctcatgcagcagacgggcctgcggcttgcccccgtcatccttcaggccgacgccacggtcggacagtgtgcgacggtcctcgtcgcggtagctcagttcgggcattggtacctctcgtctggtggtggtcacgcctccgatgctgagaagctgtcggagggaatcgggaacgcagcagctcggcttaactcgaccgtcgaagaagacctcgacatcacgagcgaacacgcggcttacctgtccacgcagcccgatcattgcgggcgcattgccgatgtactgtacccgcatgccgctgcggatgtcggtgatcttcatgtcggttccttatgccgggacggtgatgtgcttgcgcgcctcggcgctggtcgtgagcttgcgcccacggctgtagccgtcgcacacggtgcactgaagcaggaggtaggtaccgacctgcgtgcgggccggatcatcctgcgggatcatttcgttgcagccgcacttgttgcagcggtgctcgctgccgtcggccttgtagtacactgcgacgttcggatgctgcgagtaccaaccgcgcagcttcttgtactccaacttcatggacttcacgtcgatgcggttgtacgcttcgcactcgtcccatgctccgggcaggctctgcatgcaggccacccacaggtcgaagccggggaagttgtggtggtcgtacttgcgcagctccggcacgatcacgccggtggtgtactccaacttctgcgaggtgaaggcgaactcggtgcggttcagcagcatcgggtcgatcacctgcaccggagacacgggcggcaggccgaggattgcgaggcgagccttgatcttgcgaaggtcgaacttcttgccgttgcgagcgagcacgaagtcggcggcgttgagcagtgcccacagcgccttgccctgcttgcgatcatcgaacacgtcgcgcacgttgcgctggtccatgtagaacgacgcctcgtcgtccagccattcgcaagcgaacgacatcagcgaccagtcacgcttgatctgcttgacgctgaagttgttgttgaacatgccccagccatagaactcgatggggaacgtctcgatgtcgaggcagagaatcttcgggccgcgcttcggtgctcggcgaatgaactgggtaagggtcacggtgtctccttgttgatagcccgacgctttcgcgctttcgcattgcgagcgatacgcttctcgtcgtcggtcttgtaggtaggatgcaggtaccccgtgatgttggtgaggtgcgaccgcaggtagttggggatgcccgcacagaatgcgaacacgtcgcgcacgccgtaccggcctgcgttgttctcgaccttgccgagcagggagttgcatccgcgatggagcaccccgcgcacagcgccggtcttgtggtcatggtccagcaccggatcgagcggagccttcaggccgaactgtccctgacagagacagcaccggttgccttgctccgctgcgagcttgatgcgcagcagcttgacctgtgttgcagtgagtcgcttcatgctttgtatgcctccaagattgcacgcttctcgttcacgtcctcggcgaggtcatagaacgcctgcttcagcttcggcccgaacacgtcgagcttcagcacgtcgagcagttctgcgtcacgatccgtccgcatccacagcagcacggcttgctcggcgaatgtcttgcgccagtcggcacccaacacttcgctgtacttgccgctcacgatctgcaccgcttcgaggttggtcttcgtctcgaacagcagctgctccgctgtcaccttgcccaccttcggcagacccggtatgttgtcggcggtgtcgccgtggagcatctgcatccagaaccacttgtgaccgtactgcaatccgttctcgccaacgatgtcgtaagcgccgagcggaacctctgtgatgtcgtagccgtcccagtctacgtgcacgccgcagaacattcgcatgtccttgtcggcgctgtgcaccacgtgcaggatgttgtggtgcaatgctgcaccctcgttgacgtacgcgatgccatcgtcggcctcacgggtcagccagattttgggagtgaaagcgtcgccctcgtatgtctccatccactcacgaaggaacgcccagttgttgggcttgcggcctgcttggcgctgaccctgatacggctgcgtggtagcagcgaggaagcgatcacccttggtagacgcggcgtgcgtcaggtgcatgacgatcttgcccgctccgctgacatgcttcagctgtgcgcagcgggagagcacgttgcgtcgtgcatcccccgccgagcagttctcgctaccagccgcgaagtacgccatgtagtccccatcaacgtgagcgatcacgcgcgggttgtgctgacgtaccacctgcaccggcatcggggagcgctcaccggccgctgccatgagagcgctcaggtccatcaggcgatgcctgccatcgggtcgctaccgtccaccgggaacggcggcttgtcgtcggccggagcagcgtcggtgggcgcggcgttcgccacgtcgccgaccacttcgtccagcgcatcgacgccttccttggtgaccgtggtgctgcccgccaacttggcggcggcgtagtcgtagcacggaagacccttgaagttcagcgccgcagcgatgcgcagctgcgtcttgttcttcgactgcgcctcgtgggtgaccttgccggtcttctcgtccttgcgctccgggtactcgccggggatgtagatgctgtcccacatgtcggcgtcggcgaagtcccacacgaacgcacccagcggggtgatctgctgcggcaccgggatcacggtgtccacgaacttgccggtcgggatgccgttctccatttccggcaccggcatgaccggcttgcggatggaagccttgtcgatttcggcgaaggtcttgttcgggtcgcgcttgcccggcttgtggatgacttccagcagcacaccctgacccagcagctgcacgaagtggcgctcctcggtgcgcaggcggctgaagattttgaagtagtgcgccttctcgttggtggacaggccgagggtcagcgtcatgcgcaccggcaccggaccattgtcggtttcgatgtgcgggtgctgcttaccggtcagctcgaacacgatggcgacttcatcctgcgtcttcttcttgccctcgaactcgaactcgtgcttgcccagctcgtagtacccgacgatgcgggcggtggtcacaccggcagcgggcggggtgtagtcgaagctgccaccactggcgaccgactgatccttaccctgcgtggcgaccttgttcaacagtgcgtcaagactcatgcgtgttgttctccttattcaaacgacgggttgtgattacctacgaagtccttgcggatcgacgcgcggtactcgatgaccagaccggcgaactctgcgggagggttcttctcctccatcatgttgtcgcccatcttggtttcacacgggacgccaagcggcagcgtccagttgaaccaccactccatatacaccgacgcttccagcatcgaggcgtgcagcagagcagcggccttggttgcgatgtcgccgtgtgcatccacgtagacggcatcgtgcacctgattcacgagcaacgcacggcccaaccattccttcggttcggtcacgtacttccggtagaaggcgcgcaggctgacgtacatcgccgccttggcccattcaccaccggtgccttgcatcgggtagttcttgatttccgtgggcgagaacgactgcgcacagccacccttgctcgcgggcttgttggcgatgaacaccggggacggtgactcgctgaaggaatacatcttgccgtccggcgtggtccagtgcgaccggccaagctgacacgtcagcccatgcggcacgccttgctgccccgcgttgggatgcggaacgaagcgctgagtgctgacgcggttgcgcttgatgtgctcgaccatgcggtcgatgtactcgcccagctccgggtaacgctcggcctcaccgcgcaccagcgcctcgacttcttcctccgacatgccggtggtcgcagcgatcttcgccacgcccgcaccgtacgcacgctggaaggagaacaccttcgcgttgccgcgcttcttcttccacttcttgtgctcgggatgcttgtcgtccttgctcgccttcaggatgaagtcgtagtcgtacttgccttgctcaccccacgcctgctctgcacggaggcagtgcatgtcgaggccctgcttcaagtcctcgatcagctgacggcactcggtgaggattgcctgcacgtagatttcgagggaggtgtagtccgactggatgatcttgccaccccggtgccgggacacgaaggcgcgcttgatctgcgaacccttctcctccaacgtctcctcgtccagctcgcccttgctcacgttctgcaagttcggatcgctggaagacaagcggccggtaaccgtgttggtcatgttgagcttgtggtggatgatgt

SEQ ID NO: 17 - DNA, 44415 bp, unidentified
  source 1..44415: mol_type = genomic DNA
ccgtcgatgaactcgatccatgcctgccggttgagtgggccttggcagatggcgtgcaggatgtcgaacttgatgttgaacccgacgaggaactgctgcccgtaacacagctcacgcagccacccatcgggtgcgccgcccatgtactggttgtctatcccgactcgggtgtcgtagtacaggccggtgttccgtgcgtcacccttccgcttgtagccaatcgccacgatcttgttcatgtcgtagaacggattggccttgcgcttcaggatggaacggatcgtggtttcgaggtcgaaggaagtgaagctcacagcggccaccgttgcagggccagctggtacatttcatccgacgcatcgccatccaagtccagcccgtcgcgcacccaacggaacacgatgatgcggtcctgcttgtccttgatgttgcggcgcttgcagatggtggtggcctcgaccgcgcgctgataccagccggagtcggcggtcaccatgacgttgaacacgccgttgcgcagcgcataccacgtggtgctgtagtcctcgtcctcctcgtagtgtccatcggcaccggagcacagggtccatccctgatcgaccagcttttcgatggcctcgtggaagtcctgcaccagcacgaggaagtcgatgtccgtgtcggtcacgggcggctcgactgtgtagctgctgccggtgcggctggacgtgatgacgcccacgttgcgcggcaggtagatgttcggttcggtactcacggtgtgttacctccgggcttggtgatccagaacgtgaagcacgggatcagattgatgcaccagcgcttgttgtgcggcgagtagtgcacgccgatccaagtgctgtgtttgttccgcagccatccccacttccactgcggcgcgtcgttgcggccttcgatgtagcctgcgtcgtgcaccttgcgcagcagcttggcaaggtggattgcttgcgcgttgctcacgcagttgaaggtcttcgcctcggtggattcaccggggaagctgaccgacaccgtgaacccggtggctacgatgtgaattggcttgctcatgctgcctcctgatagaagcgggcacgctctgcatccatcatcacttcttcccgaacgtcacgcttgccgcctgcgcggtgcagcttgttcttcggggtgccgatgtagcggaagcgttccatcgctgggtcattgagcttgccgcccatgatgatgaagtcgcacgcaccctgcttgccggtcttgctgtccttcagtgcggactgcggcgggtactggattccctcaccctcggcgctgatctgcgaagtcgccacgcccacggcgtcgtacttcacacaccagttgcgagcggcctgatacatcgcctccaacatctgatcggtacgctgcccgccgttggtcatgccaccggtgaacgtgatgttgtcgatcatgtcgaagatgatgaagccggggttggtctgcttgatgatggcctcgacttcaccggagttgaacccgtggatgtcgtagaactgcatgcggtggatgtccccgcccatcgcatcttcgatgcgcttgcggatgctaccatccttcgcccactccaccatctcagggatggtagcgccgagcagcgactgataccaccgctgcttgatgcgcttgcccggcccctcgttgttgagccagatgccggtgcgcttctggtccggccaaacgttgtcgagctgcgtgatccagtggctggactcgctggtcaggaacgtggtcttgcctgcgtcgggacgcatggcgtagatgccgaagtcaccaccacgcagagcgcgcaggttcttcgccaacgtgggcagtcggaagtggatgccgatgtcgtgctcgtccatctgcatcagttcctcgggcgtctcctgcaccagcgggagccgcgccttgcgatccattcggtcggtgatcgtctcggccaagccgtacagctcgtcgcgcaggctgaactcagcgccgccattccactgcacgatcttgctgaccgcagtggtggcaagctccaactccaacagcttctcgatcatgccctgctctgcctcgggcgggaccggctcgcgcatctgcttcagcagaactttgagcagggacttcttgtcgtcgggctgcgtcttccacttgaactccatggcccagccatcgaacacatcgaacggcaagtccttcgtgtccgggaactccttgtagtacgcacgcaacgcatcgagcatcagcacggtcagctcgtccagcccatcacgtggtgcgctgggtaccagccggtcgaacttgccacggttggtgcacaaccgcagcagcgtggtgtcaagactcatcaggttctccttcgggttcgtacttggaatcgagctggtgataccgggtgttgcgcgtctcgaacttgcgcccgccgtccgccacatacagcaccgtcgaggtgtgcacgatgtcgcagtcgccgaggttcggatgcgcaagcacgccgccgagcgtggcacggaagccaacgacgggcgggatgatagcgcgccggtagcgcacgatgggtttgctcattgcagcttctccttgatgtagtcggtcgtgtaatacttcgggtcacgtggtgacgtgatgttcctgtagtccagaccaaacgcacgtagacgcgcagcgattactcgcgcactgtcttggccgggattgctaccgttgcttctacctctgtcgtcatcgagccacgtcgctacacgttggcctcgatcagtcagctgcttcaacactttgttgtgcagcttggtgccgagcaacgaccacgcttcggttaccagtcccaccttgtatgcactgagcgggtcttcgcacagtacgatggtgtcacctgtgcccacgccgtagcgtgcgacaagtccgtctttcggaacgtcaggtgttagccacttcggctgtctcgttgccgaccgggctgtccagtataccacgttgtcgccttcagtgatcggtagtaccacccgcccgatgcttgggcaccagtacagccgcagcttctcgatcatctgaagcgagagtcccatcttgaagaaccacaccttagcgtcgagcggccactcgcgggtgtcgtatacccgtggctctggcaactcaacagtcgcacgcactctgcgttcgctcgtctgctcggcgtggattcgtgcaagcttggcctcgatactctcgtgctcacgcttgaatcctgtgccaccgcacctgaaacagaatgcggtggacttgtcgtgctctcgtgagataagcaagggcgtaccctccccgcactcatgggccacacgtgtgcggccaccaacaggcaggcgctcggcatgtggtagccagtcgttgtcgggaagggtatcgctcatgctatcctcgcttggttattcccagacctcgaagatgtcgtggctggtggcgtacaggacggagccgttgccgtccgtgctgacgatcagacgggagccgtcttcactggtcagcttggacacgacgaacccggtgcccttcggcagcttgttggtctgccgcgtgtcgatcaggtacgcattctggccgggcttcagctcgtcgccacgcttgacgacggccacgctgggtgacggcggggcgaggctcacgactgcccgccttcgccacccgcagccttggcggcagcggcttcggcggcgaggcgctgggcctcggcaacggcggcgtcgatttcttcctgcgccttcagcacttcctcggccgacatcagcagggcgctgctgtcgatcaggttcagctcggcatccagaccttcgccggtctgcaccttcagttgcagcacgcccttgtcgttcttgccggtggcgacgatcacgccggacaggacgcgcttgttcagggcacgaccgaacaggtaggacacggcgtcgcccgccttcagcgcttcgatggcggcgctgttggcctcgacggcatccagcttggcgagcttctcgttcaggccatcgaccttggcctgcgccttggcgatgtcttccagcagctcggcgcgcttggcttcgtagtggctgacggtggtctgctcggtggtgttttcgttcgacatgtagatggttcctcttgacggttgataggatggcccgtacgtgggccagtcgtagcctacccggctcgggttactgaaagatcagctcgctgttgtacccaccgccgccattgtagaagcggcgacgcagcacgctctcctcacccagcaccagcagacggtccacgatggcgcggatggcgctcatgtactggtccaccagctcgctgtgcaagttcaggtcgaagcggatcacggtcaccgcctcgtcgtccagtgcgccggtgtccttgcggacgtacaggccacggccattggtcatggtcgcaccgccgatcagcttcacggcggcggcaatctccggctgcacgttgagcagtcggctgtcgggcacagtcacctcgacccagcttcccatgcgcaggctcatgctgcacctgccagtgcggactgcacgttgggctgcaacgatgcaccggaacgcagctcggcagcacgacgcttcatgcgggagcgcagcttgcgacgctgcttgttgttcccgccgaggctatcggccacgcgcttcagctggttgttgccgacgatgcgggtctgaccctgccccttctgcacggggaagtagtcctgccccagcatcttgcgcaggatcgggttgtcgatgggaatcagcggcacgctgacgtgcaggtgccggctggtgtccggcgcaggcggcggcgtgtcgtcgtcatcgtggcgcggcttcaccgctgcgaccaccttgtccttgacgtacttggccgcagccttgatcttgtccatgaaacccatggttacttcctcctcgttccgaagtgattgaactccaactcatgccacacgtagtacgtggtgccgagcgggtcagtgtctgccttccagttgcgctggtcgcagtagtcgttggctgcgccgaggtcatcgaacgtcagcgagaacccagtggaagccgggccggtgcggaaccggcacagcttgccgtcgtcgtcatggtactggccgacgacaacccacgggccacgacccacgatccagtacagcaggatcaggatgcgcagccagagcttacgcatagtacggctcgacacggtagcccatgttctcgccgcccagcgactcggcattgaacacggcgcgcgctgcatcgcgggtcgggaacagcacgttgtactcgctcttgttgtactcgttgccgtcgatgcgcacggtggcgctcgggtgctggttgtagcagctgacatcggagtcgctgcggtcttcggcgaaggcgtaggtgatacgccaacccagcggcttgcgcaccggcttgcggatgctctcgcccacttcgaggatgtgccagttgaagaacgacccgccgtagctgttgagcacatccgcctcggcacgcacggcggcgcggcggtcgaagatggcgagctggttcgggtacgtgccgtcacgcagcgagtccagcaggctggtggtggcacccttggtgcgcagctcggcgatcaccgcatccagttcctcttgggtcggggtgcggccggtgccattggcgacgacgccagtgatgacgccatcgttgctgttcttggggatcgagacgatgaagtataccttacgcatggtggttctcctgattgacgggtgggatttcgatttcctctatcgagtagagggtgggcaccttctcgtggtgcttgcggtggtgttcgatggcttgctcgcacgcctcgtggctggtgtgatgtccgccgaggatgtaatccccgacagccacacccttcacggtaacgagcggcagcgccttcaccacaaggcgcaggctgacctcacgcataccagcgctccacgctgtgctcatgggtcacgaactctttccactggcgcggctgctcgcacagctggatcggcttgcgctccccactacggatgcgcttgtaagttacggggatcatgcaatgtgccctcctgttgggcgtggttccaaagctacgccctcgttagaaggcgcagcggtagatcacgcgcggctcgggtgccacttcacgcggtagcggcggagacggttcggatcgttgccgacgtgcgaggcgatggcgttgcgtgcagcctgcgcagtggtgaacgtgccgctgagtccgatcacagtggacgtattccaacccagctggtgagggcgccgcgcatgcttggtgaagaactcggcggtgtagaagccgcgatccttctccgggccatcgggagtgccttcgggcaccacacggtacgcatcctcgctgatgccctgcaccttggcccgcgccttcagcatgcggtacgcagcattgcggctgcgctgcggcaggcccagctcacgcacctgcgcccagttggcgagggcgatgctgccgtggcgcagattgaactgcacgatccagcccttggtcttcgtcttgttgaccagcccggtctgcgatgcagtcagggcgacgtggcgtgcgctctggtcgtccatcaggacatccggcagcttacgcggcaggttgtcgggcattgccaggccgggcaacaccatgcggccggtcacgctgccgaggaagtccagctgcgaggcatccaacaccaccggaggcaacggagacagcaggcacgccatcacccgcgcctcgatagcagcgaagtcaagttcacgcatgccgtagcccacggtgaacgtcggcggtgcgatcaggtcgcgcagcagctgtgcctcgacatcgctgtcacggcaggccgcaatcacgtcgtcctcgaattgcaggatggcgtcacgctcgaagctctcgacaccgaagtcgcgcagctcaccgtgcagcacggcgaactcattggacagcttgcggttggagtacgggtctgcctttgcggtcagtgcacaggcgatgtgaagggccgagcgcagcagggatgcttcgcgctgggtcactcgaaggttgatcttgggttccatgttacacgttctccttcttcttggtgggcttcggcacagcgcgggcagcgttgatgacggcctgttcctcctcggtcggcacgtagccttcctcggtcgccttttccagacggcccagcagcttgtgcaggtcggcggcgaacgagaacgcctctgcgggcttctcggtcttgaagtcgtaccacgccttcgcggcggcacgttccagcacgtcggccagagcttcgccctcgactcgcttgctcttggcaaacttcatgggcgcgctcgccttggtttccttgtcgtcgttcggagccatcgggccgaactcggacaggtacaggcgcagggcttcatgcttcatgccgttgcccacggcgagacacagatcggaagcgagcgtaacgtcgccgtggatgtgtgcgtggttgatgaccgcaatcgcggcctgctgaatctggtccaccagcttggtgcgggcggtgttgatcgacttgatggcgcgcttgatgtcagcgcttccggtgatgatgtccatggtggttcccttcaggttgggtccgtgccgattgcacgacactaggccctcttgcgaaggcccagtagcttgcatttaagcgagtcggatgtcgaatgaacgcccaccgcacggcaggacgtagagcgccgacacagagccggccggatgcttcatgatggcccgattgtaggaatcgcgggcagcttccacgtagtggcgagagaacttgaaccggatcacaggtaagccctcctgtcagcggcgtggttcgcccggttcgtcccgctgttaccctcgacaacaaacacagatcgctttccggcggttccgtggcgggcttcgtagcgctcggcttggcgcttgcgctcggcaagcttgcggtcatgctccgtggtgcgcaggtccatcacgcttgccgtccgggtgaactggcagaagcggcgcttacgctgggtgcggtcgagattggcattgatcgagccttgcatgttgtgcctccattggcactggtgggaaaactaacagattgatgcgccctcagaaagccgtcgagtcggtcaatccctcattctcgattagagccgttgcatcgcctatcgtgggcgcacactgaccaccggatttgcctgcatggtcatcgcaaagggagggcgcatcaatctgctagcccttcgggctgtcaaccctactccggctagcagtgccattgtcaccgtgtggcccgtagagccttttcacgaaacgcacagtattccatgcgataggaggctcaccacctccttatgaccggcttcccaccttggcagtgggttacttcccgtggccgactctcacggcagatgggaagccctaagcgttaggcttaggtaaagcggcaccagtgttgcaagtctggtggattctatgggcctttgaaatcccagttcatccggttatccgctagtgctacgttgcagcttggcggtccacgtcaactctcggccactattggctgtggttggcacgcttcccgttacaccctacccgttagcggtagtcctacgccatccaatgtggctgctcctcagagcgtggtgccatactagcacccttgttgcatcctgtcaagcccttggctcgctcgggtctctaacccgttgggcgtcctgtcgccaccatcccaccatgtacgtcggtggtccacgtgttgcaaggcctcaaagggctatctgtgccgccttgtcaagctatccgttagaggaccatgtgcgctcctgttagtgtcttgaccggtgtcccggtctcacctcagcctcaacacccgtaatctctcacgtctagccttaccgctaggtcgctccgctgttccggtggctaccacttgccgcctatcatagctaactgctagcttagtgtcaagcgtggttcggtagctcctcgcatcccttaccagtgactcccgtgtacccttagcccacttgttggcggcgccactacggatcacgtcactcgacttgcgttgcagcttactaccattgcggccgtgtgtctactactgcttgcatcgcaagcgtcaaccgttggcctagcgggtagctaactaatcagctcgacagagtaccgatagacggtgattcaggttgagccgactgtgtgctataggtgtaccaaaaggccgaaacgatacagatggccctcgcacgcctacagctgcggttcgcatggtagcaggtagggtagcccctgtcaagccccttgcggccctcctgaagccctgtcgctgccccagtgacgccattgaaccacaccgcaccggccacgtcaacacctttcgccaagagatttattaacgattcagccaaggcagcgcggtccagccatacaggcagcaggcgcacgcccacccgcacgcccacccgcaggcacccacgcacggccacgcacacgcacgctcaggcccacgcaggcaggcacacgggtacacccacgcggaaccttgacgcgggcgcacagacgcgcacacaggcgcacacgcgggcacgcacccacgcacacccgcaggcgcgtaacgcgagggcgtacgggggcacgcgcgggagcttctattggagtgacccccgcgcatttccgaagcaaattttggtccggctacccacgtggccttactcctaagcctcgcgaactggtgcctttagcttgacgataggcccggagctgtagacatcgtgagctatcgcagcagccatggccttagccacagacttgctcgcatgataggcccctagagctagcgccttgccactgccatcgaagtacggagcctcctcgacccactgctgcttaccagtagtgaccgtgagtacgccgtccttaaccacaagcaccgtcgcggacttgccaacgtgctcctcgtagccttcgcccgctttaagcgcagcgagaaccgggcgaagcactgtgaaatccccggtgacacccagcagcacagggccggtgggtgtcgatacgggcatgatcttacgcacggtgtgcttgtggtcgccctgcgtggcctgactatcggcccacaggtgcttgccgtcccatgcgatggtggtcatttgtcacccgtacaccggcgcttaccggtaccgcacacctcggccttccacgcacgcagcgcagccttgtccttgttgcacagaacggtgtccatgcggcggtcctgcgcgagcttgaccaccttgtcctgcgaggaggtggtgcccttctccccaccgaggtaggtgatgtggcagtctgcaagcagggagtcgtcagggaccggcaggttcgcgcaggaggtcagcgacatcagcaggaacagtgccatcccggtactccggggcagcgtcaagaacttcttcagtgcgaacacgcacgtcctccttctctttgatgtaggtcgcgtacccggtagcctgcgtctgcgccgccttggcggtagcggtcgtgccgacttgggcagtttccagcttctccaccttgcgttgcaggccgtagacgtacagaccgaagcacacgaacatggtcacgaccagcagcaagccaaccagcttgccgccgagccgcgcgatcacttcacttggggtttccacggttggatcacctcgttgttggggcgcaagcacagagcaaactctgcgtcgcggcgcttggggatgccggagcaacggctgctggacagtcggcagtcgagcttaccgacgtagacccagcgcaggaactccttgcagctaccttcacgatcccctgcgttcgctttgcgcagcatggtgctgtcggcgaacgccttctcacctacgttgaacacgaagtctgtgtaggcgtcgatctggttgcggttaacgggggccttcaggtgcttgcgcacgccctgctgggcgatctgtaggtcttcgatcagccacttgtcgcactgtgccttcgttgccgtcatgcccatcgctacgcccttggtgtggccgtagcagatggtcggcacccggccggtgtcgaggtacgcagcgtagcgtaccccttcgtggccttgggtgaatgacagcagcgttgccgaaatgccgatgaagatgccgccgatcaggccgaacagccccttgttgctggtatcttggttctgctgctggttcatggttgctccttacggggtcagtgggtcgtcatccgggtccagatcgaccggagtgtgcgggccggagttcggacccgaggacgcggtgcgtgcgcccgcagcgatcagggcgtccagcacgagggtggcgtccttctggaactgcgcgagcagctgcgctgcggttgcgggatgctgctctgcgtgctccatgagggcgagcagttcgcggtgcaggtagttgccacggccgaacagacccgtgtagttgctggtgaagtcggacttctgcattggttacctccggtaacggtcgagtagggatggacggccacgttgcagcggactcttgcgggtcgctgccttcatgccggtcggatcgttgatccagtcttggaactctcgctgctgctgcttggcgatggccttgttctggtccagtgcaagctgcgcaacccagtgacgcacgctaccttccagtgcatcgagccggtcatcgtgtgcgatgctgcccttctgctgcgtgatcttcgccatctggtggaacaggctgtagacctgacgcttgccgctggtggcgtagcgctgggtgtactcgtgatccatttcaaccacggattccagcatgaccagcgagccgcgagccatgacaggttcgagagtgccgatgatacgggcttccttgttgccggtcacgaactcctcgcggatgtcgcccttgtatcccttctccgtgccgcgatcttctcgcaggacaggcaggaacaccttggcgaacgcgccgtagcccatgttcttttcgatgctgatgacgttcggcttgtacttcaccgcaatgcggcgcagttctagcaagccatcaccgtcgtagccaccgggcacagctcccacggccaacacgtacacggtggagttgaggaaggcggtcacggcgaaggccgtctcgtctccgttggcaccaccaccggccgggtcgatctgcatgtgcacgccctgcacgggggcagtctcggtgctcatgtcgtgcggcatcatcatcacgaagccgtacccactggactggaagctgcgctggtgagcgttgctcaggccacgggtgatcgtcagcgggaagcggtcgccaccaccggggatcacgatcaggttctcggtcttcagcgggaagcgcatcgcatccatcagccgcgtgttgagcatgtagttcagctgatagctggacggtccacgctgacgcagctcggactggtgcttctgctcaccggccaacagctcgtcggtgcactggccctcgtcgcccatcgggccaccaccgaacgccaacatcgggtcggcttctaggcgctgcacgatagacggtgccagatgcgggccgtagtgctcgcgctgtgccggggtcgggtagcgaccgggccagatgcgaacgtcgtagccacgtccgggcagggtgttgtagatggagtcgccggtctgcggcgtgccgaggtacaggatgcgacccggagtaccgggcttgccggtgcagatggccgagaactccaacgtgatggtcagcagcagctcacggttcgcggcagtgcggctgttcttgttggactccacgtcgtcggcgatcagcaggtccgcacgcttacccggcaggttgccggtgacgccgatgcacgccacgctcggggacttgtcgattcccttcagcgagtggtgcacgtcgaacgcatccacggaggtacggtcgcccgcgttcttgtccgggcggatgcactccaacgtcggcaccgtgaggatgatgcgctgaatcagcgtagcaatctcggatgcctgcgtgccgcctgccgatacgatcagcacacggtgagtgggatcgtggatcaggcagaagacggcgtagatggcagcgatggtggacttcgcctcgcctcgctgcgcctgcaccattgcgaggtgcgggccatactgcatgtagttggcgatgtcgtactgcatccacgtcggctcgaaccccagcaccttcataatgtcgcgcatgaaggtggcgaagtgccggtagtggttctgcaacagctccaacttcttgcggcgcacgtcggccgcttcagctgattcacgcattgttggctacgctccccggaaagtgaacgatgttgtcgagtgcacgctgcaactcgtcgtcgtcagccggaggcagcgagtgcttgcccagctcgtcttccagctcgccgagtgccttgttggcctcgcgcgtcgccgtgatgttgttgtccttcaggaacttgatcgccgcattgatgtcggctgcggtgcacagctcgccatcttggatgcgctgcatcagcgcacgcgcgaccagttcgtgcagcgcaccgagtgcgccctcacttgccggattcgacatccttgcctcccatgatctttcggtgctcgcgtgcccgccagtagaactgagcgacggcgtacagaatggcgagcgtagttacgatggcagcaccgtacgtgctgatgaagttgaggtagaccgcgccgagcgtaagcggcgaggttcggacgacctcattgaccacactcggcggggtcatgctgttctcctgtaggttagggccagtcgtcgggattgccgacgagcttccattgcaggcggttgacgttgttcatgcccaccgcaatcaggtcgccggggattcccgaggcgatcacatgttcggttgcgaagcgctcacgctgcgcgcgtacgcacaggttgctgccgttcttgtacgacaggagcacgtcgctctgcgtggcgaagacagcccgcttctcgtccatgcacaggcgcggagtggtagcaccggggatcaccatggtctgcatcgaagcagccaccgtgtcgtaccagtagaacttgcacacaccgcccgccatgtacgccacgtgcgggcgcatggtctggtcgaaggccagtgcgatctgcgtgatcccggagtcggtcagcacggtgaccggggcaacgccgtcgcggtaaacgacgacgctgctgccgtcactctcggcagtccacagcgcagcttggaggtcgtccactgctgcgttgagagtcagcccgccctgctcgaagtcaatgagcgggcgggtgcgccgattctgctgctccacccagtcaccgcgttggatgctttgggagacagtggggatcatggcgtgtaccggctccaagaaacccgcatgcgcaagttcgccgtctccgatccggtcttggtgatacccggattgaagccgacttggaaggtcacgcacgcggagagtcccattgcagccgtgatcggaccaccgggcacgttgttgatcgacatccggcaaacgcagtcacggtagtaagtacccggaacataggctacctgctgaagctgcaagtcagagaagctggcaatcgtccccggcggatactggtcggtgatagctccggtgccgtcgccagtaccgccgtagaagtagtagcacccccacacgtagtccgaccaagcgactgccgactgaccgttcataccgccgctgcggcccattgcaataggcttacaggtaacagtggtgctaacacccttgatcgtctcagtagtgacaaccggcgtggtatctgcgtacatgcgcagctcgtaagtaaccacgaggatttcatccgacagcaccgtgatggtggtcgggttacctgcggagtccttgataagcgcacgggtggtcaggatgtacgcgccggtattgttgttgtatgctttggcaccaagctccgacagaacgccagtagcggtaccagccgggaactggtactggcagcgggagtaggcgtagtacggggcagtggtagtcccaccgctgtccgaggacgtacgaccaacctgcgccacctgtgcaccaagagcggtatcggtgaatgccggggtggcgctgccactaccgactgccaagtaagcaatgaggtcgtacatgctgcgaggatagccgctgccggtatcacccagtgcgtccataccaccgtccgtgataaggttgctctgccagtcggctacaacttcgagagtatcgagggacttacccttgctgatggtgaacacgccagcaatgccgaggtgattgtggatcatgcgaagctccatgatacgaagccagaccggagtcgtgcagtcgcgtcgagcggctggttgactacagggtgctgcttcagggtgaaggaatggaaagaactcgacagcttcgccgtctccgggtcaggcgtgtagtccttacggatggatcggatgtcgaacgaaacgaaagcgctcccgtacaacgtgctctccgggtcggcggcataatcctgcctagagcttcggagttcccagcttacgaaggaggaacccagcgacgcagtatccaaaggctggagcatgtcgatgttgctgtacccagcaaagctgctggtcagcatcgcggcatcgaactggtagaagctgtagagcttggacgtaacgtagatgccctgctcctcgatacgaccggaccagtaggccacacggttcaacccgtccgtgaccttgatgctaaggaagtaggagctgtcgtcgttctgacccagtacgtacttgtggttccacttaacggtgtccacccacagcggtttgttctgcttgctgcggaacgccgacagtacaacctgcacgtacttcgtgtccttgggcgcagcgccttcggcaacggactggtgccacgcaccgttgctgccggaggaaaccatgttgccccagttgcgttgcagctcggtcccatcctccttgcggtagatgatcgacacacgagcaccggccttgcccttggagcttgcgccctgctggacctcggcggtgcatcggatgtagtcgttgaccttggcagggatcagcgggttgagcaggtcgctgccgcccgtcttgatgttggcgaagcgcgcgctgtacacgccgctgtcggtgtcgtagtctgagccagtgccaatcgaccagccttcgccattcgatccaccgcccggcaaccacgtgccgtcgtcgcctgcctcgaagtcgccgttgggcacgagggtttcctcgtccacgacttcagtgaaagccgcccacttgacgacgacttccttggtgatgttgtccacccgtaccgcagcgcccgaagggagcgtcgattcgatgacctccacggtgcagcggccgactgggttgttgatggacaggcgagactcgtaagcctcgcccgccgtgtacccttccagcacgcccgtcaccgacaggccatctgcaacctcgtccgccatgagcggtcggccgtacagcctgaagtgattagccatgcttactccttagccaagtcgcccgagagcaaccacgtgttggtgtcgccgtcgatgcacgttgcagtgatgacggagttggtgccgcgagttgcggcggtgcagccgaccgggacttcgagcgtcacgcccacgtcgccagtgatgaccacagggcctgccttctgctgcacgctgaagtagctgcccgaggcgagcttggtttcaccgtcgcccacttcggggatcaggttgatgttgacggcgcaacctccggcgtacgtgcagcgcacgagtccgtactcggtagccttggcggcgtagtaagtcggaccctctgccgtgatgatcggcacccgcaggctcgcagcggtgatcggcgcaggcccggtgtagggcttggcgtaaccacgcagcacggcgaaccagatgctgccctcggcaggaaccgtggcgaagcggatgaagctgggatcggtgccgtcagcgagcgtgacctgatagtccacgtccggctgcatgccgatgccgttgacgtacacgtcgtagaagcccgcgccggatacgtccgcgcccaccatgtcgaagtcggtgtcacccacctgatcgccagtccaagcaccggaccagacgcgcggggcgacggacacgataccaccagctgccagcaactcggtgacctgcttgtagatgttctggataatctcgttcaggtccacgatcacaccgacctgctggtcgatgctaagggtggcgatgttgagtgagtcgaacatttcctgaatgatcttcaggagctggtcgttgctgaggttaaggtttgtcttgctgatgatgctaccgttaacgtagtcaacgagcatctgctgcaccggagtgctgcggtagatgtagagcttgcgcccagcggcgacggcaggcgagactcggacggtactagcgtcatcgtcttcgctcaggacttccacggtgtgcggagtccggtcggtcagcagctgagtctcctcgtccagcagtccgctcatggcgtacacgtgggacgggttgatgtagccaccggtaaagctgatctgccagtcagtggtcacgccatcggcgtcgaacacgtctgtcgcgtagcgcagctgcgggtctggaactgccatgctgcctcctgtttgctataggtgtaccaaaagggtgggccgtccttggccctgatcttactcctccttccactggctggctgcgcccttcagcagcgggatcaccatcggcagtcgcccgcccggaatcacgtcggccagattctccggcttgccagcaatgccctgagcgaagtcgttgatgactcccagcgacggcgcgaactgcccgcccaccacttccttgcggttgccgaactgcccaccggccagctgcttcagccacgtcggaccctgcgtatcggtggcgtactcgtaccagccgcccgccacgccagtgcccacgtccagcacatcgttgagcatacccgtcgccgacacgtagttcagcgtggccttgcccagcgccagaggcgacaggatgttctggtcgatggcctcgtcgcgctcctgatcgttcatcagggccacgcgggacagcacccgcagggcttgcagcggagccgccacagccatcgcagcagcgatcaggcccgccgtctgccatgcaccgtagttgcccacgtaccggcccagctgcttctgctgcgcgaccagcgagaacgtgcggtgctggaacagcagcttcagccagccgttgtgcgcccacttgccagtctcgccgatgaaggtgtcctgaagaatctgcgaggtgccacggttgatcgcgttgtagaacgccaaccatgcctgccgatccgccagcccctcgacgttgcgcgggtctactgcttccagcttaccatccgcgccccagcgcacgacctgatcctgcgtagcccgcaggcggttcagcaggttgtcgtcaatgcccatgtccttcagggcggtgtcagcttcagcaccatcacgcaggaacttcacgcccttggcgatcagcacttccgcgaagccacgctgctgcacagcaagcacggcccgctgccccgagaggatgcggttcgcatgcgctgccttctgcaccagcgaggtcaggaagcctgcgcgctcgctaccatacatcgacgcctgcgtgtccagcgagttgaacatgtgtaggtcgtaaccggcgagaccgaagccgcgaccgctgatgaactcgaagccgtcgaggatttggttgccgctgtcctcgcccttcaggatgcgcatgatttcgctgcgcatgcggggagcgatacggattgcgtcagccacaccagcagcaccaacagcggcgaggccgttgctgtactccgctgcctgattgatgcccgcgccgcccagctggatggccgaggtcagcagacgcgcattcgccagaacagtcggatcgccggtaccgaccgggcgaccaaggaactcggacatcacctgctcgaacgccttcagctccacatcgttggcaccggtcaggcgcattgcttcgcgcgccacgttgatgcctgcgtcgccgaggatgccgtgcttcgccagagcgatgtcaccagcaacacgtcccgcgtacttgcggtagttgtccatcacgcggttgtcgagatagtccatcagacggaacttaccgtcagcgtcctcgtactgcttggtcacgtcgaggtcgatacgcgccttggtgtgcttcgcaccgccacggctgtacttgcccatgaccttctgaatctcctcctcgttgagcgacatcgcccgcagagtgtcgcgcagcgtgtccgcctgcgactccgagaagacctgacccggcgcttcgatgacacccgcagccttgcgctcgatgcgttccagatacttggtagcgaacttatcgaggaagtcgtccccatacagctcgcccatcacctcgaactgatcgcgcatcgcctgacggataccctcgcgtcgcaccggaccagcagcagcgatgctgccgcccagccacgtacgggactcgtagccctccacgtcctcctccggcagacgctgtgcgcccaccgtaccggccgcgcgctgctctgctgccatgcggttgtagccacggtccaactcacgggccattgccttcactgcctcgtgcgcatccgggatgtccccgccgttgaagcgagtctcgcggtacagcttcactgcgtactcgaagtccgcgcgagccttccagcccgtggcgaagtccttgatcgcaccgataccgcgcacgtccgcacgccacaggcgataggccgcttcccactgacgcgggcgggtgcccatgaacgactcaaaccgaccatgccgatccatcgctgcggtgctgtgtcggcctgctgcaccctcgggattctccaacagggtgatcgcaagcatgcgggcaactggcgacttggacgacattagagtcgtgctcgtagcttccagcccgaagcgctgcatgatggtggacagcttcgccgcgtcgatgccgtactgcgcactgaagcgttcggagcgtgccatcacttcggcgacctgcacacgcatcgcgtcatcactgacggacttgtccagaccggtgcgctggtagaaagccttgcgctcgcggttcgacttgaagatcgagttggcgagcatgccacgcgtctgccgggtaccggcctgcgtgtcgcgcacttccgcgccgaggttgtcaccgacgaccgacatcaggcgttcgagcgcggactcctgattcttcagacccatcactcgcgcgatcttatccttcagccactcccacgcattcgggcgggtgttgcccggcgcgggcatctgacgcagcaccgcctgcacagcgcggttcgtcaggccgtaggaaatcagctcgtcagtgttggcgaggaagcctgcctgcggctggttgatgcgcgtctccatcgcagcggtggtcagcgtggagtccacactgccgatgctgttgttgatatgggtcagcagttcttccatttcctgcccgaacaccgagttgctgcgcagctcacgcagcgtggcagcgtgcagcatttcgtgcaccaccacttccggcgtgtagttccgcatcgccatcgcgtccagtccggcgttgtagccaccggccacacgcatacccggacccatgttggcaccggcgaaccacttgtcgagttccgattccggcacgatcttcaccgtgctcagccgcccgccacgcttcagcgcgttggcgatagcacgcacgtcctccgggatagaggcgttggattccagatacttcagcacgccatcgacgttaccgcccttgatacctgcggtcttccatgcgcgttccagcagcgggtcatgctgatcgacccggccacccacgctgtcgttgtaccgcccggtcgttgcgtccacgttgcccgcgtcccgtgcgagtgcaccagtggtgcctgcggtggtggtcgtctcctgcacgtcgggacgggcgaagatacggaagtcgtcaggcacgtcggccataccagcgcgcagccaatccacagcctcctgcttggcaagctggtggatgcggttgttcaccagcaccgggttggcgtcctcgcccagctcggccacagcgcgcgccttcaggtcggccgaccacgcttcgccgtaagcggcagcgttgcctgcggacaggtcgatggttgccttgtcacgaatctgcgcagccgagcgcacgcccggaatgtgcatcgcggtgcctatggtggtagcgaatgcagcgtcggtcatgaagtccgcgaagttgcggcgctcgcccatgccaaccagcgcggcgtccgtgatgacggaaccgaccgcgttctccgcagcagccgacgcgagcgacgcgcccacgcgcccttcggcaacgagtgcagccgagccgatgcccagcgccttagcgcctgcggcagtgacgccgccgatagcccagttgcccggatcggtgaagcctgccaccatgtcgtaaccgaagctaccccagccagtctgctgatccttgatgcgcatggagtggcggcgcaggaactgtcggtcgctgacgtacttcagctcgttcggcgagtacgctgcatcgcggatgtcttcgagttcgtcggcagtcatccacggcttctcccattccttcgggtcgtacttccaaccttccggaacgttctcgtcctcgcgcgcaaactggttgctgatcgcagcaccgatgccgctgtcgaacgcagcgccccacttgtcgaggaaggtcagcgagttgcgcagctcctcgtccgcgcggtcctgcgcgagcgcctgttcggtctgatccagcagcgccttgcgagcgccggtgttcagcacgtccacttcctgacgcacccaccacggcacaacctgatccgatgcacggacagcctgagccttgcctacggcctgcgcggcggtgccaccttcctgtgctacctgacccatcgacagctcggcgatgcccgcacgaatcttgccgatgtgttccttcgctgccgacgccagagcgttgcggccttcgatgggcgcacccgtccacgcatccgggatggacgcaccggaccacgtacggtcgcgcatgttcgggttgccctgccatgcggcgttgaggtctgcctgcgtggtggtcaggctgcgcggctgcgccgacactgcgggagcggacgcaccgcccagcacgctcggtgcataggctgcgttctcctgcccccagttcttcggattggtgccgccttggtagatgcgcagcgccttcgtcacgtcgcccttggcaagctgcatgttctcgcgcatgatgtcggcatacagctcgatgctgtcttggaagttgcgcatgtcgtacttgcgaccgttgcgcgcttcccacgttgcctgcgtggtgggcatgacttggaagtcgccctgtgctcctgccttgctgcggatcacaccgtcagcgtccttggcggcacgcccgttgccggactctactcgccactgaccgcgcacgatggactccggcactcccgcataagcggcagccttggcaatctgctggtcttgggtcagccccgaaagatcgagtgccattgtctatctccttacagtttgggttggatggaaatgctctgctgaatcgtaccgtcgttcatgcgaacgtagccctgcggtaccggggcctgcaactgacgctgctgcttggtgtgcttctcgtactcgtccttgatgtcgcgcccgtacaccggcacaaccttccagcccttctcgccaacagcgttgacgtacagcaccggctcgccgttctcgctgtccttcatgcggaacacgtcagccttcagcccggtgctcggctcgatgttgacccggcgcagtgctgcgtcgatggccttctcgatggcgggtccggtttccttcgtgtccatgaagcccagccatgcaccgacgctgccgatcactcggccttcgtcgtcgcgtccgttttcccatgcgtacttgcctgcgtcttccagaccgtaggccagcttggcgtgagtagccgcagcctgcaagccttccgcagaagtgtccagcagaccaccggtgtcagtgaccgagcggacgatggcgcgagcatacgcagcgcggccagagtcgcccagcttgttgccgaacatgccgaggtacttggggttgagcttggcgatagcttccgtaacacgagcctgagtagcctcggattccttacggctgttcgcgtcgaactgcgtcggatcgtcggtggtgatttctccacgggccacctcgtaagcaagctcgaagttcacgccaccattctccaacgcttgcagcttgttgaagaacgtgttgacgctatctccgaagtacagcgcagcggtagtcgcgccagtcagtcggccctgcacgggctgaccgttcgtgtcgatgcgtgcggcggtggtctgcttcagttccttccactgctggtacagtgcagccgctgccgtgttcggctgatcgcggagcacagcgcgcgccgtggtctggaactggtcggccacacccttcagcacagcgcctcgcccggtgttggcgttccacaccagctgcgacatggcgaccttggggttcgcggccatcgtggcattccatgcctgcaccgtgttcgcctcgatcagctccttgtccacgccggggatgttgatcgtctgcgcgtacgtgccgcgcttgaacgcttcgatgccaccacggatgtcctcctcctgcgcggccagcttctgctggtcggtcagcgcggccttggccgcagcgttacgctggttgatgacggcttcctgtgcgcggatgtgcgcgcctgcggactgtgccatgatcgaagccaactgcgtaccggagtacagcggtgcgtcgcttccagtctcggcggcgtaggtcgagttcatttcctcgatcatcgcctgcgacggcttggcaccaatgccctccgatgcgtacatggagacgagcgccatcttctcggcctgctccgggttggcatcgagccagtcggaacggtaacgatcctgcgcctgcttcacgtactgctggattcccagctgcccgtccgggtcgatggcgttcagaacgcccttgctgttgaggaacttcagcgtgtggaactcgccgcgatccgcagcgccacgatagaacgcagtgatcgcggacttgtacgactcgtccgtctggtagcgcgagggcgacagtccgtccagcagggacagctgcgcctgcgtcagcgcctcggtggccttctcgtccatgggacggttggtaccgagcatcgccgtgcgcttcgccagttcgttgaagccggtggacgccgacgagttcgcagcgtactgcgccttcaccagctcctgctgctgccatgccgtgcgctccttggtgtgcaggtccatgagggaacccgcgcgatccatgaaggtcttctgcaacaccgtgtccgcgaaaccgttgccggtcatgcgggcagtggcgaggtcgttgaactccttcgccatcgcctcgggaggaagctgacgcaactccggcatacgccgaagcaagtcgctctccatttcgttgacctgcgagagcgtgttatacatgctcgcgccaatctcgtagttggtgtctccgaagattttcttgtaccacggttcggtcgcagcaatctcgtccatggtcttaccagcgcgggcggcaacgaagccgtcccacatctgctgctgcttcagcttggcggtgttcggcgctgccagctcctgcaagaactctggcaggttgctgtccggcatcgtcataccaccagtgcttgcgaaccagtcgttgccggattgaaccggcccgacctgattcacaccagcgccttgaatgctggtgttgcccgacagtgctggggtggcgttgatgccaccctgcaatgcggactgcgtgttgaaggtaaccgtgccgatgtcagccattaccatgcacctcctgagttgcctccgctgccgctatcgaaccagccgaggccggacgtagtggtggagaagttgtcgtagttgttgccgaagttgccggtgaccttcgccccagtcacggactgcttgccggtgccgtcgttgtacccgaaggtagtggacgcccacgacttgccgccgcgatcattggactgctgccacgcctgcataccgttctgcgctgcgttgctgaaggactgagaggcaccagtgaagttgccgttgtccgcctgccacgtgccgaccgcgaagtctgccacggcctcgcctgccatcggcccaccgaagtaggtagccacggccacgccgatcagcttgcccaagcgacgcttcattgcctgcggctcgatgtgctgcgagtagtcgaactgcccgaacgaacggctcatgtccatcccgttccacgcgcgcgacatgatctgcgcagtctgcgatgcgccccgcgaggcgaggagcgagacagcgttggcctgcgtctcctgatccatttccgcctgcaaccgcaccatcgaatccatcaggtctgcggacgagccgccgacaccgacagcaccagcctgcgcctgaagtgcgccacgcgcgttcgccagttggagctgggagttaagcccagccccttggcgcgcacgcagctcctcggacagcgcttccatgttggagttgtactccttcgcggcggcgtccagttgggcgttgttcttcagggaccgcatgaaatcagcgaagccggtcttggcgacctcgctgcggttctggttgtcggtctgcgcaacggctgcacggtagttcgcacgggcaacgcgggtggtgttgttcgcttgcaggatcgtattaaccgaacccattagctaaccctccgtacattgttgaaagtctgacccgtccagctcaggccggtcacccggagcgggagccaatccttgctgcgaatctcgtaggtgcactcgcgcacttcgcgcccgacgctgatgttgagctgcccccggtacaccggttgccgcgcgatcagattgtcggagtcgccgaggatgcggccctcgaagtccgtagtggtcacattgctgttgcgggttgccaccgtggcgatcatgcctgccgtgttctccacgtccaccgtcaccttgttgagggacatgcgtccatcgagtacggcctgaccgttctggtcccgagggaacggattggtcgggatcaccagagcttcggacaccacgccgtattccagcgcaccagcagcgaggtcatcgaactggttaaggaagtcagacgcctgcgcgtagggacaacccagcaggaagtacgggctagtgctattgacggcgatgcttgcgctcgcagtctgtacgcccgtaggtgtaccaaaactcgcccagctgtcgaggcacgcatgcgagtccggctcgcccttcgggtcgaacacgtcgcacgccaccagcgacccgcgcgcagtgaacacgaggccgttcttcttgtagctgctcacgccgatgatttcgcccagcgccgggtggtaccggaacttcgaccacgcatccacgatgcgctgcccgttgttcttgttgtcctcgtaccggtacaggtagaagtcctgcgggtgctcgcgagtgcggaacatgacgaggttcggcgcagtgagcggggtgatctgcaacggagtgcccgacagccacgagtccagctcgttggacatttcgtccgtcaccgtctgctgcccgttgagcgcgcccactcgcatctggtgcaggctcgtgccttcgctgccgtactgcgcataaaagatgtagttgcccgaggtctgcgccttcgcgtcaaccgaatccttgttggcactgaacgctttaatcagcggattcttcggactgaacaccgagtcgccgctgatgccgtactgctgacggtcaccgaagatcacgaggttgccgttgtagagcgtcgcgtgccggagcacatcgccctcgctgccgtgcgcgaagatttcgatggggtcgctgtcttcgatggtgacggccgagccgcgccagaagttcaggtagtccgccgagcgtgaggcgttgacgtagttctgtgcgccgatgaccagccggtcttggaagacggacagcatcgtgatcggcttgtcgatgaaccacgggatcggcgaggtcagaccatcgcctgccactcgcgcaccgtaggccggatgctcgccgctgctcggagccagagacgtgaggcccgcaccgttgcgtgcgatgtagcctacaccgttgtagatgtagagctgcgacacgaggttgtcgatggtgcactccacgccgggcgcttcgtaccagtccaccgacccgtagccggaagtctcgccgttctccaactcagcgcgcaggtagtacgactcgtccgcgcctgcaccactcggccgcacgcgaatgaccttgccgtgccagtggaacttgacggcgtaggtcgcgtctgtaatttcctgccctgcggcgtagaaggtcgtgccgtctccctcgtcgtcaaccgtgatgtccttgaactggtcatcgtcaatgatgatcccgcccttgatgtacgttgccgacacgcctgcatcgaccagcaaatccgacagctgctccgcgatgtactccgggcgcgtctgctcagcgctcgtcacgatccactcgttgaccgcagagttgtactcgttcactcggtcgttgacgtacttctggtacgccgcgtccggctccgtgccaccgggaaggtagaacgggatgtcgctggtgtcgagcgttccggggtacgatgcggtaaccgtcttgaacgttaccgtcagcaccgtgttgtccgtccgcgtcaggttcaccgtgtacgtggtgttgtacttcccggtgcgcacccatgctgcgaggcgctggatgttcgtctgctcctgccacacgttcgtgctggtggccgaggggatcgtggtgttgcccgcgatgtagacgtagctgccgatggccgtgagcgacgatgcgcctccgctgaccagcgtgttgacccacgtgctgttctcgtacaccagagggatgaacgactcgtccgtcttgttgtagaggaacgcgaaggactcgctgcccaaggtcgaggcgtcgcgccggtacagcagcgcgtactccttgccctcctgcatgaagtcgaacacgtccatgttgcgcagctcggccgaggtgacaacggcttgggaagcagcgaaccgcgtaccacgacggcgcacgaggccgttcaccggatcggacagcacgttgatctgctcgtgcgtctgtcccggccgacgacgatgcgccggtttctgactgacaccctgaaggatgtcgggataggttccgcctgcctttgccatgttgtctccttagccggggaatgtgacgtggctgtgccacgggtgaccgctgtagttccagtaacgggaacgcagcacgtccacggatgcgcgagcgaacagcgggttcgccttgatctggcggatgtgctcggccttcaagttgatgtaactgtcatcgcgctgctgcttgatcttggcgtacttggtgttgtcgccgtcgaagtcagactggaaccgcagcaccgagtcgtcgcgcacgaacatctgcacctcgtaggggaggtcatcgaagtccagcagccgcaccagcttggcctgcacgttgtggtcgaactcgtaggtgttgcgcttgcggtcgtacagtcggcgtccgcgctgcaccacgtggccgaaccggctcgggttgcagtccagcttcagcacgtccgtggggaccatgatgtacttgctcgttgcctgcggcttcagctccacccattcggtgttgaaccacagcgagagtgaggacacgtcacggtgcacgcggtcgatcaagtcaacggcgtcgtccttgtatacgtggtcatcttccagcgtgttgagcttcgtctcgcccatcgtcttcaagcaggcgttcacgatgtcgagcttggtgatgaatgccatggtgtctcctgagaggaacaaggcagagacgccggagcgcccctgccgggatgttgcttagtccgcagccagagccagagcggccggtgcgtactcgatgtcctgcgagccgatttcgtcgtccacgaaacggacacggacgacccagcctgcggtgccacgggtgtcgtagtggacgccgacgacggtaccaacggagttggcgggcagaccggccacgccagttgcggcgacgacgcggttggaaatctcgaacggtcggtcaaagaccatgatgttgctcctgtgttggtggaagaagggcgcggtttgagttacccgaaggattcagggaccgcgcccagcggattaggcaaccttgtcgatgcggcccgcgttctcgacgcgatccagaccaacggcgaaggacatccacgagtccacgaagtagcacttcgaggcatcgctccaccacaccgaggactgcaacggcagcgcttcggcgatcagcagggccttcggcgacacggccacggcgatcagggtgctgaagtcgccgtcgtagaagtcgtcgttgtcgtcgttcgacagcaggtgaccttcgatcacggtgttcggcaggttctcgctcgacagcaccgggacgccccagccgtggaaggtcgggatgccggtcagcttgttgccgtccgaggtcaggtactcgccgttgctgatctgctcggcctgctgcaacaggtagaagatcgccgggcgcacgatcaggaccacgccatcgcgctgcggcttgaccttcttctcctcctccatgcgggagaacagtttgccgatggcggcgtacaccttggccggatcgttctcgtcaccagcggcggacagcacgacctgcgtggcaccgaagtggccctcgggcgcgcggccgttgcgggtgaagatcgactgcgtggcagcagcggccttcgcggcggcgatgctgatggtcaggtccacgaactcggcgatttcctgaccctgctcgatggcgatttccttgcgggtgtcgatgtcggtgaagatttcgtccagctgccagatgctgtgacgcgacagcagcatggtatcgacggtcaccgacgccttgctgaagtccaccggggtgccgtccggcgcgtcaccgcgcttcagcttctgaagcttggtacggccgatggccttcttggtcagggtgttggtgcccttgacctgcttgcgcgggaagaacttttccagcaccgagctggacacgtaggtgtgctcgacatcgccggtgaactgttcgaggatcagggcgttctcgttgccggactggttgacctgattcggcagaaccgggacagtcgggaagatggtgctcatgctttgtgttgctccttggtcttagtggatgacgcgcgcgttgagtgcacgcagttcttcggagtgggccgcaccacggatgcccttctcggcaaccagcttgcggtactcagcgcggtactgctccttcgtgataggagcgacgccgttgatcgacgcggcgggggcggcggcgttggtagccggtgcgcccttgacggtcgtcgcgggattggcctgtgccagagccatcaggtaacgcgcggtcgcctgagcgccgaagccaccagccgacagcgattcgcttgcctgcttcagttggtcggcgggcaggttggcccgtgcgaactgctggatcgcagcccagttctctgcgccacccacggcttcgtggacagcagcaacgttcgcggcgtgcgctgcggttgcagcggcggtgacacgagcgatgctctccttcgccagagcgaggatcggtgcggaacccttggccttgtcgccgaggacttccagcttggcttccagcagggcgaagttgcccttcgctgcttcggtcagttcgcggctgtcgatgtcgaggcccacggtgttgacgaagtattcggccgcgatgttcaggccgttgtcgccgtagtccgggatcgacaccgcagtcggcgcagcgttcgccggggcggcgggctgtgcgggagcggcaggttcgagactcagcgcgtcagcagccggaggtgcagcaggagctgcgggctgtgccggtgcggccggagcgggctggccgttgggcaacagcttgtcgtctgcgggagccggagctgccggtgcgggctggttgccgttcgaggttgcgatcacggttgcgccgggaccaccgcccggaggtgcgttggaactcattgtgtctgtgtctccatgttgttggcgttgtcgatctgctgggatgcgttctgcatggcgagctgctgctgtgcacgctgctgcatcatctggccgtactcggcctcagtcagcacgtagacgttcgggtccaagccaccagcggcggcgaggtctgcgatccacgcggacagcttcagtcgttcgagaatctgcggcggcagtgcgaggacgttggcgaggttgctgccgaactccaacagccggtcacggtcacccgtacgggagagcgcggccaagccggtgatgatgacaggctccaagtccttgcctcggatgtcgcggcccgtcaggttcatcacccaaaaggcgactggtacctgcacgtccgcagcgatccgggagtagccgccacccagcccgccttccagttcttcggcgaccatgcggatttcctgcgcggtcacacgttccgcctgacgagtcaccgccgtctgcaacaggaagcctgcgccgatgcggttgatgtaggtggactggattgcttggttggtttgcagcacgccatcgacgcctgcgttaatcagctcgatgtcacccttcatgccgggaatggccgcgccattgggcgacgccatgaagtcctcgacggaggtctgacctgcggggttaaccagccaccggaactcggaggcgaggatcgcgccctgcactgcggcctcggacagcatcgagagcgactggaagtcggcctcgtagtcttcgaccaagccggagccgtagtcatcgcctgcggccaagtcccagctaaccgcccggtagggcagcttgtctgcggtgtaggtcgaggagaagttggcgggcagcttgcagttgcaaatccacacgtcttcgttgtacttgccggtcttgtggtccagcttgacccacttgtactcccacaccatgccgtcgtcatcgggcttgaagtccgggtgcgcgacaatggcagcgagcgctgcgggttccagctgggtcttgtgcaccttctcccgaaggatcagttcgtagacctcgccggtgcgggtgcgcttgaccacgtagtgccgcatgttgagcacgcggatcgtgtccttctccaacaccatgagggcgttgcccagcacgatcagcatcttcagcaggtcgtacagccgggagcggatggagcgcttgtccagttcgagactggcatcctgctcggccttcgcaagcatcgcctgcatggcctgcaagtcagcgccttgctcctgcgcagcctgcttcgccttgcgcttcagctccaaccggaagaacgggcgggacggtgcgaacagcgacatcatcagcttgttcgccagatggttcactgcctgcgcgccgagagactggaacccgtgggtcagcggctcggtgtcctgatcgcggttcttgcgagggaacagcttgggcacggtccagctcgaatagcgttcgagtcggtacatgatgccctgtcgcttgttgtcgtaagcctcgaactggcggtgagcggtttggatcggatggtccatgctcacctcacaacaggtctgacccggccacggtcgtcagccgggaagctgcggtcgtggtcacgggtcgggtgtaagtggagcgggcggtcttgcgtcggccgatcaggtcggcagtctgcaagtcgaggtcggaagttcccagccgcacatcgacggtatcgacgggggcactcagcaacttctcggcgtactcagatgcggcctgctgtgcagctgcctgtgccatctgatcggccatcgcctgaatctggtagttcgtggattgagtttggaggttggtctgcttgtcgatagcagcagcttgcttcagcgctgctcgcttggcggacccaccaccaacgatgctacccataggttaactccttcgcttggtgaattggggagcatgccgttccagcaggtagccgtagcgtgcatacatccgtgtgagtgctcgggagttccgagctagtgcaccgcctgcgctcagtgagtcgcagtggttgatgtcagccagatgttccatcacggctatgtaccggtcgaaggaactgcccggcccaattcgcagcaccatgttctcaacgaacgtagtacggttcttggagtaccacggtgtgacaatggcaaagcacagcaggtaggcttcatcaatgattactgcatccactagaccctgtgttatcagggccactgtgtaatcagggtcatcacagttgtagctcacagaagattctctgttgtctaccttactatcttctctagatgacagatacaaagcggccgttaaagccgccttgatctgctcactatcacccgtcgttggtgttcggtacggaggaatcaacggtgaaaccctcctgtaagatgttcaggacgcgggccatccccaactgcatacctgcctccaagggcgtggtattcgagttgacggacagcgacagcccggacagcttccgcacggcggccagctggttcgggtggagcgtcatcaggactttcactttggcgtcttcggccatggtgtctcctctgtgctataggtgtaccaaaaggtccggcaccggttccgcttaccttcgcggccgctccaaccggacctcagttgcctcgtgctataggtgtactgaaactccgtcagctgaagaagtacggagaatcaaggacttgccgaaggtccagctcgcccatcggcggcggctccggcaggaacgggtaggccgagtggaaggccgacagcacgtcgtgccgctcgtacatcgacacgaacacctcccggatgatccggtacagtgccgcgctgtcggcggcgtgggtgccgaagtcgtcgtgaatcatggcgaaggcgtcgatgccttcggccttggccgcgttgaccaccagcgtcaggtggcttgcgtcgaggctgtgcacgaagttcggggcgatgccgttgcggtgccgggacttcttcaccgcgtccgtgctcttgcgcagggacagcttggcgttgccgcacagcttggtgttgatgcggtgctcctcggactcccagtagacctgcaccaccgggaacccggacggcgtgatccaccggatgcggtcgtacccttggttgaggatcgacccggagccgcgctgcaaccactccatcgcgcccgctgcggcgaccacggtgtcggcgatggcctcacccatgcgcttgctcaggaagcgcgctgcggggccgtacagggccttgtcgagcgaggggaacttcccacacttcaggtagtcttcgatgatgaagtccgcccacgaggactgccgcgagccgtacggcagggtcatcacgctgcgcttcaccagcgagcgtgtgaggccgtggtcgagccacagcgtgcggtacccttcggcatcctcgtcctcgcctagcaggacggcagtcacgcggtctgccaccatctggtagatgtcattcggcagcggtgctgggatcaggttcgtcgccacgccgcctgctgcgtcgcgcagcatcgccgagaagttctgaagcccattgcacgaaccgtccatgccgactgcgatgcggctcaggaagcgatccccgaacacttgccactgctcgtactccatgcaccagctcagaaattgcagcggcttgtcggcggtcttccactcgtcgttgttcaccgggtccgcagcgaacgccatgatctggtcgtgatgctccgctacccacttcacacgatccggcagagacgccttgtcgtatccccatcggtttgctcctgtgatgcagaaccaatccttcgcgtccttagtcagcagcggcttgccatcggcgaactccaagagcgccttctgcaagtccgaaccctgcggcgacacgccggtggtctgaacgtacttgcggccacggaagtcagcgaagtacacgaagtagatgctcgggtactcggcgaacttgcgcgccaccttcattgcgttgtagaaacgattgcccttgttctgtcgcaggcgctcgtcggtgtgccagttggacatgtcgcgcttccactgcttgaactccaactcctgattgtgggacatggtttccttggtcatgtccttcgtcagccactccggcttgcgcggcttcggcagctcgccctgagaaatgatttcctccatgtcgtgcaccttggcgatggccgacacagcttccatcagtcgcttgttgatgcgccacggcacgcgctgcaatgcgttgatcgcagccatctcgttgcgcagctcggcagcgcggtactcgtcgcgggtctgagcgtaggtcttcaccatccacggattgagtcggcgcatttccttcgtgtggaatccaccgttgtcgatgtccacccagtccatcggcggctcgacgcacggcaggtagaacggcgtggcctcgatcacgaagtcgctgatctgagtaatcagcttgcgcacctcgtcggtcagcacgatcttgacgtgcgtcttggtctggaacttgcggtacgctgcgcctgcactggcagcagtctcggtgaccacgccaatctccaacatgcccagctgcgcaagctgatcgcacaggtacgcgccgacctgatcgcgctgtgcctgtccccactccacgaactcgatgccgttcttgcgtccttgcatcttcatcaccgtcatgcggtggttctcgttgacagagagcttgcggtccatgtcgttcatcaggtggtagaacagagtcggctccgcgtcggcgaactgcgtcagcaggtactcatggtacacgttgatgccaacgttcttcaacacgtcgcggtcgctgccttcgccgtgcttgtctcgcatgcaggaggtaagggcaccgcgaacggcgacgaaggccacagcctcgtaccactcgcgtgcctgttcctcggcgctgacgggctgtccacgcttgttctgacgctcgggatcgtacttggcgcgcagaagtggcacgtgcgcttgcgcacggccgattcgcggagagtcgatgtccgcacggatgcgctccgcaagcggaagcacgaaccggcgatacactgcttgggcgtaggggttgttgtccgcgccgcccttctcctcgttgcgggcgatggacttctccatgcgctccttaccgaaggcgtaggtttccagttcgagttccacttgcgagagcattgttacctccgttgctgccgcacggtgtagtcgcgcggcgggtagcgtttcaggataccgcgcatgatttccatgtgcaggtcgtggatgatgtgcggccacgcctcaccgccgatatcctcggccatgcacgtggcagcagcgccgaacaagtcggcaccgtaccgggcgcgcaccgaaacctcgacgcggcccatccatgccgaggactggctgaagtccagctccggcttctcgaaagtgatcgcgtccatcagcccctccgctcgtcaaggaacttggcgaacgcttcctgcaccttgtcgcgcagcgtctcgttcggccacagggaaccggcgtactcgccgaaaggaacgctgatgcgcagctccaccgtgtcgcgctccatgttgtgccatgcttgcacctcgacgctcacaggtctgcctccttcttgtcgtgacggatgcccttgtatcgcggctcgcgcagcaggccgtacttgctgaaggacatcgcctcgatttccacgatgcctcccacgctaggcagctcgctctcgctgtgcggcacgccgctgccaacctcctgcgtcttgccttctccgaggtcaacgacgaccgtgtacacggcgcggccggtcttctcgccgactgcttcgttgatgccgagcacacgcaggtccagcgtcagggtcggcttgatcttgacgacttcgccgttggttcccttgtcgcccttcacccacttgccgctcggcttgcgcaggatcagcccgtcgtacgcgccgccctcgcacagcagcttcgccgcttccatgctgcccagctcttggtcgatcaggaagccctgcgactcggcgtagaacaccggcgcggtgccctcggcgatggcgtggcccatgctcggcaggcggctgacgcgctcctgatacacgaggtcgctgaaaccctgctcccattcttccagcgtcacgaagtcgaacaccacgaacatcggctcggtgtactgcgtgccgtccttcttgcggaacatgccgctgacggtgggctggtcgatctgcgggtgccagtattcgccgaagtacacgccgaccgggaagaacggcgcggatgcgagagcgttctcgatgtggtgtgcgctgacgacctgctcaccggtgcgggagaacaggtcaaccacgccacgatccaccggctgcatctgcacgtcgcccaccttgatggcatgcaggcccttgttcaccgtgggcacccagtggccgcgcttgatggcgaccatgttgcagccgtcgtacttcggctgtgcgatgtactcggtgcgaagctgctcctcggtgggccgcagcttcttcttgatcttgtcctgctcgactgccttgtggacgatgtagctcatgcgtagtccctccaaatctggaacatggcgagcggcacttcgtaccacggaacgtagcgctcccagtacgtggccttgccgtcgtaccactgcacgcggaagttgcccttggtgaaggcgcggttgatcttgaagccgcgcttgcgcttcttgtagccgggagcaacccggacattctggcgaggcacatcaaacatcggcgctgtcctccttcttggtgccgtcacccagcgcggcgttgaaccgtgcgatgcgggacgacatgaactggttgacgatggtgccgatccacagcttgcgcggagcgagcgaaccacggtagccttcccacgcatcggcgatgcgggtatacagctcggcctgatcttcgtcgggcaggttcgggaacccggccttgaccgcattctgcaatgcctcctcgtggtcggcactctcgccccacgcaacggcgttctcgtaggacttgatgagcatggcggtctggttcttgtagagcattcagttctccttcgacgggaatggaacgaaacctgcgaggcccctcatcacgaggatgcagaatgcgtcgtcagggtatgtacgatgccagagtgagttggcccactcgacatcgaactgcttgcgggtacggtgctcctctaggaagcgcgcccactcggcctcatgtgggacgtaccgatgcacttggccgcagcgggcgcaggccatcagtcacccttgctgaaccagcggcggatgatgtactggcggatgaagctgatcgctgtgaacgcaatgccgatggcgtgcgccgacagcagcggatgctcgggatgccacagcaccggaagcagcgcgatgttcgctgcgtagttgatgctgtagccgatgccgatgttcacccaagcctctttgatggagcgcgccttactctgcgccactggccttctcctcctcgcgcagttccagctccaacaggaacagctcgttgatgatgtggtgcgcccggtggtggatgcccgtctccgggtccagcttctcgccgaggcagcgcttgttgtcgtgtcggtagctcgcgtcctgataccgttcgagcgccttctcgacatgctgccacgagtgcgctttgtacttctgcgcgccgaaggtcagggtgtcgatgactcgggccagtgcacgcggcacgccctcatgcagcagacgggcctgcggcttgcccccgtcatccttcaggccgacgccacggtcggacagtgtgcgacggtcctcgtcgcggtagctcagttcgggcattggtacctctcgtctggtggtggtcacgcctccgatgctgagaagctgtcggagggaatcgggaacgcagcagctcggcttaactcgaccgtcgaagaagacctcgacatcacgagcgaacacgcggcttacctgtccacgcagcccgatcattgcgggcgcattgccgatgtactgtacccgcatgccgctgcggatgtcggtgatcttcatgtcggttccttatgccgggacggtgatgtgcttgcgcgcctcggcgctggtcgtgagcttgcgcccacggctgtagccgtcgcacacggtgcactgaagcaggaggtaggtaccgacctgcgtgcgggccggatcatcctgcgggatcatttcgttgcagccgcacttgttgcagcggtgctcgctgccgtcggccttgtagtacactgcgacgttcggatgctgcgagtaccaaccgcgcagcttcttgtactccaacttcatggacttcacgtcgatgcggttgtacgcttcgcactcgtcccatgctccgggcaggctctgcatgcaggccacccacaggtcgaagccggggaagttgtggtggtcgtacttgcgcagctccggcacgatcacgccggtggtgtactccaacttctgcgaggtgaaggcgaactcggtgcggttcagcagcatcgggtcgatcacctgcaccggagacacgggcggcaggccgaggattgcgaggcgagccttgatcttgcgaaggtcgaacttcttgccgttgcgagcgagcacgaagtcggcggcgttgagcagtgcccacagcgccttgccctgcttgcgatcatcgaacacgtcgcgcacgttgcgctggtccatgtagaacgacgcctcgtcgtccagccattcgcaagcgaacgacatcagcgaccagtcacgcttgatctgcttgacgctgaagttgttgttgaacatgccccagccatagaactcgatggggaacgtctcgatgtcgaggcagagaatcttcgggccgcgcttcggtgctcggcgaatgaactgggtaagggtcacggtgtctccttgttgatagcccgacgctttcgcgctttcgcattgcgagcgatacgcttctcgtcgtcggtcttgtaggtaggatgcaggtaccccgtgatgttggtgaggtgcgaccgcaggtagttggggatgcccgcacagaatgcgaacacgtcgcgcacgccgtaccggcctgcgttgttctcgaccttgccgagcagggagttgcatccgcgatggagcaccccgcgcacagcgccggtcttgtggtcatggtccagcaccggatcgagcggagccttcaggccgaactgtccctgacagagacagcaccggttgccttgctccgctgcgagcttgatgcgcagcagcttgacctgtgttgcagtgagtcgcttcatgctttgtatgcctccaagattgcacgcttctcgttcacgtcctcggcgaggtcatagaacgcctgcttcagcttcggcccgaacacgtcgagcttcagcacgtcgagcagttctgcgtcacgatccgtccgcatccacagcagcacggcttgctcggcgaatgtcttgcgccagtcggcacccaacacttcgctgtacttgccgctcacgatctgcaccgcttcgaggttggtcttcgtctcgaacagcagctgctccgctgtcaccttgcccaccttcggcagacccggtatgttgtcggcggtgtcgccgtggagcatctgcatccagaaccacttgtgaccgtactgcaatccgttctcgccaacgatgtcgtaagcgccgagcggaacctctgtgatgtcgtagccgtcccagtctacgtgcacgccgcagaacattcgcatgtccttgtcggcgctgtgcaccacgtgcaggatgttgtggtgcaatgctgcaccctcgttgacgtacgcgatgccatcgtcggcctcacgggtcagccagattttgggagtgaaagcgtcgccctcgtatgtctccatccactcacgaaggaacgcccagttgttgggcttgcggcctgcttggcgctgaccctgatacggctgcgtggtagcagcgaggaagcgatcacccttggtagacgcggcgtgcgtcaggtgcatgacgatcttgcccgctccgctgacatgcttcagctgtgcgcagcgggagagcacgttgcgtcgtgcatcccccgccgagcagttctcgctaccagccgcgaagtacgccatgtagtccccatcaacgtgagcgatcacgcgcgggttgtgctgacgtaccacctgcaccggcatcggggagcgctcaccggccgctgccatgagagcgctcaggtccatcaggcgatgcctgccatcgggtcgctaccgtccaccgggaacggcggcttgtcgtcggccggagcagcgtcggtgggcgcggcgttcgccacgtcgccgaccacttcgtccagcgcatcgacgccttccttggtgaccgtggtgctgcccgccaacttggcggcggcgtagtcgtagcacggaagacccttgaagttcagcgccgcagcgatgcgcagctgcgtcttgttcttcgactgcgcctcgtgggtgaccttgccggtcttctcgtccttgcgctccgggtactcgccggggatgtagatgctgtcccacatgtcggcgtcggcgaagtcccacacgaacgcacccagcggggtgatctgctgcggcaccgggatcacggtgtccacgaacttgccggtcgggatgccgttctccatttccggcaccggcatgaccggcttgcggatggaagccttgtcgatttcggcgaaggtcttgttcgggtcgcgcttgcccggcttgtggatgacttccagcagcacaccctgacccagcagctgcacgaagtggcgctcctcggtgcgcaggcggctgaagattttgaagtagtgcgccttctcgttggtggacaggccgagggtcagcgtcatgcgcaccggcaccggaccattgtcggtttcgatgtgcgggtgctgcttaccggtcagctcgaacacgatggcgacttcatcctgcgtcttcttcttgccctcgaactcgaactcgtgcttgcccagctcgtagtacccgacgatgcgggcggtggtcacaccggcagcgggcggggtgtagtcgaagctgccaccactggcgaccgactgatccttaccctgcgtggcgaccttgttcaacagtgcgtcaagactcatgcgtgttgttctccttattcaaacgacgggttgtgattacctacgaagtccttgcggatcgacgcgcggtactcgatgaccagaccggcgaactctgcgggagggttcttctcctccatcatgttgtcgcccatcttggtttcacacgggacgccaagcggcagcgtccagttgaaccaccactccatatacaccgacgcttccagcatcgaggcgtgcagcagagcagcggccttggttgcgatgtcgccgtgtgcatccacgtagacggcatcgtgcacctgattcacgagcaacgcacggcccaaccattccttcggttcggtcacgtacttccggtagaaggcgcgcaggctgacgtacatcgccgccttggcccattcaccaccggtgccttgcatcgggtagttcttgatttccgtgggcgagaacgactgcgcacagccacccttgctcgcgggcttgttggcgatgaacaccggggacggtgactcgctgaaggaatacatcttgccgtccggcgtggtccagtgcgaccggccaagctgacacgtcagcccatgcggcacgccttgctgccccgcgttgggatgcggaacgaagcgctgagtgctgacgcggttgcgcttgatgtgctcgaccatgcggtcgatgtactcgcccagctccgggtaacgctcggcctcaccgcgcaccagcgcctcgacttcttcctccgacatgccggtggtcgcagcgatcttcgccacgcccgcaccgtacgcacgctggaaggagaacaccttcgcgttgccgcgcttcttcttccacttcttgtgctcgggatgcttgtcgtccttgctcgccttcaggatgaagtcgtagtcgtacttgccttgctcaccccacgcctgctctgcacggaggcagtgcatgtcgaggccctgcttcaagtcctcgatcagctgacggcactcggtgaggattgcctgcacgtagatttcgagggaggtgtagtccgactggatgatcttgccaccccggtgccgggacacgaaggcgcgcttgatctgcgaacccttctcctccaacgtctcctcgtccagctcgcccttgctcacgttctgcaagttcggatcgctggaagacaagcggccggtaaccgtgttggtcatgttgagcttgtggtggatgatgccgtccggtcccaccagcgtgagcatgcccttctgctctccggtcttctcgtccgtcgtgatgtagtacgtggacaagtccttgtggatgtcgtcgcgtctggcaagcgccttggtgaacggcaggttgcggtagcccagcgcctcgatcacgtcggcagcggtggagtacacgccgggatcgctcttgctttcccatgcagcatcaggctcggtgtagccagggaactcgaacagcatgtcctcgttgcggaacttctgcttggtcaagtcatcgaccttcaccttcttggtcttgtactctcccttgttcttgccgctgccgtacgtggtgtagcgccagaggttgtcgaagtcctcggccggtggcgtcgccgtcgtggtaccatcgaccagcacgtagtgcacctcgtccttctgcacgtaagtcggcccaccctcggtggacatgatcggaaccttggccgtgtacttcaccttgccgccgaagatcagcgcgctcttgtggaagcggctgttccagttgaaggtcaggccctcgggcagctcggggatgaagccgttgagttcggcggtcgccgttgcaagctcgacctccaactccttcgccttcgtaagcgcccagtccttgtccacgtacatgccgttgtactcggcttcgatggtgaagcacagcgcacccatgttgaggagcgccgagcgcagaccaccacgtgcacggaaggcggcgagctgtccgaggaacatcttctcggtgttaccgatgtcgcccacgtcgtcggtgtcgttggtgccgaggaggtaatccatcagcagcgtcttgtcgatgtcgcaggtgtccacgcccgcagcccacagggacttgactgcatcgtccttcaagttgccgccgtagcgtggagccgtctcgtccatgctcgccatgtggaactcttgcgtcatgccgtgcagcaggtactccgcaagctggcagtcccacaccatgccgcct

SEQ ID NO: 18 - DNA, 44415 bp, unidentified
  source 1..44415: mol_type = genomic DNA
gataggcccggagctgtagacatcgtgagctatcgcagcagccatggccttagccacagacttgctcgcatgataggcccctagagctagcgccttgccactgccatcgaagtacggagcctcctcgacccactgctgcttaccagtagtgaccgtgagtacgccgtccttaaccacaagcaccgtcgcggacttgccaacgtgctcctcgtagccttcgcccgctttaagcgcagcgagaaccgggcgaagcactgtgaaatccccggtgacacccagcagcacagggccggtgggtgtcgatacgggcatgatcttacgcacggtgtgcttgtggtcgccctgcgtggcctgactatcggcccacaggtgcttgccgtcccatgcgatggtggtcatttgtcacccgtacaccggcgcttaccggtaccgcacacctcggccttccacgcacgcagcgcagccttgtccttgttgcacagaacggtgtccatgcggcggtcctgcgcgagcttgaccaccttgtcctgcgaggaggtggtgcccttctccccaccgaggtaggtgatgtggcagtctgcaagcagggagtcgtcagggaccggcaggttcgcgcaggaggtcagcgacatcagcaggaacagtgccatcccggtactccggggcagcgtcaagaacttcttcagtgcgaacacgcacgtcctccttctctttgatgtaggtcgcgtacccggtagcctgcgtctgcgccgccttggcggtagcggtcgtgccgacttgggcagtttccagcttctccaccttgcgttgcaggccgtagacgtacagaccgaagcacacgaacatggtcacgaccagcagcaagccaaccagcttgccgccgagccgcgcgatcacttcacttggggtttccacggttggatcacctcgttgttggggcgcaagcacagagcaaactctgcgtcgcggcgcttggggatgccggagcaacggctgctggacagtcggcagtcgagcttaccgacgtagacccagcgcaggaactccttgcagctaccttcacgatcccctgcgttcgctttgcgcagcatggtgctgtcggcgaacgccttctcacctacgttgaacacgaagtctgtgtaggcgtcgatctggttgcggttaacgggggccttcaggtgcttgcgcacgccctgctgggcgatctgtaggtcttcgatcagccacttgtcgcactgtgccttcgttgccgtcatgcccatcgctacgcccttggtgtggccgtagcagatggtcggcacccggccggtgtcgaggtacgcagcgtagcgtaccccttcgtggccttgggtgaatgacagcagcgttgccgaaatgccgatgaagatgccgccgatcaggccgaacagccccttgttgctggtatcttggttctgctgctggttcatggttgctccttacggggtcagtgggtcgtcatccgggtccagatcgaccggagtgtgcgggccggagttcggacccgaggacgcggtgcgtgcgcccgcagcgatcagggcgtccagcacgagggtggcgtccttctggaactgcgcgagcagctgcgctgcggttgcgggatgctgctctgcgtgctccatgagggcgagcagttcgcggtgcaggtagttgccacggccgaacagacccgtgtagttgctggtgaagtcggacttctgcattggttacctccggtaacggtcgagtagggatggacggccacgttgcagcggactcttgcgggtcgctgccttcatgccggtcggatcgttgatccagtcttggaactctcgctgctgctgcttggcgatggccttgttctggtccagtgcaagctgcgcaacccagtgacgcacgctaccttccagtgcatcgagccggtcatcgtgtgcgatgctgcccttctgctgcgtgatcttcgccatctggtggaacaggctgtagacctgacgcttgccgctggtggcgtagcgctgggtgtactcgtgatccatttcaaccacggattccagcatgaccagcgagccgcgagccatgacaggttcgagagtgccgatgatacgggcttccttgttgccggtcacgaactcctcgcggatgtcgcccttgtatcccttctccgtgccgcgatcttctcgcaggacaggcaggaacaccttggcgaacgcgccgtagcccatgttcttttcgatgctgatgacgttcggcttgtacttcaccgcaatgcggcgcagttctagcaagccatcaccgtcgtagccaccgggcacagctcccacggccaacacgtacacggtggagttgaggaaggcggtcacggcgaaggccgtctcgtctccgttggcaccaccaccggccgggtcgatctgcatgtgcacgccctgcacgggggcagtctcggtgctcatgtcgtgcggcatcatcatcacgaagccgtacccactggactggaagctgcgctggtgagcgttgctcaggccacgggtgatcgtcagcgggaagcggtcgccaccaccggggatcacgatcaggttctcggtcttcagcgggaagcgcagcgcatccatcagccgcgtgttgagcatgtagttcagctgatagctggacggtccacgctgacgcagctcggactggtgcttctgctcaccggccaacagctcgtcggtgcactggccctcgtcgcccatcgggccaccaccgaacgccaacatcgggtcggcttctaggcgctgcacgatagacggtgccagatgcgggccgtagtgctcgcgctgtgccggggtcgggtagcgaccgggccagatgcgaacgtcgtagccacgtccgggcagggtgttgtagatggagtcgccggtctgcggcgtgccgaggtacaggatgcgacccggagtaccgggcttgccggtgcagatggccgagaactccaacgtgatggtcagcagcagctcacggttcgcggcagtgcggctgttcttgttggactccacgtcgtcggcgatcagcaggtccgcacgcttacccggcaggttgccggtgacgccgatgcacgccacgctcggggacttgtcgattcccttcagcgagtggtgcacgtcgaacgcatccacggaggtacggtcgcccgcgttcttgtccgggcggatgcactccaacgtcggcaccgtgaggatgatgcgctgaatcagcgtagcaatctcggatgcctgcgtgccgcctgccgatacgatcagcacacggtgagtgggatcgtggatcaggcagaagacggcgtagatggcagcgatggtggacttcgcctcgcctcgctgcgcctgcaccattgcgaggtgcgggccatactgcatgtagttggcgatgtcgtactgcatccacgtcggctcgaaccccagcaccttcataatgtcgcgcatgaaggtggcgaagtgccggtagtggttctgcaacagctccaacttcttgcggcgcacgtcggccgcttcagctgattcacgcattgttggctacgctccccggaaagtgaacgatgttgtcgagtgcacgctgcaactcgtcgtcgtcagccggaggcagcgagtgcttgcccagctcgtcttccagctcgccgagtgccttgttggcctcgcgcgtcgccgtgatgttgttgtccttcaggaacttgatcgccgcattgatgtcggctgcggtgcacagctcgccatcttggatgcgctgcatcagcgcacgcgcgaccagttcgtgcagcgcaccgagtgcgccctcacttgccggattcgacatccttgcctcccatgatctttcggtgctcgcgtgcccgccagtagaactgagcgacggcgtacagaatggcgagcgtagttacgatggcagcaccgtacgtgctgatgaagttgaggtagaccgcgccgagcgtaagcggcgaggttcggacgacctcattgaccacactcggcggggtcatgctgttctcctgtaggttagggccagtcgtcgggattgccgacgagcttccattgcaggcggttgacgttgttcatgcccaccgcaatcaggtcgccggggattcccgaggcgatcacatgttcggttgcgaagcgctcacgctgcgcgcgtacgcacaggttgctgccgttcttgtacgacaggagcacgtcgctctgcgtggcgaagacagcccgcttctcgtccatgcacaggcgcggagtggtagcaccggggatcaccatggtctgcatcgaagcagccaccgtgtcgtaccagtagaacttgcacacaccgcccgccatgtacgccacgtgcgggcgcatggtctggtcgaaggccagtgcgatctgcgtgatcccggagtcggtcagcacggtgaccggggcaacgccgtcgcggtaaacgacgacgctgctgccgtcactctcggcagtccacagcgcagcttggaggtcgtccactgctgcgttgagagtcagcccgccctgctcgaagtcaatgagcgggcgggtgcgccgattctgctgctccacccagtcaccgcgttggatgctttgggagacagtggggatcatggcgtgtaccggctccaagaaacccgcatgcgcaagttcgccgtctccgatccggtcttggtgatacccggattgaagccgacttggaaggtcacgcacgcggagagtcccattgcagccgtgatcggaccaccgggcacgttgttgatcgacatccggcaaacgcagtcacggtagtaagtacccggaacataggctacctgctgaagctgcaagtcagagaagctggcaatcgtccccggcggatactggtcggtgatagctccggtgccgtcgccagtaccgccgtagaagtagtagcacccccacacgtagtccgaccaagcgactgccgactgaccgttcataccgccgctgcggcccattgcaataggcttacaggtaacagtggtgctaacacccttgatcgtctcagtagtgacaaccggcgtggtatctgcgtacatgcgcagctcgtaagtaaccacgaggatttcatccgacagcaccgtgatggtggtcgggttacctgcggagtccttgataagcgcacgggtggtcaggatgtacgcgccggtattgttgttgtatgctttggcaccaagctccgacagaacgccagtagcggtaccagccgggaactggtactggcagcgggagtaggcgtagtacggggcagtggtagtcccaccgctgtccgaggacgtacgaccaacctgcgccacctgtgcaccaagagcggtatcggtgaatgccggggtggcgctgccactaccgactgccaagtaagcaatgaggtcgtacatgctgcgaggatagccgctgccggtatcacccagtgcgtccataccaccgtccgtgataaggttgctctgccagtcggctacaacttcgagagtatcgagggacttacccttgctgatggtgaacacgccagcaatgccgaggtgattgtggatcatgcgaagctccatgatacgaagccagaccggagtcgtgcagtcgcgtcgagcggctggttgactacagggtgctgcttcagggtgaaggaatggaaagaactcgacagcttcgccgtctccgggtcaggcgtgtagtccttacggatggatcggatgtcgaacgaaacgaaagcgctcccgtacaacgtgctctccgggtcggcggcataatcctgcctagagcttcggagttcccagcttacgaaggaggaacccagcgacgcagtatccaaaggctggagcatgtcgatgttgctgtacccagcaaagctgctggtcagcatcgcggcatcgaactggtagaagctgtagagcttggacgtaacgtagatgccctgctcctcgatacgaccggaccagtaggccacacggttcaacccgtccgtgaccttgatgctaaggaagtaggagctgtcgtcgttctgacccagtacgtacttgtggttccacttaacggtgtccacccacagcggtttgttctgcttgctgcggaacgccgacagtacaacctgcacgtacttcgtgtccttgggcgcagcgccttcggcaacggactggtgccacgcaccgttgctgccggaggaaaccatgttgccccagttgcgttgcagctcggtcccatcctccttgcggtagatgatcgacacacgagcaccggccttgcccttggagcttgcgccctgctggacctcggcggtgcatcggatgtagtcgttgaccttggcagggatcagcgggttgagcaggtcgctgccgcccgtcttgatgttggcgaagcgcgcgctgtacacgccgctgtcggtgtcgtagtctgagccagtgccaatcgaccagccttcgccattcgatccaccgcccggcaaccacgtgccgtcgtcgcctgcctcgaagtcgccgttgggcacgagggtttcctcgtccacgacttcagtgaaagccgcccacttgacgacgacttccttggtgatgttgtccacccgtaccgcagcgcccgaagggagcgtcgattcgatgacctccacggtgcagcggccgactgggttgttgatggacaggcgagactcgtaagcctcgcccgccgtgtacccttccagcacgcccgtcaccgacaggccatctgcaacctcgtccgccatgagcggtcggccgtacagcctgaagtgattagccatgcttactccttagccaagtcgcccgagagcaaccacgtgttggtgtcgccgtcgatgcacgttgcagtgatgacggagttggtgccgcgagttgcggcggtgcagccgaccgggacttcgagcgtcacgcccacgtcgccagtgatgaccacagggcctgccttctgctgcacgctgaagtagctgcccgaggcgagcttggtttcaccgtcgcccacttcggggatcaggttgatgttgacggcgcaacctccggcgtacgtgcagcgcacgagtccgtactcggtagccttggcggcgtagtaagtcggaccctctgccgtgatgatcggcacccgcaggctcgcagcggtgatcggcgcaggcccggtgtagggcttggcgtaaccacgcagcacggcgaaccagatgctgccctcggcaggaaccgtggcgaagcggatgaagctgggatcggtgccgtcagcgagcgtgacctgatagtccacgtccggctgcatgccgatgccgttgacgtacacgtcgtagaagcccgcgccggatacgtccgcgcccaccatgtcgaagtcggtgtcacccacctgatcgccagtccaagcaccggaccagacgcgcggggcgacggacacgataccaccagctgccagcaactcggtgacctgcttgtagatgttctggataatctcgttcaggtccacgatcacaccgacctgctggtcgatgctaagggtggcgatgttgagtgagtcgaacatttcctgaatgatcttcaggagctggtcgttgctgaggttaaggtttgtcttgctgatgatgctaccgttaacgtagtcaacgagcatctgctgcaccggagtgctgcggtagatgtagagcttgcgcccagcggcgacggcaggcgagactcggacggtactagcgtcatcgtcttcgctcaggacttccacggtgtgcggagtccggtcggtcagcagctgagtctcctcgtccagcagtccgctcatggcgtacacgtgggacgggttgatgtagccaccggtaaagctgatctgccagtcagtggtcacgccatcggcgtcgaacacgtctgtcgcgtagcgcagctgcgggtctggaactgccatgctgcctcctgtttgctataggtgtaccaaaagggtgggccgtccttggccctgatcttactcctccttccactggctggctgcgcccttcagcagcgggatcaccatcggcagtcgcccgcccggaatcacgtcggccagattctccggcttgccagcaatgccctgagcgaagtcgttgatgactcccagcgacggcgcgaactgcccgcccaccacttccttgcggttgccgaactgcccaccggccagctgcttcagccacgtcggaccctgcgtatcggtggcgtactcgtaccagccgcccgccacgccagtgcccacgtccagcacatcgttgagcatacccgtcgccgacacgtagttcagcgtggccttgcccagcgccagaggcgacaggatgttctggtcgatggcctcgtcgcgctcctgatcgttcatcagggccacgcgggacagcacccgcagggcttgcagcggagccgccacagccatcgcagcagcgatcaggcccgccgtctgccatgcaccgtagttgcccacgtaccggcccagctgcttctgctgcgcgaccagcgagaacgtgcggtgctggaacagcagcttcagccagccgttgtgcgcccacttgccagtctcgccgatgaaggtgtcctgaagaatctgcgaggtgccacggttgatcgcgttgtagaacgccaaccatgcctgccgatccgccagcccctcgacgttgcgcgggtctactgcttccagcttaccatccgcgccccagcgcacgacctgatcctgcgtagcccgcaggcggttcagcaggttgtcgtcaatgcccatgtccttcagggcggtgtcagcttcagcaccatcacgcaggaacttcacgcccttggcgatcagcacttccgcgaagccacgctgctgcacagcaagcacggcccgctgccccgagaggatgcggttcgcatgcgctgccttctgcaccagcgaggtcaggaagcctgcgcgctcgctaccatacatcgacgcctgcgtgtccagcgagttgaacatgtgtaggtcgtaaccggcgagaccgaagccgcgaccgctgatgaactcgaagccgtcgaggatttggttgccgctgtcctcgcccttcaggatgcgcatgatttcgctgcgcatgcggggagcgatacggattgcgtcagccacaccagcagcaccaacagcggcgaggccgttgctgtactccgctgcctgattgatgcccgcgccgcccagctggatggccgaggtcagcagacgcgcattcgccagaacagtcggatcgccggtaccgaccgggcgaccaaggaactcggacatcacctgctcgaacgccttcagctccacatcgttggcaccggtcaggcgcattgcttcgcgcgccacgttgatgcctgcgtcgccgaggatgccgtgcttcgccagagcgatgtcaccagcaacacgtcccgcgtacttgcggtagttgtccatcacgcggttgtcgagatagtccatcagacggaacttaccgtcagcgtcctcgtactgcttggtcacgtcgaggtcgatacgcgccttggtgtgcttcgcaccgccacggctgtacttgcccatgaccttctgaatctcctcctcgttgagcgacatcgcccgcagagtgtcgcgcagcgtgtccgcctgcgactccgagaagacctgacccggcgcttcgatgacacccgcagccttgcgctcgatgcgttccagatacttggtagcgaacttatcgaggaagtcgtccccatacagctcgcccatcacctcgaactgatcgcgcatcgcctgacggataccctcgcgtcgcaccggaccagcagcagcgatgctgccgcccagccacgtacgggactcgtagccctccacgtcctcctccggcagacgctgtgcgcccaccgtaccggccgcgcgctgctctgctgccatgcggttgtagccacggtccaactcacgggccattgccttcactgcctcgtgcgcatccgggatgtccccgccgttgaagcgagtctcgcggtacagcttcactgcgtactcgaagtccgcgcgagccttccagcccgtggcgaagtccttgatcgcaccgataccgcgcacgtccgcacgccacaggcgataggccgcttcccactgacgcgggcgggtgcccatgaacgactcaaaccgaccatgccgatccatcgctgcggtgctgtgtcggcctgctgcaccctcgggattctccaacagggtgatcgcaagcatgcgggcaactggcgacttggacgacattagagtcgtgctcgtagcttccagcccgaagcgctgcatgatggtggacagcttcgccgcgtcgatgccgtactgcgcactgaagcgttcggagcgtgccatcacttcggcgacctgcacacgcatcgcgtcatcactgacggacttgtccagaccggtgcgctggtagaaagccttgcgctcgcggttcgacttgaagatcgagttggcgagcatgccacgcgtctgccgggtaccggcctgcgtgtcgcgcacttccgcgccgaggttgtcaccgacgaccgacatcaggcgttcgagcgcggactcctgattcttcagacccatcactcgcgcgatcttatccttcagccactcccacgcattcgggcgggtgttgcccggcgcgggcatctgacgcagcaccgcctgcacagcgcggttcgtcaggccgtaggaaatcagctcgtcagtgttggcgaggaagcctgcctgcggctggttgatgcgcgtctccatcgcagcggtggtcagcgtggagtccacactgccgatgctgttgttgatatgggtcagcagttcttccatttcctgcccgaacaccgagttgctgcgcagctcacgcagcgtggcagcgtgcagcatttcgtgcaccaccacttccggcgtgtagttccgcatcgccatcgcgtccagtccggcgttgtagccaccggccacacgcatacccggacccatgttggcaccggcgaaccacttgtcgagttccgattccggcacgatcttcaccgtgctcagccgcccgccacgcttcagcgcgttggcgatagcacgcacgtcctccgggatagaggcgttggattccagatacttcagcacgccatcgacgttaccgcccttgatacctgcggtcttccatgcgcgttccagcagcgggtcatgctgatcgacccggccacccacgctgtcgttgtaccgcccggtcgttgcgtccacgttgcccgcgtcccgtgcgagtgcaccagtggtgcctgcggtggtggtcgtctcctgcacgtcgggacgggcgaagatacggaagtcgtcaggcacgtcggccataccagcgcgcagccaatccacagcctcctgcttggcaagctggtggatgcggttgttcaccagcaccgggttggcgtcctcgcccagctcggccacagcgcgcgccttcaggtcggccgaccacgcttcgccgtaagcggcagcgttgcctgcggacaggtcgatggttgccttgtcacgaatctgcgcagccgagcgcacgcccggaatgtgcatcgcggtgcctatggtggtagcgaatgcagcgtcggtcatgaagtccgcgaagttgcggcgctcgcccatgccaaccagcgcggcgtccgtgatgacggaaccgaccgcgttctccgcagcagccgacgcgagcgacgcgcccacgcgcccttcggcaacgagtgcagccgagccgatgcccagcgccttagcgcctgcggcagtgacgccgccgatagcccagttgcccggatcggtgaagcctgccaccatgtcgtaaccgaagctaccccagccagtctgctgatccttgatgcgcatggagtggcggcgcaggaactgtcggtcgctgacgtacttcagctcgttcggcgagtacgctgcatcgcggatgtcttcgagttcgtcggcagtcatccacggcttctcccattccttcgggtcgtacttccaaccttccggaacgttctcgtcctcgcgcgcaaactggttgctgatcgcagcaccgatgccgctgtcgaacgcagcgccccacttgtcgaggaaggtcagcgagttgcgcagctcctcgtccgcgcggtcctgcgcgagcgcctgttcggtctgatccagcagcgccttgcgagcgccggtgttcagcacgtccacttcctgacgcacccaccacggcacaacctgatccgatgcacggacagcctgagccttgcctacggcctgcgcggcggtgccaccttcctgtgctacctgacccatcgacagctcggcgatgcccgcacgaatcttgccgatgtgttccttcgctgccgacgccagagcgttgcggccttcgatgggcgcacccgtccacgcatccgggatggacgcaccggaccacgtacggtcgcgcatgttcgggttgccctgccatgcggcgttgaggtctgcctgcgtggtggtcaggctgcgcggctgcgccgacactgcgggagcggacgcaccgcccagcacgctcggtgcataggctgcgttctcctgcccccagttcttcggattggtgccgccttggtagatgcgcagcgccttcgtcacgtcgcccttggcaagctgcatgttctcgcgcatgatgtcggcatacagctcgatgctgtcttggaagttgcgcatgtcgtacttgcgaccgttgcgcgcttcccacgttgcctgcgtggtgggcatgacttggaagtcgccctgtgctcctgccttgctgcggatcacaccgtcagcgtccttggcggcacgcccgttgccggactctactcgccactgaccgcgcacgatggactccggcactcccgcataagcggcagccttggcaatctgctggtcttgggtcagccccgaaagatcgagtgccattgtctatctccttacagtttgggttggatggaaatgctctgctgaatcgtaccgtcgttcatgcgaacgtagccctgcggtaccggggcctgcaactgacgctgctgcttggtgtgcttctcgtactcgtccttgatgtcgcgcccgtacaccggcacaaccttccagcccttctcgccaacagcgttgacgtacagcaccggctcgccgttctcgctgtccttcatgcggaacacgtcagccttcagcccggtgctcggctcgatgttgacccggcgcagtgctgcgtcgatggccttctcgatggcgggtccggtttccttcgtgtccatgaagcccagccatgcaccgacgctgccgatcactcggccttcgtcgtcgcgtccgttttcccatgcgtacttgcctgcgtcttccagaccgtaggccagcttggcgtgagtagccgcagcctgcaagccttccgcagaagtgtccagcagaccaccggtgtcagtgaccgagcggacgatggcgcgagcatacgcagcgcggccagagtcgcccagcttgttgccgaacatgccgaggtacttggggttgagcttggcgatagcttccgtaacacgagcctgagtagcctcggattccttacggctgttcgcgtcgaactgcgtcggatcgtcggtggtgatttctccacgggccacctcgtaagcaagctcgaagttcacgccaccattctccaacgcttgcagcttgttgaagaacgtgttgacgctatctccgaagtacagcgcagcggtagtcgcgccagtcagtcggccctgcacgggctgaccgttcgtgtcgatgcgtgcggcggtggtctgcttcagttccttccactgctggtacagtgcagccgctgccgtgttcggctgatcgcggagcacagcgcgcgccgtggtctggaactggtcggccacacccttcagcacagcgcctcgcccggtgttggcgttccacaccagctgcgacatggcgaccttggggttcgcggccatcgtggcattccatgcctgcaccgtgttcgcctcgatcagctccttgtccacgccggggatgttgatcgtctgcgcgtacgtgccgcgcttgaacgcttcgatgccaccacggatgtcctcctcctgcgcggccagcttctgctggtcggtcagcgcggccttggccgcagcgttacgctggttgatgacggcttcctgtgcgcggatgtgcgcgcctgcggactgtgccatgatcgaagccaactgcgtaccggagtacagcggtgcgtcgcttccagtctcggcggcgtaggtcgagttcatttcctcgatcatcgcctgcgacggcttggcaccaatgccctccgatgcgtacatggagacgagcgccatcttctcggcctgctccgggttggcatcgagccagtcggaacggtaacgatcctgcgcctgcttcacgtactgctggattcccagctgcccgtccgggtcgatggcgttcagaacgcccttgctgttgaggaacttcagcgtgtggaactcgccgcgatccgcagcgccacgatagaacgcagtgatcgcggacttgtacgactcgtccgtctggtagcgcgagggcgacagtccgtccagcagggacagctgcgcctgcgtcagcgcctcggtggccttctcgtccatgggacggttggtaccgagcatcgccgtgcgcttcgccagttcgttgaagccggtggacgccgacgagttcgcagcgtactgcgccttcaccagctcctgctgctgccatgccgtgcgctccttggtgtgcaggtccatgagggaacccgcgcgatccatgaaggtcttctgcaacaccgtgtccgcgaaaccgttgccggtcatgcgggcagtggcgaggtcgttgaactccttcgccatcgcctcgggaggaagctgacgcaactccggcatacgccgaagcaagtcgctctccatttcgttgacctgcgagagcgtgttatacatgctcgcgccaatctcgtagttggtgtctccgaagattttcttgtaccacggttcggtcgcagcaatctcgtccatggtcttaccagcgcgggcggcaacgaagccgtcccacatctgctgctgcttcagcttggcggtgttcggcgctgccagctcctgcaagaactctggcaggttgctgtccggcatcgtcataccaccagtgcttgcgaaccagtcgttgccggattgaaccggcccgacctgattcacaccagcgccttgaatgctggtgttgcccgacagtgctggggtggcgttgatgccaccctgcaatgcggactgcgtgttgaaggtaaccgtgccgatgtcagccattaccatgcacctcctgagttgcctccgctgccgctatcgaaccagccgaggccggacgtagtggtggagaagttgtcgtagttgttgccgaagttgccggtgaccttcgccccagtcacggactgcttgccggtgccgtcgttgtacccgaaggtagtggacgcccacgacttgccgccgcgatcattggactgctgccacgcctgcataccgttctgcgctgcgttgctgaaggactgagaggcaccagtgaagttgccgttgtccgcctgccacgtgccgaccgcgaagtctgccacggcctcgcctgccatcggcccaccgaagtaggtagccacggccacgccgatcagcttgcccaagcgacgcttcattgcctgcggctcgatgtgctgcgagtagtcgaactgcccgaacgaacggctcatgtccatcccgttccacgcgcgcgacatgatctgcgcagtctgcgatgcgccccgcgaggcgaggagcgagacagcgttggcctgcgtctcctgatccatttccgcctgcaaccgcaccatcgaatccatcaggtctgcggacgagccgccgacaccgacagcaccagcctgcgcctgaagtgcgccacgcgcgttcgccagttggagctgggagttaagcccagccccttggcgcgcacgcagctcctcggacagcgcttccatgttggagttgtactccttcgcggcggcgtccagttgggcgttgttcttcagggaccgcatgaaatcagcgaagccggtcttggcgacctcgctgcggttctggttgtcggtctgcgcaacggctgcacggtagttcgcacgggcaacgcgggtggtgttgttcgcttgcaggatcgtattaaccgaacccattagctaaccctccgtacattgttgaaagtctgacccgtccagctcaggccggtcacccggagcgggagccaatccttgctgcgaatctcgtaggtgcactcgcgcacttcgcgcccgacgctgatgttgagctgcccccggtacaccggttgccgcgcgatcagattgtcggagtcgccgaggatgcggccctcgaagtccgtagtggtcacattgctgttgcgggttgccaccgtggcgatcatgcctgccgtgttctccacgtccaccgtcaccttgttgagggacatgcgtccatcgagtacggcctgaccgttctggtcccgagggaacggattggtcgggatcaccagagcttcggacaccacgccgtattccagcgcaccagcagcgaggtcatcgaactggttaaggaagtcagacgcctgcgcgtagggacaacccagcaggaagtacgggctagtgctattgacggcgatgcttgcgctcgcagtctgtacgcccgtaggtgtaccaaaactcgcccagctgtcgaggcacgcatgcgagtccggctcgcccttcgggtcgaacacgtcgcacgccaccagcgacccgcgcgcagtgaacacgaggccgttcttcttgtagctgctcacgccgatgatttcgcccagcgccgggtggtaccggaacttcgaccacgcatccacgatgcgctgcccgttgttcttgttgtcctcgtaccggtacaggtagaagtcctgcgggtgctcgcgagtgcggaacatgacgaggttcggcgcagtgagcggggtgatctgcaacggagtgcccgacagccacgagtccagctcgttggacatttcgtccgtcaccgtctgctgcccgttgagcgcgcccactcgcatctggtgcaggctcgtgccttcgctgccgtactgcgcataaaagatgtagttgcccgaggtctgcgccttcgcgtcaaccgaatccttgttggcactgaacgctttaatcagcggattcttcggactgaacaccgagtcgccgctgatgccgtactgctgacggtcaccgaagatcacgaggttgccgttgtagagcgtcgcgtgccggagcacatcgccctcgctgccgtgcgcgaagatttcgatggggtcgctgtcttcgatggtgacggccgagccgcgccagaagttcaggtagtccgccgagcgtgaggcgttgacgtagttctgtgcgccgatgaccagccggtcttggaagacggacagcatcgtgatcggcttgtcgatgaaccacgggatcggcgaggtcagaccatcgcctgccactcgcgcaccgtaggccggatgctcgccgctgctcggagccagagacgtgaggcccgcaccgttgcgtgcgatgtagcctacaccgttgtagatgtagagctgcgacacgaggttgtcgatggtgcactccacgccgggcgcttcgtaccagtccaccgacccgtagccggaagtctcgccgttctccaactcagcgcgcaggtagtacgactcgtccgcgcctgcaccactcggccgcacgcgaatgaccttgccgtgccagtggaacttgacggcgtaggtcgcgtctgtaatttcctgccctgcggcgtagaaggtcgtgccgtctccctcgtcgtcaaccgtgatgtccttgaactggtcatcgtcaatgatgatcccgcccttgatgtacgttgccgacacgcctgcatcgaccagcaaatccgacagctgctccgcgatgtactccgggcgcgtctgctcagcgctcgtcacgatccactcgttgaccgcagagttgtactcgttcactcggtcgttgacgtacttctggtacgccgcgtccggctccgtgccaccgggaaggtagaacgggatgtcgctggtgtcgagcgttccggggtacgatgcggtaaccgtcttgaacgttaccgtcagcaccgtgttgtccgtccgcgtcaggttcaccgtgtacgtggtgttgtacttcccggtgcgcacccatgctgcgaggcgctggatgttcgtctgctcctgccacacgttcgtgctggtggccgaggggatcgtggtgttgcccgcgatgtagacgtagctgccgatggccgtgagcgacgatgcgcctccgctgaccagcgtgttgacccacgtgctgttctcgtacaccagagggatgaacgactcgtccgtcttgttgtagaggaacgcgaaggactcgctgcccaaggtcgaggcgtcgcgccggtacagcagcgcgtactccttgccctcctgcatgaagtcgaacacgtccatgttgcgcagctcggccgaggtgacaacggcttgggaagcagcgaaccgcgtaccacgacggcgcacgaggccgttcaccggatcggacagcacgttgatctgctcgtgcgtctgtcccggccgacgacgatgcgccggtttctgactgacaccctgaaggatgtcgggataggttccgcctgcctttgccatgttgtctccttagccggggaatgtgacgtggctgtgccacgggtgaccgctgtagttccagtaacgggaacgcagcacgtccacggatgcgcgagcgaacagcgggttcgccttgatctggcggatgtgctcggccttcaagttgatgtaactgtcatcgcgctgctgcttgatcttggcgtacttggtgttgtcgccgtcgaagtcagactggaaccgcagcaccgagtcgtcgcgcacgaacatctgcacctcgtaggggaggtcatcgaagtccagcagccgcaccagcttggcctgcacgttgtggtcgaactcgtaggtgttgcgcttgcggtcgtacagtcggcgtccgcgctgcaccacgtggccgaaccggctcgggttgcagtccagcttcagcacgtccgtggggaccatgatgtacttgctcgttgcctgcggcttcagctccacccattcggtgttgaaccacagcgagagtgaggacacgtcacggtgcacgcggtcgatcaagtcaacggcgtcgtccttgtatacgtggtcatcttccagcgtgttgagcttcgtctcgcccatcgtcttcaagcaggcgttcacgatgtcgagcttggtgatgaatgccatggtgtctcctgagaggaacaaggcagagacgccggagcgcccctgccgggatgttgcttagtccgcagccagagccagagcggccggtgcgtactcgatgtcctgcgagccgatttcgtcgtccacgaaacggacacggacgacccagcctgcggtgccacgggtgtcgtagtggacgccgacgacggtaccaacggagttggcgggcagaccggccacgccagttgcggcgacgacgcggttggaaatctcgaacggtcggtcaaagaccatgatgttgctcctgtgttggtggaagaagggcgcggtttgagttacccgaaggattcagggaccgcgcccagcggattaggcaaccttgtcgatgcggcccgcgttctcgacgcgatccagaccaacggcgaaggacatccacgagtccacgaagtagcacttcgaggcatcgctccaccacaccgaggactgcaacggcagcgcttcggcgatcagcagggccttcggcgacacggccacggcgatcagggtgctgaagtcgccgtcgtagaagtcgtcgttgtcgtcgttcgacagcaggtgaccttcgatcacggtgttcggcaggttctcgctcgacagcaccgggacgccccagccgtggaaggtcgggatgccggtcagcttgttgccgtccgaggtcaggtactcgccgttgctgatctgctcggcctgctgcaacaggtagaagatcgccgggcgcacgatcaggaccacgccatcgcgctgcggcttgaccttcttctcctcctccatgcgggagaacagtttgccgatggcggcgtacaccttggccggatcgttctcgtcaccagcggcggacagcacgacctgcgtggcaccgaagtggccctcgggcgcgcggccgttgcgggtgaagatcgactgcgtggcagcagcggccttcgcggcggcgatgctgatggtcaggtccacgaactcggcgatttcctgaccctgctcgatggcgatttccttgcgggtgtcgatgtcggtgaagatttcgtccagctgccagatgctgtgacgcgacagcagcatggtatcgacggtcaccgacgccttgctgaagtccaccggggtgccgtccggcgcgtcaccgcgcttcagcttctgaagcttggtacggccgatggccttcttggtcagggtgttggtgcccttgacctgcttgcgcgggaagaacttttccagcaccgagctggacacgtaggtgtgctcgacatcgccggtgaactgttcgaggatcagggcgttctcgttgccggactggttgacctgattcggcagaaccgggacagtcgggaagatggtgctcatgctttgtgttgctccttggtcttagtggatgacgcgcgcgttgagtgcacgcagttcttcggagtgggccgcaccacggatgcccttctcggcaaccagcttgcggtactcagcgcggtactgctccttcgtgataggagcgacgccgttgatcgacgcggcgggggcggcggcgttggtagccggtgcgcccttgacggtcgtcgcgggattggcctgtgccagagccatcaggtaacgcgcggtcgcctgagcgccgaagccaccagccgacagcgattcgcttgcctgcttcagttggtcggcgggcaggttggcccgtgcgaactgctggatcgcagcccagttctctgcgccacccacggcttcgtggacagcagcaacgttcgcggcgtgcgctgcggttgcagcggcggtgacacgagcgatgctctccttcgccagagcgaggatcggtgcggaacccttggccttgtcgccgaggacttccagcttggcttccagcagggcgaagttgcccttcgctgcttcggtcagttcgcggctgtcgatgtcgaggcccacggtgttgacgaagtattcggccgcgatgttcaggccgttgtcgccgtagtccgggatcgacaccgcagtcggcgcagcgttcgccggggcggcgggctgtgcgggagcggcaggttcgagactcagcgcgtcagcagccggaggtgcagcaggagctgcgggctgtgccggtgcggccggagcgggctggccgttgggcaacagcttgtcgtctgcgggagccggagctgccggtgcgggctggttgccgttcgaggttgcgatcacggttgcgccgggaccaccgcccggaggtgcgttggaactcattgtgtctgtgtctccatgttgttggcgttgtcgatctgctgggatgcgttctgcatggcgagctgctgctgtgcacgctgctgcatcatctggccgtactcggcctcagtcagcacgtagacgttcgggtccaagccaccagcggcggcgaggtctgcgatccacgcggacagcttcagtcgttcgagaatctgcggcggcagtgcgaggacgttggcgaggttgctgccgaactccaacagccggtcacggtcacccgtacgggagagcgcggccaagccggtgatgatgacaggctccaagtccttgcctcggatgtcgcggcccgtcaggttcatcacccaaaaggcgactggtacctgcacgtccgcagcgatccgggagtagccgccacccagcccgccttccagttcttcggcgaccatgcggatttcctgcgcggtcacacgttccgcctgacgagtcaccgccgtctgcaacaggaagcctgcgccgatgcggttgatgtaggtggactggattgcttggttggtttgcagcacgccatcgacgcctgcgttaatcagctcgatgtcacccttcatgccgggaatggccgcgccattgggcgacgccatgaagtcctcgacggaggtctgacctgcggggttaaccagccaccggaactcggaggcgaggatcgcgccctgcactgcggcctcggacagcatcgagagcgactggaagtcggcctcgtagtcttcgaccaagccggagccgtagtcatcgcctgcggccaagtcccagctaaccgcccggtagggcagcttgtctgcggtgtaggtcgaggagaagttggcgggcagcttgcagttgcaaatccacacgtcttcgttgtacttgccggtcttgtggtccagcttgacccacttgtactcccacaccatgccgtcgtcatcgggcttgaagtccgggtgcgcgacaatggcagcgagcgctgcgggttccagctgggtcttgtgcaccttctcccgaaggatcagttcgtagacctcgccggtgcgggtgcgcttgaccacgtagtgccgcatgttgagcacgcggatcgtgtccttctccaacaccatgagggcgttgcccagcacgatcagcatcttcagcaggtcgtacagccgggagcggatggagcgcttgtccagttcgagactggcatcctgctcggccttcgcaagcatcgcctgcatggcctgcaagtcagcgccttgctcctgcgcagcctgcttcgccttgcgcttcagctccaaccggaagaacgggcgggacggtgcgaacagcgacatcatcagcttgttcgccagatggttcactgcctgcgcgccgagagactggaacccgtgggtcagcggctcggtgtcctgatcgcggttcttgcgagggaacagcttgggcacggtccagctcgaatagcgttcgagtcggtacatgatgccctgtcgcttgttgtcgtaagcctcgaactggcggtgagcggtttggatcggatggtccatgctcacctcacaacaggtctgacccggccacggtcgtcagccgggaagctgcggtcgtggtcacgggtcgggtgtaagtggagcgggcggtcttgcgtcggccgatcaggtcggcagtctgcaagtcgaggtcggaagttcccagccgcacatcgacggtatcgacgggggcactcagcaacttctcggcgtactcagatgcggcctgctgtgcagctgcctgtgccatctgatcggccatcgcctgaatctggtagttcgtggattgagtttggaggttggtctgcttgtcgatagcagcagcttgcttcagcgctgctcgcttggcggacccaccaccaacgatgctacccataggttaactccttcgcttggtgaattggggagcatgccgttccagcaggtagccgtagcgtgcatacatccgtgtgagtgctcgggagttccgagctagtgcaccgcctgcgctcagtgagtcgcagtggttgatgtcagccagatgttccatcacggctatgtaccggtcgaaggaactgcccggcccaattcgcagcaccatgttctcaacgaacgtagtacggttcttggagtaccacggtgtgacaatggcaaagcacagcaggtaggcttcatcaatgattactgcatccactagaccctgtgttatcagggccactgtgtaatcagggtcatcacagttgtagctcacagaagattctctgttgtctaccttactatcttctctagatgacagatacaaagcggccgttaaagccgccttgatctgctcactatcacccgtcgttggtgttcggtacggaggaatcaacggtgaaaccctcctgtaagatgttcaggacgcgggccatccccaactgcatacctgcctccaagggcgtggtattcgagttgacggacagcgacagcccggacagcttccgcacggcggccagctggttcgggtggagcgtcatcaggactttcactttggcgtcttcggccatggtgtctcctctgtgctataggtgtaccaaaaggtccggcaccggttccgcttaccttcgcggccgctccaaccggacctcagttgcctcgtgctataggtgtactgaaactccgtcagctgaagaagtacggagaatcaaggacttgccgaaggtccagctcgcccatcggcggcggctccggcaggaacgggtaggccgagtggaaggccgacagcacgtcgtgccgctcgtacatcgacacgaacacctcccggatgatccggtacagtgccgcgctgtcggcggcgtgggtgccgaagtcgtcgtgaatcatggcgaaggcgtcgatgccttcggccttggccgcgttgaccaccagcgtcaggtggcttgcgtcgaggctgtgcacgaagttcggggcgatgccgttgcggtgccgggacttcttcaccgcgtccgtgctcttgcgcagggacagcttggcgttgccgcacagcttggtgttgatgcggtgctcctcggactcccagtagacctgcaccaccgggaacccggacggcgtgatccaccggatgcggtcgtacccttggttgaggatcgacccggagccgcgctgcaaccactccatcgcgcccgctgcggcgaccacggtgtcggcgatggcctcacccatgcgcttgctcaggaagcgcgctgcggggccgtacagggccttgtcgagcgaggggaacttcccacacttcaggtagtcttcgatgatgaagtccgcccacgaggactgccgcgagccgtacggcagggtcatcacgctgcgcttcaccagcgagcgtgtgaggccgtggtcgagccacagcgtgcggtacccttcggcatcctcgtcctcgcctagcaggacggcagtcacgcggtctgccaccatctggtagatgtcattcggcagcggtgctgggatcaggttcgtcgccacgccgcctgctgcgtcgcgcagcatcgccgagaagttctgaagcccattgcacgaaccgtccatgccgactgcgatgcggctcaggaagcgatccccgaacacttgccactgctcgtactccatgcaccagctcagaaattgcagcggcttgtcggcggtcttccactcgtcgttgttcaccgggtccgcagcgaacgccatgatctggtcgtgatgctccgctacccacttcacacgatccggcagagacgccttgtcgtatccccatcggtttgctcctgtgatgcagaaccaatccttcgcgtccttagtcagcagcggcttgccatcggcgaactccaagagcgccttctgcaagtccgaaccctgcggcgacacgccggtggtctgaacgtacttgcggccacggaagtcagcgaagtacacgaagtagatgctcgggtactcggcgaacttgcgcgccaccttcattgcgttgtagaaacgattgcccttgttctgtcgcaggcgctcgtcggtgtgccagttggacatgtcgcgcttccactgcttgaactccaactcctgattgtgggacatggtttccttggtcatgtccttcgtcagccactccggcttgcgcggcttcggcagctcgccctgagaaatgatttcctccatgtcgtgcaccttggcgatggccgacacagcttccatcagtcgcttgttgatgcgccacggcacgcgctgcaatgcgttgatcgcagccatctcgttgcgcagctcggcagcgcggtactcgtcgcgggtctgagcgtaggtcttcaccatccacggattgagtcggcgcatttccttcgtgtggaatccaccgttgtcgatgtccacccagtccatcggcggctcgacgcacggcaggtagaacggcgtggcctcgatcacgaagtcgctgatctgagtaatcagcttgcgcacctcgtcggtcagcacgatcttgacgtgcgtcttggtctggaacttgcggtacgctgcgcctgcactggcagcagtctcggtgaccacgccaatctccaacatgcccagctgcgcaagctgatcgcacaggtacgcgccgacctgatcgcgctgtgcctgtccccactccacgaactcgatgccgttcttgcgtccttgcatcttcatcaccgtcatgcggtggttctcgttgacagagagcttgcggtccatgtcgttcatcaggtggtagaacagagtcggctccgcgtcggcgaactgcgtcagcaggtactcatggtacacgttgatgccaacgttcttcaacacgtcgcggtcgctgccttcgccgtgcttgtctcgcatgcaggaggtaagggcaccgcgaacggcgacgaaggccacagcctcgtaccactcgcgtgcctgttcctcggcgctgacgggctgtccacgcttgttctgacgctcgggatcgtacttggcgcgcagaagtggcacgtgcgcttgcgcacggccgattcgcggagagtcgatgtccgcacggatgcgctccgcaagcggaagcacgaaccggcgatacactgcttgggcgtaggggttgttgtccgcgccgcccttctcctcgttgcgggcgatggacttctccatgcgctccttaccgaaggcgtaggtttccagttcgagttccacttgcgagagcattgttacctccgttgctgccgcacggtgtagtcgcgcggcgggtagcgtttcaggataccgcgcatgatttccatgtgcaggtcgtggatgatgtgcggccacgcctcaccgccgatatcctcggccatgcacgtggcagcagcgccgaacaagtcggcaccgtaccgggcgcgcaccgaaacctcgacgcggcccatccatgccgaggactggctgaagtccagctccggcttctcgaaagtgatcgcgtccatcagcccctccgctcgtcaaggaacttggcgaacgcttcctgcaccttgtcgcgcagcgtctcgttcggccacagggaaccggcgtactcgccgaaaggaacgctgatgcgcagctccaccgtgtcgcgctccatgttgtgccatgcttgcacctcgacgctcacaggtctgcctccttcttgtcgtgacggatgcccttgtatcgcggctcgcgcagcaggccgtacttgctgaaggacatcgcctcgatttccacgatgcctcccacgctaggcagctcgctctcgctgtgcggcacgccgctgccaacctcctgcgtcttgccttctccgaggtcaacgacgaccgtgtacacggcgcggccggtcttctcgccgactgcttcgttgatgccgagcacacgcaggtccagcgtcagggtcggcttgatcttgacgacttcgccgttggttcccttgtcgcccttcacccacttgccgctcggcttgcgcaggatcagcccgtcgtacgcgccgccctcgcacagcagcttcgccgcttccatgctgcccagctcttggtcgatcaggaagccctgcgactcggcgtagaacaccggcgcggtgccctcggcgatggcgtggcccatgctcggcaggcggctgacgcgctcctgatacacgaggtcgctgaaaccctgctcccattcttccagcgtcacgaagtcgaacaccacgaacatcggctcggtgtactgcgtgccgtccttcttgcggaacatgccgctgacggtgggctggtcgatctgcgggtgccagtattcgccgaagtacacgccgaccgggaagaacggcgcggatgcgagagcgttctcgatgtggtgtgcgctgacgacctgctcaccggtgcgggagaacaggtcaaccacgccacgatccaccggctgcatctgcacgtcgcccaccttgatggcatgcaggcccttgttcaccgtgggcacccagtggccgcgcttgatggcgaccatgttgcagccgtcgtacttcggctgtgcgatgtactcggtgcgaagctgctcctcggtgggccgcagcttcttcttgatcttgtcctgctcgactgccttgtggacgatgtagctcatgcgtagtccctccaaatctggaacatggcgagcggcacttcgtaccacggaacgtagcgctcccagtacgtggccttgccgtcgtaccactgcacgcggaagttgcccttggtgaaggcgcggttgatcttgaagccgcgcttgcgcttcttgtagccgggagcaacccggacattctggcgaggcacatcaaacatcggcgctgtcctccttcttggtgccgtcacccagcgcggcgttgaaccgtgcgatgcgggacgacatgaactggttgacgatggtgccgatccacagcttgcgcggagcgagcgaaccacggtagccttcccacgcatcggcgatgcgggtatacagctcggcctgatcttcgtcgggcaggttcgggaacccggccttgaccgcattctgcaatgcctcctcgtggtcggcactctcgccccacgcaacggcgttctcgtaggacttgatgagcatggcggtctggttcttgtagagcattcagttctccttcgacgggaatggaacgaaacctgcgaggcccctcatcacgaggatgcagaatgcgtcgtcagggtatgtacgatgccagagtgagttggcccactcgacatcgaactgcttgcgggtacggtgctcctctaggaagcgcgcccactcggcctcatgtgggacgtaccgatgcacttggccgcagcgggcgcaggccatcagtcacccttgctgaaccagcggcggatgatgtactggcggatgaagctgatcgctgtgaacgcaatgccgatggcgtgcgccgacagcagcggatgctcgggatgccacagcaccggaagcagcgcgatgttcgctgcgtagttgatgctgtagccgatgccgatgttcacccaagcctctttgatggagcgcgccttactctgcgccactggccttctcctcctcgcgcagttccagctccaacaggaacagctcgttgatgatgtggtgcgcccggtggtggatgcccgtctccgggtccagcttctcgccgaggcagcgcttgttgtcgtgtcggtagctcgcgtcctgataccgttcgagcgccttctcgacatgctgccacgagtgcgctttgtacttctgcgcgccgaaggtcagggtgtcgatgactcgggccagtgcacgcggcacgccctcatgcagcagacgggcctgcggcttgcccccgtcatccttcaggccgacgccacggtcggacagtgtgcgacggtcctcgtcgcggtagctcagttcgggcattggtacctctcgtctggtggtggtcacgcctccgatgctgagaagctgtcggagggaatcgggaacgcagcagctcggcttaactcgaccgtcgaagaagacctcgacatcacgagcgaacacgcggcttacctgtccacgcagcccgatcattgcgggcgcattgccgatgtactgtacccgcatgccgctgcggatgtcggtgatcttcatgtcggttccttatgccgggacggtgatgtgcttgcgcgcctcggcgctggtcgtgagcttgcgcccacggctgtagccgtcgcacacggtgcactgaagcaggaggtaggtaccgacctgcgtgcgggccggatcatcctgcgggatcatttcgttgcagccgcacttgttgcagcggtgctcgctgccgtcggccttgtagtacactgcgacgttcggatgctgcgagtaccaaccgcgcagcttcttgtactccaacttcatggacttcacgtcgatgcggttgtacgcttcgcactcgtcccatgctccgggcaggctctgcatgcaggccacccacaggtcgaagccggggaagttgtggtggtcgtacttgcgcagctccggcacgatcacgccggtggtgtactccaacttctgcgaggtgaaggcgaactcggtgcggttcagcagcatcgggtcgatcacctgcaccggagacacgggcggcaggccgaggattgcgaggcgagccttgatcttgcgaaggtcgaacttcttgccgttgcgagcgagcacgaagtcggcggcgttgagcagtgcccacagcgccttgccctgcttgcgatcatcgaacacgtcgcgcacgttgcgctggtccatgtagaacgacgcctcgtcgtccagccattcgcaagcgaacgacatcagcgaccagtcacgcttgatctgcttgacgctgaagttgttgttgaacatgccccagccatagaactcgatggggaacgtctcgatgtcgaggcagagaatcttcgggccgcgcttcggtgctcggcgaatgaactgggtaagggtcacggtgtctccttgttgatagcccgacgctttcgcgctttcgcattgcgagcgatacgcttctcgtcgtcggtcttgtaggtaggatgcaggtaccccgtgatgttggtgaggtgcgaccgcaggtagttggggatgcccgcacagaatgcgaacacgtcgcgcacgccgtaccggcctgcgttgttctcgaccttgccgagcagggagttgcatccgcgatggagcaccccgcgcacagcgccggtcttgtggtcatggtccagcaccggatcgagcggagccttcaggccgaactgtccctgacagagacagcaccggttgccttgctccgctgcgagcttgatgcgcagcagcttgacctgtgttgcagtgagtcgcttcatgctttgtatgcctccaagattgcacgcttctcgttcacgtcctcggcgaggtcatagaacgcctgcttcagcttcggcccgaacacgtcgagcttcagcacgtcgagcagttctgcgtcacgatccgtccgcatccacagcagcacggcttgctcggcgaatgtcttgcgccagtcggcacccaacacttcgctgtacttgccgctcacgatctgcaccgcttcgaggttggtcttcgtctcgaacagcagctgctccgctgtcaccttgcccaccttcggcagacccggtatgttgtcggcggtgtcgccgtggagcatctgcatccagaaccacttgtgaccgtactgcaatccgttctcgccaacgatgtcgtaagcgccgagcggaacctctgtgatgtcgtagccgtcccagtctacgtgcacgccgcagaacattcgcatgtccttgtcggcgctgtgcaccacgtgcaggatgttgtggtgcaatgctgcaccctcgttgacgtacgcgatgccatcgtcggcctcacgggtcagccagattttgggagtgaaagcgtcgccctcgtatgtctccatccactcacgaaggaacgcccagttgttgggcttgcggcctgcttggcgctgaccctgatacggctgcgtggtagcagcgaggaagcgatcacccttggtagacgcggcgtgcgtcaggtgcatgacgatcttgcccgctccgctgacatgcttcagctgtgcgcagcgggagagcacgttgcgtcgtgcatcccccgccgagcagttctcgctaccagccgcgaagtacgccatgtagtccccatcaacgtgagcgatcacgcgcgggttgtgctgacgtaccacctgcaccggcatcggggagcgctcaccggccgctgccatgagagcgctcaggtccatcaggcgatgcctgccatcgggtcgctaccgtccaccgggaacggcggcttgtcgtcggccggagcagcgtcggtgggcgcggcgttcgccacgtcgccgaccacttcgtccagcgcatcgacgccttccttggtgaccgtggtgctgcccgccaacttggcggcggcgtagtcgtagcacggaagacccttgaagttcagcgccgcagcgatgcgcagctgcgtcttgttcttcgactgcgcctcgtgggtgaccttgccggtcttctcgtccttgcgctccgggtactcgccggggatgtagatgctgtcccacatgtcggcgtcggcgaagtcccacacgaacgcacccagcggggtgatctgctgcggcaccgggatcacggtgtccacgaacttgccggtcgggatgccgttctccatttccggcaccggcatgaccggcttgcggatggaagccttgtcgatttcggcgaaggtcttgttcgggtcgcgcttgcccggcttgtggatgacttccagcagcacaccctgacccagcagctgcacgaagtggcgctcctcggtgcgcaggcggctgaagattttgaagtagtgcgccttctcgttggtggacaggccgagggtcagcgtcatgcgcaccggcaccggaccattgtcggtttcgatgtgcgggtgctgcttaccggtcagctcgaacacgatggcgacttcatcctgcgtcttcttcttgccctcgaactcgaactcgtgcttgcccagctcgtagtacccgacgatgcgggcggtggtcacaccggcagcgggcggggtgtagtcgaagctgccaccactggcgaccgactgatccttaccctgcgtggcgaccttgttcaacagtgcgtcaagactcatgcgtgttgttctccttattcaaacgacgggttgtgattacctacgaagtccttgcggatcgacgcgcggtactcgatgaccagaccggcgaactctgcgggagggttcttctcctccatcatgttgtcgcccatcttggtttcacacgggacgccaagcggcagcgtccagttgaaccaccactccatatacaccgacgcttccagcatcgaggcgtgcagcagagcagcggccttggttgcgatgtcgccgtgtgcatccacgtagacggcatcgtgcacctgattcacgagcaacgcacggcccaaccattccttcggttcggtcacgtacttccggtagaaggcgcgcaggctgacgtacatcgccgccttggcccattcaccaccggtgccttgcatcgggtagttcttgatttccgtgggcgagaacgactgcgcacagccacccttgctcgcgggcttgttggcgatgaacaccggggacggtgactcgctgaaggaatacatcttgccgtccggcgtggtccagtgcgaccggccaagctgacacgtcagcccatgcggcacgccttgctgccccgcgttgggatgcggaacgaagcgctgagtgctgacgcggttgcgcttgatgtgctcgaccatgcggtcgatgtactcgcccagctccgggtaacgctcggcctcaccgcgcaccagcgcctcgacttcttcctccgacatgccggtggtcgcagcgatcttcgccacgcccgcaccgtacgcacgctggaaggagaacaccttcgcgttgccgcgcttcttcttccacttcttgtgctcgggatgcttgtcgtccttgctcgccttcaggatgaagtcgtagtcgtacttgccttgctcaccccacgcctgctctgcacggaggcagtgcatgtcgaggccctgcttcaagtcctcgatcagctgacggcactcggtgaggattgcctgcacgtagatttcgagggaggtgtagtccgactggatgatcttgccaccccggtgccgggacacgaaggcgcgcttgatctgcgaacccttctcctccaacgtctcctcgtccagctcgcccttgctcacgttctgcaagttcggatcgctggaagacaagcggccggtaaccgtgttggtcatgttgagcttgtggtggatgatgccgtccggtcccaccagcgtgagcatgcccttctgctctccggtcttctcgtccgtcgtgatgtagtacgtggacaagtccttgtgaatgtcgtcgcgtctggcaagcgccttggtgaacggcaggttgcggtagcccagcgcctcgatcacgtcggcagcggtggagtacacgccgggatcgctcttgctttcccatgcagcatcaggctcggtgtagccagggaactcgaacagcatgtcctcgttgcggaacttctgcttggtcaagtcatcgaccttcaccttcttggtcttgtactctcccttgttcttgccgctgccgtacgtggtgtagcgccagaggttgtcgaagtcctcggccggtggcgtcgccgtcgtggtaccatcgaccagcacgtagtgcacctcgtccttctgcacgtaagtcggcccaccctcggtggacatgatcggaaccttggccgtgtacttcaccttgccgccgaagatcagcgcgctcttgtggaagcggctgttccagttgaaggtcaggccctcgggcagctcggggatgaagccgttgagttcggcggtcgccgttgcaagctcgacctccaactccttcgccttcgtaagcgcccagtccttgtccacgtacatgccgttgtactcggcttcgatggtgaagcacagcgcacccatgttgaggagcgccgagcgcagaccaccacgtgcacggaaggcggcgagctgtccgaggaacatcttctcggtgttaccgatgtcgcccacgtcgtcggtgtcgttggtgccgaggaggtaatccatcagcagcgtcttgtcgatgtcgcaggtgtccacgcccgcagcccacagggacttgactgcatcgtccttcaagttgccgccgtagcgtggagccgtctcgtccatgctcgccatgtggaactcttgcgtcatgccgtgcagcaggtactccgcaagctggcagtcccacaccatgccgccgccgtcgatgaactcgatccatgcctgccggttgagtgggccttggcagatggcgtgcaggatgtcgaacttgatgttgaacccgacgaggaactgctgcccgtaacacagctcacgcagccacccatcgggtgcgccgcccatgtactggttgtctatcccgactcgggtgtcgtagtacaggccggtgttccgtgcgtcacccttccgcttgtagccaatcgccacgatcttgttcatgtcgtagaacggattggccttgcgcttcaggatggaacggatcgtggtttcgaggtcgaaggaagtgaagctcacagcggccaccgttgcagggccagctggtacatttcatccgacgcatcgccatccaagtccagcccgtcgcgcacccaacggaacacgatgatgcggtcctgcttgtccttgatgttgcggcgcttgcagatggtggtggcctcgaccgcgcgctgataccagccggagtcggcggtcaccatgacgttgaacacgccgttgcgcagcgcataccacgtggtgctgtagtcctcgtcctcctcgtagtgtccatcggcaccggagcacagggtccatccctgatcgaccagcttttcgatggcctcgtggaagtcctgcaccagcacgaggaagtcgatgtccgtgtcggtcacgggcggctcgactgtgtagctgctgccggtgcggctggacgtgatgacgcccacgttgcgcggcaggtagatgttcggttcggtactcacggtgtgttacctccgggcttggtgatccagaacgtgaagcacgggatcagattgatgcaccagcgcttgttgtgcggcgagtagtgcacgccgatccaagtgctgtgtttgttccgcagccatccccacttccactgcggcgcgtcgttgcggccttcgatgtagcctgcgtcgtgcaccttgcgcagcagcttggcaaggtggattgcttgcgcgttgctcacgcagttgaaggtcttcgcctcggtggattcaccggggaagctgaccgacaccgtgaacccggtggctacgatgtgaattggcttgctcatgctgcctcctgatagaagcgggcacgctctgcatccatcatcacttcttcccgaacgtcacgcttgccgcctgcgcggtgcagcttgttcttcggggtgccgatgtagcggaagcgttccatcgctgggtcattgagcttgccgcccatgatgatgaagtcgcacgcaccctgcttgccggtcttgctgtccttcagtgcggactgcggcgggtactggattccctcaccctcggcgctgatctgcgaagtcgccacgcccacggcgtcgtacttcacacaccagttgcgagcggcctgatacatcgcctccaacatctgatcggtacgctgcccgccgttggtcatgccaccggtgaacgtgatgttgtcgatcatgtcgaagatgatgaagccggggttggtctgcttgatgatggcctcgacttcaccggagttgaacccgtggatgtcgtagaactgcatgcggtggatgtccccgcccatcgcatcttcgatgcgcttgcggatgctaccatccttcgcccactccaccatctcagggatggtagcgccgagcagcgactgataccaccgctgcttgatgcgcttgcccggcccctcgttgttgagccagatgccggtgcgcttctggtccggccaaacgttgtcgagctgcgtgatccagtggctggactcgctggtcaggaacgtggtcttgcctgcgtcgggacgcatggcgtagatgccgaagtcaccaccacgcagagcgcgcaggttcttcgccaacgtgggcagtcggaagtggatgccgatgtcgtgctcgtccatctgcatcagttcctcgggcgtctcctgcaccagcgggagccgcgccttgcgatccattcggtcggtgatcgtctcggccaagccgtacagctcgtcgcgcaggctgaactcagcgccgccattccactgcacgatcttgctgaccgcagtggtggcaagctccaactccaacagcttctcgatcatgccctgctctgcctcgggcgggaccggctcgcgcatctgcttcagcagaactttgagcagggacttcttgtcgtcgggctgcgtcttccacttgaactccatggcccagccatcgaacacatcgaacggcaagtccttcgtgtccgggaactccttgtagtacgcacgcaacgcatcgagcatcagcacggtcagctcgtccagcccatcacgtggtgcgctgggtaccagccggtcgaacttgccacggttggtgcacaaccgcagcagcgtggtgtcaagactcatcaggttctccttcgggttcgtacttggaatcgagctggtgataccgggtgttgcgcgtctcgaacttgcgcccgccgtccgccacatacagcaccgtcgaggtgtgcacgatgtcgcagtcgccgaggttcggatgcgcaagcacgccgccgagcgtggcacggaagccaacgacgggcgggatgatagcgcgccggtagcgcacgatgggtttgctcattgcagcttctccttgatgtagtcggtcgtgtaatacttcgggtcacgtggtgacgtgatgttcctgtagtccagaccaaacgcacgtagacgcgcagcgattactcgcgcactgtcttggccgggattgctaccgttgcttctacctctgtcgtcatcgagccacgtcgctacacgttggcctcgatcagtcagctgcttcaacactttgttgtgcagcttggtgccgagcaacgaccacgcttcggttaccagtcccaccttgtatgcactgagcgggtcttcgcacagtacgatggtgtcacctgtgcccacgccgtagcgtgcgacaagtccgtctttcggaacgtcaggtgttagccacttcggctgtctcgttgccgaccgggctgtccagtataccacgttgtcgccttcagtgatcggtagtaccacccgcccgatgcttgggcaccagtacagccgcagcttctcgatcatctgaagcgagagtcccatcttgaagaaccacaccttagcgtcgagcggccactcgcgggtgtcgtatacccgtggctctggcaactcaacagtcgcacgcactctgcgttcgctcgtctgctcggcgtggattcgtgcaagcttggcctcgatactctcgtgctcacgcttgaatcctgtgccaccgcacctgaaacagaatgcggtggacttgtcgtgctctcgtgagataagcaagggcgtaccctccccgcactcatgggccacacgtgtgcggccaccaacaggcaggcgctcggcatgtggtagccagtcgttgtcgggaagggtatcgctcatgctatcctcgcttggttattcccagacctcgaagatgtcgtggctggtggcgtacaggacggagccgttgccgtccgtgctgacgatcagacgggagccgtcttcactggtcagcttggacacgacgaacccggtgcccttcggcagcttgttggtctgccgcgtgtcgatcaggtacgcattctggccgggcttcagctcgtcgccacgcttgacgacggccacgctgggtgacggcggggcgaggctcacgactgcccgccttcgccacccgcagccttggcggcagcggcttcggcggcgaggcgctgggcctcggcaacggcggcgtcgatttcttcctgcgccttcagcacttcctcggccgacatcagcagggcgctgctgtcgatcaggttcagctcggcatccagaccttcgccggtctgcaccttcagttgcagcacgcccttgtcgttcttgccggtggcgacgatcacgccggacaggacgcgcttgttcagggcacgaccgaacaggtaggacacggcgtcgcccgccttcagcgcttcgatggcggcgctgttggcctcgacggcatccagcttggcgagcttctcgttcaggccatcgaccttggcctgcgccttggcgatgtcttccagcagctcggcgcgcttggcttcgtagtggctgacggtggtctgctcggtggtgttttcgttcgacatgtagatggttcctcttgacggttgataggatggcccgtacgtgggccagtcgtagcctacccggctcgggttactgaaagatcagctcgctgttgtacccaccgccgccattgtagaagcggcgacgcagcacgctctcctcacccagcaccagcagacggtccacgatggcgcggatggcgctcatgtactggtccaccagctcgctgtgcaagttcaggtcgaagcggatcacggtcaccgcctcgtcgtccagtgcgccggtgtccttgcggacgtacaggccacggccattggtcatggtcgcaccgccgatcagcttcacggcggcggcaatctccggctgcacgttgagcagtcggctgtcgggcacagtcacctcgacccagcttcccatgcgcaggctcatgctgcacctgccagtgcggactgcacgttgggctgcaacgatgcaccggaacgcagctcggcagcacgacgcttcatgcgggagcgcagcttgcgacgctgcttgttgttcccgccgaggctatcggccacgcgcttcagctggttgttgccgacgatgcgggtctgaccctgccccttctgcacggggaagtagtcctgccccagcatcttgcgcaggatcgggttgtcgatgggaatcagcggcacgctgacgtgcaggtgccggctggtgtccggcgcaggcggcggcgtgtcgtcgtcatcgtggcgcggcttcaccgctgcgaccaccttgtccttgacgtacttggccgcagccttgatcttgtccatgaaacccatggttacttcctcctcgttccgaagtgattgaactccaactcatgccacacgtagtacgtggtgccgagcgggtcagtgtctgccttccagttgcgctggtcgcagtagtcgttggctgcgccgaggtcatcgaacgtcagcgagaacccagtggaagccgggccggtgcggaaccggcacagcttgccgtcgtcgtcatggtactggccgacgacaacccacgggccacgacccacgatccagtacagcaggatcaggatgcgcagccagagcttacgcatagtacggctcgacacggtagcccatgttctcgccgcccagcgactcggcattgaacacggcgcgcgctgcatcgcgggtcgggaacagcacgttgtactcgctcttgttgtactcgttgccgtcgatgcgcacggtggcgctcgggtgctggttgtagcagctgacatcggagtcgctgcggtcttcggcgaaggcgtaggtgatacgccaacccagcggcttgcgcaccggcttgcggatgctctcgcccacttcgaggatgtgccagttgaagaacgacccgccgtagctgttgagcacatccgcctcggcacgcacggcggcgcggcggtcgaagatggcgagctggttcgggtacgtgccgtcacgcagcgagtccagcaggctggtggtggcacccttggtgcgcagctcggcgatcaccgcatccagttcctcttgggtcggggtgcggccggtgccattggcgacgacgccagtgatgacgccatcgttgctgttcttggggatcgagacgatgaagtataccttacgcatggtggttctcctgattgacgggtgggatttcgatttcctctatcgagtagagggtgggcaccttctcgtggtgcttgcggtggtgttcgatggcttgctcgcacgcctcgtggctggtgtgatgtccgccgaggatgtaatccccgacagccacacccttcacggtaacgagcggcagcgccttcaccacaaggcgcaggctgacctcacgcataccagcgctccacgctgtgctcatgggtcacgaactctttccactggcgcggctgctcgcacagctggatcggcttgcgctccccactacggatgcgcttgtaagttacggggatcatgcaatgtgccctcctgttgggcgtggttccaaagctacgccctcgttagaaggcgcagcggtagatcacgcgcggctcgggtgccacttcacgcggtagcggcggagacggttcggatcgttgccgacgtgcgaggcgatggcgttgcgtgcagcctgcgcagtggtgaacgtgccgctgagtccgatcacagtggacgtattccaacccagctggtgagggcgccgcgcatgcttggtgaagaactcggcggtgtagaagccgcgatccttctccgggccatcgggagtgccttcgggcaccacacggtacgcatcctcgctgatgccctgcaccttggcccgcgccttcagcatgcggtacgcagcattgcggctgcgctgcggcaggcccagctcacgcacctgcgcccagttggcgagggcgatgctgccgtggcgcagattgaactgcacgatccagcccttggtcttcgtcttgttgaccagcccggtctgcgatgcagtcagggcgacgtggcgtgcgctctggtcgtccatcaggacatccggcagcttacgcggcaggttgtcgggcattgccaggccgggcaacaccatgcggccggtcacgctgccgaggaagtccagctgcgaggcatccaacaccaccggaggcaacggagacagcaggcacgccatcacccgcgcctcgatagcagcgaagtcaagttcacgcatgccgtagcccacggtgaacgtcggcggtgcgatcaggtcgcgcagcagctgtgcctcgacatcgctgtcacggcaggccgcaatcacgtcgtcctcgaattgcaggatggcgtcacgctcgaagctctcgacaccgaagtcgcgcagctcaccgtgcagcacggcgaactcattggacagcttgcggttggagtacgggtctgcctttgcggtcagtgcacaggcgatgtgaagggccgagcgcagcagggatgcttcgcgctgggtcactcgaaggttgatcttgggttccatgttacacgttctccttcttcttggtgggcttcggcacagcgcgggcagcgttgatgacggcctgttcctcctcggtcggcacgtagccttcctcggtcgccttttccagacggcccagcagcttgtgcaggtcggcggcgaacgagaacgcctctgcgggcttctcggtcttgaagtcgtaccacgccttcgcggcggcacgttccagcacgtcggccagagcttcgccctcgactcgcttgctcttggcaaacttcatgggcgcgctcgccttggtttccttgtcgtcgttcggagccatcgggccgaactcggacaggtacaggcgcagggcttcatgcttcatgccgttgcccacggcgagacacagatcggaagcgagcgtaacgtcgccgtggatgtgtgcgtggttgatgaccgcaatcgcggcctgctgaatctggtccaccagcttggtgcgggcggtgttgatcgacttgatggcgcgcttgatgtcagcgcttccggtgatgatgtccatggtggttcccttcaggttgggtccgtgccgattgcacgacactaggccctcttgcgaaggcccagtagcttgcatttaagcgagtcggatgtcgaatgaacgcccaccgcacggcaggacgtagagcgccgacacagagccggccggatgcttcatgatggcccgattgtaggaatcgcgggcagcttccacgtagtggcgagagaacttgaaccggatcacaggtaagccctcctgtcagcggcgtggttcgcccggttcgtcccgctgttaccctcgacaacaaacacagatcgctttccggcggttccgtggcgggcttcgtagcgctcggcttggcgcttgcgctcggcaagcttgcggtcatgctccgtggtgcgcaggtccatcacgcttgccgtccgggtgaactggcagaagcggcgcttacgctgggtgcggtcgagattggcattgatcgagccttgcatgttgtgcctccattggcactggtgggaaaactaacagattgatgcgccctcagaaagccgtcgagtcggtcaatccctcattctcgattagagccgttgcatcgcctatcgtgggcgcacactgaccaccggatttgcctgcatggtcatcgcaaagggagggcgcatcaatctgctagcccttcgggctgtcaaccctactccggctagcagtgccattgtcaccgtgtggcccgtagagccttttcacgaaacgcacagtattccatgcgataggaggctcaccacctccttatgaccggcttcccaccttggcagtgggttacttcccgtggccgactctcacggcagatgggaagccctaagcgttaggcttaggtaaagcggcaccagtgttgcaagtctggtggattctatgggcctttgaaatcccagttcatccggttatccgctagtgctacgttgcagcttggcggtccacgtcaactctcggccactattggctgtggttggcacgcttcccgttacaccctacccgttagcggtagtcctacgccatccaatgtggctgctcctcagagcgtggtgccatactagcacccttgttgcatcctgtcaagcccttggctcgctcgggtctctaacccgttgggcgtcctgtcgccaccatcccaccatgtacgtcggtggtccacgtgttgcaaggcctcaaagggctatctgtgccgccttgtcaagctatccgttagaggaccatgtgcgctcctgttagtgtcttgaccggtgtcccggtctcacctcagcctcaacacccgtaatctctcacgtctagccttaccgctaggtcgctccgctgttccggtggctaccacttgccgcctatcatagctaactgctagcttagtgtcaagcgtggttcggtagctcctcgcatcccttaccagtgactcccgtgtacccttagcccacttgttggcggcgccactacggatcacgtcactcgacttgcgttgcagcttactaccattgcggccgtgtgtctactactgcttgcatcgcaagcgtcaaccgttggcctagcgggtagctaactaatcagctcgacagagtaccgatagacggtgattcaggttgagccgactgtgtgctataggtgtaccaaaaggccgaaacgatacagatggccctcgcacgcctacagctgcggttcgcatggtagcaggtagggtagcccctgtcaagccccttgcggccctcctgaagccctgtcgctgccccagtgacgccattgaaccacaccgcaccggccacgtcaacacctttcgccaagagatttattaacgattcagccaaggcagcgcggtccagccatacaggcagcaggcgcacgcccacccgcacgcccacccgcaggcacccacgcacggccacgcacacgcacgctcaggcccacgcaggcaggcacacgggtacacccacgcggaaccttgacgcgggcgcacagacgcgcacacaggcgcacacgcgggcacgcacccacgcacacccgcaggcgcgtaacgcgagggcgtacgggggcacgcgcgggagcttctattggagtgacccccgcgcatttccgaagcaaattttggtccggctacccacgtggccttactcctaagcctcgcgaactggtgcctttagcttgac

SEQ ID NO: 19 - DNA, 44415 bp, unidentified
  source 1..44415: mol_type = genomic DNA
gcgctgccttggctgaatcgttaataaatctcttggcgaaaggtgttgacgtggccggtgcggtgtggttcaatggcgtcactggggcagcgacagggcttcaggagggccgcaaggggcttgacaggggctaccctacctgctaccatgcgaaccgcagctgtaggcgtgcgagggccatctgtatcgtttcggccttttggtacacctatagcacacagtcggctcaacctgaatcaccgtctatcggtactctgtcgagctgattagttagctacccgctaggccaacggttgacgcttgcgatgcaagcagtagtagacacacggccgcaatggtagtaagctgcaacgcaagtcgagtgacgtgatccgtagtggcgccgccaacaagtgggctaagggtacacgggagtcactggtaagggatgcgaggagctaccgaaccacgcttgacactaagctagcagttagctatgataggcggcaagtggtagccaccggaacagcggagcgacctagcggtaaggctagacgtgagagattacgggtgttgaggctgaggtgagaccgggacaccggtcaagacactaacaggagcgcacatggtcctctaacggatagcttgacaaggcggcacagatagccctttgaggccttgcaacacgtggaccaccgacgtacatggtgggatggtggcgacaggacgcccaacgggttagagacccgagcgagccaagggcttgacaggatgcaacaagggtgctagtatggcaccacgctctgaggagcagccacattggatggcgtaggactaccgctaacgggtagggtgtaacgggaagcgtgccaaccacagccaatagtggccgagagttgacgtggaccgccaagctgcaacgtagcactagcggataaccggatgaactgggatttcaaaggcccatagaatccaccagacttgcaacactggtgccgctttacctaagcctaacgcttagggcttcccatctgccgtgagagtcggccacgggaagtaacccactgccaaggtgggaagccggtcataaggaggtggtgagcctcctatcgcatggaatactgtgcgtttcgtgaaaaggctctacgggccacacggtgacaatggcactgctagccggagtagggttgacagcccgaagggctagcagattgatgcgccctccctttgcgatgaccatgcaggcaaatccggtggtcagtgtgcgcccacgataggcgatgcaacggctctaatcgagaatgagggattgaccgactcgacggctttctgagggcgcatcaatctgttagttttcccaccagtgccaatggaggcacaacatgcaaggctcgatcaatgccaatctcgaccgcacccagcgtaagcgccgcttctgccagttcacccggacggcaagcgtgatggacctgcgcaccacggagcatgaccgcaagcttgccgagcgcaagcgccaagccgagcgctacgaagcccgccacggaaccgccggaaagcgatctgtgtttgttgtcgagggtaacagcgggacgaaccgggcgaaccacgccgctgacaggagggcttacctgtgatccggttcaagttctctcgccactacgtggaagctgcccgcgattcctacaatcgggccatcatgaagcatccggccggctctgtgtcggcgctctacgtcctgccgtgcggtgggcgttcattcgacatccgactcgcttaaatgcaagctactgggccttcgcaagagggcctagtgtcgtgcaatcggcacggacccaacctgaagggaaccaccatggacatcatcaccggaagcgctgacatcaagcgcgccatcaagtcgatcaacaccgcccgcaccaagctggtggaccagattcagcaggccgcgattgcggtcatcaaccacgcacacatccacggcgacgttacgctcgcttccgatctgtgtctcgccgtgggcaacggcatgaagcatgaagccctgcgcctgtacctgtccgagttcggcccgatggctccgaacgacgacaaggaaaccaaggcgagcgcgcccatgaagtttgccaagagcaagcgagtcgagggcgaagctctggccgacgtgctggaacgtgccgccgcgaaggcgtggtacgacttcaagaccgagaagcccgcagaggcgttctcgttcgccgccgacctgcacaagctgctgggccgtctggaaaaggcgaccgaggaaggctacgtgccgaccgaggaggaacaggccgtcatcaacgctgcccgcgctgtgccgaagcccaccaagaagaaggagaacgtgtaacatggaacccaagatcaaccttcgagtgacccagcgcgaagcatccctgctgcgctcggcccttcacatcgcctgtgcactgaccgcaaaggcagacccgtactccaaccgcaagctgtccaatgagttcgccgtgctgcacggtgagctgcgcgacttcggtgtcgagagcttcgagcgtgacgccatcctgcaattcgaggacgacgtgattgcggcctgccgtgacagcgatgtcgaggcacagctgctgcgcgacctgatcgcaccgccgacgttcaccgtgggctacggcatgcgtgaacttgacttcgctgctatcgaggcgcgggtgatggcgtgcctgctgtctccgttgcctccggtggtgttggatgcctcgcagctggacttcctcggcagcgtgaccggccgcatggtgttgcccggcctggcaatgcccgacaacctgccgcgtaagctgccggatgtcctgatggacgaccagagcgcacgccacgtcgccctgactgcatcgcagaccgggctggtcaacaagacgaagaccaagggctggatcgtgcagttcaatctgcgccacggcagcatcgccctcgccaactgggcgcaggtgcgtgagctgggcctgccgcagcgcagccgcaatgctgcgtaccgcatgctgaaggcgcgggccaaggtgcagggcatcagcgaggatgcgtaccgtgtggtgcccgaaggcactcccgatggcccggagaaggatcgcggcttctacaccgccgagttcttcaccaagcatgcgcggcgccctcaccagctgggttggaatacgtccactgtgatcggactcagcggcacgttcaccactgcgcaggctgcacgcaacgccatcgcctcgcacgtcggcaacgatccgaaccgtctccgccgctaccgcgtgaagtggcacccgagccgcgcgtgatctaccgctgcgccttctaacgagggcgtagctttggaaccacgcccaacaggagggcacattgcatgatccccgtaacttacaagcgcatccgtagtggggagcgcaagccgatccagctgtgcgagcagccgcgccagtggaaagagttcgtgacccatgagcacagcgtggagcgctggtatgcgtgaggtcagcctgcgccttgtggtgaaggcgctgccgctcgttaccgtgaagggtgtggctgtcggggattacatcctcggcggacatcacaccagccacgaggcgtgcgagcaagccatcgaacaccaccgcaagcaccacgagaaggtgcccaccctctactcgatagaggaaatcgaaatcccacccgtcaatcaggagaaccaccatgcgtaaggtatacttcatcgtctcgatccccaagaacagcaacgatggcgtcatcactggcgtcgtcgccaatggcaccggccgcaccccgacccaagaggaactggatgcggtgatcgccgagctgcgcaccaagggtgccaccaccagcctgctggactcgctgcgtgacggcacgtacccgaaccagctcgccatcttcgaccgccgcgccgccgtgcgtgccgaggcggatgtgctcaacagctacggcgggtcgttcttcaactggcacatcctcgaagtgggcgagagcatccgcaagccggtgcgcaagccgctgggttggcgtatcacctacgccttcgccgaagaccgcagcgactccgatgtcagctgctacaaccagcacccgagcgccaccgtgcgcatcgacggcaacgagtacaacaagagcgagtacaacgtgctgttcccgacccgcgatgcagcgcgcgccgtgttcaatgccgagtcgctgggcggcgagaacatgggctaccgtgtcgagccgtactatgcgtaagctctggctgcgcatcctgatcctgctgtactggatcgtgggtcgtggcccgtgggttgtcgtcggccagtaccatgacgacgacggcaagctgtgccggttccgcaccggcccggcttccactgggttctcgctgacgttcgatgacctcggcgcagccaacgactactgcgaccagcgcaactggaaggcagacactgacccgctcggcaccacgtactacgtgtggcatgagttggagttcaatcacttcggaacgaggaggaagtaaccatgggtttcatggacaagatcaaggctgcggccaagtacgtcaaggacaaggtggtcgcagcggtgaagccgcgccacgatgacgacgacacgccgccgcctgcgccggacaccagccggcacctgcacgtcagcgtgccgctgattcccatcgacaacccgatcctgcgcaagatgctggggcaggactacttccccgtgcagaaggggcagggtcagacccgcatcgtcggcaacaaccagctgaagcgcgtggccgatagcctcggcgggaacaacaagcagcgtcgcaagctgcgctcccgcatgaagcgtcgtgctgccgagctgcgttccggtgcatcgttgcagcccaacgtgcagtccgcactggcaggtgcagcatgagcctgcgcatgggaagctgggtcgaggtgactgtgcccgacagccgactgctcaacgtgcagccggagattgccgccgccgtgaagctgatcggcggtgcgaccatgaccaatggccgtggcctgtacgtccgcaaggacaccggcgcactggacgacgaggcggtgaccgtgatccgcttcgacctgaacttgcacagcgagctggtggaccagtacatgagcgccatccgcgccatcgtggaccgtctgctggtgctgggtgaggagagcgtgctgcgtcgccgcttctacaatggcggcggtgggtacaacagcgagctgatctttcagtaacccgagccgggtaggctacgactggcccacgtacgggccatcctatcaaccgtcaagaggaaccatctacatgtcgaacgaaaacaccaccgagcagaccaccgtcagccactacgaagccaagcgcgccgagctgctggaagacatcgccaaggcgcaggccaaggtcgatggcctgaacgagaagctcgccaagctggatgccgtcgaggccaacagcgccgccatcgaagcgctgaaggcgggcgacgccgtgtcctacctgttcggtcgtgccctgaacaagcgcgtcctgtccggcgtgatcgtcgccaccggcaagaacgacaagggcgtgctgcaactgaaggtgcagaccggcgaaggtctggatgccgagctgaacctgatcgacagcagcgccctgctgatgtcggccgaggaagtgctgaaggcgcaggaagaaatcgacgccgccgttgccgaggcccagcgcctcgccgccgaagccgctgccgccaaggctgcgggtggcgaaggcgggcagtcgtgagcctcgccccgccgtcacccagcgtggccgtcgtcaagcgtggcgacgagctgaagcccggccagaatgcgtacctgatcgacacgcggcagaccaacaagctgccgaagggcaccgggttcgtcgtgtccaagctgaccagtgaagacggctcccgtctgatcgtcagcacggacggcaacggctccgtcctgtacgccaccagccacgacatcttcgaggtctgggaataaccaagcgaggatagcatgagcgatacccttcccgacaacgactggctaccacatgccgagcgcctgcctgttggtggccgcacacgtgtggcccatgagtgcggggagggtacgcccttgcttatctcacgagagcacgacaagtccaccgcattctgtttcaggtgcggtggcacaggattcaagcgtgagcacgagagtatcgaggccaagcttgcacgaatccacgccgagcagacgagcgaacgcagagtgcgtgcgactgttgagttgccagagccacgggtatacgacacccgcgagtggccgctcgacgctaaggtgtggttcttcaagatgggactctcgcttcagatgatcgagaagctgcggctgtactggtgcccaagcatcgggcgggtggtactaccgatcactgaaggcgacaacgtggtatactggacagcccggtcggcaacgagacagccgaagtggctaacacctgacgttccgaaagacggacttgtcgcacgctacggcgtgggcacaggtgacaccatcgtactgtgcgaagacccgctcagtgcatacaaggtgggactggtaaccgaagcgtggtcgttgctcggcaccaagctgcacaacaaagtgttgaagcagctgactgatcgaggccaacgtgtagcgacgtggctcgatgacgacagaggtagaagcaacggtagcaatcccggccaagacagtgcgcgagtaatcgctgcgcgtctacgtgcgtttggtctggactacaggaacatcacgtcaccacgtgacccgaagtattacacgaccgactacatcaaggagaagctgcaatgagcaaacccatcgtgcgctaccggcgcgctatcatcccgcccgtcgttggcttccgtgccacgctcggcggcgtgcttgcgcatccgaacctcggcgactgcgacatcgtgcacacctcgacggtgctgtatgtggcggacggcgggcgcaagttcgagacgcgcaacacccggtatcaccagctcgattccaagtacgaacccgaaggagaacctgatgagtcttgacaccacgctgctgcggttgtgcaccaaccgtggcaagttcgaccggctggtacccagcgcaccacgtgatgggctggacgagctgaccgtgctgatgctcgatgcgttgcgtgcgtactacaaggagttcccggacacgaaggacttgccgttcgatgtgttcgatggctgggccatggagttcaagtggaagacgcagcccgacgacaagaagtccctgctcaaagttctgctgaagcagatgcgcgagccggtcccgcccgaggcagagcagggcatgatcgagaagctgttggagttggagcttgccaccactgcggtcagcaagatcgtgcagtggaatggcggcgctgagttcagcctgcgcgacgagctgtacggcttggccgagacgatcaccgaccgaatggatcgcaaggcgcggctcccgctggtgcaggagacgcccgaggaactgatgcagatggacgagcacgacatcggcatccacttccgactgcccacgttggcgaagaacctgcgcgctctgcgtggtggtgacttcggcatctacgccatgcgtcccgacgcaggcaagaccacgttcctgaccagcgagtccagccactggatcacgcagctcgacaacgtttggccggaccagaagcgcaccggcatctggctcaacaacgaggggccgggcaagcgcatcaagcagcggtggtatcagtcgctgctcggcgctaccatccctgagatggtggagtgggcgaaggatggtagcatccgcaagcgcatcgaagatgcgatgggcggggacatccaccgcatgcagttctacgacatccacgggttcaactccggtgaagtcgaggccatcatcaagcagaccaaccccggcttcatcatcttcgacatgatcgacaacatcacgttcaccggtggcatgaccaacggcgggcagcgtaccgatcagatgttggaggcgatgtatcaggccgctcgcaactggtgtgtgaagtacgacgccgtgggcgtggcgacttcgcagatcagcgccgagggtgagggaatccagtacccgccgcagtccgcactgaaggacagcaagaccggcaagcagggtgcgtgcgacttcatcatcatgggcggcaagctcaatgacccagcgatggaacgcttccgctacatcggcaccccgaagaacaagctgcaccgcgcaggcggcaagcgtgacgttcgggaagaagtgatgatggatgcagagcgtgcccgcttctatcaggaggcagcatgagcaagccaattcacatcgtagccaccgggttcacggtgtcggtcagcttccccggtgaatccaccgaggcgaagaccttcaactgcgtgagcaacgcgcaagcaatccaccttgccaagctgctgcgcaaggtgcacgacgcaggctacatcgaaggccgcaacgacgcgccgcagtggaagtggggatggctgcggaacaaacacagcacttggatcggcgtgcactactcgccgcacaacaagcgctggtgcatcaatctgatcccgtgcttcacgttctggatcaccaagcccggaggtaacacaccgtgagtaccgaaccgaacatctacctgccgcgcaacgtgggcgtcatcacgtccagccgcaccggcagcagctacacagtcgagccgcccgtgaccgacacggacatcgacttcctcgtgctggtgcaggacttccacgaggccatcgaaaagctggtcgatcagggatggaccctgtgctccggtgccgatggacactacgaggaggacgaggactacagcaccacgtggtatgcgctgcgcaacggcgtgttcaacgtcatggtgaccgccgactccggctggtatcagcgcgcggtcgaggccaccaccatctgcaagcgccgcaacatcaaggacaagcaggaccgcatcatcgtgttccgttgggtgcgcgacgggctggacttggatggcgatgcgtcggatgaaatgtaccagctggccctgcaacggtggccgctgtgagcttcacttccttcgacctcgaaaccacgatccgttccatcctgaagcgcaaggccaatccgttctacgacatgaacaagatcgtggcgattggctacaagcggaagggtgacgcacggaacaccggcctgtactacgacacccgagtcgggatagacaaccagtacatgggcggcgcacccgatgggtggctgcgtgagctgtgttacgggcagcagttcctcgtcgggttcaacatcaagttcgacatcctgcacgccatctgccaaggcccactcaaccggcaggcatggatcgagttcatcgacggcggcggcatggtgtgggactgccagcttgcggagtacctgctgcacggcatgacgcaagagttccacatggcgagcatggacgagacggctccacgctacggcggcaacttgaaggacgatgcagtcaagtccctgtgggctgcgggcgtggacacctgcgacatcgacaagacgctgctgatggattacctcctcggcaccaacgacaccgacgacgtgggcgacatcggtaacaccgagaagatgttcctcggacagctcgccgccttccgtgcacgtggtggtctgcgctcggcgctcctcaacatgggtgcgctgtgcttcaccatcgaagccgagtacaacggcatgtacgtggacaaggactgggcgcttacgaaggcgaaggagttggaggtcgagcttgcaacggcgaccgccgaactcaacggcttcatccccgagctgcccgagggcctgaccttcaactggaacagccgcttccacaagagcgcgctgatcttcggcggcaaggtgaagtacacggccaaggttccgatcatgtccaccgagggtgggccgacttacgtgcagaaggacgaggtgcactacgtgctggtcgatggtaccacgacggcgacgccaccggccgaggacttcgacaacctctggcgctacaccacgtacggcagcggcaagaacaagggagagtacaagaccaagaaggtgaaggtcgatgacttgaccaagcagaagttccgcaacgaggacatgctgttcgagttccctggctacaccgagcctgatgctgcatgggaaagcaagagcgatcccggcgtgtactccaccgctgccgacgtgatcgaggcgctgggctaccgcaacctgccgttcaccaaggcgcttgccagacgcgacgacatccacaaggacttgtccacgtactacatcacgacggacgagaagaccggagagcagaagggcatgctcacgctggtgggaccggacggcatcatccaccacaagctcaacatgaccaacacggttaccggccgcttgtcttccagcgatccgaacttgcagaacgtgagcaagggcgagctggacgaggagacgttggaggagaagggttcgcagatcaagcgcgccttcgtgtcccggcaccggggtggcaagatcatccagtcggactacacctccctcgaaatctacgtgcaggcaatcctcaccgagtgccgtcagctgatcgaggacttgaagcagggcctcgacatgcactgcctccgtgcagagcaggcgtggggtgagcaaggcaagtacgactacgacttcatcctgaaggcgagcaaggacgacaagcatcccgagcacaagaagtggaagaagaagcgcggcaacgcgaaggtgttctccttccagcgtgcgtacggtgcgggcgtggcgaagatcgctgcgaccaccggcatgtcggaggaagaagtcgaggcgctggtgcgcggtgaggccgagcgttacccggagctgggcgagtacatcgaccgcatggtcgagcacatcaagcgcaaccgcgtcagcactcagcgcttcgttccgcatcccaacgcggggcagcaaggcgtgccgcatgggctgacgtgtcagcttggccggtcgcactggaccacgccggacggcaagatgtattccttcagcgagtcaccgtccccggtgttcatcgccaacaagcccgcgagcaagggtggctgtgcgcagtcgttctcgcccacggaaatcaagaactacccgatgcaaggcaccggtggtgaatgggccaaggcggcgatgtacgtcagcctgcgcgccttctaccggaagtacgtgaccgaaccgaaggaatggttgggccgtgcgttgctcgtgaatcaggtgcacgatgccgtctacgtggatgcacacggcgacatcgcaaccaaggccgctgctctgctgcacgcctcgatgctggaagcgtcggtgtatatggagtggtggttcaactggacgctgccgcttggcgtcccgtgtgaaaccaagatgggcgacaacatgatggaggagaagaaccctcccgcagagttcgccggtctggtcatcgagtaccgcgcgtcgatccgcaaggacttcgtaggtaatcacaacccgtcgtttgaataaggagaacaacacgcatgagtcttgacgcactgttgaacaaggtcgccacgcagggtaaggatcagtcggtcgccagtggtggcagcttcgactacaccccgcccgctgccggtgtgaccaccgcccgcatcgtcgggtactacgagctgggcaagcacgagttcgagttcgagggcaagaagaagacgcaggatgaagtcgccatcgtgttcgagctgaccggtaagcagcacccgcacatcgaaaccgacaatggtccggtgccggtgcgcatgacgctgaccctcggcctgtccaccaacgagaaggcgcactacttcaaaatcttcagccgcctgcgcaccgaggagcgccacttcgtgcagctgctgggtcagggtgtgctgctggaagtcatccacaagccgggcaagcgcgacccgaacaagaccttcgccgaaatcgacaaggcttccatccgcaagccggtcatgccggtgccggaaatggagaacggcatcccgaccggcaagttcgtggacaccgtgatcccggtgccgcagcagatcaccccgctgggtgcgttcgtgtgggacttcgccgacgccgacatgtgggacagcatctacatccccggcgagtacccggagcgcaaggacgagaagaccggcaaggtcacccacgaggcgcagtcgaagaacaagacgcagctgcgcatcgctgcggcgctgaacttcaagggtcttccgtgctacgactacgccgccgccaagttggcgggcagcaccacggtcaccaaggaaggcgtcgatgcgctggacgaagtggtcggcgacgtggcgaacgccgcgcccaccgacgctgctccggccgacgacaagccgccgttcccggtggacggtagcgacccgatggcaggcatcgcctgatggacctgagcgctctcatggcagcggccggtgagcgctccccgatgccggtgcaggtggtacgtcagcacaacccgcgcgtgatcgctcacgttgatggggactacatggcgtacttcgcggctggtagcgagaactgctcggcgggggatgcacgacgcaacgtgctctcccgctgcgcacagctgaagcatgtcagcggagcgggcaagatcgtcatgcacctgacgcacgccgcgtctaccaagggtgatcgcttcctcgctgctaccacgcagccgtatcagggtcagcgccaagcaggccgcaagcccaacaactgggcgttccttcgtgagtggatggagacatacgagggcgacgctttcactcccaaaatctggctgacccgtgaggccgacgatggcatcgcgtacgtcaacgagggtgcagcattgcaccacaacatcctgcacgtggtgcacagcgccgacaaggacatgcgaatgttctgcggcgtgcacgtagactgggacggctacgacatcacagaggttccgctcggcgcttacgacatcgttggcgagaacggattgcagtacggtcacaagtggttctggatgcagatgctccacggcgacaccgccgacaacataccgggtctgccgaaggtgggcaaggtgacagcggagcagctgctgttcgagacgaagaccaacctcgaagcggtgcagatcgtgagcggcaagtacagcgaagtgttgggtgccgactggcgcaagacattcgccgagcaagccgtgctgctgtggatgcggacggatcgtgacgcagaactgctcgacgtgctgaagctcgacgtgttcgggccgaagctgaagcaggcgttctatgacctcgccgaggacgtgaacgagaagcgtgcaatcttggaggcatacaaagcatgaagcgactcactgcaacacaggtcaagctgctgcgcatcaagctcgcagcggagcaaggcaaccggtgctgtctctgtcagggacagttcggcctgaaggctccgctcgatccggtgctggaccatgaccacaagaccggcgctgtgcgcggggtgctccatcgcggatgcaactccctgctcggcaaggtcgagaacaacgcaggccggtacggcgtgcgcgacgtgttcgcattctgtgcgggcatccccaactacctgcggtcgcacctcaccaacatcacggggtacctgcatcctacctacaagaccgacgacgagaagcgtatcgctcgcaatgcgaaagcgcgaaagcgtcgggctatcaacaaggagacaccgtgacccttacccagttcattcgccgagcaccgaagcgcggcccgaagattctctgcctcgacatcgagacgttccccatcgagttctatggctggggcatgttcaacaacaacttcagcgtcaagcagatcaagcgtgactggtcgctgatgtcgttcgcttgcgaatggctggacgacgaggcgtcgttctacatggaccagcgcaacgtgcgcgacgtgttcgatgatcgcaagcagggcaaggcgctgtgggcactgctcaacgccgccgacttcgtgctcgctcgcaacggcaagaagttcgaccttcgcaagatcaaggctcgcctcgcaatcctcggcctgccgcccgtgtctccggtgcaggtgatcgacccgatgctgctgaaccgcaccgagttcgccttcacctcgcagaagttggagtacaccaccggcgtgatcgtgccggagctgcgcaagtacgaccaccacaacttccccggcttcgacctgtgggtggcctgcatgcagagcctgcccggagcatgggacgagtgcgaagcgtacaaccgcatcgacgtgaagtccatgaagttggagtacaagaagctgcgcggttggtactcgcagcatccgaacgtcgcagtgtactacaaggccgacggcagcgagcaccgctgcaacaagtgcggctgcaacgaaatgatcccgcaggatgatccggcccgcacgcaggtcggtacctacctcctgcttcagtgcaccgtgtgcgacggctacagccgtgggcgcaagctcacgaccagcgccgaggcgcgcaagcacatcaccgtcccggcataaggaaccgacatgaagatcaccgacatccgcagcggcatgcgggtacagtacatcggcaatgcgcccgcaatgatcgggctgcgtggacaggtaagccgcgtgttcgctcgtgatgtcgaggtcttcttcgacggtcgagttaagccgagctgctgcgttcccgattccctccgacagcttctcagcatcggaggcgtgaccaccaccagacgagaggtaccaatgcccgaactgagctaccgcgacgaggaccgtcgcacactgtccgaccgtggcgtcggcctgaaggatgacgggggcaagccgcaggcccgtctgctgcatgagggcgtgccgcgtgcactggcccgagtcatcgacaccctgaccttcggcgcgcagaagtacaaagcgcactcgtggcagcatgtcgagaaggcgctcgaacggtatcaggacgcgagctaccgacacgacaacaagcgctgcctcggcgagaagctggacccggagacgggcatccaccaccgggcgcaccacatcatcaacgagctgttcctgttggagctggaactgcgcgaggaggagaaggccagtggcgcagagtaaggcgcgctccatcaaagaggcttgggtgaacatcggcatcggctacagcatcaactacgcagcgaacatcgcgctgcttccggtgctgtggcatcccgagcatccgctgctgtcggcgcacgccatcggcattgcgttcacagcgatcagcttcatccgccagtacatcatccgccgctggttcagcaagggtgactgatggcctgcgcccgctgcggccaagtgcatcggtacgtcccacatgaggccgagtgggcgcgcttcctagaggagcaccgtacccgcaagcagttcgatgtcgagtgggccaactcactctggcatcgtacataccctgacgacgcattctgcatcctcgtgatgaggggcctcgcaggtttcgttccattcccgtcgaaggagaactgaatgctctacaagaaccagaccgccatgctcatcaagtcctacgagaacgccgttgcgtggggcgagagtgccgaccacgaggaggcattgcagaatgcggtcaaggccgggttcccgaacctgcccgacgaagatcaggccgagctgtatacccgcatcgccgatgcgtgggaaggctaccgtggttcgctcgctccgcgcaagctgtggatcggcaccatcgtcaaccagttcatgtcgtcccgcatcgcacggttcaacgccgcgctgggtgacggcaccaagaaggaggacagcgccgatgtttgatgtgcctcgccagaatgtccgggttgctcccggctacaagaagcgcaagcgcggcttcaagatcaaccgcgccttcaccaagggcaacttccgcgtgcagtggtacgacggcaaggccacgtactgggagcgctacgttccgtggtacgaagtgccgctcgccatgttccagatttggagggactacgcatgagctacatcgtccacaaggcagtcgagcaggacaagatcaagaagaagctgcggcccaccgaggagcagcttcgcaccgagtacatcgcacagccgaagtacgacggctgcaacatggtcgccatcaagcgcggccactgggtgcccacggtgaacaagggcctgcatgccatcaaggtgggcgacgtgcagatgcagccggtggatcgtggcgtggttgacctgttctcccgcaccggtgagcaggtcgtcagcgcacaccacatcgagaacgctctcgcatccgcgccgttcttcccggtcggcgtgtacttcggcgaatactggcacccgcagatcgaccagcccaccgtcagcggcatgttccgcaagaaggacggcacgcagtacaccgagccgatgttcgtggtgttcgacttcgtgacgctggaagaatgggagcagggtttcagcgacctcgtgtatcaggagcgcgtcagccgcctgccgagcatgggccacgccatcgccgagggcaccgcgccggtgttctacgccgagtcgcagggcttcctgatcgaccaagagctgggcagcatggaagcggcgaagctgctgtgcgagggcggcgcgtacgacgggctgatcctgcgcaagccgagcggcaagtgggtgaagggcgacaagggaaccaacggcgaagtcgtcaagatcaagccgaccctgacgctggacctgcgtgtgctcggcatcaacgaagcagtcggcgagaagaccggccgcgccgtgtacacggtcgtcgttgacctcggagaaggcaagacgcaggaggttggcagcggcgtgccgcacagcgagagcgagctgcctagcgtgggaggcatcgtggaaatcgaggcgatgtccttcagcaagtacggcctgctgcgcgagccgcgatacaagggcatccgtcacgacaagaaggaggcagacctgtgagcgtcgaggtgcaagcatggcacaacatggagcgcgacacggtggagctgcgcatcagcgttcctttcggcgagtacgccggttccctgtggccgaacgagacgctgcgcgacaaggtgcaggaagcgttcgccaagttccttgacgagcggaggggctgatggacgcgatcactttcgagaagccggagctggacttcagccagtcctcggcatggatgggccgcgtcgaggtttcggtgcgcgcccggtacggtgccgacttgttcggcgctgctgccacgtgcatggccgaggatatcggcggtgaggcgtggccgcacatcatccacgacctgcacatggaaatcatgcgcggtatcctgaaacgctacccgccgcgcgactacaccgtgcggcagcaacggaggtaacaatgctctcgcaagtggaactcgaactggaaacctacgccttcggtaaggagcgcatggagaagtccatcgcccgcaacgaggagaagggcggcgcggacaacaacccctacgcccaagcagtgtatcgccggttcgtgcttccgcttgcggagcgcatccgtgcggacatcgactctccgcgaatcggccgtgcgcaagcgcacgtgccacttctgcgcgccaagtacgatcccgagcgtcagaacaagcgtggacagcccgtcagcgccgaggaacaggcacgcgagtggtacgaggctgtggccttcgtcgccgttcgcggtgcccttacctcctgcatgcgagacaagcacggcgaaggcagcgaccgcgacgtgttgaagaacgttggcatcaacgtgtaccatgagtacctgctgacgcagttcgccgacgcggagccgactctgttctaccacctgatgaacgacatggaccgcaagctctctgtcaacgagaaccaccgcatgacggtgatgaagatgcaaggacgcaagaacggcatcgagttcgtggagtggggacaggcacagcgcgatcaggtcggcgcgtacctgtgcgatcagcttgcgcagctgggcatgttggagattggcgtggtcaccgagactgctgccagtgcaggcgcagcgtaccgcaagttccagaccaagacgcacgtcaagatcgtgctgaccgacgaggtgcgcaagctgattactcagatcagcgacttcgtgatcgaggccacgccgttctacctgccgtgcgtcgagccgccgatggactgggtggacatcgacaacggtggattccacacgaaggaaatgcgccgactcaatccgtggatggtgaagacctacgctcagacccgcgacgagtaccgcgctgccgagctgcgcaacgagatggctgcgatcaacgcattgcagcgcgtgccgtggcgcatcaacaagcgactgatggaagctgtgtcggccatcgccaaggtgcacgacatggaggaaatcatttctcagggcgagctgccgaagccgcgcaagccggagtggctgacgaaggacatgaccaaggaaaccatgtcccacaatcaggagttggagttcaagcagtggaagcgcgacatgtccaactggcacaccgacgagcgcctgcgacagaacaagggcaatcgtttctacaacgcaatgaaggtggcgcgcaagttcgccgagtacccgagcatctacttcgtgtacttcgctgacttccgtggccgcaagtacgttcagaccaccggcgtgtcgccgcagggttcggacttgcagaaggcgctcttggagttcgccgatggcaagccgctgctgactaaggacgcgaaggattggttctgcatcacaggagcaaaccgatggggatacgacaaggcgtctctgccggatcgtgtgaagtgggtagcggagcatcacgaccagatcatggcgttcgctgcggacccggtgaacaacgacgagtggaagaccgccgacaagccgctgcaatttctgagctggtgcatggagtacgagcagtggcaagtgttcggggatcgcttcctgagccgcatcgcagtcggcatggacggttcgtgcaatgggcttcagaacttctcggcgatgctgcgcgacgcagcaggcggcgtggcgacgaacctgatcccagcaccgctgccgaatgacatctaccagatggtggcagaccgcgtgactgccgtcctgctaggcgaggacgaggatgccgaagggtaccgcacgctgtggctcgaccacggcctcacacgctcgctggtgaagcgcagcgtgatgaccctgccgtacggctcgcggcagtcctcgtgggcggacttcatcatcgaagactacctgaagtgtgggaagttcccctcgctcgacaaggccctgtacggccccgcagcgcgcttcctgagcaagcgcatgggtgaggccatcgccgacaccgtggtcgccgcagcgggcgcgatggagtggttgcagcgcggctccgggtcgatcctcaaccaagggtacgaccgcatccggtggatcacgccgtccgggttcccggtggtgcaggtctactgggagtccgaggagcaccgcatcaacaccaagctgtgcggcaacgccaagctgtccctgcgcaagagcacggacgcggtgaagaagtcccggcaccgcaacggcatcgccccgaacttcgtgcacagcctcgacgcaagccacctgacgctggtggtcaacgcggccaaggccgaaggcatcgacgccttcgccatgattcacgacgacttcggcacccacgccgccgacagcgcggcactgtaccggatcatccgggaggtgttcgtgtcgatgtacgagcggcacgacgtgctgtcggccttccactcggcctacccgttcctgccggagccgccgccgatgggcgagctggaccttcggcaagtccttgattctccgtacttcttcagctgacggagtttcagtacacctatagcacgaggcaactgaggtccggttggagcggccgcgaaggtaagcggaaccggtgccggaccttttggtacacctatagcacagaggagacaccatggccgaagacgccaaagtgaaagtcctgatgacgctccacccgaaccagctggccgccgtgcggaagctgtccgggctgtcgctgtccgtcaactcgaataccacgcccttggaggcaggtatgcagttggggatggcccgcgtcctgaacatcttacaggagggtttcaccgttgattcctccgtaccgaacaccaacgacgggtgatagtgagcagatcaaggcggctttaacggccgctttgtatctgtcatctagagaagatagtaaggtagacaacagagaatcttctgtgagctacaactgtgatgaccctgattacacagtggccctgataacacagggtctagtggatgcagtaatcattgatgaagcctacctgctgtgctttgccattgtcacaccgtggtactccaagaaccgtactacgttcgttgagaacatggtgctgcgaattgggccgggcagttccttcgaccggtacatagccgtgatggaacatctggctgacatcaaccactgcgactcactgagcgcaggcggtgcactagctcggaactcccgagcactcacacggatgtatgcacgctacggctacctgctggaacggcatgctccccaattcaccaagcgaaggagttaacctatgggtagcatcgttggtggtgggtccgccaagcgagcagcgctgaagcaagctgctgctatcgacaagcagaccaacctccaaactcaatccacgaactaccagattcaggcgatggccgatcagatggcacaggcagctgcacagcaggccgcatctgagtacgccgagaagttgctgagtgcccccgtcgataccgtcgatgtgcggctgggaacttccgacctcgacttgcagactgccgacctgatcggccgacgcaagaccgcccgctccacttacacccgacccgtgaccacgaccgcagcttcccggctgacgaccgtggccgggtcagacctgttgtgaggtgagcatggaccatccgatccaaaccgctcaccgccagttcgaggcttacgacaacaagcgacagggcatcatgtaccgactcgaacgctattcgagctggaccgtgcccaagctgttccctcgcaagaaccgcgatcaggacaccgagccgctgacccacgggttccagtctctcggcgcgcaggcagtgaaccatctggcgaacaagctgatgatgtcgctgttcgcaccgtcccgcccgttcttccggttggagctgaagcgcaaggcgaagcaggctgcgcaggagcaaggcgctgacttgcaggccatgcaggcgatgcttgcgaaggccgagcaggatgccagtctcgaactggacaagcgctccatccgctcccggctgtacgacctgctgaagatgctgatcgtgctgggcaacgccctcatggtgttggagaaggacacgatccgcgtgctcaacatgcggcactacgtggtcaagcgcacccgcaccggcgaggtctacgaactgatccttcgggagaaggtgcacaagacccagctggaacccgcagcgctcgctgccattgtcgcgcacccggacttcaagcccgatgacgacggcatggtgtgggagtacaagtgggtcaagctggaccacaagaccggcaagtacaacgaagacgtgtggatttgcaactgcaagctgcccgccaacttctcctcgacctacaccgcagacaagctgccctaccgggcggttagctgggacttggccgcaggcgatgactacggctccggcttggtcgaagactacgaggccgacttccagtcgctctcgatgctgtccgaggccgcagtgcagggcgcgatcctcgcctccgagttccggtggctggttaaccccgcaggtcagacctccgtcgaggacttcatggcgtcgcccaatggcgcggccattcccggcatgaagggtgacatcgagctgattaacgcaggcgtcgatggcgtgctgcaaaccaaccaagcaatccagtccacctacatcaaccgcatcggcgcaggcttcctgttgcagacggcggtgactcgtcaggcggaacgtgtgaccgcgcaggaaatccgcatggtcgccgaagaactggaaggcgggctgggtggcggctactcccggatcgctgcggacgtgcaggtaccagtcgccttttgggtgatgaacctgacgggccgcgacatccgaggcaaggacttggagcctgtcatcatcaccggcttggccgcgctctcccgtacgggtgaccgtgaccggctgttggagttcggcagcaacctcgccaacgtcctcgcactgccgccgcagattctcgaacgactgaagctgtccgcgtggatcgcagacctcgccgccgctggtggcttggacccgaacgtctacgtgctgactgaggccgagtacggccagatgatgcagcagcgtgcacagcagcagctcgccatgcagaacgcatcccagcagatcgacaacgccaacaacatggagacacagacacaatgagttccaacgcacctccgggcggtggtcccggcgcaaccgtgatcgcaacctcgaacggcaaccagcccgcaccggcagctccggctcccgcagacgacaagctgttgcccaacggccagcccgctccggccgcaccggcacagcccgcagctcctgctgcacctccggctgctgacgcgctgagtctcgaacctgccgctcccgcacagcccgccgccccggcgaacgctgcgccgactgcggtgtcgatcccggactacggcgacaacggcctgaacatcgcggccgaatacttcgtcaacaccgtgggcctcgacatcgacagccgcgaactgaccgaagcagcgaagggcaacttcgccctgctggaagccaagctggaagtcctcggcgacaaggccaagggttccgcaccgatcctcgctctggcgaaggagagcatcgctcgtgtcaccgccgctgcaaccgcagcgcacgccgcgaacgttgctgctgtccacgaagccgtgggtggcgcagagaactgggctgcgatccagcagttcgcacgggccaacctgcccgccgaccaactgaagcaggcaagcgaatcgctgtcggctggtggcttcggcgctcaggcgaccgcgcgttacctgatggctctggcacaggccaatcccgcgacgaccgtcaagggcgcaccggctaccaacgccgccgcccccgccgcgtcgatcaacggcgtcgctcctatcacgaaggagcagtaccgcgctgagtaccgcaagctggttgccgagaagggcatccgtggtgcggcccactccgaagaactgcgtgcactcaacgcgcgcgtcatccactaagaccaaggagcaacacaaagcatgagcaccatcttcccgactgtcccggttctgccgaatcaggtcaaccagtccggcaacgagaacgccctgatcctcgaacagttcaccggcgatgtcgagcacacctacgtgtccagctcggtgctggaaaagttcttcccgcgcaagcaggtcaagggcaccaacaccctgaccaagaaggccatcggccgtaccaagcttcagaagctgaagcgcggtgacgcgccggacggcaccccggtggacttcagcaaggcgtcggtgaccgtcgataccatgctgctgtcgcgtcacagcatctggcagctggacgaaatcttcaccgacatcgacacccgcaaggaaatcgccatcgagcagggtcaggaaatcgccgagttcgtggacctgaccatcagcatcgccgccgcgaaggccgctgctgccacgcagtcgatcttcacccgcaacggccgcgcgcccgagggccacttcggtgccacgcaggtcgtgctgtccgccgctggtgacgagaacgatccggccaaggtgtacgccgccatcggcaaactgttctcccgcatggaggaggagaagaaggtcaagccgcagcgcgatggcgtggtcctgatcgtgcgcccggcgatcttctacctgttgcagcaggccgagcagatcagcaacggcgagtacctgacctcggacggcaacaagctgaccggcatcccgaccttccacggctggggcgtcccggtgctgtcgagcgagaacctgccgaacaccgtgatcgaaggtcacctgctgtcgaacgacgacaacgacgacttctacgacggcgacttcagcaccctgatcgccgtggccgtgtcgccgaaggccctgctgatcgccgaagcgctgccgttgcagtcctcggtgtggtggagcgatgcctcgaagtgctacttcgtggactcgtggatgtccttcgccgttggtctggatcgcgtcgagaacgcgggccgcatcgacaaggttgcctaatccgctgggcgcggtccctgaatccttcgggtaactcaaaccgcgcccttcttccaccaacacaggagcaacatcatggtctttgaccgaccgttcgagatttccaaccgcgtcgtcgccgcaactggcgtggccggtctgcccgccaactccgttggtaccgtcgtcggcgtccactacgacacccgtggcaccgcaggctgggtcgtccgtgtccgtttcgtggacgacgaaatcggctcgcaggacatcgagtacgcaccggccgctctggctctggctgcggactaagcaacatcccggcaggggcgctccggcgtctctgccttgttcctctcaggagacaccatggcattcatcaccaagctcgacatcgtgaacgcctgcttgaagacgatgggcgagacgaagctcaacacgctggaagatgaccacgtatacaaggacgacgccgttgacttgatcgaccgcgtgcaccgtgacgtgtcctcactctcgctgtggttcaacaccgaatgggtggagctgaagccgcaggcaacgagcaagtacatcatggtccccacggacgtgctgaagctggactgcaacccgagccggttcggccacgtggtgcagcgcggacgccgactgtacgaccgcaagcgcaacacctacgagttcgaccacaacgtgcaggccaagctggtgcggctgctggacttcgatgacctcccctacgaggtgcagatgttcgtgcgcgacgactcggtgctgcggttccagtctgacttcgacggcgacaacaccaagtacgccaagatcaagcagcagcgcgatgacagttacatcaacttgaaggccgagcacatccgccagatcaaggcgaacccgctgttcgctcgcgcatccgtggacgtgctgcgttcccgttactggaactacagcggtcacccgtggcacagccacgtcacattccccggctaaggagacaacatggcaaaggcaggcggaacctatcccgacatccttcagggtgtcagtcagaaaccggcgcatcgtcgtcggccgggacagacgcacgagcagatcaacgtgctgtccgatccggtgaacggcctcgtgcgccgtcgtggtacgcggttcgctgcttcccaagccgttgtcacctcggccgagctgcgcaacatggacgtgttcgacttcatgcaggagggcaaggagtacgcgctgctgtaccggcgcgacgcctcgaccttgggcagcgagtccttcgcgttcctctacaacaagacggacgagtcgttcatccctctggtgtacgagaacagcacgtgggtcaacacgctggtcagcggaggcgcatcgtcgctcacggccatcggcagctacgtctacatcgcgggcaacaccacgatcccctcggccaccagcacgaacgtgtggcaggagcagacgaacatccagcgcctcgcagcatgggtgcgcaccgggaagtacaacaccacgtacacggtgaacctgacgcggacggacaacacggtgctgacggtaacgttcaagacggttaccgcatcgtaccccggaacgctcgacaccagcgacatcccgttctaccttcccggtggcacggagccggacgcggcgtaccagaagtacgtcaacgaccgagtgaacgagtacaactctgcggtcaacgagtggatcgtgacgagcgctgagcagacgcgcccggagtacatcgcggagcagctgtcggatttgctggtcgatgcaggcgtgtcggcaacgtacatcaagggcgggatcatcattgacgatgaccagttcaaggacatcacggttgacgacgagggagacggcacgaccttctacgccgcagggcaggaaattacagacgcgacctacgccgtcaagttccactggcacggcaaggtcattcgcgtgcggccgagtggtgcaggcgcggacgagtcgtactacctgcgcgctgagttggagaacggcgagacttccggctacgggtcggtggactggtacgaagcgcccggcgtggagtgcaccatcgacaacctcgtgtcgcagctctacatctacaacggtgtaggctacatcgcacgcaacggtgcgggcctcacgtctctggctccgagcagcggcgagcatccggcctacggtgcgcgagtggcaggcgatggtctgacctcgccgatcccgtggttcatcgacaagccgatcacgatgctgtccgtcttccaagaccggctggtcatcggcgcacagaactacgtcaacgcctcacgctcggcggactacctgaacttctggcgcggctcggccgtcaccatcgaagacagcgaccccatcgaaatcttcgcgcacggcagcgagggcgatgtgctccggcacgcgacgctctacaacggcaacctcgtgatcttcggtgaccgtcagcagtacggcatcagcggcgactcggtgttcagtccgaagaatccgctgattaaagcgttcagtgccaacaaggattcggttgacgcgaaggcgcagacctcgggcaactacatcttttatgcgcagtacggcagcgaaggcacgagcctgcaccagatgcgagtgggcgcgctcaacgggcagcagacggtgacggacgaaatgtccaacgagctggactcgtggctgtcgggcactccgttgcagatcaccccgctcactgcgccgaacctcgtcatgttccgcactcgcgagcacccgcaggacttctacctgtaccggtacgaggacaacaagaacaacgggcagcgcatcgtggatgcgtggtcgaagttccggtaccacccggcgctgggcgaaatcatcggcgtgagcagctacaagaagaacggcctcgtgttcactgcgcgcgggtcgctggtggcgtgcgacgtgttcgacccgaagggcgagccggactcgcatgcgtgcctcgacagctgggcgagttttggtacacctacgggcgtacagactgcgagcgcaagcatcgccgtcaatagcactagcccgtacttcctgctgggttgtccctacgcgcaggcgtctgacttccttaaccagttcgatgacctcgctgctggtgcgctggaatacggcgtggtgtccgaagctctggtgatcccgaccaatccgttccctcgggaccagaacggtcaggccgtactcgatggacgcatgtccctcaacaaggtgacggtggacgtggagaacacggcaggcatgatcgccacggtggcaacccgcaacagcaatgtgaccactacggacttcgagggccgcatcctcggcgactccgacaatctgatcgcgcggcaaccggtgtaccgggggcagctcaacatcagcgtcgggcgcgaagtgcgcgagtgcacctacgagattcgcagcaaggattggctcccgctccgggtgaccggcctgagctggacgggtcagactttcaacaatgtacggagggttagctaatgggttcggttaatacgatcctgcaagcgaacaacaccacccgcgttgcccgtgcgaactaccgtgcagccgttgcgcagaccgacaaccagaaccgcagcgaggtcgccaagaccggcttcgctgatttcatgcggtccctgaagaacaacgcccaactggacgccgccgcgaaggagtacaactccaacatggaagcgctgtccgaggagctgcgtgcgcgccaaggggctgggcttaactcccagctccaactggcgaacgcgcgtggcgcacttcaggcgcaggctggtgctgtcggtgtcggcggctcgtccgcagacctgatggattcgatggtgcggttgcaggcggaaatggatcaggagacgcaggccaacgctgtctcgctcctcgcctcgcggggcgcatcgcagactgcgcagatcatgtcgcgcgcgtggaacgggatggacatgagccgttcgttcgggcagttcgactactcgcagcacatcgagccgcaggcaatgaagcgtcgcttgggcaagctgatcggcgtggccgtggctacctacttcggtgggccgatggcaggcgaggccgtggcagacttcgcggtcggcacgtggcaggcggacaacggcaacttcactggtgcctctcagtccttcagcaacgcagcgcagaacggtatgcaggcgtggcagcagtccaatgatcgcggcggcaagtcgtgggcgtccactaccttcgggtacaacgacggcaccggcaagcagtccgtgactggggcgaaggtcaccggcaacttcggcaacaactacgacaacttctccaccactacgtccggcctcggctggttcgatagcggcagcggaggcaactcaggaggtgcatggtaatggctgacatcggcacggttaccttcaacacgcagtccgcattgcagggtggcatcaacgccaccccagcactgtcgggcaacaccagcattcaaggcgctggtgtgaatcaggtcgggccggttcaatccggcaacgactggttcgcaagcactggtggtatgacgatgccggacagcaacctgccagagttcttgcaggagctggcagcgccgaacaccgccaagctgaagcagcagcagatgtgggacggcttcgttgccgcccgcgctggtaagaccatggacgagattgctgcgaccgaaccgtggtacaagaaaatcttcggagacaccaactacgagattggcgcgagcatgtataacacgctctcgcaggtcaacgaaatggagagcgacttgcttcggcgtatgccggagttgcgtcagcttcctcccgaggcgatggcgaaggagttcaacgacctcgccactgcccgcatgaccggcaacggtttcgcggacacggtgttgcagaagaccttcatggatcgcgcgggttccctcatggacctgcacaccaaggagcgcacggcatggcagcagcaggagctggtgaaggcgcagtacgctgcgaactcgtcggcgtccaccggcttcaacgaactggcgaagcgcacggcgatgctcggtaccaaccgtcccatggacgagaaggccaccgaggcgctgacgcaggcgcagctgtccctgctggacggactgtcgccctcgcgctaccagacggacgagtcgtacaagtccgcgatcactgcgttctatcgtggcgctgcggatcgcggcgagttccacacgctgaagttcctcaacagcaagggcgttctgaacgccatcgacccggacgggcagctgggaatccagcagtacgtgaagcaggcgcaggatcgttaccgttccgactggctcgatgccaacccggagcaggccgagaagatggcgctcgtctccatgtacgcatcggagggcattggtgccaagccgtcgcaggcgatgatcgaggaaatgaactcgacctacgccgccgagactggaagcgacgcaccgctgtactccggtacgcagttggcttcgatcatggcacagtccgcaggcgcgcacatccgcgcacaggaagccgtcatcaaccagcgtaacgctgcggccaaggccgcgctgaccgaccagcagaagctggccgcgcaggaggaggacatccgtggtggcatcgaagcgttcaagcgcggcacgtacgcgcagacgatcaacatccccggcgtggacaaggagctgatcgaggcgaacacggtgcaggcatggaatgccacgatggccgcgaaccccaaggtcgccatgtcgcagctggtgtggaacgccaacaccgggcgaggcgctgtgctgaagggtgtggccgaccagttccagaccacggcgcgcgctgtgctccgcgatcagccgaacacggcagcggctgcactgtaccagcagtggaaggaactgaagcagaccaccgccgcacgcatcgacacgaacggtcagcccgtgcagggccgactgactggcgcgactaccgctgcgctgtacttcggagatagcgtcaacacgttcttcaacaagctgcaagcgttggagaatggtggcgtgaacttcgagcttgcttacgaggtggcccgtggagaaatcaccaccgacgatccgacgcagttcgacgcgaacagccgtaaggaatccgaggctactcaggctcgtgttacggaagctatcgccaagctcaaccccaagtacctcggcatgttcggcaacaagctgggcgactctggccgcgctgcgtatgctcgcgccatcgtccgctcggtcactgacaccggtggtctgctggacacttctgcggaaggcttgcaggctgcggctactcacgccaagctggcctacggtctggaagacgcaggcaagtacgcatgggaaaacggacgcgacgacgaaggccgagtgatcggcagcgtcggtgcatggctgggcttcatggacacgaaggaaaccggacccgccatcgagaaggccatcgacgcagcactgcgccgggtcaacatcgagccgagcaccgggctgaaggctgacgtgttccgcatgaaggacagcgagaacggcgagccggtgctgtacgtcaacgctgttggcgagaagggctggaaggttgtgccggtgtacgggcgcgacatcaaggacgagtacgagaagcacaccaagcagcagcgtcagttgcaggccccggtaccgcagggctacgttcgcatgaacgacggtacgattcagcagagcatttccatccaacccaaactgtaaggagatagacaatggcactcgatctttcggggctgacccaagaccagcagattgccaaggctgccgcttatgcgggagtgccggagtccatcgtgcgcggtcagtggcgagtagagtccggcaacgggcgtgccgccaaggacgctgacggtgtgatccgcagcaaggcaggagcacagggcgacttccaagtcatgcccaccacgcaggcaacgtgggaagcgcgcaacggtcgcaagtacgacatgcgcaacttccaagacagcatcgagctgtatgccgacatcatgcgcgagaacatgcagcttgccaagggcgacgtgacgaaggcgctgcgcatctaccaaggcggcaccaatccgaagaactgggggcaggagaacgcagcctatgcaccgagcgtgctgggcggtgcgtccgctcccgcagtgtcggcgcagccgcgcagcctgaccaccacgcaggcagacctcaacgccgcatggcagggcaacccgaacatgcgcgaccgtacgtggtccggtgcgtccatcccggatgcgtggacgggtgcgcccatcgaaggccgcaacgctctggcgtcggcagcgaaggaacacatcggcaagattcgtgcgggcatcgccgagctgtcgatgggtcaggtagcacaggaaggtggcaccgccgcgcaggccgtaggcaaggctcaggctgtccgtgcatcggatcaggttgtgccgtggtgggtgcgtcaggaagtggacgtgctgaacaccggcgctcgcaaggcgctgctggatcagaccgaacaggcgctcgcgcaggaccgcgcggacgaggagctgcgcaactcgctgaccttcctcgacaagtggggcgctgcgttcgacagcggcatcggtgctgcgatcagcaaccagtttgcgcgcgaggacgagaacgttccggaaggttggaagtacgacccgaaggaatgggagaagccgtggatgactgccgacgaactcgaagacatccgcgatgcagcgtactcgccgaacgagctgaagtacgtcagcgaccgacagttcctgcgccgccactccatgcgcatcaaggatcagcagactggctggggtagcttcggttacgacatggtggcaggcttcaccgatccgggcaactgggctatcggcggcgtcactgccgcaggcgctaaggcgctgggcatcggctcggctgcactcgttgccgaagggcgcgtgggcgcgtcgctcgcgtcggctgctgcggagaacgcggtcggttccgtcatcacggacgccgcgctggttggcatgggcgagcgccgcaacttcgcggacttcatgaccgacgctgcattcgctaccaccataggcaccgcgatgcacattccgggcgtgcgctcggctgcgcagattcgtgacaaggcaaccatcgacctgtccgcaggcaacgctgccgcttacggcgaagcgtggtcggccgacctgaaggcgcgcgctgtggccgagctgggcgaggacgccaacccggtgctggtgaacaaccgcatccaccagcttgccaagcaggaggctgtggattggctgcgcgctggtatggccgacgtgcctgacgacttccgtatcttcgcccgtcccgacgtgcaggagacgaccaccaccgcaggcaccactggtgcactcgcacgggacgcgggcaacgtggacgcaacgaccgggcggtacaacgacagcgtgggtggccgggtcgatcagcatgacccgctgctggaacgcgcatggaagaccgcaggtatcaagggcggtaacgtcgatggcgtgctgaagtatctggaatccaacgcctctatcccggaggacgtgcgtgctatcgccaacgcgctgaagcgtggcgggcggctgagcacggtgaagatcgtgccggaatcggaactcgacaagtggttcgccggtgccaacatgggtccgggtatgcgtgtggccggtggctacaacgccggactggacgcgatggcgatgcggaactacacgccggaagtggtggtgcacgaaatgctgcacgctgccacgctgcgtgagctgcgcagcaactcggtgttcgggcaggaaatggaagaactgctgacccatatcaacaacagcatcggcagtgtggactccacgctgaccaccgctgcgatggagacgcgcatcaaccagccgcaggcaggcttcctcgccaacactgacgagctgatttcctacggcctgacgaaccgcgctgtgcaggcggtgctgcgtcagatgcccgcgccgggcaacacccgcccgaatgcgtgggagtggctgaaggataagatcgcgcgagtgatgggtctgaagaatcaggagtccgcgctcgaacgcctgatgtcggtcgtcggtgacaacctcggcgcggaagtgcgcgacacgcaggccggtacccggcagacgcgtggcatgctcgccaactcgatcttcaagtcgaaccgcgagcgcaaggctttctaccagcgcaccggtctggacaagtccgtcagtgatgacgcgatgcgtgtgcaggtcgccgaagtgatggcacgctccgaacgcttcagtgcgcagtacggcatcgacgcggcgaagctgtccaccatcatgcagcgcttcgggctggaagctacgagcacgactctaatgtcgtccaagtcgccagttgcccgcatgcttgcgatcaccctgttggagaatcccgagggtgcagcaggccgacacagcaccgcagcgatggatcggcatggtcggtttgagtcgttcatgggcacccgcccgcgtcagtgggaagcggcctatcgcctgtggcgtgcggacgtgcgcggtatcggtgcgatcaaggacttcgccacgggctggaaggctcgcgcggacttcgagtacgcagtgaagctgtaccgcgagactcgcttcaacggcggggacatcccggatgcgcacgaggcagtgaaggcaatggcccgtgagttggaccgtggctacaaccgcatggcagcagagcagcgcgcggccggtacggtgggcgcacagcgtctgccggaggaggacgtggagggctacgagtcccgtacgtggctgggcggcagcatcgctgctgctggtccggtgcgacgcgagggtatccgtcaggcgatgcgcgatcagttcgaggtgatgggcgagctgtatggggacgacttcctcgataagttcgctaccaagtatctggaacgcatcgagcgcaaggctgcgggtgtcatcgaagcgccgggtcaggtcttctcggagtcgcaggcggacacgctgcgcgacactctgcgggcgatgtcgctcaacgaggaggagattcagaaggtcatgggcaagtacagccgtggcggtgcgaagcacaccaaggcgcgtatcgacctcgacgtgaccaagcagtacgaggacgctgacggtaagttccgtctgatggactatctcgacaaccgcgtgatggacaactaccgcaagtacgcgggacgtgttgctggtgacatcgctctggcgaagcacggcatcctcggcgacgcaggcatcaacgtggcgcgcgaagcaatgcgcctgaccggtgccaacgatgtggagctgaaggcgttcgagcaggtgatgtccgagttccttggtcgcccggtcggtaccggcgatccgactgttctggcgaatgcgcgtctgctgacctcggccatccagctgggcggcgcgggcatcaatcaggcagcggagtacagcaacggcctcgccgctgttggtgctgctggtgtggctgacgcaatccgtatcgctccccgcatgcgcagcgaaatcatgcgcatcctgaagggcgaggacagcggcaaccaaatcctcgacggcttcgagttcatcagcggtcgcggcttcggtctcgccggttacgacctacacatgttcaactcgctggacacgcaggcgtcgatgtatggtagcgagcgcgcaggcttcctgacctcgctggtgcagaaggcagcgcatgcgaaccgcatcctctcggggcagcgggccgtgcttgctgtgcagcagcgtggcttcgcggaagtgctgatcgccaagggcgtgaagttcctgcgtgatggtgctgaagctgacaccgccctgaaggacatgggcattgacgacaacctgctgaaccgcctgcgggctacgcaggatcaggtcgtgcgctggggcgcggatggtaagctggaagcagtagacccgcgcaacgtcgaggggctggcggatcggcaggcatggttggcgttctacaacgcgatcaaccgtggcacctcgcagattcttcaggacaccttcatcggcgagactggcaagtgggcgcacaacggctggctgaagctgctgttccagcaccgcacgttctcgctggtcgcgcagcagaagcagctgggccggtacgtgggcaactacggtgcatggcagacggcgggcctgatcgctgctgcgatggctgtggcggctccgctgcaagccctgcgggtgctgtcccgcgtggccctgatgaacgatcaggagcgcgacgaggccatcgaccagaacatcctgtcgcctctggcgctgggcaaggccacgctgaactacgtgtcggcgacgggtatgctcaacgatgtgctggacgtgggcactggcgtggcgggcggctggtacgagtacgccaccgatacgcagggtccgacgtggctgaagcagctggccggtgggcagttcggcaaccgcaaggaagtggtgggcgggcagttcgcgccgtcgctgggagtcatcaacgacttcgctcagggcattgctggcaagccggagaatctggccgacgtgattccgggcgggcgactgccgatggtgatcccgctgctgaagggcgcagccagccagtggaaggaggagtaagatcagggccaaggacggcccacccttttggtacacctatagcaaacaggaggcagcatggcagttccagacccgcagctgcgctacgcgacagacgtgttcgacgccgatggcgtgaccactgactggcagatcagctttaccggtggctacatcaacccgtcccacgtgtacgccatgagcggactgctggacgaggagactcagctgctgaccgaccggactccgcacaccgtggaagtcctgagcgaagacgatgacgctagtaccgtccgagtctcgcctgccgtcgccgctgggcgcaagctctacatctaccgcagcactccggtgcagcagatgctcgttgactacgttaacggtagcatcatcagcaagacaaaccttaacctcagcaacgaccagctcctgaagatcattcaggaaatgttcgactcactcaacatcgccacccttagcatcgaccagcaggtcggtgtgatcgtggacctgaacgagattatccagaacatctacaagcaggtcaccgagttgctggcagctggtggtatcgtgtccgtcgccccgcgcgtctggtccggtgcttggactggcgatcaggtgggtgacaccgacttcgacatggtgggcgcggacgtatccggcgcgggcttctacgacgtgtacgtcaacggcatcggcatgcagccggacgtggactatcaggtcacgctcgctgacggcaccgatcccagcttcatccgcttcgccacggttcctgccgagggcagcatctggttcgccgtgctgcgtggttacgccaagccctacaccgggcctgcgccgatcaccgctgcgagcctgcgggtgccgatcatcacggcagagggtccgacttactacgccgccaaggctaccgagtacggactcgtgcgctgcacgtacgccggaggttgcgccgtcaacatcaacctgatccccgaagtgggcgacggtgaaaccaagctcgcctcgggcagctacttcagcgtgcagcagaaggcaggccctgtggtcatcactggcgacgtgggcgtgacgctcgaagtcccggtcggctgcaccgccgcaactcgcggcaccaactccgtcatcactgcaacgtgcatcgacggcgacaccaacacgtggttgctctcgggcgacttggctaaggagtaagcatggctaatcacttcaggctgtacggccgaccgctcatggcggacgaggttgcagatggcctgtcggtgacgggcgtgctggaagggtacacggcgggcgaggcttacgagtctcgcctgtccatcaacaacccagtcggccgctgcaccgtggaggtcatcgaatcgacgctcccttcgggcgctgcggtacgggtggacaacatcaccaaggaagtcgtcgtcaagtgggcggctttcactgaagtcgtggacgaggaaaccctcgtgcccaacggcgacttcgaggcaggcgacgacggcacgtggttgccgggcggtggatcgaatggcgaaggctggtcgattggcactggctcagactacgacaccgacagcggcgtgtacagcgcgcgcttcgccaacatcaagacgggcggcagcgacctgctcaacccgctgatccctgccaaggtcaacgactacatccgatgcaccgccgaggtccagcagggcgcaagctccaagggcaaggccggtgctcgtgtgtcgatcatctaccgcaaggaggatgggaccgagctgcaacgcaactggggcaacatggtttcctccggcagcaacggtgcgtggcaccagtccgttgccgaaggcgctgcgcccaaggacacgaagtacgtgcaggttgtactgtcggcgttccgcagcaagcagaacaaaccgctgtgggtggacaccgttaagtggaaccacaagtacgtactgggtcagaacgacgacagctcctacttccttagcatcaaggtcacggacgggttgaaccgtgtggcctactggtccggtcgtatcgaggagcagggcatctacgttacgtccaagctctacagcttctaccagttcgatgccgcgatgctgaccagcagctttgctgggtacagcaacatcgacatgctccagcctttggatactgcgtcgctgggttcctccttcgtaagctgggaactccgaagctctaggcaggattatgccgccgacccggagagcacgttgtacgggagcgctttcgtttcgttcgacatccgatccatccgtaaggactacacgcctgacccggagacggcgaagctgtcgagttctttccattccttcaccctgaagcagcaccctgtagtcaaccagccgctcgacgcgactgcacgactccggtctggcttcgtatcatggagcttcgcatgatccacaatcacctcggcattgctggcgtgttcaccatcagcaagggtaagtccctcgatactctcgaagttgtagccgactggcagagcaaccttatcacggacggtggtatggacgcactgggtgataccggcagcggctatcctcgcagcatgtacgacctcattgcttacttggcagtcggtagtggcagcgccaccccggcattcaccgataccgctcttggtgcacaggtggcgcaggttggtcgtacgtcctcggacagcggtgggactaccactgccccgtactacgcctactcccgctgccagtaccagttcccggctggtaccgctactggcgttctgtcggagcttggtgccaaagcatacaacaacaataccggcgcgtacatcctgaccacccgtgcgcttatcaaggactccgcaggtaacccgaccaccatcacggtgctgtcggatgaaatcctcgtggttacttacgagctgcgcatgtacgcagataccacgccggttgtcactactgagacgatcaagggtgttagcaccactgttacctgtaagcctattgcaatgggccgcagcggcggtatgaacggtcagtcggcagtcgcttggtcggactacgtgtgggggtgctactacttctacggcggtactggcgacggcaccggagctatcaccgaccagtatccgccggggacgattgccagcttctctgacttgcagcttcagcaggtagcctatgttccgggtacttactaccgtgactgcgtttgccggatgtcgatcaacaacgtgcccggtggtccgatcacggctgcaatgggactctccgcgtgcgtgaccttccaagtcggcttcaatccgggtatcaccaagaccggatcggagacggcgaacttgcgcatgcgggtttcttggagccggtacacgccatgatccccactgtctcccaaagcatccaacgcggtgactgggtggagcagcagaatcggcgcacccgcccgctcattgacttcgagcagggcgggctgactctcaacgcagcagtggacgacctccaagctgcgctgtggactgccgagagtgacggcagcagcgtcgtcgtttaccgcgacggcgttgccccggtcaccgtgctgaccgactccgggatcacgcagatcgcactggccttcgaccagaccatgcgcccgcacgtggcgtacatggcgggcggtgtgtgcaagttctactggtacgacacggtggctgcttcgatgcagaccatggtgatccccggtgctaccactccgcgcctgtgcatggacgagaagcgggctgtcttcgccacgcagagcgacgtgctcctgtcgtacaagaacggcagcaacctgtgcgtacgcgcgcagcgtgagcgcttcgcaaccgaacatgtgatcgcctcgggaatccccggcgacctgattgcggtgggcatgaacaacgtcaaccgcctgcaatggaagctcgtcggcaatcccgacgactggccctaacctacaggagaacagcatgaccccgccgagtgtggtcaatgaggtcgtccgaacctcgccgcttacgctcggcgcggtctacctcaacttcatcagcacgtacggtgctgccatcgtaactacgctcgccattctgtacgccgtcgctcagttctactggcgggcacgcgagcaccgaaagatcatgggaggcaaggatgtcgaatccggcaagtgagggcgcactcggtgcgctgcacgaactggtcgcgcgtgcgctgatgcagcgcatccaagatggcgagctgtgcaccgcagccgacatcaatgcggcgatcaagttcctgaaggacaacaacatcacggcgacgcgcgaggccaacaaggcactcggcgagctggaagacgagctgggcaagcactcgctgcctccggctgacgacgacgagttgcagcgtgcactcgacaacatcgttcactttccggggagcgtagccaacaatgcgtgaatcagctgaagcggccgacgtgcgccgcaagaagttggagctgttgcagaaccactaccggcacttcgccaccttcatgcgcgacattatgaaggtgctggggttcgagccgacgtggatgcagtacgacatcgccaactacatgcagtatggcccgcacctcgcaatggtgcaggcgcagcgaggcgaggcgaagtccaccatcgctgccatctacgccgtcttctgcctgatccacgatcccactcaccgtgtgctgatcgtatcggcaggcggcacgcaggcatccgagattgctacgctgattcagcgcatcatcctcacggtgccgacgttggagtgcatccgcccggacaagaacgcgggcgaccgtacctccgtggatgcgttcgacgtgcaccactcgctgaagggaatcgacaagtccccgagcgtggcgtgcatcggcgtcaccggcaacctgccgggtaagcgtgcggacctgctgatcgccgacgacgtggagtccaacaagaacagccgcactgccgcgaaccgtgagctgctgctgaccatcacgttggagttctcggccatctgcaccggcaagcccggtactccgggtcgcatcctgtacctcggcacgccgcagaccggcgactccatctacaacaccctgcccggacgtggctacgacgttcgcatctggcccggtcgctacccgaccccggcacagcgcgagcactacggcccgcatctggcaccgtctatcgtgcagcgcctagaagccgacccgatgttggcgttcggtggtggcccgatgggcgacgagggccagtgcaccgacgagctgttggccggtgagcagaagcaccagtccgagctgcgtcagcgtggaccgtccagctatcagctgaactacatgctcaacacgcggctgatggatgcgctgcgcttcccgctgaagaccgagaacctgatcgtgatccccggtggtggcgaccgcttcccgctgacgatcacccgtggcctgagcaacgctcaccagcgcagcttccagtccagtgggtacggcttcgtgatgatgatgccgcacgacatgagcaccgagactgcccccgtgcagggcgtgcacatgcagatcgacccggccggtggtggtgccaacggagacgagacggccttcgccgtgaccgccttcctcaactccaccgtgtacgtgttggccgtgggagctgtgcccggtggctacgacggtgatggcttgctagaactgcgccgcattgcggtgaagtacaagccgaacgtcatcagcatcgaaaagaacatgggctacggcgcgttcgccaaggtgttcctgcctgtcctgcgagaagatcgcggcacggagaagggatacaagggcgacatccgcgaggagttcgtgaccggcaacaaggaagcccgtatcatcggcactctcgaacctgtcatggctcgcggctcgctggtcatgctggaatccgtggttgaaatggatcacgagtacacccagcgctacgccaccagcggcaagcgtcaggtctacagcctgttccaccagatggcgaagatcacgcagcagaagggcagcatcgcacacgatgaccggctcgatgcactggaaggtagcgtgcgtcactgggttgcgcagcttgcactggaccagaacaaggccatcgccaagcagcagcagcgagagttccaagactggatcaacgatccgaccggcatgaaggcagcgacccgcaagagtccgctgcaacgtggccgtccatccctactcgaccgttaccggaggtaaccaatgcagaagtccgacttcaccagcaactacacgggtctgttcggccgtggcaactacctgcaccgcgaactgctcgccctcatggagcacgcagagcagcatcccgcaaccgcagcgcagctgctcgcgcagttccagaaggacgccaccctcgtgctggacgccctgatcgctgcgggcgcacgcaccgcgtcctcgggtccgaactccggcccgcacactccggtcgatctggacccggatgacgacccactgaccccgtaaggagcaaccatgaaccagcagcagaaccaagataccagcaacaaggggctgttcggcctgatcggcggcatcttcatcggcatttcggcaacgctgctgtcattcacccaaggccacgaaggggtacgctacgctgcgtacctcgacaccggccgggtgccgaccatctgctacggccacaccaagggcgtagcgatgggcatgacggcaacgaaggcacagtgcgacaagtggctgatcgaagacctacagatcgcccagcagggcgtgcgcaagcacctgaaggcccccgttaaccgcaaccagatcgacgcctacacagacttcgtgttcaacgtaggtgagaaggcgttcgccgacagcaccatgctgcgcaaagcgaacgcaggggatcgtgaaggtagctgcaaggagttcctgcgctgggtctacgtcggtaagctcgactgccgactgtccagcagccgttgctccggcatccccaagcgccgcgacgcagagtttgctctgtgcttgcgccccaacaacgaggtgatccaaccgtggaaaccccaagtgaagtgatcgcgcggctcggcggcaagctggttggcttgctgctggtcgtgaccatgttcgtgtgcttcggtctgtacgtctacggcctgcaacgcaaggtggagaagctggaaactgcccaagtcggcacgaccgctaccgccaaggcggcgcagacgcaggctaccgggtacgcgacctacatcaaagagaaggaggacgtgcgtgttcgcactgaagaagttcttgacgctgccccggagtaccgggatggcactgttcctgctgatgtcgctgacctcctgcgcgaacctgccggtccctgacgactccctgcttgcagactgccacatcacctacctcggtggggagaagggcaccacctcctcgcaggacaaggtggtcaagctcgcgcaggaccgccgcatggacaccgttctgtgcaacaaggacaaggctgcgctgcgtgcgtggaaggccgaggtgtgcggtaccggtaagcgccggtgtacgggtgacaaatgaccaccatcgcatgggacggcaagcacctgtgggccgatagtcaggccacgcagggcgaccacaagcacaccgtgcgtaagatcatgcccgtatcgacacccaccggccctgtgctgctgggtgtcaccggggatttcacagtgcttcgcccggttctcgctgcgcttaaagcgggcgaaggctacgaggagcacgttggcaagtccgcgacggtgcttgtggttaaggacggcgtactcacggtcactactggtaagcagcagtgggtcgaggaggctccgtacttcgatggcagtggcaaggcgctagctctaggggcctatcatgcgagcaagtctgtggctaaggccatggctgctgcgatagctcacgatgtctacagctccgggcctatcgtcaagctaaaggcaccagttcgcgaggcttaggagtaaggccacgtgggtagccggaccaaaatttgcttcggaaatgcgcgggggtcactccaatagaagctcccgcgcgtgcccccgtacgccctcgcgttacgcgcctgcgggtgtgcgtgggtgcgtgcccgcgtgtgcgcctgtgtgcgcgtctgtgcgcccgcgtcaaggttccgcgtgggtgtacccgtgtgcctgcctgcgtgggcctgagcgtgcgtgtgcgtggccgtgcgtgggtgcctgcgggtgggcgtgcgggtgggcgtgcgcctgctgcctgtatggctggacc

SEQ ID NO: 20 - DNA, 44415 bp, unidentified
  source 1..44415: mol_type = genomic DNA
gctgccttggctgaatcgttaataaatctcttggcgaaaggtgttgacgtggccggtgcggtgtggttcaatggcgtcactggggcagcgacagggcttcaggagggccgcaaggggcttgacaggggctaccctacctgctaccatgcgaaccgcagctgtaggcgtgcgagggccatctgtatcgtttcggccttttggtacacctatagcacacagtcggctcaacctgaatcaccgtctatcggtactctgtcgagctgattagttagctacccgctaggccaacggttgacgcttgcgatgcaagcagtagtagacacacggccgcaatggtagtaagctgcaacgcaagtcgagtgacgtgatccgtagtggcgccgccaacaagtgggctaagggtacacgggagtcactggtaagggatgcgaggagctaccgaaccacgcttgacactaagctagcagttagctatgataggcggcaagtggtagccaccggaacagcggagcgacctagcggtaaggctagacgtgagagattacgggtgttgaggctgaggtgagaccgggacaccggtcaagacactaacaggagcgcacatggtcctctaacggatagcttgacaaggcggcacagatagccctttgaggccttgcaacacgtggaccaccgacgtacatggtgggatggtggcgacaggacgcccaacgggttagagacccgagcgagccaagggcttgacaggatgcaacaagggtgctagtatggcaccacgctctgaggagcagccacattggatggcgtaggactaccgctaacgggtagggtgtaacgggaagcgtgccaaccacagccaatagtggccgagagttgacgtggaccgccaagctgcaacgtagcactagcggataaccggatgaactgggatttcaaaggcccatagaatccaccagacttgcaacactggtgccgctttacctaagcctaacgcttagggcttcccatctgccgtgagagtcggccacgggaagtaacccactgccaaggtgggaagccggtcataaggaggtggtgagcctcctatcgcatggaatactgtgcgtttcgtgaaaaggctctacgggccacacggtgacaatggcactgctagccggagtagggttgacagcccgaagggctagcagattgatgcgccctccctttgcgatgaccatgcaggcaaatccggtggtcagtgtgcgcccacgataggcgatgcaacggctctaatcgagaatgagggattgaccgactcgacggctttctgagggcgcatcaatctgttagttttcccaccagtgccaatggaggcacaacatgcaaggctcgatcaatgccaatctcgaccgcacccagcgtaagcgccgcttctgccagttcacccggacggcaagcgtgatggacctgcgcaccacggagcatgaccgcaagcttgccgagcgcaagcgccaagccgagcgctacgaagcccgccacggaaccgccggaaagcgatctgtgtttgttgtcgagggtaacagcgggacgaaccgggcgaaccacgccgctgacaggagggcttacctgtgatccggttcaagttctctcgacactacgtggaagctgcccgcgattcctacaatcgggccatcatgaagcatccggccggctctgtgtcggcgctctacgtcctgccgtgcggtgggcgttcattcgacatccgactcgcttaaatgcaagctactgggccttcgcaagagggcctagtgtcgtgcaatcggcacggacccaacctgaagggaaccaccatggacatcatcaccggaagcgctgacatcaagcgcgccatcaagtcgatcaacaccgcccgcaccaagctggtggaccagattcagcaggccgcgattgcggtcatcaaccacgcacacatccacggcgacgttacgctcgcttccgatctgtgtctcgccgtgggcaacggcatgaagcatgaagccctgcgcctgtacctgtccgagttcggcccgatggctccgaacgacgacaaggaaaccaaggcgagcgcgcccatgaagtttgccaagagcaagcgagtcgagggcgaagctctggccgacgtgctggaacgtgccgccgcgaaggcgtggtacgacttcaagaccgagaagcccgcagaggcgttctcgttcgccgccgacctgcacaagctgctgggccgtctggaaaaggcgaccgaggaaggctacgtgccgaccgaggaggaacaggccgtcatcaacgctgcccgcgctgtgccgaagcccaccaagaagaaggagaacgtgtaacatggaacccaagatcaaccttcgagtgacccagcgcgaagcatccctgctgcgctcggcccttcacatcgcctgtgcactgaccgcaaaggcagacccgtactccaaccgcaagctgtccaatgagttcgccgtgctgcacggtgagctgcgcgacttcggtgtcgagagcttcgagcgtgacgccatcctgcaattcgaggacgacgtgattgcggcctgccgtgacagcgatgtcgaggcacagctgctgcgcgacctgatcgcaccgccgacgttcaccgtgggctacggcatgcgtgaacttgacttcgctgctatcgaggcgcgggtgatggcgtgcctgctgtctccgttgcctccggtggtgttggatgcctcgcagctggacttcctcggcagcgtgaccggccgcatggtgttgcccggcctggcaatgcccgacaacctgccgcgtaagctgccggatgtcctgatggacgaccagagcgcacgccacgtcgccctgactgcatcgcagaccgggctggtcaacaagacgaagaccaagggctggatcgtgcagttcaatctgcgccacggcagcatcgccctcgccaactgggcgcaggtgcgtgagctgggcctgccgcagcgcagccgcaatgctgcgtaccgcatgctgaaggcgcgggccaaggtgcagggcatcagcgaggatgcgtaccgtgtggtgcccgaaggcactcccgatggcccggagaaggatcgcggcttctacaccgccgagttcttcaccaagcatgcgcggcgccctcaccagctgggttggaatacgtccactgtgatcggactcagcggcacgttcaccactgcgcaggctgcacgcaacgccatcgcctcgcacgtcggcaacgatccgaaccgtctccgccgctaccgcgtgaagtggcacccgagccgcgcgtgatctaccgctgcgccttctaacgagggcgtagctttggaaccacgcccaacaggagggcacattgcatgatccccgtaacttacaagcgcatccgtagtggggagcgcaagccgatccagctgtgcgagcagccgcgccagtggaaagagttcgtgacccatgagcacagcgtggagcgctggtatgcgtgaggtcagcctgcgccttgtggtgaaggcgctgccgctcgttaccgtgaagggtgtggctgtcggggattacatcctcggcggacatcacaccagccacgaggcgtgcgagcaagccatcgaacaccaccgcaagcaccacgagaaggtgcccaccctctactcgatagaggaaatcgaaatcccacccgtcaatcaggagaaccaccatgcgtaaggtatacttcatcgtctcgatccccaagaacagcaacgatggcgtcatcactggcgtcgtcgccaatggcaccggccgcaccccgacccaagaggaactggatgcggtgatcgccgagctgcgcaccaagggtgccaccaccagcctgctggactcgctgcgtgacggcacgtacccgaaccagctcgccatcttcgaccgccgcgccgccgtgcgtgccgaggcggatgtgctcaacagctacggcgggtcgttcttcaactggcacatcctcgaagtgggcgagagcatccgcaagccggtgcgcaagccgctgggttggcgtatcacctacgccttcgccgaagaccgcagcgactccgatgtcagctgctacaaccagcacccgagcgccaccgtgcgcatcgacggcaacgagtacaacaagagcgagtacaacgtgctgttcccgacccgcgatgcagcgcgcgccgtgttcaatgccgagtcgctgggcggcgagaacatgggctaccgtgtcgagccgtactatgcgtaagctctggctgcgcatcctgatcctgctgtactggatcgtgggtcgtggcccgtgggttgtcgtcggccagtaccatgacgacgacggcaagctgtgccggttccgcaccggcccggcttccactgggttctcgctgacgttcgatgacctcggcgcagccaacgactactgcgaccagcgcaactggaaggcagacactgacccgctcggcaccacgtactacgtgtggcatgagttggagttcaatcacttcggaacgaggaggaagtaaccatgggtttcatggacaagatcaaggctgcggccaagtacgtcaaggacaaggtggtcgcagcggtgaagccgcgccacgatgacgacgacacgccgccgcctgcgccggacaccagccggcacctgcacgtcagcgtgccgctgattcccatcgacaacccgatcctgcgcaagatgctggggcaggactacttccccgtgcagaaggggcagggtcagacccgcatcgtcggcaacaaccagctgaagcgcgtggccgatagcctcggcgggaacaacaagcagcgtcgcaagctgcgctcccgcatgaagcgtcgtgctgccgagctgcgttccggtgcatcgttgcagcccaacgtgcagtccgcactggcaggtgcagcatgagcctgcgcatgggaagctgggtcgaggtgactgtgcccgacagccgactgctcaacgtgcagccggagattgccgccgccgtgaagctgatcggcggtgcgaccatgaccaatggccgtggcctgtacgtccgcaaggacaccggcgcactggacgacgaggcggtgaccgtgatccgcttcgacctgaacttgcacagcgagctggtggaccagtacatgagcgccatccgcgccatcgtggaccgtctgctggtgctgggtgaggagagcgtgctgcgtcgccgcttctacaatggcggcggtgggtacaacagcgagctgatctttcagtaacccgagccgggtaggctacgactggcccacgtacgggccatcctatcaaccgtcaagaggaaccatctacatgtcgaacgaaaacaccaccgagcagaccaccgtcagccactacgaagccaagcgcgccgagctgctggaagacatcgccaaggcgcaggccaaggtcgatggcctgaacgagaagctcgccaagctggatgccgtcgaggccaacagcgccgccatcgaagcgctgaaggcgggcgacgccgtgtcctacctgttcggtcgtgccctgaacaagcgcgtcctgtccggcgtgatcgtcgccaccggcaagaacgacaagggcgtgctgcaactgaaggtgcagaccggcgaaggtctggatgccgagctgaacctgatcgacagcagcgccctgctgatgtcggccgaggaagtgctgaaggcgcaggaagaaatcgacgccgccgttgccgaggcccagcgcctcgccgccgaagccgctgccgccaaggctgcgggtggcgaaggcgggcagtcgtgagcctcgccccgccgtcacccagcgtggccgtcgtcaagcgtggcgacgagctgaagcccggccagaatgcgtacctgatcgacacgcggcagaccaacaagctgccgaagggcaccgggttcgtcgtgtccaagctgaccagtgaagacggctcccgtctgatcgtcagcacggacggcaacggctccgtcctgtacgccaccagccacgacatcttcgaggtctgggaataaccaagcgaggatagcatgagcgatacccttcccgacaacgactggctaccacatgccgagcgcctgcctgttggtggccgcacacgtgtggcccatgagtgcggggagggtacgcccttgcttatctcacgagagcacgacaagtccaccgcattctgtttcaggtgcggtggcacaggattcaagcgtgagcacgagagtatcgaggccaagcttgcacgaatccacgccgagcagacgagcgaacgcagagtgcgtgcgactgttgagttgccagagccacgggtatacgacacccgcgagtggccgctcgacgctaaggtgtggttcttcaagatgggactctcgcttcagatgatcgagaagctgcggctgtactggtgcccaagcatcgggcgggtggtactaccgatcactgaaggcgacaacgtggtatactggacagcccggtcggcaacgagacagccgaagtggctaacacctgacgttccgaaagacggacttgtcgcacgctacggcgtgggcacaggtgacaccatcgtactgtgcgaagacccgctcagtgcatacaaggtgggactggtaaccgaagcgtggtcgttgctcggcaccaagctgcacaacaaagtgttgaagcagctgactgatcgaggccaacgtgtagcgacgtggctcgatgacgacagaggtagaagcaacggtagcaatcccggccaagacagtgcgcgagtaatcgctgcgcgtctacgtgcgtttggtctggactacaggaacatcacgtcaccacgtgacccgaagtattacacgaccgactacatcaaggagaagctgcaatgagcaaacccatcgtgcgctaccggcgcgctatcatcccgcccgtcgttggcttccgtgccacgctcggcggcgtgcttgcgcatccgaacctcggcgactgcgacatcgtgcacacctcgacggtgctgtatgtggcggacggcgggcgcaagttcgagacgcgcaacacccggtatcaccagctcgattccaagtacgaacccgaaggagaacctgatgagtcttgacaccacgctgctgcggttgtgcaccaaccgtggcaagttcgaccggctggtacccagcgcaccacgtgatgggctggacgagctgaccgtgctgatgctcgatgcgttgcgtgcgtactacaaggagttcccggacacgaaggacttgccgttcgatgtgttcgatggctgggccatggagttcaagtggaagacgcagcccgacgacaagaagtccctgctcaaagttctgctgaagcagatgcgcgagccggtcccgcccgaggcagagcagggcatgatcgagaagctgttggagttggagcttgccaccactgcggtcagcaagatcgtgcagtggaatggcggcgctgagttcagcctgcgcgacgagctgtacggcttggccgagacgatcaccgaccgaatggatcgcaaggcgcggctcccgctggtgcaggagacgcccgaggaactgatgcagatggacgagcacgacatcggcatccacttccgactgcccacgttggcgaagaacctgcgcgctctgcgtggtggtgacttcggcatctacgccatgcgtcccgacgcaggcaagaccacgttcctgaccagcgagtccagccactggatcacgcagctcgacaacgtttggccggaccagaagcgcaccggcatctggctcaacaacgaggggccgggcaagcgcatcaagcagcggtggtatcagtcgctgctcggcgctaccatccctgagatggtggagtgggcgaaggatggtagcatccgcaagcgcatcgaagatgcgatgggcggggacatccaccgcatgcagttctacgacatccacgggttcaactccggtgaagtcgaggccatcatcaagcagaccaaccccggcttcatcatcttcgacatgatcgacaacatcacgttcaccggtggcatgaccaacggcgggcagcgtaccgatcagatgttggaggcgatgtatcaggccgctcgcaactggtgtgtgaagtacgacgccgtgggcgtggcgacttcgcagatcagcgccgagggtgagggaatccagtacccgccgcagtccgcactgaaggacagcaagaccggcaagcagggtgcgtgcgacttcatcatcatgggcggcaagctcaatgacccagcgatggaacgcttccgctacatcggcaccccgaagaacaagctgcaccgcgcaggcggcaagcgtgacgttcgggaagaagtgatgatggatgcagagcgtgcccgcttctatcaggaggcagcatgagcaagccaattcacatcgtagccaccgggttcacggtgtcggtcagcttccccggtgaatccaccgaggcgaagaccttcaactgcgtgagcaacgcgcaagcaatccaccttgccaagctgctgcgcaaggtgcacgacgcaggctacatcgaaggccgcaacgacgcgccgcagtggaagtggggatggctgcggaacaaacacagcacttggatcggcgtgcactactcgccgcacaacaagcgctggtgcatcaatctgatcccgtgcttcacgttctggatcaccaagcccggaggtaacacaccgtgagtaccgaaccgaacatctacctgccgcgcaacgtgggcgtcatcacgtccagccgcaccggcagcagctacacagtcgagccgcccgtgaccgacacggacatcgacttcctcgtgctggtgcaggacttccacgaggccatcgaaaagctggtcgatcagggatggaccctgtgctccggtgccgatggacactacgaggaggacgaggactacagcaccacgtggtatgcgctgcgcaacggcgtgttcaacgtcatggtgaccgccgactccggctggtatcagcgcgcggtcgaggccaccaccatctgcaagcgccgcaacatcaaggacaagcaggaccgcatcatcgtgttccgttgggtgcgcgacgggctggacttggatggcgatgcgtcggatgaaatgtaccagctggccctgcaacggtggccgctgtgagcttcacttccttcgacctcgaaaccacgatccgttccatcctgaagcgcaaggccaatccgttctacgacatgaacaagatcgtggcgattggctacaagcggaagggtgacgcacggaacaccggcctgtactacgacacccgagtcgggatagacaaccagtacatgggcggcgcacccgatgggtggctgcgtgagctgtgttacgggcagcagttcctcgtcgggttcaacatcaagttcgacatcctgcacgccatctgccaaggcccactcaaccggcaggcatggatcgagttcatcgacggcggcggcatggtgtgggactgccagcttgcggagtacctgctgcacggcatgacgcaagagttccacatggcgagcatggacgagacggctccacgctacggcggcaacttgaaggacgatgcagtcaagtccctgtgggctgcgggcgtggacacctgcgacatcgacaagacgctgctgatggattacctcctcggcaccaacgacaccgacgacgtgggcgacatcggtaacaccgagaagatgttcctcggacagctcgccgccttccgtgcacgtggtggtctgcgctcggcgctcctcaacatgggtgcgctgtgcttcaccatcgaagccgagtacaacggcatgtacgtggacaaggactgggcgcttacgaaggcgaaggagttggaggtcgagcttgcaacggcgaccgccgaactcaacggcttcatccccgagctgcccgagggcctgaccttcaactggaacagccgcttccacaagagcgcgctgatcttcggcggcaaggtgaagtacacggccaaggttccgatcatgtccaccgagggtgggccgacttacgtgcagaaggacgaggtgcactacgtgctggtcgatggtaccacgacggcgacgccaccggccgaggacttcgacaacctctggcgctacaccacgtacggcagcggcaagaacaagggagagtacaagaccaagaaggtgaaggtcgatgacttgaccaagcagaagttccgcaacgaggacatgctgttcgagttccctggctacaccgagcctgatgctgcatgggaaagcaagagcgatcccggcgtgtactccaccgctgccgacgtgatcgaggcgctgggctaccgcaacctgccgttcaccaaggcgcttgccagacgcgacgacatccacaaggacttgtccacgtactacatcacgacggacgagaagaccggagagcagaagggcatgctcacgctggtgggaccggacggcatcatccaccacaagctcaacatgaccaacacggttaccggccgcttgtcttccagcgatccgaacttgcagaacgtgagcaagggcgagctggacgaggagacgttggaggagaagggttcgcagatcaagcgcgccttcgtgtcccggcaccggggtggcaagatcatccagtcggactacacctccctcgaaatctacgtgcaggcaatcctcaccgagtgccgtcagctgatcgaggacttgaagcagggcctcgacatgcactgcctccgtgcagagcaggcgtggggtgagcaaggcaagtacgactacgacttcatcctgaaggcgagcaaggacgacaagcatcccgagcacaagaagtggaagaagaagcgcggcaacgcgaaggtgttctccttccagcgtgcgtacggtgcgggcgtggcgaagatcgctgcgaccaccggcatgtcggaggaagaagtcgaggcgctggtgcgcggtgaggccgagcgttacccggagctgggcgagtacatcgaccgcatggtcgagcacatcaagcgcaaccgcgtcagcactcagcgcttcgttccgcatcccaacgcggggcagcaaggcgtgccgcatgggctgacgtgtcagcttggccggtcgcactggaccacgccggacggcaagatgtattccttcagcgagtcaccgtccccggtgttcatcgccaacaagcccgcgagcaagggtggctgtgcgcagtcgttctcgcccacggaaatcaagaactacccgatgcaaggcaccggtggtgaatgggccaaggcggcgatgtacgtcagcctgcgcgccttctaccggaagtacgtgaccgaaccgaaggaatggttgggccgtgcgttgctcgtgaatcaggtgcacgatgccgtctacgtggatgcacacggcgacatcgcaaccaaggccgctgctctgctgcacgcctcgatgctggaagcgtcggtgtatatggagtggtggttcaactggacgctgccgcttggcgtcccgtgtgaaaccaagatgggcgacaacatgatggaggagaagaaccctcccgcagagttcgccggtctggtcatcgagtaccgcgcgtcgatccgcaaggacttcgtaggtaatcacaacccgtcgtttgaataaggagaacaacacgcatgagtcttgacgcactgttgaacaaggtcgccacgcagggtaaggatcagtcggtcgccagtggtggcagcttcgactacaccccgcccgctgccggtgtgaccaccgcccgcatcgtcgggtactacgagctgggcaagcacgagttcgagttcgagggcaagaagaagacgcaggatgaagtcgccatcgtgttcgagctgaccggtaagcagcacccgcacatcgaaaccgacaatggtccggtgccggtgcgcatgacgctgaccctcggcctgtccaccaacgagaaggcgcactacttcaaaatcttcagccgcctgcgcaccgaggagcgccacttcgtgcagctgctgggtcagggtgtgctgctggaagtcatccacaagccgggcaagcgcgacccgaacaagaccttcgccgaaatcgacaaggcttccatccgcaagccggtcatgccggtgccggaaatggagaacggcatcccgaccggcaagttcgtggacaccgtgatcccggtgccgcagcagatcaccccgctgggtgcgttcgtgtgggacttcgccgacgccgacatgtgggacagcatctacatccccggcgagtacccggagcgcaaggacgagaagaccggcaaggtcacccacgaggcgcagtcgaagaacaagacgcagctgcgcatcgctgcggcgctgaacttcaagggtcttccgtgctacgactacgccgccgccaagttggcgggcagcaccacggtcaccaaggaaggcgtcgatgcgctggacgaagtggtcggcgacgtggcgaacgccgcgcccaccgacgctgctccggccgacgacaagccgccgttcccggtggacggtagcgacccgatggcaggcatcgcctgatggacctgagcgctctcatggcagcggccggtgagcgctccccgatgccggtgcaggtggtacgtcagcacaacccgcgcgtgatcgctcacgttgatggggactacatggcgtacttcgcggctggtagcgagaactgctcggcgggggatgcacgacgcaacgtgctctcccgctgcgcacagctgaagcatgtcagcggagcgggcaagatcgtcatgcacctgacgcacgccgcgtctaccaagggtgatcgcttcctcgctgctaccacgcagccgtatcagggtcagcgccaagcaggccgcaagcccaacaactgggcgttccttcgtgagtggatggagacatacgagggcgacgctttcactcccaaaatctggctgacccgtgaggccgacgatggcatcgcgtacgtcaacgagggtgcagcattgcaccacaacatcctgcacgtggtgcacagcgccgacaaggacatgcgaatgttctgcggcgtgcacgtagactgggacggctacgacatcacagaggttccgctcggcgcttacgacatcgttggcgagaacggattgcagtacggtcacaagtggttctggatgcagatgctccacggcgacaccgccgacaacataccgggtctgccgaaggtgggcaaggtgacagcggagcagctgctgttcgagacgaagaccaacctcgaagcggtgcagatcgtgagcggcaagtacagcgaagtgttgggtgccgactggcgcaagacattcgccgagcaagccgtgctgctgtggatgcggacggatcgtgacgcagaactgctcgacgtgctgaagctcgacgtgttcgggccgaagctgaagcaggcgttctatgacctcgccgaggacgtgaacgagaagcgtgcaatcttggaggcatacaaagcatgaagcgactcactgcaacacaggtcaagctgctgcgcatcaagctcgcagcggagcaaggcaaccggtgctgtctctgtcagggacagttcggcctgaaggctccgctcgatccggtgctggaccatgaccacaagaccggcgctgtgcgcggggtgctccatcgcggatgcaactccctgctcggcaaggtcgagaacaacgcaggccggtacggcgtgcgcgacgtgttcgcattctgtgcgggcatccccaactacctgcggtcgcacctcaccaacatcacggggtacctgcatcctacctacaagaccgacgacgagaagcgtatcgctcgcaatgcgaaagcgcgaaagcgtcgggctatcaacaaggagacaccgtgacccttacccagttcattcgccgagcaccgaagcgcggcccgaagattctctgcctcgacatcgagacgttccccatcgagttctatggctggggcatgttcaacaacaacttcagcgtcaagcagatcaagcgtgactggtcgctgatgtcgttcgcttgcgaatggctggacgacgaggcgtcgttctacatggaccagcgcaacgtgcgcgacgtgttcgatgatcgcaagcagggcaaggcgctgtgggcactgctcaacgccgccgacttcgtgctcgctcgcaacggcaagaagttcgaccttcgcaagatcaaggctcgcctcgcaatcctcggcctgccgcccgtgtctccggtgcaggtgatcgacccgatgctgctgaaccgcaccgagttcgccttcacctcgcagaagttggagtacaccaccggcgtgatcgtgccggagctgcgcaagtacgaccaccacaacttccccggcttcgacctgtgggtggcctgcatgcagagcctgcccggagcatgggacgagtgcgaagcgtacaaccgcatcgacgtgaagtccatgaagttggagtacaagaagctgcgcggttggtactcgcagcatccgaacgtcgcagtgtactacaaggccgacggcagcgagcaccgctgcaacaagtgcggctgcaacgaaatgatcccgcaggatgatccggcccgcacgcaggtcggtacctacctcctgcttcagtgcaccgtgtgcgacggctacagccgtgggcgcaagctcacgaccagcgccgaggcgcgcaagcacatcaccgtcccggcataaggaaccgacatgaagatcaccgacatccgcagcggcatgcgggtacagtacatcggcaatgcgcccgcaatgatcgggctgcgtggacaggtaagccgcgtgttcgctcgtgatgtcgaggtcttcttcgacggtcgagttaagccgagctgctgcgttcccgattccctccgacagcttctcagcatcggaggcgtgaccaccaccagacgagaggtaccaatgcccgaactgagctaccgcgacgaggaccgtcgcacactgtccgaccgtggcgtcggcctgaaggatgacgggggcaagccgcaggcccgtctgctgcatgagggcgtgccgcgtgcactggcccgagtcatcgacaccctgaccttcggcgcgcagaagtacaaagcgcactcgtggcagcatgtcgagaaggcgctcgaacggtatcaggacgcgagctaccgacacgacaacaagcgctgcctcggcgagaagctggacccggagacgggcatccaccaccgggcgcaccacatcatcaacgagctgttcctgttggagctggaactgcgcgaggaggagaaggccagtggcgcagagtaaggcgcgctccatcaaagaggcttgggtgaacatcggcatcggctacagcatcaactacgcagcgaacatcgcgctgcttccggtgctgtggcatcccgagcatccgctgctgtcggcgcacgccatcggcattgcgttcacagcgatcagcttcatccgccagtacatcatccgccgctggttcagcaagggtgactgatggcctgcgcccgctgcggccaagtgcatcggtacgtcccacatgaggccgagtgggcgcgcttcctagaggagcaccgtacccgcaagcagttcgatgtcgagtgggccaactcactctggcatcgtacataccctgacgacgcattctgcatcctcgtgatgaggggcctcgcaggtttcgttccattcccgtcgaaggagaactgaatgctctacaagaaccagaccgccatgctcatcaagtcctacgagaacgccgttgcgtggggcgagagtgccgaccacgaggaggcattgcagaatgcggtcaaggccgggttcccgaacctgcccgacgaagatcaggccgagctgtatacccgcatcgccgatgcgtgggaaggctaccgtggttcgctcgctccgcgcaagctgtggatcggcaccatcgtcaaccagttcatgtcgtcccgcatcgcacggttcaacgccgcgctgggtgacggcaccaagaaggaggacagcgccgatgtttgatgtgcctcgccagaatgtccgggttgctcccggctacaagaagcgcaagcgcggcttcaagatcaaccgcgccttcaccaagggcaacttccgcgtgcagtggtacgacggcaaggccacgtactgggagcgctacgttccgtggtacgaagtgccgctcgccatgttccagatttggagggactacgcatgagctacatcgtccacaaggcagtcgagcaggacaagatcaagaagaagctgcggcccaccgaggagcagcttcgcaccgagtacatcgcacagccgaagtacgacggctgcaacatggtcgccatcaagcgcggccactgggtgcccacggtgaacaagggcctgcatgccatcaaggtgggcgacgtgcagatgcagccggtggatcgtggcgtggttgacctgttctcccgcaccggtgagcaggtcgtcagcgcacaccacatcgagaacgctctcgcatccgcgccgttcttcccggtcggcgtgtacttcggcgaatactggcacccgcagatcgaccagcccaccgtcagcggcatgttccgcaagaaggacggcacgcagtacaccgagccgatgttcgtggtgttcgacttcgtgacgctggaagaatgggagcagggtttcagcgacctcgtgtatcaggagcgcgtcagccgcctgccgagcatgggccacgccatcgccgagggcaccgcgccggtgttctacgccgagtcgcagggcttcctgatcgaccaagagctgggcagcatggaagcggcgaagctgctgtgcgagggcggcgcgtacgacgggctgatcctgcgcaagccgagcggcaagtgggtgaagggcgacaagggaaccaacggcgaagtcgtcaagatcaagccgaccctgacgctggacctgcgtgtgctcggcatcaacgaagcagtcggcgagaagaccggccgcgccgtgtacacggtcgtcgttgacctcggagaaggcaagacgcaggaggttggcagcggcgtgccgcacagcgagagcgagctgcctagcgtgggaggcatcgtggaaatcgaggcgatgtccttcagcaagtacggcctgctgcgcgagccgcgatacaagggcatccgtcacgacaagaaggaggcagacctgtgagcgtcgaggtgcaagcatggcacaacatggagcgcgacacggtggagctgcgcatcagcgttcctttcggcgagtacgccggttccctgtggccgaacgagacgctgcgcgacaaggtgcaggaagcgttcgccaagttccttgacgagcggaggggctgatggacgcgatcactttcgagaagccggagctggacttcagccagtcctcggcatggatgggccgcgtcgaggtttcggtgcgcgcccggtacggtgccgacttgttcggcgctgctgccacgtgcatggccgaggatatcggcggtgaggcgtggccgcacatcatccacgacctgcacatggaaatcatgcgcggtatcctgaaacgctacccgccgcgcgactacaccgtgcggcagcaacggaggtaacaatgctctcgcaagtggaactcgaactggaaacctacgccttcggtaaggagcgcatggagaagtccatcgcccgcaacgaggagaagggcggcgcggacaacaacccctacgcccaagcagtgtatcgccggttcgtgcttccgcttgcggagcgcatccgtgcggacatcgactctccgcgaatcggccgtgcgcaagcgcacgtgccacttctgcgcgccaagtacgatcccgagcgtcagaacaagcgtggacagcccgtcagcgccgaggaacaggcacgcgagtggtacgaggctgtggccttcgtcgccgttcgcggtgcccttacctcctgcatgcgagacaagcacggcgaaggcagcgaccgcgacgtgttgaagaacgttggcatcaacgtgtaccatgagtacctgctgacgcagttcgccgacgcggagccgactctgttctaccacctgatgaacgacatggaccgcaagctctctgtcaacgagaaccaccgcatgacggtgatgaagatgcaaggacgcaagaacggcatcgagttcgtggagtggggacaggcacagcgcgatcaggtcggcgcgtacctgtgcgatcagcttgcgcagctgggcatgttggagattggcgtggtcaccgagactgctgccagtgcaggcgcagcgtaccgcaagttccagaccaagacgcacgtcaagatcgtgctgaccgacgaggtgcgcaagctgattactcagatcagcgacttcgtgatcgaggccacgccgttctacctgccgtgcgtcgagccgccgatggactgggtggacatcgacaacggtggattccacacgaaggaaatgcgccgactcaatccgtggatggtgaagacctacgctcagacccgcgacgagtaccgcgctgccgagctgcgcaacgagatggctgcgatcaacgcattgcagcgcgtgccgtggcgcatcaacaagcgactgatggaagctgtgtcggccatcgccaaggtgcacgacatggaggaaatcatttctcagggcgagctgccgaagccgcgcaagccggagtggctgacgaaggacatgaccaaggaaaccatgtcccacaatcaggagttggagttcaagcagtggaagcgcgacatgtccaactggcacaccgacgagcgcctgcgacagaacaagggcaatcgtttctacaacgcaatgaaggtggcgcgcaagttcgccgagtacccgagcatctacttcgtgtacttcgctgacttccgtggccgcaagtacgttcagaccaccggcgtgtcgccgcagggttcggacttgcagaaggcgctcttggagttcgccgatggcaagccgctgctgactaaggacgcgaaggattggttctgcatcacaggagcaaaccgatggggatacgacaaggcgtctctgccggatcgtgtgaagtgggtagcggagcatcacgaccagatcatggcgttcgctgcggacccggtgaacaacgacgagtggaagaccgccgacaagccgctgcaatttctgagctggtgcatggagtacgagcagtggcaagtgttcggggatcgcttcctgagccgcatcgcagtcggcatggacggttcgtgcaatgggcttcagaacttctcggcgatgctgcgcgacgcagcaggcggcgtggcgacgaacctgatcccagcaccgctgccgaatgacatctaccagatggtggcagaccgcgtgactgccgtcctgctaggcgaggacgaggatgccgaagggtaccgcacgctgtggctcgaccacggcctcacacgctcgctggtgaagcgcagcgtgatgaccctgccgtacggctcgcggcagtcctcgtgggcggacttcatcatcgaagactacctgaagtgtgggaagttcccctcgctcgacaaggccctgtacggccccgcagcgcgcttcctgagcaagcgcatgggtgaggccatcgccgacaccgtggtcgccgcagcgggcgcgatggagtggttgcagcgcggctccgggtcgatcctcaaccaagggtacgaccgcatccggtggatcacgccgtccgggttcccggtggtgcaggtctactgggagtccgaggagcaccgcatcaacaccaagctgtgcggcaacgccaagctgtccctgcgcaagagcacggacgcggtgaagaagtcccggcaccgcaacggcatcgccccgaacttcgtgcacagcctcgacgcaagccacctgacgctggtggtcaacgcggccaaggccgaaggcatcgacgccttcgccatgattcacgacgacttcggcacccacgccgccgacagcgcggcactgtaccggatcatccgggaggtgttcgtgtcgatgtacgagcggcacgacgtgctgtcggccttccactcggcctacccgttcctgccggagccgccgccgatgggcgagctggaccttcggcaagtccttgattctccgtacttcttcagctgacggagtttcagtacacctatagcacgaggcaactgaggtccggttggagcggccgcgaaggtaagcggaaccggtgccggaccttttggtacacctatagcacagaggagacaccatggccgaagacgccaaagtgaaagtcctgatgacgctccacccgaaccagctggccgccgtgcggaagctgtccgggctgtcgctgtccgtcaactcgaataccacgcccttggaggcaggtatgcagttggggatggcccgcgtcctgaacatcttacaggagggtttcaccgttgattcctccgtaccgaacaccaacgacgggtgatagtgagcagatcaaggcggctttaacggccgctttgtatctgtcatctagagaagatagtaaggtagacaacagagaatcttctgtgagctacaactgtgatgaccctgattacacagtggccctgataacacagggtctagtggatgcagtaatcattgatgaagcctacctgctgtgctttgccattgtcacaccgtggtactccaagaaccgtactacgttcgttgagaacatggtgctgcgaattgggccgggcagttccttcgaccggtacatagccgtgatggaacatctggctgacatcaaccactgcgactcactgagcgcaggcggtgcactagctcggaactcccgagcactcacacggatgtatgcacgctacggctacctgctggaacggcatgctccccaattcaccaagcgaaggagttaacctatgggtagcatcgttggtggtgggtccgccaagcgagcagcgctgaagcaagctgctgctatcgacaagcagaccaacctccaaactcaatccacgaactaccagattcaggcgatggccgatcagatggcacaggcagctgcacagcaggccgcatctgagtacgccgagaagttgctgagtgcccccgtcgataccgtcgatgtgcggctgggaacttccgacctcgacttgcagactgccgacctgatcggccgacgcaagaccgcccgctccacttacacccgacccgtgaccacgaccgcagcttcccggctgacgaccgtggccgggtcagacctgttgtgaggtgagcatggaccatccgatccaaaccgctcaccgccagttcgaggcttacgacaacaagcgacagggcatcatgtaccgactcgaacgctattcgagctggaccgtgcccaagctgttccctcgcaagaaccgcgatcaggacaccgagccgctgacccacgggttccagtctctcggcgcgcaggcagtgaaccatctggcgaacaagctgatgatgtcgctgttcgcaccgtcccgcccgttcttccggttggagctgaagcgcaaggcgaagcaggctgcgcaggagcaaggcgctgacttgcaggccatgcaggcgatgcttgcgaaggccgagcaggatgccagtctcgaactggacaagcgctccatccgctcccggctgtacgacctgctgaagatgctgatcgtgctgggcaacgccctcatggtgttggagaaggacacgatccgcgtgctcaacatgcggcactacgtggtcaagcgcacccgcaccggcgaggtctacgaactgatccttcgggagaaggtgcacaagacccagctggaacccgcagcgctcgctgccattgtcgcgcacccggacttcaagcccgatgacgacggcatggtgtgggagtacaagtgggtcaagctggaccacaagaccggcaagtacaacgaagacgtgtggatttgcaactgcaagctgcccgccaacttctcctcgacctacaccgcagacaagctgccctaccgggcggttagctgggacttggccgcaggcgatgactacggctccggcttggtcgaagactacgaggccgacttccagtcgctctcgatgctgtccgaggccgcagtgcagggcgcgatcctcgcctccgagttccggtggctggttaaccccgcaggtcagacctccgtcgaggacttcatggcgtcgcccaatggcgcggccattcccggcatgaagggtgacatcgagctgattaacgcaggcgtcgatggcgtgctgcaaaccaaccaagcaatccagtccacctacatcaaccgcatcggcgcaggcttcctgttgcagacggcggtgactcgtcaggcggaacgtgtgaccgcgcaggaaatccgcatggtcgccgaagaactggaaggcgggctgggtggcggctactcccggatcgctgcggacgtgcaggtaccagtcgccttttgggtgatgaacctgacgggccgcgacatccgaggcaaggacttggagcctgtcatcatcaccggcttggccgcgctctcccgtacgggtgaccgtgaccggctgttggagttcggcagcaacctcgccaacgtcctcgcactgccgccgcagattctcgaacgactgaagctgtccgcgtggatcgcagacctcgccgccgctggtggcttggacccgaacgtctacgtgctgactgaggccgagtacggccagatgatgcagcagcgtgcacagcagcagctcgccatgcagaacgcatcccagcagatcgacaacgccaacaacatggagacacagacacaatgagttccaacgcacctccgggcggtggtcccggcgcaaccgtgatcgcaacctcgaacggcaaccagcccgcaccggcagctccggctcccgcagacgacaagctgttgcccaacggccagcccgctccggccgcaccggcacagcccgcagctcctgctgcacctccggctgctgacgcgctgagtctcgaacctgccgctcccgcacagcccgccgccccggcgaacgctgcgccgactgcggtgtcgatcccggactacggcgacaacggcctgaacatcgcggccgaatacttcgtcaacaccgtgggcctcgacatcgacagccgcgaactgaccgaagcagcgaagggcaacttcgccctgctggaagccaagctggaagtcctcggcgacaaggccaagggttccgcaccgatcctcgctctggcgaaggagagcatcgctcgtgtcaccgccgctgcaaccgcagcgcacgccgcgaacgttgctgctgtccacgaagccgtgggtggcgcagagaactgggctgcgatccagcagttcgcacgggccaacctgcccgccgaccaactgaagcaggcaagcgaatcgctgtcggctggtggcttcggcgctcaggcgaccgcgcgttacctgatggctctggcacaggccaatcccgcgacgaccgtcaagggcgcaccggctaccaacgccgccgcccccgccgcgtcgatcaacggcgtcgctcctatcacgaaggagcagtaccgcgctgagtaccgcaagctggttgccgagaagggcatccgtggtgcggcccactccgaagaactgcgtgcactcaacgcgcgcgtcatccactaagaccaaggagcaacacaaagcatgagcaccatcttcccgactgtcccggttctgccgaatcaggtcaaccagtccggcaacgagaacgccctgatcctcgaacagttcaccggcgatgtcgagcacacctacgtgtccagctcggtgctggaaaagttcttcccgcgcaagcaggtcaagggcaccaacaccctgaccaagaaggccatcggccgtaccaagcttcagaagctgaagcgcggtgacgcgccggacggcaccccggtggacttcagcaaggcgtcggtgaccgtcgataccatgctgctgtcgcgtcacagcatctggcagctggacgaaatcttcaccgacatcgacacccgcaaggaaatcgccatcgagcagggtcaggaaatcgccgagttcgtggacctgaccatcagcatcgccgccgcgaaggccgctgctgccacgcagtcgatcttcacccgcaacggccgcgcgcccgagggccacttcggtgccacgcaggtcgtgctgtccgccgctggtgacgagaacgatccggccaaggtgtacgccgccatcggcaaactgttctcccgcatggaggaggagaagaaggtcaagccgcagcgcgatggcgtggtcctgatcgtgcgcccggcgatcttctacctgttgcagcaggccgagcagatcagcaacggcgagtacctgacctcggacggcaacaagctgaccggcatcccgaccttccacggctggggcgtcccggtgctgtcgagcgagaacctgccgaacaccgtgatcgaaggtcacctgctgtcgaacgacgacaacgacgacttctacgacggcgacttcagcaccctgatcgccgtggccgtgtcgccgaaggccctgctgatcgccgaagcgctgccgttgcagtcctcggtgtggtggagcgatgcctcgaagtgctacttcgtggactcgtggatgtccttcgccgttggtctggatcgcgtcgagaacgcgggccgcatcgacaaggttgcctaatccgctgggcgcggtccctgaatccttcgggtaactcaaaccgcgcccttcttccaccaacacaggagcaacatcatggtctttgaccgaccgttcgagatttccaaccgcgtcgtcgccgcaactggcgtggccggtctgcccgccaactccgttggtaccgtcgtcggcgtccactacgacacccgtggcaccgcaggctgggtcgtccgtgtccgtttcgtggacgacgaaatcggctcgcaggacatcgagtacgcaccggccgctctggctctggctgcggactaagcaacatcccggcaggggcgctccggcgtctctgccttgttcctctcaggagacaccatggcattcatcaccaagctcgacatcgtgaacgcctgcttgaagacgatgggcgagacgaagctcaacacgctggaagatgaccacgtatacaaggacgacgccgttgacttgatcgaccgcgtgcaccgtgacgtgtcctcactctcgctgtggttcaacaccgaatgggtggagctgaagccgcaggcaacgagcaagtacatcatggtccccacggacgtgctgaagctggactgcaacccgagccggttcggccacgtggtgcagcgcggacgccgactgtacgaccgcaagcgcaacacctacgagttcgaccacaacgtgcaggccaagctggtgcggctgctggacttcgatgacctcccctacgaggtgcagatgttcgtgcgcgacgactcggtgctgcggttccagtctgacttcgacggcgacaacaccaagtacgccaagatcaagcagcagcgcgatgacagttacatcaacttgaaggccgagcacatccgccagatcaaggcgaacccgctgttcgctcgcgcatccgtggacgtgctgcgttcccgttactggaactacagcggtcacccgtggcacagccacgtcacattccccggctaaggagacaacatggcaaaggcaggcggaacctatcccgacatccttcagggtgtcagtcagaaaccggcgcatcgtcgtcggccgggacagacgcacgagcagatcaacgtgctgtccgatccggtgaacggcctcgtgcgccgtcgtggtacgcggttcgctgcttcccaagccgttgtcacctcggccgagctgcgcaacatggacgtgttcgacttcatgcaggagggcaaggagtacgcgctgctgtaccggcgcgacgcctcgaccttgggcagcgagtccttcgcgttcctctacaacaagacggacgagtcgttcatccctctggtgtacgagaacagcacgtgggtcaacacgctggtcagcggaggcgcatcgtcgctcacggccatcggcagctacgtctacatcgcgggcaacaccacgatcccctcggccaccagcacgaacgtgtggcaggagcagacgaacatccagcgcctcgcagcatgggtgcgcaccgggaagtacaacaccacgtacacggtgaacctgacgcggacggacaacacggtgctgacggtaacgttcaagacggttaccgcatcgtaccccggaacgctcgacaccagcgacatcccgttctaccttcccggtggcacggagccggacgcggcgtaccagaagtacgtcaacgaccgagtgaacgagtacaactctgcggtcaacgagtggatcgtgacgagcgctgagcagacgcgcccggagtacatcgcggagcagctgtcggatttgctggtcgatgcaggcgtgtcggcaacgtacatcaagggcgggatcatcattgacgatgaccagttcaaggacatcacggttgacgacgagggagacggcacgaccttctacgccgcagggcaggaaattacagacgcgacctacgccgtcaagttccactggcacggcaaggtcattcgcgtgcggccgagtggtgcaggcgcggacgagtcgtactacctgcgcgctgagttggagaacggcgagacttccggctacgggtcggtggactggtacgaagcgcccggcgtggagtgcaccatcgacaacctcgtgtcgcagctctacatctacaacggtgtaggctacatcgcacgcaacggtgcgggcctcacgtctctggctccgagcagcggcgagcatccggcctacggtgcgcgagtggcaggcgatggtctgacctcgccgatcccgtggttcatcgacaagccgatcacgatgctgtccgtcttccaagaccggctggtcatcggcgcacagaactacgtcaacgcctcacgctcggcggactacctgaacttctggcgcggctcggccgtcaccatcgaagacagcgaccccatcgaaatcttcgcgcacggcagcgagggcgatgtgctccggcacgcgacgctctacaacggcaacctcgtgatcttcggtgaccgtcagcagtacggcatcagcggcgactcggtgttcagtccgaagaatccgctgattaaagcgttcagtgccaacaaggattcggttgacgcgaaggcgcagacctcgggcaactacatcttttatgcgcagtacggcagcgaaggcacgagcctgcaccagatgcgagtgggcgcgctcaacgggcagcagacggtgacggacgaaatgtccaacgagctggactcgtggctgtcgggcactccgttgcagatcaccccgctcactgcgccgaacctcgtcatgttccgcactcgcgagcacccgcaggacttctacctgtaccggtacgaggacaacaagaacaacgggcagcgcatcgtggatgcgtggtcgaagttccggtaccacccggcgctgggcgaaatcatcggcgtgagcagctacaagaagaacggcctcgtgttcactgcgcgcgggtcgctggtggcgtgcgacgtgttcgacccgaagggcgagccggactcgcatgcgtgcctcgacagctgggcgagttttggtacacctacgggcgtacagactgcgagcgcaagcatcgccgtcaatagcactagcccgtacttcctgctgggttgtccctacgcgcaggcgtctgacttccttaaccagttcgatgacctcgctgctggtgcgctggaatacggcgtggtgtccgaagctctggtgatcccgaccaatccgttccctcgggaccagaacggtcaggccgtactcgatggacgcatgtccctcaacaaggtgacggtggacgtggagaacacggcaggcatgatcgccacggtggcaacccgcaacagcaatgtgaccactacggacttcgagggccgcatcctcggcgactccgacaatctgatcgcgcggcaaccggtgtaccgggggcagctcaacatcagcgtcgggcgcgaagtgcgcgagtgcacctacgagattcgcagcaaggattggctcccgctccgggtgaccggcctgagctggacgggtcagactttcaacaatgtacggagggttagctaatgggttcggttaatacgatcctgcaagcgaacaacaccacccgcgttgcccgtgcgaactaccgtgcagccgttgcgcagaccgacaaccagaaccgcagcgaggtcgccaagaccggcttcgctgatttcatgcggtccctgaagaacaacgcccaactggacgccgccgcgaaggagtacaactccaacatggaagcgctgtccgaggagctgcgtgcgcgccaaggggctgggcttaactcccagctccaactggcgaacgcgcgtggcgcacttcaggcgcaggctggtgctgtcggtgtcggcggctcgtccgcagacctgatggattcgatggtgcggttgcaggcggaaatggatcaggagacgcaggccaacgctgtctcgctcctcgcctcgcggggcgcatcgcagactgcgcagatcatgtcgcgcgcgtggaacgggatggacatgagccgttcgttcgggcagttcgactactcgcagcacatcgagccgcaggcaatgaagcgtcgcttgggcaagctgatcggcgtggccgtggctacctacttcggtgggccgatggcaggcgaggccgtggcagacttcgcggtcggcacgtggcaggcggacaacggcaacttcactggtgcctctcagtccttcagcaacgcagcgcagaacggtatgcaggcgtggcagcagtccaatgatcgcggcggcaagtcgtgggcgtccactaccttcgggtacaacgacggcaccggcaagcagtccgtgactggggcgaaggtcaccggcaacttcggcaacaactacgacaacttctccaccactacgtccggcctcggctggttcgatagcggcagcggaggcaactcaggaggtgcatggtaatggctgacatcggcacggttaccttcaacacgcagtccgcattgcagggtggcatcaacgccaccccagcactgtcgggcaacaccagcattcaaggcgctggtgtgaatcaggtcgggccggttcaatccggcaacgactggttcgcaagcactggtggtatgacgatgccggacagcaacctgccagagttcttgcaggagctggcagcgccgaacaccgccaagctgaagcagcagcagatgtgggacggcttcgttgccgcccgcgctggtaagaccatggacgagattgctgcgaccgaaccgtggtacaagaaaatcttcggagacaccaactacgagattggcgcgagcatgtataacacgctctcgcaggtcaacgaaatggagagcgacttgcttcggcgtatgccggagttgcgtcagcttcctcccgaggcgatggcgaaggagttcaacgacctcgccactgcccgcatgaccggcaacggtttcgcggacacggtgttgcagaagaccttcatggatcgcgcgggttccctcatggacctgcacaccaaggagcgcacggcatggcagcagcaggagctggtgaaggcgcagtacgctgcgaactcgtcggcgtccaccggcttcaacgaactggcgaagcgcacggcgatgctcggtaccaaccgtcccatggacgagaaggccaccgaggcgctgacgcaggcgcagctgtccctgctggacggactgtcgccctcgcgctaccagacggacgagtcgtacaagtccgcgatcactgcgttctatcgtggcgctgcggatcgcggcgagttccacacgctgaagttcctcaacagcaagggcgttctgaacgccatcgacccggacgggcagctgggaatccagcagtacgtgaagcaggcgcaggatcgttaccgttccgactggctcgatgccaacccggagcaggccgagaagatggcgctcgtctccatgtacgcatcggagggcattggtgccaagccgtcgcaggcgatgatcgaggaaatgaactcgacctacgccgccgagactggaagcgacgcaccgctgtactccggtacgcagttggcttcgatcatggcacagtccgcaggcgcgcacatccgcgcacaggaagccgtcatcaaccagcgtaacgctgcggccaaggccgcgctgaccgaccagcagaagctggccgcgcaggaggaggacatccgtggtggcatcgaagcgttcaagcgcggcacgtacgcgcagacgatcaacatccccggcgtggacaaggagctgatcgaggcgaacacggtgcaggcatggaatgccacgatggccgcgaaccccaaggtcgccatgtcgcagctggtgtggaacgccaacaccgggcgaggcgctgtgctgaagggtgtggccgaccagttccagaccacggcgcgcgctgtgctccgcgatcagccgaacacggcagcggctgcactgtaccagcagtggaaggaactgaagcagaccaccgccgcacgcatcgacacgaacggtcagcccgtgcagggccgactgactggcgcgactaccgctgcgctgtacttcggagatagcgtcaacacgttcttcaacaagctgcaagcgttggagaatggtggcgtgaacttcgagcttgcttacgaggtggcccgtggagaaatcaccaccgacgatccgacgcagttcgacgcgaacagccgtaaggaatccgaggctactcaggctcgtgttacggaagctatcgccaagctcaaccccaagtacctcggcatgttcggcaacaagctgggcgactctggccgcgctgcgtatgctcgcgccatcgtccgctcggtcactgacaccggtggtctgctggacacttctgcggaaggcttgcaggctgcggctactcacgccaagctggcctacggtctggaagacgcaggcaagtacgcatgggaaaacggacgcgacgacgaaggccgagtgatcggcagcgtcggtgcatggctgggcttcatggacacgaaggaaaccggacccgccatcgagaaggccatcgacgcagcactgcgccgggtcaacatcgagccgagcaccgggctgaaggctgacgtgttccgcatgaaggacagcgagaacggcgagccggtgctgtacgtcaacgctgttggcgagaagggctggaaggttgtgccggtgtacgggcgcgacatcaaggacgagtacgagaagcacaccaagcagcagcgtcagttgcaggccccggtaccgcagggctacgttcgcatgaacgacggtacgattcagcagagcatttccatccaacccaaactgtaaggagatagacaatggcactcgatctttcggggctgacccaagaccagcagattgccaaggctgccgcttatgcgggagtgccggagtccatcgtgcgcggtcagtggcgagtagagtccggcaacgggcgtgccgccaaggacgctgacggtgtgatccgcagcaaggcaggagcacagggcgacttccaagtcatgcccaccacgcaggcaacgtgggaagcgcgcaacggtcgcaagtacgacatgcgcaacttccaagacagcatcgagctgtatgccgacatcatgcgcgagaacatgcagcttgccaagggcgacgtgacgaaggcgctgcgcatctaccaaggcggcaccaatccgaagaactgggggcaggagaacgcagcctatgcaccgagcgtgctgggcggtgcgtccgctcccgcagtgtcggcgcagccgcgcagcctgaccaccacgcaggcagacctcaacgccgcatggcagggcaacccgaacatgcgcgaccgtacgtggtccggtgcgtccatcccggatgcgtggacgggtgcgcccatcgaaggccgcaacgctctggcgtcggcagcgaaggaacacatcggcaagattcgtgcgggcatcgccgagctgtcgatgggtcaggtagcacaggaaggtggcaccgccgcgcaggccgtaggcaaggctcaggctgtccgtgcatcggatcaggttgtgccgtggtgggtgcgtcaggaagtggacgtgctgaacaccggcgctcgcaaggcgctgctggatcagaccgaacaggcgctcgcgcaggaccgcgcggacgaggagctgcgcaactcgctgaccttcctcgacaagtggggcgctgcgttcgacagcggcatcggtgctgcgatcagcaaccagtttgcgcgcgaggacgagaacgttccggaaggttggaagtacgacccgaaggaatgggagaagccgtggatgactgccgacgaactcgaagacatccgcgatgcagcgtactcgccgaacgagctgaagtacgtcagcgaccgacagttcctgcgccgccactccatgcgcatcaaggatcagcagactggctggggtagcttcggttacgacatggtggcaggcttcaccgatccgggcaactgggctatcggcggcgtcactgccgcaggcgctaaggcgctgggcatcggctcggctgcactcgttgccgaagggcgcgtgggcgcgtcgctcgcgtcggctgctgcggagaacgcggtcggttccgtcatcacggacgccgcgctggttggcatgggcgagcgccgcaacttcgcggacttcatgaccgacgctgcattcgctaccaccataggcaccgcgatgcacattccgggcgtgcgctcggctgcgcagattcgtgacaaggcaaccatcgacctgtccgcaggcaacgctgccgcttacggcgaagcgtggtcggccgacctgaaggcgcgcgctgtggccgagctgggcgaggacgccaacccggtgctggtgaacaaccgcatccaccagcttgccaagcaggaggctgtggattggctgcgcgctggtatggccgacgtgcctgacgacttccgtatcttcgcccgtcccgacgtgcaggagacgaccaccaccgcaggcaccactggtgcactcgcacgggacgcgggcaacgtggacgcaacgaccgggcggtacaacgacagcgtgggtggccgggtcgatcagcatgacccgctgctggaacgcgcatggaagaccgcaggtatcaagggcggtaacgtcgatggcgtgctgaagtatctggaatccaacgcctctatcccggaggacgtgcgtgctatcgccaacgcgctgaagcgtggcgggcggctgagcacggtgaagatcgtgccggaatcggaactcgacaagtggttcgccggtgccaacatgggtccgggtatgcgtgtggccggtggctacaacgccggactggacgcgatggcgatgcggaactacacgccggaagtggtggtgcacgaaatgctgcacgctgccacgctgcgtgagctgcgcagcaactcggtgttcgggcaggaaatggaagaactgctgacccatatcaacaacagcatcggcagtgtggactccacgctgaccaccgctgcgatggagacgcgcatcaaccagccgcaggcaggcttcctcgccaacactgacgagctgatttcctacggcctgacgaaccgcgctgtgcaggcggtgctgcgtcagatgcccgcgccgggcaacacccgcccgaatgcgtgggagtggctgaaggataagatcgcgcgagtgatgggtctgaagaatcaggagtccgcgctcgaacgcctgatgtcggtcgtcggtgacaacctcggcgcggaagtgcgcgacacgcaggccggtacccggcagacgcgtggcatgctcgccaactcgatcttcaagtcgaaccgcgagcgcaaggctttctaccagcgcaccggtctggacaagtccgtcagtgatgacgcgatgcgtgtgcaggtcgccgaagtgatggcacgctccgaacgcttcagtgcgcagtacggcatcgacgcggcgaagctgtccaccatcatgcagcgcttcgggctggaagctacgagcacgactctaatgtcgtccaagtcgccagttgcccgcatgcttgcgatcaccctgttggagaatcccgagggtgcagcaggccgacacagcaccgcagcgatggatcggcatggtcggtttgagtcgttcatgggcacccgcccgcgtcagtgggaagcggcctatcgcctgtggcgtgcggacgtgcgcggtatcggtgcgatcaaggacttcgccacgggctggaaggctcgcgcggacttcgagtacgcagtgaagctgtaccgcgagactcgcttcaacggcggggacatcccggatgcgcacgaggcagtgaaggcaatggcccgtgagttggaccgtggctacaaccgcatggcagcagagcagcgcgcggccggtacggtgggcgcacagcgtctgccggaggaggacgtggagggctacgagtcccgtacgtggctgggcggcagcatcgctgctgctggtccggtgcgacgcgagggtatccgtcaggcgatgcgcgatcagttcgaggtgatgggcgagctgtatggggacgacttcctcgataagttcgctaccaagtatctggaacgcatcgagcgcaaggctgcgggtgtcatcgaagcgccgggtcaggtcttctcggagtcgcaggcggacacgctgcgcgacactctgcgggcgatgtcgctcaacgaggaggagattcagaaggtcatgggcaagtacagccgtggcggtgcgaagcacaccaaggcgcgtatcgacctcgacgtgaccaagcagtacgaggacgctgacggtaagttccgtctgatggactatctcgacaaccgcgtgatggacaactaccgcaagtacgcgggacgtgttgctggtgacatcgctctggcgaagcacggcatcctcggcgacgcaggcatcaacgtggcgcgcgaagcaatgcgcctgaccggtgccaacgatgtggagctgaaggcgttcgagcaggtgatgtccgagttccttggtcgcccggtcggtaccggcgatccgactgttctggcgaatgcgcgtctgctgacctcggccatccagctgggcggcgcgggcatcaatcaggcagcggagtacagcaacggcctcgccgctgttggtgctgctggtgtggctgacgcaatccgtatcgctccccgcatgcgcagcgaaatcatgcgcatcctgaagggcgaggacagcggcaaccaaatcctcgacggcttcgagttcatcagcggtcgcggcttcggtctcgccggttacgacctacacatgttcaactcgctggacacgcaggcgtcgatgtatggtagcgagcgcgcaggcttcctgacctcgctggtgcagaaggcagcgcatgcgaaccgcatcctctcggggcagcgggccgtgcttgctgtgcagcagcgtggcttcgcggaagtgctgatcgccaagggcgtgaagttcctgcgtgatggtgctgaagctgacaccgccctgaaggacatgggcattgacgacaacctgctgaaccgcctgcgggctacgcaggatcaggtcgtgcgctggggcgcggatggtaagctggaagcagtagacccgcgcaacgtcgaggggctggcggatcggcaggcatggttggcgttctacaacgcgatcaaccgtggcacctcgcagattcttcaggacaccttcatcggcgagactggcaagtgggcgcacaacggctggctgaagctgctgttccagcaccgcacgttctcgctggtcgcgcagcagaagcagctgggccggtacgtgggcaactacggtgcatggcagacggcgggcctgatcgctgctgcgatggctgtggcggctccgctgcaagccctgcgggtgctgtcccgcgtggccctgatgaacgatcaggagcgcgacgaggccatcgaccagaacatcctgtcgcctctggcgctgggcaaggccacgctgaactacgtgtcggcgacgggtatgctcaacgatgtgctggacgtgggcactggcgtggcgggcggctggtacgagtacgccaccgatacgcagggtccgacgtggctgaagcagctggccggtgggcagttcggcaaccgcaaggaagtggtgggcgggcagttcgcgccgtcgctgggagtcatcaacgacttcgctcagggcattgctggcaagccggagaatctggccgacgtgattccgggcgggcgactgccgatggtgatcccgctgctgaagggcgcagccagccagtggaaggaggagtaagatcagggccaaggacggcccacccttttggtacacctatagcaaacaggaggcagcatggcagttccagacccgcagctgcgctacgcgacagacgtgttcgacgccgatggcgtgaccactgactggcagatcagctttaccggtggctacatcaacccgtcccacgtgtacgccatgagcggactgctggacgaggagactcagctgctgaccgaccggactccgcacaccgtggaagtcctgagcgaagacgatgacgctagtaccgtccgagtctcgcctgccgtcgccgctgggcgcaagctctacatctaccgcagcactccggtgcagcagatgctcgttgactacgttaacggtagcatcatcagcaagacaaaccttaacctcagcaacgaccagctcctgaagatcattcaggaaatgttcgactcactcaacatcgccacccttagcatcgaccagcaggtcggtgtgatcgtggacctgaacgagattatccagaacatctacaagcaggtcaccgagttgctggcagctggtggtatcgtgtccgtcgccccgcgcgtctggtccggtgcttggactggcgatcaggtgggtgacaccgacttcgacatggtgggcgcggacgtatccggcgcgggcttctacgacgtgtacgtcaacggcatcggcatgcagccggacgtggactatcaggtcacgctcgctgacggcaccgatcccagcttcatccgcttcgccacggttcctgccgagggcagcatctggttcgccgtgctgcgtggttacgccaagccctacaccgggcctgcgccgatcaccgctgcgagcctgcgggtgccgatcatcacggcagagggtccgacttactacgccgccaaggctaccgagtacggactcgtgcgctgcacgtacgccggaggttgcgccgtcaacatcaacctgatccccgaagtgggcgacggtgaaaccaagctcgcctcgggcagctacttcagcgtgcagcagaaggcaggccctgtggtcatcactggcgacgtgggcgtgacgctcgaagtcccggtcggctgcaccgccgcaactcgcggcaccaactccgtcatcactgcaacgtgcatcgacggcgacaccaacacgtggttgctctcgggcgacttggctaaggagtaagcatggctaatcacttcaggctgtacggccgaccgctcatggcggacgaggttgcagatggcctgtcggtgacgggcgtgctggaagggtacacggcgggcgaggcttacgagtctcgcctgtccatcaacaacccagtcggccgctgcaccgtggaggtcatcgaatcgacgctcccttcgggcgctgcggtacgggtggacaacatcaccaaggaagtcgtcgtcaagtgggcggctttcactgaagtcgtggacgaggaaaccctcgtgcccaacggcgacttcgaggcaggcgacgacggcacgtggttgccgggcggtggatcgaatggcgaaggctggtcgattggcactggctcagactacgacaccgacagcggcgtgtacagcgcgcgcttcgccaacatcaagacgggcggcagcgacctgctcaacccgctgatccctgccaaggtcaacgactacatccgatgcaccgccgaggtccagcagggcgcaagctccaagggcaaggccggtgctcgtgtgtcgatcatctaccgcaaggaggatgggaccgagctgcaacgcaactggggcaacatggtttcctccggcagcaacggtgcgtggcaccagtccgttgccgaaggcgctgcgcccaaggacacgaagtacgtgcaggttgtactgtcggcgttccgcagcaagcagaacaaaccgctgtgggtggacaccgttaagtggaaccacaagtacgtactgggtcagaacgacgacagctcctacttccttagcatcaaggtcacggacgggttgaaccgtgtggcctactggtccggtcgtatcgaggagcagggcatctacgttacgtccaagctctacagcttctaccagttcgatgccgcgatgctgaccagcagctttgctgggtacagcaacatcgacatgctccagcctttggatactgcgtcgctgggttcctccttcgtaagctgggaactccgaagctctaggcaggattatgccgccgacccggagagcacgttgtacgggagcgctttcgtttcgttcgacatccgatccatccgtaaggactacacgcctgacccggagacggcgaagctgtcgagttctttccattccttcaccctgaagcagcaccctgtagtcaaccagccgctcgacgcgactgcacgactccggtctggcttcgtatcatggagcttcgcatgatccacaatcacctcggcattgctggcgtgttcaccatcagcaagggtaagtccctcgatactctcgaagttgtagccgactggcagagcaaccttatcacggacggtggtatggacgcactgggtgataccggcagcggctatcctcgcagcatgtacgacctcattgcttacttggcagtcggtagtggcagcgccaccccggcattcaccgataccgctcttggtgcacaggtggcgcaggttggtcgtacgtcctcggacagcggtgggactaccactgccccgtactacgcctactcccgctgccagtaccagttcccggctggtaccgctactggcgttctgtcggagcttggtgccaaagcatacaacaacaataccggcgcgtacatcctgaccacccgtgcgcttatcaaggactccgcaggtaacccgaccaccatcacggtgctgtcggatgaaatcctcgtggttacttacgagctgcgcatgtacgcagataccacgccggttgtcactactgagacgatcaagggtgttagcaccactgttacctgtaagcctattgcaatgggccgcagcggcggtatgaacggtcagtcggcagtcgcttggtcggactacgtgtgggggtgctactacttctacggcggtactggcgacggcaccggagctatcaccgaccagtatccgccggggacgattgccagcttctctgacttgcagcttcagcaggtagcctatgttccgggtacttactaccgtgactgcgtttgccggatgtcgatcaacaacgtgcccggtggtccgatcacggctgcaatgggactctccgcgtgcgtgaccttccaagtcggcttcaatccgggtatcaccaagaccggatcggagacggcgaacttgcgcatgcgggtttcttggagccggtacacgccatgatccccactgtctcccaaagcatccaacgcggtgactgggtggagcagcagaatcggcgcacccgcccgctcattgacttcgagcagggcgggctgactctcaacgcagcagtggacgacctccaagctgcgctgtggactgccgagagtgacggcagcagcgtcgtcgtttaccgcgacggcgttgccccggtcaccgtgctgaccgactccgggatcacgcagatcgcactggccttcgaccagaccatgcgcccgcacgtggcgtacatggcgggcggtgtgtgcaagttctactggtacgacacggtggctgcttcgatgcagaccatggtgatccccggtgctaccactccgcgcctgtgcatggacgagaagcgggctgtcttcgccacgcagagcgacgtgctcctgtcgtacaagaacggcagcaacctgtgcgtacgcgcgcagcgtgagcgcttcgcaaccgaacatgtgatcgcctcgggaatccccggcgacctgattgcggtgggcatgaacaacgtcaaccgcctgcaatggaagctcgtcggcaatcccgacgactggccctaacctacaggagaacagcatgaccccgccgagtgtggtcaatgaggtcgtccgaacctcgccgcttacgctcggcgcggtctacctcaacttcatcagcacgtacggtgctgccatcgtaactacgctcgccattctgtacgccgtcgctcagttctactggcgggcacgcgagcaccgaaagatcatgggaggcaaggatgtcgaatccggcaagtgagggcgcactcggtgcgctgcacgaactggtcgcgcgtgcgctgatgcagcgcatccaagatggcgagctgtgcaccgcagccgacatcaatgcggcgatcaagttcctgaaggacaacaacatcacggcgacgcgcgaggccaacaaggcactcggcgagctggaagacgagctgggcaagcactcgctgcctccggctgacgacgacgagttgcagcgtgcactcgacaacatcgttcactttccggggagcgtagccaacaatgcgtgaatcagctgaagcggccgacgtgcgccgcaagaagttggagctgttgcagaaccactaccggcacttcgccaccttcatgcgcgacattatgaaggtgctggggttcgagccgacgtggatgcagtacgacatcgccaactacatgcagtatggcccgcacctcgcaatggtgcaggcgcagcgaggcgaggcgaagtccaccatcgctgccatctacgccgtcttctgcctgatccacgatcccactcaccgtgtgctgatcgtatcggcaggcggcacgcaggcatccgagattgctacgctgattcagcgcatcatcctcacggtgccgacgttggagtgcatccgcccggacaagaacgcgggcgaccgtacctccgtggatgcgttcgacgtgcaccactcgctgaagggaatcgacaagtccccgagcgtggcgtgcatcggcgtcaccggcaacctgccgggtaagcgtgcggacctgctgatcgccgacgacgtggagtccaacaagaacagccgcactgccgcgaaccgtgagctgctgctgaccatcacgttggagttctcggccatctgcaccggcaagcccggtactccgggtcgcatcctgtacctcggcacgccgcagaccggcgactccatctacaacaccctgcccggacgtggctacgacgttcgcatctggcccggtcgctacccgaccccggcacagcgcgagcactacggcccgcatctggcaccgtctatcgtgcagcgcctagaagccgacccgatgttggcgttcggtggtggcccgatgggcgacgagggccagtgcaccgacgagctgttggccggtgagcagaagcaccagtccgagctgcgtcagcgtggaccgtccagctatcagctgaactacatgctcaacacgcggctgatggatgcgctgcgcttcccgctgaagaccgagaacctgatcgtgatccccggtggtggcgaccgcttcccgctgacgatcacccgtggcctgagcaacgctcaccagcgcagcttccagtccagtgggtacggcttcgtgatgatgatgccgcacgacatgagcaccgagactgcccccgtgcagggcgtgcacatgcagatcgacccggccggtggtggtgccaacggagacgagacggccttcgccgtgaccgccttcctcaactccaccgtgtacgtgttggccgtgggagctgtgcccggtggctacgacggtgatggcttgctagaactgcgccgcattgcggtgaagtacaagccgaacgtcatcagcatcgaaaagaacatgggctacggcgcgttcgccaaggtgttcctgcctgtcctgcgagaagatcgcggcacggagaagggatacaagggcgacatccgcgaggagttcgtgaccggcaacaaggaagcccgtatcatcggcactctcgaacctgtcatggctcgcggctcgctggtcatgctggaatccgtggttgaaatggatcacgagtacacccagcgctacgccaccagcggcaagcgtcaggtctacagcctgttccaccagatggcgaagatcacgcagcagaagggcagcatcgcacacgatgaccggctcgatgcactggaaggtagcgtgcgtcactgggttgcgcagcttgcactggaccagaacaaggccatcgccaagcagcagcagcgagagttccaagactggatcaacgatccgaccggcatgaaggcagcgacccgcaagagtccgctgcaacgtggccgtccatccctactcgaccgttaccggaggtaaccaatgcagaagtccgacttcaccagcaactacacgggtctgttcggccgtggcaactacctgcaccgcgaactgctcgccctcatggagcacgcagagcagcatcccgcaaccgcagcgcagctgctcgcgcagttccagaaggacgccaccctcgtgctggacgccctgatcgctgcgggcgcacgcaccgcgtcctcgggtccgaactccggcccgcacactccggtcgatctggacccggatgacgacccactgaccccgtaaggagcaaccatgaaccagcagcagaaccaagataccagcaacaaggggctgttcggcctgatcggcggcatcttcatcggcatttcggcaacgctgctgtcattcacccaaggccacgaaggggtacgctacgctgcgtacctcgacaccggccgggtgccgaccatctgctacggccacaccaagggcgtagcgatgggcatgacggcaacgaaggcacagtgcgacaagtggctgatcgaagacctacagatcgcccagcagggcgtgcgcaagcacctgaaggcccccgttaaccgcaaccagatcgacgcctacacagacttcgtgttcaacgtaggtgagaaggcgttcgccgacagcaccatgctgcgcaaagcgaacgcaggggatcgtgaaggtagctgcaaggagttcctgcgctgggtctacgtcggtaagctcgactgccgactgtccagcagccgttgctccggcatccccaagcgccgcgacgcagagtttgctctgtgcttgcgccccaacaacgaggtgatccaaccgtggaaaccccaagtgaagtgatcgcgcggctcggcggcaagctggttggcttgctgctggtcgtgaccatgttcgtgtgcttcggtctgtacgtctacggcctgcaacgcaaggtggagaagctggaaactgcccaagtcggcacgaccgctaccgccaaggcggcgcagacgcaggctaccgggtacgcgacctacatcaaagagaaggaggacgtgcgtgttcgcactgaagaagttcttgacgctgccccggagtaccgggatggcactgttcctgctgatgtcgctgacctcctgcgcgaacctgccggtccctgacgactccctgcttgcagactgccacatcacctacctcggtggggagaagggcaccacctcctcgcaggacaaggtggtcaagctcgcgcaggaccgccgcatggacaccgttctgtgcaacaaggacaaggctgcgctgcgtgcgtggaaggccgaggtgtgcggtaccggtaagcgccggtgtacgggtgacaaatgaccaccatcgcatgggacggcaagcacctgtgggccgatagtcaggccacgcagggcgaccacaagcacaccgtgcgtaagatcatgcccgtatcgacacccaccggccctgtgctgctgggtgtcaccggggatttcacagtgcttcgcccggttctcgctgcgcttaaagcgggcgaaggctacgaggagcacgttggcaagtccgcgacggtgcttgtggttaaggacggcgtactcacggtcactactggtaagcagcagtgggtcgaggaggctccgtacttcgatggcagtggcaaggcgctagctctaggggcctatcatgcgagcaagtctgtggctaaggccatggctgctgcgatagctcacgatgtctacagctccgggcctatcgtcaagctaaaggcaccagttcgcgaggcttaggagtaaggccacgtgggtagccggaccaaaatttgcttcggaaatgcgcgggggtcactccaatagaagctcccgcgcgtgcccccgtacgccctcgcgttacgcgcctgcgggtgtgcgtgggtgcgtgcccgcgtgtgcgcctgtgtgcgcgtctgtgcgcccgcgtcaaggttccgcgtgggtgtacccgtgtgcctgcctgcgtgggcctgagcgtgcgtgtgcgtggccgtgcgtgggtgcctgcgggtgggcgtgcgggtgggcgtgcgcctgctgcctgtatggctggaccgc

SEQ ID NO: 21 - DNA, 44482 bp, unidentified
  source 1..44482: mol_type = genomic DNA
tcccggccacccgtcaagcacaatctgcgagagatttattaaccattcagccaaggcggcacggtccagccatacaggcagcgcaagcgtacacgcgccgtaggcgcaggcaggcgcacccgcccacgcaggcacacgcacggccgcacaggcgcgcccacacgccacgcgcaggcaggcacaggcacacacccacgcggaaccttgacgcgggcgcacagccgcgcacacaggcgcacacgcgagcacgcaggcgggcgcacccgcaggcgcgtaacgcacgggcgtatgggggcacgcgcgggagcttctattggagtgacccccgcgcatttgggaagcaaattttggtccggctacccgcgtggccttatgactaagccttgcgaactggtgcctttagcttgatgataggcccggagctgtacacatcgtgagctatcgccgcagccattgccttagccacagacttgctcgcatggtacgcccctagagctagcgccttgccgctgccatcgaagtacggagcctcctcgacccactgctgcttaccagtagtgaccgtgagtacgccgtccttaatcacaagcaccgtcgcggacttgccaacgtgctcctcgtagccttcgcccgctttaagcgcagcgagaaccgggcgaagcactgtgaagtccccggtgacacccagcagcacagggccggtgggtgtcgatacgggcatgatcttgcggacggtgtgcttgtggtcgccctgtgtggcctgactatcggcccacaggtgcttgccgtcccatgcgatggtggtcacttgtcccccgtacaccggcgcttgccggtaccgcacacttcttccttccacgcacgcagcgcggccttgtccttgttgcacagaacggtgtccatgcggcggtcttgtgcgagcttgaccaccttgtcctgactggaagtcgtcccgcgctcaccaccgaggtaggtgatgtggcagtccttcagcagatcatcgctgggaaccggcaggttcgcgcaggaggtcagcgacatcagcaggaacagtgccgtcacgatactcgggaacggcgtcgagagcttcttcagtgcgaacacgcacgtcctccttctctttgatgtaggttgcgtacccggtagcctgagtctgcgcagccttggcggtagcggtcgtgccgacttgggcagtttccagcttctccaccttgcgttgcagaccgtagacgtacagaccgaagcacacgaacatggtcacgaccagcagcaggccgatagccttgccgccgagccgcgcgatcacttcacttggggtttccacggttggatcacctcgttgttggggcgcaggcagagggcaaactctgcatcgcggcgcttgggaatgccggagcagcggctgctggacagtcggcagtcgagcttgccaacgtagacccagcgcaggaactccttgcagctaccttcacgatcccctgcgttcgccttgcgcagcatggtgctgtctgcgaacgccttctcgcctacgttgaacacgaagtccgtgtaagcgtcgatctggttgcggttaacgggaaccttcaggtgcttgcgcacgccctgctgggcgatctgtaggtcttcgatcagccacttgtcgcactgtgccttcgttgccgtcatgcccatcgctacgcccttggtgtggccgtagcagatggtcggcacccggccggtgtcgaggtacgcagcgtagcgtaccccttcgtggccttgggtgaatgacagcagcgttgccgaaatgccgatgaagatgccgccgatcaggccgaacagccccttgttgctggtatcttggttctgctgctggttcatggttgctccttacggggtcagcgggtcatcatccgggtccagatcgaccggagtgtgcgggccggagttcggacccgaggactgcgtgcgcgcaccggcagcgatcagggcgtcgagcacgagggtcgcgtccttctggaactgagcgagcagctgcgctgcggttgcgggatgctgctccgcatgctccacgagggcaagcagttcgcggtgcaggtagttgccacggccgaacaggcccgtgtagttgctggtgaagtcggacttctgcattggttacctccggtaacggtcgagtagggatggacggccacgttgcagcggactctttcgggtcgctgccttcatgccggtcggatcgttgatccagtcttggaactctcgctgctgctgcttggcgatggccttgttctggtccagtgcaagctgcgcaacccagtgacgcacgctaccttccagcgcatcgaggcggtcatcgtgtgcgatgctgcccttctgctgcgtgatcttcgccatctggtggaacaggctgtagacctgacgcttcccgctggatgcgtagcgctgggtgtactcgtgatccatttcaaccacggattccagcatgaccagcgagccacgagccatgacaggttcgagcgtgccgatgatgcgggcttccttgttgccggtcacgaactcctcgcggatgtcacccttgtatcccttctcggtaccgcgatcttctcgcagcacaggcaggaacaccttggcgaacgcgccgtagcccatgttcttttcgatgctgatgacgtttggcttgtacttcaccgcgatgcggcggagttcgagcaggccgtcaccgtcgtagccaccgggcacagcgcccacggccaacacgtacacggtggagttgaggaaggcggtcacggcgaacgccgtctcgtctccgtttgcaccgccaccggccgggtcgatctgcatgtgcacaccctgcaccggggcagtctcggtgctcatgtcgtgcggcatcatcatcacgaagccgtagccgctggactggaagctgcgctggtgcgcgttgctcaggccacgagtgatcgtcagcgggaagcggtcgccgccacccggaatcacgatcaggttctccgtcttcagcgggaagcggagcgcgtccatcagccgcgtgttgagcatgtagttcagctggtagctggacggtccacgctgacgcagttcggactggtgcttctgctcaccggccaacagctcgtcggtgcactgcccctcgtcgcccatcgggccaccaccgaacgccaacatcgggtcggcttcgagacgctgcacgatggacggtgccagatgcgggccgtagtgctcgcgctgtgccggggtcggatagcgaccgggccagatgcgaacgtcgtagccacgtccgggcagggtgttgtagatggagtcgccggtctgcggcgtgccgaggtacaggatgcgccccggagtgccgggcttgccggtgcagatcgcggagaactccaacgtgatggtcagcagcagctcgcggttcgcggcagtgcggctgttcttgttggactccacgtcgtcggcgatcaggaggtcggctcgcttacccggcaggttgccggtgacgccgatacacgccacgctcggggacttgtcgatgcccttcagcgagtggtgcacgtcgaaggcgtccacactggtgcggtcgcccgcgttcttgtccgggcggatgcactccaacgtcggcaccgtgaggatgatgcgctgaattagcgtagcaatctcggatgcctgcgtgccgcctgccgatacgatcagcacacggtgggtgggatcgtggatcaagcagaagacggcgtagatcgcggcgatggtggacttcgcctcgcctcgctgcgcctgcaccattgcgaggtgcgggccgtactgcatgtagttggcgatgtcgtactgcatccacgtcggctcgaaccccagcaccttcataatgtcgcgcatgaaggtggcgaagtggcggtagtggttctgcaacagctccaacttgcggcgacggatgtctgccgcttcggctgattcacgcattggctacgctccccggaaagttcacgatgttgtcgagcgctgcttgcagctcggtgtcgtcggcctgcggcagcgagtgcttgccgagttcgtcttccagttcgccgagcgccttgttggcctcgcgcgtagccgtgatgttgttgtccttcaggaacttgatcgcggcattgatgtcggctgcggtacacagctcgccgttggcgaggcgttccttcagtaccgtggcgacaagttcgtggagtgcgccaagcgcgccctcacttgcggggttcgacatccttccctcccatgatcttgcggtgctcgcgcgcgcgccagtagaactgggcgactgcgtacagaatggcgagcgtagttacgatggcagcaccatacgtgctgatgaagttgaggtagaccgcgccgagcgtaagcggcgaggttcggacgacctcattgaccacactcggcggggtcatgctgttctcctgtaggttagggccagtcgtcgggattgccgacgagcttccattgcaggcggttgacgttgttcataccaaccgcgatcaggtcaccggggattccggtggcgatcacgtgttcggttgcgaagcgctcgcgctgtgctcggacgcacaggttgctcccgttcttgtaggacagtagcacgtcgctctgcgtggcgaagatcgcccgcttctcgtccatgcacagacgtggcgtagtagcaccggggatcaccatggtctgcatggaagcagccaccgtgtcgtaccagtagaacttgcacacaccacctgccatgtacgcgatgtgtgggcgcatggtctggtcgaatgccagtgcgatctgcgtgatgcccgagtctgtcagcacggtgacaggagcaacgccgtcgcggtaaacgacaacgctgctgccatcactctcggcggtccacaacgcggcctgaaggtcgtccacggatgcgttgagagccagcccgccctgctcgaagtcgatgagcgggcgggtgcgccgattctgctgctctacccagtcaccacgttggatgctttgggagacagtggggatcatggcgtgtaccggctccaagaaactcgcatgcgcaggttcgccgtctccgagccggtcttggtgatgcccggactgaagccaacttggaacgaggcgcaagccgagaggcccatagcagccgtgatcggaccaccgggtacgttgttgatcgacatgcgacacaccacgtcccgatagtggctaccggcaacgtaggccacatactgaatatgcaagtccgagtagctgacgttggttcccggaggatactggtctgtgatcgcgccggtcccgtctccggttccgccgtagaagtagtagcagccccaaacgtagtccgaccacgcaatggccgattgcccactgagcgaaccactccggccgagggcgatgggcttgcaagtcacagtggtgctgacgcccttgatcgtctcagtcgtcaccaccggagtcgtgtcgatgtagagacgcagctcgtaggtcaccacgaggatttcatccgacagcaccgtgatggtggtcgggttacctgcggagtccttgataagcgcgcgcgtggtgaggatgtaggtaccgttgctgctgttgtacgccttggcacccagttcggaaaggacgccggtagcggtgcctgccgggaactggtactggcagcgggagtaggcgtagtacggagccgtggtggtgccgccgttgtccgaagtcgtacggccaacctgcgcaacctgcgcgccgagagcagtgtcggtgaacgcaggggttgcgctaccgctgcccactgccaagtaggcaatgaggtcgtacatgctgcggggatacccgctgccggagtcacccagtgcgtccatgccaccgtcggtgataaggttgctctgccagtcggcgacaacttccagagtgtcgagggacttacccttgctgatagtgaacacaccggcgatgccgaggtgattgtggatcatgagaagctccatgatacgaagccggaccggagtcgagcagtcgcgtcgagcggctgattgacaacaaggtgctgcttcatggtgaaggaatggaaggaactcgacagtcgcgccatctccgggtcgggtgtgtagtccttgcgaatggatcggatgtcgaacgaaacgaaagagctaccgtaggaaaggctctcctcagcggcgtaatcctgacgcgagctgcgcagttcccagcttacgaaggaggaacccagcgacgcagtatccaaaggaggcagcatgtcgatgttgctgtacccagcaaagctgctggtcagcatcgcggcatcgaactggtagaagctgtagagcttcgacgtaacgtagatgccctgctcctcgatacgaccggaccagtaggccacacggttcaacccatccgtgaccttgatgctcaggaagtaggagctgtcgtcgttctgacccagcacgtacttgtggttccacttaacggtgtccacccacagcggcttgttctgcttgctgcggaacgccgacagcacaacctgcacgtacttcgtgtccttgggcgcggcaccttcggcaacagactggtgccacgcaccgttgctgccggaggaaaccatgttgccccagttacgttgtagctcggtcccatcttccttgcggtagatgatcgacacgcgagcaccagccttgcccttggagcttgcgccctgctggacttcggcggtgcatcggatgtagtcgttgaccttggcagggatcagagggttgagtaagtcgctaccgcccgtcttgatgttggcgaagcgcgcgctgtatacgccgctgtccgtgtcgtagtccgagccggtgccaatcgaccagccttcgccgttcgatccgccgcccggcacccacgtgccgtcgtcgcctgcctcgaagtcgccgttgggtacgagggtttcctcatccacgacttcagtgaaagccgcccactttacgacgacttccttggtgatgttgtccacccgtaccgcagcgcccgaagggagcgtcgattcgatgacctccacggtgcagcggccgactgggttgttgatggacaggcgagactcgtaagcctcgcccgccgtgtacccttccagcacgcccgtcaccgacaggccatctgcaacctcgtccgccatcagcggtcggccgtacagcctgaagtgattagccatgcttactccttagccaagtcgcccgagagcaaccacgtgttggtgtcgccgtcgatgcacgttgcagtgacgacggagttggtgccgcgagtcgcggcggtgcagccgaccgggacttcgatggtcacgcctgcgtcgccagtgatgaccactgggcctgccttctgctggacgctgaagtagctgcccgaggcgagcttcgtctcaccgtcgcccacttcggggatcaggttgatgttgacggcgcagcctccggcatacgtgcagcgcacgaggccgtactcggtatccttggcggcgtagtaggtcggaccctctgccgggatgatcggcactcgcaggctcgcagcggtgatcggcgcaggcccggtgtaaggcttggcgtaaccacgcagcacggcgaaccagatgctgccctcggcgggaaccgtggcgaagcggatgaagctgggatcggtatcgtcggccagagtgacctgatagtccacgtccggctgcatgccgataccgttgacgtacacgtcgtagaagccagcgccggacacgtccgcgcccaccatgtcgaagtcggtgtcgtccacctgatcgccggtccatgcaccggaccagacgcgcggggcgacggacacgataccaccagcggccagcaactcggtgacctgcttgtagatgttctggataatctcgttcaggtccacgatcacaccgacctgctggtcaatgctaagggtggcgatgttgagcgagtcgaacatttcctgaatgatcttcaggagctggtcgttgctgaggttaaggttggtcttgctgatgatgctaccgttaacgtagtcaacgagcatctgctgcaccggagtgctgcggtagatgtagagcttgcgcccagcggcgactgcaggcgagacacggacggtgctagcgtcatcgtcctcgctcaggacttccacggtgtgcggagtccggtcggtcagcagctgagtctcctcgtccagcagtccgctcatggcgtacacgtgggacgggttgatgtagccaccggtaaagctgatctgccagtcagtggtcacgccatcggcgtcgaacacgtctgtcgcgtagcgcagctgcgggtctggaactgccatgctgcctcctgtttgctataggtgtaccaaaaagggtgggccatccttggccctgattctcactcctccttccactggctggccgcgcccttcagcagcgggatcaccatgggcagtcgcccgcccggaatcacgtcggccagattctccggcttgccagcgatgccctgagcgaagtcgttgatgacgcccagcgcgggcgcgaactgcccgcccaccacttccttgcggttgccgaactgcccaccggccagctgcttcagccacgtcggaccctgcgtgtcggtggcgtactcgtaccagccaccagccacaccggtgcccacgtccagcacatcgttgagcatgcccgtcgccgacacgtagttcagcgtggccttgcccagcgccagaggcgacaggatgttctggtcgatggcttcgtcgcgctcctgatcgttcatcaggaccacgcgggacagcacgcgcagggcttgcagcggcgcagccacggccatcgccgcagcgatcaggcccgcagtctgccacgcaccgtagttgcccacgtagcggcccagctgcttctgctgcgcgaccagcgagaacgtgcggtgctggaacagcagcttcaaccaaccgttgtgcgcccacttgccagtctcgccgatgaaggtgtcctgaagaatctgcgaggtgccacggttgatcgcgttgtagaacgccaaccatgcctgccgatccgccagtccctcgacgttgcgcgggtccaccgcttccagcttaccgtcagcgccccagcgcacgacccgatcctgcgtcgcccgcaggcggttcagcaggttgtcgtcaatgcccatgtccttcagggcggtgtcagcctcggcaccatcgcgcaggaacttcacgcccttggcgatcagcacttccgcgaagccgcgctgctgcacggcgagcacagcccgctgccccgaaaggatgcggttcgcatgcgctgccttctgcaccagcgaggtcaggaagcccgcgcgctcgctgccgtacatcgacgcctgcgtgtccaacgagttgaacatgtgcaggtcgtaaccggcgaggccgaagccgcgaccgctgatgaactcgaagccgtcgaggatttggttgccgctgtcctcgcccttcaggatgcgcatgatttcgctgcgcatgcgaggagcgatgcgaatcgcgtcagccacaccagcagcaccaacagcggcgaggccgttgctgtactctgctgcctgattgatgcccgcaccgcccagctggatagccgaagtcagcaggcgtgcgttcgccagaacagtcggatcaccggtgcccaccgggcgaccgaggaactcggacatcacctgctcgaacgccttcagctccacgtcgttggcaccggtcaggcgcattgcttcgcgcgccacgttgatgcctgcgtcaccgaggataccgtgcttcgccagagcgatgtcaccagcaacccggcccgcgtacttgcggtagttgtccatcactcggttgtcgaggtagtccatcagacggaacttaccgtcagcatcttcgtactgcttggtcacgtcgaggtcgatacgcgccttggtgtgcttcgcaccgccacggctgtacttgcccatcaccttctgaatctcctcctcgttgagcgacatcgcccgcagagtgtcgcgcagcgtgtccgcctgcgactccgagaagacctgacccggtgcttcgatgatacccgcagccttgcgctcgatgcgttccagatacttggtagcgaacttgtcgaggaagtcatccccgtacagctcacccatcacctcgaactgatcgcgcattgcctgacggatgccctcacggcgaaccggaccagcagcagcgatgctaccacccagccacgtacgggactcgtagccctccacgtcttcctccggcagacgctgtgcgcccaccgtaccggccgcgcgctgctctgctgccatgcggttgtagccacggtccagctcacgggccattgccttcactgcctcgtgcgcatccgggatgtccccgccgttgaagcgagtctcgcggtacagcttcactgcgtactcgaagtccgcacgtgccttccagcccgtggcgaagtccttgatcgcaccgatgccgcgcacgtccgcacgccacaagcggtaggccgcttcccactgacgcgggcgcgtacccatgaacgactcgaaccgaccatgccgatccatcgccgctgtgctgtgtcggcctgctgcaccctccgggttctccaacagggtgatcgcaagcatgcgagcgacaggcgacttggacgacatcagggtcgtgctcgtagcttccagcccgaagcgctgcatgatggtggacagcttcgcagcgtcgatgccgtactgcgcactgaagcgctccgagcgtgccatcacctctgcgacctgcactcgcatcgcgtcgtcgctgacggacttgtccagaccggtgcgctggtagaacgccttgcgctcgcggttcgacttgaagatcgagttggcgagcatgccacgggtctgccgggacgcggcctgagtgtcgcgcacttcagcaccgaggttgtcaccgaccacagacatcagacgttcgagcgcggactcctgattcttcaggcccatcactcgcgcgatcttgtccttcagccactcccacgcattcggacgggtgttgcccggcgcaggcatctgacgcagcaccgcctgcacggcgcggttcgtcaggccgtaggaaatcagctcgtcggtgttggcgaggaagcctgcctgcggctggttgatgcgcgtctccatcgcagcggtggtcagcgtggagtccacactgccgatgctgttgttgatgtgggtcagcagttcttccatttcctgaccgaacaccgagttgctgcgcagctcacgcagggtggcagcgtgcagcatttcgtgcaccaccacttccggcgtgtagttccgcatcgccatcgcgtccagcccggcgttgtagccaccggccactcgcatacccggacccatgttggcaccggcaaaccacttgtcgagttcagactccggcacgatcttcaccgtgctcagacgaccgccgcgcttcagcgcattggcgatagcacgcacgtcctcggggatcgaggcgttggattccagatacttcagcacgccatcgacgttgccgccacggatgcctgcggccttccacgcacgttccagcagcggatcatgctgatcgactcgaccacccacgctgtcgttgtaacgaccggtcgaggcgtccacgttgtccacgtcacgcgccagtgcaccagtggtgcctgcggtggtggtcgtctcctgcacgtcgggacgcgcgaagatgcggaagtcgtccggcacatcagccataccagcgcgcagccaatcgactgcttcctgcttggcaagctggtggatgcggttgttgaccagcaccgggttggcgttgtcgccaagctcggccacagctcgcgccttcaggtcagccgaccacgcttcgccgtaagcggcagcgttgcctgcggacaggtcgatggtagccttgtcccgaatctgcgcagccgagcgcacgcccggaatgtgcatcgcggtaccgatggtggtggcgaacgctgcgtcggtcataaagtccgcgaagttgcggcgctcacccataccaaccagcgcggcgtccgtaatgacggaaccgaccgcgttctccgcagcagcggacgcgagggacgcaccgacgcggccttcggcaaccagagccgccgagcctacgcccagcaccttggcacccgcagcagtcacgccgccgatggcccagttgcccggatcggtgaagcctgccactaggtcgtagccgaagctcgaccagccggtctgctgatccttgatgcgcattgagctgcgacgcatgtactgtcggtcgctcacgtacttcagctcgttcggcgagtacgcagcatcgcggatgtcttccagttcgtcggcagtcatccacgacttctcccactccttcgggtcgtacttccaaccttccggcacgttctcgtcctcacgcgcgagctggttgctgatcgcagcaccgatgccgctatcgaaagcagcgccccacttgtcgaggaaggtaagcgagttgcgcagttcctcgtccgcacggtcctgtgcgagagcctgctcggtctgatccagcagcgccttgcgtgcgccggtgttcagaacgtccacttcctgacgaacccaccacggcacaacctgatccgatgcacggacagcctgcgccttacccacagcctccgctgcggtgccgccttcctgagccacctgccccatcgacagttcggcgatgcccgcgcgaatcttgccgatgtgttccttcgctgccgacgccagagcgttgcggccttcgatgggcgcgccagtccacgcatccgggatggatgcaccggaccacgtgcggtcgcgcatgttcgggtttccctgccatgcggcgttgaggtctgcctgtgtggtagtcaggctgcgcggctgcgatgacactgcgggagcggatgcgccgcccagcacactcggtgcgtaagccgcgttctcttgcccccagttcttctggttggtaccaccttggtagatgcgcagcgccttcgtcacgtcacccttggcaagctgcatgttctcgcgcatgatgtcggcatacagctcgatgctgtcttggaagttgcgcatgtcgtacttgcgaccgttgcgcgcttcccacgttgcctgcgtggtgggcatgacttggaagtcgccctgtgctcctgccttgctgcggatcacaccgtcagcgtccttggcggcgcgcccgttgccggactctactcgccactgaccgcgcacgatggactccggcactcccgcataagcggcagccttggcaatctgctggtcttgggtcagccccgaaagatcgagtgccattgtctatctccttacagtttgggttggatggaaatgctctgctgaatcgtaccgtcgttcatacgaacgtagccctgcggtaccggggcctgcaactgacgctgctgcttggtgtgcttctcgtactcggccttgatgtcgcgcccatacaccggcacaaccttccagcccttctcgccaacagcgttgacgtacagcaccggctcgccgttctcgctatccttcatgcggaacacgtcagccttcaggccagctcccggctcgatgttgacccggcgtagcgctgcgtcgatggccttctcgatagcgggtccggtttccttcgtgtccatgaagcccagccatgcaccgacgcctccggtcactcgaccttcatcatcgcgcccgttctcccacgcgtacttgcctgcgtcttccagaccgtaggccagcttggcgtgagtagccgcagcctgcaagccttccgcagacgtgtccagcagaccaccgctgtcggtgaccgagcgtacgatggcgcgagcatacgcagcgcggccagagtcgcccagcttgttgccgaacatgccgaggtacttggggttgagcttggcgatagcttccgtaacacgagcctgagtagcctcggattccttacggctggtcgcgtcgaactgcgtagggtcttcggtggtgatttctccacgggccacctcgtaggcaagctcgaagttcacgccaccattctccagagcttgcagcttgttgaagaacgtgttgacgctatccccgaagtacagcgcagcagtagtcgcgccagtcagtcggccctgtacgggctgaccgttcgtgtcgatgcgtgcggcggtggtctgcttcagctccttccactgctggtacagtgcggccgctgccgtgttaggctgatcgcggagcacagcgcgtgccgtggtctggaactggtcggccacccccttcagcacagcgcctcgaccggtgttggcgttccacaccagctgcgacatggcgaccttggggttcgatgccatcgtggcgttccatgcctgcaccgtgtttgcttcgatcagctccttgtccactccggggatgttgatcgtctgcgcgtacgtgccgcgcttgaacgcttcgatgccaccacggatgtcctcctcctgcgcggccagcttctgctgatcggtcagcgcggccttggccgcagcgttgcgctggttgatgacggcttcctgtgcgcggatgtgtgcgcctgcggactgcgccatgatcgaagccagctgtgtgccggagtacagcggtgcgtcgcttcccgtctcggcggcgtaggtcgagttcatttcctcgatcatcgcctgcgacggcttggcaccaatgccctccgatgcgtacatggagacgagcgccatcttctcggcctgctccgggttggcgtcgagccagtcggaacggtaccggtcctgcgcttgcttcacgtactgctggattccaagctgcccatcagggtcaatggcgctcagcacgcccttgctgttgaggaacttcagcgtgtggaactcgccacgatccgcagcgccacggtagaacgccgtgatcgcggacttgtaggactcgtccgtctggtagcgcgaaggcgacagcccatccagcaaggacagctgcgcctgcgtcagcgcctcggtagccttctcgtccattggccggttggtgccgagcatcgccgtgcgcttcgccagttcgttgaagccggtggacgccgacgagttcgcagcgtactgtgctttcaccagctcctgctgctgccacgccgtacgctccttggtgtgcaggtccatgagagaaccagcgcgatccatgaaggtcttctgcaacaccgtgtccgcgaaaccgttgccggtcatccgggcagtggcgaggtcgttgaactccttcgccatcgcctcgggaggaagctgccgcaactccggcatgcggcgcagcaagtcgctctccatttcattgacctgcgagagcgtgttatacatgctcgcgccaatctcgtagttggtgtcgccgaagattttcttgtaccacggttcggtcgcagcaatctcgtccatggtcttaccagcgcgggcggctacgaagccatcccacatctgctgctgcttcagcttggcggtgttcggcgctgccagctcctgcaagaactctggcaggttgctgtccggcatcgtcataccaccagtgcttgcgaaccagtcgttgccggattgaaccgggccgaccggattcacaccagcgccttgaatgctggtgttgcccgacagtgcgggggtggcgttgatgccaccctgcaatgcggactgcgtgttgaaggtaaccgtgccgatgtcagccattaccatgcacctcctgagttgcccccgctgccgctatcgaaccagccgaggccggacgtagtggtggagaagttgtcgtagttgttgccgaagttgccagtgaccttcgccccagtcacggcctgcttgccggtgccgtcgttgtacccgaaggtagtggacgcccacgacttgccgccgcgatcattggactgctgccatgcctgcatgccgttctgcgctgcgttgctgaaggactgagaggcaccagtgaagttgccgttgtccgcctgccacgtgccgaccgcgaagtctgccacggcctcgcccgccatcggcccaccgaagtaggtagcaacggccacgccgatcagcttgcccaagcgacgcttcatcgcctgcggctcgatgtgctgcgagtagtcgaactgcccgaacgaacggctcatgtccatcccgttccacgcacgcgacatgacctgcgcagtctgcgaggcaccacgcgaggcgaggagagcaacagcgttggcctgcgtctcctgatccatttccgcctgcaaccgcaccatcgaatccatcaggtctgcggacgagccgccgacaccgacagcaccggcctgcgcctgaagtgcaccccgcgcgttcgccagttggagctgggagttaagcccagccccttggcgcgcacgcagctcctccgacagcgcctccatgttggagttgtactccttcgcggctgcgtccagttgggcgttgttcttcagggaccgcatgaaatcagcgaagccggtcttggcgacctcgctgcggttctgattgtcggtctgcgcaacggctgcacggtagttcgcacgggcaactcgggtggtgttgttcgcttgcaggatcgtattaaccgaacccattagctaaccctccgtacattgttgaaagtctgacccgtccagctcaggccggtcacccggagcgggagccaatccttgctgcgaatctcgtaggtgcactcgcgcacttcgcgtccaacgctgatgttgagctgcccccggtacaccggttgccgcgcgatcaggttgtcggagtcgccgaggatgcggccctcgaagtccgtggtggtcacgttgctgttgcgtgtggtcaccgcagcgagcatgcccgcagtatcctctacgtccaccgtcaccttgttgagtgacatgcgtccgtcgagtacggcctgaccattctgatcccgagggaacgggttggtcgggatcaccacagcctcggacaccacaccgtattccagcgcaccagcgtcgaggtcatcgaactgggtaaggaagtcggacgcctgagcgtaaggacagccgagcaggaagtacgggctagtgctattgacggcgatgctcgcgctcgcggtcagtacgcccgtaggtgtaccaaaactcgcccagctatcgaggcacgcatgcgagtccggctcgcccttcgggtcgaacacgtcgcacgccaccagcgatccgcgtgcggtgaacacgaggccgttcttcttgtagctgctcacgccgatgatttcgcccagcgccgggtggtattggaacttcgaccacgagtccacgacacgctgcccgttgttcttgttgtcctcgtaccggtacaggtagaagtcctgcgggtgctctcgcgtgcggaacatgacgaggttcggtgccgtgagcggagtgatctgcaacggcgtgcccgacagccacgagtccagctcgttggacatttcgtccgtcaccgtctgctgcccgttgagtgcgccgactcgcatctgatgcaggctcgtgccttcgctgccgtactgcgcgtagaagatgtagttgcccgaggtctgcgccttcgcatccaccgaatccttgttggcactgaacgccttaatcagtggattcttgggactgaacaccgagtcgccgctgatgccatactgctgccggtcaccgaagatcacgaggtttccgttgtagagcgtagcgtgccggagcacgtcgccctcgctaccgtgagcgaagatttcgatggggtcgctgtcttcgatggtaacggcagagccacgccagaagttcaggtagtccgccgagcgcgaggagttgacgtagttctgtgctccgatcaccagccggtcttggaagacggacagcatcgtgatcggcttgtcgatgaaccacgggatcggcgaggtcagcccgtcgcctgccacccgcgcgccgtaagccggatgctcaccgctgcccggagccagagacgtgaggccagcgccgttacgcgcgatgtagcccacaccgttgtagatgtagagctgggacacgaggttgtcgatggtgcactccacgccgggcgcttcataccagtccaccgagccgtagcccgaagtctccccgttctccaactccgcacgcaggtagtacgactcgtcagcgcctgcaccgctcgggcgcacgcggatgatcttgccgtgccaatggaacttgacggcataggtcgcgtcggtaatctcctgccctgcggcatagaaggtcgtgccgtcgccctcgtcgtcaaccgttatgtccttgaactggtcgtcgtcaatcacgataccgcccttgatgtacgtcgccgacacgcctgcatcgaccagcaaatccgacagctgctcggcgatgtactccgggcgcgtctgctcggcgctcgtcacgatccactcgttgactgcggagttgtactcgttcactctgtcgttgacatacttctggtacgccgggtccggctccgtaccaccgggtaggtagaacgggatgtcgctggtgtcgagcgtgccgggatacgatgcggtcaccgtcttgaacgtcaccgtaagcaccgtgttgtccgtccgcgtcaggttcaccgtgtacgtggtgttgtacttaccgctgcgcacccacgctgcgaggcgctggatgttcgtctgctcctgccacacgttcgtgctagtggcggacgggatcgtggtgttgcccgcgatgtagacgtagctgccgatggctgcgagcgacgatgcgccaccgctgaccagcgtgttgacccacgtgctgttctcgtacaccagcgggatgaacgactcgtccgtcttgttgtagaggaacgcgaaggactcgcttcccaaggtcgaggcgtcgcgccgatacagcagtgcatactccttgccctcctgcatgaagtcgaacacgtccatgttgcgcagctcggccgaggtgacaacggcttgggaagcagcgaaccgcgtaccacgacggcgcacgaggccgttcaccggatcggacagcacgttgatctgctcgtgcgtctggcccggacgacgacggtgcgccggtttctgactgacaccctgaaggatgtcgggataggttccgcctgcctttgccatgttgcctccttagccggggaaagtgtagtggctatgccacgggtgtccgctgtagttgaagtaccgctgacgcagcacgtccacggatgcacgagcgaacagcgggttcgccttgatctggcggatgtgctcggacttcaggttgatgtagctgtcgtcgcgctgctgcttgatctttgcgtacttggtgttgtcgccatcgaagtccgactggaagcgcagcactgcgtcgtcgcgcacgaacatctgcacctcgtaggggaggtcatcgaagtccagcagccgaaccatcttggcctgcacgttgtgatcgaactcgtatgtgttgcgcttgcggtcgtacagtcggcgtccgcgctgtaccacgtggccgaaccggctcgggttacagtccagcttcagcacgtccgtggggaccatgatgtacttgctcgttgcctgcggcttcagctccacccattcggtgttgaaccacagcgcgagcgacgacacgtcgcgggtaacgcggtcgatcaagtcaactgcgtcgtccttgtatacgtggtcatcttccagcgtgttgagcttcgtctcgcccatcgtcttcaagcaggcgttcacgatgtcgagcttggtgatgaatgccatggtgtctcctgagaggaacaaggcagagacgccggagcgccccctgccgggatgttgcttagtccgcagccagagccagcgaggccggtgcgtactcgatgtcctgcgagccgatttcgtcatcaacgaaacggacgcgcacgacccagcccgagccgatggcgtcgtaatggacgcctacgacggtgccaacggagttggcgggcagaccggccacgccagttgcggcgacgacgcggttggaaatctcgaacggtcgatcaaagaccatgatgttgctcctgtgttggtggaaggcgaggcgcggtttgagttacccgaaggattcagggaccgcgcctagcggattaggcaaccttgtcgatgcggcccgcgttctcgacgcgatccagaccaacggcgaaggacatccacgagtccacgaagtagcacttcgaggcgtcgctccaccacaccgaggactgcaacggcagcgcttcggcgatcagcagggccttcggcgacacggccacagcgatcagggtgctgaagtcgccgtcgtagaagtcgtcgttgtcgtcgttcgacagcaggtgaccttcgatcacggtgttcggcaggttctcgctcgacagcaccgggacgccccagccgtggaaggtcgggatgccggtcagcttgttgccgtccgaggtcaggtactcgccgttgctgatctgctctgcctgctgcaacaggtagaagatcgccgggcgcacgatcaggaccacgccatcacgctgcggcttgaccttcttctcctcctccatgcgggagaacagcttgccgatggcggcgtacaccttggccggatcgttctcgtcaccggcggcggcgagcacgacctgcgtggcaccgaagtggccctcgggcgcgcggccgttgcgggtgaagatcgactgcgtggcagcagcggccttggcggcggcgatgctgatggtcaggtccacgaactcggcgatttcctgaccctgctcgatggcgatttccttgcgggtgtcgatgtcggtgaagatttcgtccagctgccagatgctgtgacgcgacagcagcatggtatcgacggtcaccgacgccttgctgaagtccaccggggtgccgtccggcgcgtcaccgcgcttcagcttctgaagcttggtacggccgatggccttcttggtcagggtgttggtgcccttgacctgcttgcgcgggaagaacttttccagcaccgagctggacacgtaggtgtgctcgacatcgccggtgaactgttcgaggatcagcgcgttctcgttgccggactggttgacctgattcggcagaaccgggacggtcgggaagatggtgctcatgctttatgttgctccttggttcttagtggatgacgcgcgcgttgagtgcacgcagttcttcggagtgggccgcaccacggatgcccttctcggcaaccagcttgcggtactcagcgcggtactgctccttcgtgagaggagcgacgccgttgatcgacgcggcgggagcggcggcattggtagccggtgcgcccttgacggtcgtcgcgggattggcctgtgccagagccatcaggtaacgcgcggtcgcctgagcgccgaagccaccagccgacagcgattcgcttgcctgcttcagttggtcggcgggcaggttggcccgtgcgaactgctggatcgcagcccagttctctgcgccacccacggcctcgtggacagcagcaacgttcgcggtgtgtgctgcggttgcggcagcggtgacgcgagcgatgctctccttcgccagagcgaggatcggtgcggaacccttggccttgtcgccgaggacttccagcttggcttccagcagggcgaagttgcccttcgctgcttcggtcagttcgcggctgtcgatgtcgaggcccacggtgttgacgaagtattcggccgcgatgttcaggccgttgtcgccgtagtccgggatcgccacagcagtcggcgcgccattcgccggggcggcgggctgtgcgggagccgcaggttcgagactcagcgcgtcagcagccggaggtgcagcaggagctgcgggctgtgccggtgcggcgggtgcaggctgaccgttgggcagcagcttgtcgtccacgggagccggagctgccggtgcgggctggttgccgttcgaggttgcgatcacggttgcgccgggaccaccgcccggaggtgcgttggaactcattgtgtctgtgtctccatgttgttggcgttatcgacctgctgcgatgcgttctgcatgaccagctgctgctgtgcacgctgctgcatcatctggccgtactcggcctcagtcagtacgtagatgttcgggtccaagccaccagcggcggcgaggtctgcgatccacgcggacagcttcagtcgttcgagaatctgcggcggcagcgcgaggacgttggctaggttgctgccgaactccaacagccggtcacggtcacccgtacgggagagcgcggccaagccggtgatgatgacaggctccaagtccttgcctcggatgtcgcggcccgtcaggttcatcacccaaaaggcaacgggtacctgcacgtcagcggcgatacgggagtaaccaccacccagcccgccttccagttcttcggcgaccatgcggatttcctgcgcggtcacacgttccgcctgacgagtcaccgccgtctgcaacaggaagcctgcgccgatgcggttgatgtaggtggactggattgcttggttggtttgcagcacaccatcgacgcctgcgttaatcagctcgatgtcgcccttcatgccgggaatggccgcgccgtttggcgatgccatgaagtcctcgacggaggtctgacctgcggggttcaccagccaccggaactcggaagcgaggatcgcgccctgtactgcggcctcggacagcatcgagagcgactggaagtcggcctcgtagtcttcgaccaagccggagccgtagtcatcgcctgcggccaagtcccagctcaccgcccggtagggcagcttgtctgcggtgtaggtcgaggagaagttggcgggcagcttgcagttgcaaatccacacgtcttcgttgtacttgccggtcttgtggtccagcttgacccacttgtactcccacaccattccgtcgtcatcgggcttgaagtccgggtgcgcgacaatggcagcgagtgcggctggttccagctgggtcttgtgcaccttctcccgaaggatcagctcgtacacctcgccggtgcgggtgcgcttgaccacgtagtgccgcatgttgagcacgcggatcgtgtccttctccaacaccatgagggcgttgcctagtacgatcagcatcttcagcaggtcgtacagtcgggatcggattgagcgcttgtccagttcgagactggcatcctgctcggccttcgcaagcatcgcctgcatggcctgcaagtcagcgccctgttcctgagcagcctgcttcgccttgcgcttcagctccaatcggaagaagggtcgggacggagcgaacagcgacatcatcagcttgttcgccagatggttcactgcctgcgcgccgagagactggaacccgtgggtcagcggctcggtatcctgatcgcggttcttgcgagggaacagcttcggcacagtccagcccgaatagcgttcgagtcggtacatgatgccctgacgcttgttgtcgtaagcctcgaactggcggtgagcggtttggatcgaatggtccatgctcacctcacaacaggtctgacccggccacagtcgtcagccgggaagctgcggtcgtggtcacgggtcgggtgtaggtggagcgggcggtcttgcgtcggccgatcaggtcggcagtctgcaagtcgaggtcggaagttcccagccgcacatcgacggtatcgacgggggcactcagcaacttctcggcgtactcagatgcggcctgctgtgcagctgcctgtgccatctgatcggccatcgcctgaatctggtagttcgtggattgagtttggaggttggtctgcttgtcgatagcagcagcttgcttcagcgctgcccgcttggcggacccaccaccaacgatgctacccataggttaactccttcgcttggtgaattggggagcatgccgttccagcaggtagccgtagcgtgcatacatccgtgtgagcgctcgtgagttccgagctagtgcaccgcctgcgctcagtgagtcgcagtggttgatgtcagccagatgttccatcacggctatgtaccggtcgaaggaactgcccggcccaattcgcagcaccatgttctcaacgaacgtagtacggttcttggagtaccacggtgtgacaatggcaaagcatagtaggtaagcttcatcaatgattactgcatccactagaccctgtgttatcagggccactgtgtaatcaggatcatcacagttgtagctcacagaagattctctgttgtctaccttactatcttctctagatgacagatacaaagcggccgttaaagccgccttgatctgctcactatcacccgtcgttggtgttcggtacggaggaatcaacggtgaaaccctcctgtaagatgttcaggacgcgggccatccccaactgcatacctgcctccaagggcgtggtatttgagttgacggacagcgacagcccggacagtcgccgcacggcggccagctggttcgggtggagcgtcatcaggactttcactttggcgtcttcggccatggtgtctcctctgtgctataggtgtaccaaaaggtccggcaccggttccgcttactctcgcggccgctccaaccggacctcagttgcctcgtgctataggtgtactgaaactccgtcagctgaagaagtacggagaatcaaggacttgccgcaggtccagctcgcccatcggcggcggctccggcaggaacgggtaggccgagtggaaggccgagagcacatcgtgccgctcgtacatcgacacgaacacctcccggatgatccggtacagggccgcgctgtcggcggcatgggtgccgaagtcgtcgtggatcatggcgaaggcgtcgatgccctcggccttggccgcgttgaccaccagcgtcaggtggcttgcgtcgaggctgtgcacgaagttcggggcgatgccgttgcggtgccgggacttcttcaccgcgtccgtgctcttgcgcagggacagcttggcgttgccgcacagcttggtgttgatgcggtgctcctcggattcccagtagacctgcaccaccgggaatccggacggcgtgatccaccggatgcggtcgtacccttggttgaggatcgacccggagccgcgctgcaaccactccatcgcgcccgctgcggcgaccacggtgtcggcgatggcctcacccatgcgcttgctcaggaagcgcgctgcggggccgtacagggccttgtcgagcgaggggaacttgccgcacttcaggtagtcttcgatgatgaagtccgcccacgaagactgccgggagccgtagggcagggtcatcacgctacgcttcaccagcgaacgtgtgaggccatggtcgagccacagcgtacggtacccttcggcatcctcgtcctcgcccagcaggatcgcagtcacgcggtctgcgaccatctggtagatgtcattcggcagcggtgccgggatcaggttagtcgccaccccgcctgctgcgtcgcgcagcatcgccgagaagttctgaagcccattgcacgaaccgtccatgccgactgcgatgcggctcaggaagcgatccccgaacacttgccactgctcgtactccatgcaccagctcagaaattgcagcggcttgtcggcggtcttccactcgtcgttgtgcaccgggtccgcagcgaacgccattatctggtcgtgatgctccgctacccacttcacacgatccggcagagacgccttgtcgtatccccatcggtttgctcctgtgatgcagaaccaatccttcgcgtccttcgtcagcaacggcttaccatcggcgaactccaagagtgccttctgcaagtccgaaccctgcggcgacacgccggtcgtctgcacgtacttgcggccgcggaagtcagcgaagtacacgaagtagatgctcgggtactcggcgaacttgcgcgccaccttcattgcgttgtagaatcgattgcccttgttctgccgcaggcgctcgtcggtgtgccagttggacatgtcgcgcttccactgcttgaactccaactcctgattgtgggacatggtttccttggtcatgtccttcgtcagccactccggcttgcgcggcttcggcagctcgccttgcgaaatgatttcctccatgtcgtgcaccttggcgatggccgacacggcttccatcagccgcttgttgatgcgccacggcacgcgctgcaatgcgttgatcgcggacatttcgttgcgcagctcggcggcgcggtactcgtctcgcgtctgagcgtaggtcttcaccatccacggattgagccgacgcatttccttcgtgtggaatccaccgttgtcgatgtccacccagtccatcggcggttcgacgcacggaagatagaacggcgtagcctcaatcacaaagtcgctgatctgcgtaatcagcttgcgcacctcgtcagtcagcacgatcttgacgtgagtcttggtctggaacttgcggtacgctgcgcctgcactggcagcagtctcggttactacgccaatctccaacatgcccaactgggcgagctgatcgcacaggtacgcgccgacctgatcgcgctgcgcttgcccccactccatgaactcgatgccgttcttgcggccctgcatcttcatcaccgtcatgcggtggttctcgttgacagagagcttgcggtccatgtcgttcatcaggtggtagaacagcgtcggctcagcgtcggcgaactgcgtcagcaggtactcgtggtacacgttgatgccaacgttcttcagcacgtcgcggtcgctgccttcgccgtgcttgtcccgcatgcaggaggtaagggcaccacgaacggcaacgaaggccacagcctcgtaccactcgcgtgcctgttcctcggcgctgacgggctgtccacgcttgttctgacgctcgggatcatacttggcgcgcagaagtggcacgtgcgcttgggcacgaccgatgcgcggggagtcgatgtccgcacggatgcgctccgcaagcggaagcacgaaccggcgatacactgcttgggcgtaggggttgttgtccgcgccgcccttctcctcgttgcgggcgatggacttctccatgcgctccttaccgaaggcgtaggtttccagttcgagttccacttgcgagagcatgctacctccgttgcttgatggtgaagtccgtcggcgggtagcgcttcaggatcatgcagaccagtgcggtgtgcatttcgttgatgatgtgcggccacgcaggaccaccgacctcgtagctcgggatgcactggcggttgaagaactgctcggtgccgcaccacgcggtggcagtcacagtgacgtgacctccaccgtagggagagaagcggtcaccgtcgaaatccagctcgggctttccgaatcgaatgtccatcagcccctccgttcggcgaggaagcggtccagcgattcgatcaccgcatcgcgcaccgtctcgttcggccacagggaaccggcgtactcacggaacgggatgctcactcgcacctccaccgtgtcgcgctccatgttatgccacacttcggtctgaacgttgctcaccggtcggcctccttcttgtcatggcggatgcccttgtagcgcggctcgcgcagcaggccgtacttgctgaaggacatggcttcgatttccacgatgtcgccgactacgggaacttgcgaaagctggtgcggcacgccgctcccgacctcctgctccttaccatcgccgaggtccacgaacacggtgtagacatcgcgcccggtcttctcgccgacagcacggccgatgcgtagcacacgcaggtccagcgtcagggtaggcttgaccttgacgacttcgccgttcgtgcccttgtcgcccttcacccacttaccgctcggcttgcgcaggatcaggccgtcgtatgcgccgccctcgcacaacagcttcgccgcctccatgctgcccagctcttggtcgatcaggaagccctgcgactctgcgtagaacaccggagcggtgccctctgcgatggcatggcccatgctcggcaggcggctgacgcgctcctgatacacgaggtcgctgaaaccctgctcccattcttccagcgtcacgaagtcgaacaccacgaacatcggctcggtgtactgcgtgccatccttcttgcggaacatgccgctgacggtgggctggtcgatctgcgggtgccagtattccccgaagtacacgccgaccgggaagaacggcgcggatgcgagagcgttctcgatgtggtgcgcgctgacgacctgctcgccagtccgagagaacaggtcaaccaccccgcgatccaccggctgcatctgcacgtcgcccaccttgattgcgtgcagacccttgttcactgtcggcacccagtggccgcgcttgatggcgaccatgttgcacccgtcgtacttcggctgtgcgatgtactcggtgcgcagctgctcctcggtaggccgcagcttcttcttgatcttgtcctgctcgactgccttgtggacgatgtagctcatgcgtggtccctccaaatctggaacatggcgagcggcacttcgtaccacggaacgtaacgctcccagtacgtggccttgccgtcgtaccactgcacgcggaagttgcccttggtgaaggcgcggttgatcttgaagccgcgcttgcgcttcttgtagccgggagcgacccggacattgctgcgaggcacatcaaacatcggcgctgtcctccttcttggtgccgtcacccagtgcagcgttgaactgcgcgatgcgggatgacatgaacttgttgacgatgccgccgatccacagcttgcgaggggcgagggaaccacggtacccttcccactcgtcggcgatgcgggtatacagctcggcctgagcctcgtcgggcaggttcgggaacccggccttgaccgcgttctgcaacgcctcctcgtggtcagcactctcgccccacgcaacggcgttctcgtaggacttgataagcatggcggtctggttcttgtagagcattcatttctccttcgacgggaatggaacgaaacctgcgaggcccttcatcacgaggatgcagaaggcgtcgtcagggtatgtacgatgccagagcgagttggcccacccggcatcgaactgcttgcgggtacggtgctcctctaggaagcgcgcccactcggcctcatgtgggacgtaccgatgcacttggccgcagcgggcgcaggccattagtcacccttgctgaaccaacggcggatgatgtactggcggatgaagcttatcgccgtgaacgcaatgccgatggcgtgcgccgaaagcagcgggtgctcgggatgccacagcaccggcagcagggcgatgttcgctgcgtagttgatgctgtacccgatgccgatgttcacccaagcctctttgatcgagcgcgccttactctgcgccacgggccttctcctcctcgcgcagttccagctccaacaggaacagctcgttgatgatgtggtgcgcccggtggtggattcccgtctccgggtccagcttctcgccgaggcagcgcttgttgtcgtgccggtagctcgcgtcctgataacgttcgagcgccttctccacgtgctgccacgaatgcgccttgtacttctgcgcaccgaaggtcagggtgtcgatgacacgggccagtgcacgcggcacgccctcgtgcagcagccgcgcctgcggcttaccgccatcatccttcagcccgacaccacggtcggacagtgtgcgacgatcttcgtcacggtagttcagtgcttctggcaagggaacctcccttcgtgcggtggtgacacctcccacgcccatcaggcgagtgaggaactgcgggcggatgatagattccttcagctgcccgtcgaacagaactccaacatcaacggcgctgatcgagcgaaccacgccggacctaccgacgaggcccggagcggagccggtatagcgtacgcggtcgccgtggcgaacgtcggtaagtctcatgcgcttctccttacgcgggaacggtgatgtgcttgcgagcctcggcgctggtcgtgagcttgcgcccacggctgtagccgtcgcacacggtgcactgaagcaggaggtacgttccgacctgcgtacgggccggatcatcctgcgggatcatttcgttgcagccgcacttgttgcagcgatgctcgctgccatcggccttgtagtacactgcgacgttcgggtgctgcgagtaccaaccgcgcagcttcttgtactccaacttcatggacttcacgtcgattcggttgtacgcttcgcactcgtcccatgcgccgggcaagctctgcatgcaggccacccacaggtcgaagccggggaagttgtggtggtcgtacttgcgcagctccggcacgatcacgccggtggtgtactccaacttctgcgaggtgaaggcgaactcggtgcggttcagcagcagtgggtcgatcacctgcaccggagacacgggcgggaacccgaggatggcgaggcgcgccttgatcttgcgcaggtcgaacttcttgccgttgcgagcgagcacgaagtcggcggcgttgagcagtgcccacagcgccttgccttgcttgcgatcatcgaacacatcacgcacgttgcgctgatccatgtagaacgactcgtcatcgtccagccactcgcaagcgaacgacatcagcgaccagtcacgcttgatctgcttgacgctgaagttgttgttgaacatgccccagccgtagaactcgatggggaatgtctcgatgtcgaggcagagaatcttcgggccgcgcttcggtgctcggcgaatgaactgggtaagggtcacggtgtctccttgttgatagcccgacgctttcgcgccttcgcattgcgagcgatgcgcttctcgtcgtcggtcttgaaggtaggatgcaggtaccccgtgatgttggtgaggtgcgaccgcaggtagttggggatgcccgcacagaatgcgaacacgtcgcgcacgccgtaccggcctgcgttgttctcgaccttgccaagcagcgagttgcatccgcgatggagcaccccgcgcacagcgccggtcttgtggtcgtggtcgagcaccggatcgagcggagccttcaggccgaactgtccctgacagagacagcaccggttgccttgctccgctgcgagcttgatgcgcagcagcttgacctgtgttgcagtgagtcgcttcatgctttgtatgcctccaagattgcgcgcttctcgttcacgtcctcggcgaggtcatagaacgcctgcttcagcttcggcccaaacacgtcgagcttcagcacgtcgagcagttcagcgtcacgatccgtccgcatccacaacagcacggcttgctcggcgaaggtcttgcgccagtcggaacccagcacctcgctgtacttgccacgcaccagcatcgctgcctcggcgttgtccttggtaccgaacagcaacgtctcggcagtgaccttgcccacgtcaggcaggccggggatgtggtcggcgctgtcaccgtggagcatctgcatccagaaccacttgtggccgtactgcaaaccgttctcgcccacgatgtcgtaagcgccaagcggaacctcggtgatgtcgtagccgtcccagtctacgtgcacgccgcagaacattcgcatgtccttgtcggcgctgtgcaccacgtgcaggatgttgtggtgcaatgctgcaccctcgttgacgtacgcgatgccgtcgtcggcctcacgagtcagccagattttgggagtgaaagcgtcgccctcgtatgtctccatccactcacgaaggaacgcccagttgttgggcttgcggcctgcttggcgctgaccctgatacggctgcgtggtagcagcgaggaagcgatcacccttggtagacgcggcgtgcgtcaggtgcatgacgatcttgcccgctccgctgacatgcttcagctgtgcgcagcgggagagcacgttgcgtcgtgcatcccccgccgagcagttctcgctaccagccgcgaagtacgccatgtagtccccgtcaacgtgagcgatcacgcgcgggttgtgctgacgtaccacttgcaccggcatcggggagcgctcaccggccgctgccatgagagcgctcaggtccatcaggcgatgcccgccatcgggtcgctaccatccaccgggaacggcggcttgtcgtcagccggagcagcgtcggtagccgcagcgttcgccacgtcgccgaccacttcgtccagcgcatcgacgccttccttggtgaccgtgctgctgcccgacaacttggcggcggcgtagtcgtagcacggcaggcccttgaagttcagcgccgcagcgatgcgcagctgcgtcttgttcttcgactgcgcttcgtgagtgaccttgccggtcttctcgtccttgcgctccgggtactcgccggggatgtagatgctgtcccacatgtcggcatcggcgaagtcccacacgaacgcacccagcggggtgatctgctgcggtaccgggatcacggtgtccacgaacttgccggtggggataccgttctccatttccggcaccggcatgaccggcttgcggatggaagccttgtcgatttcggcgaaggtcttgttcgggtcgcgcttgcccggcttgtggatgacttccagcagcacgccctgacccagcagctgcacgaagtgtcgctcctcggtgcgcaggcggctgaagattttgaagtagtgcgccttctcgttggtggacaggccgagggtcagcgtcatgcgcaccggcaccggaccgttgtccgtgtcgatgtgcgggtgctgcttgccggtcagctcgaacacgatggcgacttcatcctgcgtcttcttcttgccctcgaactcgaactcgtgcttgcccagctcgtagtacccgacgatgcgggcggtggtcacaccagcagcgggcggggtgtagtcgaagttgccaccactggcaaccgactgatccttaccctgcgtggcgaccttgttcaacagtgcgtcaagactcatgcgtgttgttctccttattcaaacgacgggttgtgattaccaacgaagtccttgcggatcgacgctcggtactcgatgaccagaccggcgaactctgcgggagggttcttctcctccatcatgttgtcgcccatcttggtttcacacgggacgccaagtggcagcgtccagttgaaccaccactccatatacaccgacgcttccagcatcgaggcgtgcagcagagcagaggccttggttgcgatgtcgccgtgtgcatccacgtagacggcatcgtgcacctgattcacgagcagcgcgcggcccaaccattccttcggttcggtcacgtacttccggtagaaggcgcgcaggctgacgtacatcgccgccttggcccactcaccaccggtgccctgcatcgggtagttcttgatttccgtaggcgagaacgactgcgcacagccacccttgctcgcgggcttgttggcgatgaacaccggggacggtgactcgctgaaggaatacatcttgccgtccggagtggtccagtgcgaccggccaagctgacacgtaagcccatgtggcacgccttgctgcccggcgttgggatgcggaacgaagcgttgcgtgctgacgcggttgcgcttgatgtgctcgaccatgcggtcgatgtactcgcccagctccgggtaacgctcggcctcaccacgcaccagcgcctcgacttcttcctccgacatgccggtggtcgcagcgatcttcgccacgcccgcaccgtacgcacgctggaaggagaacaccttcgcgtttccgcgcttcttcttccacttcttgtgctcgggatgcttgtcgtccttgctcgccttcaggatgaagtcgtagtcgtacttgccttgctcgccccacgcctgctctgcacgcaagcagtgcatgtcgaggccccgcttcaagtcctcgatcagctgacggcactcggtgaggattgcctgcacgtagatttcgagggaggtgtagtccgactggatgatcttgccacccttgtgtcgggacacgaaggcgcgcttgatctgcgaacccttctcctccaacgtctcctcgtccagctcacccttactcacgttctgcaagttcggatcgctggaagacaagcggcccgtgaccgtgttggtcatgttgagcttgtggtggatgatgccgtccggcccgaccagcgtgagcattcccttctgctcgccagtcttctcgtccgtcgtgatgtagtacgtggacaagtccttgtgcaagtcagcgcgccgggcaagcgccttggtgaacggcaggttgcggtagcccagcgcctcgatcacatcggcggcggtggagtacacaccctcgtcgctcttgctttcccacgcagcatcaggctcggtgtagccggggaactcgaacagcatgtcctcgttgcggaacttctgcttggtcaagtcatcgaccttaaccttcttggtcttgtactcccccttgttcttgccgctgccgtacgtggtgtagcgccacaggttgtcgaagtcctcggccgggggcgtcgccgtcgtagtaccatcgaccagcacgtagtgcacctcgtccttctgcacgtacgtcggcccgccctcggtggacatgatcggaaccttggccgtgtacttcaccttgccaccgaagatcagcgcgctcttgtggaagcggctgttccagttgaaggtcagaccctcgggcaactcggggatgaagccgttgagttcggcggtcgccgttgcaagctcgacctccaactccttcgccttcgcaagcgcccagtccttgtccacgtacatgccgttgtactcggcttcgatggtgaagcacagcgcacccatgttgagcagcgccgagcgcaaaccaccacgtgcacggaaggcagcgagctgaccgaggaacatcttctcggtgttgccgatgtcgcccacgtcgtcggtgtcgttggtgccgaggagataatccatcagcagcgtcttgtcgatgtcgcaggtgtccacgcccgcagcccacagggacttgactgcatcgtccttcaggttgccgccgtagcgtggggccgtctcgtccatgctcgccatgtggaactcttgcgtcataccatgaagcaggtactccgcaagctggcagtcccacaccatgccgccgccgtcgatgaactcgatccatgcctgccgattgagcgggccttggcagatggcgtgcaggatgtcgaacttgatgttgaacccgacgaggaactgctgcccgtaacacagctcgcgcagccacccatcgggtgcgccgcccatgtactggttgtcgattccgatgcgggtgtcgtagtacaggccggtgttccgtgcgtcgcccttccgcttgtagccaatcgccacgatcttgttcatatcgtagaacggattggccttgcgcttcaggatggcacggatcgtggtttcgaggtcgaaggaagtgaagctcacagcggccaccgttgcagggccagctcgtacatttcgtcggacgcatcgccatccaagtcaagcccgtcacgcacccaacggaacacgatgatgcggtcctgcttgtccttgatgttgcggcgcttgcagatggtggtggcctcgaccgcgcgctgataccagccggagtcggcggtcaccatgacgttgaacacgccgttgcgcagcgcataccacgtgtcgctgtagtcctcgtcctcctcgtagtgcccatcggcaccggagcacagggtccatcccgcctcgaccagcttggcgatggcctcgtggaagtcctgcaccagcacgaggtagtcgatgtccgtgttggttacgggcggctcgacggtgtagctgctgccggtacgactggacgtgatgacgcccacgttgcgcggcaggtagatattcggttcggtactcacggcgtgttacctccgggcttggtgatccacagcgtgaagcacgggatcaggttgatgcaccagcgcttgttgtgcggcgagtagtgcacgccgatccatgtgctgtgcttgttgcgcaaccatccccacttccactgcggagcatcgttgcggccttcgatgtagcctgcgtcgtgtaccttgcgcatcataccagcgaggaagttagcctgcgctgtcgatgcacactggtacgactgcccaccgaagtggacctgcgcacacccatcgacgtggattttgtccttcgtcatgctgcctcctgatagaagcgggcacgctctgcgtccatcatcacttcttcccgaacgtcacgcttaccgcctgcgcggtgcagcttgttcttcggggtgccgatgtagcggaagcgttccatcgctgggtcattgagcttgccgcccatgatgatgaagtcgcacgcaccctgcttgccggtcttgctgtccttcagtgcggactgcggcgggtactgaatgccctcaccctcagcgctgatctgcgaagtcgccacgcccacggcgtcgtacttcacacaccagttgcgagcggcctgatacatcgcctccaacatctgatcggtacgctgtccgccgttggtcatgccaccggtgaacgtgatgttgtcgatcatgtcgaagatgatgaagccggggttggtctgcttgatgatggcctcgacctcaccggagttgaacccgtggatgtcgtagaactgcatgcggtggatgtccccgcccatcgcatcttcgatgcgcttgcggatgctgccatccttcgcccactccaccatctcagggatggtagcgccgagcagcgactgataccaccgctgcttgatgcgcttgcccggtccctcgttgttgagccagatgccggtgcgcttctggtccggccacaccgcatcgagctgcgtgatccagtgactagactcgctcgttaggaacgtggtcttgcctgcgtcgggacgcatggcgtagataccgaagtcaccgccacgcatagcacgcaggttgcgcgccaatgtgggcagtcggaagtggatgccgatgtcgtgctcgtccatttccatcagttcttccggcgtctccttgaccagcgggagccgcgccttacgatccatccggtcggtgatagtctcggccaatccgtacagctcgtcgcgcaggctgaactccgctccgccattccactgcacgatcttactgaccgcagtggtggcaagctccaactccaacagcttctcgatcatgccctgctctgcctcgggcgggaccggctcgcgcatctgcttcagcagaactttgagcagggacttcttgtcgtcggcctgcgtcttccacttgaactccatggcccagccatcgaacacatcgaacggcaagtccttcgtgtccgggaactccttgtagtacgcacgcaacgcatcgagcatcagcacggtcagctcgtccagcccatcacgtggtgcactgggtaccagccggtcgaacttgccacggttggtgcacaaccgcagcagcgtggtgtcaagactcatcaggttctccttcgggttcgtacttggaatcgagctggtgataccgtgtgttgcgcgtctcgaacttgcgcccgccgtccgtcacgtacagcaccgtcgaggtgtgcacgatgtcgcagtcgccgaggttcggatgcgcaagcacgtcgccgagcgtggcacggaagccaacgacgggcgggatgatggcgcgccgatagcgcacgatgggtttgctcattgcagcttctccttgatgtagtcggtcgtgtaatacttcgggtcacgtggtgacgtgatgttcctgtagtccagaccaaacgcacgtagacgcgcagcgattactcgcgcgctgtcttggccgggattgctaccgttgcttctacctctgtcgtcatcgagccacgttgctacacgttggcctcgatcagtcagctgcttcaacactttgttgtgcagcttggtgccgagcaacgaccacgcttctgtgcactggcccaccttgaaggcggatagcgggtcttcgcatagcacgatggtgtcccccttgcccacgccgtagcgtgcgacaagcccatccttcggcacatcaggagtcagccatttgggctgacggcttgtgcttcgtgctgtccagtacacaacgtcgtcgccttcagtgatcggtagtaccacccgcccgatgctcgggcaccagtacagccgcagcttgtcgatcatctgaagcgagagtcccatcttaaagaaccacaccttcgcatcgagcggccactctcgggtgtcgtatacccgtggctctggcaactcaacagtcgcacgcactctgcgttcgctcgtctgctcggcgtggattcgtgcaagcttggcctctatactctcgtgctcacgcttgaatcctgtgccaccgcacctgaaacagaatgcggtggacttgtcatgctcccgagtgataagcaagggagtcccttccccgcaatcatgcggcactcgggtgcggtggccgacctgtagtcgctccgcatggtgcagccaatcgctgtcgggaagggtctcgctcatgctatcctcgcttgattactcgaacacctcgaagatgtcgttgtcggtggcgtacagcacggagccgttgccatcggtgctgacgatcagccggtcaccagactcgctggtcagcttggacaccacgaaaggcgtgcccttggtcagcttgttggtctgccgggtgtcgatcaggtacgcggtggtgccgggcttcagctcgtcgccgcgcttgactgatgcactgaccggggccgggctggacaggctcacgactgcccgccttcaccggcagcagccttggcggcggcagcttcggcggcgaggcgctgtgcctcggcaacggcggcgtcgatttcttcctgcgccttcagcacttcttcggccgacatcagcagggcgctgctgtcgatcaggttcagctcggcatccagaccttcgccggtctgcaccttcagttgcagcacgcccttgtcgttcttgccggtggcgacgatcacgccggacaggacacgcttgttcagggcacgaccgaacaggtaggacacggcgtcgccggacttcagcgcttcgatggctgcgctgttggcctcgaccgcatccagcttggcgagcttgtcgttcagcgcatcgaccttggcctgcgccttggcgatgtcttccagcagctcggcgcgcttggcttcgtagtggctgacggaggtggtctgttcggtggtgttttcgttcgacatgcggtgtatctcctttcattgacgggtttggttggtggaccgtaacgtgggccagtcggcacagttcagtgctggattactggaagatcagctcgctgttgtacccaccgccgccattgtagaagcgacggcgcagcacgctctcctcgccgagcaccagcaggcggtccacgatggcgcggatggcgctcatgtactggtccaccagctcgctctgcaagttcatgtcgaagcggatcacggtcaccgcctcgtcatccagtgcgccggtatccttgcggacgtacaggccacgggcattggtcatcgtcgcgccaccgatcagcttgacggcggcggcaatctccggctgcacgttgagcagtcggctgtcgggcacggtcacctcgacccagcttcccatgcgcaggctcatgctgcacctgccagtgcggactgcacgttcggctgcaacgatgcaccagcacgcagctcggcagcacgacgcttcatgcgggagcgcagcttgcggcgctgcttgttgttgtcgccgaggctatcggccacacgcttcagctggttgttgccgacgatgcgggtctgaccctgccccttctgcacggggaagtagtcctgccccagcatcttgcgcagcaccgggttgtcgatggggatcagcggcacgctgacgtgcaggtaccggctggtatccggtgcgggcggcggcgtgtcatcgtcgtcgtgctgcggcttcaccgctgcaaccaccttgtccttcacccagttggcggcaccgcgaatcttgccgccgacgttcttgatcttttccatgaatcccatggtttacttcctcctcgtgccgaagtgattgaactccgtctcgtgccacacatagtacgtggtgccgagcgggtcggtgtctgcctgccagttgcgctgggtgcagtagtcgttggctgcgtcgaggtcatcgaacgtcagcgagaacccggtggaagccgggccggtgcggaaccggcacagcctaccgtcgtcgtcatggtactgcccgacgacaacccacggtccacgacccacgatccagtacagcaggatcaggatacgcagccagagtttacgcatacaccgcctcgatgtagtagcccgagggattctgcttgctgcgcttgtcaccgatggtattatcgatgatgtcacgggcggcggcgcgagtcgggaacagcaggttgtcctcgctgttgttctcttcgtcaccatcgacgcgcaccgttgcgccgtctttgtagcagctggtgtagtcaccgtcgtacttgatacgctagcccttcacctgacgcaccggcttgcggatgctatcgcccacttcgatgatgtgccagttgaacaggccaccaccgttgaaggagttcaggatgtcggcctcggcacgggcggcggcacggcgctcgaaggcggacaccgggccgggataggtggcgtcgcgcaggctgtccagcagggactgcgttgcgcccttggtgcgcagcagctcgaccagtgccgtcacttcctcggcggtggcgttgcggcccgtgccattggcgacgacgccagtgatgacgccatcctttgcggtggccgggatcgaagcgatgaagtacagcttacgcatggtggttctcctcattgacgggtgggatttcgatttcctctacggtgtagagagtgggcaccttctcgtggtgcagacggtggtgtgcgatggcctgctcgcacgcctcgtggctggtgtggtgcccgccgaggatataatccccgacagcccaaccctgcacggtaacgagcggcagcgccttcaccacaaggcgcaggctgacctcacgcataccagcgctccacgctgtgctcatgggtcacgaactctttccactggcggggcttctcgcacagctggatcggcttgcgctttccactacggatgcgcttgtagacgatagggatcatgcaatatgccctcctgttgggcgtggttccaaagctacgccctcgttagaaggcgcagcggtagatcacgcgtggttcgggtgccacttcactcggtagcgacgcagacggttcgcatcgttgccgacgtgcgcagcgatggcattgcgtgcagcttgcgcagtggtgaccgttccgttgagaccggtcacgctggacgtgttccatcccagctgcgactgacgggcggcgtgcttggtgaagaactcggcggtgtagaagccgcgatccttctccgggccatcgggagtaccttccggcaccacacggtacgcatcctcgctgataccctgcgccttggcccgcgccttcagcatgcggtacgctgcattgcggctgcgctgcggcaggcccagctcacgcacctgtgcccagttggcaagggcgatgccgccgtggcgcagattgaactgcacgatccagcccttggcctgcggcttgttgaccagcccggtctgcgatgcagtcagggccacgtggcgtgcgctctgatcgtccatcagtacatccggcagcttacgcggcaggttgtcgggcattgccgggccgggcaacaccatgcggccggtcacgctgccgaggaagtccagctgcgaggcatccaacaccaccggaggcaacggagacagcaggcacgccatcacccgcgcctcgatagcagcgaagtcaagttcacgcatgccgtagcccacggtgaacgtcggcggtgcgaacaggtcacgcagcagctgcgcctcggcattgctgtcccggcaggccgcgataacgtcgtcctcgaattgcaggataccgtcacggtcgaagctctcgattccgaagtctcgcagctcaccgtgcagagtggagaactcgtcggcgaggtctttgcgagcatacggctgcgctttggcggtcagcgcacaggcaatgtgcagggcagcacgcagcagggacgcttcgcgctgggtcactcgcaagttgatcttgggttccatcatggctccttgaatcggtgggtgtggaaggctgtgcggtcgccgaagtcatcgacaaccacccagtattcgggaaaggtgaatccgttctccatcgtgacgctcgggaccacctcgactacggtgtattccttgccgccagtcaggcggaacagggccgtgtgcttggatacaacgacggtcccggattccatcacgcagtcgccttcaccttggcaggcttgggcacggcgcgggcagcgttgatgacggcctgttcttcctcggtcgggacataaccgccctcggtcgccttttccagacggcccagcagcttgtgcaggtcggcggcgaaggagaacgcctcggcgggcttctcggtcttgaagtcgtaccacgccttcgcggcggcacgttccagcatttcggccagagcttcgccctcgacgcgcttgctcttggcaaacttcatcggcgcgctcgccttggtttccttgtcgtcgttcggagccatcgggccgaactcggacaggtacaggcgcagggcctcatgcttcatgccgttgcccacggcgagacacagatcggaggcaagcgtaacgtcgccgtggatgtgtgcatggttgatgaccgcaatcgcggcctgctgaatctggtccaccagcttggtgcgggcggtgttgatcgacttgatggtgcgcttgatgtcagcgcttccggtgatgatgtccatggtggttcccttcaggttgggtccgtgccgattgcacgacactaggccctcttgcgaaggcccagtagcttgcattcagtggatggtgggtgcagcgagcttgatgtcataggtccagcgtgcgccggtccattgcaggttcgatacagcgcccggcggatgcttcgccattgcccgttcgtggcttgccatggcgttgcggctgtaccctgcggcgaagtagaatcggatcacaggtaagccctccggtcagcggcgtggttcgcccggttcgtcccgctgttgccctcgacaacaaacacagatcgctttccagcggttccgtggcgggcttcgtagcgttcggcttgtcgcttgcgctcggcgagcttgcggtcatgctccgtggtgcgcaggtccatcacgcttgcagtccgggtgaactggcagaagcggcgcttacgctgggtgcggtcgagattggcattgatcgagccttgcatgttgtgcctccatttggcactggtgggaaaaactaacagattgatgcgccctcagaaagccgtcgagtcggtcaatccctcattctcgattagagccgttgcatcgcctatcgtgggcgcacactgaccaccggatttgcctgcatggtcatcgcaaagggagggcgcatcaatctgctagcccttcgggctgtcaaccctactccggctagcagtgccattgtcaccgtgtggcccatagagccttttcacgaaacgcacagtattccatgcgataggaggctcaccacctccttatgaccggcttcccacctttggcagtgggttacgctgcgtggccgactctcacggcaaatgcaggccctaagcgttaggcttaggtaaagcggcaccagtgttgctagtctggtggattctatgggcctttgacatcccagttcatccggttatccgctagtgctacgttgtagcttggcgttccacccgtgggcttcacgttacaccctacccgttagcggtagtcctacccggtccagtgccggtggtcctcagaccgtggtgccatactagcaccctgtttgcatcctgtcaagcccttggctcgattcgggtctctaacccgttgggcgtcctgtcgccaccatcctaccatgtatgccggtagtccgcaaggtgctagctgctccgctgttccggtggctaccacttgccgcctatcatagctcactgctagcttagtgtcaagcgtggttcggtagctcctcgcatcccttaccagtgactcccatgtgcccttagcccacttgttggcggcgccactacggatcacgtcactcgacttgcgttgcagcttactaccattgcggccgtgtgtcaaccgttggcctagcgggtagctaactaatcagctcgacagagtaccgatagacggtgattcaggttgagccgactgtgtgctataggtgtaccaaaaggccgaaacgatacagatggccctcacacgcctacagctgcggttcgcatggtacccggtaggtatgtacctgtcaagccccttgcggccctcctgcggccctgtcgctgcgcctgacgcggtgtcaggtgtcgcggtagctcctcagtgacgccagtagaccacac

SEQ ID NO: 22 - DNA, 44415 bp, unidentified
  source 1..44415: mol_type = genomic DNA
tgattgcggtgggcatgaacaacgtcaaccgcctgcaatggaagctcgtcggcaatcccgacgactggccctaacctacaggagaacagcatgaccccgccgagtgtggtcaatgaggtcgtccgaacctcgccgcttacgctcggcgcggtctacctcaacttcatcagcacgtacggtgctgccatcgtaactacgctcgccattctgtacgccgtcgctcagttctactggcgggcacgcgagcaccgaaagatcatgggaggcaaggatgtcgaatccggcaagtgagggcgcactcggtgcgctgcacgaactggtcgcgcgtgcgctgatgcagcgcatccaagatggcgagctgtgcaccgcagccgacatcaatgcggcgatcaagttcctgaaggacaacaacatcacggcgacgcgcgaggccaacaaggcactcggcgagctggaagacgagctgggcaagcactcgctgcctccggctgacgacgacgagttgcagcgtgcactcgacaacatcgttcactttccggggagcgtagccaacaatgcgtgaatcagctgaagcggccgacgtgcgccgcaagaagttggagctgttgcagaaccactaccggcacttcgccaccttcatgcgcgacattatgaaggtgctggggttcgagccgacgtggatgcagtacgacatcgccaactacatgcagtatggcccgcacctcgcaatggtgcaggcgcagcgaggcgaggcgaagtccaccatcgctgccatctacgccgtcttctgcctgatccacgatcccactcaccgtgtgctgatcgtatcggcaggcggcacgcaggcatccgagattgctacgctgattcagcgcatcatcctcacggtgccgacgttggagtgcatccgcccggacaagaacgcgggcgaccgtacctccgtggatgcgttcgacgtgcaccactcgctgaagggaatcgacaagtccccgagcgtggcgtgcatcggcgtcaccggcaacctgccgggtaagcgtgcggacctgctgatcgccgacgacgtggagtccaacaagaacagccgcactgccgcgaaccgtgagctgctgctgaccatcacgttggagttctcggccatctgcaccggcaagcccggtactccgggtcgcatcctgtacctcggcacgccgcagaccggcgactccatctacaacaccctgcccggacgtggctacgacgttcgcatctggcccggtcgctacccgaccccggcacagcgcgagcactacggcccgcatctggcaccgtctatcgtgcagcgcctagaagccgacccgatgttggcgttcggtggtggcccgatgggcgacgagggccagtgcaccgacgagctgttggccggtgagcagaagcaccagtccgagctgcgtcagcgtggaccgtccagctatcagctgaactacatgctcaacacgcggctgatggatgcgctgcgcttcccgctgaagaccgagaacctgatcgtgatccccggtggtggcgaccgcttcccgctgacgatcacccgtggcctgagcaacgctcaccagcgcagcttccagtccagtgggtacggcttcgtgatgatgatgccgcacgacatgagcaccgagactgcccccgtgcagggcgtgcacatgcagatcgacccggccggtggtggtgccaacggagacgagacggccttcgccgtgaccgccttcctcaactccaccgtgtacgtgttggccgtgggagctgtgcccggtggctacgacggtgatggcttgctagaactgcgccgcattgcggtgaagtacaagccgaacgtcatcagcatcgaaaagaacatgggctacggcgcgttcgccaaggtgttcctgcctgtcctgcgagaagatcgcggcacggagaagggatacaagggcgacatccgcgaggagttcgtgaccggcaacaaggaagcccgtatcatcggcactctcgaacctgtcatggctcgcggctcgctggtcatgctggaatccgtggttgaaatggatcacgagtacacccagcgctacgccaccagcggcaagcgtcaggtctacagcctgttccaccagatggcgaagatcacgcagcagaagggcagcatcgcacacgatgaccggctcgatgcactggaaggtagcgtgcgtcactgggttgcgcagcttgcactggaccagaacaaggccatcgccaagcagcagcagcgagagttccaagactggatcaacgatccgaccggcatgaaggcagcgacccgcaagagtccgctgcaacgtggccgtccatccctactcgaccgttaccggaggtaaccaatgcagaagtccgacttcaccagcaactacacgggtctgttcggccgtggcaactacctgcaccgcgaactgctcgccctcatggagcacgcagagcagcatcccgcaaccgcagcgcagctgctcgcgcagttccagaaggacgccaccctcgtgctggacgccctgatcgctgcgggcgcacgcaccgcgtcctcgggtccgaactccggcccgcacactccggtcgatctggacccggatgacgatccactgaccccgtaaggagcaaccatgaaccagcagcagaaccaagataccagcaacaaggggctgttcggcctgatcggcggcatcttcatcggcatttcggcaacgctgctgtcattcacccaaggccacgaaggggtacgctacgctgcgtacctcgacaccggccgggtgccgaccatctgctacggccacaccaagggcgtagcgatgggcatgacggcaacgaaggcacagtgcgacaagtggctgatcgaagacctacagatcgcccagcagggcgtgcgcaagcacctgaaggcccccgttaaccgcaaccagatcgacgcctacacagacttcgtgttcaacgtaggtgagaaggcgttcgccgacagcaccatgctgcgcaaagcgaacgcaggggatcgtgaaggtagctgcaaggagttcctgcgctgggtctacgtcggtaagctcgactgccgactgtccagcagccgttgctccggcatccccaagcgccgcgacgcagagtttgctctgtgcttgcgccccaacaacgaggtgatccaaccgtggaaaccccaagtgaagtgatcgcgcggctcggcggcaagctggttggcttgctgctggtcgtgaccatgttcgtgtgcttcggtctgtacgtctacggcctgcaacgcaaggtggagaagctggaaactgcccaagtcggcacgaccgctaccgccaaggcggcgcagacgcaggctaccgggtacgcgacctacatcaaagagaaggaggacgtgcgtgttcgcactgaagaagttcttgacgctgccccggagtaccgggatggcactgttcctgctgatgtcgctgacctcctgcgcgaacctgccggtccctgacgactccctgcttgcagactgccacatcacctacctcggtggggagaagggcaccacctcctcgcaggacaaggtggtcaagctcgcgcaggaccgccgcatggacaccgttctgtgcaacaaggacaaggctgcgctgcgtgcgtggaaggccgaggtgtgcggtaccggtaagcgccggtgtacgggtgacaaatgaccaccatcgcatgggacggcaagcacctgtgggccgatagtcaggccacgcagggcgaccacaagcacaccgtgcgtaagatcatgcccgtatcgacacccaccggccctgtgctgctgggtgtcaccggggatttcacagtgcttcgcccggttctcgctgcgcttaaagcgggcgaaggctacgaggagcacgttggcaagtccgcgacggtgcttgtggttaaggacggcgtactcacggtcactactggtaagcagcagtgggtcgaggaggctccgtacttcgatggcagtggcaaggcgctagctctaggggcctatcatgcgagcaagtctgtggctaaggccatggctgctgcgatagctcacgatgtctacagctccgggcctatcgtcaagctaaaggcaccagttcgcgaggcttaggagtaaggccacgtgggtagccggaccaaaatttgcttcggaaatgcgcgggggtcactccaatagaagctcccgcgcgtgcccccgtacgccctcgcgttacgcgcctgcgggtgtgcgtgggtgcgtgcccgcgtgtgcgcctgtgtgcgcgtctgtgcgcccgcgtcaaggttccgcgtgggtgtacccgtgtgcctgcctgcgtgggcctgagcgtgcgtgtgcgtggccgtgcgtgggtgcctgcgggtgggcgtgcgggtgggcgtgcgcctgctgcctgtatggctggaccgcgctgccttggctgaatcgttaataaatctcttggcgaaaggtgttgacgtggccggtgcggtgtggttcaatggcgtcactggggcagcgacagggcttcaggagggccgcaaggggcttgacaggggctaccctacctgctaccatgcgaaccgcagctgtaggcgtgcgagggccatctgtatcgtttcggccttttggtacacctatagcacacagtcggctcaacctgaatcaccgtctatcggtactctgtcgagctgattagttagctacccgctaggccaacggttgacgcttgcgatgcaagcagtagtagacacacggccgcaatggtagtaagctgcaacgcaagtcgagtgacgtgatccgtagtggcgccgccaacaagtgggctaagggtacacgggagtcactggtaagggatgcgaggagctaccgaaccacgcttgacactaagctagcagttagctatgataggcggcaagtggtagccaccggaacagcggagcgacctagcggtaaggctagacgtgagagattacgggtgttgaggctgaggtgagaccgggacaccggtcaagacactaacaggagcgcacatggtcctctaacggatagcttgacaaggcggcacagatagccctttgaggccttgcaacacgtggaccaccgacgtacatggtgggatggtggcgacaggacgcccaacgggttagagacccgagcgagccaagggcttgacaggatgcaacaagggtgctagtatggcaccacgctctgaggagcagccacattggatggcgtaggactaccgctaacgggtagggtgtaacgggaagcgtgccaaccacagccaatagtggccgagagttgacgtggaccgccaagctgcaacgtagcactagcggataaccggatgaactgggatttcaaaggcccatagaatccaccagacttgcaacactggtgccgctttacctaagcctaacgcttagggcttcccatctgccgtgagagtcggccacgggaagtaacccactgccaaggtgggaagccggtcataaggaggtggtgagcctcctatcgcatggaatactgtgcgtttcgtgaaaaggctctacgggccacacggtgacaatggcactgctagccggagtagggttgacagcccgaagggctagcagattgatgcgccctccctttgcgatgaccatgcaggcaaatccggtggtcagtgtgcgcccacgataggcgatgcaacggctctaatcgagaatgagggattgaccgactcgacggctttctgagggcgcatcaatctgttagttttcccaccagtgccaatggaggcacaacatgcaaggctcgatcaatgccaatctcgaccgcacccagcgtaagcgccgcttctgccagttcacccggacggcaagcgtgatggacctgcgcaccacggagcatgaccgcaagcttgccgagcgcaagcgccaagccgagcgctacgaagcccgccacggaaccgccggaaagcgatctgtgtttgttgtcgagggtaacagcgggacgaaccgggcgaaccacgccgctgacaggagggcttacctgtgatccggttcaagttctctcgccactacgtggaagctgcccgcgattcctacaatcgggccatcatgaagcatccggccggctctgtgtcggcgctctacgtcctgccgtgcggtgggcgttcattcgacatccgactcgcttaaatgcaagctactgggccttcgcaagagggcctagtgtcgtgcaatcggcacggacccaacctgaagggaaccaccatggacatcatcaccggaagcgctgacatcaagcgcgccatcaagtcgatcaacaccgcccgcaccaagctggtggaccagattcagcaggccgcgattgcggtcatcaaccacgcacacatccacggcgacgttacgctcgcttccgatctgtgtctcgccgtgggcaacggcatgaagcatgaagccctgcgcctgtacctgtccgagttcggcccgatggctccgaacgacgacaaggaaaccaaggcgagcgcgcccatgaagtttgccaagagcaagcgagtcgagggcgaagctctggccgacgtgctggaacgtgccgccgcgaaggcgtggtacgacttcaagaccgagaagcccgcagaggcgttctcgttcgccgccgacctgcacaagctgctgggccgtctggaaaaggcgaccgaggaaggctacgtgccgaccgaggaggaacaggccgtcatcaacgctgcccgcgctgtgccgaagcccaccaagaagaaggagaacgtgtaacatggaacccaagatcaaccttcgagtgacccagcgcgaagcatccctgctgcgctcggcccttcacatcgcctgtgcactgaccgcaaaggcagacccgtactccaaccgcaagctgtccaatgagttcgccgtgctgcacggtgagctgcgcgacttcggtgtcgagagcttcgagcgtgacgccatcctgcaattcgaggacgacgtgattgcggcctgccgtgacagcgatgtcgaggcacagctgctgcgcgacctgatcgcaccgccgacgttcaccgtgggctacggcatgcgtgaacttgacttcgctgctatcgaggcgcgggtgatggcgtgcctgctgtctccgttgcctccggtggtgttggatgcctcgcagctggacttcctcggcagcgtgaccggccgcatggtgttgcccggcctggcaatgcccgacaacctgccgcgtaagctgccggatgtcctgatggacgaccagagcgcacgccacgtcgccctgactgcatcgcagaccgggctggtcaacaagacgaagaccaagggctggatcgtgcagttcaatctgcgccacggcagcatcgccctcgccaactgggcgcaggtgcgtgagctgggcctgccgcagcgcagccgcaatgctgcgtaccgcatgctgaaggcgcgggccaaggtgcagggcatcagcgaggatgcgtaccgtgtggtgcccgaaggcactcccgatggcccggagaaggatcgcggcttctacaccgccgagttcttcaccaagcatgcgcggcgccctcaccagctgggttggaatacgtccactgtgatcggactcagcggcacgttcaccactgcgcaggctgcacgcaacgccatcgcctcgcacgtcggcaacgatccgaaccgtctccgccgctaccgcgtgaagtggcacccgagccgcgcgtgatctaccgctgcgccttctaacgagggcgtagctttggaaccacgcccaacaggagggcacattgcatgatccccgtaacttacaagcgcatccgtagtggggagcgcaagccgatccagctgtgcgagcagccgcgccagtggaaagagttcgtgacccatgagcacagcgtggagcgctggtatgcgtgaggtcagcctgcgccttgtggtgaaggcgctgccgctcgttaccgtgaagggtgtggctgtcggggattacatcctcggcggacatcacaccagccacgaggcgtgcgagcaagccatcgaacaccaccgcaagcaccacgagaaggtgcccaccctctactcgatagaggaaatcgaaatcccacccgtcaatcaggagaaccaccatgcgtaaggtatacttcatcgtctcgatccccaagaacagcaacgatggcgtcatcactggcgtcgtcgccaatggcaccggccgcaccccgacccaagaggaactggatgcggtgatcgccgagctgcgcaccaagggtgccaccaccagcctgctggactcgctgcgtgacggcacgtacccgaaccagctcgccatcttcgaccgccgcgccgccgtgcgtgccgaggcggatgtgctcaacagctacggcgggtcgttcttcaactggcacatcctcgaagtgggcgagagcatccgcaagccggtgcgcaagccgctgggttggcgtatcacctacgccttcgccgaagaccgcagcgactccgatgtcagctgctacaaccagcacccgagcgccaccgtgcgcatcgacggcaacgagtacaacaagagcgagtacaacgtgctgttcccgacccgcgatgcagcgcgcgccgtgttcaatgccgagtcgctgggcggcgagaacatgggctaccgtgtcgagccgtactatgcgtaagctctggctgcgcatcctgatcctgctgtactggatcgtgggtcgtggcccgtgggttgtcgtcggccagtaccatgacgacgacggcaagctgtgccggttccgcaccggcccggcttccactgggttctcgctgacgttcgatgacctcggcgcagccaacgactactgcgaccagcgcaactggaaggcagacactgacccgctcggcaccacgtactacgtgtggcatgagttggagttcaatcacttcggaacgaggaggaagtaaccatgggtttcatggacaagatcaaggctgcggccaagtacgtcaaggacaaggtggtcgcagcggtgaagccgcgccacgatgacgacgacacgccgccgcctgcgccggacaccagccggcacctgcacgtcagcgtgccgctgattcccatcgacaacccgatcctgcgcaagatgctggggcaggactacttccccgtgcagaaggggcagggtcagacccgcatcgtcggcaacaaccagctgaagcgcgtggccgatagcctcggcgggaacaacaagcagcgtcgcaagctgcgctcccgcatgaagcgtcgtgctgccgagctgcgttccggtgcatcgttgcagcccaacgtgcagtccgcactggcaggtgcagcatgagcctgcgcatgggaagctgggtcgaggtgactgtgcccgacagccgactgctcaacgtgcagccggagattgccgccgccgtgaagctgatcggcggtgcgaccatgaccaatggccgtggcctgtacgtccgcaaggacaccggcgcactggacgacgaggcggtgaccgtgatccgcttcgacctgaacttgcacagcgagctggtggaccagtacatgagcgccatccgcgccatcgtggaccgtctgctggtgctgggtgaggagagcgtgctgcgtcgccgcttctacaatggcggcggtgggtacaacagcgagctgatctttcagtaacccgagccgggtaggctacgactggcccacgtacgggccatcctatcaaccgtcaagaggaaccatctacatgtcgaacgaaaacaccaccgagcagaccaccgtcagccactacgaagccaagcgcgccgagctgctggaagacatcgccaaggcgcaggccaaggtcgatggcctgaacgagaagctcgccaagctggatgccgtcgaggccaacagcgccgccatcgaagcgctgaaggcgggcgacgccgtgtcctacctgttcggtcgtgccctgaacaagcgcgtcctgtccggcgtgatcgtcgccaccggcaagaacgacaagggcgtgctgcaactgaaggtgcagaccggcgaaggtctggatgccgagctgaacctgatcgacagcagcgccctgctgatgtcggccgaggaagtgctgaaggcgcaggaagaaatcgacgccgccgttgccgaggcccagcgcctcgccgccgaagccgctgccgccaaggctgcgggtggcgaaggcgggcagtcgtgagcctcgccccgccgtcacccagcgtggccgtcgtcaagcgtggcgacgagctgaagcccggccagaatgcgtacctgatcgacacgcggcagaccaacaagctgccgaagggcaccgggttcgtcgtgtccaagctgaccagtgaagacggctcccgtctgatcgtcagcacggacggcaacggctccgtcctgtacgccaccagccacgacatcttcgaggtctgggaataaccaagcgaggatagcatgagcgatacccttcccgacaacgactggctaccacatgccgagcgcctgcctgttggtggccgcacacgtgtggcccatgagtgcggggagggtacgcccttgcttatctcacgagagcacgacaagtccaccgcattctgtttcaggtgcggtggcacaggattcaagcgtgagcacgagagtatcgaggccaagcttgcacgaatccacgccgagcagacgagcgaacgcagagtgcgtgcgactgttgagttgccagagccacgggtatacgacacccgcgagtggccgctcgacgctaaggtgtggttcttcaagatgggactctcgcttcagatgatcgagaagctgcggctgtactggtgcccaagcatcgggcgggtggtactaccgatcactgaaggcgacaacgtggtatactggacagcccggtcggcaacgagacagccgaagtggctaacacctgacgttccgaaagacggacttgtcgcacgctacggcgtgggcacaggtgacaccatcgtactgtgcgaagacccgctcagtgcatacaaggtgggactggtaaccgaagcgtggtcgttgctcggcaccaagctgcacaacaaagtgttgaagcagctgactgatcgaggccaacgtgtagcgacgtggctcgatgacgacagaggtagaagcaacggtagcaatcccggccaagacagtgcgcgagtaatcgctgcgcgtctacgtgcgtttggtctggactacaggaacatcacgtcaccacgtgacccgaagtattacacgaccgactacatcaaggagaagctgcaatgagcaaacccatcgtgcgctaccggcgcgctatcatcccgcccgtcgttggcttccgtgccacgctcggcggcgtgcttgcgcatccgaacctcggcgactgcgacatcgtgcacacctcgacggtgctgtatgtggcggacggcgggcgcaagttcgagacgcgcaacacccggtatcaccagctcgattccaagtacgaacccgaaggagaacctgatgagtcttgacaccacgctgctgcggttgtgcaccaaccgtggcaagttcgaccggctggtacccagcgcaccacgtgatgggctggacgagctgaccgtgctgatgctcgatgcgttgcgtgcgtactacaaggagttcccggacacgaaggacttgccgttcgatgtgttcgatggctgggccatggagttcaagtggaagacgcagcccgacgacaagaagtccctgctcaaagttctgctgaagcagatgcgcgagccggtcccgcccgaggcagagcagggcatgatcgagaagctgttggagttggagcttgccaccattgcggtcagcaagatcgtgcagtggaatggcggcgctgagttcagcctgcgcgacgagctgtacggcttggccgagacgatcaccgaccgaatggatcgcaaggcgcggctcccgctggtgcaggagacgcccgaggaactgatgcagatggacgagcacgacatcggcatccacttccgactgcccacgttggcgaagaacctgcgcgctctgcgtggtggtgacttcggcatctacgccatgcgtcccgacgcaggcaagaccacgttcctgaccagcgagtccagccactggatcacgcagctcgacaacgtttggccggaccagaagcgcaccggcatctggctcaacaacgaggggccgggcaagcgcatcaagcagcggtggtatcagtcgctgctcggcgctaccatccctgagatggtggagtgggcgaaggatggtagcatccgcaagcgcatcgaagatgcgatgggcggggacatccaccgcatgcagttctacgacatccacgggttcaactccggtgaagtcgaggccatcatcaagcagaccaaccccggcttcatcatcttcgacatgatcgacaacatcacgttcaccggtggcatgaccaacggcgggcagcgtaccgatcagatgttggaggcgatgtatcaggccgctcgcaactggtgtgtgaagtacgacgccgtgggcgtggcgacttcgcagatcagcgccgagggtgagggaatccagtacccgccgcagtccgcactgaaggacagcaagaccggcaagcagggtgcgtgcgacttcatcatcatgggcggcaagctcaatgacccagcgatggaacgcttccgctacatcggcaccccgaagaacaagctgcaccgcgcaggcggcaagcgtgacgttcgggaagaagtgatgatggatgcagagcgtgcccgcttctatcaggaggcagcatgagcaagccaattcacatcgtagccaccgggttcacggtgtcggtcagcttccccggtgaatccaccgaggcgaagaccttcaactgcgtgagcaacgcgcaagcaatccaccttgccaagctgctgcgcaaggtgcacgacgcaggctacatcgaaggccgcaacgacgcgccgcagtggaagtggggatggctgcggaacaaacacagcacttggatcggcgtgcactactcgccgcacaacaagcgctggtgcatcaatctgatcccgtgcttcacgttctggatcaccaagcccggaggtaacacaccgtgagtaccgaaccgaacatctacctgccgcgcaacgtgggcgtcatcacgtccagccgcaccggcagcagctacacagtcgagccgcccgtgaccgacacggacatcgacttcctcgtgctggtgcaggacttccacgaggccatcgaaaagctggtcgatcagggatggaccctgtgctccggtgccgatggacactacgaggaggacgaggactacagcaccacgtggtatgcgctgcgcaacggcgtgttcaacgtcatggtgaccgccgactccggctggtatcagcgcgcggtcgaggccaccaccatctgcaagcgccgcaacatcaaggacaagcaggaccgcatcatcgtgttccgttgggtgcgcgacgggctggacttggatggcgatgcgtcggatgaaatgtaccagctggccctgcaacggtggccgctgtgagcttcacttccttcgacctcgaaaccacgatccgttccatcctgaagcgcaaggccaatccgttctacgacatgaacaagatcgtggcgattggctacaagcggaagggtgacgcacggaacaccggcctgtactacgacacccgagtcgggatagacaaccagtacatgggcggcgcacccgatgggtggctgcgtgagctgtgttacgggcagcagttcctcgtcgggttcaacatcaagttcgacatcctgcacgccatctgccaaggcccactcaaccggcaggcatggatcgagttcatcgacggcggcggcatggtgtgggactgccagcttgcggagtacctgctgcacggcatgacgcaagagttccacatggcgagcatggacgagacggctccacgctacggcggcaacttgaaggacgatgcagtcaagtccctgtgggctgcgggcgtggacacctgcgacatcgacaagacgctgctgatggattacctcctcggcaccaacgacaccgacgacgtgggcgacatcggtaacaccgagaagatgttcctcggacagctcgccgccttccgtgcacgtggtggtctgcgctcggcgctcctcaacatgggtgcgctgtgcttcaccatcgaagccgagtacaacggcatgtacgtggacaaggactgggcgcttacgaaggcgaaggagttggaggtcgagcttgcaacggcgaccgccgaactcaacggcttcatccccgagctgcccgagggcctgaccttcaactggaacagccgcttccacaagagcgcgctgatcttcggcggcaaggtgaagtacacggccaaggttccgatcatgtccaccgagggtgggccgacttacgtgcagaaggacgaggtgcactacgtgctggtcgatggtaccacgacggcgacgccaccggccgaggacttcgacaacctctggcgctacaccacgtacggcagcggcaagaacaagggagagtacaagaccaagaaggtgaaggtcgatgacttgaccaagcagaagttccgcaacgaggacatgctgttcgagttccctggctacaccgagcctgatgctgcatgggaaagcaagagcgatcccggcgtgtactccaccgctgccgacgtgatcgaggcgctgggctaccgcaacctgccgttcaccaaggcgcttgccagacgcgacgacatccacaaggacttgtccacgtactacatcacgacggacgagaagaccggagagcagaagggcatgctcacgctggtgggaccggacggcatcatccaccacaagctcaacatgaccaacacggttaccggccgcttgtcttccagcgatccgaacttgcagaacgtgagcaagggcgagctggacgaggagacgttggaggagaagggttcgcagatcaagcgcgccttcgtgtcccggcaccggggtggcaagatcatccagtcggactacacctccctcgaaatctacgtgcaggcaatcctcaccgagtgccgtcagctgatcgaggacttgaagcagggcctcgacatgcactgcctccgtgcagagcaggcgtggggtgagcaaggcaagtacgactacgacttcatcctgaaggcgagcaaggacgacaagcatcccgagcacaagaagtggaagaagaagcgcagcaacgcgaaggtgttctccttccagcgtgcgtacggtgcgggcgtggcgaagatcgctgcgaccaccggcatgtcggaggaagaagtcgaggcgctggtgcgcggtgaggccgagcgttacccggagctgggcgagtacatcgaccgcatggtcgagcacatcaagcgcaaccgcgtcagcactcagcgcttcgttccgcatcccaacgcggggcagcaaggcgtgccgcatgggctgacgtgtcagcttggccggtcgcactggaccacgccggacggcaagatgtattccttcagcgagtcaccgtccccggtgttcatcgccaacaagcccgcgagcaagggtggctgtgcgcagtcgttctcgcccacggaaatcaagaactacccgatgcaaggcaccggtggtgaatgggccaaggcggcgatgtacgtcagcctgcgcgccttctaccggaagtacgtgaccgaaccgaaggaatggttgggccgtgcgttgctcgtgaatcaggtgcacgatgccgtctacgtggatgcacacggcgacatcgcaaccaaggccgctgctctgctgcacgcctcgatgctggaagcgtcggtgtatatggagtggtggttcaactggacgctgccgcttggcgtcccgtgtgaaaccaagatgggcgacaacatgatggaggagaagaaccctcccgcagagttcgccggtctggtcatcgagtaccgcgcgtcgatccgcaaggacttcgtaggtaatcacaacccgtcgtttgaataaggagaacaacacgcatgagtcttgacgcactgttgaacaaggtcgccacgcagggtaaggatcagtcggtcgccagtggtggcagcttcgactacaccccgcccgctgccggtgtgaccaccgcccgcatcgtcgggtactacgagctgggcaagcacgagttcgagttcgagggcaagaagaagacgcaggatgaagtcgccatcgtgttcgagctgaccggtaagcagcacccgcacatcgaaaccgacaatggtccggtgccggtgcgcatgacgctgaccctcggcctgtccaccaacgagaaggcgcactacttcaaaatcttcagccgcctgcgcaccgaggagcgccacttcgtgcagctgctgggtcagggtgtgctgctggaagtcatccacaagccgggcaagcgcgacccgaacaagaccttcgccgaaatcgacaaggcttccatccgcaagccggtcatgccggtgccggaaatggagaacggcatcccgaccggcaagttcgtggacaccgtgatcccggtgccgcagcagatcaccccgctgggtgcgttcgtgtgggacttcgccgacgccgacatgtgggacagcatctacatccccggcgagtacccggagcgcaaggacgagaagaccggcaaggtcacccacgaggcgcagtcgaagaacaagacgcagctgcgcatcgctgcggcgctgaacttcaagggtcttccgtgctacgactacgccgccgccaagttggcgggcagcaccacggtcaccaaggaaggcgtcgatgcgctggacgaagtggtcggcgacgtggcgaacgccgcgcccaccgacgctgctccggccgacgacaagccgccgttcccggtggacggtagcgacccgatggcaggcatcgcctgatggacctgagcgctctcatggcagcggccggtgagcgctccccgatgccggtgcaggtggtacgtcagcacaacccgcgcgtgatcgctcacgttgatggggactacatggcgtacttcgcggctggtagcgagaactgctcggcgggggatgcacgacgcaacgtgctctcccgctgcgcacagctgaagcatgtcagcggagcgggcaagatcgtcatgcacctgacgcacgccgcgtctaccaagggtgatcgcttcctcgctgctaccacgcagccgtatcagggtcagcgccaagcaggccgcaagcccaacaactgggcgttccttcgtgagtggatggagacatacgagggcgacgctttcactcccaaaatctggctgacccgtgaggccgacgatggcatcgcgtacgtcaacgagggtgcagcattgcaccacaacatcctgcacgtggtgcacagcgccgacaaggacatgcgaatgttctgcggcgtgcacgtagactgggacggctacgacatcacagaggttccgctcggcgcttacgacatcgttggcgagaacggattgcagtacggtcacaagtggttctggatgcagatgctccacggcgacaccgccgacaacataccgggtctgccgaaggtgggcaaggtgacagcggagcagctgctgttcgagacgaagaccaacctcgaagcggtgcagatcgtgagcggcaagtacagcgaagtgttgggtgccgactggcgcaagacattcgccgagcaagccgtgctgctgtggatgcggacggatcgtgacgcagaactgctcgacgtgctgaagctcgacgtgttcgggccgaagctgaagcaggcgttctatgacctcgccgaggacgtgaacgagaagcgtgcaatcttggaggcatacaaagcatgaagcgactcactgcaacacaggtcaagctgctgcgcatcaagctcgcagcggagcaaggcaaccggtgctgtctctgtcagggacagttcggcctgaaggctccgctcgatccggtgctggaccatgaccacaagaccggcgctgtgcgcggggtgctccatcgcggatgcaactccctgctcggcaaggtcgagaacaacgcaggccggtacggcgtgcgcgacgtgttcgcattctgtgcgggcatccccaactacctgcggtcgcacctcaccaacatcacggggtacctgcatcctacctacaagaccgacgacgagaagcgtatcgctcgcaatgcgaaagcgcgaaagcgtcgggctatcaacaaggagacaccgtgacccttacccagttcattcgccgagcaccgaagcgcggcccgaagattctctgcctcgacatcgagacgttccccatcgagttctatggctggggcatgttcaacaacaacttcagcgtcaagcagatcaagcgtgactggtcgctgatgtcgttcgcttgcgaatggctggacgacgaggcgtcgttctacatggaccagcgcaacgtgcgcgacgtgttcgatgatcgcaagcagggcaaggcgctgtgggcactgctcaacgccgccgacttcgtgctcgctcgcaacggcaagaagttcgaccttcgcaagatcaaggctcgcctcgcaatcctcggcctgccgcccgtgtctccggtgcaggtgatcgacccgatgctgctgaaccgcaccgagttcgccttcacctcgcagaagttggagtacaccaccggcgtgatcgtgccggagctgcgcaagtacgaccaccacaacttccccggcttcgacctgtgggtggcctgcatgcagagcctgcccggagcatgggacgagtgcgaagcgtacaaccgcatcgacgtgaagtccatgaagttggagtacaagaagctgcgcggttggtactcgcagcatccgaacgtcgcagtgtactacaaggccgacggcagcgagcaccgctgcaacaagtgcggctgcaacgaaatgatcccgcaggatgatccggcccgcacgcaggtcggtacctacctcctgcttcagtgcaccgtgtgcgacggctacagccgtgggcgcaagctcacgaccagcgccgaggcgcgcaagcacatcaccgtcccggcataaggaaccgacatgaagatcaccgacatccgcagcggcatgcgggtacagtacatcggcaatgcgcccgcaatgatcgggctgcgtggacaggtaagccgcgtgttcgctcgtgatgtcgaggtcttcttcgacggtcgagttaagccgagctgctgcgttcccgattccctccgacagcttctcagcatcggaggcgtgaccaccaccagacgagaggtaccaatgcccgaactgagctaccgcgacgaggaccgtcgcacactgtccgaccgtggcgtcggcctgaaggatgacgggggcaagccgcaggcccgtctgctgcatgagggcgtgccgcgtgcactggcccgagtcatcgacaccctgaccttcggcgcgcagaagtacaaagcgcactcgtggcagcatgtcgagaaggcgctcgaacggtatcaggacgcgagctaccgacacgacaacaagcgctgcctcggcgagaagctggacccggagacgggcatccaccaccgggcgcaccacatcatcaacgagctgttcctgttggagctggaactgcgcgaggaggagaaggccagtggcgcagagtaaggcgcgctccatcaaagaggcttgggtgaacatcggcatcggctacagcatcaactacgcagcgaacatcgcgctgcttccggtgctgtggcatcccgagcatccgctgctgtcggcgcacgccatcggcattgcgttcacagcgatcagcttcatccgccagtacatcatccgccgctggttcagcaagggtgactgatggcctgcgcccgctgcggccaagtgcatcggtacgtcccacatgaggccgagtgggcgcgcttcctagaggagcaccgtacccgcaagcagttcgatgtcgagtgggccaactcactctggcatcgtacataccctgacgacgcattctgcatcctcgtgatgaggggcctcgcaggtttcgttccattcccgtcgaaggagaactgaatgctctacaagaaccagaccgccatgctcatcaagtcctacgagaacgccgttgcgtggggcgagagtgccgaccacgaggaggcattgcagaatgcggtcaaggccgggttcccgaacctgcccgacgaagatcaggccgagctgtatacccgcatcgccgatgcgtgggaaggctaccgtggttcgctcgctccgcgcaagctgtggatcggcaccatcgtcaaccagttcatgtcgtcccgcatcgcacggttcaacgccgcgctgggtgacggcaccaagaaggaggacagcgccgatgtttgatgtgcctcgccagaatgtccgggttgctcccggctacaagaagcgcaagcgcggcttcaagatcaaccgcgccttcaccaagggcaacttccgcgtgcagtggtacgacggcaaggccacgtactgggagcgctacgttccgtggtacgaagtgccgctcgccatgttccagatttggagggactacgcatgagctacatcgtccacaaggcagtcgagcaggacaagatcaagaagaagctgcggcccaccgaggagcagcttcgcaccgagtacatcgcacagccgaagtacgacggctgcaacatggtcgccatcaagcgcggccactgggtgcccacggtgaacaagggcctgcatgccatcaaggtgggcgacgtgcagatgcagccggtggatcgtggcgtggttgacctgttctcccgcaccggtgagcaggtcgtcagcgcacaccacatcgagaacgctctcgcatccgcgccgttcttcccggtcggcgtgtacttcggcgaatactggcacccgcagatcgaccagcccaccgtcagcggcatgttccgcaagaaggacggcacgcagtacaccgagccgatgttcgtggtgttcgacttcgtgacgctggaagaatgggagcagggtttcagcgacctcgtgtatcaggagcgcgtcagccgcctgccgagcatgggccacgccatcgccgagggcaccgcgccggtgttctacgccgagtcgcagggcttcctgatcgaccaagagctgggcagcatggaagcggcgaagctgctgtgcgagggcggcgcgtacgacgggctgatcctgcgcaagccgagcggcaagtgggtgaagggcgacaagggaaccaacggcgaagtcgtcaagatcaagccgaccctgacgctggacctgcgtgtgctcggcatcaacgaagcagtcggcgagaagaccggccgcgccgtgtacacggtcgtcgttgacctcggagaaggcaagacgcaggaggttggcagcggcgtgccgcacagcgagagcgagctgcctagcgtgggaggcatcgtggaaatcgaggcgatgtccttcagcaagtacggcctgctgcgcgagccgcgatacaagggcatccgtcacgacaagaaggaggcagacctgtgagcgtcgaggtgcaagcatggcacaacatggagcgcgacacggtggagctgcgcatcagcgttcctttcggcgagtacgccggttccctgtggccgaacgagacgctgcgcgacaaggtgcaggaagcgttcgccaagttccttgacgagcggaggggctgatggacgcgatcactttcgagaagccggagctggacttcagccagtcctcggcatggatgggccgcgtcgaggtttcggtgcgcgcccggtacggtgccgacttgttcggcgctgctgccacgtgcatggccgaggatatcggcggtgaggcgtggccgcacatcatccacgacctgcacatggaaatcatgcgcggtatcctgaaacgctacccgccgcgcgactacaccgtgcggcagcaacggaggtaacaatgctctcgcaagtggaactcgaactggaaacctacgccttcggtaaggagcgcatggagaagtccatcgcccgcaacgaggagaagggcggcgcggacaacaacccctacgcccaagcagtgtatcgccggttcgtgcttccgcttgcggagcgcatccgtgcggacatcgactctccgcgaatcggccgtgcgcaagcgcacgtgccacttctgcgcgccaagtacgatcccgagcgtcagaacaagcgtggacagcccgtcagcgccgaggaacaggcacgcgagtggtacgaggctgtggccttcgtcgccgttcgcggtgcccttacctcctgcatgcgagacaagcacggcgaaggcagcgaccgcgacgtgttgaagaacgttggcatcaacgtgtaccatgagtacctgctgacgcagttcgccgacgcggagccgactctgttctaccacctgatgaacgacatggaccgcaagctctctgtcaacgagaaccaccgcatgacggtgatgaagatgcaaggacgcaagaacggcatcgagttcgtggagtggggacaggcacagcgcgatcaggtcggcgcgtacctgtgcgatcagcttgcgcagctgggcatgttggagattggcgtggtcaccgagactgctgccagtgcaggcgcagcgtaccgcaagttccagaccaagacgcacgtcaagatcgtgctgaccgacgaggtgcgcaagctgattactcagatcagcgacttcgtgatcgaggccacgccgttctacctgccgtgcgtcgagccgccgatggactgggtggacatcgacaacggtggattccacacgaaggaaatgcgccgactcaatccgtggatggtgaagacctacgctcagacccgcgacgagtaccgcgctgccgagctgcgcaacgagatggctgcgatcaacgcattgcagcgcgtgccgtggcgcatcaacaagcgactgatggaagctgtgtcggccatcgccaaggtgcacgacatggaggaaatcatttctcagggcgagctgccgaagccgcgcaagccggagtggctgacgaaggacatgaccaaggaaaccatgtcccacaatcaggagttggagttcaagcagtggaagcgcgacatgtccaactggcacaccgacgagcgcctgcgacagaacaagggcaatcgtttctacaacgcaatgaaggtggcgcgcaagttcgccgagtacccgagcatctacttcgtgtacttcgctgacttccgtggccgcaagtacgttcagaccaccggcgtgtcgccgcagggttcggacttgcagaaggcgctcttggagttcgccgatggcaagccgctgctgactaaggacgcgaaggattggttctgcatcacaggagcaaaccgatggggatacgacaaggcgtctctgccggatcgtgtgaagtgggtagcggagcatcacgaccagatcatggcgttcgctgcggacccggtgaacaacgacgagtggaagaccgccgacaagccgctgcaatttctgagctggtgcatggagtacgagcagtggcaagtgttcggggatcgcttcctgagccgcatcgcagtcggcatggacggttcgtgcaatgggcttcagaacttctcggcgatgctgcgcgacgcagcaggcggcgtggcgacgaacctgatcccagcaccgctgccgaatgacatctaccagatggtggcagaccgcgtgactgccgtcctgctaggcgaggacgaggatgccgaagggtaccgcacgctgtggctcgaccacggcctcacacgctcgctggtgaagcgcagcgtgatgaccctgccgtacggctcgcggcagtcctcgtgggcggacttcatcatcgaagactacctgaagtgtgggaagttcccctcgctcgacaaggccctgtacggccccgcagcgcgcttcctgagcaagcgcatgggtgaggccatcgccgacaccgtggtcgccgcagcgggcgcgatggagtggttgcagcgcggctccgggtcgatcctcaaccaagggtacgaccgcatccggtggatcacgccgtccgggttcccggtggtgcaggtctactgggagtccgaggagcaccgcatcaacaccaagctgtgcggcaacgccaagctgtccctgcgcaagagcacggacgcggtgaagaagtcccggcaccgcaacggcatcgccccgaacttcgtgcacagcctcgacgcaagccacctgacgctggtggtcaacgcggccaaggccgaaggcatcgacgccttcgccatgattcacgacgacttcggcacccacgccgccgacagcgcggcactgtaccggatcatccgggaggtgttcgtgtcgatgtacgagcggcacgacgtgctgtcggccttccactcggcctacccgttcctgccggagccgccgccgatgggcgagctggaccttcggcaagtccttgattctccgtacttcttcagctgacggagtttcagtacacctatagcacgaggcaactgaggtccggttggagcggccgcgaaggtaagcggaaccggtgccggaccttttggtacacctatagcacagaggagacaccatggccgaagacgccaaagtgaaagtcctgatgacgctccacccgaaccagctggccgccgtgcggaagctgtccgggctgtcgctgtccgtcaactcgaataccacgcccttggaggcaggtatgcagttggggatggcccgcgtcctgaacatcttacaggagggtttcaccgttgattcctccgtaccgaacaccaacgacgggtgatagtgagcagatcaaggcggctttaacggccgctttgtatctgtcatctagagaagatagtaaggtagacaacagagaatcttctgtgagctacaactgtgatgaccctgattacacagtggccctgataacacagggtctagtggatgcagtaatcattgatgaagcctacctgctgtgctttgccattgtcacaccgtggtactccaagaaccgtactacgttcgttgagaacatggtgctgcgaattgggccgggcagttccttcgaccggtacatagccgtgatggaacatctggctgacatcaaccactgcgactcactgagcgcaggcggtgcactagctcggaactcccgagcactcacacggatgtatgcacgctacggctacctgctggaacggcatgctccccaattcaccaagcgaaggagttaacctatgggtagcatcgttggtggtgggtccgccaagcgagcagcgctgaagcaagctgctgctatcgacaagcagaccaacctccaaactcaatccacgaactaccagattcaggcgatggccgatcagatggcacaggcagctgcacagcaggccgcatctgagtacgccgagaagttgctgagtgcccccgtcgataccgtcgatgtgcggctgggaacttccgacctcgacttgcagactgccgacctgatcggccgacgcaagaccgcccgctccacttacacccgacccgtgaccacgaccgcagcttcccggctgacgaccgtggccgggtcagacctgttgtgaggtgagcatggaccatccgatccaaaccgctcaccgccagttcgaggcttacgacaacaagcgacagggcatcatgtaccgactcgaacgctattcgagctggaccgtgcccaagctgttccctcgcaagaaccgcgatcaggacaccgagccgctgacccacgggttccagtctctcggcgcgcaggcagtgaaccatctggcgaacaagctgatgatgtcgctgttcgcaccgtcccgcccgttcttccggttggagctgaagcgcaaggcgaagcaggctgcgcaggagcaaggcgctgacttgcaggccatgcaggcgatgcttgcgaaggccgagcaggatgccagtctcgaactggacaagcgctccatccgctcccggctgtacgacctgctgaagatgctgatcgtgctgggcaacgccctcatggtgttggagaaggacacgatccgcgtgctcaacatgcggcactacgtggtcaagcgcacccgcaccggcgaggtctacgaactgatccttcgggagaaggtgcacaagacccagctggaacccgcagcgctcgctgccattgtcgcgcacccggacttcaagcccgatgacgacggcatggtgtgggagtacaagtgggtcaagctggaccacaagaccggcaagtacaacgaagacgtgtggatttgcaactgcaagctgcccgccaacttctcctcgacctacaccgcagacaagctgccctaccgggcggttagctgggacttggccgcaggcgatgactacggctccggcttggtcgaagactacgaggccgacttccagtcgctctcgatgctgtccgaggccgcagtgcagggcgcgatcctcgcctccgagttccggtggctggttaaccccgcaggtcagacctccgtcgaggacttcatggcgtcgcccaatggcgcggccattcccggcatgaagggtgacatcgagctgattaacgcaggcgtcgatggcgtgctgcaaaccaaccaagcaatccagtccacctacatcaaccgcatcggcgcaggcttcctgttgcagacggcggtgactcgtcaggcggaacgtgtgaccgcgcaggaaatccgcatggtcgccgaagaactggaaggcgggctgggtggcggctactcccggatcgctgcggacgtgcaggtaccagtcgccttttgggtgatgaacctgacgggccgcgacatccgaggcaaggacttggagcctgtcatcatcaccggcttggccgcgctctcccgtacgggtgaccgtgaccggctgttggagttcggcagcaacctcgccaacgtcctcgcactgccgccgcagattctcgaacgactgaagctgtccgcgtggatcgcagacctcgccgccgctggtggcttggacccgaacgtctacgtgctgactgaggccgagtacggccagatgatgcagcagcgtgcacagcagcagctcgccatgcagaacgcatcccagcagatcgacaacgccaacaacatggagacacagacacaatgagttccaacgcacctccgggcggtggtcccggcgcaaccgtgatcgcaacctcgaacggcaaccagcccgcaccggcagctccggctcccgcagacgacaagctgttgcccaacggccagcccgctccggccgcaccggcacagcccgcagctcctgctgcacctccggctgctgacgcgctgagtctcgaacctgccgctcccgcacagcccgccgccccggcgaacgctgcgccgactgcggtgtcgatcccggactacggcgacaacggcctgaacatcgcggccgaatacttcgtcaacaccgtgggcctcgacatcgacagccgcgaactgaccgaagcagcgaagggcaacttcgccctgctggaagccaagctggaagtcctcggcgacaaggccaagggttccgcaccgatcctcgctctggcgaaggagagcatcgctcgtgtcaccgccgctgcaaccgcagcgcacgccgcgaacgttgctgctgtccacgaagccgtgggtggcgcagagaactgggctgcgatccagcagttcgcacgggccaacctgcccgccgaccaactgaagcaggcaagcgaatcgctgtcggctggtggcttcggcgctcaggcgaccgcgcgttacctgatggctctggcacaggccaatcccgcgacgaccgtcaagggcgcaccggctaccaacgccgccgcccccgccgcgtcgatcaacggcgtcgctcctatcacgaaggagcagtaccgcgctgagtaccgcaagctggttgccgagaagggcatccgtggtgcggcccactccgaagaactgcgtgcactcaacgcgcgcgtcatccactaagaccaaggagcaacacaaagcatgagcaccatcttcccgactgtcccggttctgccgaatcaggtcaaccagtccggcaacgagaacgccctgatcctcgaacagttcaccggcgatgtcgagcacacctacgtgtccagctcggtgctggaaaagttcttcccgcgcaagcaggtcaagggcaccaacaccctgaccaagaaggccatcggccgtaccaagcttcagaagctgaagcgcggtgacgcgccggacggcaccccggtggacttcagcaaggcgtcggtgaccgtcgataccatgctgctgtcgcgtcacagcatctggcagctggacgaaatcttcaccgacatcgacacccgcaaggaaatcgccatcgagcagggtcaggaaatcgccgagttcgtggacctgaccatcagcatcgccgccgcgaaggccgctgctgccacgcagtcgatcttcacccgcaacggccgcgcgcccgagggccacttcggtgccacgcaggtcgtgctgtccgccgctggtgacgagaacgatccggccaaggtgtacgccgccatcggcaaactgttctcccgcatggaggaggagaagaaggtcaagccgcagcgcgatggcgtggtcctgatcgtgcgcccggcgatcttctacctgttgcagcaggccgagcagatcagcaacggcgagtacctgacctcggacggcaacaagctgaccggcatcccgaccttccacggctggggcgtcccggtgctgtcgagcgagaacctgccgaacaccgtgatcgaaggtcacctgctgtcgaacgacgacaacgacgacttctacgacggcgacttcagcaccctgatcgccgtggccgtgtcgccgaaggccctgctgatcgccgaagcgctgccgttgcagtcctcggtgtggtggagcgatgcctcgaagtgctacttcgtggactcgtggatgtccttcgccgttggtctggatcgcgtcgagaacgcgggccgcatcgacaaggttgcctaatccgctgggcgcggtccctgaatccttcgggtaactcaaaccgcgcccttcttccaccaacacaggagcaacatcatggtctttgaccgaccgttcgagatttccaaccgcgtcgtcgccgcaactggcgtggccggtctgcccgccaactccgttggtaccgtcgtcggcgtccactacgacacccgtggcaccgcaggctgggtcgtccgtgtccgtttcgtggacgacgaaatcggctcgcaggacatcgagtacgcaccggccgctctggctctggctgcggactaagcaacatcccggcaggggcgctccggcgtctctgccttgttcctctcaggagacaccatggcattcatcaccaagctcgacatcgtgaacgcctgcttgaagacgatgggcgagacgaagctcaacacgctggaagatgaccacgtatacaaggacgacgccgttgacttgatcgaccgcgtgcaccgtgacgtgtcctcactctcgctgtggttcaacaccgaatgggtggagctgaagccgcaggcaacgagcaagtacatcatggtccccacggacgtgctgaagctggactgcaacccgagccggttcggccacgtggtgcagcgcggacgccgactgtacgaccgcaagcgcaacacctacgagttcgaccacaacgtgcaggccaagctggtgcggctgctggacttcgatgacctcccctacgaggtgcagatgttcgtgcgcgacgactcggtgctgcggttccagtctgacttcgacggcgacaacaccaagtacgccaagatcaagcagcagcgcgatgacagttacatcaacttgaaggccgagcacatccgccagatcaaggcgaacccgctgttcgctcgcgcatccgtggacgtgctgcgttcccgttactggaactacagcggtcacccgtggcacagccacgtcacattccccggctaaggagacaacatggcaaaggcaggcggaacctatcccgacatccttcagggtgtcagtcagaaaccggcgcatcgtcgtcggccgggacagacgcacgagcagatcaacgtgctgtccgatccggtgaacggcctcgtgcgccgtcgtggtacgcggttcgctgcttcccaagccgttgtcacctcggccgagctgcgcaacatggacgtgttcgacttcatgcaggagggcaaggagtacgcgctgctgtaccggcgcgacgcctcgaccttgggcagcgagtccttcgcgttcctctacaacaagacggacgagtcgttcatccctctggtgtacgagaacagcacgtgggtcaacacgctggtcagcggaggcgcatcgtcgctcacggccatcggcagctacgtctacatcgcgggcaacaccacgatcccctcggccaccagcacgaacgtgtggcaggagcagacgaacatccagcgcctcgcagcatgggtgcgcaccgggaagtacaacaccacgtacacggtgaacctgacgcggacggacaacacggtgctgacggtaacgttcaagacggttaccgcatcgtaccccggaacgctcgacaccagcgacatcccgttctaccttcccggtggcacggagccggacgcggcgtaccagaagtacgtcaacgaccgagtgaacgagtacaactctgcggtcaacgagtggatcgtgacgagcgctgagcagacgcgcccggagtacatcgcggagcagctgtcggatttgctggtcgatgcaggcgtgtcggcaacgtacatcaagggcgggatcatcattgacgatgaccagttcaaggacatcacggttgacgacgagggagacggcacgaccttctacgccgcagggcaggaaattacagacgcgacctacgccgtcaagttccactggcacggcaaggtcattcgcgtgcggccgagtggtgcaggcgcggacgagtcgtactacctgcgcgctgagttggagaacggcgagacttccggctacgggtcggtggactggtacgaagcgcccggcgtggagtgcaccatcgacaacctcgtgtcgcagctctacatctacaacggtgtaggctacatcgcacgcaacggtgcgggcctcacgtctctggctccgagcagcggcgagcatccggcctacggtgcgcgagtggcaggcgatggtctgacctcgccgatcccgtggttcatcgacaagccgatcacgatgctgtccgtcttccaagaccggctggtcatcggcgcacagaactacgtcaacgcctcacgctcggcggactacctgaacttctggcgcggctcggccgtcaccatcgaagacagcgaccccatcgaaatcttcgcgcacggcagcgagggcgatgtgctccggcacgcgacgctctacaacggcaacctcgtgatcttcggtgaccgtcagcagtacggcatcagcggcgactcggtgttcagtccgaagaatccgctgattaaagcgttcagtgccaacaaggattcggttgacgcgaaggcgcagacctcgggcaactacatcttttatgcgcagtacggcagcgaaggcacgagcctgcaccagatgcgagtgggcgcgctcaacgggcagcagacggtgacggacgaaatgtccaacgagctggactcgtggctgtcgggcactccgttgcagatcaccccgctcactgcgccgaacctcgtcatgttccgcactcgcgagcacccgcaggacttctacctgtaccggtacgaggacaacaagaacaacgggcagcgcatcgtggatgcgtggtcgaagttccggtaccacccggcgctgggcgaaatcatcggcgtgagcagctacaagaagaacggcctcgtgttcactgcgcgcgggtcgctggtggcgtgcgacgtgttcgacccgaagggcgagccggactcgcatgcgtgcctcgacagctgggcgagttttggtacacctacgggcgtacagactgcgagcgcaagcatcgccgtcaatagcactagcccgtacttcctgctgggttgtccctacgcgcaggcgtctgacttccttaaccagttcgatgacctcgctgctggtgcgctggaatacggcgtggtgtccgaagctctggtgatcccgaccaatccgttccctcgggaccagaacggtcaggccgtactcgatggacgcatgtccctcaacaaggtgacggtggacgtggagaacacggcaggcatgatcgccacggtggcaacccgcaacagcaatgtgaccactacggacttcgagggccgcatcctcggcgactccgacaatctgatcgcgcggcaaccggtgtaccgggggcagctcaacatcagcgtcgggcgcgaagtgcgcgagtgcacctacgagattcgcagcaaggattggctcccgctccgggtgaccggcctgagctggacgggtcagactttcaacaatgtacggagggttagctaatgggttcggttaatacgatcctgcaagcgaacaacaccacccgcgttgcccgtgcgaactaccgtgcagccgttgcgcagaccgacaaccagaaccgcagcgaggtcgccaagaccggcttcgctgatttcatgcggtccctgaagaacaacgcccaactggacgccgccgcgaaggagtacaactccaacatggaagcgctgtccgaggagctgcgtgcgcgccaaggggctgggcttaactcccagctccaactggcgaacgcgcgtggcgcacttcaggcgcaggctggtgctgtcggtgtcggcggctcgtccgcagacctgatggattcgatggtgcggttgcaggcggaaatggatcaggagacgcaggccaacgctgtctcgctcctcgcctcgcggggcgcatcgcagactgcgcagatcatgtcgcgcgcgtggaacgggatggacatgagccgttcgttcgggcagttcgactactcgcagcacatcgagccgcaggcaatgaagcgtcgcttgggcaagctgatcggcgtggccgtggctacctacttcggtgggccgatggcaggcgaggccgtggcagacttcgcggtcggcacgtggcaggcggacaacggcaacttcactggtgcctctcagtccttcagcaacgcagcgcagaacggtatgcaggcgtggcagcagtccaatgatcgcggcggcaagtcgtgggcgtccactaccttcgggtacaacgacggcaccggcaagcagtccgtgactggggcgaaggtcaccggcaacttcggcaacaactacgacaacttctccaccactacgtccggcctcggctggttcgatagcggcagcggaggcaactcaggaggtgcatggtaatggctgacatcggcacggttaccttcaacacgcagtccgcattgcagggtggcatcaacgccaccccagcactgtcgggcaacaccagcattcaaggcgctggtgtgaatcaggtcgggccggttcaatccggcaacgactggttcgcaagcactggtggtatgacgatgccggacagcaacctgccagagttcttgcaggagctggcagcgccgaacaccgccaagctgaagcagcagcagatgtgggacggcttcgttgccgcccgcgctggtaagaccatggacgagattgctgcgaccgaaccgtggtacaagaaaatcttcggagacaccaactacgagattggcgcgagcatgtataacacgctctcgcaggtcaacgaaatggagagcgacttgcttcggcgtatgccggagttgcgtcagcttcctcccgaggcgatggcgaaggagttcaacgacctcgccactgcccgcatgaccggcaacggtttcgcggacacggtgttgcagaagaccttcatggatcgcgcgggttccctcatggacctgcacaccaaggagcgcacggcatggcagcagcaggagctggtgaaggcgcagtacgctgcgaactcgtcggcgtccaccggcttcaacgaactggcgaagcgcacggcgatgctcggtaccaaccgtcccatggacgagaaggccaccgaggcgctgacgcaggcgcagctgtccctgctggacggactgtcgccctcgcgctaccagacggacgagtcgtacaagtccgcgatcactgcgttctatcgtggcgctgcggatcgcggcgagttccacacgctgaagttcctcaacagcaagggcgttctgaacgccatcgacccggacgggcagctgggaatccagcagtacgtgaagcaggcgcaggatcgttaccgttccgactggctcgatgccaacccggagcaggccgagaagatggcgctcgtctccatgtacgcatcggagggcattggtgccaagccgtcgcaggcgatgatcgaggaaatgaactcgacctacgccgccgagactggaagcgacgcaccgctgtactccggtacgcagttggcttcgatcatggcacagtccgcaggcgcgcacatccgcgcacaggaagccgtcatcaaccagcgtaacgctgcggccaaggccgcgctgaccgaccagcagaagctggccgcgcaggaggaggacatccgtggtggcatcgaagcgttcaagcgcggcacgtacgcgcagacgatcaacatccccggcgtggacaaggagctgatcgaggcgaacacggtgcaggcatggaatgccacgatggccgcgaaccccaaggtcgccatgtcgcagctggtgtggaacgccaacaccgggcgaggcgctgtgctgaagggtgtggccgaccagttccagaccacggcgcgcgctgtgctccgcgatcagccgaacacggcagcggctgcactgtaccagcagtggaaggaactgaagcagaccaccgccgcacgcatcgacacgaacggtcagcccgtgcagggccgactgactggcgcgactaccgctgcgctgtacttcggagatagcgtcaacacgttcttcaacaagctgcaagcgttggagaatggtggcgtgaacttcgagcttgcttacgaggtggcccgtggagaaatcaccaccgacgatccgacgcagttcgacgcgaacagccgtaaggaatccgaggctactcaggctcgtgttacggaagctatcgccaagctcaaccccaagtacctcggcatgttcggcaacaagctgggcgactctggccgcgctgcgtatgctcgcgccatcgtccgctcggtcactgacaccggtggtctgctggacacttctgcggaaggcttgcaggctgcggctactcacgccaagctggcctacggtctggaagacgcaggcaagtacgcatgggaaaacggacgcgacgacgaaggccgagtgatcggcagcgtcggtgcatggctgggcttcatggacacgaaggaaaccggacccgccatcgagaaggccatcgacgcagcactgcgccgggtcaacatcgagccgagcaccgggctgaaggctgacgtgttccgcatgaaggacagcgagaacggcgagccggtgctgtacgtcaacgctgttggcgagaagggctggaaggttgtgccggtgtacgggcgcgacatcaaggacgagtacgagaagcacaccaagcagcagcgtcagttgcaggccccggtaccgcagggctacgttcgcatgaacgacggtacgattcagcagagcatttccatccaacccaaactgtaaggagatagacaatggcactcgatctttcggggctgacccaagaccagcagattgccaaggctgccgcttatgcgggagtgccggagtccatcgtgcgcggtcagtggcgagtagagtccggcaacgggcgtgccgccaaggacgctgacggtgtgatccgcagcaaggcaggagcacagggcgacttccaagtcatgcccaccacgcaggcaacgtgggaagcgcgcaacggtcgcaagtacgacatgcgcaacttccaagacagcatcgagctgtatgccgacatcatgcgcgagaacatgcagcttgccaagggcgacgtgacgaaggcgctgcgcatctaccaaggcggcaccaatccgaagaactgggggcaggagaacgcagcctatgcaccgagcgtgctgggcggtgcgtccgctcccgcagtgtcggcgcagccgcgcagcctgaccaccacgcaggcagacctcaacgccgcatggcagggcaacccgaacatgcgcgaccgtacgtggtccggtgcgtccatcccggatgcgtggacgggtgcgcccatcgaaggccgcaacgctctggcgtcggcagcgaaggaacacatcggcaagattcgtgcgggcatcgccgagctgtcgatgggtcaggtagcacaggaaggtggcaccgccgcgcaggccgtaggcaaggctcaggctgtccgtgcatcggatcaggttgtgccgtggtgggtgcgtcaggaagtggacgtgctgaacaccggcgctcgcaaggcgctgctggatcagaccgaacaggcgctcgcgcaggaccgcgcggacgaggagctgcgcaactcgctgaccttcctcgacaagtggggcgctgcgttcgacagcggcatcggtgctgcgatcagcaaccagtttgcgcgcgaggacgagaacgttccggaaggttggaagtacgacccgaaggaatgggagaagccgtggatgactgccgacgaactcgaagacatccgcgatgcagcgtactcgccgaacgagctgaagtacgtcagcgaccgacagttcctgcgccgccactccatgcgcatcaaggatcagcagactggctggggtagcttcggttacgacatggtggcaggcttcaccgatccgggcaactgggctatcggcggcgtcactgccgcaggcgctaaggcgctgggcatcggctcggctgcactcgttgccgaagggcgcgtgggcgcgtcgctcgcgtcggctgctgcggagaacgcggtcggttccgtcatcacggacgccgcgctggttggcatgggcgagcgccgcaacttcgcggacttcatgaccgacgctgcattcgctaccaccataggcaccgcgatgcacattccgggcgtgcgctcggctgcgcagattcgtgacaaggcaaccatcgacctgtccgcaggcaacgctgccgcttacggcgaagcgtggtcggccgacctgaaggcgcgcgctgtggccgagctgggcgaggacgccaacccggtgctggtgaacaaccgcatccaccagcttgccaagcaggaggctgtggattggctgcgcgctggtatggccgacgtgcctgacgacttccgtatcttcgcccgtcccgacgtgcaggagacgaccaccaccgcaggcaccactggtgcactcgcacgggacgcgggcaacgtggacgcaacgaccgggcggtacaacgacagcgtgggtggccgggtcgatcagcatgacccgctgctggaacgcgcatggaagaccgcaggtatcaagggcggtaacgtcgatggcgtgctgaagtatctggaatccaacgcctctatcccggaggacgtgcgtgctatcgccaacgcgctgaagcgtggcgggcggctgagcacggtgaagatcgtgccggaatcggaactcgacaagtggttcgccggtgccaacatgggtccgggtatgcgtgtggccggtggctacaacgccggactggacgcgatggcgatgcggaactacacgccggaagtggtggtgcacgaaatgctgcacgctgccacgctgcgtgagctgcgcagcaactcggtgttcgggcaggaaatggaagaactgctgacccatatcaacaacagcatcggcagtgtggactccacgctgaccaccgctgcgatggagacgcgcatcaaccagccgcaggcaggcttcctcgccaacactgacgagctgatttcctacggcctgacgaaccgcgctgtgcaggcggtgctgcgtcagatgcccgcgccgggcaacacccgcccgaatgcgtgggagtggctgaaggataagatcgcgcgagtgatgggtctgaagaatcaggagtccgcgctcgaacgcctgatgtcggtcgtcggtgacaacctcggcgcggaagtgcgcgacacgcaggccggtacccggcagacgcgtggcatgctcgccaactcgatcttcaagtcgaaccgcgagcgcaaggctttctaccagcgcaccggtctggacaagtccgtcagtgatgacgcgatgcgtgtgcaggtcgccgaagtgatggcacgctccgaacgcttcagtgcgcagtacggcatcgacgcggcgaagctgtccaccatcatgcagcgcttcgggctggaagctacgagcacgactctaatgtcgtccaagtcgccagttgcccgcatgcttgcgatcaccctgttggagaatcccgagggtgcagcaggccgacacagcaccgcagcgatggatcggcatggtcggtttgagtcgttcatgggcacccgcccgcgtcagtgggaagcggcctatcgcctgtggcgtgcggacgtgcgcggtatcggtgcgatcaaggacttcgccacgggctggaaggctcgcgcggacttcgagtacgcagtgaagctgtaccgcgagactcgcttcaacggcggggacatcccggatgcgcacgaggcagtgaaggcaatggcccgtgagttggaccgtggctacaaccgcatggcagcagagcagcgcgcggccggtacggtgggcgcacagcgtctgccggaggaggacgtggagggctacgagtcccgtacgtggctgggcggcagcatcgctgctgctggtccggtgcgacgcgagggtatccgtcaggcgatgcgcgatcagttcgaggtgatgggcgagctgtatggggacgacttcctcgataagttcgctaccaagtatctggaacgcatcgagcgcaaggctgcgggtgtcatcgaagcgccgggtcaggtcttctcggagtcgcaggcggacacgctgcgcgacactctgcgggcgatgtcgctcaacgaggaggagattcagaaggtcatgggcaagtacagccgtggcggtgcgaagcacaccaaggcgcgtatcgacctcgacgtgaccaagcagtacgaggacgctgacggtaagttccgtctgatggactatctcgacaaccgcgtgatggacaactaccgcaagtacgcgggacgtgttgctggtgacatcgctctggcgaagcacggcatcctcggcgacgcaggcatcaacgtggcgcgcgaagcaatgcgcctgaccggtgccaacgatgtggagctgaaggcgttcgagcaggtgatgtccgagttccttggtcgcccggtcggtaccggcgatccgactgttctggcgaatgcgcgtctgctgacctcggccatccagctgggcggcgcgggcatcaatcaggcagcggagtacagcaacggcctcgccgctgttggtgctgctggtgtggctgacgcaatccgtatcgctccccgcatgcgcagcgaaatcatgcgcatcctgaagggcgaggacagcggcaaccaaatcctcgacggcttcgagttcatcagcggtcgcggcttcggtctcgccggttacgacctacacatgttcaactcgctggacacgcaggcgtcgatgtatggtagcgagcgcgcaggcttcctgacctcgctggtgcagaaggcagcgcatgcgaaccgcatcctctcggggcagcgggccgtgcttgctgtgcagcagcgtggcttcgcggaagtgctgatcgccaagggcgtgaagttcctgcgtgatggtgctgaagctgacaccgccctgaaggacatgggcattgacgacaacctgctgaaccgcctgcgggctacgcaggatcaggtcgtgcgctggggcgcggatggtaagctggaagcagtagacccgcgcaacgtcgaggggctggcggatcggcaggcatggttggcgttctacaacgcgatcaaccgtggcacctcgcagattcttcaggacaccttcatcggcgagactggcaagtgggcgcacaacggctggctgaagctgctgttccagcaccgcacgttctcgctggtcgcgcagcagaagcagctgggccggtacgtgggcaactacggtgcatggcagacggcgggcctgatcgctgctgcgatggctgtggcggctccgctgcaagccctgcgggtgctgtcccgcgtggccctgatgaacgatcaggagcgcgacgaggccatcgaccagaacatcctgtcgcctctggcgctgggcaaggccacgctgaactacgtgtcggcgacgggtatgctcaacgatgtgctggacgtgggcactggcgtggcgggcggctggtacgagtacgccaccgatacgcagggtccgacgtggctgaagcagctggccggtgggcagttcggcaaccgcaaggaagtggtgggcgggcagttcgcgccgtcgctgggagtcatcaacgacttcgctcagggcattgctggcaagccggagaatctggccgacgtgattccgggcgggcgactgccgatggtgatcccgctgctgaagggcgcagccagccagtggaaggaggagtaagatcagggccaaggacggcccacccttttggtacacctatagcaaacaggaggcagcatggcagttccagacccgcagctgcgctacgcgacagacgtgttcgacgccgatggcgtgaccactgactggcagatcagctttaccggtggctacatcaacccgtcccacgtgtacgccatgagcggactgctggacgaggagactcagctgctgaccgaccggactccgcacaccgtggaagtcctgagcgaagacgatgacgctagtaccgtccgagtctcgcctgccgtcgccgctgggcgcaagctctacatctaccgcagcactccggtgcagcagatgctcgttgactacgttaacggtagcatcatcagcaagacaaaccttaacctcagcaacgaccagctcctgaagatcattcaggaaatgttcgactcactcaacatcgccacccttagcatcgaccagcaggtcggtgtgatcgtggacctgaacgagattatccagaacatctacaagcaggtcaccgagttgctggcagctggtggtatcgtgtccgtcgccccgcgcgtctggtccggtgcttggactggcgatcaggtgggtgacaccgacttcgacatggtgggcgcggacgtatccggcgcgggcttctacgacgtgtacgtcaacggcatcggcatgcagccggacgtggactatcaggtcacgctcgctgacggcaccgatcccagcttcatccgcttcgccacggttcctgccgagggcagcatctggttcgccgtgctgcgtggttacgccaagccctacaccgggcctgcgccgatcaccgctgcgagcctgcgggtgccgatcatcacggcagagggtccgacttactacgccgccaaggctaccgagtacggactcgtgcgctgcacgtacgccggaggttgcgccgtcaacatcaacctgatccccgaagtgggcgacggtgaaaccaagctcgcctcgggcagctacttcagcgtgcagcagaaggcaggccctgtggtcatcactggcgacgtgggcgtgacgctcgaagtcccggtcggctgcaccgccgcaactcgcggcaccaactccgtcatcactgcaacgtgcatcgacggcgacaccaacacgtggttgctctcgggcgacttggctaaggagtaagcatggctaatcacttcaggctgtacggccgaccgctcatggcggacgaggttgcagatggcctgtcggtgacgggcgtgctggaagggtacacggcgggcgaggcttacgagtctcgcctgtccatcaacaacccagtcggccgctgcaccgtggaggtcatcgaatcgacgctcccttcgggcgctgcggtacgggtggacaacatcaccaaggaagtcgtcgtcaagtgggcggctttcactgaagtcgtggacgaggaaaccctcgtgcccaacggcgacttcgaggcaggcgacgacggcacgtggttgccgggcggtggatcgaatggcgaaggctggtcgattggcactggctcagactacgacaccgacagcggcgtgtacagcgcgcgcttcgccaacatcaagacgggcggcagcgacctgctcaacccgctgatccctgccaaggtcaacgactacatccgatgcaccgccgaggtccagcagggcgcaagctccaagggcaaggccggtgctcgtgtgtcgatcatctaccgcaaggaggatgggaccgagctgcaacgcaactggggcaacatggtttcctccggcagcaacggtgcgtggcaccagtccgttgccgaaggcgctgcgcccaaggacacgaagtacgtgcaggttgtactgtcggcgttccgcagcaagcagaacaaaccgctgtgggtggacaccgttaagtggaaccacaagtacgtactgggtcagaacgacgacagctcctacttccttagcatcaaggtcacggacgggttgaaccgtgtggcctactggtccggtcgtatcgaggagcagggcatctacgttacgtccaagctctacagcttctaccagttcgatgccgcgatgctgaccagcagctttgctgggtacagcaacatcgacatgctccagcctttggatactgcgtcgctgggttcctccttcgtaagctgggaactccgaagctctaggcaggattatgccgccgacccggagagcacgttgtacgggagcgctttcgtttcgttcgacatccgatccatccgtaaggactacacgcctgacccggagacggcgaagctgtcgagttctttccattccttcaccctgaagcagcaccctgtagtcaaccagccgctcgacgcgactgcacgactccggtctggcttcgtatcatggagcttcgcatgatccacaatcacctcggcattgctggcgtgttcaccatcagcaagggtaagtccctcgatactctcgaagttgtagccgactggcagagcaaccttatcacggacggtggtatggacgcactgggtgataccggcagcggctatcctcgcagcatgtacgacctcattgcttacttggcagtcggtagtggcagcgccaccccggcattcaccgataccgctcttggtgcacaggtggcgcaggttggtcgtacgtcctcggacagcggtgggactaccactgccccgtactacgcctactcccgctgccagtaccagttcccggctggtaccgctactggcgttctgtcggagcttggtgccaaagcatacaacaacaataccggcgcgtacatcctgaccacccgtgcgcttatcaaggactccgcaggtaacccgaccaccatcacggtgctgtcggatgaaatcctcgtggttacttacgagctgcgcatgtacgcagataccacgccggttgtcactactgagacgatcaagggtgttagcaccactgttacctgtaagcctattgcaatgggccgcagcggcggtatgaacggtcagtcggcagtcgcttggtcggactacgtgtgggggtgctactacttctacggcggtactggcgacggcaccggagctatcaccgaccagtatccgccggggacgattgccagcttctctgacttgcagcttcagcaggtagcctatgttccgggtacttactaccgtgactgcgtttgccggatgtcgatcaacaacgtgcccggtggtccgatcacggctgcaatgggactctccgcgtgcgtgaccttccaagtcggcttcaatccgggtatcaccaagaccggatcggagacggcgaacttgcgcatgcgggtttcttggagccggtacacgccatgatccccactgtctcccaaagcatccaacgcggtgactgggtggagcagcagaatcggcgcacccgcccgctcattgacttcgagcagggcgggctgactctcaacgcagcagtggacgacctccaagctgcgctgtggactgccgagagtgacggcagcagcgtcgtcgtttaccgcgacggcgttgccccggtcaccgtgctgaccgactccgggatcacgcagatcgcactggccttcgaccagaccatgcgcccgcacgtggcgtacatggcgggcggtgtgtgcaagttctactggtacgacacggtggctgcttcgatgcagaccatggtgatccccggtgctaccactccgcgcctgtgcatggacgagaagcgggctgtcttcgccacgcagagcgacgtgctcctgtcgtacaagaacggcagcaacctgtgcgtacgcgcgcagcgtgagcgcttcgcaaccgaacatgtgatcgcctcgggaatccccggcgacc

SEQ ID NO: 23 - DNA, 44427 bp, unidentified
  source 1..44427: mol_type = genomic DNA
gcgctgccttggctgaatcgttaataaatctcttggcgaaaggtgttgacgtggccggtgcggtgtggttcaatggcgtcactggggcagcgacagggcttcaggagggccgcaaggggcttgacaggggctaccctacctgctaccatgcgaaccgcagctgtaggcgtgcgagggccatctgtatcgtttcggccttttggtacacctatagcacacagtcggctcaacctgaatcaccgtctatcggtactctgtcgagctgattagttagctacccgctaggccaacggttgacgcttgcgatgcaagcagtagtagacacacggccgcaatggtagtaagctgcaacgcaagtcgagtgacgtgatccgtagtggcgccgccaacaagtgggctaagggtacacgggagtcactggtaagggatgcgaggagctaccgaaccacgcttgacactaagctagcagttagctatgataggcggcaagtggtagccaccggaacagcggagcgacctagcggtaaggctagacgtgagagattacgggtgttgaggctgaggtgagaccgggacaccggtcaagacactaacaggagcgcacatggtcctctaacggatagcttgacaaggcggcacagatagccctttgaggccttgcaacacgtggaccaccgacgtacatggtgggatggtggcgacaggacgcccaacgggttagagacccgagcgagccaagggcttgacaggatgcaacaagggtgctagtatggcaccacgctctgaggagcagccacattggatggcgtaggactaccgctaacgggtagggtgtaacgggaagcgtgccaaccacagccaatagtggccgagagttgacgtggaccgccaagctgcaacgtagcactagcggataaccggatgaactgggatttcaaaggcccatagaatccaccagacttgcaacactggtgccgctttacctaagcctaacgcttagggcttcccatctgccgtgagagtcggccacgggaagtaacccactgccaaggtgggaagccggtcataaggaggtggtgagcctcctatcgcatggaatactgtgcgtttcgtgaaaaggctctacgggccacacggtgacaatggcactgctagccggagtagggttgacagcccgaagggctagcagattgatgcgccctccctttgcgatgaccatgcaggcaaatccggtggtcagtgtgcgcccacgataggcgatgcaacggctctaatcgagaatgagggattgaccgactcgacggctttctgagggcgcatcaatctgttagttttcccaccagtgccaatggaggcacaacatgcaaggctcgatcaatgccaatctcgaccgcacccagcgtaagcgccgcttctgccagttcacccggacggcaagcgtgatggacctgcgcaccacggagcatgaccgcaagcttgccgagcgcaagcgccaagccgagcgctacgaagcccgccacggaaccgccggaaagcgatctgtgtttgttgtcgagggtaacagcgggacgaaccgggcgaaccacgccgctgacaggagggcttacctgtgatccggttcaagttctctcgccactacgtggaagctgcccgcgattcctacaatcgggccatcatgaagcatccggccggctctgtgtcggcgctctacgtcctgccgtgcggtgggcgttcattcgacatccgactcgcttaaatgcaagctactgggccttcgcaagagggcctagtgtcgtgcaatcggcacggacccaacctgaagggaaccaccatggacatcatcaccggaagcgctgacatcaagcgcgccatcaagtcgatcaacaccgcccgcaccaagctggtggaccagattcagcaggccgcgattgcggtcatcaaccacgcacacatccacggcgacgttacgctcgcttccgatctgtgtctcgccgtgggcaacggcatgaagcatgaagccctgcgcctgtacctgtccgagttcggcccgatggctccgaacgacgacaaggaaaccaaggcgagcgcgcccatgaagtttgccaagagcaagcgagtcgagggcgaagctctggccgacgtgctggaacgtgccgccgcgaaggcgtggtacgacttcaagaccgagaagcccgcagaggcgttctcgttcgccgccgacctgcacaagctgctgggccgtctggaaaaggcgaccgaggaaggctacgtgccgaccgaggaggaacaggccgtcatcaacgctgcccgcgctgtgccgaagcccaccaagaagaaggagaacgtgtaacatggaacccaagatcaaccttcgagtgacccagcgcgaagcatccctgctgcgctcggcccttcacatcgcctgtgcactgaccgcaaaggcagacccgtactccaaccgcaagctgtccaatgagttcgccgtgctgcacggtgagctgcgcgacttcggtgtcgagagcttcgagcgtgacgccatcctgcaattcgaggacgacgtgattgcggcctgccgtgacagcgatgtcgaggcacagctgctgcgcgacctgatcgcaccgccgacgttcaccgtgggctacggcatgcgtgaacttgacttcgctgctatcgaggcgcgggtgatggcgtgcctgctgtctccgttgcctccggtggtgttggatgcctcgcagctggacttcctcggcagcgtgaccggccgcatggtgttgcccggcctggcaatgcccgacaacctgccgcgtaagctgccggatgtcctgatggacgaccagagcgcacgccacgtcgccctgactgcatcgcagaccgggctggtcaacaagacgaagaccaagggctggatcgtgcagttcaatctgcgccacggcagcatcgccctcgccaactgggcgcaggtgcgtgagctgggcctgccgcagcgcagccgcaatgctgcgtaccgcatgctgaaggcgcgggccaaggtgcagggcatcagcgaggatgcgtaccgtgtggtgcccgaaggcactcccgatggcccggagaaggatcgcggcttctacaccgccgagttcttcaccaagcatgcgcggcgccctcaccagctgggttggaatacgtccactgtgatcggactcagcggcacgttcaccactgcgcaggctgcacgcaacgccatcgcctcgcacgtcggcaacgatccgaaccgtctccgccgctaccgcgtgaagtggcacccgagccgcgcgtgatctaccgctgcgccttctaacgagggcgtagctttggaaccacgcccaacaggagggcacattgcatgatccccgtaacttacaagcgcatccgtagtggggagcgcaagccgatccagctgtgcgagcagccgcgccagtggaaagagttcgtgacccatgagcacagcgtggagcgctggtatgcgtgaggtcagcctgcgccttgtggtgaaggcgctgccgctcgttaccgtgaagggtgtggctgtcggggattacatcctcggcggacatcacaccagccacgaggcgtgcgagcaagccatcgaacaccaccgcaagcaccacgagaaggtgcccaccctctactcgatagaggaaatcgaaatcccacccgtcaatcaggagaaccaccatgcgtaaggtatacttcatcgtctcgatccccaagaacagcaacgatggcgtcatcactggcgtcgtcgccaatggcaccggccgcaccccgacccaagaggaactggatgcggtgatcgccgagctgcgcaccaagggtgccaccaccagcctgctggactcgctgcgtgacggcacgtacccgaaccagctcgccatcttcgaccgccgcgccgccgtgcgtgccgaggcggatgtgctcaacagctacggcgggtcgttcttcaactggcacatcctcgaagtgggcgagagcatccgcaagccggtgcgcaagccgctgggttggcgtatcacctacgccttcgccgaagaccgcagcgactccgatgtcagctgctacaaccagcacccgagcgccaccgtgcgcatcgacggcaacgagtacaacaagagcgagtacaacgtgctgttcccgacccgcgatgcagcgcgcgccgtgttcaatgccgagtcgctgggcggcgagaacatgggctaccgtgtcgagccgtactatgcgtaagctctggctgcgcatcctgatcctgctgtactggatcgtgggtcgtggcccgtgggttgtcgtcggccagtaccatgacgacgacggcaagctgtgccggttccgcaccggcccggcttccactgggttctcgctgacgttcgatgacctcggcgcagccaacgactactgcgaccagcgcaactggaaggcagacactgacccgctcggcaccacgtactacgtgtggcatgagttggagttcaatcacttcggaacgaggaggaagtaaccatgggtttcatggacaagatcaaggctgcggccaagtacgtcaaggacaaggtggtcgcagcggtgaagccgcgccacgatgacgacgacacgccgccgcctgcgccggacaccagccggcacctgcacgtcagcgtgccgctgattcccatcgacaacccgatcctgcgcaagatgctggggcaggactacttccccgtgcagaaggggcagggtcagacccgcatcgtcggcaacaaccagctgaagcgcgtggccgatagcctcggcgggaacaacaagcagcgtcgcaagctgcgctcccgcatgaagcgtcgtgctgccgagctgcgttccggtgcatcgttgcagcccaacgtgcagtccgcactggcaggtgcagcatgagcctgcgcatgggaagctgggtcgaggtgactgtgcccgacagccgactgctcaacgtgcagccggagattgccgccgccgtgaagctgatcggcggtgcgaccatgaccaatggccgtggcctgtacgtccgcaaggacaccggcgcactggacgacgaggcggtgaccgtgatccgcttcgacctgaacttgcacagcgagctggtggaccagtacatgagcgccatccgcgccatcgtggaccgtctgctggtgctgggtgaggagagcgtgctgcgtcgccgcttctacaatggcggcggtgggtacaacagcgagctgatctttcagtaacccgagccgggtaggctacgactggcccacgtacgggccatcctatcaaccgtcaagaggaaccatctacatgtcgaacgaaaacaccaccgagcagaccaccgtcagccactacgaagccaagcgcgccgagctgctggaagacatcgccaaggcgcaggccaaggtcgatggcctgaacgagaagctcgccaagctggatgccgtcgaggccaacagcgccgccatcgaagcgctgaaggcgggcgacgccgtgtcctacctgttcggtcgtgccctgaacaagcgcgtcctgtccggcgtgatcgtcgccaccggcaagaacgacaagggcgtgctgcaactgaaggtgcagaccggcgaaggtctggatgccgagctgaacctgatcgacagcagcgccctgctgatgtcggccgaggaagtgctgaaggcgcaggaagaaatcgacgccgccgttgccgaggcccagcgcctcgccgccgaagccgctgccgccaaggctgcgggtggcgaaggcgggcagtcgtgagcctcgccccgccgtcacccagcgtggccgtcgtcaagcgtggcgacgagctgaagcccggccagaatgcgtacctgatcgacacgcggcagaccaacaagctgccgaagggcaccgggttcgtcgtgtccaagctgaccagtgaagacggctcccgtctgatcgtcagcacggacggcaacggctccgtcctgtacgccaccagccacgacatcttcgaggtctgggaataaccaagcgaggatagcatgagcgatacccttcccgacaacgactggctaccacatgccgagcgcctgcctgttggtggccgcacacgtgtggcccatgagtgcggggagggtacgcccttgcttatctcacgagagcacgacaagtccaccgcattctgtttcaggtgcggtggcacaggattcaagcgtgagcacgagagtatcgaggccaagcttgcacgaatccacgccgagcagacgagcgaacgcagagtgcgtgcgactgttgagttgccagagccacgggtatacgacacccgcgagtggccgctcgacgctaaggtgtggttcttcaagatgggactctcgcttcagatgatcgagaagctgcggctgtactggtgcccaagcatcgggcgggtggtactaccgatcactgaaggcgacaacgtggtatactggacagcccggtcggcaacgagacagccgaagtggctaacacctgacgttccgaaagacggacttgtcgcacgctacggcgtgggcacaggtgacaccatcgtactgtgcgaagacccgctcagtgcatacaaggtgggactggtaaccgaagcgtggtcgttgctcggcaccaagctgcacaacaaagtgttgaagcagctgactgatcgaggccaacgtgtagcgacgtggctcgatgacgacagaggtagaagcaacggtagcaatcccggccaagacagtgcgcgagtaatcgctgcgcgtctacgtgcgtttggtctggactacaggaacatcacgtcaccacgtgacccgaagtattacacgaccgactacatcaaggagaagctgcaatgagcaaacccatcgtgcgctaccggcgcgctatcatcccgcccgtcgttggcttccgtgccacgctcggcggcgtgcttgcgcatccgaacctcggcgactgcgacatcgtgcacacctcgacggtgctgtatgtggcggacggcgggcgcaagttcgagacgcgcaacacccggtatcaccagctcgattccaagtacgaacccgaaggagaacctgatgagtcttgacaccacgctgctgcggttgtgcaccaaccgtggcaagttcgaccggctggtacccagcgcaccacgtgatgggctggacgagctgaccgtgctgatgctcgatgcgttgcgtgcgtactacaaggagttcccggacacgaaggacttgccgttcgatgtgttcgatggctgggccatggagttcaagtggaagacgcagcccgacgacaagaagtccctgctcaaagttctgctgaagcagatgcgcgagccggtcccgcccgaggcagagcagggcatgatcgagaagctgttggagttggagcttgccaccactgcggtcagcaagatcgtgcagtggaatggcggcgctgagttcagcctgcgcgacgagctgtacggcttggccgagacgatcaccgaccgaatggatcgcaaggcgcggctcccgctggtgcaggagacgcccgaggaactgatgcagatggacgagcacgacatcggcatccacttccgactgcccacgttggcgaagaacctgcgcgctctgcgtggtggtgacttcggcatctacgccatgcgtcccgacgcaggcaagaccacgttcctgaccagcgagtccagccactggatcacgcagctcgacaacgtttggccggaccagaagcgcaccggcatctggctcaacaacgaggggccgggcaagcgcatcaagcagcggtggtatcagtcgctgctcggcgctaccatccctgagatggtggagtgggcgaaggatggtagcatccgcaagcgcatcgaagatgcgatgggcggggacatccaccgcatgcagttctacgacatccacgggttcaactccggtgaagtcgaggccatcatcaagcagaccaaccccggcttcatcatcttcgacatgatcgacaacatcacgttcaccggtggcatgaccaacggcgggcagcgtaccgatcagatgttggaggcgatgtatcaggccgctcgcaactggtgtgtgaagtacgacgccgtgggcgtggcgacttcgcagatcagcgccgagggtgagggaatccagtacccgccgcagtccgcactgaaggacagcaagaccggcaagcagggtgcgtgcgacttcatcatcatgggcggcaagctcaatgacccagcgatggaacgcttccgctacatcggcaccccgaagaacaagctgcaccgcgcaggcggcaagcgtgacgttcgggaagaagtgatgatggatgcagagcgtgcccgcttctatcaggaggcagcatgagcaagccaattcacatcgtagccaccgggttcacggtgtcggtcagcttccccggtgaatccaccgaggcgaagaccttcaactgcgtgagcaacgcgcaagcaatccaccttgccaagctgctgcgcaaggtgcacgacgcaggctacatcgaaggccgcaacgacgcgccgcagtggaagtggggatggctgcggaacaaacacagcacttggatcggcgtgcactactcgccgcacaacaagcgctggtgcatcaatctgatcccgtgcttcacgttctggatcaccaagcccggaggtaacacaccgtgagtaccgaaccgaacatctacctgccgcgcaacgtgggcgtcatcacgtccagccgcaccggcagcagctacacagtcgagccgcccgtgaccgacacggacatcgacttcctcgtgctggtgcaggacttccacgaggccatcgaaaagctggtcgatcagggatggaccctgtgctccggtgccgatggacactacgaggaggacgaggactacagcaccacgtggtatgcgctgcgcaacggcgtgttcaacgtcatggtgaccgccgactccggctggtatcagcgcgcggtcgaggccaccaccatctgcaagcgccgcaacatcaaggacaagcaggaccgcatcatcgtgttccgttgggtgcgcgacgggctggacttggatggcgatgcgtcggatgaaatgtaccagctggccctgcaacggtggccgctgtgagcttcacttccttcgacctcgaaaccacgatccgttccatcctgaagcgcaaggccaatccgttctacgacatgaacaagatcgtggcgattggctacaagcggaagggtgacgcacggaacaccggcctgtactacgacacccgagtcgggatagacaaccagtacatgggcggcgcacccgatgggtggctgcgtgagctgtgttacgggcagcagttcctcgtcgggttcaacatcaagttcgacatcctgcacgccatctgccaaggcccactcaaccggcaggcatggatcgagttcatcgacggcggcggcatggtgtgggactgccagcttgcggagtacctgctgcacggcatgacgcaagagttccacatggcgagcatggacgagacggctccacgctacggcggcaacttgaaggacgatgcagtcaagtccctgtgggctgcgggcgtggacacctgcgacatcgacaagacgctgctgatggattacctcctcggcaccaacgacaccgacgacgtgggcgacatcggtaacaccgagaagatgttcctcggacagctcgccgccttccgtgcacgtggtggtctgcgctcggcgctcctcaacatgggtgcgctgtgcttcaccatcgaagccgagtacaacggcatgtacgtggacaaggactgggcgcttacgaaggcgaaggagttggaggtcgagcttgcaacggcgaccgccgaactcaacggcttcatccccgagctgcccgagggcctgaccttcaactggaacagccgcttccacaagagcgcgctgatcttcggcggcaaggtgaagtacacggccaaggttccgatcatgtccaccgagggtgggccgacttacgtgcagaaggacgaggtgcactacgtgctggtcgatggtaccacgacggcgacgccaccggccgaggacttcgacaacctctggcgctacaccacgtacggcagcggcaagaacaagggagagtacaagaccaagaaggtgaaggtcgatgacttgaccaagcagaagttccgcaacgaggacatgctgttcgagttccctggctacaccgagcctgatgctgcatgggaaagcaagagcgatcccggcgtgtactccaccgctgccgacgtgatcgaggcgctgggctaccgcaacctgccgttcaccaaggcgcttgccagacgcgacgacatccacaaggacttgtccacgtactacatcacgacggacgagaagaccggagagcagaagggcatgctcacgctggtgggaccggacggcatcatccaccacaagctcaacatgaccaacacggttaccggccgcttgtcttccagcgatccgaacttgcagaacgtgagcaagggcgagctggacgaggagacgttggaggagaagggttcgcagatcaagcgcgccttcgtgtcccggcaccggggtggcaagatcatccagtcggactacacctccctcgaaatctacgtgcaggcaatcctcaccgagtgccgtcagctgatcgaggacttgaagcagggcctcgacatgcactgcctccgtgcagagcaggcgtggggtgagcaaggcaagtacgactacgacttcatcctgaaggcgagcaaggacgacaagcatcccgagcacaagaagtggaagaagaagcgcggcaacgcgaaggtgttctccttccagcgtgcgtacggtgcgggcgtggcgaagatcgctgcgaccaccggcatgtcggaggaagaagtcgaggcgctggtgcgcggtgaggccgagcgttacccggagctgggcgagtacatcgaccgcatggtcgagcacatcaagcgcaaccgcgtcagcactcagcgcttcgttccgcatcccaacgcggggcagcaaggcgtgccgcatgggctgacgtgtcagcttggccggtcgcactggaccacgccggacggcaagatgtattccttcagcgagtcaccgtccccggtgttcatcgccaacaagcccgcgagcaagggtggctgtgcgcagtcgttctcgcccacggaaatcaagaactacccgatgcaaggcaccggtggtgaatgggccaaggcggcgatgtacgtcagcctgcgcgccttctaccggaagtacgtgaccgaaccgaaggaatggttgggccgtgcgttgctcgtgaatcaggtgcacgatgccgtctacgtggatgcacacggcgacatcgcaaccaaggccgctgctctgctgcacgcctcgatgctggaagcgtcggtgtatatggagtggtggttcaactggacgctgccgcttggcgtcccgtgtgaaaccaagatgggcgacaacatgatggaggagaagaaccctcccgcagagttcgccggtctggtcatcgagtaccgcgcgtcgatccgcaaggacttcgtaggtaatcacaacccgtcgtttgaataaggagaacaacacgcatgagtcttgacgcactgttgaacaaggtcgccacgcagggtaaggatcagtcggtcgccagtggtggcagcttcgactacaccccgcccgctgccggtgtgaccaccgcccgcatcgtcgggtactacgagctgggcaagcacgagttcgagttcgagggcaagaagaagacgcaggatgaagtcgccatcgtgttcgagctgaccggtaagcagcacccgcacatcgaaaccgacaatggtccggtgccggtgcgcatgacgctgaccctcggcctgtccaccaacgagaaggcgcactacttcaaaatcttcagccgcctgcgcaccgaggagcgccacttcgtgcagctgctgggtcagggtgtgctgctggaagtcatccacaagccgggcaagcgcgacccgaacaagaccttcgccgaaatcgacaaggcttccatccgcaagccggtcatgccggtgccggaaatggagaacggcatcccgaccggcaagttcgtggacaccgtgatcccggtgccgcagcagatcaccccgctgggtgcgttcgtgtgggacttcgccgacgccgacatgtgggacagcatctacatccccggcgagtacccggagcgcaaggacgagaagaccggcaaggtcacccacgaggcgcagtcgaagaacaagacgcagctgcgcatcgctgcggcgctgaacttcaagggtcttccgtgctacgactacgccgccgccaagttggcgggcagcaccacggtcaccaaggaaggcgtcgatgcgctggacgaagtggtcggcgacgtggcgaacgccgcgcccaccgacgctgctccggccgacgacaagccgccgttcccggtggacggtagcgacccgatggcaggcatcgcctgatggacctgagcgctctcatggcagcggccggtgagcgctccccgatgccggtgcaggtggtacgtcagcacaacccgcgcgtgatcgctcacgttgatggggactacatggcgtacttcgcggctggtagcgagaactgctcggcgggggatgcacgacgcaacgtgctctcccgctgcgcacagctgaagcatgtcagcggagcgggcaagatcgtcatgcacctgacgcacgccgcgtctaccaagggtgatcgcttcctcgctgctaccacgcagccgtatcagggtcagcgccaagcaggccgcaagcccaacaactgggcgttccttcgtgagtggatggagacatacgagggcgacgctttcactcccaaaatctggctgacccgtgaggccgacgatggcatcgcgtacgtcaacgagggtgcagcattgcaccacaacatcctgcacgtggtgcacagcgccgacaaggacatgcgaatgttctgcggcgtgcacgtagactgggacggctacgacatcacagaggttccgctcggcgcttacgacatcgttggcgagaacggattgcagtacggtcacaagtggttctggatgcagatgctccacggcgacaccgccgacaacataccgggtctgccgaaggtgggcaaggtgacagcggagcagctgctgttcgagacgaagaccaacctcgaagcggtgcagatcgtgagcggcaagtacagcgaagtgttgggtgccgactggcgcaagacattcgccgagcaagccgtgctgctgtggatgcggacggatcgtgacgcagaactgctcgacgtgctgaagctcgacgtgttcgggccgaagctgaagcaggcgttctatgacctcgccgaggacgtgaacgagaagcgtgcaatcttggaggcatacaaagcatgaagcgactcactgcaacacaggtcaagctgctgcgcatcaagctcgcagcggagcaaggcaaccggtgctgtctctgtcagggacagttcggcctgaaggctccgctcgatccggtgctggaccatgaccacaagaccggcgctgtgcgcggggtgctccatcgcggatgcaactccctgctcggcaaggtcgagaacaacgcaggccggtacggcgtgcgcgacgtgttcgcattctgtgcgggcatccccaactacctgcggtcgcacctcaccaacatcacggggtacctgcatcctacctacaagaccgacgacgagaagcgtatcgctcgcaatgcgaaagcgcgaaagcgtcgggctatcaacaaggagacaccgtgacccttacccagttcattcgccgagcaccgaagcgcggcccgaagattctctgcctcgacatcgagacgttccccatcgagttctatggctggggcatgttcaacaacaacttcagcgtcaagcagatcaagcgtgactggtcgctgatgtcgttcgcttgcgaatggctggacgacgaggcgtcgttctacatggaccagcgcaacgtgcgcgacgtgttcgatgatcgcaagcagggcaaggcgctgtgggcactgctcaacgccgccgacttcgtgctcgctcgcaacggcaagaagttcgaccttcgcaagatcaaggctcgcctcgcaatcctcggcctgccgcccgtgtctccggtgcaggtgatcgacccgatgctgctgaaccgcaccgagttcgccttcacctcgcagaagttggagtacaccaccggcgtgatcgtgccggagctgcgcaagtacgaccaccacaacttccccggcttcgacctgtgggtggcctgcatgcagagcctgcccggagcatgggacgagtgcgaagcgtacaaccgcatcgacgtgaagtccatgaagttggagtacaagaagctgcgcggttggtactcgcagcatccgaacgtcgcagtgtactacaaggccgacggcagcgagcaccgctgcaacaagtgcggctgcaacgaaatgatcccgcaggatgatccggcccgcacgcaggtcggtacctacctcctgcttcagtgcaccgtgtgcgacggctacagccgtgggcgcaagctcacgaccagcgccgaggcgcgcaagcacatcaccgtcccggcataaggaaccgacatgaagatcaccgacatccgcagcggcatgcgggtacagtacatcggcaatgcgcccgcaatgatcgggctgcgtggacaggtaagccgcgtgttcgctcgtgatgtcgaggtcttcttcgacggtcgagttaagccgagctgctgcgttcccgattccctccgacagcttctcagcatcggaggcgtgaccaccaccagacgagaggtaccaatgcccgaactgagctaccgcgacgaggaccgtcgcacactgtccgaccgtggcgtcggcctgaaggatgacgggggcaagccgcaggcccgtctgctgcatgagggcgtgccgcgtgcactggcccgagtcatcgacaccctgaccttcggcgcgcagaagtacaaagcgcactcgtggcagcatgtcgagaaggcgctcgaacggtatcaggacgcgagctaccgacacgacaacaagcgctgcctcggcgagaagctggacccggagacgggcatccaccaccgggcgcaccacatcatcaacgagctgttcctgttggagctggaactgcgcgaggaggagaaggccagtggcgcagagtaaggcgcgctccatcaaagaggcttgggtgaacatcggcatcggctacagcatcaactacgcagcgaacatcgcgctgcttccggtgctgtggcatcccgagcatccgctgctgtcggcgcacgccatcggcattgcgttcacagcgatcagcttcatccgccagtacatcatccgccgctggttcagcaagggtgactgatggcctgcgcccgctgcggccaagtgcatcggtacgtcccacatgaggccgagtgggcgcgcttcctagaggagcaccgtacccgcaagcagttcgatgtcgagtgggccaactcactctggcatcgtacataccctgacgacgcattctgcatcctcgtgatgaggggcctcgcaggtttcgttccattcccgtcgaaggagaactgaatgctctacaagaaccagaccgccatgctcatcaagtcctacgagaacgccgttgcgtggggcgagagtgccgaccacgaggaggcattgcagaatgcggtcaaggccgggttcccgaacctgcccgacgaagatcaggccgagctgtatacccgcatcgccgatgcgtgggaaggctaccgtggttcgctcgctccgcgcaagctgtggatcggcaccatcgtcaaccagttcatgtcgtcccgcatcgcacggttcaacgccgcgctgggtgacggcaccaagaaggaggacagcgccgatgtttgatgtgcctcgccagaatgtccgggttgctcccggctacaagaagcgcaagcgcggcttcaagatcaaccgcgccttcaccaagggcaacttccgcgtgcagtggtacgacggcaaggccacgtactgggagcgctacgttccgtggtacgaagtgccgctcgccatgttccagatttggagggactacgcatgagctacatcgtccacaaggcagtcgagcaggacaagatcaagaagaagctgcggcccaccgaggagcagcttcgcaccgagtacatcgcacagccgaagtacgacggctgcaacatggtcgccatcaagcgcggccactgggtgcccacggtgaacaagggcctgcatgccatcaaggtgggcgacgtgcagatgcagccggtggatcgtggcgtggttgacctgttctcccgcaccggtgagcaggtcgtcagcgcacaccacatcgagaacgctctcgcatccgcgccgttcttcccggtcggcgtgtacttcggcgaatactggcacccgcagatcgaccagcccaccgtcagcggcatgttccgcaagaaggacggcacgcagtacaccgagccgatgttcgtggtgttcgacttcgtgacgctggaagaatgggagcagggtttcagcgacctcgtgtatcaggagcgcgtcagccgcctgccgagcatgggccacgccatcgccgagggcaccgcgccggtgttctacgccgagtcgcagggcttcctgatcgaccaagagctgggcagcatggaagcggcgaagctgctgtgcgagggcggcgcgtacgacgggctgatcctgcgcaagccgagcggcaagtgggtgaagggcgacaagggaaccaacggcgaagtcgtcaagatcaagccgaccctgacgctggacctgcgtgtgctcggcatcaacgaagcagtcggcgagaagaccggccgcgccgtgtacacggtcgtcgttgacctcggagaaggcaagacgcaggaggttggcagcggcgtgccgcacagcgagagcgagctgcctagcgtgggaggcatcgtggaaatcgaggcgatgtccttcagcaagtacggcctgctgcgcgagccgcgatacaagggcatccgtcacgacaagaaggaggcagacctgtgagcgtcgaggtgcaagcatggcacaacatggagcgcgacacggtggagctgcgcatcagcgttcctttcggcgagtacgccggttccctgtggccgaacgagacgctgcgcgacaaggtgcaggaagcgttcgccaagttccttgacgagcggaggggctgatggacgcgatcactttcgagaagccggagctggacttcagccagtcctcggcatggatgggccgcgtcgaggtttcggtgcgcgcccggtacggtgccgacttgttcggcgctgctgccacgtgcatggccgaggatatcggcggtgaggcgtggccgcacatcatccacgacctgcacatggaaatcatgcgcggtatcctgaaacgctacccgccgcgcgactacaccgtgcggcagcaacggaggtaacaatgctctcgcaagtggaactcgaactggaaacctacgccttcggtaaggagcgcatggagaagtccatcgcccgcaacgaggagaagggcggcgcggacaacaacccctacgcccaagcagtgtatcgccggttcgtgcttccgcttgcggagcgcatccgtgcggacatcgactctccgcgaatcggccgtgcgcaagcgcacgtgccacttctgcgcgccaagtacgatcccgagcgtcagaacaagcgtggacagcccgtcagcgccgaggaacaggcacgcgagtggtacgaggctgtggccttcgtcgccgttcgcggtgcccttacctcctgcatgcgagacaagcacggcgaaggcagcgaccgcgacgtgttgaagaacgttggcatcaacgtgtaccatgagtacctgctgacgcagttcgccgacgcggagccgactctgttctaccacctgatgaacgacatggaccgcaagctctctgtcaacgagaaccaccgcatgacggtgatgaagatgcaaggacgcaagaacggcatcgagttcgtggagtggggacaggcacagcgcgatcaggtcggcgcgtacctgtgcgatcagcttgcgcagctgggcatgttggagattggcgtggtcaccgagactgctgccagtgcaggcgcagcgtaccgcaagttccagaccaagacgcacgtcaagatcgtgctgaccgacgaggtgcgcaagctgattactcagatcagcgacttcgtgatcgaggccacgccgttctacctgccgtgcgtcgagccgccgatggactgggtggacatcgacaacggtggattccacacgaaggaaatgcgccgactcaatccgtggatggtgaagacctacgctcagacccgcgacgagtaccgcgctgccgagctgcgcaacgagatggctgcgatcaacgcattgcagcgcgtgccgtggcgcatcaacaagcgactgatggaagctgtgtcggccatcgccaaggtgcacgacatggaggaaatcatttctcagggcgagctgccgaagccgcgcaagccggagtggctgacgaaggacatgaccaaggaaaccatgtcccacaatcaggagttggagttcaagcagtggaagcgcgacatgtccaactggcacaccgacgagcgcctgcgacagaacaagggcaatcgtttctacaacgcaatgaaggtggcgcgcaagttcgccgagtacccgagcatctacttcgtgtacttcgctgacttccgtggccgcaagtacgttcagaccaccggcgtgtcgccgcagggttcggacttgcagaaggcgctcttggagttcgccgatggcaagccgctgctgactaaggacgcgaaggattggttctgcatcacaggagcaaaccgatggggatacgacaaggcgtctctgccggatcgtgtgaagtgggtagcggagcatcacgaccagatcatggcgttcgctgcggacccggtgaacaacgacgagtggaagaccgccgacaagccgctgcaatttctgagctggtgcatggagtacgagcagtggcaagtgttcggggatcgcttcctgagccgcatcgcagtcggcatggacggttcgtgcaatgggcttcagaacttctcggcgatgctgcgcgacgcagcaggcggcgtggcgacgaacctgatcccagcaccgctgccgaatgacatctaccagatggtggcagaccgcgtgactgccgtcctgctaggcgaggacgaggatgccgaagggtaccgcacgctgtggctcgaccacggcctcacacgctcgctggtgaagcgcagcgtgatgaccctgccgtacggctcgcggcagtcctcgtgggcggacttcatcatcgaagactacctgaagtgtgggaagttcccctcgctcgacaaggccctgtacggccccgcagcgcgcttcctgagcaagcgcatgggtgaggccatcgccgacaccgtggtcgccgcagcgggcgcgatggagtggttgcagcgcggctccgggtcgatcctcaaccaagggtacgaccgcatccggtggatcacgccgtccgggttcccggtggtgcaggtctactgggagtccgaggagcaccgcatcaacaccaagctgtgcggcaacgccaagctgtccctgcgcaagagcacggacgcggtgaagaagtcccggcaccgcaacggcatcgccccgaacttcgtgcacagcctcgacgcaagccacctgacgctggtggtcaacgcggccaaggccgaaggcatcgacgccttcgccatgattcacgacgacttcggcacccacgccgccgacagcgcggcactgtaccggatcatccgggaggtgttcgtgtcgatgtacgagcggcacgacgtgctgtcggccttccactcggcctacccgttcctgccggagccgccgccgatgggcgagctggaccttcggcaagtccttgattctccgtacttcttcagctgacggagtttcagtacacctatagcacgaggcaactgaggtccggttggagcggccgcgaaggtaagcggaaccggtgccggaccttttggtacacctatagcacagaggagacaccatggccgaagacgccaaagtgaaagtcctgatgacgctccacccgaaccagctggccgccgtgcggaagctgtccgggctgtcgctgtccgtcaactcgaataccacgcccttggaggcaggtatgcagttggggatggcccgcgtcctgaacatcttacaggagggtttcaccgttgattcctccgtaccgaacaccaacgacgggtgatagtgagcagatcaaggcggctttaacggccgctttgtatctgtcatctagagaagatagtaaggtagacaacagagaatcttctgtgagctacaactgtgatgaccctgattacacagtggccctgataacacagggtctagtggatgcagtaatcattgatgaagcctacctgctgtgctttgccattgtcacaccgtggtactccaagaaccgtactacgttcgttgagaacatggtgctgcgaattgggccgggcagttccttcgaccggtacatagccgtgatggaacatctggctgacatcaaccactgcgactcactgagcgcaggcggtgcactagctcggaactcccgagcactcacacggatgtatgcacgctacggctacctgctggaacggcatgctccccaattcaccaagcgaaggagttaacctatgggtagcatcgttggtggtgggtccgccaagcgagcagcgctgaagcaagctgctgctatcgacaagcagaccaacctccaaactcaatccacgaactaccagattcaggcgatggccgatcagatggcacaggcagctgcacagcaggccgcatctgagtacgccgagaagttgctgagtgcccccgtcgataccgtcgatgtgcggctgggaacttccgacctcgacttgcagactgccgacctgatcggccgacgcaagaccgcccgctccacttacacccgacccgtgaccacgaccgcagcttcccggctgacgaccgtggccgggtcagacctgttgtgaggtgagcatggaccatccgatccaaaccgctcaccgccagttcgaggcttacgacaacaagcgacagggcatcatgtaccgactcgaacgctattcgagctggaccgtgcccaagctgttccctcgcaagaaccgcgatcaggacaccgagccgctgacccacgggttccagtctctcggcgcgcaggcagtgaaccatctggcgaacaagctgatgatgtcgctgttcgcaccgtcccgcccgttcttccggttggagctgaagcgcaaggcgaagcaggctgcgcaggagcaaggcgctgacttgcaggccatgcaggcgatgcttgcgaaggccgagcaggatgccagtctcgaactggacaagcgctccatccgctcccggctgtacgacctgctgaagatgctgatcgtgctgggcaacgccctcatggtgttggagaaggacacgatccgcgtgctcaacatgcggcactacgtggtcaagcgcacccgcaccggcgaggtctacgaactgatccttcgggagaaggtgcacaagacccagctggaacccgcagcgctcgctgccattgtcgcgcacccggacttcaagcccgatgacgacggcatggtgtgggagtacaagtgggtcaagctggaccacaagaccggcaagtacaacgaagacgtgtggatttgcaactgcaagctgcccgccaacttctcctcgacctacaccgcagacaagctgccctaccgggcggttagctgggacttggccgcaggcgatgactacggctccggcttggtcgaagactacgaggccgacttccagtcgctctcgatgctgtccgaggccgcagtgcagggcgcgatcctcgcctccgagttccggtggctggttaaccccgcaggtcagacctccgtcgaggacttcatggcgtcgcccaatggcgcggccattcccggcatgaagggtgacatcgagctgattaacgcaggcgtcgatggcgtgctgcaaaccaaccaagcaatccagtccacctacatcaaccgcatcggcgcaggcttcctgttgcagacggcggtgactcgtcaggcggaacgtgtgaccgcgcaggaaatccgcatggtcgccgaagaactggaaggcgggctgggtggcggctactcccggatcgctgcggacgtgcaggtaccagtcgccttttgggtgatgaacctgacgggccgcgacatccgaggcaaggacttggagcctgtcatcatcaccggcttggccgcgctctcccgtacgggtgaccgtgaccggctgttggagttcggcagcaacctcgccaacgtcctcgcactgccgccgcagattctcgaacgactgaagctgtccgcgtggatcgcagacctcgccgccgctggtggcttggacccgaacgtctacgtgctgactgaggccgagtacggccagatgatgcagcagcgtgcacagcagcagctcgccatgcagaacgcatcccagcagatcgacaacgccaacaacatggagacacagacacaatgagttccaacgcacctccgggcggtggtcccggcgcaaccgtgatcgcaacctcgaacggcaaccagcccgcaccggcagctccggctcccgcagacgacaagctgttgcccaacggccagcccgctccggccgcaccggcacagcccgcagctcctgctgcacctccggctgctgacgcgctgagtctcgaacctgccgctcccgcacagcccgccgccccggcgaacgctgcgccgactgcggtgtcgatcccggactacggcgacaacggcctgaacatcgcggccgaatacttcgtcaacaccgtgggcctcgacatcgacagccgcgaactgaccgaagcagcgaagggcaacttcgccctgctggaagccaagctggaagtcctcggcgacaaggccaagggttccgcaccgatcctcgctctggcgaaggagagcatcgctcgtgtcaccgccgctgcaaccgcagcgcacgccgcgaacgttgctgctgtccacgaagccgtgggtggcgcagagaactgggctgcgatccagcagttcgcacgggccaacctgcccgccgaccaactgaagcaggcaagcgaatcgctgtcggctggtggcttcggcgctcaggcgaccgcgcgttacctgatggctctggcacaggccaatcccgcgacgaccgtcaagggcgcaccggctaccaacgccgccgcccccgccgcgtcgatcaacggcgtcgctcctatcacgaaggagcagtaccgcgctgagtaccgcaagctggttgccgagaagggcatccgtggtgcggcccactccgaagaactgcgtgcactcaacgcgcgcgtcatccactaagaccaaggagcaacacaaagcatgagcaccatcttcccgactgtcccggttctgccgaatcaggtcaaccagtccggcaacgagaacgccctgatcctcgaacagttcaccggcgatgtcgagcacacctacgtgtccagctcggtgctggaaaagttcttcccgcgcaagcaggtcaagggcaccaacaccctgaccaagaaggccatcggccgtaccaagcttcagaagctgaagcgcggtgacgcgccggacggcaccccggtggacttcagcaaggcgtcggtgaccgtcgataccatgctgctgtcgcgtcacagcatctggcagctggacgaaatcttcaccgacatcgacacccgcaaggaaatcgccatcgagcagggtcaggaaatcgccgagttcgtggacctgaccatcagcatcgccgccgcgaaggccgctgctgccacgcagtcgatcttcacccgcaacggccgcgcgcccgagggccacttcggtgccacgcaggtcgtgctgtccgccgctggtgacgagaacgatccggccaaggtgtacgccgccatcggcaaactgttctcccgcatggaggaggagaagaaggtcaagccgcagcgcgatggcgtggtcctgatcgtgcgcccggcgatcttctacctgttgcagcaggccgagcagatcagcaacggcgagtacctgacctcggacggcaacaagctgaccggcatcccgaccttccacggctggggcgtcccggtgctgtcgagcgagaacctgccgaacaccgtgatcgaaggtcacctgctgtcgaacgacgacaacgacgacttctacgacggcgacttcagcaccctgatcgccgtggccgtgtcgccgaaggccctgctgatcgccgaagcgctgccgttgcagtcctcggtgtggtggagcgatgcctcgaagtgctacttcgtggactcgtggatgtccttcgccgttggtctggatcgcgtcgagaacgcgggccgcatcgacaaggttgcctaatccgctgggcgcggtccctgaatccttcgggtaactcaaaccgcgcccttcttccaccaacacaggagcaacatcatggtctttgaccgaccgttcgagatttccaaccgcgtcgtcgccgcaactggcgtggccggtctgcccgccaactccgttggtaccgtcgtcggcgtccactacgacacccgtggcaccgcaggctgggtcgtccgtgtccgtttcgtggacgacgaaatcggctcgcaggacatcgagtacgcaccggccgctctggctctggctgcggactaagcaacatcccggcaggggcgctccggcgtctctgccttgttcctctcaggagacaccatggcattcatcaccaagctcgacatcgtgaacgcctgcttgaagacgatgggcgagacgaagctcaacacgctggaagatgaccacgtatacaaggacgacgccgttgacttgatcgaccgcgtgcaccgtgacgtgtcctcactctcgctgtggttcaacaccgaatgggtggagctgaagccgcaggcaacgagcaagtacatcatggtccccacggacgtgctgaagctggactgcaacccgagccggttcggccacgtggtgcagcgcggacgccgactgtacgaccgcaagcgcaacacctacgagttcgaccacaacgtgcaggccaagctggtgcggctgctggacttcgatgacctcccctacgaggtgcagatgttcgtgcgcgacgactcggtgctgcggttccagtctgacttcgacggcgacaacaccaagtacgccaagatcaagcagcagcgcgatgacagttacatcaacttgaaggccgagcacatccgccagatcaaggcgaacccgctgttcgctcgcgcatccgtggacgtgctgcgttcccgttactggaactacagcggtcacccgtggcacagccacgtcacattccccggctaaggagacaacatggcaaaggcaggcggaacctatcccgacatccttcagggtgtcagtcagaaaccggcgcatcgtcgtcggccgggacagacgcacgagcagatcaacgtgctgtccgatccggtgaacggcctcgtgcgccgtcgtggtacgcggttcgctgcttcccaagccgttgtcacctcggccgagctgcgcaacatggacgtgttcgacttcatgcaggagggcaaggagtacgcgctgctgtaccggcgcgacgcctcgaccttgggcagcgagtccttcgcgttcctctacaacaagacggacgagtcgttcatccctctggtgtacgagaacagcacgtgggtcaacacgctggtcagcggaggcgcatcgtcgctcacggccatcggcagctacgtctacatcgcgggcaacaccacgatcccctcggccaccagcacgaacgtgtggcaggagcagacgaacatccagcgcctcgcagcatgggtgcgcaccgggaagtacaacaccacgtacacggtgaacctgacgcggacggacaacacggtgctgacggtaacgttcaagacggttaccgcatcgtaccccggaacgctcgacaccagcgacatcccgttctaccttcccggtggcacggagccggacgcggcgtaccagaagtacgtcaacgaccgagtgaacgagtacaactctgcggtcaacgagtggatcgtgacgagcgctgagcagacgcgcccggagtacatcgcggagcagctgtcggatttgctggtcgatgcaggcgtgtcggcaacgtacatcaagggcgggatcatcattgacgatgaccagttcaaggacatcacggttgacgacgagggagacggcacgaccttctacgccgcagggcaggaaattacagacgcgacctacgccgtcaagttccactggcacggcaaggtcattcgcgtgcggccgagtggtgcaggcgcggacgagtcgtactacctgcgcgctgagttggagaacggcgagacttccggctacgggtcggtggactggtacgaagcgcccggcgtggagtgcaccatcgacaacctcgtgtcgcagctctacatctacaacggtgtaggctacatcgcacgcaacggtgcgggcctcacgtctctggctccgagcagcggcgagcatccggcctacggtgcgcgagtggcaggcgatggtctgacctcgccgatcccgtggttcatcgacaagccgatcacgatgctgtccgtcttccaagaccggctggtcatcggcgcacagaactacgtcaacgcctcacgctcggcggactacctgaacttctggcgcggctcggccgtcaccatcgaagacagcgaccccatcgaaatcttcgcgcacggcagcgagggcgatgtgctccggcacgcgacgctctacaacggcaacctcgtgatcttcggtgaccgtcagcagtacggcatcagcggcgactcggtgttcagtccgaagaatccgctgattaaagcgttcagtgccaacaaggattcggttgacgcgaaggcgcagacctcgggcaactacatcttttatgcgcagtacggcagcgaaggcacgagcctgcaccagatgcgagtgggcgcgctcaacgggcagcagacggtgacggacgaaatgtccaacgagctggactcgtggctgtcgggcactccgttgcagatcaccccgctcactgcgccgaacctcgtcatgttccgcactcgcgagcacccgcaggacttctacctgtaccggtacgaggacaacaagaacaacgggcagcgcatcgtggatgcgtggtcgaagttccggtaccacccggcgctgggcgaaatcatcggcgtgagcagctacaagaagaacggcctcgtgttcactgcgcgcgggtcgctggtggcgtgcgacgtgttcgacccgaagggcgagccggactcgcatgcgtgcctcgacagctgggcgagttttggtacacctacgggcgtacagactgcgagcgcaagcatcgccgtcaatagcactagcccgtacttcctgctgggttgtccctacgcgcaggcgtctgacttccttaaccagttcgatgacctcgctgctggtgcgctggaatacggcgtggtgtccgaagctctggtgatcccgaccaatccgttccctcgggaccagaacggtcaggccgtactcgatggacgcatgtccctcaacaaggtgacggtggacgtggagaacacggcaggcatgatcgccacggtggcaacccgcaacagcaatgtgaccactacggacttcgagggccgcatcctcggcgactccgacaatctgatcgcgcggcaaccggtgtaccgggggcagctcaacatcagcgtcgggcgcgaagtgcgcgagtgcacctacgagattcgcagcaaggattggctcccgctccgggtgaccggcctgagctggacgggtcagactttcaacaatgtacggagggttagctaatgggttcggttaatacgatcctgcaagcgaacaacaccacccgcgttgcccgtgcgaactaccgtgcagccgttgcgcagaccgacaaccagaaccgcagcgaggtcgccaagaccggcttcgctgatttcatgcggtccctgaagaacaacgcccaactggacgccgccgcgaaggagtacaactccaacatggaagcgctgtccgaggagctgcgtgcgcgccaaggggctgggcttaactcccagctccaactggcgaacgcgcgtggcgcacttcaggcgcaggctggtgctgtcggtgtcggcggctcgtccgcagacctgatggattcgatggtgcggttgcaggcggaaatggatcaggagacgcaggccaacgctgtctcgctcctcgcctcgcggggcgcatcgcagactgcgcagatcatgtcgcgcgcgtggaacgggatggacatgagccgttcgttcgggcagttcgactactcgcagcacatcgagccgcaggcaatgaagcgtcgcttgggcaagctgatcggcgtggccgtggctacctacttcggtgggccgatggcaggcgaggccgtggcagacttcgcggtcggcacgtggcaggcggacaacggcaacttcactggtgcctctcagtccttcagcaacgcagcgcagaacggtatgcaggcgtggcagcagtccaatgatcgcggcggcaagtcgtgggcgtccactaccttcgggtacaacgacggcaccggcaagcagtccgtgactggggcgaaggtcaccggcaacttcggcaacaactacgacaacttctccaccactacgtccggcctcggctggttcgatagcggcagcggaggcaactcaggaggtgcatggtaatggctgacatcggcacggttaccttcaacacgcagtccgcattgcagggtggcatcaacgccaccccagcactgtcgggcaacaccagcattcaaggcgctggtgtgaatcaggtcgggccggttcaatccggcaacgactggttcgcaagcactggtggtatgacgatgccggacagcaacctgccagagttcttgcaggagctggcagcgccgaacaccgccaagctgaagcagcagcagatgtgggacggcttcgttgccgcccgcgctggtaagaccatggacgagattgctgcgaccgaaccgtggtacaagaaaatcttcggagacaccaactacgagattggcgcgagcatgtataacacgctctcgcaggtcaacgaaatggagagcgacttgcttcggcgtatgccggagttgcgtcagcttcctcccgaggcgatggcgaaggagttcaacgacctcgccactgcccgcatgaccggcaacggtttcgcggacacggtgttgcagaagaccttcatggatcgcgcgggttccctcatggacctgcacaccaaggagcgcacggcatggcagcagcaggagctggtgaaggcgcagtacgctgcgaactcgtcggcgtccaccggcttcaacgaactggcgaagcgcacggcgatgctcggtaccaaccgtcccatggacgagaaggccaccgaggcgctgacgcaggcgcagctgtccctgctggacggactgtcgccctcgcgctaccagacggacgagtcgtacaagtccgcgatcactgcgttctatcgtggcgctgcggatcgcggcgagttccacacgctgaagttcctcaacagcaagggcgttctgaacgccatcgacccggacgggcagctgggaatccagcagtacgtgaagcaggcgcaggatcgttaccgttccgactggctcgatgccaacccggagcaggccgagaagatggcgctcgtctccatgtacgcatcggagggcattggtgccaagccgtcgcaggcgatgatcgaggaaatgaactcgacctacgccgccgagactggaagcgacgcaccgctgtactccggtacgcagttggcttcgatcatggcacagtccgcaggcgcgcacatccgcgcacaggaagccgtcatcaaccagcgtaacgctgcggccaaggccgcgctgaccgaccagcagaagctggccgcgcaggaggaggacatccgtggtggcatcgaagcgttcaagcgcggcacgtacgcgcagacgatcaacatccccggcgtggacaaggagctgatcgaggcgaacacggtgcaggcatggaatgccacgatggccgcgaaccccaaggtcgccatgtcgcagctggtgtggaacgccaacaccgggcgaggcgctgtgctgaagggtgtggccgaccagttccagaccacggcgcgcgctgtgctccgcgatcagccgaacacggcagcggctgcactgtaccagcagtggaaggaactgaagcagaccaccgccgcacgcatcgacacgaacggtcagcccgtgcagggccgactgactggcgcgactaccgctgcgctgtacttcggagatagcgtcaacacgttcttcaacaagctgcaagcgttggagaatggtggcgtgaacttcgagcttgcttacgaggtggcccgtggagaaatcaccaccgacgatccgacgcagttcgacgcgaacagccgtaaggaatccgaggctactcaggctcgtgttacggaagctatcgccaagctcaaccccaagtacctcggcatgttcggcaacaagctgggcgactctggccgcgctgcgtatgctcgcgccatcgtccgctcggtcactgacaccggtggtctgctggacacttctgcggaaggcttgcaggctgcggctactcacgccaagctggcctacggtctggaagacgcaggcaagtacgcatgggaaaacggacgcgacgacgaaggccgagtgatcggcagcgtcggtgcatggctgggcttcatggacacgaaggaaaccggacccgccatcgagaaggccatcgacgcagcactgcgccgggtcaacatcgagccgagcaccgggctgaaggctgacgtgttccgcatgaaggacagcgagaacggcgagccggtgctgtacgtcaacgctgttggcgagaagggctggaaggttgtgccggtgtacgggcgcgacatcaaggacgagtacgagaagcacaccaagcagcagcgtcagttgcaggccccggtaccgcagggctacgttcgcatgaacgacggtacgattcagcagagcatttccatccaacccaaactgtaaggagatagacaatggcactcgatctttcggggctgacccaagaccagcagattgccaaggctgccgcttatgcgggagtgccggagtccatcgtgcgcggtcagtggcgagtagagtccggcaacgggcgtgccgccaaggacgctgacggtgtgatccgcagcaaggcaggagcacagggcgacttccaagtcatgcccaccacgcaggcaacgtgggaagcgcgcaacggtcgcaagtacgacatgcgcaacttccaagacagcatcgagctgtatgccgacatcatgcgcgagaacatgcagcttgccaagggcgacgtgacgaaggcgctgcgcatctaccaaggcggcaccaatccgaagaactgggggcaggagaacgcagcctatgcaccgagcgtgctgggcggtgcgtccgctcccgcagtgtcggcgcagccgcgcagcctgaccaccacgcaggcagacctcaacgccgcatggcagggcaacccgaacatgcgcgaccgtacgtggtccggtgcgtccatcccggatgcgtggacgggtgcgcccatcgaaggccgcaacgctctggcgtcggcagcgaaggaacacatcggcaagattcgtgcgggcatcgccgagctgtcgatgggtcaggtagcacaggaaggtggcaccgccgcgcaggccgtaggcaaggctcaggctgtccgtgcatcggatcaggttgtgccgtggtgggtgcgtcaggaagtggacgtgctgaacaccggcgctcgcaaggcgctgctggatcagaccgaacaggcgctcgcgcaggaccgcgcggacgaggagctgcgcaactcgctgaccttcctcgacaagtggggcgctgcgttcgacagcggcatcggtgctgcgatcagcaaccagtttgcgcgcgaggacgagaacgttccggaaggttggaagtacgacccgaaggaatgggagaagccgtggatgactgccgacgaactcgaagacatccgcgatgcagcgtactcgccgaacgagctgaagtacgtcagcgaccgacagttcctgcgccgccactccatgcgcatcaaggatcagcagactggctggggtagcttcggttacgacatggtggcaggcttcaccgatccgggcaactgggctatcggcggcgtcactgccgcaggcgctaaggcgctgggcatcggctcggctgcactcgttgccgaagggcgcgtgggcgcgtcgctcgcgtcggctgctgcggagaacgcggtcggttccgtcatcacggacgccgcgctggttggcatgggcgagcgccgcaacttcgcggacttcatgaccgacgctgcattcgctaccaccataggcaccgcgatgcacattccgggcgtgcgctcggctgcgcagattcgtgacaaggcaaccatcgacctgtccgcaggcaacgctgccgcttacggcgaagcgtggtcggccgacctgaaggcgcgcgctgtggccgagctgggcgaggacgccaacccggtgctggtgaacaaccgcatccaccagcttgccaagcaggaggctgtggattggctgcgcgctggtatggccgacgtgcctgacgacttccgtatcttcgcccgtcccgacgtgcaggagacgaccaccaccgcaggcaccactggtgcactcgcacgggacgcgggcaacgtggacgcaacgaccgggcggtacaacgacagcgtgggtggccgggtcgatcagcatgacccgctgctggaacgcgcatggaagaccgcaggtatcaagggcggtaacgtcgatggcgtgctgaagtatctggaatccaacgcctctatcccggaggacgtgcgtgctatcgccaacgcgctgaagcgtggcgggcggctgagcacggtgaagatcgtgccggaatcggaactcgacaagtggttcgccggtgccaacatgggtccgggtatgcgtgtggccggtggctacaacgccggactggacgcgatggcgatgcggaactacacgccggaagtggtggtgcacgaaatgctgcacgctgccacgctgcgtgagctgcgcagcaactcggtgttcgggcaggaaatggaagaactgctgacccatatcaacaacagcatcggcagtgtggactccacgctgaccaccgctgcgatggagacgcgcatcaaccagccgcaggcaggcttcctcgccaacactgacgagctgatttcctacggcctgacgaaccgcgctgtgcaggcggtgctgcgtcagatgcccgcgccgggcaacacccgcccgaatgcgtgggagtggctgaaggataagatcgcgcgagtgatgggtctgaagaatcaggagtccgcgctcgaacgcctgatgtcggtcgtcggtgacaacctcggcgcggaagtgcgcgacacgcaggccggtacccggcagacgcgtggcatgctcgccaactcgatcttcaagtcgaaccgcgagcgcaaggctttctaccagcgcaccggtctggacaagtccgtcagtgatgacgcgatgcgtgtgcaggtcgccgaagtgatggcacgctccgaacgcttcagtgcgcagtacggcatcgacgcggcgaagctgtccaccatcatgcagcgcttcgggctggaagctacgagcacgactctaatgtcgtccaagtcgccagttgcccgcatgcttgcgatcaccctgttggagaatcccgagggtgcagcaggccgacacagcaccgcagcgatggatcggcatggtcggtttgagtcgttcatgggcacccgcccgcgtcagtgggaagcggcctatcgcctgtggcgtgcggacgtgcgcggtatcggtgcgatcaaggacttcgccacgggctggaaggctcgcgcggacttcgagtacgcagtgaagctgtaccgcgagactcgcttcaacggcggggacatcccggatgcgcacgaggcagtgaaggcaatggcccgtgagttggaccgtggctacaaccgcatggcagcagagcagcgcgcggccggtacggtgggcgcacagcgtctgccggaggaggacgtggagggctacgagtcccgtacgtggctgggcggcagcatcgctgctgctggtccggtgcgacgcgagggtatccgtcaggcgatgcgcgatcagttcgaggtgatgggcgagctgtatggggacgacttcctcgataagttcgctaccaagtatctggaacgcatcgagcgcaaggctgcgggtgtcatcgaagcgccgggtcaggtcttctcggagtcgcaggcggacacgctgcgcgacactctgcgggcgatgtcgctcaacgaggaggagattcagaaggtcatgggcaagtacagccgtggcggtgcgaagcacaccaaggcgcgtatcgacctcgacgtgaccaagcagtacgaggacgctgacggtaagttccgtctgatggactatctcgacaaccgcgtgatggacaactaccgcaagtacgcgggacgtgttgctggtgacatcgctctggcgaagcacggcatcctcggcgacgcaggcatcaacgtggcgcgcgaagcaatgcgcctgaccggtgccaacgatgtggagctgaaggcgttcgagcaggtgatgtccgagttccttggtcgcccggtcggtaccggcgatccgactgttctggcgaatgcgcgtctgctgacctcggccatccagctgggcggcgcgggcatcaatcaggcagcggagtacagcaacggcctcgccgctgttggtgctgctggtgtggctgacgcaatccgtatcgctccccgcatgcgcagcgaaatcatgcgcatcctgaagggcgaggacagcggcaaccaaatcctcgacggcttcgagttcatcagcggtcgcggcttcggtctcgccggttacgacctacacatgttcaactcgctggacacgcaggcgtcgatgtatggtagcgagcgcgcaggcttcctgacctcgctggtgcagaaggcagcgcatgcgaaccgcatcctctcggggcagcgggccgtgcttgctgtgcagcagcgtggcttcgcggaagtgctgatcgccaagggcgtgaagttcctgcgtgatggtgctgaagctgacaccgccctgaaggacatgggcattgacgacaacctgctgaaccgcctgcgggctacgcaggatcaggtcgtgcgctggggcgcggatggtaagctggaagcagtagacccgcgcaacgtcgaggggctggcggatcggcaggcatggttggcgttctacaacgcgatcaaccgtggcacctcgcagattcttcaggacaccttcatcggcgagactggcaagtgggcgcacaacggctggctgaagctgctgttccagcaccgcacgttctcgctggtcgcgcagcagaagcagctgggccggtacgtgggcaactacggtgcatggcagacggcgggcctgatcgctgctgcgatggctgtggcggctccgctgcaagccctgcgggtgctgtcccgcgtggccctgatgaacgatcaggagcgcgacgaggccatcgaccagaacatcctgtcgcctctggcgctgggcaaggccacgctgaactacgtgtcggcgacgggtatgctcaacgatgtgctggacgtgggcactggcgtggcgggcggctggtacgagtacgccaccgatacgcagggtccgacgtggctgaagcagctggccggtgggcagttcggcaaccgcaaggaagtggtgggcgggcagttcgcgccgtcgctgggagtcatcaacgacttcgctcagggcattgctggcaagccggagaatctggccgacgtgattccgggcgggcgactgccgatggtgatcccgctgctgaagggcgcagccagccagtggaaggaggagtaagatcagggccaaggacggcccacccttttggtacacctatagcaaacaggaggcagcatggcagttccagacccgcagctgcgctacgcgacagacgtgttcgacgccgatggcgtgaccactgactggcagatcagctttaccggtggctacatcaacccgtcccacgtgtacgccatgagcggactgctggacgaggagactcagctgctgaccgaccggactccgcacaccgtggaagtcctgagcgaagacgatgacgctagtaccgtccgagtctcgcctgccgtcgccgctgggcgcaagctctacatctaccgcagcactccggtgcagcagatgctcgttgactacgttaacggtagcatcatcagcaagacaaaccttaacctcagcaacgaccagctcctgaagatcattcaggaaatgttcgactcactcaacatcgccacccttagcatcgaccagcaggtcggtgtgatcgtggacctgaacgagattatccagaacatctacaagcaggtcaccgagttgctggcagctggtggtatcgtgtccgtcgccccgcgcgtctggtccggtgcttggactggcgatcaggtgggtgacaccgacttcgacatggtgggcgcggacgtatccggcgcgggcttctacgacgtgtacgtcaacggcatcggcatgcagccggacgtggactatcaggtcacgctcgctgacggcaccgatcccagcttcatccgcttcgccacggttcctgccgagggcagcatctggttcgccgtgctgcgtggttacgccaagccctacaccgggcctgcgccgatcaccgctgcgagcctgcgggtgccgatcatcacggcagagggtccgacttactacgccgccaaggctaccgagtacggactcgtgcgctgcacgtacgccggaggttgcgccgtcaacatcaacctgatccccgaagtgggcgacggtgaaaccaagctcgcctcgggcagctacttcagcgtgcagcagaaggcaggccctgtggtcatcactggcgacgtgggcgtgacgctcgaagtcccggtcggctgcaccgccgcaactcgcggcaccaactccgtcatcactgcaacgtgcatcgacggcgacaccaacacgtggttgctctcgggcgacttggctaaggagtaagcatggctaatcacttcaggctgtacggccgaccgctcatggcggacgaggttgcagatggcctgtcggtgacgggcgtgctggaagggtacacggcgggcgaggcttacgagtctcgcctgtccatcaacaacccagtcggccgctgcaccgtggaggtcatcgaatcgacgctcccttcgggcgctgcggtacgggtggacaacatcaccaaggaagtcgtcgtcaagtgggcggctttcactgaagtcgtggacgaggaaaccctcgtgcccaacggcgacttcgaggcaggcgacgacggcacgtggttgccgggcggtggatcgaatggcgaaggctggtcgattggcactggctcagactacgacaccgacagcggcgtgtacagcgcgcgcttcgccaacatcaagacgggcggcagcgacctgctcaacccgctgatccctgccaaggtcaacgactacatccgatgcaccgccgaggtccagcagggcgcaagctccaagggcaaggccggtgctcgtgtgtcgatcatctaccgcaaggaggatgggaccgagctgcaacgcaactggggcaacatggtttcctccggcagcaacggtgcgtggcaccagtccgttgccgaaggcgctgcgcccaaggacacgaagtacgtgcaggttgtactgtcggcgttccgcagcaagcagaacaaaccgctgtgggtggacaccgttaagtggaaccacaagtacgtactgggtcagaacgacgacagctcctacttccttagcatcaaggtcacggacgggttgaaccgtgtggcctactggtccggtcgtatcgaggagcagggcatctacgttacgtccaagctctacagcttctaccagttcgatgccgcgatgctgaccagcagctttgctgggtacagcaacatcgacatgctccagcctttggatactgcgtcgctgggttcctccttcgtaagctgggaactccgaagctctaggcaggattatgccgccgacccggagagcacgttgtacgggagcgctttcgtttcgttcgacatccgatccatccgtaaggactacacgcctgacccggagacggcgaagctgtcgagttctttccattccttcaccctgaagcagcaccctgtagtcaaccagccgctcgacgcgactgcacgactccggtctggcttcgtatcatggagcttcgcatgatccacaatcacctcggcattgctggcgtgttcaccatcagcaagggtaagtccctcgatactctcgaagttgtagccgactggcagagcaaccttatcacggacggtggtatggacgcactgggtgataccggcagcggctatcctcgcagcatgtacgacctcattgcttacttggcagtcggtagtggcagcgccaccccggcattcaccgataccgctcttggtgcacaggtggcgcaggttggtcgtacgtcctcggacagcggtgggactaccactgccccgtactacgcctactcccgctgccagtaccagttcccggctggtaccgctactggcgttctgtcggagcttggtgccaaagcatacaacaacaataccggcgcgtacatcctgaccacccgtgcgcttatcaaggactccgcaggtaacccgaccaccatcacggtgctgtcggatgaaatcctcgtggttacttacgagctgcgcatgtacgcagataccacgccggttgtcactactgagacgatcaagggtgttagcaccactgttacctgtaagcctattgcaatgggccgcagcggcggtatgaacggtcagtcggcagtcgcttggtcggactacgtgtgggggtgctactacttctacggcggtactggcgacggcaccggagctatcaccgaccagtatccgccggggacgattgccagcttctctgacttgcagcttcagcaggtagcctatgttccgggtacttactaccgtgactgcgtttgccggatgtcgatcaacaacgtgcccggtggtccgatcacggctgcaatgggactctccgcgtgcgtgaccttccaagtcggcttcaatccgggtatcaccaagaccggatcggagacggcgaacttgcgcatgcgggtttcttggagccggtacacgccatgatccccactgtctcccaaagcatccaacgcggtgactgggtggagcagcagaatcggcgcacccgcccgctcattgacttcgagcagggcgggctgactctcaacgcagcagtggacgacctccaagctgcgctgtggactgccgagagtgacggcagcagcgtcgtcgtttaccgcgacggcgttgccccggtcaccgtgctgaccgactccgggatcacgcagatcgcactggccttcgaccagaccatgcgcccgcacgtggcgtacatggcgggcggtgtgtgcaagttctactggtacgacacggtggctgcttcgatgcagaccatggtgatccccggtgctaccactccgcgcctgtgcatggacgagaagcgggctgtcttcgccacgcagagcgacgtgctcctgtcgtacaagaacggcagcaacctgtgcgtacgcgcgcagcgtgagcgcttcgcaaccgaacatgtgatcgcctcgggaatccccggcgacctgattgcggtgggcatgaacaacgtcaaccgcctgcaatggaagctcgtcggcaatcccgacgactggccctaacctacaggagaacagcatgaccccgccgagtgtggtcaatgaggtcgtccgaacctcgccgcttacgctcggcgcggtctacctcaacttcatcagcacgtacggtgctgccatcgtaactacgctcgccattctgtacgccgtcgctcagttctactggcgggcacgcgagcaccgaaagatcatgggaggcaaggatgtcgaatccggcaagtgagggcgcactcggtgcgctgcacgaactggtcgcgcgtgcgctgatgcagcgcatccaagatggcgagctgtgcaccgcagccgacatcaatgcggcgatcaagttcctgaaggacaacaacatcacggcgacgcgcgaggccaacaaggcactcggcgagctggaagacgagctgggcaagcactcgctgcctccggctgacgacgacgagttgcagcgtgcactcgacaacatcgttcactttccggggagcgtagccaacaatgcgtgaatcagctgaagcggccgacgtgcgccgcaagaagttggagctgttgcagaaccactaccggcacttcgccaccttcatgcgcgacattatgaaggtgctggggttcgagccgacgtggatgcagtacgacatcgccaactacatgcagtatggcccgcacctcgcaatggtgcaggcgcagcgaggcgaggcgaagtccaccatcgctgccatctacgccgtcttctgcctgatccacgatcccactcaccgtgtgctgatcgtatcggcaggcggcacgcaggcatccgagattgctacgctgattcagcgcatcatcctcacggtgccgacgttggagtgcatccgcccggacaagaacgcgggcgaccgtacctccgtggatgcgttcgacgtgcaccactcgctgaagggaatcgacaagtccccgagcgtggcgtgcatcggcgtcaccggcaacctgccgggtaagcgtgcggacctgctgatcgccgacgacgtggagtccaacaagaacagccgcactgccgcgaaccgtgagctgctgctgaccatcacgttggagttctcggccatctgcaccggcaagcccggtactccgggtcgcatcctgtacctcggcacgccgcagaccggcgactccatctacaacaccctgcccggacgtggctacgacgttcgcatctggcccggtcgctacccgaccccggcacagcgcgagcactacggcccgcatctggcaccgtctatcgtgcagcgcctagaagccgacccgatgttggcgttcggtggtggcccgatgggcgacgagggccagtgcaccgacgagctgttggccggtgagcagaagcaccagtccgagctgcgtcagcgtggaccgtccagctatcagctgaactacatgctcaacacgcggctgatggatgcgctgcgcttcccgctgaagaccgagaacctgatcgtgatccccggtggtggcgaccgcttcccgctgacgatcacccgtggcctgagcaacgctcaccagcgcagcttccagtccagtgggtacggcttcgtgatgatgatgccgcacgacatgagcaccgagactgcccccgtgcagggcgtgcacatgcagatcgacccggccggtggtggtgccaacggagacgagacggccttcgccgtgaccgccttcctcaactccaccgtgtacgtgttggccgtgggagctgtgcccggtggctacgacggtgatggcttgctagaactgcgccgcattgcggtgaagtacaagccgaacgtcatcagcatcgaaaagaacatgggctacggcgcgttcgccaaggtgttcctgcctgtcctgcgagaagatcgcggcacggagaagggatacaagggcgacatccgcgaggagttcgtgaccggcaacaaggaagcccgtatcatcggcactctcgaacctgtcatggctcgcggctcgctggtcatgctggaatccgtggttgaaatggatcacgagtacacccagcgctacgccaccagcggcaagcgtcaggtctacagcctgttccaccagatggcgaagatcacgcagcagaagggcagcatcgcacacgatgaccggctcgatgcactggaaggtagcgtgcgtcactgggttgcgcagcttgcactggaccagaacaaggccatcgccaagcagcagcagcgagagttccaagactggatcaacgatccgaccggcatgaaggcagcgacccgcaagagtccgctgcaacgtggccgtccatccctactcgaccgttaccggaggtaaccaatgcagaagtccgacttcaccagcaactacacgggtctgttcggccgtggcaactacctgcaccgcgaactgctcgccctcatggagcacgcagagcagcatcccgcaaccgcagcgcagctgctcgcgcagttccagaaggacgccaccctcgtgctggacgccctgatcgctgcgggcgcacgcaccgcgtcctcgggtccgaactccggcccgcacactccggtcgatctggacccggatgacgacccactgaccccgtaaggagcaaccatgaaccagcagcagaaccaagataccagcaacaaggggctgttcggcctgatcggcggcatcttcatcggcatttcggcaacgctgctgtcattcacccaaggccacgaaggggtacgctacgctgcgtacctcgacaccggccgggtgccgaccatctgctacggccacaccaagggcgtagcgatgggcatgacggcaacgaaggcacagtgcgacaagtggctgatcgaagacctacagatcgcccagcagggcgtgcgcaagcacctgaaggcccccgttaaccgcaaccagatcgacgcctacacagacttcgtgttcaacgtaggtgagaaggcgttcgccgacagcaccatgctgcgcaaagcgaacgcaggggatcgtgaaggtagctgcaaggagttcctgcgctgggtctacgtcggtaagctcgactgccgactgtccagcagccgttgctccggcatccccaagcgccgcgacgcagagtttgctctgtgcttgcgccccaacaacgaggtgatccaaccgtggaaaccccaagtgaagtgatcgcgcggctcggcggcaagctggttggcttgctgctggtcgtgaccatgttcgtgtgcttcggtctgtacgtctacggcctgcaacgcaaggtggagaagctggaaactgcccaagtcggcacgaccgctaccgccaaggcggcgcagacgcaggctaccgggtacgcgacctacatcaaagagaaggaggacgtgcgtgttcgcactgaagaagttcttgacgctgccccggagtaccgggatggcactgttcctgctgatgtcgctgacctcctgcgcgaacctgccggtccctgacgactccctgcttgcagactgccacatcacctacctcggtggggagaagggcaccacctcctcgcaggacaaggtggtcaagctcgcgcaggaccgccgcatggacaccgttctgtgcaacaaggacaaggctgcgctgcgtgcgtggaaggccgaggtgtgcggtaccggtaagcgccggtgtacgggtgacaaatgaccaccatcgcatgggacggcaagcacctgtgggccgatagtcaggccacgcagggcgaccacaagcacaccgtgcgtaagatcatgcccgtatcgacacccaccggccctgtgctgctgggtgtcaccggggatttcacagtgcttcgcccggttctcgctgcgcttaaagcgggcgaaggctacgaggagcacgttggcaagtccgcgacggtgcttgtggttaaggacggcgtactcacggtcactactggtaagcagcagtgggtcgaggaggctccgtacttcgatggcagtggcaaggcgctagctctaggggcctatcatgcgagcaagtctgtggctaaggccatggctgctgcgatagctcacgatgtctacagctccgggcctatcgtcaagctaaaggcaccagttcgcgaggcttaggagtaaggccacgtgggtagccggaccaaaatttgcttcggaaatgcgcgggggtcactccaatagaagctcccgcgcgtgcccccgtacgccctcgcgttacgcgcctgcgggtgtgcgtgggtgcgtgcccgcgtgtgcgcctgtgtgcgcgtctgtgcgcccgcgtcaaggttccgcgtgggtgtacccgtgtgcctgcctgcgtgggcctgagcgtgcgtgtgcgtggccgtgcgtgggtgcctgcgggtgggcgtgcgggtgggcgtgcgggtgggcgtgcgcctgctgcctgtatggctggacc

SEQ ID NO: 24 - DNA, 44415 bp, unidentified
  source 1..44415: mol_type = genomic DNA
ctgcttgtccttgatgttgcggcgcttgcagatggtggtggcctcgaccgcgcgctgataccagccggagtcggcggtcaccatgacgttgaacacgccgttgcgcagcgcataccacgtggtgctgtagtcctcgtcctcctcgtagtgtccatcggcaccggagcacagggtccatccctgatcgaccagcttttcgatggcctcgtggaagtcctgcaccagcacgaggaagtcgatgtccgtgtcggtcacgggcggctcgactgtgtagctgctgccggtgcggctggacgtgatgacgcccacgttgcgcggcaggtagatgttcggttcggtactcacggtgtgttacctccgggcttggtgatccagaacgtgaagcacgggatcagattgatgcaccagcgcttgttgtgcggcgagtagtgcacgccgatccaagtgctgtgtttgttccgcagccatccccacttccactgcggcgcgtcgttgcggccttcgatgtagcctgcgtcgtgcaccttgcgcagcagcttggcaaggtggattgcttgcgcgttgctcacgcagttgaaggtcttcgcctcggtggattcaccggggaagctgaccgacaccgtgaacccggtggctacgatgtgaattggcttgctcatgctgcctcctgatagaagcgggcacgctctgcatccatcatcacttcttcccgaacgtcacgcttgccgcctgcgcggtgcagcttgttcttcggggtgccgatgtagcggaagcgttccatcgctgggtcattgagcttgccgcccatgatgatgaagtcgcacgcaccctgcttgccggtcttgctgtccttcagtgcggactgcggcgggtactggattccctcaccctcggcgctgatctgcgaagtcgccacgcccacggcgtcgtacttcacacaccagttgcgagcggcctgatacatcgcctccaacatctgatcggtacgctgcccgccgttggtcatgccaccggtgaacgtgatgttgtcgatcatgtcgaagatgatgaagccggggttggtctgcttgatgatggcctcgacttcaccggagttgaacccgtggatgtcgtagaactgcatgcggtggatgtccccgcccatcgcatcttcgatgcgcttgcggatgctaccatccttcgcccactccaccatctcagggatggtagcgccgagcagcgactgataccaccgctgcttgatgcgcttgcccggcccctcgttgttgagccagatgccggtgcgcttctggtccggccaaacgttgtcgagctgcgtgatccagtggctggactcgctggtcaggaacgtggtcttgcctgcgtcgggacgcatggcgtagatgccgaagtcaccaccacgcagagcgcgcaggttcttcgccaacgtgggcagtcggaagtggatgccgatgtcgtgctcgtccatctgcatcagttcctcgggcgtctcctgcaccagcgggagccgcgccttgcgatccattcggtcggtgatcgtctcggccaagccgtacagctcgtcgcgcaggctgaactcagcgccgccattccactgcacgatcttgctgaccgcagtggtggcaagctccaactccaacagcttctcgatcatgccctgctctgcctcgggcgggaccggctcgcgcatctgcttcagcagaactttgagcagggacttcttgtcgtcgggctgcgtcttccacttgaactccatggcccagccatcgaacacatcgaacggcaagtccttcgtgtccgggaactccttgtagtacgcacgcaacgcatcgagcatcagcacggtcagctcgtccagcccatcacgtggtgcgctgggtaccagccggtcgaacttgccacggttggtgcacaaccgcagcagcgtggtgtcaagactcatcaggttctccttcgggttcgtacttggaatcgagctggtgataccgggtgttgcgcgtctcgaacttgcgcccgccgtccgccacatacagcaccgtcgaggtgtgcacgatgtcgcagtcgccgaggttcggatgcgcaagcacgccgccgagcgtggcacggaagccaacgacgggcgggatgatagcgcgccggtagcgcacgatgggtttgctcattgcagcttctccttgatgtagtcggtcgtgtaatacttcgggtcacgtggtgacgtgatgttcctgtagtccagaccaaacgcacgtagacgcgcagcgattactcgcgcactgtcttggccgggattgctaccgttgcttctacctctgtcgtcatcgagccacgtcgctacacgttggcctcgatcagtcagctgcttcaacactttgttgtgcagcttggtgccgagcaacgaccacgcttcggttaccagtcccaccttgtatgcactgagcgggtcttcgcacagtacgatggtgtcacctgtgcccacgccgtagcgtgcgacaagtccgtctttcggaacgtcaggtgttagccacttcggctgtctcgttgccgaccgggctgtccagtataccacgttgtcgccttcagtgatcggtagtaccacccgcccgatgcttgggcaccagtacagccgcagcttctcgatcatctgaagcgagagtcccatcttgaagaaccacaccttagcgtcgagcggccactcgcgggtgtcgtatacccgtggctctggcaactcaacagtcgcacgcactctgcgttcgctcgtctgctcggcgtggattcgtgcaagcttggcctcgatactctcgtgctcacgcttgaatcctgtgccaccgcacctgaaacagaatgcggtggacttgtcgtgctctcgtgagataagcaagggcgtaccctccccgcactcatgggccacacgtgtgcggccaccaacaggcaggcgctcggcatgtggtagccagtcgttgtcgggaagggtatcgctcatgctatcctcgcttggttattcccagacctcgaagatgtcgtggctggtggcgtacaggacggagccgttgccgtccgtgctgacgatcagacgggagccgtcttcactggtcagcttggacacgacgaacccggtgcccttcggcagcttgttggtctgccgcgtgtcgatcaggtacgcattctggccgggcttcagctcgtcgccacgcttgacgacggccacgctgggtgacggcggggcgaggctcacgactgcccgccttcgccacccgcagccttggcggcagcggcttcggcggcgaggcgctgggcctcggcaacggcggcgtcgatttcttcctgcgccttcagcacttcctcggccgacatcagcagggcgctgctgtcgatcaggttcagctcggcatccagaccttcgccggtctgcaccttcagttgcagcacgcccttgtcgttcttgccggtggcgacgatcacgccggacaggacgcgcttgttcagggcacgaccgaacaggtaggacacggcgtcgcccgccttcagcgcttcgatggcggcgctgttggcctcgacggcatccagcttggcgagcttctcgttcaggccatcgaccttggcctgcgccttggcgatgtcttccagcagctcggcgcgcttggcttcgtagtggctgacggtggtctgctcggtggtgttttcgttcgacatgtagatggttcctcttgacggttgataggatggcccgtacgtgggccagtcgtagcctacccggctcgggttactgaaagatcagctcgctgttgtacccaccgccgccattgtagaagcggcgacgcagcacgctctcctcacccagcaccagcagacggtccacgatggcgcggatggcgctcatgtactggtccaccagctcgctgtgcaagttcaggtcgaagcggatcacggtcaccgcctcgtcgtccagtgcgccggtgtccttgcggacgtacaggccacggccattggtcatggtcgcaccgccgatcagcttcacggcggcggcaatctccggctgcacgttgagcagtcggctgtcgggcacagtcacctcgacccagcttcccatgcgcaggctcatgctgcacctgccagtgcggactgcacgttgggctgcaacgatgcaccggaacgcagctcggcagcacgacgcttcatgcgggagcgcagcttgcgacgctgcttgttgttcccgccgaggctatcggccacgcgcttcagctggttgttgccgacgatgcgggtctgaccctgccccttctgcacggggaagtagtcctgccccagcatcttgcgcaggatcgggttgtcgatgggaatcagcggcacgctgacgtgcaggtgccggctggtgtccggcgcaggcggcggcgtgtcgtcgtcatcgtggcgcggcttcaccgctgcgaccaccttgtccttgacgtacttggccgcagccttgatcttgtccatgaaacccatggttacttcctcctcgttccgaagtgattgaactccaactcatgccacacgtagtacgtggtgccgagcgggtcagtgtctgccttccagttgcgctggtcgcagtagtcgttggctgcgccgaggtcatcgaacgtcagcgagaacccagtggaagccgggccggtgcggaaccggcacagcttgccgtcgtcgtcatggtactggccgacgacaacccacgggccacgacccacgatccagtacagcaggatcaggatgcgcagccagagcttacgcatagtacggctcgacacggtagcccatgttctcgccgcccagcgactcggcattgaacacggcgcgcgctgcatcgcgggtcgggaacagcacgttgtactcgctcttgttgtactcgttgccgtcgatgcgcacggtggcgctcgggtgctggttgtagcagctgacatcggagtcgctgcggtcttcggcgaaggcgtaggtgatacgccaacccagcggcttgcgcaccggcttgcggatgctctcgcccacttcgaggatgtgccagttgaagaacgacccgccgtagctgttgagcacatccgcctcggcacgcacggcggcgcggcggtcgaagatggcgagctggttcgggtacgtgccgtcacgcagcgagtccagcaggctggtggtggcacccttggtgcgcagctcggcgatcaccgcatccagttcctcttgggtcggggtgcggccggtgccattggcgacgacgccagtgatgacgccatcgttgctgttcttggggatcgagacgatgaagtataccttacgcatggtggttctcctgattgacgggtgggatttcgatttcctctatcgagtagagggtgggcaccttctcgtggtgcttgcggtggtgttcgatggcttgctcgcacgcctcgtggctggtgtgatgtccgccgaggatgtaatccccgacagccacacccttcacggtaacgagcggcagcgccttcaccacaaggcgcaggctgacctcacgcataccagcgctccacgctgtgctcatgggtcacgaactctttccactggcgcggctgctcgcacagctggatcggcttgcgctccccactacggatgcgcttgtaagttacggggatcatgcaatgtgccctcctgttgggcgtggttccaaagctacgccctcgttagaaggcgcagcggtagatcacgcgcggctcgggtgccacttcacgcggtagcggcggagacggttcggatcgttgccgacgtgcgaggcgatggcgttgcgtgcagcctgcgcagtggtgaacgtgccgctgagtccgatcacagtggacgtattccaacccagctggtgagggcgccgcgcatgcttggtgaagaactcggcggtgtagaagccgcgatccttctccgggccatcgggagtgccttcgggcaccacacggtacgcatcctcgctgatgccctgcaccttggcccgcgccttcagcatgcggtacgcagcattgcggctgcgctgcggcaggcccagctcacgcacctgcgcccagttggcgagggcgatgctgccgtggcgcagattgaactgcacgatccagcccttggtcttcgtcttgttgaccagcccggtctgcgatgcagtcagggcgacgtggcgtgcgctctggtcgtccatcaggacatccggcagcttacgcggcaggttgtcgggcattgccaggccgggcaacaccatgcggccggtcacgctgccgaggaagtccagctgcgaggcatccaacaccaccggaggcaacggagacagcaggcacgccatcacccgcgcctcgatagcagcgaagtcaagttcacgcatgccgtagcccacggtgaacgtcggcggtgcgatcaggtcgcgcagcagctgtgcctcgacatcgctgtcacggcaggccgcaatcacgtcgtcctcgaattgcaggatggcgtcacgctcgaagctctcgacaccgaagtcgcgcagctcaccgtgcagcacggcgaactcattggacagcttgcggttggagtacgggtctgcctttgcggtcagtgcacaggcgatgtgaagggccgagcgcagcagggatgcttcgcgctgggtcactcgaaggttgatcttgggttccatgttacacgttctccttcttcttggtgggcttcggcacagcgcgggcagcgttgatgacggcctgttcctcctcggtcggcacgtagccttcctcggtcgccttttccagacggcccagcagcttgtgcaggtcggcggcgaacgagaacgcctctgcgggcttctcggtcttgaagtcgtaccacgccttcgcggcggcacgttccagcacgtcggccagagcttcgccctcgactcgcttgctcttggcaaacttcatgggcgcgctcgccttggtttccttgtcgtcgttcggagccatcgggccgaactcggacaggtacaggcgcagggcttcatgcttcatgccgttgcccacggcgagacacagatcggaagcgagcgtaacgtcgccgtggatgtgtgcgtggttgatgaccgcaatcgcggcctgctgaatctggtccaccagcttggtgcgggcggtgttgatcgacttgatggcgcgcttgatgtcagcgcttccggtgatgatgtccatggtggttcccttcaggttgggtccgtgccgattgcacgacactaggccctcttgcgaaggcccagtagcttgcatttaagcgagtcggatgtcgaatgaacgcccaccgcacggcaggacgtagagcgccgacacagagccggccggatgcttcatgatggcccgattgtaggaatcgcgggcagcttccacgtagtggcgagagaacttgaaccggatcacaggtaagccctcctgtcagcggcgtggttcgcccggttcgtcccgctgttaccctcgacaacaaacacagatcgctttccggcggttccgtggcgggcttcgtagcgctcggcttggcgcttgcgctcggcaagcttgcggtcatgctccgtggtgcgcaggtccatcacgcttgccgtccgggtgaactggcagaagcggcgcttacgctgggtgcggtcgagattggcattgatcgagccttgcatgttgtgcctccattggcactggtgggaaaactaacagattgatgcgccctcagaaagccgtcgagtcggtcaatccctcattctcgattagagccgttgcatcgcctatcgtgggcgcacactgaccaccggatttgcctgcatggtcatcgcaaagggagggcgcatcaatctgctagcccttcgggctgtcaaccctactccggctagcagtgccattgtcaccgtgtggcccgtagagccttttcacgaaacgcacagtattccatgcgataggaggctcaccacctccttatgaccggcttcccaccttggcagtgggttacttcccgtggccgactctcacggcagatgggaagccctaagcgttaggcttaggtaaagcggcaccagtgttgcaagtctggtggattctatgggcctttgaaatcccagttcatccggttatccgctagtgctacgttgcagcttggcggtccacgtcaactctcggccactattggctgtggttggcacgcttcccgttacaccctacccgttagcggtagtcctacgccatccaatgtggctgctcctcagagcgtggtgccatactagcacccttgttgcatcctgtcaagcccttggctcgctcgggtctctaacccgttgggcgtcctgtcgccaccatcccaccatgtacgtcggtggtccacgtgttgcaaggcctcaaagggctatctgtgccgccttgtcaagctatccgttagaggaccatgtgcgctcctgttagtgtcttgaccggtgtcccggtctcacctcagcctcaacacccgtaatctctcacgtctagccttaccgctaggtcgctccgctgttccggtggctaccacttgccgcctatcatagctaactgctagcttagtgtcaagcgtggttcggtagctcctcgcatcccttaccagtgactcccgtgtacccttagcccacttgttggcggcgccactacggatcacgtcactcgacttgcgttgcagcttactaccattgcggccgtgtgtctactactgcttgcatcgcaagcgtcaaccgttggcctagcgggtagctaactaatcagctcgacagagtaccgatagacggtgattcaggttgagccgactgtgtgctataggtgtaccaaaaggccgaaacgatacagatggccctcgcacgcctacagctgcggttcgcatggtagcaggtagggtagcccctgtcaagccccttgcggccctcctgaagccctgtcgctgccccagtgacgccattgaaccacaccgcaccggccacgtcaacacctttcgccaagagatttattaacgattcagccaaggcagcgcggtccagccatacaggcagcaggcgcacgcccacccgcacgcccacccgcaggcacccacgcacggccacgcacacgcacgctcaggcccacgcaggcaggcacacgggtacacccacgcggaaccttgacgcgggcgcacagacgcgcacacaggcgcacacgcgggcacgcacccacgcacacccgcaggcgcgtaacgcgagggcgtacgggggcacgcgcgggagcttctattggagtgacccccgcgcatttccgaagcaaattttggtccggctacccacgtggccttactcctaagcctcgcgaactggtgcctttagcttgacgataggcccggagctgtagacatcgtgagctatcgcagcagccatggccttagccacagacttgctcgcatgataggcccctagagctagcgccttgccactgccatcgaagtacggagcctcctcgacccactgctgcttaccagtagtgaccgtgagtacgccgtccttaaccacaagcaccgtcgcggacttgccaacgtgctcctcgtagccttcgcccgctttaagcgcagcgagaaccgggcgaagcactgtgaaatccccggtgacacccagcagcacagggccggtgggtgtcgatacgggcatgatcttacgcacggtgtgcttgtggtcgccctgcgtggcctgactatcggcccacaggtgcttgccgtcccatgcgatggtggtcatttgtcacccgtacaccggcgcttaccggtaccgcacacctcggccttccacgcacgcagcgcagccttgtccttgttgcacagaacggtgtccatgcggcggtcctgcgcgagcttgaccaccttgtcctgcgaggaggtggtgcccttctccccaccgaggtaggtgatgtggcagtctgcaagcagggagtcgtcagggaccggcaggttcgcgcaggaggtcagcgacatcagcaggaacagtgccatcccggtactccggggcagcgtcaagaacttcttcagtgcgaacacgcacgtcctccttctctttgatgtaggtcgcgtacccggtagcctgcgtctgcgccgccttggcggtagcggtcgtgccgacttgggcagtttccagcttctccaccttgcgttgcaggccgtagacgtacagaccgaagcacacgaacatggtcacgaccagcagcaagccaaccagcttgccgccgagccgcgcgatcacttcacttggggtttccacggttggatcacctcgttgttggggcgcaagcacagagcaaactctgcgtcgcggcgcttggggatgccggagcaacggctgctggacagtcggcagtcgagcttaccgacgtagacccagcgcaggaactccttgcagctaccttcacgatcccctgcgttcgctttgcgcagcatggtgctgtcggcgaacgccttctcacctacgttgaacacgaagtctgtgtaggcgtcgatctggttgcggttaacgggggccttcaggtgcttgcgcacgccctgctgggcgatctgtaggtcttcgatcagccacttgtcgcactgtgccttcgttgccgtcatgcccatcgctacgcccttggtgtggccgtagcagatggtcggcacccggccggtgtcgaggtacgcagcgtagcgtaccccttcgtggccttgggtgaatgacagcagcgttgccgaaatgccgatgaagatgccgccgatcaggccgaacagccccttgttgctggtatcttggttctgctgctggttcatggttgctccttacggggtcagtgggtcgtcatccgggtccagatcgaccggagtgtgcgggccggagttcggacccgaggacgcggtgcgtgcgcccgcagcgatcagggcgtccagcacgagggtggcgtccttctggaactgcgcgagcagctgcgctgcggttgcgggatgctgctctgcgtgctccatgagggcgagcagttcgcggtgcaggtagttgccacggccgaacagacccgtgtagttgctggtgaagtcggacttctgcattggttacctccggtaacggtcgagtagggatggacggccacgttgcagcggactcttgcgggtcgctgccttcatgccggtcggatcgttgatccagtcttggaactctcgctgctgctgcttggcgatggccttgttctggtccagtgcaagctgcgcaacccagtgacgcacgctaccttccagtgcatcgagccggtcatcgtgtgcgatgctgcccttctgctgcgtgatcttcgccatctggtggaacaggctgtagacctgacgcttgccgctggtggcgtagcgctgggtgtactcgtgatccatttcaaccacggattccagcatgaccagcgagccgcgagccatgacaggttcgagagtgccgatgatacgggcttccttgttgccggtcacgaactcctcgcggatgtcgcccttgtatcccttctccgtgccgcgatcttctcgcaggacaggcaggaacaccttggcgaacgcgccgtagcccatgttcttttcgatgctgatgacgttcggcttgtacttcaccgcaatgcggcgcagttctagcaagccatcaccgtcgtagccaccgggcacagctcccacggccaacacgtacacggtggagttgaggaaggcggtcacggcgaaggccgtctcgtctccgttggcaccaccaccggccgggtcgatctgcatgtgcacgccctgcacgggggcagtctcggtgctcatgtcgtgcggcatcatcatcacgaagccgtacccactggactggaagctgcgctggtgagcgttgctcaggccacgggtgatcgtcagcgggaagcggtcgccaccaccggggatcacgatcaggttctcggtcttcagcgggaagcgcagcgcatccatcagccgcgtgttgagcatgtagttcagctgatagctggacggtccacgctgacgcagctcggactggtgcttctgctcaccggccaacagctcgtcggtgcactggccctcgtcgcccatcgggccaccaccgaacgccaacatcgggtcggcttctaggcgctgcacgatagacggtgccagatgcgggccgtagtgctcgcgctgtgccggggtcgggtagcgaccgggccagatgcgaacgtcgtagccacgtccgggcagggtgttgtagatggagtcgccggtctgcggcgtgccgaggtacaggatgcgacccggagtaccgggcttgccggtgcagatggccgagaactccaacgtgatggtcagcagcagctcacggttcgcggcagtgcggctgttcttgttggactccacgtcgtcggcgatcagcaggtccgcacgcttacccggcaggttgccggtgacgccgatgcacgccacgctcggggacttgtcgattcccttcagcgagtggtgcacgtcgaacgcatccacggaggtacggtcgcccgcgttcttgtccgggcggatgcactccaacgtcggcaccgtgaggatgatgcgctgaatcagcgtagcaatctcggatgcctgcgtgccgcctgccgatacgatcagcacacggtgagtgggatcgtggatcaggcagaagacggcgtagatggcagcgatggtggacttcgcctcgcctcgctgcgcctgcaccattgcgaggtgcgggccatactgcatgtagttggcgatgtcgtactgcatccacgtcggctcgaaccccagcaccttcataatgtcgcgcatgaaggtggcgaagtgccggtagtggttctgcaacagctccaacttcttgcggcgcacgtcggccgcttcagctgattcacgcattgttggctacgctccccggaaagtgaacgatgttgtcgagtgcacgctgcaactcgtcgtcgtcagccggaggcagcgagtgcttgcccagctcgtcttccagctcgccgagtgccttgttggcctcgcgcgtcgccgtgatgttgttgtccttcaggaacttgatcgccgcattgatgtcggctgcggtgcacagctcgccatcttggatgcgctgcatcagcgcacgcgcgaccagttcgtgcagcgcaccgagtgcgccctcacttgccggattcgacatccttgcctcccatgatctttcggtgctcgcgtgcccgccagtagaactgagcgacggcgtacagaatggcgagcgtagttacgatggcagcaccgtacgtgctgatgaagttgaggtagaccgcgccgagcgtaagcggcgaggttcggacgacctcattgaccacactcggcggggtcatgctgttctcctgtaggttagggccagtcgtcgggattgccgacgagcttccattgcaggcggttgacgttgttcatgcccaccgcaatcaggtcgccggggattcccgaggcgatcacatgttcggttgcgaagcgctcacgctgcgcgcgtacgcacaggttgctgccgttcttgtacgacaggagcacgtcgctctgcgtggcgaagacagcccgcttctcgtccatgcacaggcgcggagtggtagcaccggggatcaccatggtctgcatcgaagcagccaccgtgtcgtaccagtagaacttgcacacaccgcccgccatgtacgccacgtgcgggcgcatggtctggtcgaaggccagtgcgatctgcgtgatcccggagtcggtcagcacggtgaccggggcaacgccgtcgcggtaaacgacgacgctgctgccgtcactctcggcagtccacagcgcagcttggaggtcgtccactgctgcgttgagagtcagcccgccctgctcgaagtcaatgagcgggcgggtgcgccgattctgctgctccacccagtcaccgcgttggatgctttgggagacagtggggatcatggcgtgtaccggctccaagaaacccgcatgcgcaagttcgccgtctccgatccggtcttggtgatacccggattgaagccgacttggaaggtcacgcacgcggagagtcccattgcagccgtgatcggaccaccgggcacgttgttgatcgacatccggcaaacgcagtcacggtagtaagtacccggaacataggctacctgctgaagctgcaagtcagagaagctggcaatcgtccccggcggatactggtcggtgatagctccggtgccgtcgccagtaccgccgtagaagtagtagcacccccacacgtagtccgaccaagcgactgccgactgaccgttcataccgccgctgcggcccattgcaataggcttacaggtaacagtggtgctaacacccttgatcgtctcagtagtgacaaccggcgtggtatctgcgtacatgcgcagctcgtaagtaaccacgaggatttcatccgacagcaccgtgatggtggtcgggttacctgcggagtccttgataagcgcacgggtggtcaggatgtacgcgccggtattgttgttgtatgctttggcaccaagctccgacagaacgccagtagcggtaccagccgggaactggtactggcagcgggagtaggcgtagtacggggcagtggtagtcccaccgctgtccgaggacgtacgaccaacctgcgccacctgtgcaccaagagcggtatcggtgaatgccggggtggcgctgccactaccgactgccaagtaagcaatgaggtcgtacatgctgcgaggatagccgctgccggtatcacccagtgcgtccataccaccgtccgtgataaggttgctctgccagtcggctacaacttcgagagtatcgagggacttacccttgctgatggtgaacacgccagcaatgccgaggtgattgtggatcatgcgaagctccatgatacgaagccagaccggagtcgtgcagtcgcgtcgagcggctggttgactacagggtgctgcttcagggtgaaggaatggaaagaactcgacagcttcgccgtctccgggtcaggcgtgtagtccttacggatggatcggatgtcgaacgaaacgaaagcgctcccgtacaacgtgctctccgggtcggcggcataatcctgcctagagcttcggagttcccagcttacgaaggaggaacccagcgacgcagtatccaaaggctggagcatgtcgatgttgctgtacccagcaaagctgctggtcagcatcgcggcatcgaactggtagaagctgtagagcttggacgtaacgtagatgccctgctcctcgatacgaccggaccagtaggccacacggttcaacccgtccgtgaccttgatgctaaggaagtaggagctgtcgtcgttctgacccagtacgtacttgtggttccacttaacggtgtccacccacagcggtttgttctgcttgctgcggaacgccgacagtacaacctgcacgtacttcgtgtccttgggcgcagcgccttcggcaacggactggtgccacgcaccgttgctgccggaggaaaccatgttgccccagttgcgttgcagctcggtcccatcctccttgcggtagatgatcgacacacgagcaccggccttgcccttggagcttgcgccctgctggacctcggcggtgcatcggatgtagtcgttgaccttggcagggatcagcgggttgagcaggtcgctgccgcccgtcttgatgttggcgaagcgcgcgctgtacacgccgctgtcggtgtcgtagtctgagccagtgccaatcgaccagccttcgccattcgatccaccgcccggcaaccacgtgccgtcgtcgcctgcctcgaagtcgccgttgggcacgagggtttcctcgtccacgacttcagtgaaagccgcccacttgacgacgacttccttggtgatgttgtccacccgtaccgcagcgcccgaagggagcgtcgattcgatgacctccacggtgcagcggccgactgggttgttgatggacaggcgagactcgtaagcctcgcccgccgtgtacccttccagcacgcccgtcaccgacaggccatctgcaacctcgtccgccatgagcggtcggccgtacagcctgaagtgattagccatgcttactccttagccaagtcgcccgagagcaaccacgtgttggtgtcgccgtcgatgcacgttgcagtgatgacggagttggtgccgcgagttgcggcggtgcagccgaccgggacttcgagcgtcacgcccacgtcgccagtgatgaccacagggcctgccttctgctgcacgctgaagtagctgcccgaggcgagcttggtttcaccgtcgcccacttcggggatcaggttgatgttgacggcgcaacctccggcgtacgtgcagcgcacgagtccgtactcggtagccttggcggcgtagtaagtcggaccctctgccgtgatgatcggcacccgcaggctcgcagcggtgatcggcgcaggcccggtgtagggcttggcgtaaccacgcagcacggcgaaccagatgctgccctcggcaggaaccgtggcgaagcggatgaagctgggatcggtgccgtcagcgagcgtgacctgatagtccacgtccggctgcatgccgatgccgttgacgtacacgtcgtagaagcccgcgccggatacgtccgcgcccaccatgtcgaagtcggtgtcacccacctgatcgccagtccaagcaccggaccagacgcgcggggcgacggacacgataccaccagctgccagcaactcggtgacctgcttgtagatgttctggataatctcgttcaggtccacgatcacaccgacctgctggtcgatgctaagggtggcgatgttgagtgagtcgaacatttcctgaatgatcttcaggagctggtcgttgctgaggttaaggtttgtcttgctgatgatgctaccgttaacgtagtcaacgagcatctgctgcaccggagtgctgcggtagatgtagagcttgcgcccagcggcgacggcaggcgagactcggacggtactagcgtcatcgtcttcgctcaggacttccacggtgtgcggagtccggtcggtcagcagctgagtctcctcgtccagcagtccgctcatggcgtacacgtgggacgggttgatgtagccaccggtaaagctgatctgccagtcagtggtcacgccatcggcgtcgaacacgtctgtcgcgtagcgcagctgcgggtctggaactgccatgctgcctcctgtttgctataggtgtaccaaaagggtgggccgtccttggccctgatcttactcctccttccactggctggctgcgcccttcagcagcgggatcaccatcggcagtcgcccgcccggaatcacgtcggccagattctccggcttgccagcaatgccctgagcgaagtcgttgatgactcccagcgacggcgcgaactgcccgcccaccacttccttgcggttgccgaactgcccaccggccagctgcttcagccacgtcggaccctgcgtatcggtggcgtactcgtaccagccgcccgccacgccagtgcccacgtccagcacatcgttgagcatacccgtcgccgacacgtagttcagcgtggccttgcccagcgccagaggcgacaggatgttctggtcgatggcctcgtcgcgctcctgatcgttcatcagggccacgcgggacagcacccgcagggcttgcagcggagccgccacagccatcgcagcagcgatcaggcccgccgtctgccatgcaccgtagttgcccacgtaccggcccagctgcttctgctgcgcgaccagcgagaacgtgcggtgctggaacagcagcttcagccagccgttgtgcgcccacttgccagtctcgccgatgaaggtgtcctgaagaatctgcgaggtgccacggttgatcgcgttgtagaacgccaaccatgcctgccgatccgccagcccctcgacgttgcgcgggtctactgcttccagcttaccatccgcgccccagcgcacgacctgatcctgcgtagcccgcaggcggttcagcaggttgtcgtcaatgcccatgtccttcagggcggtgtcagcttcagcaccatcacgcaggaacttcacgcccttggcgatcagcacttccgcgaagccacgctgctgcacagcaagcacggcccgctgccccgagaggatgcggttcgcatgcgctgccttctgcaccagcgaggtcaggaagcctgcgcgctcgctaccatacatcgacgcctgcgtgtccagcgagttgaacatgtgtaggtcgtaaccggcgagaccgaagccgcgaccgctgatgaactcgaagccgtcgaggatttggttgccgctgtcctcgcccttcaggatgcgcatgatttcgctgcgcatgcggggagcgatacggattgcgtcagccacaccagcagcaccaacagcggcgaggccgttgctgtactccgctgcctgattgatgcccgcgccgcccagctggatggccgaggtcagcagacgcgcattcgccagaacagtcggatcgccggtaccgaccgggcgaccaaggaactcggacatcacctgctcgaacgccttcagctccacatcgttggcaccggtcaggcgcattgcttcgcgcgccacgttgatgcctgcgtcgccgaggatgccgtgcttcgccagagcgatgtcaccagcaacacgtcccgcgtacttgcggtagttgtccatcacgcggttgtcgagatagtccatcagacggaacttaccgtcagcgtcctcgtactgcttggtcacgtcgaggtcgatacgcgccttggtgtgcttcgcaccgccacggctgtacttgcccatgaccttctgaatctcctcctcgttgagcgacatcgcccgcagagtgtcgcgcagcgtgtccgcctgcgactccgagaagacctgacccggcgcttcgatgacacccgcagccttgcgctcgatgcgttccagatacttggtagcgaacttatcgaggaagtcgtccccatacagctcgcccatcacctcgaactgatcgcgcatcgcctgacggataccctcgcgtcgcaccggaccagcagcagcgatgctgccgcccagccacgtacgggactcgtagccctccacgtcctcctccggcagacgctgtgcgcccaccgtaccggccgcgcgctgctctgctgccatgcggttgtagccacggtccaactcacgggccattgccttcactgcctcgtgcgcatccgggatgtccccgccgttgaagcgagtctcgcggtacagcttcactgcgtactcgaagtccgcgcgagccttccagcccgtggcgaagtccttgatcgcaccgataccgcgcacgtccgcacgccacaggcgataggccgcttcccactgacgcgggcgggtgcccatgaacgactcaaaccgaccatgccgatccatcgctgcggtgctgtgtcggcctgctgcaccctcgggattctccaacagggtgatcgcaagcatgcgggcaactggcgacttggacgacattagagtcgtgctcgtagcttccagcccgaagcgctgcatgatggtggacagcttcgccgcgtcgatgccgtactgcgcactgaagcgttcggagcgtgccatcacttcggcgacctgcacacgcatcgcgtcatcactgacggacttgtccagaccggtgcgctggtagaaagccttgcgctcgcggttcgacttgaagatcgagttggcgagcatgccacgcgtctgccgggtaccggcctgcgtgtcgcgcacttccgcgccgaggttgtcaccgacgaccgacatcaggcgttcgagcgcggactcctgattcttcagacccatcactcgcgcgatcttatccttcagccactcccacgcattcgggcgggtgttgcccggcgcgggcatctgacgcagcaccgcctgcacagcgcggttcgtcaggccgtaggaaatcagctcgtcagtgttggcgaggaagcctgcctgcggctggttgatgcgcgtctccatcgcagcggtggtcagcgtggagtccacactgccgatgctgttgttgatatgggtcagcagttcttccatttcctgcccgaacaccgagttgctgcgcagctcacgcagcgtggcagcgtgcagcatttcgtgcaccaccacttccggcgtgtagttccgcatcgccatcgcgtccagtccggcgttgtagccaccggccacacgcatacccggacccatgttggcaccggcgaaccacttgtcgagttccgattccggcacgatcttcaccgtgctcagccgcccgccacgcttcagcgcgttggcgatagcacgcacgtcctccgggatagaggcgttggattccagatacttcagcacgccatcgacgttaccgcccttgatacctgcggtcttccatgcgcgttccagcagcgggtcatgctgatcgacccggccacccacgctgtcgttgtaccgcccggtcgttgcgtccacgttgcccgcgtcccgtgcgagtgcaccagtggtgcctgcggtggtggtcgtctcctgcacgtcgggacgggcgaagatacggaagtcgtcaggcacgtcggccataccagcgcgcagccaatccacagcctcctgcttggcaagctggtggatgcggttgttcaccagcaccgggttggcgtcctcgcccagctcggccacagcgcgcgccttcaggtcggccgaccacgcttcgccgtaagcggcagcgttgcctgcggacaggtcgatggttgccttgtcacgaatctgcgcagccgagcgcacgcccggaatgtgcatcgcggtgcctatggtggtagcgaatgcagcgtcggtcatgaagtccgcgaagttgcggcgctcgcccatgccaaccagcgcggcgtccgtgatgacggaaccgaccgcgttctccgcagcagccgacgcgagcgacgcgcccacgcgcccttcggcaacgagtgcagccgagccgatgcccagcgccttagcgcctgcggcagtgacgccgccgatagcccagttgcccggatcggtgaagcctgccaccatgtcgtaaccgaagctaccccagccagtctgctgatccttgatgcgcatggagtggcggcgcaggaactgtcggtcgctgacgtacttcagctcgttcggcgagtacgctgcatcgcggatgtcttcgagttcgtcggcagtcatccacggcttctcccattccttcgggtcgtacttccaaccttccggaacgttctcgtcctcgcgcgcaaactggttgctgatcgcagcaccgatgccgctgtcgaacgcagcgccccacttgtcgaggaaggtcagcgagttgcgcagctcctcgtccgcgcggtcctgcgcgagcgcctgttcggtctgatccagcagcgccttgcgagcgccggtgttcagcacgtccacttcctgacgcacccaccacggcacaacctgatccgatgcacggacagcctgagccttgcctacggcctgcgcggcggtgccaccttcctgtgctacctgacccatcgacagctcggcgatgcccgcacgaatcttgccgatgtgttccttcgctgccgacgccagagcgttgcggccttcgatgggcgcacccgtccacgcatccgggatggacgcaccggaccacgtacggtcgcgcatgttcgggttgccctgccatgcggcgttgaggtctgcctgcgtggtggtcaggctgcgcggctgcgccgacactgcgggagcggacgcaccgcccagcacgctcggtgcataggctgcgttctcctgcccccagttcttcggattggtgccgccttggtagatgcgcagcgccttcgtcacgtcgcccttggcaagctgcatgttctcgcgcatgatgtcggcatacagctcgatgctgtcttggaagttgcgcatgtcgtacttgcgaccgttgcgcgcttcccacgttgcctgcgtggtgggcatgacttggaagtcgccctgtgctcctgccttgctgcggatcacaccgtcagcgtccttggcggcacgcccgttgccggactctactcgccactgaccgcgcacgatggactccggcactcccgcataagcggcagccttggcaatctgctggtcttgggtcagccccgaaagatcgagtgccattgtctatctccttacagtttgggttggatggaaatgctctgctgaatcgtaccgtcgttcatgcgaacgtagccctgcggtaccggggcctgcaactgacgctgctgcttggtgtgcttctcgtactcgtccttgatgtcgcgcccgtacaccggcacaaccttccagcccttctcgccaacagcgttgacgtacagcaccggctcgccgttctcgctgtccttcatgcggaacacgtcagccttcagcccggtgctcggctcgatgttgacccggcgcagtgctgcgtcgatggccttctcgatggcgggtccggtttccttcgtgtccatgaagcccagccatgcaccgacgctgccgatcactcggccttcgtcgtcgcgtccgttttcccatgcgtacttgcctgcgtcttccagaccgtaggccagcttggcgtgagtagccgcagcctgcaagccttccgcagaagtgtccagcagaccaccggtgtcagtgaccgagcggacgatggcgcgagcatacgcagcgcggccagagtcgcccagcttgttgccgaacatgccgaggtacttggggttgagcttggcgatagcttccgtaacacgagcctgagtagcctcggattccttacggctgttcgcgtcgaactgcgtcggatcgtcggtggtgatttctccacgggccacctcgtaagcaagctcgaagttcacgccaccattctccaacgcttgcagcttgttgaagaacgtgttgacgctatctccgaagtacagcgcagcggtagtcgcgccagtcagtcggccctgcacgggctgaccgttcgtgtcgatgcgtgcggcggtggtctgcttcagttccttccactgctggtacagtgcagccgctgccgtgttcggctgatcgcggagcacagcgcgcgccgtggtctggaactggtcggccacacccttcagcacagcgcctcgcccggtgttggcgttccacaccagctgcgacatggcgaccttggggttcgcggccatcgtggcattccatgcctgcaccgtgttcgcctcgatcagctccttgtccacgccggggatgttgatcgtctgcgcgtacgtgccgcgcttgaacgcttcgatgccaccacggatgtcctcctcctgcgcggccagcttctgctggtcggtcagcgcggccttggccgcagcgttacgctggttgatgacggcttcctgtgcgcggatgtgcgcgcctgcggactgtgccatgatcgaagccaactgcgtaccggagtacagcggtgcgtcgcttccagtctcggcggcgtaggtcgagttcatttcctcgatcatcgcctgcgacggcttggcaccaatgccctccgatgcgtacatggagacgagcgccatcttctcggcctgctccgggttggcatcgagccagtcggaacggtaacgatcctgcgcctgcttcacgtactgctggattcccagctgcccgtccgggtcgatggcgttcagaacgcccttgctgttgaggaacttcagcgtgtggaactcgccgcgatccgcagcgccacgatagaacgcagtgatcgcggacttgtacgactcgtccgtctggtagcgcgagggcgacagtccgtccagcagggacagctgcgcctgcgtcagcgcctcggtggccttctcgtccatgggacggttggtaccgagcatcgccgtgcgcttcgccagttcgttgaagccggtggacgccgacgagttcgcagcgtactgcgccttcaccagctcctgctgctgccatgccgtgcgctccttggtgtgcaggtccatgagggaacccgcgcgatccatgaaggtcttctgcaacaccgtgtccgcgaaaccgttgccggtcatgcgggcagtggcgaggtcgttgaactccttcgccatcgcctcgggaggaagctgacgcaactccggcatacgccgaagcaagtcgctctccatttcgttgacctgcgagagcgtgttatacatgctcgcgccaatctcgtagttggtgtctccgaagattttcttgtaccacggttcggtcgcagcaatctcgtccatggtcttaccagcgcgggcggcaacgaagccgtcccacatctgctgctgcttcagcttggcggtgttcggcgctgccagctcctgcaagaactctggcaggttgctgtccggcatcgtcataccaccagtgcttgcgaaccagtcgttgccggattgaaccggcccgacctgattcacaccagcgccttgaatgctggtgttgcccgacagtgctggggtggcgttgatgccaccctgcaatgcggactgcgtgttgaaggtaaccgtgccgatgtcagccattaccatgcacctcctgagttgcctccgctgccgctatcgaaccagccgaggccggacgtagtggtggagaagttgtcgtagttgttgccgaagttgccggtgaccttcgccccagtcacggactgcttgccggtgccgtcgttgtacccgaaggtagtggacgcccacgacttgccgccgcgatcattggactgctgccacgcctgcataccgttctgcgctgcgttgctgaaggactgagaggcaccagtgaagttgccgttgtccgcctgccacgtgccgaccgcgaagtctgccacggcctcgcctgccatcggcccaccgaagtaggtagccacggccacgccgatcagcttgcccaagcgacgcttcattgcctgcggctcgatgtgctgcgagtagtcgaactgcccgaacgaacggctcatgtccatcccgttccacgcgcgcgacatgatctgcgcagtctgcgatgcgccccgcgaggcgaggagcgagacagcgttggcctgcgtctcctgatccatttccgcctgcaaccgcaccatcgaatccatcaggtctgcggacgagccgccgacaccgacagcaccagcctgcgcctgaagtgcgccacgcgcgttcgccagttggagctgggagttaagcccagccccttggcgcgcacgcagctcctcggacagcgcttccatgttggagttgtactccttcgcggcggcgtccagttgggcgttgttcttcagggaccgcatgaaatcagcgaagccggtcttggcgacctcgctgcggttctggttgtcggtctgcgcaacggctgcacggtagttcgcacgggcaacgcgggtggtgttgttcgcttgcaggatcgtattaaccgaacccattagctaaccctccgtacattgttgaaagtctgacccgtccagctcaggccggtcacccggagcgggagccaatccttgctgcgaatctcgtaggtgcactcgcgcacttcgcgcccgacgctgatgttgagctgcccccggtacaccggttgccgcgcgatcagattgtcggagtcgccgaggatgcggccctcgaagtccgtagtggtcacattgctgttgcgggttgccaccgtggcgatcatgcctgccgtgttctccacgtccaccgtcaccttgttgagggacatgcgtccatcgagtacggcctgaccgttctggtcccgagggaacggattggtcgggatcaccagagcttcggacaccacgccgtattccagcgcaccagcagcgaggtcatcgaactggttaaggaagtcagacgcctgcgcgtagggacaacccagcaggaagtacgggctagtgctattgacggcgatgcttgcgctcgcagtctgtacgcccgtaggtgtaccaaaactcgcccagctgtcgaggcacgcatgcgagtccggctcgcccttcgggtcgaacacgtcgcacgccaccagcgacccgcgcgcagtgaacacgaggccgttcttcttgtagctgctcacgccgatgatttcgcccagcgccgggtggtaccggaacttcgaccacgcatccacgatgcgctgcccgttgttcttgttgtcctcgtaccggtacaggtagaagtcctgcgggtgctcgcgagtgcggaacatgacgaggttcggcgcagtgagcggggtgatctgcaacggagtgcccgacagccacgagtccagctcgttggacatttcgtccgtcaccgtctgctgcccgttgagcgcgcccactcgcatctggtgcaggctcgtgccttcgctgccgtactgcgcataaaagatgtagttgcccgaggtctgcgccttcgcgtcaaccgaatccttgttggcactgaacgctttaatcagcggattcttcggactgaacaccgagtcgccgctgatgccgtactgctgacggtcaccgaagatcacgaggttgccgttgtagagcgtcgcgtgccggagcacatcgccctcgctgccgtgcgcgaagatttcgatggggtcgctgtcttcgatggtgacggccgagccgcgccagaagttcaggtagtccgccgagcgtgaggcgttgacgtagttctgtgcgccgatgaccagccggtcttggaagacggacagcatcgtgatcggcttgtcgatgaaccacgggatcggcgaggtcagaccatcgcctgccactcgcgcaccgtaggccggatgctcgccgctgctcggagccagagacgtgaggcccgcaccgttgcgtgcgatgtagcctacaccgttgtagatgtagagctgcgacacgaggttgtcgatggtgcactccacgccgggcgcttcgtaccagtccaccgacccgtagccggaagtctcgccgttctccaactcagcgcgcaggtagtacgactcgtccgcgcctgcaccactcggccgcacgcgaatgaccttgccgtgccagtggaacttgacggcgtaggtcgcgtctgtaatttcctgccctgcggcgtagaaggtcgtgccgtctccctcgtcgtcaaccgtgatgtccttgaactggtcatcgtcaatgatgatcccgcccttgatgtacgttgccgacacgcctgcatcgaccagcaaatccgacagctgctccgcgatgtactccgggcgcgtctgctcagcgctcgtcacgatccactcgttgaccgcagagttgtactcgttcactcggtcgttgacgtacttctggtacgccgcgtccggctccgtgccaccgggaaggtagaacgggatgtcgctggtgtcgagcgttccggggtacgatgcggtaaccgtcttgaacgttaccgtcagcaccgtgttgtccgtccgcgtcaggttcaccgtgtacgtggtgttgtacttcccggtgcgcacccatgctgcgaggcgctggatgttcgtctgctcctgccacacgttcgtgctggtggccgaggggatcgtggtgttgcccgcgatgtagacgtagctgccgatggccgtgagcgacgatgcgcctccgctgaccagcgtgttgacccacgtgctgttctcgtacaccagagggatgaacgactcgtccgtcttgttgtagaggaacgcgaaggactcgctgcccaaggtcgaggcgtcgcgccggtacagcagcgcgtactccttgccctcctgcatgaagtcgaacacgtccatgttgcgcagctcggccgaggtgacaacggcttgggaagcagcgaaccgcgtaccacgacggcgcacgaggccgttcaccggatcggacagcacgttgatctgctcgtgcgtctgtcccggccgacgacgatgcgccggtttctgactgacaccctgaaggatgtcgggataggttccgcctgcctttgccatgttgtctccttagccggggaatgtgacgtggctgtgccacgggtgaccgctgtagttccagtaacgggaacgcagcacgtccacggatgcgcgagcgaacagcgggttcgccttgatctggcggatgtgctcggccttcaagttgatgtaactgtcatcgcgctgctgcttgatcttggcgtacttggtgttgtcgccgtcgaagtcagactggaaccgcagcaccgagtcgtcgcgcacgaacatctgcacctcgtaggggaggtcatcgaagtccagcagccgcaccagcttggcctgcacgttgtggtcgaactcgtaggtgttgcgcttgcggtcgtacagtcggcgtccgcgctgcaccacgtggccgaaccggctcgggttgcagtccagcttcagcacgtccgtggggaccatgatgtacttgctcgttgcctgcggcttcagctccacccattcggtgttgaaccacagcgagagtgaggacacgtcacggtgcacgcggtcgatcaagtcaacggcgtcgtccttgtatacgtggtcatcttccagcgtgttgagcttcgtctcgcccatcgtcttcaagcaggcgttcacgatgtcgagcttggtgatgaatgccatggtgtctcctgagaggaacaaggcagagacgccggagcgcccctgccgggatgttgcttagtccgcagccagagccagagcggccggtgcgtactcgatgtcctgcgagccgatttcgtcgtccacgaaacggacacggacgacccagcctgcggtgccacgggtgtcgtagtggacgccgacgacggtaccaacggagttggcgggcagaccggccacgccagttgcggcgacgacgcggttggaaatctcgaacggtcggtcaaagaccatgatgttgctcctgtgttggtggaagaagggcgcggtttgagttacccgaaggattcagggaccgcgcccagcggattaggcaaccttgtcgatgcggcccgcgttctcgacgcgatccagaccaacggcgaaggacatccacgagtccacgaagtagcacttcgaggcatcgctccaccacaccgaggactgcaacggcagcgcttcggcgatcagcagggccttcggcgacacggccacggcgatcagggtgctgaagtcgccgtcgtagaagtcgtcgttgtcgtcgttcgacagcaggtgaccttcgatcacggtgttcggcaggttctcgctcgacagcaccgggacgccccagccgtggaaggtcgggatgccggtcagcttgttgccgtccgaggtcaggtactcgccgttgctgatctgctcggcctgctgcaacaggtagaagatcgccgggcgcacgatcaggaccacgccatcgcgctgcggcttgaccttcttctcctcctccatgcgggagaacagtttgccgatggcggcgtacaccttggccggatcgttctcgtcaccagcggcggacagcacgacctgcgtggcaccgaagtggccctcgggcgcgcggccgttgcgggtgaagatcgactgcgtggcagcagcggccttcgcggcggcgatgctgatggtcaggtccacgaactcggcgatttcctgaccctgctcgatggcgatttccttgcgggtgtcgatgtcggtgaagatttcgtccagctgccagatgctgtgacgcgacagcagcatggtatcgacggtcaccgacgccttgctgaagtccaccggggtgccgtccggcgcgtcaccgcgcttcagcttctgaagcttggtacggccgatggccttcttgatcagggtgttggtgcccttgacctgcttgcgcgggaagaacttttccagcaccgagctggacacgtaggtgtgctcgacatcgccggtgaactgttcgaggatcagggcgttctcgttgccggactggttgacctgattcggcagaaccgggacagtcgggaagatggtgctcatgctttgtgttgctccttggtcttagtggatgacgcgcgcgttgagtgcacgcagttcttcggagtgggccgcaccacggatgcccttctcggcaaccagcttgcggtactcagcgcggtactgctccttcgtgataggagcgacgccgttgatcgacgcggcgggggcggcggcgttggtagccggtgcgcccttgacggtcgtcgcgggattggcctgtgccagagccatcaggtaacgcgcggtcgcctgagcgccgaagccaccagccgacagcgattcgcttgcctgcttcagttggtcggcgggcaggttggcccgtgcgaactgctggatcgcagcccagttctctgcgccacccacggcttcgtggacagcagcaacgttcgcggcgtgcgctgcggttgcagcggcggtgacacgagcgatgctctccttcgccagagcgaggatcggtgcggaacccttggccttgtcgccgaggacttccagcttggcttccagcagggcgaagttgcccttcgctgcttcggtcagttcgcggctgtcgatgtcgaggcccacggtgttgacgaagtattcggccgcgatgttcaggccgttgtcgccgtagtccgggatcgacaccgcagtcggcgcagcgttcgccggggcggcgggctgtgcgggagcggcaggttcgagactcagcgcgtcagcagccggaggtgcagcaggagctgcgggctgtgccggtgcggccggagcgggctggccgttgggcaacagcttgtcgtctgcgggagccggagctgccggtgcgggctggttgccgttcgaggttgcgatcacggttgcgccgggaccaccgcccggaggtgcgttggaactcattgtgtctgtgtctccatgttgttggcgttgtcgatctgctgggatgcgttctgcatggcgagctgctgctgtgcacgctgctgcatcatctggccgtactcggcctcagtcagcacgtagacgttcgggtccaagccaccagcggcggcgaggtctgcgatccacgcggacagcttcagtcgttcgagaatctgcggcggcagtgcgaggacgttggcgaggttgctgccgaactccaacagccggtcacggtcacccgtacgggagagcgcggccaagccggtgatgatgacaggctccaagtccttgcctcggatgtcgcggcccgtcaggttcatcacccaaaaggcgactggtacctgcacgtccgcagcgatccgggagtagccgccacccagcccgccttccagttcttcggcgaccatgcggatttcctgcgcggtcacacgttccgcctgacgagtcaccgccgtctgcaacaggaagcctgcgccgatgcggttgatgtaggtggactggattgcttggttggtttgcagcacgccatcgacgcctgcgttaatcagctcgatgtcacccttcatgccgggaatggccgcgccattgggcgacgccatgaagtcctcgacggaggtctgacctgcggggttaaccagccaccggaactcggaggcgaggatcgcgccctgcactgcggcctcggacagcatcgagagcgactggaagtcggcctcgtagtcttcgaccaagccggagccgtagtcatcgcctgcggccaagtcccagctaaccgcccggtagggcagcttgtctgcggtgtaggtcgaggagaagttggcgggcagcttgcagttgcaaatccacacgtcttcgttgtacttgccggtcttgtggtccagcttgacccacttgtactcccacaccatgccgtcgtcatcgggcttgaagtccgggtgcgcgacaatggcagcgagcgctgcgggttccagctgggtcttgtgcaccttctcccgaaggatcagttcgtagacctcgccggtgcgggtgcgcttgaccacgtagtgccgcatgttgagcacgcggatcgtgtccttctccaacaccatgagggcgttgcccagcacgatcagcatcttcagcaggtcgtacagccgggagcggatggagcgcttgtccagttcgagactggcatcctgctcggccttcgcaagcatcgcctgcatggcctgcaagtcagcgccttgctcctgcgcagcctgcttcgccttgcgcttcagctccaaccggaagaacgggcgggacggtgcgaacagcgacatcatcagcttgttcgccagatggttcactgcctgcgcgccgagagactggaacccgtgggtcagcggctcggtgtcctgatcgcggttcttgcgagggaacagcttgggcacggtccagctcgaatagcgttcgagtcggtacatgatgccctgtcgcttgttgtcgtaagcctcgaactggcggtgagcggtttggatcggatggtccatgctcacctcacaacaggtctgacccggccacggtcgtcagccgggaagctgcggtcgtggtcacgggtcgggtgtaagtggagcgggcggtcttgcgtcggccgatcaggtcggcagtctgcaagtcgaggtcggaagttcccagccgcacatcgacggtatcgacgggggcactcagcaacttctcggcgtactcagatgcggcctgctgtgcagctgcctgtgccatctgatcggccatcgcctgaatctggtagttcgtggattgagtttggaggttggtctgcttgtcgatagcagcagcttgcttcagcgctgctcgcttggcggacccaccaccaacgatgctacccataggttaactccttcgcttggtgaattggggagcatgccgttccagcaggtagccgtagcgtgcatacatccgtgtgagtgctcgggagttccgagctagtgcaccgcctgcgctcagtgagtcgcagtggttgatgtcagccagatgttccatcacggctatgtaccggtcgaaggaactgcccggcccaattcgcagcaccatgttctcaacgaacgtagtacggttcttggagtaccacggtgtgacaatggcaaagcacagcaggtaggcttcatcaatgattactgcatccactagaccctgtgttatcagggccactgtgtaatcagggtcatcacagttgtagctcacagaagattctctgttgtctaccttactatcttctctagatgacagatacaaagcggccgttaaagccgccttgatctgctcactatcacccgtcgttggtgttcggtacggaggaatcaacggtgaaaccctcctgtaagatgttcaggacgcgggccatccccaactgcatacctgcctccaagggcgtggtattcgagttgacggacagcgacagcccggacagcttccgcacggcggccagctggttcgggtggagcgtcatcaggactttcactttggcgtcttcggccatggtgtctcctctgtgctataggtgtaccaaaaggtccggcaccggttccgcttaccttcgcggccgctccaaccggacctcagttgcctcgtgctataggtgtactgaaactccgtcagctgaagaagtacggagaatcaaggacttgccgaaggtccagctcgcccatcggcggcggctccggcaggaacgggtaggccgagtggaaggccgacagcacgtcgtgccgctcgtacatcgacacgaacacctcccggatgatccggtacagtgccgcgctgtcggcggcgtgggtgccgaagtcgtcgtgaatcatggcgaaggcgtcgatgccttcggccttggccgcgttgaccaccagcgtcaggtggcttgcgtcgaggctgtgcacgaagttcggggcgatgccgttgcggtgccgggacttcttcaccgcgtccgtgctcttgcgcagggacagcttggcgttgccgcacagcttggtgttgatgcggtgctcctcggactcccagtagacctgcaccaccgggaacccggacggcgtgatccaccggatgcggtcgtacccttggttgaggatcgacccggagccgcgctgcaaccactccatcgcgcccgctgcggcgaccacggtgtcggcgatggcctcacccatgcgcttgctcaggaagcgcgctgcggggccgtacagggccttgtcgagcgaggggaacttcccacacttcaggtagtcttcgatgatgaagtccgcccacgaggactgccgcgagccgtacggcagggtcatcacgctgcgcttcaccagcgagcgtgtgaggccgtggtcgagccacagcgtgcggtacccttcggcatcctcgtcctcgcctagcaggacggcagtcacgcggtctgccaccatctggtagatgtcattcggcagcggtgctgggatcaggttcgtcgccacgccgcctgctgcgtcgcgcagcatcgccgagaagttctgaagcccattgcacgaaccgtccatgccgactgcgatgcggctcaggaagcgatccccgaacacttgccactgctcgtactccatgcaccagctcagaaattgcagcggcttgtcggcggtcttccactcgtcgttgttcaccgggtccgcagcgaacgccatgatctggtcgtgatgctccgctacccacttcacacgatccggcagagacgccttgtcgtatccccatcggtttgctcctgtgatgcagaaccaatccttcgcgtccttagtcagcagcggcttgccatcggcgaactccaagagcgccttctgcaagtccgaaccctgcggcgacacgccggtggtctgaacgtacttgcggccacggaagtcagcgaagtacacgaagtagatgctcgggtactcggcgaacttgcgcgccaccttcattgcgttgtagaaacgattgcccttgttctgtcgcaggcgctcgtcggtgtgccagttggacatgtcgcgcttccactgcttgaactccaactcctgattgtgggacatggtttccttggtcatgtccttcgtcagccactccggcttgcgcggcttcggcagctcgccctgagaaatgatttcctccatgtcgtgcaccttggcgatggccgacacagcttccatcagtcgcttgttgatgcgccacggcacgcgctgcaatgcgttgatcgcagccatctcgttgcgcagctcggcagcgcggtactcgtcgcgggtctgagcgtaggtcttcaccatccacggattgagtcggcgcatttccttcgtgtggaatccaccgttgtcgatgtccacccagtccatcggcggctcgacgcacggcaggtagaacggcgtggcctcgatcacgaagtcgctgatctgagtaatcagcttgcgcacctcgtcggtcagcacgatcttgacgtgcgtcttggtctggaacttgcggtacgctgcgcctgcactggcagcagtctcggtgaccacgccaatctccaacatgcccagctgcgcaagctgatcgcacaggtacgcgccgacctgatcgcgctgtgcctgtccccactccacgaactcgatgccgttcttgcgtccttgcatcttcatcaccgtcatgcggtggttctcgttgacagagagcttgcggtccatgtcgttcatcaggtggtagaacagagtcggctccgcgtcggcgaactgcgtcagcaggtactcatggtacacgttgatgccaacgttcttcaacacgtcgcggtcgctgccttcgccgtgcttgtctcgcatgcaggaggtaagggcaccgcgaacggcgacgaaggccacagcctcgtaccactcgcgtgcctgttcctcggcgctgacgggctgtccacgcttgttctgacgctcgggatcgtacttggcgcgcagaagtggcacgtgcgcttgcgcacggccgattcgcggagagtcgatgtccgcacggatgcgctccgcaagcggaagcacgaaccggcgatacactgcttgggcgtaggggttgttgtccgcgccgcccttctcctcgttgcgggcgatggacttctccatgcgctccttaccgaaggcgtaggtttccagttcgagttccacttgcgagagcattgttacctccgttgctgccgcacggtgtagtcgcgcggcgggtagcgtttcaggataccgcgcatgatttccatgtgcaggtcgtggatgatgtgcggccacgcctcaccgccgatatcctcggccatgcacgtggcagcagcgccgaacaagtcggcaccgtaccgggcgcgcaccgaaacctcgacgcggcccatccatgccgaggactggctgaagtccagctccggcttctcgaaagtgatcgcgtccatcagcccctccgctcgtcaaggaacttggcgaacgcttcctgcaccttgtcgcgcagcgtctcgttcggccacagggaaccggcgtactcgccgaaaggaacgctgatgcgcagctccaccgtgtcgcgctccatgttgtgccatgcttgcacctcgacgctcacaggtctgcctccttcttgtcgtgacggatgcccttgtatcgcggctcgcgcagcaggccgtacttgctgaaggacatcgcctcgatttccacgatgcctcccacgctaggcagctcgctctcgctgtgcggcacgccgctgccaacctcctgcgtcttgccttctccgaggtcaacgacgaccgtgtacacggcgcggccggtcttctcgccgactgcttcgttgatgccgagcacacgcaggtccagcgtcagggtcggcttgatcttgacgacttcgccgttggttcccttgtcgcccttcacccacttgccgctcggcttgcgcaggatcagcccgtcgtacgcgccgccctcgcacagcagcttcgccgcttccatgctgcccagctcttggtcgatcaggaagccctgcgactcggcgtagaacaccggcgcggtgccctcggcgatggcgtggcccatgctcggcaggcggctgacgcgctcctgatacacgaggtcgctgaaaccctgctcccattcttccagcgtcacgaagtcgaacaccacgaacatcggctcggtgtactgcgtgccgtccttcttgcggaacatgccgctgacggtgggctggtcgatctgcgggtgccagtattcgccgaagtacacgccgaccgggaagaacggcgcggatgcgagagcgttctcgatgtggtgtgcgctgacgacctgctcaccggtgcgggagaacaggtcaaccacgccacgatccaccggctgcatctgcacgtcgcccaccttgatggcatgcaggcccttgttcaccgtgggcacccagtggccgcgcttgatggcgaccatgttgcagccgtcgtacttcggctgtgcgatgtactcggtgcgaagctgctcctcggtgggccgcagcttcttcttgatcttgtcctgctcgactgccttgtggacgatgtagctcatgcgtagtccctccaaatctggaacatggcgagcggcacttcgtaccacggaacgtagcgctcccagtacgtggccttgccgtcgtaccactgcacgcggaagttgcccttggtgaaggcgcggttgatcttgaagccgcgcttgcgcttcttgtagccgggagcaacccggacattctggcgaggcacatcaaacatcggcgctgtcctccttcttggtgccgtcacccagcgcggcgttgaaccgtgcgatgcgggacgacatgaactggttgacgatggtgccgatccacagcttgcgcggagcgagcgaaccacggtagccttcccacgcatcggcgatgcgggtatacagctcggcctgatcttcgtcgggcaggttcgggaacccggccttgaccgcattctgcaatgcctcctcgtggtcggcactctcgccccacgcaacggcgttctcgtaggacttgatgagcatggcggtctggttcttgtagagcattcagttctccttcgacgggaatggaacgaaacctgcgaggcccctcatcacgaggatgcagaatgcgtcgtcagggtatgtacgatgccagagtgagttggcccactcgacatcgaactgcttgcgggtacggtgctcctctaggaagcgcgcccactcggcctcatgtgggacgtaccgatgcacttggccgcagcgggcgcaggccatcagtcacccttgctgaaccagcggcggatgatgtactggcggatgaagctgatcgctgtgaacgcaatgccgatggcgtgcgccgacagcagcggatgctcgggatgccacagcaccggaagcagcgcgatgttcgctgcgtagttgatgctgtagccgatgccgatgttcacccaagcctctttgatggagcgcgccttactctgcgccactggccttctcctcctcgcgcagttccagctccaacaggaacagctcgttgatgatgtggtgcgcccggtggtggatgcccgtctccgggtccagcttctcgccgaggcagcgcttgttgtcgtgtcggtagctcgcgtcctgataccgttcgagcgccttctcgacatgctgccacgagtgcgctttgtacttctgcgcgccgaaggtcagggtgtcgatgactcgggccagtgcacgcggcacgccctcatgcagcagacgggcctgcggcttgcccccgtcatccttcaggccgacgccacggtcggacagtgtgcgacggtcctcgtcgcggtagctcagttcgggcattggtacctctcgtctggtggtggtcacgcctccgatgctgagaagctgtcggagggaatcgggaacgcagcagctcggcttaactcgaccgtcgaagaagacctcgacatcacgagcgaacacgcggcttacctgtccacgcagcccgatcattgcgggcgcattgccgatgtactgtacccgcatgccgctgcggatgtcggtgatcttcatgtcggttccttatgccgggacggtgatgtgcttgcgcgcctcggcgctggtcgtgagcttgcgcccacggctgtagccgtcgcacacggtgcactgaagcaggaggtaggtaccgacctgcgtgcgggccggatcatcctgcgggatcatttcgttgcagccgcacttgttgcagcggtgctcgctgccgtcggccttgtagtacactgcgacgttcggatgctgcgagtaccaaccgcgcagcttcttgtactccaacttcatggacttcacgtcgatgcggttgtacgcttcgcactcgtcccatgctccgggcaggctctgcatgcaggccacccacaggtcgaagccggggaagttgtggtggtcgtacttgcgcagctccggcacgatcacgccggtggtgtactccaacttctgcgaggtgaaggcgaactcggtgcggttcagcagcatcgggtcgatcacctgcaccggagacacgggcggcaggccgaggattgcgaggcgagccttgatcttgcgaaggtcgaacttcttgccgttgcgagcgagcacgaagtcggcggcgttgagcagtgcccacagcgccttgccctgcttgcgatcatcgaacacgtcgcgcacgttgcgctggtccatgtagaacgacgcctcgtcgtccagccattcgcaagcgaacgacatcagcgaccagtcacgcttgatctgcttgacgctgaagttgttgttgaacatgccccagccatagaactcgatggggaacgtctcgatgtcgaggcagagaatcttcgggccgcgcttcggtgctcggcgaatgaactgggtaagggtcacggtgtctccttgttgatagcccgacgctttcgcgctttcgcattgcgagcgatacgcttctcgtcgtcggtcttgtaggtaggatgcaggtaccccgtgatgttggtgaggtgcgaccgcaggtagttggggatgcccgcacagaatgcgaacacgtcgcgcacgccgtaccggcctgcgttgttctcgaccttgccgagcagggagttgcatccgcgatggagcaccccgcgcacagcgccggtcttgtggtcatggtccagcaccggatcgagcggagccttcaggccgaactgtccctgacagagacagcaccggttgccttgctccgctgcgagcttgatgcgcagcagcttgacctgtgttgcagtgagtcgcttcatgctttgtatgcctccaagattgcacgcttctcgttcacgtcctcggcgaggtcatagaacgcctgcttcagcttcggcccgaacacgtcgagcttcagcacgtcgagcagttctgcgtcacgatccgtccgcatccacagcagcacggcttgctcggcgaatgtcttgcgccagtcggcacccaacacttcgctgtacttgccgctcacgatctgcaccgcttcgaggttggtcttcgtctcgaacagcagctgctccgctgtcaccttgcccaccttcggcagacccggtatgttgtcggcggtgtcgccgtggagcatctgcatccagaaccacttgtgaccgtactgcaatccgttctcgccaacgatgtcgtaagcgccgagcggaacctctgtgatgtcgtagccgtcccagtctacgtgcacgccgcagaacattcgcatgtccttgtcggcgctgtgcaccacgtgcaggatgttgtggtgcaatgctgcaccctcgttgacgtacgcgatgccatcgtcggcctcacgggtcagccagattttgggagtgaaagcgtcgccctcgtatgtctccatccactcacgaaggaacgcccagttgttgggcttgcggcctgcttggcgctgaccctgatacggctgcgtggtagcagcgaggaagcgatcacccttggtagacgcggcgtgcgtcaggtgcatgacgatcttgcccgctccgctgacatgcttcagctgtgcgcagcgggagagcacgttgcgtcgtgcatcccccgccgagcagttctcgctaccagccgcgaagtacgccatgtagtccccatcaacgtgagcgatcacgcgcgggttgtgctgacgtaccacctgcaccggcatcggggagcgctcaccggccgctgccatgagagcgctcaggtccatcaggcgatgcctgccatcgggtcgctaccgtccaccgggaacggcggcttgtcgtcggccggagcagcgtcggtgggcgcggcgttcgccacgtcgccgaccacttcgtccagcgcatcgacgccttccttggtgaccgtggtgctgcccgccaacttggcggcggcgtagtcgtagcacggaagacccttgaagttcagcgccgcagcgatgcgcagctgcgtcttgttcttcgactgcgcctcgtgggtgaccttgccggtcttctcgtccttgcgctccgggtactcgccggggatgtagatgctgtcccacatgtcggcgtcggcgaagtcccacacgaacgcacccagcggggtgatctgctgcggcaccgggatcacggtgtccacgaacttgccggtcgggatgccgttctccatttccggcaccggcatgaccggcttgcggatggaagccttgtcgatttcggcgaaggtcttgttcgggtcgcgcttgcccggcttgtggatgacttccagcagcacaccctgacccagcagctgcacgaagtggcgctcctcggtgcgcaggcggctgaagattttgaagtagtgcgccttctcgttggtggacaggccgagggtcagcgtcatgcgcaccggcaccggaccattgtcggtttcgatgtgcgggtgctgcttaccggtcagctcgaacacgatggcgacttcatcctgcgtcttcttcttgccctcgaactcgaactcgtgcttgcccagctcgtagtacccgacgatgcgggcggtggtcacaccggcagcgggcggggtgtagtcgaagctgccaccactggcgaccgactgatccttaccctgcgtggcgaccttgttcaacagtgcgtcaagactcatgcgtgttgttctccttattcaaacgacgggttgtgattacctacgaagtccttgcggatcgacgcgcggtactcgatgaccagaccggcgaactctgcgggagggttcttctcctccatcatgttgtcgcccatcttggtttcacacgggacgccaagcggcagcgtccagttgaaccaccactccatatacaccgacgcttccagcatcgaggcgtgcagcagagcagcggccttggttgcgatgtcgccgtgtgcatccacgtagacggcatcgtgcacctgattcacgagcaacgcacggcccaaccattccttcggttcggtcacgtacttccggtagaaggcgcgcaggctgacgtacatcgccgccttggcccattcaccaccggtgccttgcatcgggtagttcttgatttccgtgggcgagaacgactgcgcacagccacccttgctcgcgggcttgttggcgatgaacaccggggacggtgactcgctgaaggaatacatcttgccgtccggcgtggtccagtgcgaccggccaagctgacacgtcagcccatgcggcacgccttgctgccccgcgttgggatgcggaacgaagcgctgagtgctgacgcggttgcgcttgatgtgctcgaccatgcggtcgatgtactcgcccagctccgggtaacgctcggcctcaccgcgcaccagcgcctcgacttcttcctccgacatgccggtggtcgcagcgatcttcgccacgcccgcaccgtacgcacgctggaaggagaacaccttcgcgttgccgcgcttcttcttccacttcttgtgctcgggatgcttgtcgtccttgctcgccttcaggatgaagtcgtagtcgtacttgccttgctcaccccacgcctgctctgcacggaggcagtgcatgtcgaggccctgcttcaagtcctcgatcagctgacggcactcggtgaggattgcctgcacgtagatttcgagggaggtgtagtccgactggatgatcttgccaccccggtgccgggacacgaaggcgcgcttgatctgcgaacccttctcctccaacgtctcctcgtccagctcgcccttgctcacgttctgcaagttcggatcgctggaagacaagcggccggtaaccgtgttggtcatgttgagcttgtggtggatgatgccgtccggtcccaccagcgtgagcatgcccttctgctctccggtcttctcgtccgtcgtgatgtagtacgtggacaagtccttgtggatgtcgtcgcgtctggcaagcgccttggtgaacggcaggttgcggtagcccagcgcctcgatcacgtcggcagcggtggagtacacgccgggatcgctcttgctttcccatgcagcatcaggctcggtgtagccagggaactcgaacagcatgtcctcgttgcggaacttctgcttggtcaagtcatcgaccttcaccttcttggtcttgtactctcccttgttcttgccgctgccgtacgtggtgtagcgccagaggttgtcgaagtcctcggccggtggcgtcgccgtcgtggtaccatcgaccagcacgtagtgcacctcgtccttctgcacgtaagtcggcccaccctcggtggacatgatcggaaccttggccgtgtacttcaccttgccgccgaagatcagcgcgctcttgtggaagcggctgttccagttgaaggtcaggccctcgggcagctcggggatgaagccgttgagttcggcggtcgccgttgcaagctcgacctccaactccttcgccttcgtaagcgcccagtccttgtccacgtacatgccgttgtactcggcttcgatggtgaagcacagcgcacccatgttgaggagcgccgagcgcagaccaccacgtgcacggaaggcggcgagctgtccgaggaacatcttctcggtgttaccgatgtcgcccacgtcgtcggtgtcgttggtgccgaggaggtaatccatcagcagcgtcttgtcgatgtcgcaggtgtccacgcccgcagcccacagggacttgactgcatcgtccttcaagttgccgccgtagcgtggagccgtctcgtccatgctcgccatgtggaactcttgcgtcatgccgtgcagcaggtactccgcaagctggcagtcccacaccatgccgccgccgtcgatgaactcgatccatgcctgccggttgagtgggccttggcagatggcgtgcaggatgtcgaacttgatgttgaacccgacgaggaactgctgcccgtaacacagctcacgcagccacccatcgggtgcgccgcccatgtactggttgtctatcccgactcgggtgtcgtagtacaggccggtgttccgtgcgtcacccttccgcttgtagccaatcgccacgatcttgttcatgtcgtagaacggattggccttgcgcttcaggatggaacggatcgtggtttcgaggtcgaaggaagtgaagctcacagcggccaccgttgcagggccagctggtacatttcatccgacgcatcgccatccaagtccagcccgtcgcgcacccaacggaacacgatgatgcggtc

SEQ ID NO: 25 - DNA, 44415 bp, unidentified
  source 1..44415: mol_type = genomic DNA
gcgagaacatgggctaccgtgtcgagccgtactatgcgtaagctctggctgcgcatcctgatcctgctgtactggatcgtgggtcgtggcccgtgggttgtcgtcggccagtaccatgacgacgacggcaagctgtgccggttccgcaccggcccggcttccactgggttctcgctgacgttcgatgacctcggcgcagccaacgactactgcgaccagcgcaactggaaggcagacactgacccgctcggcaccacgtactacgtgtggcatgagttggagttcaatcacttcggaacgaggaggaagtaaccatgggtttcatggacaagatcaaggctgcggccaagtacgtcaaggacaaggtggtcgcagcggtgaagccgcgccacgatgacgacgacacgccgccgcctgcgccggacaccagccggcacctgcacgtcagcgtgccgctgattcccatcgacaacccgatcctgcgcaagatgctggggcaggactacttccccgtgcagaaggggcagggtcagacccgcatcgtcggcaacaaccagctgaagcgcgtggccgatagcctcggcgggaacaacaagcagcgtcgcaagctgcgctcccgcatgaagcgtcgtgctgccgagctgcgttccggtgcatcgttgcagcccaacgtgcagtccgcactggcaggtgcagcatgagcctgcgcatgggaagctgggtcgaggtgactgtgcccgacagccgactgctcaacgtgcagccggagattgccgccgccgtgaagctgatcggcggtgcgaccatgaccaatggccgtggcctgtacgtccgcaaggacaccggcgcactggacgacgaggcggtgaccgtgatccgcttcgacctgaacttgcacagcgagctggtggaccagtacatgagcgccatccgcgccatcgtggaccgtctgctggtgctgggtgaggagagcgtgctgcgtcgccgcttctacaatggcggcggtgggtacaacagcgagctgatctttcagtaacccgagccgggtaggctacgactggcccacgtacgggccatcctatcaaccgtcaagaggaaccatctacatgtcgaacgaaaacaccaccgagcagaccaccgtcagccactacgaagccaagcgcgccgagctgctggaagacatcgccaaggcgcaggccaaggtcgatggcctgaacgagaagctcgccaagctggatgccgtcgaggccaacagcgccgccatcgaagcgctgaaggcgggcgacgccgtgtcctacctgttcggtcgtgccctgaacaagcgcgtcctgtccggcgtgatcgtcgccaccggcaagaacgacaagggcgtgctgcaactgaaggtgcagaccggcgaaggtctggatgccgagctgaacctgatcgacagcagcgccctgctgatgtcggccgaggaagtgctgaaggcgcaggaagaaatcgacgccgccgttgccgaggcccagcgcctcgccgccgaagccgctgccgccaaggctgcgggtggcgaaggcgggcagtcgtgagcctcgccccgccgtcacccagcgtggccgtcgtcaagcgtggcgacgagctgaagcccggccagaatgcgtacctgatcgacacgcggcagaccaacaagctgccgaagggcaccgggttcgtcgtgtccaagctgaccagtgaagacggctcccgtctgatcgtcagcacggacggcaacggctccgtcctgtacgccaccagccacgacatcttcgaggtctgggaataaccaagcgaggatagcatgagcgatacccttcccgacaacgactggctaccacatgccgagcgcctgcctgttggtggccgcacacgtgtggcccatgagtgcggggagggtacgcccttgcttatctcacgagagcacgacaagtccaccgcattctgtttcaggtgcggtggcacaggattcaagcgtgagcacgagagtatcgaggccaagcttgcacgaatccacgccgagcagacgagcgaacgcagagtgcgtgcgactgttgagttgccagagccacgggtatacgacacccgcgagtggccgctcgacgctaaggtgtggttcttcaagatgggactctcgcttcagatgatcgagaagctgcggctgtactggtgcccaagcatcgggcgggtggtactaccgatcactgaaggcgacaacgtggtatactggacagcccggtcggcaacgagacagccgaagtggctaacacctgacgttccgaaagacggacttgtcgcacgctacggcgtgggcacaggtgacaccatcgtactgtgcgaagacccgctcagtgcatacaaggtgggactggtaaccgaagcgtggtcgttgctcggcaccaagctgcacaacaaagtgttgaagcagctgactgatcgaggccaacgtgtagcgacgtggctcgatgacgacagaggtagaagcaacggtagcaatcccggccaagacagtgcgcgagtaatcgctgcgcgtctacgtgcgtttggtctggactacaggaacatcacgtcaccacgtgacccgaagtattacacgaccgactacatcaaggagaagctgcaatgagcaaacccatcgtgcgctaccggcgcgctatcatcccgcccgtcgttggcttccgtgccacgctcggcggcgtgcttgcgcatccgaacctcggcgactgcgacatcgtgcacacctcgacggtgctgtatgtggcggacggcgggcgcaagttcgagacgcgcaacacccggtatcaccagctcgattccaagtacgaacccgaaggagaacctgatgagtcttgacaccacgctgctgcggttgtgcaccaaccgtggcaagttcgaccggctggtacccagcgcaccacgtgatgggctggacgagctgaccgtgctgatgctcgatgcgttgcgtgcgtactacaaggagttcccggacacgaaggacttgccgttcgatgtgttcgatggctgggccatggagttcaagtggaagacgcagcccgacgacaagaagtccctgctcaaagttctgctgaagcagatgcgcgagccggtcccgcccgaggcagagcagggcatgatcgagaagctgttggagttggagcttgccaccactgcggtcagcaagatcgtgcagtggaatggcggcgctgagttcagcctgcgcgacgagctgtacggcttggccgagacgatcaccgaccgaatggatcgcaaggcgcggctcccgctggtgcaggagacgcccgaggaactgatgcagatggacgagcacgacatcggcatccacttccgactgcccacgttggcgaagaacctgcgcgctctgcgtggtggtgacttcggcatctacgccatgcgtcccgacgcaggcaagaccacgttcctgaccagcgagtccagccactggatcacgcagctcgacaacgtttggccggaccagaagcgcaccggcatctggctcaacaacgaggggccgggcaagcgcatcaagcagcggtggtatcagtcgctgctcggcgctaccatccctgagatggtggagtgggcgaaggatggtagcatccgcaagcgcatcgaagatgcgatgggcggggacatccaccgcatgcagttctacgacatccacgggttcaactccggtgaagtcgaggccatcatcaagcagaccaaccccggcttcatcatcttcgacatgatcgacaacatcacgttcaccggtggcatgaccaacggcgggcagcgtaccgatcagatgttggaggcgatgtatcaggccgctcgcaactggtgtgtgaagtacgacgccgtgggcgtggcgacttcgcagatcagcgccgagggtgagggaatccagtacccgccgcagtccgcactgaaggacagcaagaccggcaagcagggtgcgtgcgacttcatcatcatgggcggcaagctcaatgacccagcgatggaacgcttccgctacatcggcaccccgaagaacaagctgcaccgcgcaggcggcaagcgtgacgttcgggaagaagtgatgatggatgcagagcgtgcccgcttctatcaggaggcagcatgagcaagccaattcacatcgtagccaccgggttcacggtgtcggtcagcttccccggtgaatccaccgaggcgaagaccttcaactgcgtgagcaacgcgcaagcaatccaccttgccaagctgctgcgcaaggtgcacgacgcaggctacatcgaaggccgcaacgacgcgccgcagtggaagtggggatggctgcggaacaaacacagcacttggatcggcgtgcactactcgccgcacaacaagcgctggtgcatcaatctgatcccgtgcttcacgttctggatcaccaagcccggaggtaacacaccgtgagtaccgaaccgaacatctacctgccgcgcaacgtgggcgtcatcacgtccagccgcaccggcagcagctacacagtcgagccgcccgtgaccgacacggacatcgacttcctcgtgctggtgcaggacttccacgaggccatcgaaaagctggtcgatcagggatggaccctgtgctccggtgccgatggacactacgaggaggacgaggactacagcaccacgtggtatgcgctgcgcaacggcgtgttcaacgtcatggtgaccgccgactccggctggtatcagcgcgcggtcgaggccaccaccatctgcaagcgccgcaacatcaaggacaagcaggaccgcatcatcgtgttccgttgggtgcgcgacgggctggacttggatggcgatgcgtcggatgaaatgtaccagctggccctgcaacggtggccgctgtgagcttcacttccttcgacctcgaaaccacgatccgttccatcctgaagcgcaaggccaatccgttctacgacatgaacaagatcgtggcgattggctacaagcggaagggtgacgcacggaacaccggcctgtactacgacacccgagtcgggatagacaaccagtacatgggcggcgcacccgatgggtggctgcgtgagctgtgttacgggcagcagttcctcgtcgggttcaacatcaagttcgacatcctgcacgccatctgccaaggcccactcaaccggcaggcatggatcgagttcatcgacggcggcggcatggtgtgggactgccagcttgcggagtacctgctgcacggcatgacgcaagagttccacatggcgagcatggacgagacggctccacgctacggcggcaacttgaaggacgatgcagtcaagtccctgtgggctgcgggcgtggacacctgcgacatcgacaagacgctgctgatggattacctcctcggcaccaacgacaccgacgacgtgggcgacatcggtaacaccgagaagatgttcctcggacagctcgccgccttccgtgcacgtggtggtctgcgctcggcgctcctcaacatgggtgcgctgtgcttcaccatcgaagccgagtacaacggcatgtacgtggacaaggactgggcgcttacgaaggcgaaggagttggaggtcgagcttgcaacggcgaccgccgaactcaacggcttcatccccgagctgcccgagggcctgaccttcaactggaacagccgcttccacaagagcgcgctgatcttcggcggcaaggtgaagtacacggccaaggttccgatcatgtccaccgagggtgggccgacttacgtgcagaaggacgaggtgcactacgtgctggtcgatggtaccacgacggcgacgccaccggccgaggacttcgacaacctctggcgctacaccacgtacggcagcggcaagaacaagggagagtacaagaccaagaaggtgaaggtcgatgacttgaccaagcagaagttccgcaacgaggacatgctgttcgagttccctggctacaccgagcctgatgctgcatgggaaagcaagagcgatcccggcgtgtactccaccgctgccgacgtgatcgaggcgctgggctaccgcaacctgccgttcaccaaggcgcttgccagacgcgacgacatccacaaggacttgtccacgtactacatcacgacggacgagaagaccggagagcagaagggcatgctcacgctggtgggaccggacggcatcatccaccacaagctcaacatgaccaacacggttaccggccgcttgtcttccagcgatccgaacttgcagaacgtgagcaagggcgagctggacgaggagacgttggaggagaagggttcgcagatcaagcgcgccttcgtgtcccggcaccggggtggcaagatcatccagtcggactacacctccctcgaaatctacgtgcaggcaatcctcaccgagtgccgtcagctgatcgaggacttgaagcagggcctcgacatgcactgcctccgtgcagagcaggcgtggggtgagcaaggcaagtacgactacgacttcatcctgaaggcgagcaaggacgacaagcatcccgagcacaagaagtggaagaagaagcgcggcaacgcgaaggtgttctccttccagcgtgcgtacggtgcgggcgtggcgaagatcgctgcgaccaccggcatgtcggaggaagaagtcgaggcgctggtgcgcggtgaggccgagcgttacccggagctgggcgagtacatcgaccgcatggtcgagcacatcaagcgcaaccgcgtcagcactcagcgcttcgttccgcatcccaacgcggggcagcaaggcgtgccgcatgggctgacgtgtcagcttggccggtcgcactggaccacgccggacggcaagatgtattccttcagcgagtcaccgtccccggtgttcatcgccaacaagcccgcgagcaagggtggctgtgcgcagtcgttctcgcccacggaaatcaagaactacccgatgcaaggcaccggtggtgaatgggccaaggcggcgatgtacgtcagcctgcgcgccttctaccggaagtacgtgaccgaaccgaaggaatggttgggccgtgcgttgctcgtgaatcaggtgcacgatgccgtctacgtggatgcacacggcgacatcgcaaccaaggccgctgctctgctgcacgcctcgatgctggaagcgtcggtgtatatggagtggtggttcaactggacgctgccgcttggcgtcccgtgtgaaaccaagatgggcgacaacatgatggaggagaagaaccctcccgcagagttcgccggtctggtcatcgagtaccgcgcgtcgatccgcaaggacttcgtaggtaatcacaacccgtcgtttgaataaggagaacaacacgcatgagtcttgacgcactgttgaacaaggtcgccacgcagggtaaggatcagtcggtcgccagtggtggcagcttcgactacaccccgcccgctgccggtgtgaccaccgcccgcatcgtcgggtactacgagctgggcaagcacgagttcgagttcgagggcaagaagaagacgcaggatgaagtcgccatcgtgttcgagctgaccggtaagcagcacccgcacatcgaaaccgacaatggtccggtgccggtgcgcatgacgctgaccctcggcctgtccaccaacgagaaggcgcactacttcaaaatcttcagccgcctgcgcaccgaggagcgccacttcgtgcagctgctgggtcagggtgtgctgctggaagtcatccacaagccgggcaagcgcgacccgaacaagaccttcgccgaaatcgacaaggcttccatccgcaagccggtcatgccggtgccggaaatggagaacggcatcccgaccggcaagttcgtggacaccgtgatcccggtgccgcagcagatcaccccgctgggtgcgttcgtgtgggacttcgccgacgccgacatgtgggacagcatctacatccccggcgagtacccggagcgcaaggacgagaagaccggcaaggtcacccacgaggcgcagtcgaagaacaagacgcagctgcgcatcgctgcggcgctgaacttcaagggtcttccgtgctacgactacgccgccgccaagttggcgggcagcaccacggtcaccaaggaaggcgtcgatgcgctggacgaagtggtcggcgacgtggcgaacgccgcgcccaccgacgctgctccggccgacgacaagccgccgttcccggtggacggtagcgacccgatggcaggcatcgcctgatggacctgagcgctctcatggcagcggccggtgagcgctccccgatgccggtgcaggtggtacgtcagcacaacccgcgcgtgatcgctcacgttgatggggactacatggcgtacttcgcggctggtagcgagaactgctcggcgggggatgcacgacgcaacgtgctctcccgctgcgcacagctgaagcatgtcagcggagcgggcaagatcgtcatgcacctgacgcacgccgcgtctaccaagggtgatcgcttcctcgctgctaccacgcagccgtatcagggtcagcgccaagcaggccgcaagcccaacaactgggcgttccttcgtgagtggatggagacatacgagggcgacgctttcactcccaaaatctggctgacccgtgaggccgacgatggcatcgcgtacgtcaacgagggtgcagcattgcaccacaacatcctgcacgtggtgcacagcgccgacaaggacatgcgaatgttctgcggcgtgcacgtagactgggacggctacgacatcacagaggttccgctcggcgcttacgacatcgttggcgagaacggattgcagtacggtcacaagtggttctggatgcagatgctccacggcgacaccgccgacaacataccgggtctgccgaaggtgggcaaggtgacagcggagcagctgctgttcgagacgaagaccaacctcgaagcggtgcagatcgtgagcggcaagtacagcgaagtgttgggtgccgactggcgcaagacattcgccgagcaagccgtgctgctgtggatgcggacggatcgtgacgcagaactgctcgacgtgctgaagctcgacgtgttcgggccgaagctgaagcaggcgttctatgacctcgccgaggacgtgaacgagaagcgtgcaatcttggaggcatacaaagcatgaagcgactcactgcaacacaggtcaagctgctgcgcatcaagctcgcagcggagcaaggcaaccggtgctgtctctgtcagggacagttcggcctgaaggctccgctcgatccggtgctggaccatgaccacaagaccggcgctgtgcgcggggtgctccatcgcggatgcaactccctgctcggcaaggtcgagaacaacgcaggccggtacggcgtgcgcgacgtgttcgcattctgtgcgggcatccccaactacctgcggtcgcacctcaccaacatcacggggtacctgcatcctacctacaagaccgacgacgagaagcgtatcgctcgcaatgcgaaagcgcgaaagcgtcgggctatcaacaaggagacaccgtgacccttacccagttcattcgccgagcaccgaagcgcggcccgaagattctctgcctcgacatcgagacgttccccatcgagttctatggctggggcatgttcaacaacaacttcagcgtcaagcagatcaagcgtgactggtcgctgatgtcgttcgcttgcgaatggctggacgacgaggcgtcgttctacatggaccagcgcaacgtgcgcgacgtgttcgatgatcgcaagcagggcaaggcgctgtgggcactgctcaacgccgccgacttcgtgctcgctcgcaacggcaagaagttcgaccttcgcaagatcaaggctcgcctcgcaatcctcggcctgccgcccgtgtctccggtgcaggtgatcgacccgatgctgctgaaccgcaccgagttcgccttcacctcgcagaagttggagtacaccaccggcgtgatcgtgccggagctgcgcaagtacgaccaccacaacttccccggcttcgacctgtgggtggcctgcatgcagagcctgcccggagcatgggacgagtgcgaagcgtacaaccgcatcgacgtgaagtccatgaagttggagtacaagaagctgcgcggttggtactcgcagcatccgaacgtcgcagtgtactacaaggccgacggcagcgagcaccgctgcaacaagtgcggctgcaacgaaatgatcccgcaggatgatccggcccgcacgcaggtcggtacctacctcctgcttcagtgcaccgtgtgcgacggctacagccgtgggcgcaagctcacgaccagcgccgaggcgcgcaagcacatcaccgtcccggcataaggaaccgacatgaagatcaccgacatccgcagcggcatgcgggtacagtacatcggcaatgcgcccgcaatgatcgggctgcgtggacaggtaagccgcgtgttcgctcgtgatgtcgaggtcttcttcgacggtcgagttaagccgagctgctgcgttcccgattccctccgacagcttctcagcatcggaggcgtgaccaccaccagacgagaggtaccaatgcccgaactgagctaccgcgacgaggaccgtcgcacactgtccgaccgtggcgtcggcctgaaggatgacgggggcaagccgcaggcccgtctgctgcatgagggcgtgccgcgtgcactggcccgagtcatcgacaccctgaccttcggcgcgcagaagtacaaagcgcactcgtggcagcatgtcgagaaggcgctcgaacggtatcaggacgcgagctaccgacacgacaacaagcgctgcctcggcgagaagctggacccggagacgggcatccaccaccgggcgcaccacatcatcaacgagctgttcctgttggagctggaactgcgcgaggaggagaaggccagtggcgcagagtaaggcgcgctccatcaaagaggcttgggtgaacatcggcatcggctacagcatcaactacgcagcgaacatcgcgctgcttccggtgctgtggcatcccgagcatccgctgctgtcggcgcacgccatcggcattgcgttcacagcgatcagcttcatccgccagtacatcatccgccgctggttcagcaagggtgactgatggcctgcgcccgctgcggccaagtgcatcggtacgtcccacatgaggccgagtgggcgcgcttcctagaggagcaccgtacccgcaagcagttcgatgtcgagtgggccaactcactctggcatcgtacataccctgacgacgcattctgcatcctcgtgatgaggggcctcgcaggtttcgttccattcccgtcgaaggagaactgaatgctctacaagaaccagaccgccatgctcatcaagtcctacgagaacgccgttgcgtggggcgagagtgccgaccacgaggaggcattgcagaatgcggtcaaggccgggttcccgaacctgcccgacgaagatcaggccgagctgtatacccgcatcgccgatgcgtgggaaggctaccgtggttcgctcgctccgcgcaagctgtggatcggcaccatcgtcaaccagttcatgtcgtcccgcatcgcacggttcaacgccgcgctgggtgacggcaccaagaaggaggacagcgccgatgtttgatgtgcctcgccagaatgtccgggttgctcccggctacaagaagcgcaagcgcggcttcaagatcaaccgcgccttcaccaagggcaacttccgcgtgcagtggtacgacggcaaggccacgtactgggagcgctacgttccgtggtacgaagtgccgctcgccatgttccagatttggagggactacgcatgagctacatcgtccacaaggcagtcgagcaggacaagatcaagaagaagctgcggcccaccgaggagcagcttcgcaccgagtacatcgcacagccgaagtacgacggctgcaacatggtcgccatcaagcgcggccactgggtgcccacggtgaacaagggcctgcatgccatcaaggtgggcgacgtgcagatgcagccggtggatcgtggcgtggttgacctgttctcccgcaccggtgagcaggtcgtcagcgcacaccacatcgagaacgctctcgcatccgcgccgttcttcccggtcggcgtgtacttcggcgaatactggcacccgcagatcgaccagcccaccgtcagcggcatgttccgcaagaaggacggcacgcagtacaccgagccgatgttcgtggtgttcgacttcgtgacgctggaagaatgggagcagggtttcagcgacctcgtgtatcaggagcgcgtcagccgcctgccgagcatgggccacgccatcgccgagggcaccgcgccggtgttctacgccgagtcgcagggcttcctgatcgaccaagagctgggcagcatggaagcggcgaagctgctgtgcgagggcggcgcgtacgacgggctgatcctgcgcaagccgagcggcaagtgggtgaagggcgacaagggaaccaacggcgaagtcgtcaagatcaagccgaccctgacgctggacctgcgtgtgctcggcatcaacgaagcagtcggcgagaagaccggccgcgccgtgtacacggtcgtcgttgacctcggagaaggcaagacgcaggaggttggcagcggcgtgccgcacagcgagagcgagctgcctagcgtgggaggcatcgtggaaatcgaggcgatgtccttcagcaagtacggcctgctgcgcgagccgcgatacaagggcatccgtcacgacaagaaggaggcagacctgtgagcgtcgaggtgcaagcatggcacaacatggagcgcgacacggtggagctgcgcatcagcgttcctttcggcgagtacgccggttccctgtggccgaacgagacgctgcgcgacaaggtgcaggaagcgttcgccaagttccttgacgagcggaggggctgatggacgcgatcactttcgagaagccggagctggacttcagccagtcctcggcatggatgggccgcgtcgaggtttcggtgcgcgcccggtacggtgccgacttgttcggcgctgctgccacgtgcatggccgaggatatcggcggtgaggcgtggccgcacatcatccacgacctgcacatggaaatcatgcgcggtatcctgaaacgctacccgccgcgcgactacaccgtgcggcagcaacggaggtaacaatgctctcgcaagtggaactcgaactggaaacctacgccttcggtaaggagcgcatggagaagtccatcgcccgcaacgaggagaagggcggcgcggacaacaacccctacgcccaagcagtgtatcgccggttcgtgcttccgcttgcggagcgcatccgtgcggacatcgactctccgcgaatcggccgtgcgcaagcgcacgtgccacttctgcgcgccaagtacgatcccgagcgtcagaacaagcgtggacagcccgtcagcgccgaggaacaggcacgcgagtggtacgaggctgtggccttcgtcgccgttcgcggtgcccttacctcctgcatgcgagacaagcacggcgaaggcagcgaccgcgacgtgttgaagaacgttggcatcaacgtgtaccatgagtacctgctgacgcagttcgccgacgcggagccgactctgttctaccacctgatgaacgacatggaccgcaagctctctgtcaacgagaaccaccgcatgacggtgatgaagatgcaaggacgcaagaacggcatcgagttcgtggagtggggacaggcacagcgcgatcaggtcggcgcgtacctgtgcgatcagcttgcgcagctgggcatgttggagattggcgtggtcaccgagactgctgccagtgcaggcgcagcgtaccgcaagttccagaccaagacgcacgtcaagatcgtgctgaccgacgaggtgcgcaagctgattactcagatcagcgacttcgtgatcgaggccacgccgttctacctgccgtgcgtcgagccgccgatggactgggtggacatcgacaacggtggattccacacgaaggaaatgcgccgactcaatccgtggatggtgaagacctacgctcagacccgcgacgagtaccgcgctgccgagctgcgcaacgagatggctgcgatcaacgcattgcagcgcgtgccgtggcgcatcaacaagcgactgatggaagctgtgtcggccatcgccaaggtgcacgacatggaggaaatcatttctcagggcgagctgccgaagccgcgcaagccggagtggctgacgaaggacatgaccaaggaaaccatgtcccacaatcaggagttggagttcaagcagtggaagcgcgacatgtccaactggcacaccgacgagcgcctgcgacagaacaagggcaatcgtttctacaacgcaatgaaggtggcgcgcaagttcgccgagtacccgagcatctacttcgtgtacttcgctgacttccgtggccgcaagtacgttcagaccaccggcgtgtcgccgcagggttcggacttgcagaaggcgctcttggagttcgccgatggcaagccgctgctgactaaggacgcgaaggattggttctgcatcacaggagcaaaccgatggggatacgacaaggcgtctctgccggatcgtgtgaagtgggtagcggagcatcacgaccagatcatggcgttcgctgcggacccggtgaacaacgacgagtggaagaccgccgacaagccgctgcaatttctgagctggtgcatggagtacgagcagtggcaagtgttcggggatcgcttcctgagccgcatcgcagtcggcatggacggttcgtgcaatgggcttcagaacttctcggcgatgctgcgcgacgcagcaggcggcgtggcgacgaacctgatcccagcaccgctgccgaatgacatctaccagatggtggcagaccgcgtgactgccgtcctgctaggcgaggacgaggatgccgaagggtaccgcacgctgtggctcgaccacggcctcacacgctcgctggtgaagcgcagcgtgatgaccctgccgtacggctcgcggcagtcctcgtgggcggacttcatcatcgaagactacctgaagtgtgggaagttcccctcgctcgacaaggccctgtacggccccgcagcgcgcttcctgagcaagcgcatgggtgaggccatcgccgacaccgtggtcgccgcagcgggcgcgatggagtggttgcagcgcggctccgggtcgatcctcaaccaagggtacgaccgcatccggtggatcacgccgtccgggttcccggtggtgcaggtctactgggagtccgaggagcaccgcatcaacaccaagctgtgcggcaacgccaagctgtccctgcgcaagagcacggacgcggtgaagaagtcccggcaccgcaacggcatcgccccgaacttcgtgcacagcctcgacgcaagccacctgacgctggtggtcaacgcggccaaggccgaaggcatcgacgccttcgccatgattcacgacgacttcggcacccacgccgccgacagcgcggcactgtaccggatcatccgggaggtgttcgtgtcgatgtacgagcggcacgacgtgctgtcggccttccactcggcctacccgttcctgccggagccgccgccgatgggcgagctggaccttcggcaagtccttgattctccgtacttcttcagctgacggagtttcagtacacctatagcacgaggcaactgaggtccggttggagcggccgcgaaggtaagcggaaccggtgccggaccttttggtacacctatagcacagaggagacaccatggccgaagacgccaaagtgaaagtcctgatgacgctccacccgaaccagctggccgccgtgcggaagctgtccgggctgtcgctgtccgtcaactcgaataccacgcccttggaggcaggtatgcagttggggatggcccgcgtcctgaacatcttacaggagggtttcaccgttgattcctccgtaccgaacaccaacgacgggtgatagtgagcagatcaaggcggctttaacggccgctttgtatctgtcatctagagaagatagtaaggtagacaacagagaatcttctgtgagctacaactgtgatgaccctgattacacagtggccctgataacacagggtctagtggatgcagtaatcattgatgaagcctacctgctgtgctttgccattgtcacaccgtggtactccaagaaccgtactacgttcgttgagaacatggtgctgcgaattgggccgggcagttccttcgaccggtacatagccgtgatggaacatctggctgacatcaaccactgcgactcactgagcgcaggcggtgcactagctcggaactcccgagcactcacacggatgtatgcacgctacggctacctgctggaacggcatgctccccaattcaccaagcgaaggagttaacctatgggtagcatcgttggtggtgggtccgccaagcgagcagcgctgaagcaagctgctgctatcgacaagcagaccaacctccaaactcaatccacgaactaccagattcaggcgatggccgatcagatggcacaggcagctgcacagcaggccgcatctgagtacgccgagaagttgctgagtgcccccgtcgataccgtcgatgtgcggctgggaacttccgacctcgacttgcagactgccgacctgatcggccgacgcaagaccgcccgctccacttacacccgacccgtgaccacgaccgcagcttcccggctgacgaccgtggccgggtcagacctgttgtgaggtgagcatggaccatccgatccaaaccgctcaccgccagttcgaggcttacgacaacaagcgacagggcatcatgtaccgactcgaacgctattcgagctggaccgtgcccaagctgttccctcgcaagaaccgcgatcaggacaccgagccgctgacccacgggttccagtctctcggcgcgcaggcagtgaaccatctggcgaacaagctgatgatgtcgctgttcgcaccgtcccgcccgttcttccggttggagctgaagcgcaaggcgaagcaggctgcgcaggagcaaggcgctgacttgcaggccatgcaggcgatgcttgcgaaggccgagcaggatgccagtctcgaactggacaagcgctccatccgctcccggctgtacgacctgctgaagatgctgatcgtgctgggcaacgccctcatggtgttggagaaggacacgatccgcgtgctcaacatgcggcactacgtggtcaagcgcacccgcaccggcgaggtctacgaactgatccttcgggagaaggtgcacaagacccagctggaacccgcagcgctcgctgccattgtcgcgcacccggacttcaagcccgatgacgacggcatggtgtgggagtacaagtgggtcaagctggaccacaagaccggcaagtacaacgaagacgtgtggatttgcaactgcaagctgcccgccaacttctcctcgacctacaccgcagacaagctgccctaccgggcggttagctgggacttggccgcaggcgatgactacggctccggcttggtcgaagactacgaggccgacttccagtcgctctcgatgctgtccgaggccgcagtgcagggcgcgatcctcgcctccgagttccggtggctggttaaccccgcaggtcagacctccgtcgaggacttcatggcgtcgcccaatggcgcggccattcccggcatgaagggtgacatcgagctgattaacgcaggcgtcgatggcgtgctgcaaaccaaccaagcaatccagtccacctacatcaaccgcatcggcgcaggcttcctgttgcagacggcggtgactcgtcaggcggaacgtgtgaccgcgcaggaaatccgcatggtcgccgaagaactggaaggcgggctgggtggcggctactcccggatcgctgcggacgtgcaggtaccagtcgccttttgggtgatgaacctgacgggccgcgacatccgaggcaaggacttggagcctgtcatcatcaccggcttggccgcgctctcccgtacgggtgaccgtgaccggctgttggagttcggcagcaacctcgccaacgtcctcgcactgccgccgcagattctcgaacgactgaagctgtccgcgtggatcgcagacctcgccgccgctggtggcttggacccgaacgtctacgtgctgactgaggccgagtacggccagatgatgcagcagcgtgcacagcagcagctcgccatgcagaacgcatcccagcagatcgacaacgccaacaacatggagacacagacacaatgagttccaacgcacctccgggcggtggtcccggcgcaaccgtgatcgcaacctcgaacggcaaccagcccgcaccggcagctccggctcccgcagacgacaagctgttgcccaacggccagcccgctccggccgcaccggcacagcccgcagctcctgctgcacctccggctgctgacgcgctgagtctcgaacctgccgctcccgcacagcccgccgccccggcgaacgctgcgccgactgcggtgtcgatcccggactacggcgacaacggcctgaacatcgcggccgaatacttcgtcaacaccgtgggcctcgacatcgacagccgcgaactgaccgaagcagcgaagggcaacttcgccctgctggaagccaagctggaagtcctcggcgacaaggccaagggttccgcaccgatcctcgctctggcgaaggagagcatcgctcgtgtcaccgccgctgcaaccgcagcgcacgccgcgaacgttgctgctgtccacgaagccgtgggtggcgcagagaactgggctgcgatccagcagttcgcacgggccaacctgcccgccgaccaactgaagcaggcaagcgaatcgctgtcggctggtggcttcggcgctcaggcgaccgcgcgttacctgatggctctggcacaggccaatcccgcgacgaccgtcaagggcgcaccggctaccaacgccgccgcccccgccgcgtcgatcaacggcgtcgctcctatcacgaaggagcagtaccgcgctgagtaccgcaagctggttgccgagaagggcatccgtggtgcggcccactccgaagaactgcgtgcactcaacgcgcgcgtcatccactaagaccaaggagcaacacaaagcatgagcaccatcttcccgactgtcccggttctgccgaatcaggtcaaccagtccggcaacgagaacgccctgatcctcgaacagttcaccggcgatgtcgagcacacctacgtgtccagctcggtgctggaaaagttcttcccgcgcaagcaggtcaagggcaccaacaccctgaccaagaaggccatcggccgtaccaagcttcagaagctgaagcgcggtgacgcgccggacggcaccccggtggacttcagcaaggcgtcggtgaccgtcgataccatgctgctgtcgcgtcacagcatctggcagctggacgaaatcttcaccgacatcgacacccgcaaggaaatcgccatcgagcagggtcaggaaatcgccgagttcgtggacctgaccatcagcatcgccgccgcgaaggccgctgctgccacgcagtcgatcttcacccgcaacggccgcgcgcccgagggccacttcggtgccacgcaggtcgtgctgtccgccgctggtgacgagaacgatccggccaaggtgtacgccgccatcggcaaactgttctcccgcatggaggaggagaagaaggtcaagccgcagcgcgatggcgtggtcctgatcgtgcgcccggcgatcttctacctgttgcagcaggccgagcagatcagcaacggcgagtacctgacctcggacggcaacaagctgaccggcatcccgaccttccacggctggggcgtcccggtgctgtcgagcgagaacctgccgaacaccgtgatcgaaggtcacctgctgtcgaacgacgacaacgacgacttctacgacggcgacttcagcaccctgatcgccgtggccgtgtcgccgaaggccctgctgatcgccgaagcgctgccgttgcagtcctcggtgtggtggagcgatgcctcgaagtgctacttcgtggactcgtggatgtccttcgccgttggtctggatcgcgtcgagaacgcgggccgcatcgacaaggttgcctaatccgctgggcgcggtccctgaatccttcgggtaactcaaaccgcgcccttcttccaccaacacaggagcaacatcatggtctttgaccgaccgttcgagatttccaaccgcgtcgtcgccgcaactggcgtggccggtctgcccgccaactccgttggtaccgtcgtcggcgtccactacgacacccgtggcaccgcaggctgggtcgtccgtgtccgtttcgtggacgacgaaatcggctcgcaggacatcgagtacgcaccggccgctctggctctggctgcggactaagcaacatcccggcaggggcgctccggcgtctctgccttgttcctctcaggagacaccatggcattcatcaccaagctcgacatcgtgaacgcctgcttgaagacgatgggcgagacgaagctcaacacgctggaagatgaccacgtatacaaggacgacgccgttgacttgatcgaccgcgtgcaccgtgacgtgtcctcactctcgctgtggttcaacaccgaatgggtggagctgaagccgcaggcaacgagcaagtacatcatggtccccacggacgtgctgaagctggactgcaacccgagccggttcggccacgtggtgcagcgcggacgccgactgtacgaccgcaagcgcaacacctacgagttcgaccacaacgtgcaggccaagctggtgcggctgctggacttcgatgacctcccctacgaggtgcagatgttcgtgcgcgacgactcggtgctgcggttccagtctgacttcgacggcgacaacaccaagtacgccaagatcaagcagcagcgcgatgacagttacatcaacttgaaggccgagcacatccgccagatcaaggcgaacccgctgttcgctcgcgcatccgtggacgtgctgcgttcccgttactggaactacagcggtcacccgtggcacagccacgtcacattccccggctaaggagacaacatggcaaaggcaggcggaacctatcccgacatccttcagggtgtcagtcagaaaccggcgcatcgtcgtcggccgggacagacgcacgagcagatcaacgtgctgtccgatccggtgaacggcctcgtgcgccgtcgtggtacgcggttcgctgcttcccaagccgttgtcacctcggccgagctgcgcaacatggacgtgttcgacttcatgcaggagggcaaggagtacgcgctgctgtaccggcgcgacgcctcgaccttgggcagcgagtccttcgcgttcctctacaacaagacggacgagtcgttcatccctctggtgtacgagaacagcacgtgggtcaacacgctggtcagcggaggcgcatcgtcgctcacggccatcggcagctacgtctacatcgcgggcaacaccacgatcccctcggccaccagcacgaacgtgtggcaggagcagacgaacatccagcgcctcgcagcatgggtgcgcaccgggaagtacaacaccacgtacacggtgaacctgacgcggacggacaacacggtgctgacggtaacgttcaagacggttaccgcatcgtaccccggaacgctcgacaccagcgacatcccgttctaccttcccggtggcacggagccggacgcggcgtaccagaagtacgtcaacgaccgagtgaacgagtacaactctgcggtcaacgagtggatcgtgacgagcgctgagcagacgcgcccggagtacatcgcggagcagctgtcggatttgctggtcgatgcaggcgtgtcggcaacgtacatcaagggcgggatcatcattgacgatgaccagttcaaggacatcacggttgacgacgagggagacggcacgaccttctacgccgcagggcaggaaattacagacgcgacctacgccgtcaagttccactggcacggcaaggtcattcgcgtgcggccgagtggtgcaggcgcggacgagtcgtactacctgcgcgctgagttggagaacggcgagacttccggctacgggtcggtggactggtacgaagcgcccggcgtggagtgcaccatcgacaacctcgtgtcgcagctctacatctacaacggtgtaggctacatcgcacgcaacggtgcgggcctcacgtctctggctccgagcagcggcgagcatccggcctacggtgcgcgagtggcaggcgatggtctgacctcgccgatcccgtggttcatcgacaagccgatcacgatgctgtccgtcttccaagaccggctggtcatcggcgcacagaactacgtcaacgcctcacgctcggcggactacctgaacttctggcgcggctcggccgtcaccatcgaagacagcgaccccatcgaaatcttcgcgcacggcagcgagggcgatgtgctccggcacgcgacgctctacaacggcaacctcgtgatcttcggtgaccgtcagcagtacggcatcagcggcgactcggtgttcagtccgaagaatccgctgattaaagcgttcagtgccaacaaggattcggttgacgcgaaggcgcagacctcgggcaactacatcttttatgcgcagtacggcagcgaaggcacgagcctgcaccagatgcgagtgggcgcgctcaacgggcagcagacggtgacggacgaaatgtccaacgagctggactcgtggctgtcgggcactccgttgcagatcaccccgctcactgcgccgaacctcgtcatgttccgcactcgcgagcacccgcaggacttctacctgtaccggtacgaggacaacaagaacaacgggcagcgcatcgtggatgcgtggtcgaagttccggtaccacccggcgctgggcgaaatcatcggcgtgagcagctacaagaagaacggcctcgtgttcactgcgcgcgggtcgctggtggcgtgcgacgtgttcgacccgaagggcgagccggactcgcatgcgtgcctcgacagctgggcgagttttggtacacctacgggcgtacagactgcgagcgcaagcatcgccgtcaatagcactagcccgtacttcctgctgggttgtccctacgcgcaggcgtctgacttccttaaccagttcgatgacctcgctgctggtgcgctggaatacggcgtggtgtccgaagctctggtgatcccgaccaatccgttccctcgggaccagaacggtcaggccgtactcgatggacgcatgtccctcaacaaggtgacggtggacgtggagaacacggcaggcatgatcgccacggtggcaacccgcaacagcaatgtgaccactacggacttcgagggccgcatcctcggcgactccgacaatctgatcgcgcggcaaccggtgtaccgggggcagctcaacatcagcgtcgggcgcgaagtgcgcgagtgcacctacgagattcgcagcaaggattggctcccgctccgggtgaccggcctgagctggacgggtcagactttcaacaatgtacggagggttagctaatgggttcggttaatacgatcctgcaagcgaacaacaccacccgcgttgcccgtgcgaactaccgtgcagccgttgcgcagaccgacaaccagaaccgcagcgaggtcgccaagaccggcttcgctgatttcatgcggtccctgaagaacaacgcccaactggacgccgccgcgaaggagtacaactccaacatggaagcgctgtccgaggagctgcgtgcgcgccaaggggctgggcttaactcccagctccaactggcgaacgcgcgtggcgcacttcaggcgcaggctggtgctgtcggtgtcggcggctcgtccgcagacctgatggattcgatggtgcggttgcaggcggaaatggatcaggagacgcaggccaacgctgtctcgctcctcgcctcgcggggcgcatcgcagactgcgcagatcatgtcgcgcgcgtggaacgggatggacatgagccgttcgttcgggcagttcgactactcgcagcacatcgagccgcaggcaatgaagcgtcgcttgggcaagctgatcggcgtggccgtggctacctacttcggtgggccgatggcaggcgaggccgtggcagacttcgcggtcggcacgtggcaggcggacaacggcaacttcactggtgcctctcagtccttcagcaacgcagcgcagaacggtatgcaggcgtggcagcagtccaatgatcgcggcggcaagtcgtgggcgtccactaccttcgggtacaacgacggcaccggcaagcagtccgtgactggggcgaaggtcaccggcaacttcggcaacaactacgacaacttctccaccactacgtccggcctcggctggttcgatagcggcagcggaggcaactcaggaggtgcatggtaatggctgacatcggcacggttaccttcaacacgcagtccgcattgcagggtggcatcaacgccaccccagcactgtcgggcaacaccagcattcaaggcgctggtgtgaatcaggtcgggccggttcaatccggcaacgactggttcgcaagcactggtggtatgacgatgccggacagcaacctgccagagttcttgcaggagctggcagcgccgaacaccgccaagctgaagcagcagcagatgtgggacggcttcgttgccgcccgcgctggtaagaccatggacgagattgctgcgaccgaaccgtggtacaagaaaatcttcggagacaccaactacgagattggcgcgagcatgtataacacgctctcgcaggtcaacgaaatggagagcgacttgcttcggcgtatgccggagttgcgtcagcttcctcccgaggcgatggcgaaggagttcaacgacctcgccactgcccgcatgaccggcaacggtttcgcggacacggtgttgcagaagaccttcatggatcgcgcgggttccctcatggacctgcacaccaaggagcgcacggcatggcagcagcaggagctggtgaaggcgcagtacgctgcgaactcgtcggcgtccaccggcttcaacgaactggcgaagcgcacggcgatgctcggtaccaaccgtcccatggacgagaaggccaccgaggcgctgacgcaggcgcagctgtccctgctggacggactgtcgccctcgcgctaccagacggacgagtcgtacaagtccgcgatcactgcgttctatcgtggcgctgcggatcgcggcgagttccacacgctgaagttcctcaacagcaagggcgttctgaacgccatcgacccggacgggcagctgggaatccagcagtacgtgaagcaggcgcaggatcgttaccgttccgactggctcgatgccaacccggagcaggccgagaagatggcgctcgtctccatgtacgcatcggagggcattggtgccaagccgtcgcaggcgatgatcgaggaaatgaactcgacctacgccgccgagactggaagcgacgcaccgctgtactccggtacgcagttggcttcgatcatggcacagtccgcaggcgcgcacatccgcgcacaggaagccgtcatcaaccagcgtaacgctgcggccaaggccgcgctgaccgaccagcagaagctggccgcgcaggaggaggacatccgtggtggcatcgaagcgttcaagcgcggcacgtacgcgcagacgatcaacatccccggcgtggacaaggagctgatcgaggcgaacacggtgcaggcatggaatgccacgatggccgcgaaccccaaggtcgccatgtcgcagctggtgtggaacgccaacaccgggcgaggcgctgtgctgaagggtgtggccgaccagttccagaccacggcgcgcgctgtgctccgcgatcagccgaacacggcagcggctgcactgtaccagcagtggaaggaactgaagcagaccaccgccgcacgcatcgacacgaacggtcagcccgtgcagggccgactgactggcgcgactaccgctgcgctgtacttcggagatagcgtcaacacgttcttcaacaagctgcaagcgttggagaatggtggcgtgaacttcgagcttgcttacgaggtggcccgtggagaaatcaccaccgacgatccgacgcagttcgacgcgaacagccgtaaggaatccgaggctactcaggctcgtgttacggaagctatcgccaagctcaaccccaagtacctcggcatgttcggcaacaagctgggcgactctggccgcgctgcgtatgctcgcgccatcgtccgctcggtcactgacaccggtggtctgctggacacttctgcggaaggcttgcaggctgcggctactcacgccaagctggcctacggtctggaagacgcaggcaagtacgcatgggaaaacggacgcgacgacgaaggccgagtgatcggcagcgtcggtgcatggctgggcttcatggacacgaaggaaaccggacccgccatcgagaaggccatcgacgcagcactgcgccgggtcaacatcgagccgagcaccgggctgaaggctgacgtgttccgcatgaaggacagcgagaacggcgagccggtgctgtacgtcaacgctgttggcgagaagggctggaaggttgtgccggtgtacgggcgcgacatcaaggacgagtacgagaagcacaccaagcagcagcgtcagttgcaggccccggtaccgcagggctacgttcgcatgaacgacggtacgattcagcagagcatttccatccaacccaaactgtaaggagatagacaatggcactcgatctttcggggctgacccaagaccagcagattgccaaggctgccgcttatgcgggagtgccggagtccatcgtgcgcggtcagtggcgagtagagtccggcaacgggcgtgccgccaaggacgctgacggtgtgatccgcagcaaggcaggagcacagggcgacttccaagtcatgcccaccacgcaggcaacgtgggaagcgcgcaacggtcgcaagtacgacatgcgcaacttccaagacagcatcgagctgtatgccgacatcatgcgcgagaacatgcagcttgccaagggcgacgtgacgaaggcgctgcgcatctaccaaggcggcaccaatccgaagaactgggggcaggagaacgcagcctatgcaccgagcgtgctgggcggtgcgtccgctcccgcagtgtcggcgcagccgcgcagcctgaccaccacgcaggcagacctcaacgccgcatggcagggcaacccgaacatgcgcgaccgtacgtggtccggtgcgtccatcccggatgcgtggacgggtgcgcccatcgaaggccgcaacgctctggcgtcggcagcgaaggaacacatcggcaagattcgtgcgggcatcgccgagctgtcgatgggtcaggtagcacaggaaggtggcaccgccgcgcaggccgtaggcaaggctcaggctgtccgtgcatcggatcaggttgtgccgtggtgggtgcgtcaggaagtggacgtgctgaacaccggcgctcgcaaggcgctgctggatcagaccgaacaggcgctcgcgcaggaccgcgcggacgaggagctgcgcaactcgctgaccttcctcgacaagtggggcgctgcgttcgacagcggcatcggtgctgcgatcagcaaccagtttgcgcgcgaggacgagaacgttccggaaggttggaagtacgacccgaaggaatgggagaagccgtggatgactgccgacgaactcgaagacatccgcgatgcagcgtactcgccgaacgagctgaagtacgtcagcgaccgacagttcctgcgccgccactccatgcgcatcaaggatcagcagactggctggggtagcttcggttacgacatggtggcaggcttcaccgatccgggcaactgggctatcggcggcgtcactgccgcaggcgctaaggcgctgggcatcggctcggctgcactcgttgccgaagggcgcgtgggcgcgtcgctcgcgtcggctgctgcggagaacgcggtcggttccgtcatcacggacgccgcgctggttggcatgggcgagcgccgcaacttcgcggacttcatgaccgacgctgcattcgctaccaccataggcaccgcgatgcacattccgggcgtgcgctcggctgcgcagattcgtgacaaggcaaccatcgacctgtccgcaggcaacgctgccgcttacggcgaagcgtggtcggccgacctgaaggcgcgcgctgtggccgagctgggcgaggacgccaacccggtgctggtgaacaaccgcatccaccagcttgccaagcaggaggctgtggattggctgcgcgctggtatggccgacgtgcctgacgacttccgtatattcgcccgtcccgacgtgcaggagacgaccaccaccgcaggcaccactggtgcactcgcacgggacgcgggcaacgtggacgcaacgaccgggcggtacaacgacagcgtgggtggccgggtcgatcagcatgacccgctgctggaacgcgcatggaagaccgcaggtatcaagggcggtaacgtcgatggcgtgctgaagtatctggaatccaacgcctctatcccggaggacgtgcgtgctatcgccaacgcgctgaagcgtggcgggcggctgagcacggtgaagatcgtgccggaatcggaactcgacaagtggttcgccggtgccaacatgggtccgggtatgcgtgtggccggtggctacaacgccggactggacgcgatggcgatgcggaactacacgccggaagtggtggtgcacgaaatgctgcacgctgccacgctgcgtgagctgcgcagcaactcggtgttcgggcaggaaatggaagaactgctgacccatatcaacaacagcatcggcagtgtggactccacgctgaccaccgctgcgatggagacgcgcatcaaccagccgcaggcaggcttcctcgccaacactgacgagctgatttcctacggcctgacgaaccgcgctgtgcaggcggtgctgcgtcagatgcccgcgccgggcaacacccgcccgaatgcgtgggagtggctgaaggataagatcgcgcgagtgatgggtctgaagaatcaggagtccgcgctcgaacgcctgatgtcggtcgtcggtgacaacctcggcgcggaagtgcgcgacacgcaggccggtacccggcagacgcgtggcatgctcgccaactcgatcttcaagtcgaaccgcgagcgcaaggctttctaccagcgcaccggtctggacaagtccgtcagtgatgacgcgatgcgtgtgcaggtcgccgaagtgatggcacgctccgaacgcttcagtgcgcagtacggcatcgacgcggcgaagctgtccaccatcatgcagcgcttcgggctggaagctacgagcacgactctaatgtcgtccaagtcgccagttgcccgcatgcttgcgatcaccctgttggagaatcccgagggtgcagcaggccgacacagcaccgcagcgatggatcggcatggtcggtttgagtcgttcatgggcacccgcccgcgtcagtgggaagcggcctatcgcctgtggcgtgcggacgtgcgcggtatcggtgcgatcaaggacttcgccacgggctggaaggctcgcgcggacttcgagtacgcagtgaagctgtaccgcgagactcgcttcaacggcggggacatcccggatgcgcacgaggcagtgaaggcaatggcccgtgagttggaccgtggctacaaccgcatggcagcagagcagcgcgcggccggtacggtgggcgcacagcgtctgccggaggaggacgtggagggctacgagtcccgtacgtggctgggcggcagcatcgctgctgctggtccggtgcgacgcgagggtatccgtcaggcgatgcgcgatcagttcgaggtgatgggcgagctgtatggggacgacttcctcgataagttcgctaccaagtatctggaacgcatcgagcgcaaggctgcgggtgtcatcgaagcgccgggtcaggtcttctcggagtcgcaggcggacacgctgcgcgacactctgcgggcgatgtcgctcaacgaggaggagattcagaaggtcatgggcaagtacagccgtggcggtgcgaagcacaccaaggcgcgtatcgacctcgacgtgaccaagcagtacgaggacgctgacggtaagttccgtctgatggactatctcgacaaccgcgtgatggacaactaccgcaagtacgcgggacgtgttgctggtgacatcgctctggcgaagcacggcatcctcggcgacgcaggcatcaacgtggcgcgcgaagcaatgcgcctgaccggtgccaacgatgtggagctgaaggcgttcgagcaggtgatgtccgagttccttggtcgcccggtcggtaccggcgatccgactgttctggcgaatgcgcgtctgctgacctcggccatccagctgggcggcgcgggcatcaatcaggcagcggagtacagcaacggcctcgccgctgttggtgctgctggtgtggctgacgcaatccgtatcgctccccgcatgcgcagcgaaatcatgcgcatcctgaagggcgaggacagcggcaaccaaatcctcgacggcttcgagttcatcagcggtcgcggcttcggtctcgccggttacgacctacacatgttcaactcgctggacacgcaggcgtcgatgtatggtagcgagcgcgcaggcttcctgacctcgctggtgcagaaggcagcgcatgcgaaccgcatcctctcggggcagcgggccgtgcttgctgtgcagcagcgtggcttcgcggaagtgctgatcgccaagggcgtgaagttcctgcgtgatggtgctgaagctgacaccgccctgaaggacatgggcattgacgacaacctgctgaaccgcctgcgggctacgcaggatcaggtcgtgcgctggggcgcggatggtaagctggaagcagtagacccgcgcaacgtcgaggggctggcggatcggcaggcatggttggcgttctacaacgcgatcaaccgtggcacctcgcagattcttcaggacaccttcatcggcgagactggcaagtgggcgcacaacggctggctgaagctgctgttccagcaccgcacgttctcgctggtcgcgcagcagaagcagctgggccggtacgtgggcaactacggtgcatggcagacggcgggcctgatcgctgctgcgatggctgtggcggctccgctgcaagccctgcgggtgctgtcccgcgtggccctgatgaacgatcaggagcgcgacgaggccatcgaccagaacatcctgtcgcctctggcgctgggcaaggccacgctgaactacgtgtcggcgacgggtatgctcaacgatgtgctggacgtgggcactggcgtggcgggcggctggtacgagtacgccaccgatacgcagggtccgacgtggctgaagcagctggccggtgggcagttcggcaaccgcaaggaagtggtgggcgggcagttcgcgccgtcgctgggagtcatcaacgacttcgctcagggcattgctggcaagccggagaatctggccgacgtgattccgggcgggcgactgccgatggtgatcccgctgctgaagggcgcagccagccagtggaaggaggagtaagatcagggccaaggacggcccacccttttggtacacctatagcaaacaggaggcagcatggcagttccagacccgcagctgcgctacgcgacagacgtgttcgacgccgatggcgtgaccactgactggcagatcagctttaccggtggctacatcaacccgtcccacgtgtacgccatgagcggactgctggacgaggagactcagctgctgaccgaccggactccgcacaccgtggaagtcctgagcgaagacgatgacgctagtaccgtccgagtctcgcctgccgtcgccgctgggcgcaagctctacatctaccgcagcactccggtgcagcagatgctcgttgactacgttaacggtagcatcatcagcaagacaaaccttaacctcagcaacgaccagctcctgaagatcattcaggaaatgttcgactcactcaacatcgccacccttagcatcgaccagcaggtcggtgtgatcgtggacctgaacgagattatccagaacatctacaagcaggtcaccgagttgctggcagctggtggtatcgtgtccgtcgccccgcgcgtctggtccggtgcttggactggcgatcaggtgggtgacaccgacttcgacatggtgggcgcggacgtatccggcgcgggcttctacgacgtgtacgtcaacggcatcggcatgcagccggacgtggactatcaggtcacgctcgctgacggcaccgatcccagcttcatccgcttcgccacggttcctgccgagggcagcatctggttcgccgtgctgcgtggttacgccaagccctacaccgggcctgcgccgatcaccgctgcgagcctgcgggtgccgatcatcacggcagagggtccgacttactacgccgccaaggctaccgagtacggactcgtgcgctgcacgtacgccggaggttgcgccgtcaacatcaacctgatccccgaagtgggcgacggtgaaaccaagctcgcctcgggcagctacttcagcgtgcagcagaaggcaggccctgtggtcatcactggcgacgtgggcgtgacgctcgaagtcccggtcggctgcaccgccgcaactcgcggcaccaactccgtcatcactgcaacgtgcatcgacggcgacaccaacacgtggttgctctcgggcgacttggctaaggagtaagcatggctaatcacttcaggctgtacggccgaccgctcatggcggacgaggttgcagatggcctgtcggtgacgggcgtgctggaagggtacacggcgggcgaggcttacgagtctcgcctgtccatcaacaacccagtcggccgctgcaccgtggaggtcatcgaatcgacgctcccttcgggcgctgcggtacgggtggacaacatcaccaaggaagtcgtcgtcaagtgggcggctttcactgaagtcgtggacgaggaaaccctcgtgcccaacggcgacttcgaggcaggcgacgacggcacgtggttgccgggcggtggatcgaatggcgaaggctggtcgattggcactggctcagactacgacaccgacagcggcgtgtacagcgcgcgcttcgccaacatcaagacgggcggcagcgacctgctcaacccgctgatccctgccaaggtcaacgactacatccgatgcaccgccgaggtccagcagggcgcaagctccaagggcaaggccggtgctcgtgtgtcgatcatctaccgcaaggaggatgggaccgagctgcaacgcaactggggcaacatggtttcctccggcagcaacggtgcgtggcaccagtccgttgccgaaggcgctgcgcccaaggacacgaagtacgtgcaggttgtactgtcggcgttccgcagcaagcagaacaaaccgctgtgggtggacaccgttaagtggaaccacaagtacgtactgggtcagaacgacgacagctcctacttccttagcatcaaggtcacggacgggttgaaccgtgtggcctactggtccggtcgtatcgaggagcagggcatctacgttacgtccaagctctacagcttctaccagttcgatgccgcgatgctgaccagcagctttgctgggtacagcaacatcgacatgctccagcctttggatactgcgtcgctgggttcctccttcgtaagctgggaactccgaagctctaggcaggattatgccgccgacccggagagcacgttgtacgggagcgctttcgtttcgttcgacatccgatccatccgtaaggactacacgcctgacccggagacggcgaagctgtcgagttctttccattccttcaccctgaagcagcaccctgtagtcaaccagccgctcgacgcgactgcacgactccggtctggcttcgtatcatggagcttcgcatgatccacaatcacctcggcattgctggcgtgttcaccatcagcaagggtaagtccctcgatactctcgaagttgtagccgactggcagagcaaccttatcacggacggtggtatggacgcactgggtgataccggcagcggctatcctcgcagcatgtacgacctcattgcttacttggcagtcggtagtggcagcgccaccccggcattcaccgataccgctcttggtgcacaggtggcgcaggttggtcgtacgtcctcggacagcggtgggactaccactgccccgtactacgcctactcccgctgccagtaccagttcccggctggtaccgctactggcgttctgtcggagcttggtgccaaagcatacaacaacaataccggcgcgtacatcctgaccacccgtgcgcttatcaaggactccgcaggtaacccgaccaccatcacggtgctgtcggatgaaatcctcgtggttacttacgagctgcgcatgtacgcagataccacgccggttgtcactactgagacgatcaagggtgttagcaccactgttacctgtaagcctattgcaatgggccgcagcggcggtatgaacggtcagtcggcagtcgcttggtcggactacgtgtgggggtgctactacttctacggcggtactggcgacggcaccggagctatcaccgaccagtatccgccggggacgattgccagcttctctgacttgcagcttcagcaggtagcctatgttccgggtacttactaccgtgactgcgtttgccggatgtcgatcaacaacgtgcccggtggtccgatcacggctgcaatgggactctccgcgtgcgtgaccttccaagtcggcttcaatccgggtatcaccaagaccggatcggagacggcgaacttgcgcatgcgggtttcttggagccggtacacgccatgatccccactgtctcccaaagcatccaacgcggtgactgggtggagcagcagaatcggcgcacccgcccgctcattgacttcgagcagggcgggctgactctcaacgcagcagtggacgacctccaagctgcgctgtggactgccgagagtgacggcagcagcgtcgtcgtttaccgcgacggcgttgccccggtcaccgtgctgaccgactccgggatcacgcagatcgcactggccttcgaccagaccatgcgcccgcacgtggcgtacatggcgggcggtgtgtgcaagttctactggtacgacacggtggctgcttcgatgcagaccatggtgatccccggtgctaccactccgcgcctgtgcatggacgagaagcgggctgtcttcgccacgcagagcgacgtgctcctgtcgtacaagaacggcagcaacctgtgcgtacgcgcgcagcgtgagcgcttcgcaaccgaacatgtgatcgcctcgggaatccccggcgacctgattgcggtgggcatgaacaacgtcaaccgcctgcaatggaagctcgtcggcaatcccgacgactggccctaacctacaggagaacagcatgaccccgccgagtgtggtcaatgaggtcgtccgaacctcgccgcttacgctcggcgcggtctacctcaacttcatcagcacgtacggtgctgccatcgtaactacgctcgccattctgtacgccgtcgctcagttctactggcgggcacgcgagcaccgaaagatcatgggaggcaaggatgtcgaatccggcaagtgagggcgcactcggtgcgctgcacgaactggtcgcgcgtgcgctgatgcagcgcatccaagatggcgagctgtgcaccgcagccgacatcaatgcggcgatcaagttcctgaaggacaacaacatcacggcgacgcgcgaggccaacaaggcactcggcgagctggaagacgagctgggcaagcactcgctgcctccggctgacgacgacgagttgcagcgtgcactcgacaacatcgttcactttccggggagcgtagccaacaatgcgtgaatcagctgaagcggccgacgtgcgccgcaagaagttggagctgttgcagaaccactaccggcacttcgccaccttcatgcgcgacattatgaaggtgctggggttcgagccgacgtggatgcagtacgacatcgccaactacatgcagtatggcccgcacctcgcaatggtgcaggcgcagcgaggcgaggcgaagtccaccatcgctgccatctacgccgtcttctgcctgatccacgatcccactcaccgtgtgctgatcgtatcggcaggcggcacgcaggcatccgagattgctacgctgattcagcgcatcatcctcacggtgccgacgttggagtgcatccgcccggacaagaacgcgggcgaccgtacctccgtggatgcgttcgacgtgcaccactcgctgaagggaatcgacaagtccccgagcgtggcgtgcatcggcgtcaccggcaacctgccgggtaagcgtgcggacctgctgatcgccgacgacgtggagtccaacaagaacagccgcactgccgcgaaccgtgagctgctgctgaccatcacgttggagttctcggccatctgcaccggcaagcccggtactccgggtcgcatcctgtacctcggcacgccgcagaccggcgactccatctacaacaccctgcccggacgtggctacgacgttcgcatctggcccggtcgctacccgaccccggcacagcgcgagcactacggcccgcatctggcaccgtctatcgtgcagcgcctagaagccgacccgatgttggcgttcggtggtggcccgatgggcgacgagggccagtgcaccgacgagctgttggccggtgagcagaagcaccagtccgagctgcgtcagcgtggaccgtccagctatcagctgaactacatgctcaacacgcggctgatggatgcgctgcgcttcccgctgaagaccgagaacctgatcgtgatccccggtggtggcgaccgcttcccgctgacgatcacccgtggcctgagcaacgctcaccagcgcagcttccagtccagtgggtacggcttcgtgatgatgatgccgcacgacatgagcaccgagactgcccccgtgcagggcgtgcacatgcagatcgacccggccggtggtggtgccaacggagacgagacggccttcgccgtgaccgccttcctcaactccaccgtgtacgtgttggccgtgggagctgtgcccggtggctacgacggtgatggcttgctagaactgcgccgcattgcggtgaagtacaagccgaacgtcatcagcatcgaaaagaacatgggctacggcgcgttcgccaaggtgttcctgcctgtcctgcgagaagatcgcggcacggagaagggatacaagggcgacatccgcgaggagttcgtgaccggcaacaaggaagcccgtatcatcggcactctcgaacctgtcatggctcgcggctcgctggtcatgctggaatccgtggttgaaatggatcacgagtacacccagcgctacgccaccagcggcaagcgtcaggtctacagcctgttccaccagatggcgaagatcacgcagcagaagggcagcatcgcacacgatgaccggctcgatgcactggaaggtagcgtgcgtcactgggttgcgcagcttgcactggaccagaacaaggccatcgccaagcagcagcagcgagagttccaagactggatcaacgatccgaccggcatgaaggcagcgacccgcaagagtccgctgcaacgtggccgtccatccctactcgaccgttaccggaggtaaccaatgcagaagtccgacttcaccagcaactacacgggtctgttcggccgtggcaactacctgcaccgcgaactgctcgccctcatggagcacgcagagcagcatcccgcaaccgcagcgcagctgctcgcgcagttccagaaggacgccaccctcgtgctggacgccctgatcgctgcgggcgcacgcaccgcgtcctcgggtccgaactccggcccgcacactccggtcgatctggacccggatgacgacccactgaccccgtaaggagcaaccatgaaccagcagcagaaccaagataccagcaacaaggggctgttcggcctgatcggcggcatcttcatcggcatttcggcaacgctgctgtcattcacccaaggccacgaaggggtacgctacgctgcgtacctcgacaccggccgggtgccgaccatctgctacggccacaccaagggcgtagcgatgggcatgacggcaacgaaggcacagtgcgacaagtggctgatcgaagacctacagatcgcccagcagggcgtgcgcaagcacctgaaggcccccgttaaccgcaaccagatcgacgcctacacagacttcgtgttcaacgtaggtgagaaggcgttcgccgacagcaccatgctgcgcaaagcgaacgcaggggatcgtgaaggtagctgcaaggagttcctgcgctgggtctacgtcggtaagctcgactgccgactgtccagcagccgttgctccggcatccccaagcgccgcgacgcagagtttgctctgtgcttgcgccccaacaacgaggtgatccaaccgtggaaaccccaagtgaagtgatcgcgcggctcggcggcaagctggttggcttgctgctggtcgtgaccatgttcgtgtgcttcggtctgtacgtctacggcctgcaacgcaaggtggagaagctggaaactgcccaagtcggcacgaccgctaccgccaaggcggcgcagacgcaggctaccgggtacgcgacctacatcaaagagaaggaggacgtgcgtgttcgcactgaagaagttcttgacgctgccccggagtaccgggatggcactgttcctgctgatgtcgctgacctcctgcgcgaacctgccggtccctgacgactccctgcttgcagactgccacatcacctacctcggtggggagaagggcaccacctcctcgcaggacaaggtggtcaagctcgcgcaggaccgccgcatggacaccgttctgtgcaacaaggacaaggctgcgctgcgtgcgtggaaggccgaggtgtgcggtaccggtaagcgccggtgtacgggtgacaaatgaccaccatcgcatgggacggcaagcacctgtgggccgatagtcaggccacgcagggcgaccacaagcacaccgtgcgtaagatcatgcccgtatcgacacccaccggccctgtgctgctgggtgtcaccggggatttcacagtgcttcgcccggttctcgctgcgcttaaagcgggcgaaggctacgaggagcacgttggcaagtccgcgacggtgcttgtggttaaggacggcgtactcacggtcactactggtaagcagcagtgggtcgaggaggctccgtacttcgatggcagtggcaaggcgctagctctaggggcctatcatgcgagcaagtctgtggctaaggccatggctgctgcgatagctcacgatgtctacagctccgggcctatcgtcaagctaaaggcaccagttcgcgaggcttaggagtaaggccacgtgggtagccggaccaaaatttgcttcggaaatgcgcgggggtcactccaatagaagctcccgcgcgtgcccccgtacgccctcgcgttacgcgcctgcgggtgtgcgtgggtgcgtgcccgcgtgtgcgcctgtgtgcgcgtctgtgcgcccgcgtcaaggttccgcgtgggtgtacccgtgtgcctgcctgcgtgggcctgagcgtgcgtgtgcgtggccgtgcgtgggtgcctgcgggtgggcgtgcgggtgggcgtgcgcctgctgcctgtatggctggaccgcgctgccttggctgaatcgttaataaatctcttggcgaaaggtgttgacgtggccggtgcggtgtggttcaatggcgtcactggggcagcgacagggcttcaggagggccgcaaggggcttgacaggggctaccctacctgctaccatgcgaaccgcagctgtaggcgtgcgagggccatctgtatcgtttcggccttttggtacacctatagcacacagtcggctcaacctgaatcaccgtctatcggtactctgtcgagctgattagttagctacccgctaggccaacggttgacgcttgcgatgcaagcagtagtagacacacggccgcaatggtagtaagctgcaacgcaagtcgagtgacgtgatccgtagtggcgccgccaacaagtgggctaagggtacacgggagtcactggtaagggatgcgaggagctaccgaaccacgcttgacactaagctagcagttagctatgataggcggcaagtggtagccaccggaacagcggagcgacctagcggtaaggctagacgtgagagattacgggtgttgaggctgaggtgagaccgggacaccggtcaagacactaacaggagcgcacatggtcctctaacggatagcttgacaaggcggcacagatagccctttgaggccttgcaacacgtggaccaccgacgtacatggtgggatggtggcgacaggacgcccaacgggttagagacccgagcgagccaagggcttgacaggatgcaacaagggtgctagtatggcaccacgctctgaggagcagccacattggatggcgtaggactaccgctaacgggtagggtgtaacgggaagcgtgccaaccacagccaatagtggccgagagttgacgtggaccgccaagctgcaacgtagcactagcggataaccggatgaactgggatttcaaaggcccatagaatccaccagacttgcaacactggtgccgctttacctaagcctaacgcttagggcttcccatctgccgtgagagtcggccacgggaagtaacccactgccaaggtgggaagccggtcataaggaggtggtgagcctcctatcgcatggaatactgtgcgtttcgtgaaaaggctctacgggccacacggtgacaatggcactgctagccggagtagggttgacagcccgaagggctagcagattgatgcgccctccctttgcgatgaccatgcaggcaaatccggtggtcagtgtgcgcccacgataggcgatgcaacggctctaatcgagaatgagggattgaccgactcgacggctttctgagggcgcatcaatctgttagttttcccaccagtgccaatggaggcacaacatgcaaggctcgatcaatgccaatctcgaccgcacccagcgtaagcgccgcttctgccagttcacccggacggcaagcgtgatggacctgcgcaccacggagcatgaccgcaagcttgccgagcgcaagcgccaagccgagcgctacgaagcccgccacggaaccgccggaaagcgatctgtgtttgttgtcgagggtaacagcgggacgaaccgggcgaaccacgccgctgacaggagggcttacctgtgatccggttcaagttctctcgccactacgtggaagctgcccgcgattcctacaatcgggccatcatgaagcatccggccggctctgtgtcggcgctctacgtcctgccgtgcggtgggcgttcattcgacatccgactcgcttaaatgcaagctactgggccttcgcaagagggcctagtgtcgtgcaatcggcacggacccaacctgaagggaaccaccatggacatcatcaccggaagcgctgacatcaagcgcgccatcaagtcgatcaacaccgcccgcaccaagctggtggaccagattcagcaggccgcgattgcggtcatcaaccacgcacacatccacggcgacgttacgctcgcttccgatctgtgtctcgccgtgggcaacggcatgaagcatgaagccctgcgcctgtacctgtccgagttcggcccgatggctccgaacgacgacaaggaaaccaaggcgagcgcgcccatgaagtttgccaagagcaagcgagtcgagggcgaagctctggccgacgtgctggaacgtgccgccgcgaaggcgtggtacgacttcaagaccgagaagcccgcagaggcgttctcgttcgccgccgacctgcacaagctgctgggccgtctggaaaaggcgaccgaggaaggctacgtgccgaccgaggaggaacaggccgtcatcaacgctgcccgcgctgtgccgaagcccaccaagaagaaggagaacgtgtaacatggaacccaagatcaaccttcgagtgacccagcgcgaagcatccctgctgcgctcggcccttcacatcgcctgtgcactgaccgcaaaggcagacccgtactccaaccgcaagctgtccaatgagttcgccgtgctgcacggtgagctgcgcgacttcggtgtcgagagcttcgagcgtgacgccatcctgcaattcgaggacgacgtgattgcggcctgccgtgacagcgatgtcgaggcacagctgctgcgcgacctgatcgcaccgccgacgttcaccgtgggctacggcatgcgtgaacttgacttcgctgctatcgaggcgcgggtgatggcgtgcctgctgtctccgttgcctccggtggtgttggatgcctcgcagctggacttcctcggcagcgtgaccggccgcatggtgttgcccggcctggcaatgcccgacaacctgccgcgtaagctgccggatgtcctgatggacgaccagagcgcacgccacgtcgccctgactgcatcgcagaccgggctggtcaacaagacgaagaccaagggctggatcgtgcagttcaatctgcgccacggcagcatcgccctcgccaactgggcgcaggtgcgtgagctgggcctgccgcagcgcagccgcaatgctgcgtaccgcatgctgaaggcgcgggccaaggtgcagggcatcagcgaggatgcgtaccgtgtggtgcccgaaggcactcccgatggcccggagaaggatcgcggcttctacaccgccgagttcttcaccaagcatgcgcggcgccctcaccagctgggttggaatacgtccactgtgatcggactcagcggcacgttcaccactgcgcaggctgcacgcaacgccatcgcctcgcacgtcggcaacgatccgaaccgtctccgccgctaccgcgtgaagtggcacccgagccgcgcgtgatctaccgctgcgccttctaacgagggcgtagctttggaaccacgcccaacaggagggcacattgcatgatccccgtaacttacaagcgcatccgtagtggggagcgcaagccgatccagctgtgcgagcagccgcgccagtggaaagagttcgtgacccatgagcacagcgtggagcgctggtatgcgtgaggtcagcctgcgccttgtggtgaaggcgctgccgctcgttaccgtgaagggtgtggctgtcggggattacatcctcggcggacatcacaccagccacgaggcgtgcgagcaagccatcgaacaccaccgcaagcaccacgagaaggtgcccaccctctactcgatagaggaaatcgaaatcccacccgtcaatcaggagaaccaccatgcgtaaggtatacttcatcgtctcgatccccaagaacagcaacgatggcgtcatcactggcgtcgtcgccaatggcaccggccgcaccccgacccaagaggaactggatgcggtgatcgccgagctgcgcaccaagggtgccaccaccagcctgctggactcgctgcgtgacggcacgtacccgaaccagctcgccatcttcgaccgccgcgccgccgtgcgtgccgaggcggatgtgctcaacagctacggcgggtcgttcttcaactggcacatcctcgaagtgggcgagagcatccgcaagccggtgcgcaagccgctgggttggcgtatcacctacgccttcgccgaagaccgcagcgactccgatgtcagctgctacaaccagcacccgagcgccaccgtgcgcatcgacggcaacgagtacaacaagagcgagtacaacgtgctgttcccgacccgcgatgcagcgcgcgccgtgttcaatgccgagtcgctgggcg

SEQ ID NO: 26 - DNA, 44287 bp, unidentified
  source 1..44287: mol_type = genomic DNA
gtagtcgcgccggggatcaccatggtctgcatcgaagcagccaccgtgtcgtaccagtagaacttgcacacaccgcttgccatgtacgccacgtgcgggcgcatagtctggtcgaatgccagtgcgatctgcgtgataccggagtcggtcagcaccgtgaccggggcaacgccgtcgcggtaaacgacgacgctgctgccgtcactctcggcggtccacagcgcggcttgtaggttgtccactgccgcgttgagagtcagcccgccctgctcgaagtcaatgagcgggcgggtgcgccgattctgctgctccacccagtcaccacgttggatgctttgggagacagtggggatcatggcgtgtagcgactccacgaaacccgcatgcgcaggttggcagtctccgaggtcgtcttggtaactcccggattgaatccaacctgccagctgatagccgcactgattccggcagcggcagtgatgggcgctccggggttgttgttgatcgacatacggcagatgcaatcccggtagtacgtacccggcacgtatggaacgcgctgaagttgcagctcggagaaactgacgtttctgccgggagggtactgatcggtgaccgcgcccgtgccatcaccagtgccgccggtgaagtagtagcagccccacacgtaatcgctccaaaccacagaagacgcgccgctgaggccaccgctgctacccaaggcaagcggcttgcacgttacagtggtgctcacgcccttgatcgtctccgtggtgaccacgggagtcaggtcgggatacaggcgaatctcgtaagttaccacgaggatttcatcggacagcaccgtgatggtggtgggattgcccgaggaatccttgatgagtgcgtgggtagtcagaacgtaagcgccggtgtcgttgttgtagccgaaaccgcccagctctgacagcacaccggttgccgtacccgctgggaactggaactgcatgcgcccgtaagcgtagtagggtgccgtcgtagtcccgccgttgtcgcttgacgtgtaggacacacgagcaacctgagcgccgagcgcagtgtcggtaaacgcgggctcggcactaccactgccaacaccgaggtacccgattaccgtgtagagggactgcggatactcgcggcctccgatgaagtccataccgccgttggtaatgaggttgttttgccagtctgccactacttcaagggagtccagcgacttgcccttgctgatggtgaacacaccagccactcccatcttattgtggatcatgcaaagctccatgatacgaaggcgctctttgccatcgcgctcgcgtctagcggctgattgacaatagggtgctgcttcagggtgaaagaaatgaatcccgaggtaaccttggcactctcggaacctgcgtcgtactccttgcggatcgacttgatttcccagctcacaaacgaggagcctagctcggcatactcgggtgaggctgcgtaatcctgacggctgctgcggacctcccaactcacgaaggaagaaccgaccagcgtgctatccacgggaggaagcatgtcgatgttggagtacccagcaaagctgctggtcagcagcgctgcgtcgaattggtagaagttgtagagcttcgacgtaacgtagatgccctgctcctcgatacggccggaccagtaggccacacggttcaacccgtccgtgaccttgatgctcaggaagtaggagctgtcgtcgttctgcccgagcacgtacttgtggttccacttaacggtgtctacccacagcggcttgttttgcttgctgcggaaagccgacagtacaacctgcacgtacttcgtgtccttgggtgcagcgccctcggcaaccgactggtgccagttaccattgctgccgctgctcaccatgttgccccagttgcgttgcagctcggtcccgtcttccttgcggtagatgatcgacacgcgcgcaccagccttgcccttcgagcttgcgccctgctggacttcggcggtgcatcggatgtagtcgttgacctcggccggtatcagggggttgagcaggtcactgccacccgtcttgatgttggcgaagcgcgcgctgtatacgccgctgtccgtgtcgtagtccgagccagtgccaatcgaccagccttcgccgttcgatccaccgcccggtacccacgtaccgtcgtcgcctgcctcgaagtctccgttgggtacgagagtttcctcgtccacgacttcagtgaaagccgcccacttgacgacgacttccttggtgatgttgtccacccgtaccgcagcgcccgaagggagcgtcgattcgatgacctccacggtgcagcggccgactgggttgttgatggacaggcgagactcgtaagcctcgcccgccgtgtacccttccagcacgcccgtcaccgacaggccatctgcaacctcgtccgccatcagcggtcggccgtacagcctgaagtgattagccatgcttactccttagccaagtcgcccgagagcaaccacgtgttggtgtcgccgtcgatgcacgttgcagtgacgacggagttggtgccgcgagttgcggcggtgcagcctaccgggacttcgagcgttacgcccacgtcgccggtgatgaccacagggcctgccttctgctgcacgctgaagtagctgcccgaggcaagcttcgtctcaccgtcgcccacttcagggatcaggctgatgttgacggcgcagcccccggcgtacgtgcaacgcacgaggccgtactcggtagccttggcggcgtagtaggtcgggccttctgccgggatgataggcacgcgcaagctcgcagcggtgatcggcgcaggcccggtgtagggcttggcgtaaccacgcagcacggcgaaccagatgctgccctcagcgggaaccgtggcgaagcggatgaagctcgggtcggtgtcgtccgcaagcgtgacctgatagtccacgtccggctgcatgccgataccgttgacgtacacgtcgtagaagcccgcgccggacacgtccgcgcccaccatgtcgaagtcggtatcgtccgcctgatcgccagtccaagcaccggaccagacgcgcggggcgacggacacgataccaccagcggccagcaactcggtgacctgcttgtagatgttctggataatctcgttcaggtccacgatcacgccgacctgttggtcgatgctaagggtggcgatgttgagcgagtcgaacatttcctgaatgatcttcaggagctgatcgttgctgaggttaaggttggtcttgctgatgatgctaccgttaacgtagtcaacgagcatctgctgcaccggagtgctgcggtagatgtagagcttgcgcccagcggcgacggcaggcgagactcggacggtactagcgtcatcgtcttcgctgaggacttccacggtatgcggagtccggtcggtcagcagctgagtctcctcgtccagcagtccgctcatggcgtacacgtgggacgggttgatgtagccaccggtaaagctgatctgccagtcagtggtcacgccatcggcgtcgaacacgtctgtcgcgtagcgcagctgcgggtctggaactgccatgctgcctcctgtttgctataggtgtaccaaaagggtgggccgtccttggccctgatcttactcctccttccactggctggctgctcccttcagcagcgggatcaccatcggcagtcgcccgcccggaatcacgtcggccagattctccggcttgccagcaacgccctgagcgaagtcgttgacgactccaagcgacggtgcgaactgcccgccgatcacctccttgcggttgccgaactgcccaccggccagctgcttcagccacgtcggaccttgcgtgtcggtggcgtactcgtaccacccgcccgccacaccggtgcccacgtccaacacatcgttgagcatgcccgtcgccgacacgtagttcagcgtggccttgcccagcgccagaggcgacaggatgttctggtcgatggcctcgtcgcgctcctgatcgttcatcagggccacgcgagagagcacgcgcagggcttgcagcggagccgccacagccatcgccgcagcgatcaggcccgcagtctgccacgcaccgtagttgcccacatagcggcctagctgcttctgttgtgcgaccagcgagaacgtgcggtgctggaacagcagcttcagccagccgttgtgtgcccacttgccagtctcgccgatgaaggtgttctgaagaatctgcgaggtgccacggttgatcgcgttgtagaacgccaaccatgcctgccgatccgccagcccttcgacgttgcgcgggtccactgcttccagcttaccgtcagcgccccagcgaacaacctgatcctgcgtagcccgaaggcgattcagcaggttgtcgtcaatgcccatgtccttcagggcggtgtcagcctcagcgccatcacgcaggaacttcacgcccttggcgatcagcacctccgcgaatccacgctgctgcacggcgagcacagcccgttgccccgagaggatacggttcgcatgcgcagccttctgcaccagagaggtcaggaagcctgcgcgctcgctgccgtacatcgacgcctgagtgtccagcgagttgaacatgtgcaggtcgtaaccggcgaggccgaagccacgaccgctaatgaactcgaagccgtcgaggatttggttgccgctgtcctctcccttcaggatgcgcatgatttcgccacgcatacgaggagcgattcggatggcgtcagccacaccggcagcgccaacagctgcgaggccgttgctgtactccgccgcctgattgatgcccgcgccgcccagctggatagccgaggtcagcaggcgtgcattcgccagaacagtcggatcgccggtgccgacaggacgaccaaggaactcggacatcacctgctcgaacgccttcagctccacatcgttggcaccagtcaggcgcattgcctcgcgcgccacgttgatgcctgcgtcgccgaggatgccgtgcttagccagagcgatgtcacccgcaacacggcccgcgtacttgcggtagttatccatcacgcggttgtcgaggtagtccatcaggcggaacttgccatcggcatcttcgtactgcttggtcacgtcgaggtcgatacgcgccttggtgtgcttcgcaccgccacggctgtacttgcccatcaccttctgaatctcctcctcgttgagcgacatcgcccgcagagtgtcgcgcagcgtgtccgcctgcgactccgagaagacctgacccggtgcttcgatgatccccgcagccttgcgctcgatccgttccagatacttggtggcaaacttttcgaggaagtcatccccgtacagctcacccatcacctcgaactgatcgcgcatagcctgacggatgccctctcggcgaaccggacccgcagctgcaatgctgccgcccagccacgtgcgagactcgtagccctccacgtcttcctccggcagacgctgtgcgcccaccgtaccggccgcgcgctgctctgctgccatgcggttgtagccacgatccagctcacgggccattgccttaactgcctcgtgcgcggccgggatgtcgccaccgttgaagcgagtctcgcggtacagcttcactgcgtactcgaaatcagcgcgcgccttccagcccgttgcgaagtccttgatcgcaccgatgccgcgatcgtccgcacgccacaggcgataggccgcttcccactgacgcggccgcgtgcccatgaacgactcgaaccggccatgccgatccatcgccgccgtgctgtgccggcctgctgcgccctcgggattctccaacagggtgatcgcgagcatgcgggcaactggcgacttggacgacatgagggtcgtgctcgtagcttccagcccgaagcgctgcatgatggtggacagcttcgccgcgtcgatgccgtactgagcactgaagcgttcggagcgggccatcacttctgcgacctgcacacgcatcgcgtcatcgctgacggacttgtccaacccggtgcgctggtagaaagccttgcgctcgcggttcgacttgaagatggagttggcgagcatgccacgggtctgccgggtaccggcctgcgtgtctcgcacttccgctccgaggttgtcaccgaccacagacatcagccgttcgagagcggactcctgattcttcagtcccatcacccgcgcgatcttgtccttcaaccactcccacgcattggggcgggtgttgcccggagcgggcatctgacgcagcaccgcctgcacagcgcggttcgtcaggccgtaggaaatcagctcgtcggtgttggcgaggaagcctgcctgcggctggttgattcgcgtctccatcgcagcggtggtcagcgtggagtccacactgccgatgctgttgttgatgtgcgtcagcagttcttccatttcctgcccgaacaccgagttgctgcgcagctcacgcaaggtagcagcgtgcagcatttcgtgcaccaccacttccggtgtatagttccgcatcgccatcgcatccaatccggcgttgtagccacctgccacgcgcatacccggacccatgttggcaccggcgaaccacttgtcgagttccgattccggcacgatcttcaccgtgctcaggcgtccgccacgcttcagcgcattggcgatagcacgcacgtcctccgggatagaggcgttggattccagatacttcagcacaccctcgacgttgccgccacggatgcccgccgtcttccatgcacgttccagcagcgggtcatgctgatcgacgcgaccacccacactgtcgttgtactgacccgtggttgcgtccacgttgtccacgtccctcgccagtgcaccagtggtgcctgcggtagtggtcgtttcctgcacgtcggggcgggcgaagatgcggaagtcgtccggcacatctgccatgcctgcacgcagccagtccacagcttcctgctttgcaagctggtggatgcggttgttcaccagcaccgggttagcgttctcgcccagctcggccacggcgcgtgccttcaggtcagccgaccacgcttcgccgtaagcggcagcgttgcctgcggacaggtcgatggtagccttgtcacgaatctgcgcagccgagcgcacgcccggaatgtgcatcgcggtgccgatggtcgtggcgaacgctgcgtcggtcataaagtccgcgaagttgcggcgctcacccataccaaccagcgcggcgtccgtaatgacggaaccgaccgcgttctccgcagcagcggacgcgagggacgcaccgacgcggccttcggcaaccagagccgccgagcctacgcccagcaccttggcacccgcagcagtcacgccgccgatggcccagttgcccggatcggtgaagcctgccactaggtcgtagccgaagctcgaccagccggtctgctgatccttgatgcgcattgagctgcgacgcatgtactgtcggtcgctcacgtacttcagctcgttcggcgagtacgcagcatcgcggatgtcttccagttcgtcggcagtcatccacgacttctcccactccttcgggtcgtacttccaaccttccggcacgttctcgtcctcacgcgcgagctggttgctgatcgcagcaccgatgccgctatcgaaagcagcgccccacttgtcgaggaaggtaagcgagttgcgcagttcctcgtccgcacggtcctgtgcgagagcctgctcggtctgatccagcagcgccttgcgtgcgccggtgttcagaacgtccacttcctgacgaacccaccacggcacaacctgatccgatgcacggacagcctgcgccttacccacagcctccgctgcggtgccgccttcctgagccacctgccccatcgacagttcggcgatgcccgcgcgaatcttgccgatgtgttccttcgctgccgacgccagagcgttgcggccttcgatgggcgcgccagtccacgcatccgggatggatgcaccggaccacgtgcggtcgcgcatgttcgggtttccctgccatgcggcgttgaggtctgcctgtgtggtagtcaggctgcgcggctgcgatgacactgcgggagcggatgcgccgcccagcacactcggtgcgtaagccgcgttctcttgcccccagttcttctggttggtaccaccttggtagatgcgcagcgccttcgtcacgtcacccttggcaagctgcatgttctcgcgcatgatgtcggcatacagctcgatgctgtcttggaagttgcgcatgtcgtacttgcgaccgttgcgcgcttcccacgttgcctgcgtggtgggcatgacttggaagtcgccctgtgctcctgccttgctgcggatcacaccgtcagcgtccttggcggcgcgcccgttgccggactctactcgccactgaccgcgcacgatggactccggcactcccgcataagcggcagccttggcaatctgctggtcttgggtcagccccgaaagatcgagtgccattgtctatctccttacagtttgggttggatggaaatgctctgctgaatcgtaccgtcgttcatacgaacgtagccctgcggtaccggggcctgcaactgacgctgctgcttggtgtgcttctcgtactcggccttgatgtcgcgcccatacaccggcacaaccttccagcccttctcgccaacagcgttgacgtacagcaccggctcgccgttctcgctatccttcatgcggaacacgtcagccttcaggccagctcccggctcgatgttgacccggcgtagcgctgcgtcgatggccttctcgatagcgggtccggtttccttcgtgtccatgaagcccagccatgcaccgacgcctccggtcactcgaccttcatcatcgcgcccgttctcccacgcgtacttgcctgcgtcttccagaccgtaggccagcttggcgtgagtagccgcagcctgcaagccttccgcagacgtgtccagcagaccaccgctgtcggtgaccgagcgtacgatggcgcgagcatacgcagcgcggccagagtcgcccagcttgttgccgaacatgccgaggtacttggggttgagcttggcgatagcttccgtaacacgagcctgagtagcctcggattccttacggctggtcgcgtcgaactgcgtagggtcttcggtggtgatttctccacgggccacctcgtaggcaagctcgaagttcacgccaccattctccagagcttgcagcttgttgaagaacgtgttgacgctatccccgaagtacagcgcagcagtagtcgcgccagtcagtcggccctgtacgggctgaccgttcgtgtcgatgcgtgcggcggtggtctgcttcagctccttccactgctggtacagtgcggccgctgccgtgttaggctgatcgcggagcacagcgcgtgccgtggtctggaactggtcggccacccccttcagcacagcgcctcgaccggtgttggcgttccacaccagctgcgacatggcgaccttggggttcgatgccatcgtggcgttccatgcctgcaccgtgtttgcttcgatcagctccttgtccactccggggatgttgatcgtctgcgcgtacgtgccgcgcttgaacgcttcgatgccaccacggatgtcctcctcctgcgcggccagcttctgctgatcggtcagcgcggccttggccgcagcgttgcgctggttgatgacggcttcctgtgcgcggatgtgtgcgcctgcggactgcgccatgatcgaagccagctgtgtgccggagtacagcggtgcgtcgcttcccgtctcggcggcgtaggtcgagttcatttcctcgatcatcgcctgcgacggcttggcaccaatgccctccgatgcgtacatggagacgagcgccatcttctcggcctgctccgggttggcgtcgagccagtcggaacggtaccggtcctgcgcttgcttcacgtactgctggattccaagctgcccatcagggtcaatggcgctcagcacgcccttgctgttgaggaacttcagcgtgtggaactcgccacgatccgcagcgccacggtagaacgccgtgatcgcggacttgtaggactcgtccgtctggtagcgcgaaggcgacagcccatccagcaaggacagctgcgcctgcgtcagcgcctcggtagccttctcgtccattggccggttggtgccgagcatcgccgtgcgcttcgccagttcgttgaagccggtggacgccgacgagttcgcagcgtactgtgctttcaccagctcctgctgctgccacgccgtacgctccttggtgtgcaggtccatgagagaaccagcgcgatccatgaaggtcttctgcaacaccgtgtccgcgaaaccgttgccggtcatccgggcagtggcgaggtcgttgaactccttcgccatcgcctcgggaggaagctgccgcaactccggcatgcggcgcagcaagtcgctctccatttcattgacctgcgagagcgtgttatacatgctcgcgccaatctcgtagttggtgtcgccgaagattttcttgtaccacggttcggtcgcagcaatctcgtccatggtcttaccagcgcgggcggctacgaagccatcccacatctgctgctgcttcagcttggcggtgttcggcgctgccagctcctgcaagaactctggcaggttgctgtccggcatcgtcataccaccagtgcttgcgaaccagtcgttgccggattgaaccgggccgaccggattcacaccagcgccttgaatgctggtgttgcccgacagtgcgggggtggcgttgatgccaccctgcaatgcgggctgcgtgttgaaggtaaccgtgccgatgtcagccattaccatgcacctcctgagttgcccccgctgccgctatcgaaccagccgaggccggacgtagtggtggagaagttgtcgtagttgttgccgaagttgccagtgaccttcgccccagtcacggcctgcttgccggtgccgtcgttgtacccgaaggtagtggacgcccacgacttgccgccgcgatcattggactgctgccatgcctgcatgccgttctgcgctgcgttgctgaaggactgagaggcaccagtgaagttgccgttgtccgcctgccacgtgccgaccgcgaagtctgccacggcctcgcccgccatcggcccaccgaagtaggtagcaacggccacgccgatcagcttgcccaagcgacgcttcatcgcctgcggctcgatgtgctgcgagtagtcgaactgcccgaacgaacggctcatgtccatcccgttccacgcacgcgacatgacctgcgcagtctgcgaggcaccacgcgaggcgaggagagcaacagcgttggcctgcgtctcctgatccatttccgcctgcaaccgcaccatcgaatccatcaggtctgcggacgagccgccgacaccgacagcaccggcctgcgcctgaagtgcaccccgcgcgttcgccagttggagctgggagttaagcccagccccttggcgcgcacgcagctcctccgacagcgcctccatgttggagttgtactccttcgcggctgcgtccagttgggcgttgttcttcagggaccgcatgaaatcagcgaagccggtcttggcgacctcgctgcggttctgattgtcggtctgcgcaacggctgcacggtagttcgcacgggcaactcgggtggtgttgttcgcttgcaggatcgtattaaccgaacccattagctaaccctccgtacattgttgaaagtctgacccgtccagctcaggccggtcacccggagcgggagccaatccttgctgcgaatctcgtaggtgcactcgcgcacttcgcgtccaacgctgatgttgagctgcccccggtacaccggttgccgcgcgatcaggttgtcggagtcgccgaggatgcggccctcgaagtccgtggtggtcacgttgctgttgcgtgtggtcaccgcagcgagcatgcccgcagtatcctctacgtccaccgtcaccttgttgagtgacatgcgtccgtcgagtacggcctgaccattctgatcccgagggaacgggttggtcgggatcaccacagcctcggacaccacaccgtattccagcgcaccagcgtcgaggtcatcgaactgggtaaggaagtcggacgcctgagcgtaaggacagccgagcaggaagtacgggctagtgctattgacggcgatgctcgcgctcgcggtcagtacgcccgtaggtgtaccaaaactcgcccagctatcgaggcacgcatgcgagtccggctcgcccttcgggtcgaacacgtcgcacgccaccagcgatccgcgtgcggtgaacacgaggccgttcttcttgtagctgctcacgccgatgatttcgcccagcgccgggtggtattggaacttcgaccacgagtccacgacacgctgcccgttgttcttgttgtcctcgtaccggtacaggtagaagtcctgcgggtgctctcgcgtgcggaacatgacgaggttcggtgccgtgagcggagtgatctgcaacggcgtgcccgacagccacgagtccagctcgttggacatttcgtccgtcaccgtctgctgcccgttgagtgcgccgactcgcatctgatgcaggctcgtgccttcgctgccgtactgcgcgtagaagatgtagttgcccgaggtctgcgccttcgcatccaccgaatccttgttggcactgaacgccttaatcagtggattcttgggactgaacaccgagtcgccgctgatgccatactgctgccggtcaccgaagatcacgaggtttccgttgtagagcgtagcgtgccggagcacgtcgccctcgctaccgtgagcgaagatttcgatggggtcgctgtcttcgatggtaacggcagagccacgccagaagttcaggtagtccgccgagcgcgaggagttgacgtagttctgtgctccgatcaccagccggtcttggaagacggacagcatcgtgatcggcttgtcgatgaaccacgggatcggcgaggtcagcccgtcgcctgccacccgcgcgccgtaagccggatgctcaccgctgcccggagccagagacgtgaggccagcgccgttacgcgcgatgtagcccacaccgttgtagatgtagagctgggacacgaggttgtcgatggtgcactccacgccgggcgcttcataccagtccaccgagccgtagcccgaagtctccccgttctccaactccgcacgcaggtagtacgactcgtcagcgcctgcaccgctcgggcgcacgcggatgatcttgccgtgccaatggaacttgacggcataggtcgcgtcggtaatctcctgccctgcggcatagaaggtcgtgccgtcgccctcgtcgtcaaccgttatgtccttgaactggtcgtcgtcaatcacgataccgcccttgatgtacgtcgccgacacgcctgcatcgaccagcaaatccgacagctgctcggcgatgtactccgggcgcgtctgctcggcgctcgtcacgatccactcgttgactgcggagttgtactcgttcactctgtcgttgacatacttctggtacgccgggtccggctccgtaccaccgggtaggtagaacgggatgtcgctggtgtcgagcgtgccgggatacgatgcggtcaccgtcttgaacgtcaccgtaagcaccgtgttgtccgtccgcgtcaggttcaccgtgtacgtggtgttgtacttaccgctgcgcacccacgctgcgaggcgctggatgttcgtctgctcctgccacacgttcgtgctagtggcggacgggatcgtggtgttgcccgcgatgtagacgtagctgccgatggctgcgagcgacgatgcgccaccgctgaccagcgtgttgacccacgtgctgttctcgtacaccagcgggatgaacgactcgtccgtcttgttgtagaggaacgcgaaggactcgcttcccaaggtcgaggcgtcgcgccgatacagcagtgcatactccttgccctcctgcatgaagtcgaacacgtccatgttgcgcagctcggccgaggtgacaacggcttgggaagcagcgaaccgcgtaccacgacggcgcacgaggccgttcaccggatcggacagcacgttgatctgctcgtgcgtctggcccggacgacgacggtgcgccggtttctgactgacaccctgaaggatgtcgggataggttccgcctgcctttgccatgttgcctccttagccggggaaagtgtagtggctatgccacgggtgtccgctgtagttgaagtaccgctgacgcagcacgtccacggatgcacgagcgaacagcgggttcgccttgatctggcggatgtgctcggacttcaggttgatgtagctgtcgtcgcgctgctgcttgatctttgcgtacttggtgttgtcgccatcgaagtccgactggaagcgcagcactgcgtcgtcgcgcacgaacatctgcacctcgtaggggaggtcatcgaagtccagcagccgaaccatcttggcctgcacgttgtgatcgaactcgtatgtgttgcgcttgcggtcgtacagtcggcgtccgcgctgtaccacgtggccgaaccggctcgggttacagtccagcttcagcacgtccgtggggaccatgatgtacttgctcgttgcctgcggcttcagctccacccattcggtgttgaaccacagcgcgagcgacgacacgtcgcgggtaacgcggtcgatcaagtcaactgcgtcgtccttgtatacgtggtcatcttccagcgtgttgagcttcgtctcgcccatcgtcttcaagcaggcgttcacgatgtcgagcttggtgatgaatgccatggtgtctcctgagaggaacaaggcagagacgccggagcgcccctgccgggatgttgcttagtccgcagccagagccagcgaggccggtgcgtactcgatgtcctgcgagccgatttcgtcatcaacgaaacggacgcgcacgacccagcccgagccgatggcgtcgtaatggacgcctacgacggtgccaacggagttggcgggcagaccggccacgccagttgcggcgacgacgcggttggaaatctcgaacggtcgatcaaagaccatgatgttgctcctgtgttggtggaaggcgaggcgcggtttgagttacccgaaggattcagggaccgcgcctagcggattaggcaaccttgtcgatgcggcccgcgttctcgacgcgatccagaccaacggcgaaggacatccacgagtccacgaagtagcacttcgaggcgtcgctccaccacaccgaggactgcaacggcagcgcttcggcgatcagcagggccttcggcgacacggccacagcgatcagggtgctgaagtcgccgtcgtagaagtcgtcgttgtcgtcgttcgacagcaggtgaccttcgatcacggtgttcggcaggttctcgctcgacagcaccgggacgccccagccgtggaaggtcgggatgccggtcagcttgttgccgtccgaggtcaggtactcgccgttgctgatctgctctgcctgctgcaacaggtagaagatcgccgggcgcacgatcaggaccacgccatcacgctgcggcttgaccttcttctcctcctccatgcgggagaacagcttgccgatggcggcgtacaccttggccggatcgttctcgtcaccggcggcggcgagcacgacctgcgtggcaccgaagtggccctcgggcgcgcggccgttgcgggtgaagatcgactgcgtggcagcagcggccttggcggcggcgatgctgatggtcaggtccacgaactcggcgatttcctgaccctgctcgatggcgatttccttgcgggtgtcgatgtcggtgaagatttcgtccagctgccagatgctgtgacgcgacagcagcatggtatcgacggtcaccgacgccttgctgaagtccaccggggtgccgtccggcgcgtcaccgcgcttcagcttctgaagcttggtacggccgatggccttcttggtcagggtgttggtgcccttgacctgcttgcgcgggaagaacttttccagcaccgagctggacacgtaggtgtgctcgacatcgccggtgaactgttcgaggatcagcgcgttctcgttgccggactggttgacctgattcggcagaaccgggacggtcgggaagatggtgctcatgctttatgttgctccttggttcttagtggatgacgcgcgcgttgagtgcacgcagttcttcggagtgggccgcaccacggatgcccttctcggcaaccagcttgcggtactcagcgcggtactgctccttcgtgagaggagcgacgccgttgatcgacgcggcgggagcggcggcattggtagccggtgcgcccttgacggtcgtcgcgggattggcctgtgccagagccatcaggtaacgcgcggtcgcctgagcgccgaagccaccagccgacagcgattcgcttgcctgcttcagttggtcggcgggcaggttggcccgtgcgaactgctggatcgcagcccagttctctgcgccacccacggcctcgtggacagcagcaacgttcgcggtgtgtgctgcggttgcggcagcggtgacgcgagcgatgctctccttcgccagagcgaggatcggtgcggaacccttggccttgtcgccgaggacttccagcttggcttccagcagggcgaagttgcccttcgctgcttcggtcagttcgcggctgtcgatgtcgaggcccacggtgttgacgaagtattcggccgcgatgttcaggccgttgtcgccgtagtccgggatcgccacagcagtcggcgcgccattcgccggggcggcgggctgtgcgggagccgcaggttcgagactcagcgcgtcagcagccggaggtgcagcaggagctgcgggctgtgccggtgcggcgggtgcaggctgaccgttgggcagcagcttgtcgtccacgggagccggagctgccggtgcgggctggttgccgttcgaggttgcgatcacggttgcgccgggaccaccgcccggaggtgcgttggaactcattgtgtctgtgtctccatgttgttggcgttatcgacctgctgcgatgcgttctgcatgaccagctgctgctgtgcacgctgctgcatcatctggccgtactcggcctcagtcagtacgtagatgttcgggtccaagccaccagcggcggcgaggtctgcgatccacgcggacagcttcagtcgttcgagaatctgcggcggcagcgcgaggacgttggctaggttgctgccgaactccaacagccggtcacggtcacccgtacgggagagcgcggccaagccggtgatgatgacaggctccaagtccttgcctcggatgtcgcggcccgtcaggttcatcacccaaaaggcaacgggtacctgcacgtcagcggcgatacgggagtaaccaccacccagcccgccttccagttcttcggcgaccatgcggatttcctgcgcggtcacacgttccgcctgacgagtcaccgccgtctgcaacaggaagcctgcgccgatgcggttgatgtaggtggactggattgcttggttggtttgcagcacaccatcgacgcctgcgttaatcagctcgatgtcgcccttcatgccgggaatggctgcgccgtttggcgatgccatgaagtcctcgacggaggtctgacctgcggggttcaccagccaccggaactcggaagcgaggatcgcgccctgtactgcggcctcggacagcatcgagagcgactggaagtcggcctcgtagtcttcgaccaagccggagccgtagtcatcgcctgcggccaagtcccagctcaccgcccggtagggcagcttgtctgcggtgtaggtcgaggagaagttggcgggcagcttgcagttgcaaatccacacgtcttcgttgtacttgccggtcttgtggtccagcttgacccacttgtactcccacaccattccgtcgtcatcgggcttgaagtccgggtgcgcgacaatggcagcgagtgcggctggttccagctgggtcttgtgcaccttctcccgaaggatcagctcgtacacctcgccggtgcgggtgcgcttgaccacgtagtgccgcatgttgagcacgcggatcgtgtccttctccaacaccatgagggcgttgcctagtacgatcagcatcttcagcaggtcgtacagtcgggatcggattgagcgcttgtccagttcgagactggcatcctgctcggccttcgcaagcatcgcctgcatggcctgcaagtcagcgccctgttcctgagcagcctgcttcgccttgcgcttcagctccaatcggaagaagggtcgggacggagcgaacagcgacatcatcagcttgttcgccagatggttcactgcctgcgcgccgagagactggaacccgtgggtcagcggctcggtatcctgatcgcggttcttgcgagggaacagcttcggcacagtccagcccgaatagcgttcgagtcggtacatgatgccctgacgcttgttgtcgtaagcctcgaactggcggtgagcggtttggatcgaatggtccatgctcacctcacaacaggtctgacccggccacagtcgtcagccgggaagctgcggtcgtggtcacgggtcgggtgtaggtggagcgggcggtcttgcgtcggccgatcaggtcggcagtctgcaagtcgaggtcggaagttcccagccgcacatcgacggtatcgacgggggcactcagcaacttctcggcgtactcagatgcggcctgctgtgcagctgcctgtgccatctgatcggccatcgcctgaatctggtagttcgtggattgagtttggaggttggtctgcttgtcgatagcagcagcttgcttcagcgctgcccgcttggcggacccaccaccaacgatgctacccataggttaactccttcgcttggtgaattggggagcatgccgttccagcaggtagccgtagcgtgcatacatccgtgtgagcgctcgtgagttccgagctagtgcaccgcctgcgctcagtgagtcgcagtggttgatgtcagccagatgttccatcacggctatgtaccggtcgaaggaactgcccggcccaattcgcagcaccatgttctcaacgaacgtagtacggttcttggagtaccacggtgtgacaatggcaaagcatagtaggtaagcttcatcaatgattactgcatccactagaccctgtgttatcagggccactgtgtaatcaggatcatcacagttgtagctcacagaagattctctgttgtctaccttactatcttctctagatgacagatacaaagcggccgttaaagccgccttgatctgctcactatcacccgtcgttggtgttcggtacggaggaatcaacggtgaaaccctcctgtaagatgttcaggacgcgggccatccccaactgcatacctgcctccaagggcgtggtatttgagttgacggacagcgacagcccggacagtcgccgcacggcggccagctggttcgggtggagcgtcatcaggactttcactttggcgtcttcggccatggtgtctcctctgtgctataggtgtaccaaaaggtccggcaccggttccgcttactctcgcggccgctccaaccggacctcagttgcctcgtgctataggtgtactgaaactccgtcagctgaagaagtacggagaatcaaggacttgccgcaggtccagctcgcccatcggcggcggctccggcaggaacgggtaggccgagtggaaggccgagagcacatcgtgccgctcgtacatcgacacgaacacctcccggatgatccggtacagggccgcgctgtcggcggcatgggtgccgaagtcgtcgtggatcatggcgaaggcgtcgatgccctcggccttggccgcgttgaccaccagcgtcaggtggcttgcgtcgaggctgtgcacgaagttcggggcgatgccgttgcggtgccgggacttcttcaccgcgtccgtgctcttgcgcagggacagcttggcgttgccgcacagcttggtgttgatgcggtgctcctcggattcccagtagacctgcaccaccgggaatccggacggcgtgatccaccggatgcggtcgtacccttggttgaggatcgacccggagccgcgctgcaaccactccatcgcgcccgctgcggcgaccacggtgtcggcgatggcctcacccatgcgcttgctcaggaagcgcgctgcggggccgtacagggccttgtcgagcgaggggaacttgccgcacttcaggtagtcttcgatgatgaagtccgcccacgaagactgccgggagccgtagggcagggtcatcacgctacgcttcaccagcgaacgtgtgaggccatggtcgagccacagcgtacggtacccttcggcatcctcgtcctcgcccagcaggatcgcagtcacgcggtctgcgaccatctggtagatgtcattcggcagcggtgccgggatcaggttagtcgccaccccgcctgctgcgtcgcgcagcatcgccgagaagttctgaagcccattgcacgaaccgtccatgccgactgcgatgcggctcaggaagcgatccccgaacacttgccactgctcgtactccatgcaccagctcagaaattgcagcggcttgtcggcggtcttccactcgtcgttgtgcaccgggtccgcagcgaacgccattatctggtcgtgatgctccgctacccacttcacacgatccggcagagacgccttgtcgtatccccatcggtttgctcctgtgatgcagaaccaatccttcgcgtccttcgtcagcaacggcttaccatcggcgaactccaagagtgccttctgcaagtccgaaccctgcggcgacacgccggtcgtctgcacgtacttgcggccgcggaagtcagcgaagtacacgaagtagatgctcgggtactcggcgaacttgcgcgccaccttcattgcgttgtagaatcgattgcccttgttatgccgcaggcgctcgtcggtgtgccagttggacatgtcgcgcttccactgcttgaactccaactcctgattgtgggacatggtttccttggtcatgtccttcgtcagccactccggcttgcgcggcttcggcagctcgccttgcgaaatgatttcctccatgtcgtgcaccttggcgatggccgacacggcttccatcagccgcttgttgatgcgccacggcacgcgctgcaatgcgttgatcgcggacatttcgttgcgcagctcggcggcgcggtactcgtctcgcgtctgagcgtaggtcttcaccatccacggattgagccgacgcatttccttcgtgtggaatccaccgttgtcgatgtccacccagtccatcggcggttcgacgcacggaagatagaacggcgtagcctcaatcacaaagtcgctgatctgcgtaatcagcttgcgcacctcgtcagtcagcacgatcttgacgtgagtcttggtctggaacttgcggtacgctgcgcctgcactggcagcagtctcggttactacgccaatctccaacatgcccaactgggcgagctgatcgcacaggtacgcgccgacctgatcgcgctgcgcttgcccccactccatgaactcgatgccgttcttgcggccctgcatcttcatcaccgtcatgcggtggttctcgttgacagagagcttgcggtccatgtcgttcatcaggtggtagaacagcgtcggctcagcgtcggcgaactgcgtcagcaggtactcgtggtacacgttgatgccaacgttcttcagcacgtcgcggtcgctgccttcgccgtgcttgtcccgcatgcaggaggtaagggcaccacgaacggcaacgaaggccacagcctcgtaccactcgcgtgcctgttcctcggcgctgacgggctgtccactcttgttctgacgctcgggatcatacttggcgcgcagaagtggcacgtgcgcttgggcacgaccgatgcgcggggagtcgatgtccgcacggatgcgctccgcaagcggaagcacgaaccggcgatacactgcttgggcgtaggggttgttgtccgcgccgcccttctcctcgttgcgggcgatggacttctccatgcgctccttaccgaaggcgtaggtttccagttcgagttccacttgcgagagcatgctacctccgttgcttgatggtgaagtccgtcggcgggtagcgcttcaggatcatgcagaccagtgcggtgtgcatttcgttgatgatgtgcggccacgcaggaccaccgacctcgtagctcgggatgcactggcggttgaagaactgctcggtgccgcaccacgcggtggcagtcacagtgacgtgacctccaccgtagggagagaagcggtcaccgtcgaaatccagctcgggctttccgaatcgaatgtccatcagcccctccgttcggcgaggaagcggtccagcgattcgatcaccgcatcgcgcaccgtctcgttcggccacagggaaccggcgtactcacggaacgggatgctcactcgcacctccaccgtgtcgcgctccatgttatgccacacttcggtctgaacgttgctcaccggtcggcctccttcttgtcatggcggatgcccttgtagcgcggctcgcgcagcaggccgtacttgctgaaggacatggcttcgatttccacgatgtcgccgactacgggaacttgcgaaagctggtgcggcacgccgctcccgacctcctgctccttaccatcgccgaggtccacgaacacggtgtagacatcgcgcccggtcttctcgccgacagcacggccgatgcgtagcacacgcaggtccagcgtcagggtaggcttgaccttgacgacttcgccgttcgtgcccttgtcgcccttcacccacttaccgctcggcttgcgcaggatcaggccgtcgtatgcgccgccctcgcacaacagcttcgccgcctccatgctgcccagctcttggtcgatcaggaagccctgcgactctgcgtagaacaccggagcggtgccctctgcgatggcatggcccatgctcggcaggcggctgacgcgctcctgatacacgaggtcgctgaaaccctgctcccattcttccagcgtcacgaagtcgaacaccacgaacatcggctcggtgtactgcgtgccatccttcttgcggaacatgccgctgacggtgggctggtcgatctgcgggtgccagtattccccgaagtacacgccgaccgggaagaacggcgcggatgcgagagcgttctcgatgtggtgcgcgctgacgacctgctcgccagtccgagagaacaggtcaaccaccccgcgatccaccggctgcatctgcacgtcgcccaccttgattgcgtgcagacccttgttcactgtcggcacccagtggccgcgcttgatggcgaccatgttgcacccgtcgtacttcggctgtgcgatgtactcggtgcgcagctgctcctcggtaggccgcagcttcttcttgatcttgtcctgctcgactgccttgtggacgatgtagctcatgcgtggtccctccaaatctggaacatggcgagcggcacttcgtaccacggaacgtaacgctcccagtacgtggccttgccgtcgtaccactgcacgcggaagttgcccttggtgaaggcgcggttgatcttgaagccgcgcttgcgcttcttgtagccgggagcgacccggacattgctgcgaggcacatcaaacatcggcgctgtcctccttcttggtgccgtcacccagtgcagcgttgaactgcgcgatgcgggatgacatgaacttgttgacgatgccgccgatccacagcttgcgaggggcgagggaaccacggtacccttcccactcgtcggcgatgcgggtatacagctcggcctgagcctcgtcgggcaggttcgggaacccggccttgaccgcgttctgcaacgcctcctcgtggtcagcactctcgccccacgcaacggcgttctcgtaggacttgataagcatggcggtctggttcttgtagagcattcatttctccttcgacgggaatggaacgaaacctgcgaggcccttcatcacgaggatgcagaaggcgtcgtcagggtatgtacgatgccagagcgagttggcccacacggcatcgaactgcttgcgggtacggtgctcctctaggaagcgcgcccactcggcctcatgtgggacgtaccgatgcacttggccgcagcgggcgcaggccattagtcacccttgctgaaccaacggcggatgatgtactggcggatgaagcttatcgccgtgaacgcaatgccgatggcgtgcgccgaaagcagcgggtgctcgggatgccacagcaccggcagcagggcgatgttcgctgcgtagttgatgctgtacccgatgccgatgttcacccaagcctctttgatcgagcgcgccttactctgcgccacggaccttctcctcctcgcgcagttccagctccaacaggaacagctcgttgatgatgtggtgcgcccggtggtggattcccgtctccgggtccagcttctcgccgaggcagcgcttgttgtcgtgccggtagctcgcgtcctgataacgttcgagcgccttctccacgtgctgccacgaatgcgccttgtacttctgcgcaccgaaggtcagggtgtcgatgacacgggccagtgcacgcggcacgccctcgtgcagcagccgcgcctgcggcttaccgccatcatccttcagcccgacaccacggtcggacagtgtgcgacgatcttcgtcacggtagttcagtgcttctggcaagggaacctcccttcgtgcggtggtgacacctcccacgcccatcaggcgagtgaggaactgcgggcggatgatagattccttcagctgcccgtcgaacagaactccaacatcaacggcgctgatcgagcgaaccacgccggacctaccgacgaggcccggagcggagccggtatagcgtacgcggtcgccgtggcgaacgtcggtaagtctcatgcgcttctccttacgcgggaacggtgatgtgcttgcgagcctcggcgctggtcgtgagcttgcgcccacggctgtagccgtcgcacacggtgcactgaagcaggaggtacgttccgacctgcgtacgggccggatcatcctgcgggatcatttcgttgcagccgcacttgttgcagcgatgctcgctgccatcggccttgtagtacactgcgacgttcgggtgctgcgagtaccaaccgcgcagcttcttgtactccaacttcatggacttcacgtcgattcggttgtacgcttcgcactcgtcccatgcgccgggcaagctctgcatgcaggccacccacaggtcgaagccggggaagttgtggtggtcgtacttgcgcagctccggcacgatcacgccggtggtgtactccaacttctgcgaggtgaaggcgaactcggtgcggttcagcagcagtgggtcgatcacctgcaccggagacacgggcgggaacccgaggatggcgaggcgcgccttgatcttgcgcaggtcgaacttcttgccgttgcgagcgagcacgaagtcggcggcgttgagcagtgcccacagcgccttgccttgcttgcgatcatcgaacacatcacgcacgttgcgctgatccatgtagaacgactcgtcatcgtccagccactcgcaagcgaacgacatcagcgaccagtcacgcttgatctgcttgacgctgaagttgttgttgaacatgccccagccgtagaactcgatggggaatgtctcgatgtcgaggcagagaatcttcgggccgcgcttcggtgctcggcgaatgaactgggtaagggtcacggtgtctccttgttgatagcccgacgctttcgcgccttcgcattgcgagcgatgcgcttctcgtcgtcggtcttgaaggtaggatgcaggtaccccgtgatgttggtgaggtgcgaccgcaggtagttggggatgcccgcacagaatgcgaacacgtcgcgcacgccgtaccggcctgcgttgttctcgaccttgccaagcagcgagttgcatccgcgatggagcaccccgcgcacagcgccggtcttgtggtcgtggtcgagcaccggatcgagcggagccttcaggccgaactgtccctgacagagacagcaccggttgccttgctccgctgcgagcttgatgcgcagcagcttgacctgtgttgcagtgagtcgcttcatgctttgtatgcctccaagattgcgcgcttctcgttcacgtcctcggcgaggtcatagaacgcctgcttcagcttcggcccaaacacgtcgagcttcagcacgtcgagcagttcagcgtcacgatccgtccgcatccacaacagcacggcttgctcggcgaaggtcttgcgccagtcggaacccagcacctcgctgtacttgccacgcaccagcatcgctgcctcggcgttgtccttggtaccgaacagcaacgtctcggcagtgaccttgcccacgtcaggcaggccggggatgtggtcggcgctgtcaccgtggagcatctgcatccagaaccacttgtggccgtactgcaaaccgttctcgcccacgatgtcgtaagcgccaagcggaacctcggtgatgtcgtagccgtcccagtctacgtgcacgccgcagaacattcgcatgtccttgtcggcgctgtgcaccacgtgcaggatgttgtggtgcaatgctgcaccctcgttgacgtacgcgatgccgtcgtcggcctcacgagtcagccagattttgggagtgaaagcgtcgccctcgtatgtctccatccactcacgaaggaacgcccagttgttgggcttgcggcctgcttggcgctgaccctgatacggctgcgtggtagcagcgaggaagcgatcacccttggtagacgcggcgtgcgtcaggtgcatgacgatcttgcccgctccgctgacatgcttcagctgtgcgcagcgggagagcacgttgcgtcgtgcatcccccgccgagcagttctcgctaccagccgcgaagtacgccatgtagtccccgtcaacgtgagcgatcacgcgcgggttgtgctgacgtaccacttgcaccggcatcggggagcgctcaccggccgctgccatgagagcgctcaggtccatcaggcgatgcccgccatcgggtcgctaccatccaccgggaacggcggcttgtcgtcagccggagcagcgtcggtagccgcagcgttcgccacgtcgccgaccacttcgtccagcgcatcgacgccttccttggtgaccgtgctgctgcccgacaacttggcggcggcgtagtcgtagcacggcaggcccttgaagttcagcgccgcagcgatgcgcagctgcgtcttgttcttcgactgcgcttcgtgagtgaccttgccggtcttctcgtccttgcgctccgggtactcgccggggatgtagatgctgtcccacatgtcggcatcggcgaagtcccacacgaacgcacccagcggggtgatctgctgcggtaccgggatcacggtgtccacgaacttgccggtggggataccgttctccatttccggcaccggcatgaccggcttgcggatggaagccttgtcgatttcggcgaaggtcttgttcgggtcgcgcttgcccggcttgtggatgacttccagcagcacgccctgacccagcagctgcacgaagtgtcgctcctcggtgcgcaggcggctgaagattttgaagtagtgcgccttctcgttggtggacaggccgagggtcagcgtcatgcgcaccggcaccggaccgttgtccgtgtcgatgtgcgggtgctgcttgccggtcagctcgaacacgatggcgacttcatcctgcgtcttcttcttgccctcgaactcgaactcgtgcttgcccagctcgtagtacccgacgatgcgggcggtggtcacaccagcagcgggcggggtgtagtcgaagttgccaccactggcaaccgactgatccttaccctgcgtggcgaccttgttcaacagtgcgtcaagactcatgcgtgttgttctccttattcaaacgacgggttgtgattaccaacgaagtccttgcggatcgacgctcggtactcgatgaccagaccggcgaactctgcgggagggttcttctcctccatcatgttgtcgcccatcttggtttcacacgggacgccaagtggcagcgtccagttgaaccaccactccatatacaccgacgcttccagcatcgaggcgtgcagcagagcagaggccttggttgcgatgtcgccgtgtgcatccacgtagacggcatcgtgcacctgattcacgagcagcgcgcggcccaaccattccttcggttcggtcacgtacttccggtagaaggcgcgcaggctgacgtacatcgccgccttggcccactcaccaccggtgccctgcatcgggtagttcttgatttccgtaggcgagaacgactgcgcacagccacccttgctcgcgggcttgttggcgatgaacaccggggacggtgactcgctgaaggaatacatcttgccgtccggagtggtccagtgcgaccggccaagctgacacgtaagcccatgtggcacgccttgctgcccggcgttgggatgcggaacgaagcgttgcgtgctgacgcggttgcgcttgatgtgctcgaccatgcggtcgatgtactcgcccagctccgggtaacgctcggcctcaccacgcaccagcgcctcgacttcttcctccgacatgccggtggtcgcagcgatcttcgccacgcccgcaccgtacgcacgctggaaggagaacaccttcgcgtttccgcgcttcttcttccacttcttgtgctcgggatgcttgtcgtccttgctcgccttcaggatgaagtcgtagtcgtacttgccttgctcgccccacgcctgctctgcacgcaagcagtgcatgtcgaggccccgcttcaagtcctcgatcagctgacggcactcggtgaggattgcctgcacgtagatttcgagggaggtgtagtccgactggatgatcttgccacccttgtgtcgggacacgaaggcgcgcttgatctgcgaacccttctcctccaacgtctcctcgtccagctcacccttactcacgttctgcaagttcggatcgctggaagacaagcggcccgtgaccgtgttggtcatgttgagcttgtggtggatgatgccgtccggcccgaccagcgtgagcattcccttctgctcgccagtcttctcgtccgtcgtgatgtagtacgtggacaagtccttgtgcaagtcagcgcgccgggcaagcgccttggtgaacggcaggttgcggtagcccagcgcctcgatcacatcggcggcggtggagtacacaccctcgtcgctcttgctttcccacgcagcatcaggctcggtgtagccggggaactcgaacagcatgtcctcgttgcggaacttctgcttggtcaagtcatcgaccttaaccttcttggtcttgtactcccccttgttcttgccgctgccgtacgtggtgtagcgccacaggttgtcgaagtcctcggccgggggcgtcgccgtcgtagtaccatcgaccagcacgtagtgcacctcgtccttctgcacgtacgtcggcccgccctcggtggacatgatcggaaccttggccgtgtacttcaccttgccaccgaagatcagcgcgctcttgtggaagcggctgttccagttgaaggtcagaccctcgggcaactcggggatgaagccgttgagttcggcggtcgccgttgcaagctcgacctccaactccttcgccttcgcaagcgcccagtccttgtccacgtacatgccgttgtactcggcttcgatggtgaagcacagcgcacccatgttgagcagcgccgagcgcaaaccaccacgtgcacggaaggcagcgagctgaccgaggaacatcttctcggtgttgccgatgtcgcccacgtcgtcggtgtcgttggtgccgaggagataatccatcagcagcgtcttgtcgatgtcgcaggtgtccacgcccgcagcccacagggacttgactgcatcgtccttcaggttgccgccgtagcgtggggccgtctcgtccatgctcgccatgtggaactcttgcgtcataccatgaagcaggtactccgcaagctggcagtcccacaccatgccgccgccgtcgatgaactcgatccatgcctgccgattgagcgggccttggcagatggcgtgcaggatgtcgaacttgatgttgaacccgacgaggaactgctgcccgtaacacagctcgcgcagccacccatcgggtgcgccgcccatgtactggttgtcgattccgatgcgggtgtcgtagtacaggccggtgttccgtgcgtcgcccttccgcttgtagccaatcgccacgatcttgttcatatcgtagaacggattggccttgcgcttcaggatggcacggatcgtggtttcgaggtcgaaggaagtgaagctcacagcggccaccgttgcagggccagctcgtacatttcgtcggacgcatcgccatccaagtcaagcccgtcacgcacccaacggaacacgatgatgcggtcctgcttgtccttgatgttgcggcgcttgcagatggtggtggcctcgaccgcgcgctgataccagccggagtcggcggtcaccatgacgttgaacacgccgttgcgcagcgcataccacgtgtcgctgtagtcctcgtcctcctcgtagtgcccatcggcaccggagcacagggtccatcccgcctcgaccagcttggcgatggcctcgtggaagtcctgcaccagcacgaggtagtcgatgtccgtgttggttacgggcggctcgacggtgtagctgctgccggtacgactggacgtgatgacgcccacgttgcgcggcaggtagatattcggttcggtactcacggcgtgttacctccgggcttggtgatccacagcgtgaagcacgggatcaggttgatgcaccagcgcttgttgtgcggcgagtagtgcacgccgatccatgtgctgtgcttgttgcgcaaccatccccacttccactgcggagcatcgttgcggccttcgatgtagcctgcgtcgtgtaccttgcgcatcataccagcgaggaagttagcctgcgctgtcgatgcacactggtacgactgcccaccgaagtggacctgcgcacacccatcgacgtggattttgtccttcgtcatgctgcctcctgatagaagcgggcacgctctgcgtccatcatcacttcttcccgaacgtcacgcttaccgcctgcgcggtgcagcttgttcttcggggtgccgatgtagcggaagcgttccatcgctgggtcattgagcttgccgcccatgatgatgaagtcgcacgcaccctgcttgccggtcttgctgtccttcagtgcggactgcggcgggtactgaatgccctcaccctcagcgctgatctgcgaagtcgccacgcccacggcgtcgtacttcacacaccagttgcgagcggcctgatacatcgcctccaacatctgatcggtacgctgtccgccgttggtcatgccaccggtgaacgtgatgttgtcgatcatgtcgaagatgatgaagccggggttggtctgcttgatgatggcctcgacctcaccggagttgaacccgtggatgtcgtagaactgcatgcggtggatgtccccgcccatcgcatcttcgatgcgcttgcggatgctgccatccttcgcccactccaccatctcagggatggtagcgccgagcagcgactgataccaccgctgcttgatgcgcttgcccggtccctcgttgttgagccagatgccggtgcgcttctggtccggccacaccgcatcgagctgcgtgatccagtgactagactcgctcgttaggaacgtggtcttgcctgcgtcgggacgcatggcgtagataccgaagtcaccgccacgcatagcacgcaggttgcgcgccaatgtgggcagtcggaagtggatgccgatgtcgtgctcgtccatttccatcagttcttccggcgtctccttgaccagcgggagccgcgccttacgatccatccggtcggtgatagtctcggccaatccgtacagctcgtcgcgcaggctgaactccgctccgccattccactgcacgatcttactgaccgcagtggtggcaagctccaactccaacagcttctcgatcatgccctgctctgcctcgggcgggaccggctcgcgcatctgcttcagcagaactttgagcagggacttcttgtcgtcggcctgcgtcttccacttgaactccatggcccagccatcgaacacatcgaacggcaagtccttcgtgtccgggaactccttgtagtacgcacgcaacgcatcgagcatcagcacggtcagctcgtccagcccatcacgtggtgcactgggtaccagccggtcgaacttgccacggttggtgcacaaccgcagcagcgtggtgtcaagactcatcaggttctccttcgggttcgtacttggaatcgagctggtgataccgtgtgttgcgcgtctctaacttgcgcccgccgtccgtcacgtacagcaccgtcgaggtgtgcacgatgtcgcagtcgccgaggttcggatgcgcaagcacgtcgccgagcgtggcacggaagccaacgacgggcgggatgatggcgcgccgatagcgcacgatgggtttgctcattgcagcttctccttgatgtagtcggtcgtgtaatacttcgggtcacgtggtgacgtgatgttcctgtagtccagaccaaacgcacgtagacgcgcagcgattactcgcgcgctgtcttggccgggattgctaccgttgcttctacctctgtcgtcatcgagccacgttgctacacgttggcctcgatcagtcagctgcttcaacactttgttgtgcagcttggtgccgagcaacgaccacgcttctgtgcactggcccaccttgaaggcggatagcgggtcttcgcatagcacgatggtgtcccccttgcccacgccgtagcgtgcgacaagcccatccttcggcacatcaggagtcagccatttgggctgacggcttgtgcttcgtgctgtccagtacacaacgtcgtcgccttcagtgatcggtagtaccacccgcccgatgctcgggcaccagtacagccgcagcttgtcgatcatctgaagcgagagtcccatcttaaagaaccacaccttcgcatcgagcggccactctcgggtgtcgtatacccgtggctctggcaactcaacagtcgcacgcactctgcgttcgctcgtctgctcggcgtggattcgtgcaagcttggcctctatactctcgtgctcacgcttgaatcctgtgccaccgcacctgaaacagaatgcggtggacttgtcatgctcccgagtgataagcaagggagtcccttccccgcaatcatgcggcactcgggtgcggtggccgacctgtagtcgctccgcatggtgcagccaatcgctgtcgggaagggtctcgctcatgctatcctcgcttgattactcgaacacctcgaagatgtcgttgtcggtggcgtacagcacggagccgttgccatcggtgctgacgatcagccggtcaccagactcgctggtcagcttggacaccacgaaaggcgtgcccttggtcagcttgttggtctgccgggtgtcgatcaggtacgcggtggtgccgggcttcagctcgtcgccgcgcttgactgatgcactgaccggggccgggctggacaggctcacgactgcccgccttcaccggcagcagccttggcggcggcagcttcggcggcgaggcgctgtgcctcggcaacggcggcgtcgatttcttcctgcgccttcagcacttcttcggccgacatcagcagggcgctgctgtcgatcaggttcagctcggcatccagaccttcgccggtctgcaccttcagttgcagcacgcccttgtcgttcttgccggtggcgacgatcacgccggacaggacacgcttgttcagggcacgaccgaacaggtaggacacggcgtcgccggacttcagcgcttcgatggctgcgctgttggcctcgaccgcatccagcttggcgagcttgtcgttcagcgcatcgaccttggcctgcgccttggcgatgtcttccagcagctcggcgcgcttggcttcgtagtggctgacggaggtggtctgttcggtggtgttttcgttcgacatgcggtgtatctcctttcattgacgggtttggttggtggaccgtaacgtgggccagtcggcacagttcagtgctggattactggaagatcagctcgctgttgtacccaccgccgccattgtagaagcgacggcgcagcacgctctcctcgccgagcaccagcaggcggtccacgatggcgcggatggcgctcatgtactggtccaccagctcgctctgcaagttcatgtcgaagcggatcacggtcaccgcctcgtcatccagtgcgccggtatccttgcggacgtacaggccacgggcattggtcatcgtcgcgccaccgatcagcttgacggcggcggcaatctccggctgcacgttgagcagtcggctgtcgggcacggtcacctcgacccagcttcccatgcgcaggctcatgctgcacctgccagtgcggactgcacgttcggctgcaacgatgcaccagcacgcagctcggcagcacgacgcttcatgcgggagcgcagcttgcggcgctgcttgttgttgtcgccgaggctatcggccacacgcttcagctggttgttgccgacgatgcgggtctgaccctgccccttctgcacggggaagtagtcctgccccagcatcttgcgcagcaccgggttgtcgatggggatcagcggcacgctgacgtgcaggtaccggctggtatccggtgcgggcggcggcgtgtcatcgtcgtcgtgctgcggcttcaccgctgcaaccaccttgtccttcacccagttggcggcaccgcgaatcttgccgccgacgttcttgatcttttccatgaatcccatggtttacttcctcctcgtgccgaagtgattgaactccgtctcgtgccacacatagtacgtggtgccgagcgggtcggtgtctgcctgccagttgcgctgggtgcagtagtcgttggctgcgtcgaggtcatcgaacgtcagcgagaacccggtggaagccgggccggtgcggaaccggcacagcctaccgtcgtcgtcatggtactgcccgacgacaacccacggtccacgacccacgatccagtacagcaggatcaggatacgcagccagagtttacgcatacaccgcctcgatgtagtagcccgagggattctgcttgctgcgcttgtcaccgatggtattatcgatgatgtcacgggcggcggcgcgagtcgggaacagcaggttgtcctcgctgttgttctcttcgtcaccatcgacgcgcaccgttgcgccgtcttcgacggagttgtagcagctggtgtagtcaccgtcgtacttgatacgccagcccttcacctgacgcaccggcttgcggatgctatcgcccacttcgatgatgtgccagttgaacaggccaccaccgttgaaggagttcaggatgtcggcctcggcacgggcggcggcacggcgctcgaaggcggacaccgggccgggataggtggcgtcgcgcaggctgtccagcagggactgcgttgcgcccttggtgcgcagcagctcgaccagtgccgtcacttcctcggcggtggcgttgcggcccgtgccattggcgacgacgccagtgatgacgccatcctttgcggtggccgggatcgaagcgatgaagtacagcttacgcatggtggttctcctcattgacgggtgggatttcgatttcctctacggtgtagagagtgggcaccttctcgtggtgcagacggtggtgtgcgatggcctgctcgcacgcctcgtggctggtgtggtgcccgccgaggatataatccccgacagcccaaccctgcacggtaacgagcggcagcgccttcaccacaaggcgcaggctgacctcacgcataccagcgctccacgctgtgctcatgggtcacgaactctttccactggcggggcttctcgcacagctggatcggcttgcgctttccactacggatgcgcttgtagacgatagggatcatgcaatatgccctcctgttgggcgtggttccaaagctacgccctcgttagaaggcgcagcggtagatcacgcgtggttcgggtgccacttcactcggtagcgacgcagacggttcgcatcgttgccgacgtgcgcagcgatggcattgcgtgcagcttgcgcagtggtgaccgttccgttgagaccggtcacgctggacgtgttccatcccagctgcgactgacgggcggcgtgcttggtgaagaactcggcggtgtagaagccgcgatccttctccgggccatcgggagtaccttccggcaccacacggtacgcatcctcgctgataccctgcgccttggcccgcgccttcagcatgcggtacgctgcattgcggctgcgctgcggcaggcccagctcacgcacctgtgcccagttggcaagggcgatgccgccgtggcgcagattgaactgcacgatccagcccttggcctgcggcttgttgaccagcccggtctgcgatgcagtcagggccacgtggcgtgcgctctgatcgtccatcagtacatccggcagcttacgcggcaggttgtcgggcattgccgggccgggcaacaccatgcggccggtcacgctgccgaggaagtccagctgcgaggcatccaacaccaccggaggcaacggagacagcaggcacgccatcacccgcgcctcgatagcagcgaagtcaagttcacgcatgccgtagcccacggtgaacgtcggcggtgcgaacaggtcacgcagcagctgcgcctcggcattgctgtcccggcaggccgcgataacgtcgtcctcgaattgcaggataccgtcacggtcgaagctctcgattccgaagtctcgcagctcaccgtgcagagtggagaactcgtcggcgaggtctttgcgagcatacggctgcgctttggcggtcagcgcacaggcaatgtgcagggcagcacgcagcagggacgcttcgcgctgggtcactcgcaagttgatcttgggttccatcatggctccttgaatcggtgggtgtggaaggctgtgcggtcgccgaagtcatcgacaaccacccagtattcgggaaaggtgaatccgttctccatcgtgacgctcgggaccacctcgactacggtgtattccttgccgccagtcaggcggaacagggccgtgtgcttggatacaacgacggtcccggattccatcacgcagtcgccttcaccttggcaggcttgggcacggcgcgggcagcgttgatgacggcctgttcttcctcggtcgggacataacctccctcggtcgccttttccagacggcccagcagcttgtgcaggtcggcggcgaaggagaacgcctcggcgggcttctcggtcttgaagtcgtaccacgccttcgcggcggcacgttccagcatttcggccagagcttcgccctcgacgcgcttgctcttggcaaacttcatcggcgcgctcgccttggtttccttgtcgtcgttcggagccatcgggccgaactcggacaggtacaggcgcagggcctcatgcttcatgccgttgcccacggcgagacacagatcggaggcaagcgtaacgtcgccgtggatgtgtgcatggttgatgaccgcaatcgcggcctgctgaatctggtccaccagcttggtgcgggcggtgttgatcgacttgatggtgcgcttgatgtcagcgcttccggtgatgatgtccatggtggttcccttcaggttgggtccgtgccgattgcacgacactaggccctcttgcgaaggcccagtagcttgcattcagtggatggtgggtgcagcgagcttgatgtcataggtccagcgtgcgccggtccattgcaggttcgatacagcgcccggcggatgcttcgccattgcccgttcgtggcttgccatggcgttgcggctgtaccctgcggcgaagtagaatcggatcacaggtaagccctccggtcagcggcgtggttcgcccggttcgtcccgctgttgccctcgacaacaaacacagatcgctttccagcggttccgtggcgggcttcgtagcgttcggcttgtcgcttgcgctcggcgagcttgcggtcatgctccgtggtgcgcaggtccatcacgcttgcagtccgggtgaactggcagaagcggcgcttacgctgggtgcggtcgagattggcattggtcgagccttgcatgttgtgcctccatttggcactggtgggaaaactaacagattgatgcgccctcagaaagccgtcgagtcggtcaatccctcattctcgattagagccgttgcatcgcctatcgtgggcgcacactgaccaccggatttgcctgcatggtcatcgcaaagggagggcgcatcaatctgctagcccttcgggctgtcaaccctactccggctagcagtgccattgtcaccgtgtggcccatagagccttttcacgaaacgcacagtattccatgcgataggaggctcaccacctccttatgaccggcttcccacctttggcagtgggttacgctgcgtggccgactctcacggcaaatgcaggccctaagcgttaggcttaggtaaagcggcaccagtgttgctagtctggtggattctatgggcctttgacatcccagttcatccggttatccgctagtgctacgttgtagcttggcgttccacccgtgggcttcacgttacaccctacccgttagcggtagtcctacccggtccagtgccggtggtcctcagaccgtggtgccatactagcaccctgtttgcatcctgtcaagcccttggctcgattcgggtctctaacccgttgggcgtcctgtcgccaccatcctaccatgtatgccggtagtccgcaaggtgctagctgctccgctgttccggtggctaccacttgccgcctatcatagctcactgctagcttagtgtcaagcgtggttcggtagctcctcgcatcccttaccagtgactcccatgtgcccttagcccacttgttggcggcgccactacggatcacgtcactcgacttgcgttgcagcttactaccattgcggccgtgtgtcaactgttggcctagcgggtagctaactaatcagctcgacagagtaccgatagacggtgattcaggttgagccgactctgtgctataggtgtaccaaaaggtccgaaacgatacagatggccctcacacgcctacagctgcgggtcgcatggtagcaggtaggtatgcacctgtcaagccccttgcggccctcctgaagccctgtcgctgccccagtgacgccattggatcacaccaacggcaccacgtcaacacctttcggcgggagatttatgtacgattcagctagcccaccacgtgccacggcaggagaggaaccacaggcgcacacgcgagcacgcacccatgcgcacccgcaggcgcgtaacgcgagggcgtacgggggcacgcgcgggagcttctattggagtgacccccgcgcatttgggaagcaaattttggtccggctacccgcgtggccttatgactaagccttgcgaactggtgcctttagcttgatgataggcccggagctgtacacatcgtgagctatcgccgcagccattgccttagccacagacttgctcgcatggtacgcccctagagctagcgccttgccgctgccatcgaagtacggagcctcctcgacccactgctgcttaccagtagtgaccgtgagtacgccgtccttaatcacaagcaccgtcgcggacttgccaacgtgctcctcgtagccttcgccgctttaagcgcagcgagaaccgggcgaagcactgtgaagtccccggtgacacccagcagcacagggccggtgggtgtcgatacgggcatgatcttgcgcacggtgtgcttgtggtcaccctgcgtggcctgactatcggcccacagatgcttgccgtcccatgcgatggtggtcatttgtcacccgtgcaccggcgcttaccggtaccgcacacctcggccttccacgcacgcagcgcagccttgtccttgttgcacagaacggtgtccattcggcggtcttgcgcgagcttgaccaccttgtcctgactggaagtgctgcccttcgcgccaccgaggtaggtgatagagcagtccttcagcaggtcatcgctcggaaccggaaggttcgcgcaggaggtcagcaacatcagcaggcacactgccatcgcggtactctggagctgcgtccagaacttcttcggtgcgtacacgcacatcctccttctctttgatgtaggttgcgtagccggtagcctgagtcttggccgcagtggacgacgcggaggtcaccacttgggcgttctccaacttatcgaccttgcgctgcaagccccacacgtacagacccgcgcagacgatgagcaccacgccgagcagcaggccgatggccttaccagcaagacgcgcactcatttcggttggggtttccatggttggattacctcactgttgggccgcatgcacagagctgcctctgcatcgcggcgcttggggataccagcacaacggctggaagacaggcggcagtcgagtttcccgacgtacacccagcggtagaactccttgcagctaccagctcgatcccctgagttcgccttgcgcagcatcgtgctgccgacgaagttcccctcacccacattgaacacgaagctcgtgtaggcgtcgatctggttccgctctgccggtactttcaggtgcttgcgcaccgccttctgcgcgatggcgaggtcttcgaccagccactgcttgcattgagcctcggtcgcggtcatgcccatacgcaccccggccgtgtggccgtagcagatggtgggcactttgccggtgtcgaggtacgccgagtagcgtaccccttcgtggccggtgacaatcgtcagcagcgtggccgatacgccgatcaggatgccgccgacgaggccgaatagccccttgttgctctggtcgttctgctgctgactcatggcttacggctcctcgggttcttccggcgcgggcagcgggccgctgttcgggccactggactcggtgcgggcctgcgcggcggtcagagccgcctgcacgacggcgacatcgccggtgaagatggcctgcaactgctcggcagactgcggatgctgctcggcgtactctaccagaagcagcagctcgcggcggatgtagtcgccacggccatacaggccggtgtactggctggggaaatcggacttcaacattgggttacctccggtaacggtcgagtagggatggacggccacgttgcatcggactcttgcgggtcgctgccttcatgccggttggatcgttgatccagtcttggaactctcgctgctgctgcttggcgatggccttgttctggtccagtgcaagctgcgcaacccagtggcgcacgctaccttcgagtgcatcgagcctgtcatcgtgtgcgatgctgcccttctgctgcgtgatcttcgccatctggtggaacaggctgtatacctgacgcttgccgctggatgcgtagcgctgggtgtactcgtgatccatttcaaccacggattccagcacgaccagcgagccgcgagccatgacaggttcgagcgtgccgatgatgcgggcttccttgttgccggtcacgaactcctcgcggatgtcgcccttgtatcccttctccgtgccgcgatcttctcgcaggacgggcaggaacaccttggcgaacgcaccgtagcccatgttcttttcgatgctgatgacgttcggcttgtacttcaccgcgatgcggcggagttcgagcaggccatcgccatcgtagccaccgggaacagcgcccacggccaacacgtacacggtggagttgaggaaggcggtcacggcgaaggccgtctcgtctccgttggcaccaccaccggccgggtcgatctgcatgtgcacgccctgcacgggggcagtctcggtgctcatgtcgtgcggcatcatcatcacgaagccgtacccgctggactggaagctgcgctggtgcgcgttgctcaggccacgggtgatagtcagcgggaagcggtcgccaccaccggggatcacgaccagattctcggtcttcagcgggaagcgaagcgcatccatcaaccgcgtgttgagcatgtagttcagctggtagctggacggtccacgctgacgcagttcggactggtgcttctgctcaccggccaacagctcgtcggtgcactggccctcgtcgcccatcgggccaccaccgaacgccaacatcgggtcggcttcgaggcgctgcacgatagctggtgccagatgcgggccgtagtgctcgcgctgtgccggggtcgggtagcgaccgggccagatgcgaacgtcgtagcctcgtccgggcagggtgttgtagatggagtcgccagtctgcggcgtgccgaggtacaggattcggccgggagtaccgggcttgccggtgcagatggccgagaactccaacgtgatggtcagcagcagctcgcggttcgcggcggtgcggctgttcttgttggactccacatcgtcggcgatcagcaggtccgctcgcttacccggcaggttgccggtgacgccgatacacgccacgctcggtgacttgtcgatgcccttcagtgagtgatgcacgtcgaacgcatccacggaggtgcggtcgcccgcgttcttgtccgggcggatgcactccaacgtcggcaccgtgaggatgatgcgctgaatcagcgtagcaatctcggatgcctgcgtgccgcctgccgatacgatcagcacacggtgggtgggatcgtggatcaggcagaagacggcgtagatcgcagcgatggtagacttcgcctcgcctcgctgtgcctgcaccattgcgaggtgcgggccgtactgcatgtagttggcgatgtcgtactgcatccacgtcggctcgaaccccagcaccttcataatgtcgcgcatgaaggtggcgaagtggcggtagtggttctgcaacagctccaacttgcggcgacggatgtctgccgcttcggctgattcacgcatggttggctacactccccggaaagttcacgatgttgtcgagcgctgcttgcagctcggtgtcgtcggcctgcggcagcgagtgcttgccgagttcgtcttccagttcgccgagcgccttgttggcctcacgcgtcgccgtgatgttgttgtccttcaggaacttgatcgcggcattgatgtcggcggcagtgcacagctcgccattggcgagacgttccttcagtaccgtggcgacgagttcgtgtagcgcgccaagcgcaccctcacttgctgggttcgacatccttacctcccatgatcttgcggtgctcgcgtgtgcgccagtagaactgggcgactgcatacagaatggcgagcgtagttacgatggcagcaccgtacgtgctgatgaagttgaggtagaccgcgccgagcgtaagcggcgaggttcggacgacctcattgaccacactcggcggggtcatgctgttctcctgtaggttaaggccagtcgtcgggattgccgacgagcttccattgcaggcggttgacgttgttcatgccaaccgcgatcaggtcgccggggattccagaggcgatcacgtgttcggttgcgaagcgctcacgctgcgcgcggacgcacaggttgctgccattcttgtacgacagcagtacgtcgctttgtgtggagaagatcgcccgcttctcgtccatgcacaggcggggt

SEQ ID NO: 27 - DNA, 42769 bp, unidentified
  source 1..42769: mol_type = genomic DNA
cgctagaacttacaccgagctccgtaacattgcctacgacagcaccctgtgcgaactggaagtagcgagtgcgggaaccccatacggtggtagcggttcgcatttgctcttcggtggagccggcaagggtatcgctctggtaagtgctgctagtgtaagcgagactcgacgcgagctggatgtcggtgaattctggtgtggtagtgcccacaccaacgtgacagtaggtgaggtagccattggcagttcccaactgatccatgccgctgttggtaatcaggttatcgaacttttcagtgagcttgcggacatgccgcacaccccgctcgtcaactcgtgcagcgaacagctggaactgtccgcgcacctgagcattaagaatcatgttttggtcatccctatgatagttggcataccagtcttagttctatcgacgtagcccgacgtgcggacaacgactttagcgctggtacctccggtgatggtcggcatgctggtcttggtgtagtcttccttcggcagaatgaggcggttaaccgcagactttgaagacatacctacgatatacggcatagcggcgagagcaggggtgtcttccagcacagcaacgcgaagaacggcggatcggctggacaaagacacgacacccggcatacctgctgtggcgtagtctagaaggttggcaccggcaccgagattgagttgtgtagtcggcatgtgtgccgcagcgtcgtcgtaaaccgagacgggatacagctggccgattacgtaagttgcatcgattccgataccgccacgccagtaggccacacggttggcaccgtctgtcaccttgatgtagagcgagtagtcgctgtcatcgtcttggcctagcacgtacttgtggttccacttaacggtgtccacccacagtggcttgttctgcttgcttcggaatgctgacagcaccacttgcacgtactttgtgtccttaggcgcggcgccttcggcgactgactgatgccacgcaccgttgctcccggacttcactaggttgccggagttgcgttgcagctcggttccatcctccttgcggtagatgatcgagacgcgcgcgccggccttgcccttggagcttgcgccctgctgaacttcagcggtgcagcggatgtagtcgttgaccttggcagggacaagcgggttgagcaagtcgctaccgcccgtcttgatgttggcgaagcgcgcgctgtacacgccgctatcggtgtcgtagtctgagccagtaccaatcgaccagccttcgccgttcgatccaccgcccggcacccacgtgccatcgtcgcctgcctcgaagtcgccgttaggcacgagtgtttcctcgtccacgacttcagtgaaagccgcccacttgacgacgacttccttggtgatgttgtccacacgtaccgcagcgcccgaagggagcgtcgattcgatgacctccacggtgcagcggccgactgggttattgatggacaggcgagactcgtaagcctcgcccgccgtgtacccttccagcacgcccgtcaccgacaggctatctgcaacctcgtccgccatcagcggtcggccgtacagcctgaagtgattagccatgcttactccttagccaagtcgcccgagagcaaccacgtgttggtgtcgccgtcgatgcacgttgcagtgacgacggaattggtgccgcgagttgcggcggtgcagccgaccggtacttcgagggtcacgccaacgtcgccggtgatgaccaccgggcctgccttctgctgaacgctgaagtagctgcccgaggctagcttcgtctcaccgtcacccacttcggggatcaggttgatgttgacggcgcagcctccagcatacgtgcagcgcacgagtccgtactcggtagccttcgcggcgtagtagatagggccttctgccgggatgatcggcacgcgcaggctcgcagcagtgatcggaggaggcccggtgtagggcttggcgtaaccacgcagcacggcgaaccagatgctgccctcggcaggaatcgtggcgaagcggatgaagctgggatcgctgccgtcggccagcgtgacctgatagtccacgtccggctgcataccgataccgttgacgtacacgtcgtagaagccagcgccggacacgtcagcgccaaccatgtcgaagtcggtgtcgcccacctgatcaccagtccaagaaccggaccagacgcgcggggctacggacacgataccaccagcggccagtaactcggtgacctgcttgtagatgttctggattatctcgttcaggtccaccaccacacctacctgctggtcgatgctaagggtggcgatgttcagcgaatcgaacatttcctggatgatcttcagcaactggtcattgctgaggttaaggttggtcttgctgatgatgctgccgttaacgtagtcaacgagcatctgctgcaccggagtgctgcggtagatgtagagcttgcgcccatccgcgacggcgggctcaactcgcacggtcgaggagttttcgtcctcggacagtacctccacggtgtgggaggtccggtcggtaagcagctgcgtttcctcgtccagaatgccgctcatcgcgtacacgtgggacgggtcgatgtagccgcccgtgaagctgatttgccagtcagtagtgacgccgttagcgtcaaatacgtccgtcgcgtagcgcagctggggatcgggaactgccatgctgcctcctgtgtttgtcgtatgtgtaccaaaagtcgggccgtccttggcccgccagccttattcctccatctgcgccgccgcgcccttcagtagcgggatcacgtacggcaggcgaccgcccggcagcacgtccgcaaggttctcgggacgcccgctcacgccctgcgcgaagtcgttgatgacccccagcgcaggggcgaagctgccgcccacgatttccttccggttgccgagctggccgcccgcgagctgccgcacccagtccggggagccggtgtcggttgcgtgctcataccagccacccgccacacccgtccccacttccagcacgtcgccgaggaaggccgtcgcgctgatgtagttcatggtgctacggcccatcgccagaggcgacagggcatcctcgatggcctgatcgcgctgctcctccggcaggagggcggcacgcgaggcgacacgcagggcttgcagcggagcgaccacagccatcgccgaagcgatgatgcctgccgtaccccatgcaccgtacaggcccacgtagcgacccagctgcttctgctgtgcgaccagcgagaacgtgcggtgctggaacagcatcttcagccaaccgttgtgcgcccacttgccggtctcaccgatgaaggtgtcctgcaagatttggttagtaccacggtcgatggtgttgtagaacgcgagccacgcctgacggtcgtgcaggttctccagaccacgcgggtccacagcctccagcttaccgtccgcgccccagcgcaccacctgatcctgcgtctgccgcagccgagcaagcagcgtgtcgtcgaggcccatgtccttcagggcagtatcggcagacttaccgtcccgcaggaacttcacacccttggcgatcagcacttccgcgaagccacgctgctgcacagccagtaccgcgcgctgccccgagaggatgcggttggcgttggcagtgcgctggaccagagcagtcaggaagcctgcgcgctcggagccgtacagcgaagcctgcgtgtccatcgagttgaacatgtgcaggtcgtaacccgcgaggccgaagccgcgcccactgatgaactcgaagcccccgaggatgctgttatccgggtcttcgccgcgcagaatcttgccaatctctgcacgcatgcggggagcaatgcggatggcttccgccacaccagcagcacccacagccgggaggccgttggaatactccgccgcttggtttatgcccgcgccgcccagctgtattgccgaggtcagcagtcgcgcattcgccagaacagtcgggtcacccgtgccgattacacgaccagtgaactcggacatcacctgatcgaacgcacgcagctccacgtcgttggcacccgtagcctgcatggccttgcgcaggacagacacacctgcgtcgcccatgatgccgtgcttcgccagagcgatgtcaccagccacacggcccgcgtacttgcggtagttgtccatcacgcggttgtccaagtagtccatcaggcggaactcgccctcggcatccttgtacttgcgcgtcacgtccaagtcgatacggctcttggtgtgtttcgcaccaccacgcgagtaccggcccatcaccttctggatttcctcctcgttgagcgacagcgcgcgcagagtatcacgcagcgtgtcggactggttgtcggagaacaggttgtccggcgcgcggttcatgcccgcagcccgctcctcgatccgctccagatacttgatgctcaggtcgtcgaggaacttgtccccgtacatttcacccatcacgtcgaactgatccctcagtgcctgccggataccttcacgacgcacgcgcccagccgcagcgatcttaccgcccagccaagtgcgggactcgtaaccggccacgtcaccatcgggcaggcgggcagaacccaccgtgccgacagcacgctgctcggcagccatacggttgtagccctcgtccagcgccttcgccatctgcttgatggactcgtgggcgtcggcaatatcgcggcccatatacatggtctcgcggtacagcttcacctcgtactcgaactcgttgcgcatcttccagccggttgcgaagtccttaatcgcaccagccttccgcacgtccgcacgccacaggcgataggccgcttcccactgtctcgggcgcgcacccatgaacgactcgaagcgaccacggcgatccatcgctgctgtgctgtgacgaccagccgcgccttccgggttctccagcagggtgacggcgatcatgcgagcgaccggggactgcgacgacatgagcgtggtgctcgttgcctccagcccgaacttctgcatgatggtggacagcttatccgcgtcgatggcgtacttgccactgaagcgttctgcacggccgattacctcggcaacttggatgcgagttgcattgtcgctgatctgcttgtccagcccggtgcgctgcatgaaagccttgcgctcgcggttgctcttgaagatcgagttgaccagcatgccacgggtctgctgcgatgcagcctgcggagagcgaatctcctgacccaagttctcgccgaccacattcatcaggcgctccaacgcggactccttcccggtcaggcccagcacgcgggcgatcttgtccttcagccattcccacgcggtctgctgcgtcgcacccggaggggcgctgatgttgcgcagcactgcctgcacgtcgcggttggtcagaccgtacgacaccagctcgtcgctgttggcgaggaagcccatgctctgctgatccacacgtccctgcatcgcctgagtcatcaggttgcggtccgcctcggacaggttcgcattgacgtgcgtcagcagctcgtccatctgcgccttgaagttcgcatcctgccgcagcgagcggaaggtagcggcgtgcagcatttcgtgcagcaccacctcggcattgtgtgcggagctgcgcatcgccatcgcgttgagcgacgggttgtacccaccggccacgttcggctggttcgggaaccactgggccagctctgcatcgggagcgatgcggacaccgttcaaccggccgctacgcttcagcgtgttggcgattgcacggaagtcttccggcacgttattcgaggattcgaggtagcgcaggatgtcgtccggcgtgcccttgataccgctcgccttccacgcacgagtcagcagcgggtcagccggagcgttccactccacgctcccgcccacgttgtcggcgtagttgccagtgctcgggtccacgttctccacgtcacgggccagagagccggtggcgttcgaggtggtcggggcttcctgcgccacgtccggacgagcgaacaggcggaagtcatccggcacgtcagccatgcccgcacgaatccagtccattacctcagcgcgcgcgagggagtgaaccttcgcattgagcgccaccgggttgccatcgcccacttcggccacggcgcgggcgcggaggtccgcgttccacgcctcgccgtacatggcggcgttaccggaggccaagtcgatggttgccttgtcacgcaaggccgccgcgctgcggatgcctcgtaggttcatcgccgtgccgataccagctgagaaggcggcgtcggtcataaagtcggcgacggtgcggttctcgcccatgcccaccagtgctgcgtccgtgatgacggaagcagcggcgttctcggcaacgctcgaagcgatgcccgcagccacgcggccctcagcgaacagcgccgccgagccaacgccaagcgcgcgcgcgccaccggaggccaagccacccgttgcccagttgccaggatcggtcaggcccgccacgaggtcatatccaaagctgccccatccggactggttctccttgatccgcatgctgtggcggcgcgtgtcgatgcgatccgacacgtacgacagctcatccggggagtacgctgcatcgcgtatgtcttccagctcatcggctgtgtagtacggcttctcccactgcttcgggtcgtacgtccaaccctccggggtcagctcccgatcacgggtgatctggttggacagcgccgcgccaatgccactatcgaacgacgcgccccacttgtcgaggaacgtgagcgaatcgcggaaggccacctcgtcccggtcggcctgcgtagctgcgatggcagcgcgggtgttgcgctcgttgctctgcgtgtcgatggcagagacttcctgccgcacccaccatgggaccacctcgtcactaccgcgaacggcctgcgcagcagccacgccctgctcggcggtgccaccttccacgacgttctgacccatagccagctcgcccagcccttcgcgcaccttgccgatgtactccttcgtagctctggcaagaccgccacccgcgccttcgatagcatctccccgccatgctgcggggatgcttgccccactccacgtctccgtggtcatgttgcctgcaccggcccaagcggcactgatgctgccctggccgtccgcaccatgcgaagccacagcgggagccgtatcactacccagcactgccggcgcgtatgccgcattttctttaccccaccctcgacggtttggtccgccttggtagatacgcaaagcggtggagatgtcccccttagccatctgcatgttctcgcgcatgatgtgcgcgtacatttcaaggttgtcttggaagttccgtacgtcatacttcttaccagtgcgagcctcgatggtggcctgtgtcggaggcatgacttggaagtcaccttgtgctcccttcttagagcggataaccccatccggatcacgctttgcagtaccactaccggattctacgcgccactgtccacgcacaaccgactccggcactcccgcgtaagcggcagccgcagcgatctgctggtcttgggtcagccccgaaagatcgagtgccattgtctagttctccttagagttttggttggatggaaatgctctgttggatgctaccgtccggcatgcggacgtagccttgcggcaccgggaactcggtgcgggttgctgccttgcggcgcttctcgtactcggccttgatgtctgcgccggtgacggccacgaccttccagccgcgctcgccaacggtgttgacgtacagcaccggctcgccgctctcgctgtcacgcatacggaacacgtcagccttcaggctcttgctcggctccacgttgttggcgcggagggtggcgtcgatggctgcctcgatagcaggcccggtctccttggtgtccaggaagcccagccatgcaccgacgctgcctatgacgtgcccttcgtcgtcacgcccgttctcccagtaatacttgcccgcatcctcgccgccgtacttcagcttggcaaggttgagcgcagcagtgataccttcggaggacgtgtcgagcagcccgccagtttcgcccacggcacgcacgattgcacgtgcagctgcggctcggccggagtctcccagcttgttgccgaagtatccgaagtaggccgggttcgccttctgcaagacgctcgccactcgggactgcaacgcctcggactccttgcgactgttcgcactgaactcggtcgggtcggcggtggtgatttcaccacgcgcaacctcgtaggccagctcgaagttcacgccggattcctccagcgcttgcagcttgttgaacatcgtgttcacgccatcgccgaagtacagggctgctgtggtagcaccggacagcttgccctcgacggggttgccgttgatgtcgatacgcttggcagtcgtgttcttcagcatgcgccactggttgtagaggtcgcgcgctgcgtcgttcggctgctcacgcaggactgcgcgggccgtagtctggtactggtcggccacgcccttcagcacagcaccgcgcccagtgttggcgttccacaccagctgcgacatcgccacttcggggttcttctgcaaggtctggttgaagccctgcaccacgtttgcctccagcagctccttgtccacgcctgggacgttgatcgtctgagcgtaggtgccatgacgccacgagtcgatagcagcacggatgtcctcctgctgcgcagccagctttgcctgctcggtctgcgccaccttggcagccgccgcacgctcacgcatcaccgcttcctgcgcgcggatgtgcgcgcctgcggactgagccatcatgctcatgcgctgggtgccggagtacagcggatcgtcgctgccggtcgcagccgcgtagcccatgttgagctggtcgatctgcgcctcggtcggcttcgcaccgatgccctcggcagcgtacagcgacacgagcgccatctgctccgtagcctgcgggttactgtccagccactcggacttgtactgcgcctgcttctgcttgacgtacgcctgcaactgcaaggcatcgtccgggtccagcgccgacagcacaccacgctggttgaggaacttcagcgtgtagaactctccacggtcagcagcgccacgcacgaacgcggtcatcgccgccttgtagctatcgtccgtctggtaggcggaaggagacagcccatccagcatgctgatctgtgattgcaccagcttctcggcctcggcttcgtcgccgggtgccttgttgcccagcagcgccacccgcttcgccatttcgttgtagctggtggagttgctactgttgctagcatactgcgccttgaccagctcgctctgctgccacgccacacgctccttggtgtgcaggtccatcagcggaccagcacggtccatgaaggtcttctgcaacacggcatccgcataaccgttgccggtcatctgcgactgtgcgagcttgttgaactcctgcgccattgcttccggcggcagcttgcgcagctccggcatgcggtggatcaggtcttgctccatgtctgagaccgaacgcagcacgttgtagttctgcgcgccaatctcatagttcgtagggccgaacagcttgctgtaccacggctgctcggcagagatttcgtccatcgtctgcccgctgcgcgctgcaacgaagccatcccacatctgctgctgttccagcgccttacggttcggggcagtaatctcctccaagaactctgggagattgctgtctggcatagtcatgccgccagtatcggcgaaccaatcatttccgctgcgtaccgcctgaagcggggccacgccactaccttgcacaccggtctgtggaacggcagcggtcgcaccaagcgaaccgccaccgaccgtttcggtgctgaaggtgatcgtacccggatcaccgatagccatgtttcctccttagaaccacccaagcccagaagtgctggtggcgaagttgtcgtagttgttaccaaactgtgtggtgattttagcaggtgcctgccgcccagtaccgtcgttgtagttaaaggtgctggacgcccacgacttgccacctcgtttggacataccctgccacgccccgataccaccttggattgcggagtccatgctcttggacatgccttggaagtccccgttgcttgcctgccactggctgacagcaaggtctgccaccgcctcaccagccataggcccaccgaagtagcttgcgagagcaatacccacaccccacgcgaaccgatttttcatagccttcggctcgatgtgctgctggtaatcgaactgaccgaacgtccggctgatgtccattcccttgtaggcgttggacatgatctgtgccgtctgcgaagctccgcgacttgccatgaggcttatcgcgttctgctgcgtttccaaatccatttcggattgcaggcgcaccatagtatccattaggtcggaggacgagccaccgacaccaacgaagccagattgcgcagccagggcaccgcgcgcggctgcgagttgcacctgtgtattgaggcttgctccttgctttgcacgcagctcctcagacagctgctccatctggaagttgtactcctttgaggccgcgttcaccttcacttggttgttgagcgtgcgcatgtactccgagaagtttcccttcgccacttctagggcgttggtgttcttcgtcttcgcctcagcggcgcgccagttcgctcgtgcaacccgcgtggtgttgttggcctgaaggatagtgtttacgctacccattagctaactctcctgacgttgttaaaggtctgtccaacccacgacaggcccgtcactcggagcgggagccagtccttggagctgatcgtgtaactgcactcgcggacctcgcggcccacggggatcgacagctgcccggaatacaccggctgctgcccgaccaagttgtcgctgtcgccgaggattcggccctcgaagtcgatgctgctctgcactcggttgcgcgtggcgaccacggccaccatacctgcggtgttctgcacgtcggcggtgactcggttgagggccattcgcccgtccagcacagcctgaccgttctggtcacgcgggaacggattggttggcgtcaccgatgcgggactcaccacgccgaactccagcgatgcagggtcgaggtcgtcgaactgggataagaactccgcgatgcgtgccagtggcgtgcccagcaggaagtagtcgctggttgcgttcaccaccaccgagccatccgccacaccattctctgcgcggttcgcgtacgcgatgcgggagtcgatgtacccgtgctcgtccagctcgcccttgaagtccagcacgtccgccaccacaccactcgcgcgtccggtgaacacgatgcccgacttcttgtgggagctgattccgaggatgttgccaagcgtcggtgcgtaggcgaacttgctccacgcctccagctgccgctgcccgttgttcttgttgtcctcgtagcggtacaggtagaacgtgctgggctggttcctcgtgcggaacatcaccacgttcggcgcagtcaccgtggcaatctgcaacggctcacccttcagccagttgtcctgctcctcgctcagctcgtcggtcacggtctgctgcccgttgagggcacccacgcgcatctggtgcaggctcacgccctcgctaccgtactgcgagtagaagatgaagttgccggaggtctgagccttcgcgtcggtgctgtccttgttggcgctcaccgcccggatcaacggagacttcggagtcagcagcgcatcgccgctcacgccgtactgctgccgctcaccgaagatgatgaggttgccgttgtagagcaccgcatgccgcagtacgtcaccctcggaaccgaacgcgaacatttccactgggtcgtcgtcggcgatggtcacgacacttccgcgccagaagtcgaggtagtccccgctcatgcttgcattgacgtagttcgcactaccaacgatcagccggtcttggaagactgacagcatcgtgatgggcttgtcgatgaaccacgggatcggggaggttaggccgtcgccgaccttgcgtgcgccgtaagcggggtggtccccactcgctgggaagatgctcgtaatgcccgcgccgttgcgcgcgatgcacgcctgcccgttgtagatgtagagctgcgcgacgaggttgtcgatggtgcaagtaatgcccgcagtctcgaaccagtccaccgagccgaagcctgaggtctcaccgctttccagctccgctcgcaggtagtacgcctcgtccgtgccagcgccgctcgggcgcacacgaatgacctttccgtggaagtggtacttggtggcgtaggttgcatcggtgatttcctgcccagacgcgaagaacgtggttccatctccttcatcgtccacagtgatgtccacgaactggtcatcgtctattaggatggaacccttcaggtaggttgaggccacgccaccatcaactagcaagtccgacagcttctcggcgatgtactcgggcctagtttgctcggcgctggtgacgatccactcgttaactgcggagttgtattcgttaactcggtcgttgacgtgcttctgataagccgggtcaggctccgtgccgccaggtaggtagaatgggatgtcactggtatccagcgtgccggggtaggcagccgtcaccgtcttgtacgtcacctgcaacgtggtaccgtctgctcggtgcatggtcacggtgtaggtggtgttgaacttgccggtgcgaatccacgcagcaagtcggcgcaggttggtctcctcctgccagaggttggtgctggtcgcgctcgggaggttgtcgttgccagcgatgtagacgtagctgccgatggccgcgagtgacgatgcgccgcctgccaccagcgtgttgacccacgcgctgttctcgtacgtgatcgggatgaactgctcgcccgtcttgtcgtacaggaacgcgaagctcgcggagccgagcgccgaagcctttcggcgatacagcagcgcgtactcgcggccctcctgcgtgaagtcaaatacgtccatgtcttgcagctcgacgcgcgctgcctcgctaagggctagaggcagccgggcagcgaagcgcgtaccgcggcgacgcacaagcccttcgacgggatcggacagaatgttgatctgctcggtcgtctgtcccggtcgccgacgatgcggcggcttgccgctcacgccttgtacaatgtccgggtaggttccgcctgcctttgccatgatgcctccttagccggggaatgtggtgtggctgtgccacgggtgcccgctgtagttgaacacgcgctgacgaagaacgtccacgcttgcccgcgcatacaggggattcgccttgatctgacggatgtgctccgaccgcaggttgatccatgagtcgttgcgctgttgcataatcttctggtacttggtgttgtcgccgtcgaagtccgactggaaacgcagcacgctgtcgtcgcgcacgaacatctgcacctcgtaagggcagtcctcgaagtccagcagcctggccaccttgacggtgacggggccatcgaactcgtacttgttgcgtgcgacatcgtacaggcgtcggccgcgctgggctactcgccgcgcgccgcactgcggcaccgggtccaccttcagcacgtcggtcggaaccatgatgtacttgctggtggcctgcggctggagcttcaaccactccacgttgaaccacagcgcgagcgacgaggtgtcgcgcagcacacggtccacgaggtcgagggcatcatccttgtacgggtgatcttcctccagagtgttgagcttcgtttcgcccatcgtcttcaggcaggcgttcactacgtccaactttgtgatgaacatgatgcctcctagggaacaaggcagagagagcgctgtgctctccctgccggtggatcagtcggccgcgagggtcacggcggacggtgccagctcgaagtcctgcgagccgttctcgtcatcctccacgcgcacgacgatacgccacgcattgtcgcggccgaagacggcgacgacggtgcccagcgtaccggcctcgatgcccagcggcgcgatggcggcggtgatagaaacgcggttggaaatctcgaaggggcggtcatagaccattgtgtcttactccttggtagagggcgcagtttgagttacccgaaggattcagggactgcgcccggacggattagggagccgcgtcgatgcgaccggccagttcgacgcggttgaagccgacggcgaacgacatccagctgtctacgaagaagcacttcgaggcgtcggaccaccacacgctcgactggagcggcagcgcctcggcgatcagcagggcgcgaggcgagaccgccacggccacgaggccggtgaagtcgccgtcgtagaagttgtcgttgtcctcgttcgacagcaggtggccttcgaccacgccgttcggcaggttctcgctcgacaggaccgggacgccccacgccttgaagaccgggatgccggtcagcttgttgccgtcgctggtcaggtactcgccgttgacgatctgctcggcctgctggagggtgtagaacacggtcgggcggacgatcaggacgatgccgtcgcgctgcggcttgaccttcttggtctcctccatttcggagaacagcttgccgatggcagcgtacagcttggccggatcgttctcgtcaccggcagcggcgagcacgacctgcgtggcaccgaagtggccctcgggcgcgcggccgttcttggtgaaggccgaggtggtcatggcggcagccttggcagcagcgatgctgatggtggcgtccacgaactcggcaatctcctgaccctgctcgacagcgatttccttgcgggtgtcgatgtcggtgaagatgtcgtccagctgccagatggagtggcgcgacagcagcatggtgtccacggtcacggacgccttgctgaagtccacctgcgtgccgtccggcgcgtcgccgcgcttcagcttctggagcttggtgcggccgatggccttcttggtcagtgtgttggtgcccttgaccggctttcgcgggaagaacttctccagcacggagctggaaacgaaggtgtgctccacgtcgccggtgaactgctccagaatcagggcgttctcgttgccctgctggttgatctggttcgggaggaccggaacggtcgggaagatggtgctcatgttgtagtgatgctccttggttgttagtggatgacgcgagcgttcagagccttcagctcatcggacttcgctgcaccgctgattcccagcttgtccaccagcttacggtactctgcacggtactgttcgcgggtgagcggggcgacgccctgcaacgactcggacacggcagccggattggtagcgggctgtccctgcacggagacgttcgggttcgaggacgcgaggccgagcaaatgccgggccatcgcaacggcagccaagccgcccgaggacagagcctcactggcctgcttcagctgatcggcgggcaggttggtgcgtgcgtactgctgcacggccttccagttcgcctcaccacccacggcctcgtggaccttggtggcggtttccttgtgcttcgcgtcggcggcggcagtgatgcgcgacaccgagtccttcgccagagcgaggatcgggcctgcgcccttcgccttgtcgcccagcacttcgatcttggcttccagcaggtggaagttgcccttcgccgcttcggtcagctcacggctgttgatgtcgagacccagcgtgttgacgaagtagtcggccgcgatgttcaggccgttgtcgccgtagtccggcagctcggcagcagctggagcctgcggcgcattcggtgccggggcttgcggggcgggttcgaggttcagcgcgttcgggtcggtcacgaccggggctgcgggagcctgcggctgtgccggtgcgaccggctggttcggctggaccttggtctggtcgtcggcgggctgcgtgttgccgttgggctgcgcggtcgagacgatcacgtttgcgttggggccaccgcccggaggtgcgttctgactcattgggtctccatattgttctggttgtcgatctgctgcgaggcgttctgcatggcgagctgctgctgctgtcgcatctgcatcatctgactgtactcctcctcgctcagaacgtaggttgcgggatcaagtccgcgcgctgcggcgaggtcggcgatccacgcggacagcttcaggcggtcgagaatctgcggaggcagactcagcacgccgctgatgtcctgaccgaagcccagcagacggtcacggtccccggtgcgcgagagcgcggcgaggccagtgatgatgacgggttcgatgtcagaaccggcgatgctcttgtcgataagctccatgacccagtaggccacgggaacctgcacgtccacggcaatgcggctgtaaccgccgcccagtccaccttccagctcctcggccaccatgcggatttcttccgccgtcacgcgctcggcttgacgagtcaccgccgtctggagcaggaagcctgcgccgatgcggttgatgtagagctgctggatgttgagattggtctgtagcgtgccttcgacgccggagctaatcagctcgatgtcgcccttctgtccggggattgccgcgccgttgggcgaggccacgaagtcttctactgaagtctgaccagcagggttcaccaaccaccggaactcggaggcaaggatcgctgcttggatggtcgcttcgctcaggagggacagcgcttggaagtcgccctcgtagtcttccacgaggccggtgccgtagtcgtcgcctgccgccaagtcccacgtcacagcgcggtagggcagcttctccaaagtatagttcgacgagaagttggcgggtagctgtacgttgtccagccacacggtctcctcaaacttcgtcccgttgaacttaacccacttgtactcccagcagttaccatcgtcgtccggcttgaactccgggttgccgatgactgcggcgagtgctgcgggcttgatcgcggacttgtgaatcttttcgcggatgatgagttcgcacaccgaaccttggcggtcgcgcttgacgacgtaattgcggaggttcagcacgcgcaccgtgtccttgtcgaacaccatgagtgcattgccaagcactatcagcatcttcagcaggtcgtacagccgggcgcgaatggagcgcttgtctagctccagagaggcttcctgctccagcttcgcaagctgggtctggattgccttcgggtctacacctgactcgctcatcgaggctctggccttgcggttcgcttccagccggaagaacgggcgggacggtgcgaacagggacatcatcagcttgttggcgaggtggttcaccgcctgcgctcccagcgactggaagccgtgggtcagcggctcggtgtcctgatcgcggttcttcttggggaacagcttcgggatggtccacgaagcgtagcgctctagccggttaaggatgccgttacgcttcccgtccagcttctcgaagcgctgttccgcagtggtcgggcacattggattgtccatgctcacctcacaataggtcggtgccggacgtaccggtcagccgtgattgtgctgtggggatgatgcgctggtactgctgccgggtggtacgtcggcggccgatcaggtcatcggtcttcaggtcgaggtcggaggtgccaagggtaacatccaccgtttcgatgggagcactcagcaacttctcggcatactcgctcgcagcctgttgggcggcagcggtagccatctgatcggccatcgcctgaatctggtaattggtctgttgggtctgaaggttggtctgacggtcgatggcagccgcttgcttcagggctgccttcttcgccgagccacctccgacgagggaacccataggctatctccttcgtttggtgagttgcggcgaaccatcctccagctcgaagccgaagcgttggtacagccgagtgattgcccgagatgatcgagctagtgctccgcctgtgactatggcatcgcaatcgttggtctcggctagatgctccagtgtggctactactgcccggaaggaactgcctttaccgatccgtagtaccaagtcctcagacaggactaacctgttcttagagtaccaaggtttaactacagagaataccagtaggtagctttcgtctatcactactgcatctaccatattctgtactaccatttccacagtgtattgtggatcgtcacagaggtagcttaccgaggagctactatgctcactctcactcggggctaaagacagatacagggcagcgtctagcgccaccctgatctgctctctatcacccgtcgttggtgttcggattgctggactcaacggtgaatccctcctgcaagatgcggagaactcgtgccattccgagctgcacacctgcctctaatggcgtggtgttggaattgacggagaggacggaacccgcctgtcgctgcacggcagccagttgcttcgggtccagtcggtagatgatcttggtttcggacatgaggtctcctctgtcgtatgtgtaccaaaagggtttgatgcctgcccacgaagggcgaggcacctttgtcgtatgtgtaccgaaactccatcagctgaagaagtacggagaatcaatgacttgcgagaggtcgaggtcgcccatcggcggcggctcgggcaggaaaccataggccgccctgaactcctccagcacgtcgtgcctggagtacatgtccacgaagacctcccggatgatttcgtacaggcgggccgtgtcggcggcgtgggtgccatagtcgtcgtggatcatggcgaaggcgttgatgccatcggccttggcccggttgaccaccagcgtcaggtggctggcgtcgaggctgtggacgaagttgggggcgatgccgttgcggtgccgggacttcttcacctcgtctgtgcttcggcgcacagagagcttggtgttgccgcacagcttggtgttgatccggtgctcctcagtctcccagtacacctgcgtcaccgggaagccggacggcgtgatccacttgatgcggtcgtagccctcgcgcaggatcgccgtggatgccttctggagccacgccattgcatcggctgccgccactaccgtgtcagcgatggcgacgccgaggcgcttgctcaggaagcgtgcggccctgtcgtagagcttcttgtccagctcagggaacttgtcagccttcaggtagtcgctcacgatgaagtccgcccagctcgattgccgagagccgtatggcagggtcatcaccgagcgcttaaccagcgagcgggtcaggccgtggtccagccacagcctacggaacccttcctcgtcgtccccctcggcttcgaggagcttggtcacgaggtccgccaccatctggtagatgtcattcggcagcggtgccgggatcaggttggtagccttcccgcctgcactgtcgcgcagcattgcggagaagttctgaagcccattgcaggaaccatccatgccgactgcgatgcggctctggaagcgatccccgaacacttgccactgctcgtactccaagcaccaagcgaggaattgcagcggcttgtctgcggtcttccactcgtcgttgttcaccgggtccgcagcaaacgccagaatctggtcgtgatgctcggccacccacttcacacgatccggcagagacgccttgtcgtatccccaccggtttgctcctgtgatgcagaaccagtccttagctgacttggtgagcaagggcttaccctcgccgaactccagcagtgccttctgcaagtccgaaccctgcggagatacgccggtggtctggacatacttgcggccacggaagtccacgaagtaaacgaagtagattgcttggtagtctacgaacttgcgcgccactcgcatggcgttgtagaaccgattgctcttgctgttgcgcagtcgctcgtcggtgtgccagtcggccacctcacgcttccacttcttgaactcgcgctgctgggattcggacatgtcctccttggtcattcctttcgccaaccactccggcttgcgtggcttcggcagctcggcctgcgaaatgatttcctccatgtcgtggacctgtgccactgcggacacagcctccagcatgcgtcggttgattctccactttacctgctgcaacgcattgaccgcagccatttcgttacgcagctcggcggagcggtagtcgtcgcgggtctgagcgtaggtcttcaccatccacgggtgcagcctgcgcatttcgttggtgtggaatccgccgttgtccacgtcggtccagtccttcggtggctcgacgcacggcaggaagtacggggtgctctcgatgacgaactcgctgatctggtggatcagcttgcgcacgtcctcggtaagctcgacgtgcaggttggtcttcgtcctgcgacgtccaccagccacgatggtctcgttcaccacaccggcattcaccatgcccatctgcgcaagctggtcaacgaggtagccaccgacctgatcgcgctgcgcctgcccccactcgtggaactcgacgccgttcttcctgccctgcatcttcatcactgtcatgcggtgcgtctcgttgacgctcagcttacggtccatgtcgttcatcaggtggtagaacagcgtcggctccgcgtctgcgaactgggtcagcaggtactcgtggtacacattggtgccaacctgcttcaccacctcacgaccggcagccttatccttcttgccctgctcggcgatgcaagctgccaagcaaccacggacggccacgaaggcgatagcctcgtaccattcggtggcttgttcttcggcagtgatggcctgcccacgcttgtcctttcgctccgggtcgtacttcgcccgcagaagtggcacatgggcctgcgctctcccgatgcgcggcttgtcgatgtcagcccggattcgctccgcaagcggaagcacgaaccggcgatacaccgcctgagcgtacgggttgttcggcgcaccgccgttctcctcgttgcgctcaatggccttacgcatgcgctcttggccgaaagcgtaggtctccagttcgagttccgcttgtgtgagcatgctacctccgttacctgattgtaaagtccatcacctgtccgccaccgccttgtcgtggcggattcccttgtatcgcggctcgcgcagcaggccgtacttgctgtaggacatggcctcgatctccacgatgtccccgatgcagggcagctggtccgcgctgtgcggcacgccgctgccgacctcctgctccttgccttcgccgaggtccacgaccaccgtccacacgtcgcgcccggtcttctcgccggtgctaatgttgacgtgcatcactcgcaggtccagagtcagggtcggcttgatcttgatgacctcgcccttcgtgcccttgtcgcccttcgtccacgtgccgctcggcttgcgcaggatcaggccatcgtacgggccgctctcgcacaacaggcgggcggcttccatcggcgacagctcctgatccacgaggaagccctgcgactccgcgaggaagaacggagccttgcactcctcgatcttgctcagggtcggcggcagtcggcccacgcggtcaaggtaggtcagcgggctgaatccctgctcccactccccgatgctcacgaagtcgaacaccacgaagaacggttcggtgtactgcgtgccgtccttcttgcggaacatcccgctcacggtcggctggtcgatggtcgggtgccagtattcgccaaggtacacgccgatgggagcgaacggcgcagcggccaacgcttccttgatgtggttcgcggacatcacctcctcgccagtgcggctgaagatcgtgatgtgctcgacggagttggcagcctttaccaccacgcagttgcagccgtcgtacttgggctgcgcgaggtactcggttcgcagcatgtcgtcgctggggcgctgacgcttctgcaccttgtccagctcgacggccttgtgtacgatgtagggcttactcatcggccttggcctccttggtcgggaggttgtttcggacggtcagcccgccgacgttcgatgcgattcggccagacatgaagtctgtgacgatctggccgatccacagcttgcgcggcaccatgccgttgcggtagccttcccacgcatcggcgatgcgagcgtacaactcggctttgccttcgtcgttcagaccggggaacgcagtgttgaccgcatcctgcaacgcttcatcatgatcgccattgccccaagcaacggcaccctcgtaggactggatcagacgctgggtgttggacttgtagttcattcggtctccttcgacgcggtggaagtgttggttgctcgtggcgctcgcggcgctccttcttcttcgagcttcagctgtagcagtgcagcagcacgccacagcacgccttcgtagtcgccctcctgcaagtgtcgcaggatgcaatcttcgtgatcgccactcttgtcacgactccattgcaatggcataccggggttgtgcttctggttactcttgtacgcatgatgcgccagagcattcatggctgctgggaagtacccgaacaacaccgagtacaccggatactccttacgttcctcgctaccgtttggcagattgcttgggaagcgtgccccgtcgttgagcttgtgggtgcgctcgtcctcattacggtagttcagctcgggcagtacaacctcacgccgtgctgtggtaacacctcccacacctataaggcgtgcgagtaactctggctttacgaggctcgtagcgagtgggcggtcatccgttttaatccgcacccacttatcgtcgatcccaaccaccaccccggatttaccgacgaggttgttggctgatccggtgtagcgaacgcggtctctgatgcggacatctgtaagtctcatgttacctccttatgctggaacggtgatgtggcgacgctgctcgatgttggtcgtcagcttgcggccacggctgtgcccaccgcactgtgtgcattgcagcagcaggtaggtgccgacctgagtgcgggccggtgccttctgcgggatcatttcgttgtgcccgcacttgttgcagcggtgctcgctgccgtcggccttgtagtacaccgcgatgttcgggtgcctgctgtaccagccacgcagcttgcggtactcggccttcatggacttcacgtcgatgatgttgtactcctcgcactcgtcccatgcgccgggcaagccctgcatgcacgccacccacaggtcgaagccggggaagttcgcatggtcgtacttgcgcagctcgggaacgatgactccggtggtgtactccagcttctgcgaggtgaacgcgaactcgtcgcggttcagcagcatcgggtcgatcacgctgaccggggagagcggagggaagccgaggatggcaaggcgagccttcaccttgcgcaggtcgaacttcttgccgttgcgagcaagaacgaagtccgccgcgttgagcagggcgtggagaaccttggcctgcttgcggtcgttgaacacgtccttctcgcggcgctggtccacgtagatcgtggcctcgtcgttgtccagccactccgcagcgaacgacatgagagaccagtcgcgcttgatctgcttcgggctgaagttgttgttgaacatctgccatccccaaaactcgatggggaaggtctcgatgtcgaggcacaggatcttcggcccgtgcttcggggcgtgcttcaggaatgtggtgaggttcacgggttctccttcttcattgctcgggccttacgcgctttcgcattgcgagcggtgcgcttctcgtcctcggtcttgtgggtgggatgcagatagcccgtgatgttggtcatgtgctttcgcaggtaattcgcaagtcccccgcagaaggcgaggatgtcccgcactccataacgtgggccattgttctcgaccttgcccagcagcgagttgcacccacgatggagtacgccccgcactgcgccagtgcggtgatcgtgatccagcaccgggtcgagcggtgccttcagtccgagctgcccgccgcacaatgcgcagcggttgctctgctctgctgcgagtttaacccgcaccagcttcacctgtgttgctgtcagacgcttcatcgtttcagttcctccagcgctgcgcgcttatcgttgacatcctcggcgaggtcgtagaacgcctgcttcagcttgtcgccgaacacgtccagctgtagaacgtccagcagatttgcgtcgcgatccgtacgcatccacagcagcaccgcctgctcggcgaagtaccgctgccatccttcgcccttcacctcggcgtacttaccgtacaccaggggcgcggcttcggcgttgctcttggttccgaacagtagctcctccgccgtcaccttgcctaccttcggcaagccggggatgaagtccgccgtatctcccatgagcatctgcatccagaaccacttgtgcccatactgcaagccgtctgcgcccacgaggtcgtaggtgccgagcggaacgtccacgatgtggtagtcctcccacgtgatgtgggtgccgcagaacatacgcatgtccttgtcggcggtgtggatcacgtgcagcacgttgccgtgcttggctgctccggtgctaacgaaggccattccatcgtccgcctcgcgggtcgtccagattttcggtgtgaagtgcgggccgtcgtacgtctccatccactcgcggaggaaggcccagttgttcggcttgcgtcctgactggcgctgcccctgatacggctgagtcgtagcagcgaggaacctgtcacccttcgatgacgcgccatgtgtgaggtgcatgactacacgatccgctccgctgatatgcttcagatgcgagacgcgggagagcacgttgcgtcgtgcgtcccccgcagaacagttctcgctaccagcgcagaagtacgcagcgtagtccccgtccacgtgagcgatcacgtttcggttgtgctgtcgtacttccacgatgggcatcggggagcgctccgcagccgcagccatcagagcgctcaggtccatcaggcgacgcccgccatcgggtcgtccatgtcgaatggcggcttgtcgtcctcgtcgccctgcgcgttgtccacgtcaccgaccgcctcgtccagcgcatccacgccttccttggtgacggtgccgccgaccagcttggaggccgcgtagtcgtagcacggcagccccttgaagttcagcgccttggcgatttccagctggatggtgttcttgctgcgcgcctcggcgatgaccttgccggtcttctcgtccttgcgctccgggtactcgccttcgatgtagatgctgtcccacatgtcggcatcggcgaagtcccacacgaatgccttcagctcggtcatggccgcgcccaccgggaacacctgctccagcaggttgccggtcggctctccgtcttccagctcggggacttggatgatcggcttgcggatggattccttgtcgatgttggcgtacgtcttcttcttgccttccgggccgcgctccacgtggaccacgttcagcagcaccggcttgcccagcagctggacgaagtgcttctcgtcggtgcgcaggcgggagaacatcttgaagtacgcggccttctcgttggtagagaggttgaggcgcaggctcaggcggaccggaatcttgacgccaccatccagttccttcggcggatgcttcttgccgatcagctcgaacacgatgatgacttcgttgttggtcttcttcttgccctcgaactcgctctcgtgctggcccacctcgtagtaggcgacgatgcgagcgccggtctgcccggcctcgggcggagtgtagtcgccgccaccggcggacgccacggactggtcctgacccttttcctgcacctgcttcagcagcttgtcgagactcatgcgttggtttctccttattcaaacgacggattgtgattaccgatgaagtccttgcggatttgcatgcggtactcggggaacaagacggcgaactctgccggagggttgtgctcctccatcatgttgtcgcccatcttggtttcgcatggcacgccgagaggcagcggccacttgaaccaccactccatgtaaacggaggcttcgagcatgcttgcatgcaggagcgccgccgcttccgtggcgatggatgctgcgctgtccacgtataccgcatcgtggacctgattcaccagcagggcttggccgagccagcgctcgggctgggtgacgtacatgcggtagaaggcccgcagcgagacgtacatgctcgccttggcccactctccgccagtaccctgcaccgggtagttcttgatttccgtgggtgagaacgactgcgccacgccgccacgtgaggcgggtttggttgcgatgaacttgggcgaaggcgactcgctgaaggagtacatcttgccatccggcgtggtgaagtgggagcggcccagctgacaggtcagccccggcacgtccggatgctgcacgaagcggccagtcgtcacacggttggccttgatgacctccaccatgtggtcgatgtactcgcccagctccgggtaacgctcggcctcggcgcgcaccagcttctccacttcctcctcggtcatgcccgtggtcgctgcgatcttcgcaacgcctgcgccgtacgcacgctggaaggagaagaccttcgcgttgccgcgcatcttcttccacttgctgtgctccgggtgcgtctcgtccttcgctgccttcaggatgtaggcgtagtccttgccttcggctgcaccccatgcctgctcggcacgcaggacgtgcatgtccagaccagccttcaagtcttcgatcagctttcggcattgggtgaggatcgcctgcacgtagatttccagcgacgtgaagtccgactggatgatcttgccaccggcgtgtcggctgatgaacgcgcgcttgatctggctgcccttctccttaccggtctcctcgtcgtactcccccttgctcacgttctgcaagttcgggtcgctcgacgacaggcggccggtcacggtgttggtcatgttgagcttgtggtgtatgataccgtctggccccaccagagtgagcatgcccttctgctccccagtcttctcgtccgtcgtgatgaagtatgtggacaagtccttgtggatgtcggcgcgcttggcgagcgccttcaggaacgggatgtcacgagcgcccagctcctcaatcacctcggctgcggtggagtacacgcccttgtcggacttgctctcccatcgctcgctgccttcggtgtaaccggggaacacaaacaccatgtcctcgttgcggaacttgggcttggtcaggtcatcgaccttgaccttcttggtcttgcgctcgcccttgttcttgccaccagcgaacaccaccggctccttgccctccggtactccacccgcatcccaccactcggtcgccgcgcagtggtcccaccactcgcaggccatcgtggtgccgtcttcgaggatgtaatgcagctcatccttctggacgtactgctgcttgccggtctcaggcaccagcaccggcaccttcgccacgtacttcacctcgccgccgaagatcagcgcgctcttgtggaagcggctgttccagttgaaggtcaagccctcgggcagctcggggatgtaggactccagctctgccgttgcgtttgcaagctcctgctccagcttcttcgcatgctccagcgcccacggcttgtccacgaacatgccgttgtactcggcttcgatggtaaagcacagcgcgcccatgttgagcagcgccgagcgcagaccgttgcgtgcccggaaggcatcgagctgaccgaggaacatcttctcggtgttgccgatgtcgcccacgtcgtccgtgtcgttggtgcctacgaggtagtccataagcagggtcttatcgatgtcgcacgtatccacccctgcattccacagggacttcaccgcgtcgtccttcaggttgccgccgtacctcggggccacctcgtccatcgcgcacatgtggaactcctgggtcatgccgtacagcaggtactcggcaagctggcagtcccacaccatgccgccacggtcgatgaactcgatccatgccatgcgattctgcgggccttggcagatggcgtgcaggatgtcgaacttgatgttgaatccgacgaggtactgcgcgccgtagcatagctccttcagccaaccatccggcgcaccgccgacgtagttgttgtcttcgtcgcgcccggtggtgaagtaccgaccgctgttcttggcgtcgcccttgcgcttgtggccgatggcgacgatgcggttgaggttgtagaacgggttcgccttgcgcttcagcgtggcgcggatcgtggtctccaagtcgaaggacacgtagctcatagcggccaccgttgcagagccagatggtacatttcatccgacgcatcgccatccaagtcgagaccatcgcgcacccagcggaacacgatgatgcgatcctgcttgtccttgatgttgcgctgcttgcagatggtggtggcctctaccgcgcgctgataccagccgggatcggcagtcaccatgacgttgaacgcgccgttgcgaagcgcataccacgtgctgctgtagtcctcgtcttcctcgtagtgcccatcggcaccagagcatatggtccacccagccttgaccagctgatctagtgcctctccgaagtcctcgaccagcacgaggaaatcaatgtccgtgtcagtcacgggaggttcgacggtgtagctgctgccggtgcggctggacgcgatgacgcccaacgtgggcggcaggtggacgttctgttcggtactcatacttcctccttgacgaagcggcgggcgtggcaccagactttcttgccgtagtcgtcctccaccatcacgtaagcgggccacgtgaagttctgatcgggatactccggctggtagtcgatgacctcgtacaccttgttggtcgtgaagaagtagcctcgggagcctacgcacctcaccttgtctcccacgctcatttcgatcttcatgcttcctcctcgtagaaccgggcgcggtctgcgtcgaacatcacctcggcgcgaggatcacgcttaccgcctgcgcggtgcagcttgttcttcggagtgccgatgtatcggaagcgatccatcgcaggatcgttgagctttccgcccatgatgatgaagtcgcacgcgccctgctttccagtcttgctgtctttcagtgcggactgcggcgggaactggccgccctcgccctcggcgctgatctgcgaagtcgccacgcccacggcgtcgtacttcacgcaccagttgcgcgcggcttggtacatggcttcgagcatctgatcggtacgctgcccaccgttggtcatgcctccggtgaacgtgatgttgtcgatcatgtcgaagatgatgaagccggggttggtctgcttgatgatggcctcgacctctccggaggtgaagccgtggatgtcgtagaactgcatgcggtggatgtcgccacccatcgcttcctcgatccgctttcggatgctgccgtccttcgcccactccaccatttcggggatcgttgcgttgaggagagactgataccagcgctgcttgatgcgcttgcccggcccctcgttgttcaaccagatgccggtgcgcttctggtccggccacacgtcgtccagctgcggcagccagaatgtggactcgctggtgaggaacgtggtcttgcctgcgtcgggacgcatggcgtagatgccgaagtcgcctccgcgcatcgggcgcaggttgcggctcaggctcggcagtcggaagtggattccgatgtcgccctcgtccattgccatcagttcttccggcgtctcctgcaccagcggcagccgggccttgcggtccatgcgctcggtgatgccttcggccagagctgacagctcatcgcgcagggagaactccgcgccaccattccactgcacgatcttgctgacggcggacgtggcaagctccagctccagcatcttttcgatcatgccctgctccgcctcgggcgggacagcctcgcgcatcgcacgcagctgcaacttcagcagggatttcttgtcgtcggggagttgcttgaacttgaactccatcgcccagccgtcgaacacgtcgtgcggcagagccttggtgtcggggaactccttgtagtacgcgcgcagtgcatccagcatcagcacggtcagctcgtccagcccctcgcgcggagcgttcgggaccagccgctcgaacttacccttgtcgctgcacaatcgcagcagtgtgaggtcaagactcatcgggttcctcctcccattcgtacggtgaactcatgtcagttcctcctgccgtttagcttgttgagttctagcacaaaatccagtgctctccggtctcttcccgagaacacccagctagacacgtgataccagtgttggaaccgggaggaccaccggatgcgttctttcacagcagcttctcctctatgtactcggtcggataatacttcgggtcacggtcgctcgtgatgttccgatagtccaagccgaacgcacgaaggcgcgcggcgatttgtttcgcagcatcctgaccgggattgctcccgttcgatctgcccttgtcgtcgtcgagccacgtcgctacacgttggcctcgctcaatcagctgcatcagcaccttgttgtgcagcttggtgccgagcaacgaccacgcttctgtcaccagtcccaccttgtatgcggagagcgggtcttcgcatagaacgatggtgtctcccttgcccacgccgtagcgtgcgacgagtccgtctttcgggacatcgggagtcagccacttcggttgcctcgtagaggaccgggctgtccagtacacagggcggtcgccttccatgatgggtagtatcacgcgcccgatgtccgggcaccagtacaggccaagttcccctatcatgcgaagcgagaggcccatcttgtagaaccacaccttgtcacgcagcggccactcggttgtttcgtagacacgtggctctggcaactcaacagttgcgcgcactctgcgctcgctggtttgctcggcatgggttcgtactagcttggcttctaagctctcgtgctcacgcttgaatcctgtgccaccacacctgaaacagtatgcggtggacttgtcgtgcgagcgagtgatgagcaacgagtttccctcaccacacgcatggttgatccgagtacgggtgccgaccttcagtcgttccgcatgcggcagccagtcgctgtcaggtagttcgttgctcatcttgtcctcgcttagattgtcggaacctgtccgccgctcggcaggaagtacacgaagaaccagtacaccacgtacaaccagcccagcaggaagtgcaggatggcccacgcgatggacttgctcacggtgtaggacaggaacgcgccgccgaagcagccgatcagtgcgacgagccggttcaccagatggcccacacgctggtcgggcttgcggccacggtggtgccggagtgccgctcgatcaggagcgggttgcccttcttgtccttctggtcggtgacgatgaagacgttatcgccgtcgctcgccgcgtcggagtcctgacccagcagcagggttacgtactggcccggcaccagagcaccgggacgcaggatcgtggctgcggtgtaggaacgggaggtagcaggagcgcactgcgcctgcggctggctcgggccgatcattcggcaccgccttcgctgcccttctcggcggaagccttggccgcgtcgatgtcggcctgcgccttctcgatttcttcggcggtgaacagcagggcggtggcgtcgatcaggtggaactcggcgtcgaagccttcaccgtgctcgaccttcagctgcacgatgcccttgtcgttcttcttggtggccgacacggtgccggacaggacgcgcttgttcatggcgcggccatagacgtaggccacggcgtcgcccgccttcagcgcttcgattgcagcctcgttcgcggcgtcgttctccagcgcagcgatcttctcgtcgatcttgttgaccttttccatcgccttcaggcggtcttcgcgcagctcggccagcttgacttcggtgtgcgagacggactgggtggtggtttcgttcgacatttggtgtatctccttgacgttgtgattgagagtgcctcgtaacgtgaggcagacgactctccgagtaggttagtgcttggtcgggccgaagatcagctcggacgtgtagccgccctgcgcccacgggcggccgtagtgcctgcggcggagtacgcactcctcgcccagctccagcagcgtgtccaccaccttgcgggtggcggccctcacttggttgatgtcctcgcgctggatgttgaagtcccagcgcaccacgatgacgtgctcgtagtctgtgctgccgttgtcgttgcggacgtagaagccccgaccctcggtcagagtggcaccgccgatgatggcgacggtgttgtccagcgcctcgcgcagcccgtcgtcggacatgcgggtgctcgggatggtgacttcgatccagctaccgagaagggcgctcattgcgcacccgccaaggcgttgcggacgctcgggttcagcggcgcaccggcacgcagctcggctgctcggcgcttgatcttggaacgcaggcggcggcgctgcttgttgttcgcacccagagaatcagctgcgcgcttcatctcgttgttgcccacgttacgggtctgcccacggcccgacatgtagtcctgacacatcagcttccgcagcagcgggtcttcgattggaaccagcggcaccgagacgtgcaggtagcgggaggtgtccggcgcaggaggcggcgtgttgtcgtcatcatgctgcggcttgaacgcctgcaccaccttgtccttcacgtacttggccgcgcccttgatcttgtcgaggaagcccatcagcgtttctccttgttgtggaagtagttgaactccagctcgtgccacacgtagtacgtggtgccgagcgggtcggtcatttcctgctcgttgcgcagcgtgcagtagtcgttggcctcgtcgaggttgtcgtaggtgcggacccacagcccatcgggagttgccgggatggtgcggaaccggcacagcctaccgtcatcgtcatggtactggccgatgacgatccacggaccacgcccgacgatccagtagagcaggataagtagacgcagggcgagcttacgcatcggcatataccgcttcgatgtagtagccgtacgggttgcccttgctgcgcttgtcgccgatggtgtccagcacggggcgggcggcggcgcgggtcgggaacagtagattgctctcgtcgttgttctcctcgttgccgtcgatgcggacggtggcaccgtgttcgatgctgttgtaggcgctggtgtagtcgccgtcgtacttcagacgccaacccagcacgggctgcacacggcgcaccttgtcgccgaactcgcccacgccgtaatcgaagtgcggggactcgaatgattccagctcgccgatggcggcacgtgcggcagcgcgcttgtcccacaccaccacggtgttcgggtaggtgccgtcgcgcagcgcatcggcgaggctcggcgtcgcagcgggcttgatggtggacaggatggcctgcacttcctcgggggtgaccgggcgagcgccggtcaggttcgtgttggcgacgacaccgacgatggtgttggtgcccttggcacgggtgatgccgaagtaggtcttgctcatggttgattctcctcgttgacgggtgggatttcgtgctcggtgtgggtcacgatgtagccgtgttcctccatcatgccgcaccaagcatcggacatgcgagggtattccaaggtgctgcccgtcctcgggtcgagcacttcggttacgaacaggagccggacctcacgcataccagcgttccacgctgtgctcgttggtcacgaactctttccactggcgcggcttctcgcacagctgggccggcttgcgctttccactacggatgcgcttgtagattacggggatcatgcgttcacactctctttggtcagttcgtcgatcaggaaggacagcaggcggcggctccggccatactcgctgtcctcgtcgtacatgttgccgttgtacagggcgtactcgtccactgcgtcgaagtaggcggcagcggcggcatcgggatcgtcccagtccactgagtccatatcgttgtcggaacggtactcgtagatcatgtcgtcatcttcgcccgacgccgggaccgggtacgtgctgcacccgctccactccggccactcacgatagagctgcgtgcggaggtccacggcagaacccacatcatccgacgtgaggccgtcgcggtatcgtatgtcccgcatctggtcggcgatcttctcgcacagcgcctcgccgagattgttctcgtcgtcgatgtccgcacgggcggcaatggccgcagcgaggaggagcgcaacaacgcgctccccgtagattcccgtgaggcggctcatgccttcacctcggcgctcttgcgcttggtggcgggcttcggcaccttgtgcgcggcctcgatcacggcgcgctcctcgtcgctcggcgtatagccgccatcgacggccttttccagacggcccagcagcttgtgcaggtcggcggcgaagctgaagtcctcggcgggcttctcggtcttgaagtcatgccacatcttggcggcggcgcgctccagcatggcggccagctcctcgccctccagacgcttgctcttggcgtacttcatcggcatggcggccttggtctccttgtcgtcgtttggagccatcggaccgaactcggacaggtacaggcgcagcgcctcgtgcttcatgccgttgcccacggcaaggcacaggtcggcagcgagcgtcacgtcgccgtggacgtgggcatggttaatgacggcgattgcggtctgctgaatcgtgtccaccagcttggtgcgtgccgtattgatggacttgatgctcttgcggatgttggccgcgttggtctcgatgttcatggtatggtcccttcaggttgggtccgtgccgattgcacgacactaggccctcttgcgaaggcctagtagcttgcattacgggagccggatgctgtatgagcgcccgccgcatggtaggatgctcaggcaggacacagcgccctgcggatgcttcaggatggcccgattgtagctgtcgcgggcagattcaacgtggaagcgagagaatttgagcaggatcacaggaaagccctccggtcagcggcatggttcgcccgattggtcccgctatttcctccagcaacaaacacagatcgcttacctgcggtcccgtgtcgtgcctcatagcgctcagcttggcgcttgcgctcggccatgcgtcggtcctgctcggtggtacgcaggtccataacgcttgcagtccgggtgaactggcaaaagcggcgcttggtgctggttcgttcgagattggcgttaccgtgcatcgtttagtcctccttctggacggaattgatttgaatccaatcgaacccagattcggcgcggcgtttccagaactctttgcgcgcctcggattcggaactagcagaaaccatatcagcgtattcccggccgtgctcgccgatacctgcgaggtagaagaaaccgtacatatttgtgcctccattttggcactgtgagaaagcgaaaacatacagattgaagctcactcaggaaagccgtcgagtcggacgatccctcattctcgattagagccgacaagcaaggtttgcgcagtgcactaccgaatgccgggagtgagattcaatctgtatgccccttcgggctgtcaaccttactccgggcatacagtgccatagtcactatgcgagcggagcgctctgttcacaacccgccagattaccggcaaggtgggcaaggtgtcgcgtctgttagggtgcacattccgtgtgccgaattatggactaatccaacctagacgcggcttgcctcttgtgaccggcttcccgtattccgacgggttacgctgctgggccgactctcacggcagatgcaggtcctaggcgttagtcctaggtaaagcggcactggtgttgctagtccagtggattctatgggccttttatatcccagttcatccggttttccgctagtgctacgtttcagcttggcgatccacccatctaggcttctcgttacaccctacccgttagcggtagtcttatatcccggtccatgatgccggtggtccgcagaccgtgaagccatagtaccctatcctacctcccgtgtcaagccctgtggcttaacccgtagcgtcctgtcgccaccatcctaccatgtaagccggtagtccgcttactgatcgctccgcctttaggcttcctgaccgttactgcatagtagcctactattggcttcctgtcaagctatccgggtgtacgctcatttgcgccttgaccggaagtctcacccatgtacccttagcccattgcaagcggcgccactacggtagacttatcactagactgaccactagcttaccactacgctaactgtctgtcaaccccttggctgtcaatgcttgccgtgtggcttgcatcggcgaccggttcctagcttcacgacgctaggagtggagcgtagggaggatgctaggctatctgtagcttactgtcaagcccctgatacactttccggctaaagaccgatacgataatcgtggcaagccattctgtcgtatgtgtaccaaaaggaaaacgatacagatgccgtcctcccgtccctcactgcgtcccaatcatcgcccggtaggtatgcacctgccatgccatgcgtgcgccgtgtaggcccatcggcggccacgtgccgcgcctccaatgggcgggctgtgcttccaacgtggagccattgaatcacactcccaaccagccgtcaagcaccaatcgcaagagatttattaacgattcagtcagcctcctagtgcagtggtgtactacctggccaacacacctccacgcgagaggagagaggcacccgcgcgcacaacacgcgcccacgcgcacgcacaggcacccacaggcgcacgcgcgcacaggcacgggcacacccacacacccgcgctacgcacgcccgtaggcgcgcataggcgcacgcgcatcacgcgggagggcgcacgggggcgcacacgcgagctttgattggagtggcccccgcgcaattctaaatcaaaatttggtccagctcccgatcagcccgtcttaagtctaacgatgggcgcagcggagtacatgtcgatagcgcacgcggcagccacggccttagccgcagatttgctcacgtggtacgctccacgagcaatacccgcgccgctgccaatgaagatcggagcgtcatccggccaagacttcttaccgctaatgacggtcgcctgtccgtccttgatgataagcacggtggagttgccactgaccagcggctcgatggcttctccgcctttgagggcggctaccacggagcggaggacgtgaatctcaccggctacggcgcagaagaccggaccctccgtggtttggacccggagagccttggtcatcgtgcccttcatgtcgtccgcagtgacttggctgtcggcatacaggtgcttgccgtcccacacgatggtcgtcatgggctacttctccaccttgcagcgccaaccgcaggcttgcttgtagccgtcgtaccacgcacgcagggcgcgcttgtccacgttgcagagcttcacgtcgaactccctgtcaatagcgagcttcgctacgtcagagttggtcggatgctcctcggtgaggtacgttacggcgcaatcttcaaggtactgcgcgggcggcgccggtatcgtgacgcaggaggtcagcgacatcagcaggaacagtcccatcagcccactcaggactgcgagcaatggcttgatcgagcgcgacatgcgcgttctccttctcgattactacggttttcagttccttagccgcagtggtagcggccgaggcgttgcccgacgcctgctggtagtcctcttggacgttggcgcgagagttacggaggtgcagagtgtacgcggacaggaggattacggccagaagcagcagccctccgatcagcagttcgattttacggaagatagacataaggtccgtccttcaggcacatggcctgctcctcgtatcgtctggtcacgagaccgcgcagtaccattttgttggcgtaaatccaccgaggatactggttgcagctcccacggcggtctccggcgttgaccttgcgaagcagggtcgatgcccggagattcgactcacccacgttgaagacgaaggacaccatcgcgtcgtactctccctgcttcagaggcacgcgcacgttgcgctgtacggcccgctcagcgacgcggaggtcttcagcataccactggtcgcactgctcgtgtgtggcccgcatgccaggtcggacgcccttggtgtgccctcggcagatggtccaaggtgcgccgccagtggccgggtccgggtaggccaccagccgatagccttcgttggaagcgatctgctgcgccccgtcgagcgagaggtaggttgccccacctccagccagtgcgagggccagcaacgcggccatgacgcgcttgctgacgttcatcatcagccctccggttccggctcaggatcagtcggcaggatttcgccaccggggccggacgattccgtacgggactgggcagcggtaatggcagcctgcacccgtgccacgtcggcgttgaacagagccgccagctgggccgcagtctgcgggtgcttctcggcgtgctcgaccagagccagcagctcgcggacgagatagttgccacggccgaacaggccggtgtagttggagaaattggacttcagcatgttacctccggtaacggtcaaggatggatgggcggcctgcgcggatcggccctcgccgggtcgctgccttcatgccggttggatcgttgatccagtcttggaactccttctgcgcctgcttctcgatggccttgttctggtccagtgcgagcttgctcacccagtgccgcacgctaccttccagtgcgtcgatgcggtcatcatgcgcaaggctgccgcgttgactggtgatcttggcgatctggtggaacagggaatacaccgagcgcttgccgctgttggcgtgccgctgcgtgtactcgtgatccatttcgaccacgctctccagcaccacgagcgagccacgggcgatcacaggctccaaggtgccgatgatacgggcctccttgttgcctgtcacgaactcctcgaccagcgagccgttccacttctcccgcaggatcggaaggaacaccttggcgaaggcaccgtggcccatgttcttctcgatggagaggacgttgggcttgtatttggcggcgatttccgcgaggtggcgcaggccatccccgtcgtaaccacccggcaccgcgccaactgcgagcacgtacacggtggagttgaggaagccagtcactgcgaacgcggtctcgtctccgttggcaccgccaccggcagggtcgatctgcatgtggacaccctgaagctccgcagtctccccggagatttcgtgcggggccatcatcaggaagccgatgccactggactggaacgtgcgctggtgctgctgggacatgccacgagtgatcgtcagcgggtagcgggttccgccgcccggaatcacgatcaggttctccgtcttcagagggaagcgcatggcgtccatgagtcgggtgttcagcatgtagttcagctggaacgaggacgggcctcggtccttcagcttcgcttgcagcttggcctcgtcgtaaatctgctcgtcggtcggctgcccctcgtcgcccatcggaccaccgccaaaggcgagggacgggtctgcttcgaggcgctgtacgatagacggggccagatgcgggccatacgcctcgcgctgtgccggggtagggtagcgaccgggccagatgcgaacgtcgaagccacgacctgggagcgtgttgtagatgctctcgctggtctgcggcgtgccgaggtacaggatgcgtgccgggatgcccggacgacctgtgcagatggcggagaactccagtgtgatgttcagcagcagctcgcggttagcggcggtgcggctgttcttgttggattccacgtcgtcggcgatcagaaggtccgcgcgcttacccggcaggttgccggtgacgccgatacacgccacggatggcgagcggtcgatgcccttcaggctatgatgcacgtcgaaagcctcaaccgaagtgcggtcgcccgcattcttgtcagggcgaaggcattcgagctgcggcacggtcaggatgatgcgctggatcagcgtcgctgtctcgttggcgttggttccgcccgccgaaatcacgaggattcggtgctgcgggtcttggatcagctgccacaccgcgaagatcgcggtgatagtggtcttcgcttctccacgctgcgcctgcaccatcaggttgttcggcccgaattgcaggtagttggcgatgtcgtactgcatccacgtgggcgtgaagcccagcaccttcattatgtcgcgcatgaagacggcgaagtgggcgtagtgcttctggagcacagccagtttcttgcggcgcagctctgccgcttctgcggactcatgcgccattggctacgctccccggaaagttgacaatgttgtccagcgctgcttgcagctcggcctcctcggcctcggacacgtccttgttctccagcgtatcggccagttcgtcgagcgccttgttggcctcgcgcgtggcttggatgttgttgtccttcaggaacttgatcgcggcgttgatgtcggcggcagtgcagagttcatcattgcgtagacggtctttaaggaccgtcgccacgattacgtgcagctcacctagcgcgccttcacttgcgggatttgtcattgtggtctcccatgatctttcggtgctcgcgtgagcgccagtagaactgggcgaccgcatacagaatggcgagcgtagttacgattgcagcaccgtacgtgctgatgaagttgaggtagaccgcgccgagtgtaagcggcgaggtacggacgacctcattgaccacactcggcggggtcatgctgttctccttaaagttttgggtacaccttccactgaaggcggcggttgtttgccattcctacgttgagcagcttactggctgcaaccaacccggagagcagaacgtgctcggtcagcatgcgctctctctgcacacgacacactacctgactgctgttcttcacagcactcactagaacgtcagacagcgcctgcgattcagtctccaccacgtcgaggttgacgcagatgtctttgtagccagcgtactctaccgtgaccatgctaccgaccgaggagtcgtaccaccacaggaaggccgacgacccaccagtctggtagcccacaacggggcgcatcagctggtcgaagtcgaaggccacacgggtgacgttcggaacggagagtagtgttacagcagagccgccatccggcgtagcttggatgttggctccgtcgtagctgctcgtccacagggtgtctcgcttggcgctaaggccaacagctgaggaacccatagcgtagtccacgagcggcgcggtgaagcgccgactcgggagaacgtaggtgctcggatcaatgcctgacaccggtacagggatcatggcgtgtaccgcgaccacgcctgacgaactacgagcgaccacgtgtagttggaagtcttcgtcaggttatccgggaactcgattcggtagttcatccagccaacgtcatacgctacgccgtaccaacgcccgttcgcagcggaaggcggtgcgctgattgtgtactcgaacacaaagctcccgggaacataagtgcttgcaacaaggctagtgccgttgtaagaagacggcgcattcgcagtgcgcccaccagaccacgctgaggacgagagacgaatgtagtttcgactcgctgatccgttgttcttggacatggcgttgccgatgaagttcccgatgctggaagcacccacttggccactcgtgctgtacaaacccgaggtgtagttgtaggtgttaccgtcgaatacgaaggttccggacacgtcagttgcgtcgaggtagaccgacaaggtgtaagcgacgtacaggtactcggacgcgagcaccgtcacgctagtgggatttccttcggagtccttaatcagagtgcgagagaacagtggatagctgctaccggtacctc

SEQ ID NO: 28 - DNA, 43721 bp, unidentified
  source 1..43721: mol_type = genomic DNA
atgggccactgggcgcgcgcccggcgctgctggtccgactacaccggggaaccgctgctgtgaccgacgacaccggcatcagcaccaccccggtaccggagacggccggccagcgcatccgccgctggcgcgagcatccgggccagatggtccgcgaactgttcaacaccacgcccgacgcctggcaggacgacgtgctggcggccttcccgacgaacccgcgcctggccatgaaggcgtgtaaggggccaggcaaaaccgccgtgctggcctggctgtgctggaacttcatgctgtgctacctgcacccgaagatcgcggccgtgtcgatcaccgcggacaacctggccgatggcctgtggtccgaaatgtcgaagtggcagaagcgcgccccgctgctgcaggcgaccttcacctggacgaagacccggatttacgagaacgcgaaccccgaaacctggttcatgtcgtttcggtcctgggccaagggcggcagcgccgagcaacaggccgacaccctggcgggcttgcacgccgacaacatcatgttcgtgatcgatgaggccggcgggatccccgatgcggtgatggcggcggccgaagccggcctggccaacgcggacggcatcaacctgcacgcgcacctggtgatggccggcaaccccacgcacctgtccggccccctgtaccgggcgaccaccagcgagcgccatctgtggtggctggtggaaatcacgtcggacccggacgacccgaagcgcacgccgcgcgtgtccgccgagtgggcgcgccagcagatcgagaagtacggccgcgacaacccgtgggtgcttgtcaacgtgttcggcaagttcccgccgtccagcatgaacgccctgctggggccggacgacgtggccgcggccatgaagcgccagcccaccgaccagtcgtggcgcgccctggcccgcatcatcggcgtggacgtggcccggttcggcgacgacgccagctgcaaggcccgccgcaacggcaatgtgctgttccccctggaaatcggccgcaacatggaaagcctgcagggcgctggctgggtcgcccaggacgcccgcgacttctacaaggaccagtcgaacgccaagcccgacgcggtgttcgtggacgacacgggcggctggggcgccggctggatcgaccagctgcgcgccctgaactacaccgtgaccggggtgggcttcgccggcaaggccgacgatccgcgctacttcaacaagcgcaccgaaatgtatttccgcctggcgcacgccatcaagcacgaaggcctgtgcttgccgaacgatcccgacctgtcccgcgaactgaccgcccacacctactacttccagggcgacaagatgcgcgtggtggaaaaggaccaggtgaaggaagaactgggccattcaccggaccgttcagacgccgcggcgttgacgtatgcttacgacgtggcgccgggggatcggagccaggagaacaccggccaccctcgcatccagtccctggcggcgcaggtggccgaatcgtatgggtccggcccggccggcgaaccttacaacccgatgggataacgccatgaaactggtttcgatgaagaaggaaggcggccacggcaaggactgccattgctgtgaagccgtgccggccggctgcagtgaacccgactacccgtggggcacgcgcatcagcctggaagaggatcagattgcggccctgggcctgaaagccatgcccgccgtgggcgcgccggtcggcgtggaagcggtggccatggtgatcggcgtcaatgaggaacagcgcgacggcaagaccttccgccgcctggaactgcagatcaccgacctggccctggctgccgccggcaccaacaagtacgcccgcatgtacgcggacgacccgagcatgaaggactgaccaccatgtgcagcagcgccccgaaagtgaagcccgtagcatcggcccccgtggtcggccccgaatccgtggatgatgccgctgtcgccgagcgcgaccgcgagcgcaaccggatccgcagccgcggcgggcgccagtccacgatcctggccggcaacaccggcacggctcccaccgctcccgtgaagactgccctggggatgtgacgccatgtgcaattcgaccaccatgggcaaggtgatggacccggccaagctcctgaccggcaacagcgcgcgctgggcggatccgttgggcgtgacgaagacggccgtgggcgacccgaccggccagctgcgccgcaacgccgaaaccgagcgcgtgcgccaggacgttcgcaacggcggccccgagcgccgcgccgcggccaccaactaccagcagcagcttgccgcccagcggcagttcgccgcgcccccgaagaccgtgctgggatcctgaccgatgaagaccacccgcaagtatctggcccggcccctggtggcatcgctgccctgggccatccgttccatcctggtgcagcagggcgcgcatgatctgcgccccttcggcgtctgataggggaagccatggaaatcgaagccgcccgcgcgaagctcgacgccgccgcgacccagccgacgctgcagctgcgccagcactgcgaccgtcgccgggcggcgatgattgccgcgcgtgaaacctggatgccggactggatgcaggtaaccgagtacatcgacccggcccgcggccagttcaatggcgagggcagcaccaccacccggaagaagcgcagccggtccaagatcatcaacggcaccgccacgaagtgcgtgcgcgtggccaccgccggcatgtcctcgcacatgaccagcaaggcccggccctggttcaacctgaccaccccggacccggccatgggccagctgcaggacgtgcgcgtgtggctggacaacgtgaccaccatcctgcgcgacaccctggcgaagtccaatttctacaaggccatgccggtctgctacaccgaagacctgtcctacggcgttgcggccatgatgatcgtggagaacgccgaagaggtcgtgcgcttccacccgctgaccatcggcagctatgccatcgcgctggacgacgctggcaaggtcgattcgctgtggcgctgctacacgaagaccgcgcgccagctggtgcagaagtacggccgcctggacccgcagacggggcagcgcgtgccggacgaatccaagctgccggaacgcatcatccaggcgtacaagaacagcccggaccaggaattcacggtggaagcgctgtacgagccgaacccggacgcgcgccctggcatgggtccgctgggcgtccaggcacccaggtaccgcccgttccgtgaagtggtgtggatcgccggcagcggggatgcgaagcacggcgtgctggacatcggcgggcactacgaacagccgttcgtgtccatccgcttcaacccggtaggcgacgacacctattccgcctgccctggcaccgactcgctgggcgacatcaagcagctgcagtacctggaaggccagaagctgcggctgatcgacttgatggccgaaccgccggtcaccgtgccggacaccatgcgcaacatcggcgccagcctggccccgcggacgaagaactacctgccgcagaatcagaacggcgccaagatcgaagccacctacaccccgcagccggggtcgttgcagtgggttcagcaggaaatccgcgaggtcgaagcgcgcatccaggattcgttctactacaacctgttcctgatgctggaatcgctgggcgaggcatcgggccgcacggccacggaaatcgccgagcgcaaggaagagaaggccacggtgctggggccgacgctggaaatcgtcaccgacgaaggcctggacccgaccgtggtgcgggtgttccgcctgtgcgaacgcgccggcttgatcccgccgccgccggccatcctcgcccgcatccccttgaagatcgagtacaccagcatcctggcccaggccatgaaggcgtccggcaccagcggcatcgagcgcacggccggcttcgtggcgcagatggcgcaggtgttcggcccgtccgccctggacaagttcgacgccgaccaggcggtggacgaatacagcgagcgcacgggcgcgccggccagcatcgtccgcgacgacgacgccgtgctggccatccgccagggccgcgccgcgcaggaagcgcagcaggcggcgctggccgcggccaagcctatggccgatggcgcccaggccatcaagacgttgaacgaagcggtgccgcagcccggtagcctgggtgaaggcctggccgaacagctgcgcgggggacaagccgcatgacgcaccccgccgaccgtgaggccatcgaagcccagcagcgtgccgagcgccagggcgaaaagtggttccaggaacagctgcgggccgacgtgcagcaggtgatgaatctgcccgccgcgcgtcgtatcctgtggctgttcatgcaacagaccgggctggacgcttcgccgttcgccaccaacgccatggcgcagtcccacgcaatcgggatgcaggacgcggcgaagtggtggctgaacctggtgcgcgaccactgcccggagaaggaagcgcagatccgccgggaaggcctggcgcaggccaagccgaaaaccaccgaacaggaacccgaagaatgaacaccgaaaacaccaacaccgccgacagccagcaacccaatcctggcgaaggcgcaggtgcagccaccgatgcagcgaacccgaacgggcagtcggccaccgcgccggctgcagcgccaggtcagggcgagggtggcgataagaccggcagcgatgccggcaaccagggcgaccagggcaaggcgggcgacgaagggaagactggcgacggccagggcaagaccgacgacgaacagcccgtactgactggcgcgcccgaagcgtacacggacttcacgctgccggacggcttcacgctggacggcgaacggaaggacgtggcgctgtcgctgttccgcgacctgggcctgtcccaggcgggagcgcagcgggccatcgaccacttcatcaagacggtgggcgaggacgcggcgatgcagcagcaggccatggaagccgctgtggcgcagcagcgcgacgactggggtaagcaggcgaaggcggaactgggcgaccagtacgatgccgaagtgaaattcgccaccacggcggttcacgctctgcagaatccgaagctggtggcggcgttcgatgaactgggatggggcaaccacccggaactcatcaaggcgttcgccatgttcggcaagatgatgcgggattcgcctgtcgatggcatcggcagcggcgggtccgcgaagccggacgtgaagccgtggaaccgcctgtaccccgacatgtaacaccctcaaaccctgacctgaccatctgaaaaaggaatcgcaccatggcaatcctcgccaacggccagccgacgcttgcgagcgcggcggccctgaccactgattccggcgccgctgtcaccatcgcggaactgctggaacagacgaacccggctttcaacgacattccgtgggaagaggccaatagcaccaccggccacaaggtgtcggcgcgccagaagctgccggaaacctacctgcgccgcatcaatcagggcatcaagccgagcgcgtcgggctacggctccgtgctggaatcggccggcctgttcaacgcgctgggccaggtggacagcaagctggtcgaactggccgtggacaaggcccgtttccgcttcatggagaacaagggccacatcgagtcgatgggccagcgcttcttccagtccatgctgtacggcgatccgaacgtggtgccggaagacttcctgggcatcgcgccgcgttacgccagcctggccgccgctgaccgcaccgcggtgcagatcatcgacgcgggcggcaccggttcggacctgacttcggtctacctggtcggctggggcgaaggctcggtgatgggcttctacccgaagggtacgcaggccggcatcaagcacaagcccttcccggaagcgatgatcgatgacggcaatggtggccagtacgcaggcttccaggactggttcgacctgaacgccggtattgcggtcaaggattaccgcaacatcgtccgcatcgccaacatcgacgtttcggacctgcagtcgggcgatcccatcaccggcatcactgccggcgccaagctcatcaacctgatgaccatggccatggagcagatcaacaacccgaacggcctgaacctggtgttctacgctccgcgcgtggtcggtaccttcctgcgcctgcagatcgtgaacaaggcgaacgtgtgggtgaccacccgcgaaatcgccggccagaaggtcacggacttcgatggcgcgccggtccgccgtatggacgccatttccctcaacgaaacccgcgtcgtcgtctaatcgacggcgccggcccttcacaaggaatcgaacccatgatcctcgatcagctgctgtacttctccgacaaccaggcggtgcttgccgatggcatttccaatgtcatcgaccgcggtgccaacgctccggttctggccaacttctcgcccggcttcgctggcgacctgttcctggtcgtgcagaccggcaccgctttcacgggtgccaccgcgctggaagtgaagctggcttccgacagcaccgccgacctggccacgtcgccgaccacccacgtttccacgggcgccattccggtggccaacctgggggcgaacaaggtggttgccgttctgccggtcccgccgggcgactacgaacggtatgtgggcctcatctacgacatcaccggcaccggtaccgccggcaccatccgcgccttcctgacgcagacccccggttactatcgcaagatggcggccaacaacccgcaggcccgtaactgaccgccctggatccggccctacggggccggctccactgaccaaggaaccgcatcatgagcaacacgaagccgctcaacccccgcaccgcgcgcacgccggccggcggggaacagcagtacgtcatcgcgcagggcgcgccgcagcactacgtggacggctatggcctctgcaacgccgggcgcatcgtcaccctggcgcccggcgtggatcccggccgctggatggtcgaagtggcaccggaagacgccgagaaggcccaggcgtctgaagccgatgcccagcgcctggcagtgctggccgccgccaagatcaaggcgaaggccaacagccaggacgtgagccgcaagcaggccgctgaccaggcggcgcaggcgcaggccgctgccgatgcccaggcgaaagcccaggcggaagccgatgccatcgccaagctggcggaatcggacgcgaaggcgagggccgccgcggaccaggccaccgcggagaagcagcgcgccgatgaactgcaggcgcagctggacaaggcgaacgccgatctggccgcggcgcagtcgcagctggaaaaggccaacgcagccgaagccgaaaaggccaagggtgccgacaccaaggctgacgccaagccggccggcaacgccaagtaattcccgcctccccggcgggcgtgcagtcggggtcggcgtattgccggcccctctttttaggtgcagaccgtggccacgcagaccgacattttcaacctggcgctttacaagctcgcccagtccatcgccatcccggcggtcactgacgaatccaaggccgccgacgtgatgaaccgcctgtgggagccgatgcgcgacctggtgctgaccgaacgggtgtggccgtgggcggtgcgctcgcaggcgctggcgctggacgtggaagccgcgcagccggggtggtactaccgttatgcgtacccgaacgattgcctgaccgcctacgcggtcacggatgccaacggcatcgccgccgccggcaagctctcgcgcttcacgaatggcgactacatcgccagcgtgtggggatcgggcgccttcgactgggacaccagctacggcgaacaggccaccacgatcaacacgaacgtgcgcaacgcctacctggtgtatgcgggccgcgtggaagacaccggccggtacccgccgcagttcgtcaatgcgctggcctgccggctggccgccgaagccgcgccgccgttgatcggcgaagtgggactgaacaacaaaacccagctgctgcaggaatacacgctggcgctgaccaacgcaggcgcgcatgccatgaacgaatcgcgcacggacgccgactacgtgacgcctgccctggccgcgcgcgacagcaacgtgtggccgggccgggggccgtactgatatggccaagttcctgcagccctccctgtccggtggcgaactgtcgcccggcatgcgcggccgcgtcgatctggcgcgctacgcgatcagcctgggcaagtcgcgcaacttcatcacgaagccgaccggcggcggcgccaagcgccccggcaccatcttccgcggccgggtgaagttctccaacaagctgacgcgcctggtgcccttcatctactccaccagcgtcaagtacctcatcgaaatgggggacggctatttccggttttgggtcaatggcgcgctgctgaccaacgcgcagaagcccatcgaaggcatcacccaggcgaaccccgcggtggtcacgtccaccggccacggctaccaggccggcgaccaggttgtggttaccggtgtgcgcggtatgtccaaggtcaacggccgcaccttcaccatcgccgcggtcaccgccaacaccttccagctggtcggcttcgattccagcatcctgaccgcctacgcgggcggcggcagcgtggaccgcatcgtggaagtggccacgccctacgacgaagcgaagctgcgcagcgtgcgcttcacccagtcggcggacgttctctacatcgtccacgggcaggtgcagcagaaggaactgcgccgcctggcggtcaaccagttcgaactgcgcgacttcgcgttcaagcgcggcccgttccgcccgttcaacagcgacgaagcgctcatcatggcggtgtctggcaccaccggcatcgtgacggtcagcaccaacgtggacaccttcaccgccgacatggtggggtcgctgctgtacgtagaggaaaaggaactgcgcggcgtgaagccgtgggcatcggccgaaaagaatgtgccggtgggcgcgctgcgccggtcggacagcaaggtgtaccggtgcgtgagtatcccgccgagcctgggcggcaagggcacgccctactgggtcgccggcaacgtgcgcccgatccacgacagcggccgcgcgttcgacgggccgcaggacatcaaggacgacggcgtgaacagctacgcggtcggcgtggaatgggagttcttgcacaacaccttcggcatcctgcaggtgcagtcgtacaccgacgcgcgccacgtgcaggccgtggtgatcgagcgcgtgccggacagcatcgtgggcaccgcgccggcaccggccaacagctggacgttcagcggcgacggcagcaccaaggtgttcagcatcacgggcgccctgagcggttcgaccctggactacaaggtgaacatcgacggccagccgatccagccgaacccgtactacggcggcggcggcggggtgaacggcagcggcggcggcagcgtgcgccccggcggcagcagcaacgtgcaacaggaggcgctctaatggcgcagggctggaccatcaaccccaccgcggacacgatcacgttctacgaagcgccgcccgtgggcacgaacaacatcctggtgaacgaactggccgatgctggccagggtggcaccgacgtgtgggcggtcggctcctggtcgggtcgctacggctacccctcggaagtcgagttcttcgccgaccgcctgtggttcgccggcacgcctgcggacccccaaaccatttgggcgtcctgcatcggcgattaccccaacttcggccggtcctcgcccatcgtggacagcgacacggtgacgttcgtcatcaacgcgcgccaggtcaacacggtgaaagacctggtgccgctggacaacctgctggtgatgaccacgggcggcgaatacaaggtgaccggcgggcaggacgacgtggtgacgcccagcaccatcggcgtcaagaaccagggcaacgccggcagcggcgatgtgcagtccaagctgatcggggaatcggccatcttcatccaggaagagggccagaagatccgcgatctgcgctaccagttcgaaaaggacgggttccgcggcaacgacatcagcgtgtgggccgatcacctgttcgccggcttcgaagtcaagtggatcgaatactggaaggcgccctggcaagtggtgtggttcacccgcgacgacggcgtgcgcgtgggctgcacctacatgcccgaacaggaggtcgtgggctggcactggcacgacaccgatggccttttccttgacgcctgcgcgctgccggggaagaaggaatcggaatgctacttcctggtggaacggctcatcgacggcgaggtggtgcagtgcatcgaacagcaggccagcacgcgcgcggaaacggaatcggatctgtggttcgtggattgtggggtgcagtacgacggccggaacaccaccagcaccacgatccagctgggcagcagcgccggctggaccgagcaggacgaactgaccatcacggcttccgccgcgctgttcgtcggcgccacggatgtcggtgatggcttcgaactgtggcgcgacgtgaccacggtggaagacggcatcgccagcacccagcggtacaaggtgaggctggtgatcgactcctacgtggacgcgacgcacgtggtggcgcgcagcatcggcacggtgccggcggcgctgcgaggcgtggccctggccacctggacgttgcagcgcgacaccatcgacaacctgtggcacctggaaggcaagcgcgtcgtggtgctgcaggacgccgcggtggcaggcccgtacatggtgaccggcggcaagatcagcctggccacgccgggcggcgtgtgcaacatcggcctgccctatgcctgcgaggtcgaaacgctggaactgaactcgccgggtggtgattcgatgcgcgatcagcagaagctggcgtacaaggtcagcatcctgctgctggcgtcccgcggggtgaaggccggcggcgtcgtggacaagctctacccggtgaaggaacgccgcttcgaaccctacgggcaaccgccctacctgaaaactggcgtgttcgactgcgacatcccggcgggttggggcgtggatgccgggcgcgtgcgcatcgtgtcggacgatccgctgcccatggaaatcctgtcgatcaccaccagggcggtgtcgtccaacggccaggccggcggcgctgggggcaagggatgatccacgccaccatcgtgccggcaaccgtggaacacgcgcatgccatcgcggccaacccgcgcgcggcggacctggccgaactgtgggcatgcagccgcagcacgccgctggatgcgatgctgcggggcatggagcgcaccgccgagccgttcactgccatatacaagggccgcccggcctgcatgttcggggcttcgccgttctccatcatgggcgggatgggcgcggcctggatgatcggcagcagcgtgctgaaccagcacggcgcgcagaaggatctgctgcggctgtccgaaccggtggtcgagtacatgcaagaccagttcccgaaccttctttacaatttcgtggaccagcggaacatcgccgcgatccgctggctgcgctggctgggtttccagttcagcgatccgattgcctatggcgtggacggcctgccgttcctgcccttctaccgtcgccggggtgcgtgatgtgtgagccgattactatttcgaccggcgccgcctgggcgcttggcgctgcagctgccgccaccgcggcggccacctatgtgtccgtggacgccaacaagaaggcgggcgaggcgaaccagcaggtggccgagaacaacgcgcgcctggccgccgacgatgccgctgctgcccaggccatgggcgaccgggaatcccaggcgcagacctggcgcacgcgcgccatcatgggccagcagcgggccgccatcgccgccaacggcattgatgccgggatcgggacgccggccgaaatcctgggcgaaaccgccctgttcggcgaggtggaccagcaggccatccggctgaacaccgcgcgcaccgcctggggcttcaactcccaggtgcgcaacatccagaaccaggccggcatcgaccggttcaacacgaaggccaagggcaccgcgacggtgctttcgggcatttccagcatcgccagcagcgccggggggttctacgggtaatggctaccatcattccgcgcgtcaccggcccccaggtcgaggtccagcaggggccgcaggtacgcaacaccgcccgcgtcgatgactctggcgcgcaggcgctggccggcgccatcggcagcttcgcgcgtccggccctggaatacgcccagcgcgaacaggagcgcaacgacaccaccgccgtgatggcggcacgcaagcagctgtcggactgggaggccagcaccttcaacccggagaacccggaaggcatcaacaagtacaagggcaagaacgccctgggcgccgacgaagtgctgctgccggatctggacaagaccgtgggcagcatcagcgccagcctgacgccgcgccagcgccagcagttcgaaggcgtggccatgaacttccgcgacagcgtggccggtcggctgaacggctacatggaccgggagcattccggctatatcagcgccgaacagaaggcagcggtggacaacctgggcgccgatgcggtgtctgccggcgtggcgggcgacttctcccggcaggaccgggtggcgaacgaactgctggccatgaaccgcgcgcgccgccaggcggacggcctgggcgaagaactcatcaaggctgaggaacgcggcctggtgtccagcgtccggtcgcagaccatcgaaggcatggccacggcgcgcccgttcgaagcccaggcctacttcgaacggtatgccgatcagatgacgcccgaagaccgggcgaaggtggaccgcctgctgtacccggtggtgtccgatgccgccgcgcaggacgacgcggacgcgatcctggccggcgcccagcccgcggcataccgcgatccggggcagcgtggccgcggcccgtcgccggctgtggccaagatcctggacgaagaagccgacgcggccggtgtgccgcgggaatacctgtacgcgctggccgaacaagaatccggcttcaaccctggcgcggtgaacccggaagtgctggatgacggcgacaacgccaccggcctgttccagtaccgcgccaccagcgccaagggcttcgaccggacggatgcccgcgcatccgcgcgcgccgcggcccgtgagtttgcccagcgcgccaagaccggcggcgtggaattcgcggtcgccgcgcacttcgccggggaaggtggcgccgaagccgtcgtgcagcgcggccggcgtgcggagaacccgaagaccgcccggtatgtggaagaggtcatgggtcgcgcgtcgcgctggcgtggcgatgcgccggccacccaggtgggccgtaccgcgccgccgagcgaagccgatgccatcgcgcgcgcgcaggcgatccccgacccgcgccgccgcgctgccgtggtcagcaagatccgcgaacgtttccagctgtcggatctgcgccggcaggaagaggaccgcgccgcgtcggaaggggcgtacacggccatcaaccaggccgccaacccgaacgcgccgctgcgcgaaatcctgggcgcgcaggtgtacgcctgggccgagcggaagggacatctgaacacgctggaaaacctgcggaagaacaaggtggccggcacgttcacccaggacgacgccgtgctggtcgaatccttggaacgtgaggctgtgctgtcgccgcagaccttcgcgcggcgcgacattcatgcgctggccgaccgcatttccacgcagaccctgggcgagttgatcggcaagcagaagcaggcgaacgatccgtcgaagcgggccgactgggcgaaccagtcgcagcgcatcgaatcgggcctgcgcatcctgggcctggacgaaaccggcgacaaccgcaacgccgaaggcgagttcgtcgccaagccgccgaagaagaaggtggaggaacgtaaggtgcagcgcgcccagttcgcgcaggtgtaccgcgaggccgaacgcgccttcatccagcgccacggcaaggatccgacgccggccgaggcggaccagctgctgcgcgccgtcgtgcgcaatgtggccaccgacatccccggcaagctgtcgcgggctggcgccatcgaagggttcggcgcggcgctgccggccgctgaccggtcggaaatcatcagcgacttccgggcatcgaccgggcgcgacccgaccgaagccgaaatcgttaggattggggcacggtatcggatgcagtccaacagcgcggggtcgaactgaacatggggaagtattcggaaatcatcgcggcaacccaggccgaagatgaccaggcgcgcgcgcgcgcggccggcatcacggcgccgcaggtggagccggacgccatgggccgggccatgcgcctggccgaccagcgcggcctgccgccgggcgtcgtagccgacaacctgccggagtacgaccagcagcagcagctggacgcgctgggcgacgctgcgagcgcttcgccggtcctggcgcggtggttgggcgacccgaaccacacggcgctgtccaaggacgacacgggcgtgctgggcggcctgggccgccagttcaacagtggcctgctgtcggcgaaggaaacgctgccgtggctcccgctgccgcagtcggccatggacctggacaaggaacgcaaggccgcggccgcgcgcgggccgcagatgatggccagccccgacccgtcgtggttcagcgaactggtgggcaagttccaatcgggatgggaacagggcaaggcggccacggccatcaccatcgacggcatcaatccggtccggtacgacgaaaccgtggcccgcggcctggggtatgccgacgcggccagcggcaatgccgccctgctggcgaccagcgtggccgattcgcagcgccgggcgcaggccgccgacgtggagacggccgccaccacggccggcttcaaggaaattgcggacgcggagaagaccaaggacaccggcaagatcgcgcgggccgtggtcacgaacccgcgcgccgtcatggccgtggtggcgcagtcgctgggcaacaccgcgccgcagctggcgctgtcggccgccatgccggccagccggatcgtggccggcgtcaccgcgggcaccggctccttcgccaccgaacagggcatgaccatcctggacgtgatgggcgatgccggcgtggaaaccagcgacccggccgcggtgtcggcgttcctgcgcaacaagccggcgatggagaaggcccgccagaaggcgctgacgcgcggcgtggccgtgggcacgttcgacgcccttaccgctgggttcgcgggtcgcctgattgcgaacagccggcgcacggccgtttccatcggtgggcgcgtggctggcgaagcggcagtgcaggccggcggcggcgccgcgggcgaggcgaccgcgcagctggccagcgaaggcaagatcaccagccagtcggacattttcctggaagcggcggccgaaatgcccaccttcctggccgaaggccgcgggcagatcgcggaagcgcgccgcgccgccatgcacaacgccgaccgcttcgacgcgcaccaggaacagcgggcgatcagcgacctggtgaatctggcgtcccagtcgaagacgcgcgagcgttccgccacccggttcgaatcgctcatccgcgacatgaccagcgagggcgaggacaccatctacctgtccgcagatggcgcgcagcgcctgttccagtcggccaacagcgagggcggcccggacctgggcgcgctggtggacgcggacgcgctgcgcgaggccatcgctaccggtggcgaagtggccatcccgctggccaagtacgccaccctggtgacgccggaactgcatgcggccgttgccgaccaggtgcggctgcagcccggcgggcgccacgacgtgccggcggtgtcgtcggaagaaatccaggacgcgatcaccgccggcctggccgaagcgcagcagcaggagtcgcgcgagaacgggccggccggtcaggtatacgacgacgtggtggggcagctgctgtcccgccaggacgaacagctggcacggcagaacgcggccgtggtgcagtccgtgtatcggaacctggccgagcgcgtcggtaccgacgccagctggcacggcagaacgcggccgtggtgcagtccgtgtatcggaacctggccgagcgcgtcggtaccgacgcctggacgctgtaccagcagttcaagctgcgcatccccggcgccaccaccgacacgcgcgcccgcccgcgcggggtggacatcgacgtggacccgttcctggacgcgctgcgtagcggcaagctgccgaccgaccgcgaggtgtacggcgatactctggtgtcggcgctgcacgccgctggcggcctgcgcgattccggcggcgagttggccaacatggacgccgcgaaggcgcggccgggcctggtgaacaacctggccggcatgtccctggacgatgcactggtgtgggcataccaggaaggcttcatcacccaggcgccgacgaaccagcaggaaggcgccttcgatggcgacgccccggacatcaacacgctgctggacatgctggcccaggatcttggcgggaacccggtgtaccggccggcggcgatgaacgccgagcgcgccgcgttccgggaaaacgcccagtcgctgcaggatgaacttgaccagcgcggcatcgacctgcagcagaccgacaacgccaccgcgcgccaggcgctgggctacgcgaaccgcacgctggaacaggcgccgcagccggtggagacggacggcgtggactatgcggtacgcgacctggtgaccggtgccagcggccggcccgagagcgccgccacgcgcgcgctggtggaccaggcggtggcagatggcgacctggccaagatgctgcgcggcatcgccgcccaggaagggatcgacgccgaccaagcagcgcttgccctgcgcctggcggaaatcacgcccgaactgaacgtgacgatggtgccggcgccggcaaacgccaacgcggcgggcatctacaacaacaccacgaacgaaatctggatccaccaggctgtgccgtctgtcgtcttgcacgaagtgctgcacggcgtcacgtcggccatgatgaccagcccgacgctgcgccgcgcgaatccgaccgtggcgcgcgccgtggccgagttcaacgacttgctgggcgttgcccaggcccacttcgccggcatggaaaccgatggcgccgacgtgccggccgcgctgcgcgcgacgctgcaggatccgcgtgggccgctgtcgaacatcaaggaattgctgacctacggcatgaccgacaagcggttccaggaatggcttgccactgtgccggcgccggctggccgtgaggaagcgcgcaccgcctggcagtggttcaaggatgccatcgccaccatgctgggcgtgaccgggaaggagcgcaccgcgctggatgccttgatcgaatccaccagcgacctggtggacttcgcgcaggccaacccgcgcgcggccaacttcgcgcagatgagcgaggcgagccggttgggcgtgccgatcaccgacgccgcggcactgaaccagggcggcgacaagccgcgcggcgcggtgacgttcgaaggcgtgcccggcgcgcgggttttcaacatcgaactgctgaaaggcatggacgccagcaccttcatgcacgaaatggggcacgtgtacctggaagtgctgaatgatctggccgcgcgcgagggcgccccggcgcagatcgtcaacgacatggccacgatcaacgcctggctgggtcggaaaggcggaatgcctcctgtggcaccggggaaggtgcgtgtttaccacggtggttcgctgtccgacgccgacgtgggggatgtgtatttctcgacggacccgaagtacgcggaaggctaccgcggccagaatggcggcgatggcgtgtactggctggacgtggacgaatccctgctggaccgcgatctggcaatgggcgaggtgggccgcaattccatcgcgctgccgagcgagcaagccaaggcaatggcgcctgtttctgacggtccgcagccattcaccgtggaccagcacgaacagttcgcgcgcggctttgaagcctacctgcgcgagggcaaggcgccgtcgtctgcactgcgccgcacgttcgccgcgttcaaggtgtggctgaccgcgctgtaccgcagcgtgcgcagcctcaacgtggacctgacggacgatgtgcgcaacgtcatggatcgcatcgtggccagcgatgcggagattgaagacgcccgcgccgggcagtaccagggcgcgctgattgccgatggcatggctgtgggcatgacgttcgaacagctgcaggcctacaacgaagcggtgaacgccgcgcgcgcagatgcggaagcgaccgtggccgccgaagtgctgctggccgaacgccgcgaacaacaggcgtggtacaaccgcgagaagcgggaagtgcgtgcccaggtgcttgaagaggtccgcaatctgccggtatatcgcgcgcagcgcctgctgcggaacggcaagctgccgaacggcgagctggcccccgacgaactgcgcgtgaagctgtcgaaggacgaactgctggacctgtacgggcagtccttcctgcgcaacctggtcggcatgtactcggtcgaaggcggcgtgcgcgcagatgaggcagcggccatctacgggttcggctccggccgcgaactggtggaatcgctggtcaacgcgccgcgcctggccgatgccgtcgccagcgaaaccgattcgcgcatgaaggaccggtacccggacccgatgacagatggcacgctgcccgaccgcgccatgatcgcggcgcaccgcgaccgccaggcggacgtgatggtgcgcgagattcgcgcgctggaacagcacgtcagcgggcgccaggtgtcgcaagccgcggtcatcaagggcgtggcccggcagatcatccaggacaagaagctgcgccacctgcagccggccacctatcggtcggccgaagcgcgggccgggcgcgaggcattcgaagctgcagcgaagcaggactggggcactgccctggccgcgcgccgccggcagctgctgaacttcgaactgttccgcgaggctgtgcgcgcgcgcgatgaggccgcccgcaccgcgaagtacctggccaagttcagcgagacgaagacccgcgcgcgcctgggcaaggccggcgccgactacctggaccaggtggatggcctgctggaccggttcgacttccgcaagatcagcgacaaggcggcagaccgccgttcctcgctggccacgtggatcgaggtgcaggcgcagaagggaatcgacgtgaacctgccgcccaagatcatggacgaagcgttcaccattccgtaccgggaaatgaccgtggcggacctggccaccctgcgcgatgccgtccgttccatcgaccacctggcgcggttgaagggcaagctgctgctggccggcgaagtgcgcgacgccgcagaaatcgatgaggctatggctgccagcctggccgctgcgcacgcggcgcgcccggtcagcaccggggaccgcggtccgaaggacaagctgcgccaggccttcatgcaggggcgcgtgatccaggccaccgccaccgacatcgcccgcgaactggatgggttcaaggaccagggcgccatctggatgaacaccgtgggcgtgatgcgcgacgcggtgaacaaccgattgaacccggccctgcagcaggcgcaggacgaactggcccaggtgtacgtgaagcactacagcaaggcggaaatccgcgccttctctgagcgcgtgccgatgccggaagtgaacggcgacctgtggagcaagtcccgcctgttggggctggcgctgaactggggcaacgccggcaaccgggaagcgatcctgacccaggcccgtggccggatgtcgccggaacaggtcaacgcgctgctgtcgaagctggattcgcgcgactgggctttcgtggaagacgtgtggcgcctcatcgactcgcagtggcccgccatcgccgaagctcagaagcgccgcacgggactggtgccggagcgcgtgcaggccagcgccttcacggtgcagaccagcgacgggaaaaccctgcagatccccggcggttactacccgctgaaatacgaatccgattccgtcaagaccatgaaggacgaagcggacgacttctacaacagcattcgcaccgggcgcaccgccaaggccgccacgcgcaacggtcataccatcgagcgcgtcggatcgggcgggcgcactgtgcggctggacacgggcgtggtgcagcagcacctgcgcgacgtgctgcgcgatgtccacctgggcgatgcggtcaactacgtccacaacgtgctgaacggccaggagttcaaggaagccgtggacagcaccggcacccaggagtaccgccaggcgctggaagtgtggttgaaggacgcggcggccggcgagattgggccgcgcgtgtggcacgaacgcgccatgcgcgccgcccgccagaacttcaccgcgtcggttctgaccttcaaagtcaccagcgcgctgctgcagctgtcgggcgtggtgcccaccatcgtcaccatcggccagggccacaccatggccggcatcggccagtacctgggcaagccgcgcgcgatgacgcgctacgtgcgcgaggcgtcgccgtacatggacagccgcctgcgcacgcacatcgaagcggtgcagaccgtgatggatgcggaagcgggccggttcgccgcggggaaggccgccagcatccggttcggttactggatgatcggccgcgtgcaggggctggtggataccgtgacctggctggccgccgaacaggcgggcatggccaagttcggcaacgacgtgggccgcgcccgcgcctatgccgacgacgtggtgacgcgcgcccagggttcgggcgagttcatcgacaagtcgccgctgcagcgcggcacgctgggcgacaacgtgcgccaaacggaatggatcaaggccaccaccgccctgcagggctacatgatcgcaaaggggaatctggcctacgaacagacccgcaaggcgaatctgcgaaacccgcgccaggcgatgaagtgggccgccgacatggtgatgctgttctccgtggaaggcctgctgaccgcggccctgaccgcgaagctgccgaacgatgacgacgacgacggcctgtgggatgacctgggcgaatgggcgatcaaggatgcgctgtccacgttcttcggcgtgatccccggcggcggcgtgctggttgaccagttccgcggctacgattccagcggcgtggtggccggcgcctggcgcgcctacgccgaactgctggaaaagctgacccccggcgaggacggcgaagtgaacctggacaagggcgtggcgaaggcggcagtgtccgcggccggcgtcacgctgggcctgccgtccacccaggtcaataagaccatcgacgctattgcggcgcgcgcggacggccgcgacgtgtcgccatacgaatacctgaccggccccaagaaggaacccaaataatgaccgtttccgccaacagccgccgccgcgaataccagggcaacggcgtcacccaggtgttcaacgggccgatggcctatgcgcgcgcgcacgtctacgccttcctggtgaagggcaacacgatgaccctggtgcccagcgccagcttcgacgtggaaaagctggggtacgagtcgggtacccgcgtcacgatgcacacgccgccggccgccgacgaaatgctgctgctgctgcgcacgatgccgtacacccaggaaaccgacatcaccaaccagggcgccttccacgccgaaaccatcgaaaaggggttcgacgcgctggaaatgcagatccagcagctggtcgatggcacgatccagctggtgttcgaagacggcgaattcgtgtgggacgcgaagggtagccgcatcgtgcgcgtgggcgacccgcgcgcggaccaggacgcggtgaacctgcgcacgttgtacctggtcatcgaacagatccagaacggcggcggatcggtcggcgtcagcccgaaatactgggaaatcacgggcgacggcgaggataccgacttcgaactgcccggctccgacgtgtcggatttgctgttctacgacgtggtggtggaaggcctgtcgaaggagccttacgacgaatacaccatcgtggcggcgtccgatggatccgactttgcggtgaggttcccggcgccgctgccgaatggcgccgaaggcttcgtgatcctgcgcggctatgccaagccgttcaccggtaacaccccggtgcagacccttcgcattccgatcatcgacgtggacggcaccacctacaccgtggacaagtccagcgaattcgccctgctgcgcaccaccaacgtcaacccctgcctgctcaccctgcgcgccaaccagggcgatctgttcgacatggcggacggcagctatttcagcgtgtgccagcgcggcgatggccaggcgcgcatcgttgccgatacgggtgtgacgctggttcttccggaagggttcctgccctacacgcgcgcgccgggctccattatctcggccgtctgcgagtacgcggagggcgacacctgggtgctgtccggcgacctggcgcagagctaaaagaccatgaccagcccgcacattttgttcaccgccccgctggggcttcggttcatcggtcagccgccgctgcaggtggtcggccagctggacggctacgtggcgggccaggcctacgaaggccgcctgcagatcatcaacaacatcggcgattgcacggtgcaatgggtgtccgggacgatgccgccgggcacgtcggtgcgtgtggataacgacacctacgaagtggtggtggcgtggcccgagtacgcgccgccggacccgaacaccaccgtggtgccgaatggcagtttcgaagccggtgacgtgaattggtcgaagggcggcggctggctcattggccagggttctggcttcgacgccttcgacggcacgtggtcagctgcctacaccggccgcggcaccgccagcctggaaggcacgcgcgtgccggtcatcgtgggcaccagcatcaccggcagcatccaggtgcagcagggagggtccagcaagggcaacgtggtcgcaggtgtgatgctgctgtggtacgacgccgccggcaatctcatttcctacaacgtgggcaacatcgtccggtccggcagcaacggcgcgtggcacatttccacggtcaccgcggcagcgccggccggcagcttctatgtggccctgggcgtgaccgcgaaccggaagcgccagaaccgccggctgtgggtcgatcaagcgcgctggaatcactcctacgccagcggcgcgaacagcgacgacgattattgcctggtgctgctggtgcgcgattcggctggccgcgaagccctgtgggaaggatgcgtgggcgaacaggcgatctactacacgacgcagccctacgcgctggaagtcctggaaggcatcgatgccggcctggcccctatcgacggcgggctgcgggtgccgccgcaggtgttcgcggtcgaaggggccgaagcgttcctgtccattgtctccggcgagcttcgcacgccgctgctgactttcacggccccgccggaatccatcgacacgctgggcgttaccatcttgtcgggtgaactgcgccagatccagcgcgcctatgaagtgccgccggaaggcttggatgtcacgctgggcattgccagcggcaccctggtgcaacagctgattaccaacaacatgacgccggaaggcgtcgatgtctccaccaccatcgtttcgggaaccctcgtatgaacgctgaattgaacatccacaccacggccgcgggccggttcctcatcgaagcgttccgcatagacgcggacggcatcgaagtccctggatcgcgccgcgtcgccgcggaatggttcccgaacctgattaccgacaacggcctgaatcgcatgggtagaaacagcgattatctgggcaactgcatggtgggttcgggtagcgcggcgcctgcaaataccgacacgtcgctgcaatcgctggtggccagcaccgcgaccatccaggccgacaccaacggcaacaacgcttccccgcgctacgggtggcgccgcaaaaccttccgcttcggaacgggagttgccgccggcaacctgtccgaagtaggcgtgggctacaccaccaccgcggtgttcagccgggcactgattctggatggcggtggtagccccaccacgatcaccgttctggccgacgaagtgctggacgtgacctacgaactgcgcttctacatttccgaagcggacgtggcgttcaatgtggacatcagcggcgtgacctacgcctgcgttgttcgccctgccagcatcaccgaaggcatcggcacccaggtgggcgatgccatcaccgtcaacgcctcgggccgcgccaacgggatcaaagcctatgaaacgcaggtgcttggcgccgtaggaagcgagccgtccggcactgcttacgatgtgggctacacgaacagcgcttacaccgccggcaccttttatcgcaacacggtggccagcgcatctttgaaccaggccaacacgcccaccggtatcggagccatgcggatcgataacaccttctgcgattggcaggtgagcttcacccctaagattccgaaggatgccaccaaagtgctgacgctcaatgtgcgcagttcgtgggcgcgccatgtttaacaacaacaccctttccacgctgcccgtgccctcggctttcatcgaacaggtgagtcggcgcacggtgccgctggtggattacgaaatgggcggggtgaacgtggccgatgccagccagggcttgaacgtcaagctgtggaagctggaatcgaacggcgcgcagatgctgctgtctgccgatggcgtgcctgccatcgacctgttcacccgccccaacgtgtcgcaggttgcgctggcgttcgatcagaacatgcggccgcacgttgcgttcatgcaggaaggtgttgcgtggctttggtggtatgactcggtggcgggtgccatggtgttttcgtctttccctggcgtcaccacgccgcggctggccaccgacgaaaagcgcccgaaccaggcttcgaactcggacgttatcttggcctacgtgcgcgcgaacaacctgtatttcaggatgcagcgcgaacgcttccagaccgaacacctgttgaaatcggcggtcaacgccgaactgattgccatagggatgaaccgcgggaaccggctgcaatttcggatgcgccctaccgcatagaagaagggccgggtgatccccggccctttcctgttacgccttcggcagcgggagcgcgtagaagcgcagcctgtgcccgtcgtccaccgcgacgatggcgtgtcccagcttcctggcggtgcgcagtgcggtgggcaccacgctgtcgctgctagggaagtcgtgggtggcgatgttcaccccgtccgggtagtcggacacccacgccgcgcggcggcgctcttcttcgtcttccagctgcgccacgcggcgcttcaacgcctgcgcctcggactgggtgatccccctgcggcggcgcttcacggcgcaccgccagcagcttccagcgcggcctgtgcgtcctcggtcacttcggccagcaggtgcggcggcaggatgtccaggacgttggtgatggcgggcacgccccggcgcccgccgcgagcgttggcgattgccgccgcggcgcgcttcacctggtcaggcgtgatcggatccttgggcatggccatcgccgtttcggcgtcggcgatagcctcgcgcaggccaccccagtccgtgcagtcgttgcagggcggcgacaggtggcagctgcagttgcgcgacggcgggtggtcggtcacttccagcagccgttccagggctgcttccaggctggcttcacggctcatcgtcttctgctccatcgttgtcccagtacgacatgtcatcgtcggcggcgtcggccggcgcatcccacgtcgccggatcgatgccgtgttcgtccttctgctgcctggcgcactcttcggcgtaggccgcagcctcgccgatgtccagcccgccgcggtcgatgaaccgctgcgcgcaggttttcagccattggtcccgtgtcattggtatcccctgcaggttgtggcgccccgtgccggcggcgcctggtggtcagtcggcgctgcgcgcgaactgttcgatgggcggcgcatccggcgaacgctcgccgccttccggcagtccgccagccgtgcgcggcagagtgtcctgcaggcggaagcccagcagctgccacacctggtcaacggcgcgctggcgggaatacttgttccccagttcggcgttgaagttctcgatgctcacgcacgcggacatgccttcgacggtgaacccgttgtccagggtcagctgacagaccgtggtgcgcccgttcggcaggacggtgtaggtttcgccgacgatggcggcttccacctgttcgggggtaacgctccgcgcgttaccgaatgcgttactggtttcgttactttccatggtgctggcctcctttggccggtggtgggcgggttacttcgaaatgtctttcagcagcgcctgcagctggcgcagcttggcgccgtcctggccgctacgctcgatggtttccgccacgtcgatggcggcggcatccagggcgtcggcctttgccagcagctggcgcgcctgctcgcgcagggtttcggcaatctctgccaggttggccatcgggtcgctgctgttcgttgcgggcatgtcgtcttcctggtgctggatggtgggagtgcgagcggcgaccaggcgggggcgctgctcaatgcgctggaactgcccgtcgctctcgcggatcagcccctgttccttcaatgagcgaaggcacccatgcaccttcgcgtgttcgtacaccaggccgttgcgccccagttcggccgacacctgggcgagcgtccacccttcttggatcggcaccgtgtcgtacaccttcctggcgatgccggttaggccgtggatgatcgactgcatgcgtgctgcgttcatggtgtgcggtcctcagaacggaatgtcgtcgtcggcgaagtcgtccatgggcggcgcctggcgctggggcgcctgctgctggcgctgcggtgcctggcgctgcgtgcgctcgccatcggcagggcgtgcgtccagcatcttcatctggtcgcacgcgatgtcggtggtgtagtgggtcacgccgtccttgtcgtatttgccgtaacggatcatgccggccactgcgatcttcgaacccttgcgcaggtattcgccggcaatctcggccagcttcccgaagaacaccacgcggtgccactgggtttcctcgacctgttcgccttcgcggttcttccgcttcgacgtggtggccagggaaatgcgggtgatggccatgccgccctgcgtgtacttcacttccgggtcgttgcccaggttgccgatcaggcgcacgtcgttttcgatgttcatgccatagccttgatctgtgcgaccagggcatccagttcacgaatgaacagctgcaattcctggttcagggtggagaggtagggcagatcgcggtacacgcgcacgcgcagttccggcaggcccggccagtagctgcggaagtcgcaccactgccggccggacaccagcagctggccctgcacctgggccacgtggtcgctgggcaacttgcccgccagcactgcttcgatctgcaggtgcggtagcttcgttttgatttccagcaggccttcgtcgcccaccagggtgtccgggctgcagccgatccggccgcggcgcatgaacccgacctggcggcagtccagcgtgctggtggccatgtagaggtcgcgcacctgcggttccatcacgtgcccgcgctcggtgtgcttgttgccatcccaggtcggcacgtactccccggtgatcgtctcggccgccagctggtacagcagcttcttgcgcgtctcgctgggcgcgccgccgcggcccttggccagcaccgtgtgaaacaccgatgccgtgacgacgccgcagcgcgccgcgtgccattcgggcgtgccctgttccaggtcttcgaaaatctgcagttcgtcaagcatcggtcggttccttcgggatggcgtgcgcgtcgcgctggtggtcgtgcaggcccgccgccttgacgcgctttccgcacgtcgggcacgggatcttcgtggctttcggcaccgcaggttcgcggtcctttcggcaccgcttgctgcagtaccgcgggtaacccggcgattcgccgtccagggagacgccgcagccctcgcacagcgtcccgtccagcatcatgtcggcgatgtcacccattggtggcaccctcctgcggcttgttgtcggccagcttctgcttgcgcaggcggcccagctggtcgtgaatccggttgtagcagtcggccggcacctcttccagtgcctggatctgctggttacggcacgcgccgcgcagccagtccatgaacttgccttcgttgaccacgtaggcgtcgatcagatcgcgcaggatggccacctgttcgtcggtgatgaactccacctggggcgcgccaccggtcatcccatcgtcgtccatgtccttcgccgccacgccggtcgcggccatcagcgtgtagcgctgcaggtatgccacggtgctggccacctgctgaatcgcgttcttcttgccgctgttgtcgggggcggcgaacatttccaccgactcgctgtggccgtcgcggtgggccacgatgcaggccacggtgatctgcccggcctcctgcttcacgtcccagcggtgcgacaggccgtgcttgcccagggcggcgaccacgccatccaccacgtcggccagggtggcgtgcttgtagccgacgaacccgccgtcgctggtgctgtagcccacggccttggtcttgcggatgtcgatgggttcggccttgaacgatgccatggcggccacgaacgccttgcgcgcctgctcggcgtcccatttcagttgcaggtccagcagcttttcgaactggtccatggcgcccttctccatggcaatcacggccatctgctggaaggggttggtggagttggtcagcgcggtggactgcgccggctgggcggcgggcatgctgtccagcacttcgccttcgatggtggtggaagtattcatgcgcccaccgcctgcgcgaacgtcagcagttcgacccactgttcgtcgctgtggtcgtaccagccgttcccgcggtcttccaggtagtaggtgccggcctcggcatcgaagccgatgcccagcttgatcgcgcggccctgcacgtagtccaggcggatttccttgcggtactggttatccccagcgtccgaacgcaccaggatctgctgcagcacttcgtcggggatcccgccgggcttggcatgcaggaagcccatgccctgcggctggctcaggtcgtaggccttggcgatgaccttgggcaggttgtcgcgggtgatggtgacacgggtggtcggggtgttcattgctggtttccttcttcggtggcatcggccagcggaagcgtctggacaaagccggtcatggtggttgtggctactgcgaacttcttgtgcgcctcggtcatagcagtgcaggcggaaacaatttcctggcggaagttgtagccctcggcgattgggtaatccatgccaggctgcagcagcttcgccagttccttgccgtcccggtacgccgacttgttggcgacctttgcgatttcgtccagggtgatttccacgatgaaaacttcctcatcgcggtagttaacccggcggttggcaacgccaagaaccttcacggctgcaccgccgggatcagcacttccttgtcgcccgacatccatgcttcctgcatgtcgtcgtcggtgatcggcttggccggcgcgtagatccgtgcatccggcttcacgtcggaccagttcatgttattcacggcccagtcctggacctcgtaggggctggcctcaaacagcggcatggtgtcttcgtccaggctgcgttccacgtcgccgtcgaactcgctggcgtagtgcttcgcgcggtcgcgggcgatggtcagcaccgggacggcccagcggcttccgtccggggcgttgacgatgaacagcatggcagcgcgcctatatgcctcggcctcggcctgtgcgcgctcctgctcggcggcggcctgctcggcggcctcacggtcgcggcgttcctggtctgccttctcctgggcttcccgctgcgcctgggcggcttcgtcgtcccgctggcgctgctctgccgcctggcggtccagttcggcctgacgttccgcctgctcggcctggacgcgctcgcgctccacgcggtcagcttcggcctgctcggcgcgcaggcggtcttcctcggccaggcgcgcggcgcgctcggcgtcttccttctcctgctgctcgcggcgggccttggcctcggcgtcggccttggcctgcgcctcggcggccaggcggtcacgctcggcctgggcggcttcgtcggcgatgcggcgctgctcggcggcctcggcgtcgcgcgcggcctgctcctggcgctggcgttccagctgggcggcctgttcgtccaatgcctggcgctcggccagcatcttgcgcagcgcgtccagggcggtgtcgcgggtctgctgcgcggtcggcagatagacttcatcgaagccatccagttcgtcggcggccacgcggtcgatggcctgctgcagttccgcggcgctggcgcccactgcctgcagcggcatgttgcggatgttgtccaggcgcgcgttcatggcgccgatgcgctcggcctcggcctggcgcttcgcttcgcgctcctgctccttccggtcttcctcggccttgatctgcttatcgatggggtcttcgatggccaggatggcgtccttgatcgtgccggcgcgctcgttgatttccttgcccagcttcgacagctggctggtcttttccttgcggatgttctcggccttgtagcgcggttcgcggatcgcggcgcgcgctgccttggcttcgtccatgcccttcgtggtggtcacgtcgaacacgacgcccttgtacttggcggccaggtcagccaggccggcttctacgctttccagttcctgcatggcggcggtgcgcagcgccagggcgccggccttcgctgcggtggtggcgtcctggtcctgctcggtcgccgggtcgatttcgtgtgtcatcgttcgatccttggtgtggtggtgccggcgggaatccccgccggctgtggtgcgcgtcgcgctgttgaaccccagttacggggtgaaggtgccgatggtcatgctggcggattcgccgacctcgcccagcagcagcgccttgaactgcttggcgatttcgtcctgctcctgttccagggcgatgacgcggaagcgcagcgacggttcgcggccggtggtggaaaccgacacgcgcatgtggaacgtgcgttccggcaggcccaggtacggttcggtgcggaacgaaagaacgtccggcaggccttcatcgctggacgcggccaccgattccagcacgctgcgcgactgctggaagttgccttcggtctgctcggtggtggattcggccttgatcttcaccttgcggatggcagcgatggcgcgggccagcgggatcggcgagaacgcgccgtcgtcgctgacctggtgggcgccgatcaggtgggaccagtcttcgatgaagtccagggcgtcgcgctggctgaacgccttgccgccagcggcgagcatggccacgtaggcgggggtcgcctgcagggtcaggcgcgcggtgtggtcggcgtggcccggcgtggtggcgtcgcccaggttgaagaacacggtggcgcccagcttgtcggtgtcgatgaagccgtggccaccttcgcgtgccttcacgtaggtaacgaagtccgggatgctgctggtggtcagcttgccgcggaagcgggtgcggccggccagctgggcttccacgttctgcagggtgacgccgttggggacggcgaccaggtgcgcgatgctggccgggatctgttcctgggtggccttggccgcggcggcgctggaattctggatcgcttcgattgcgctcttgtccatgtggttcggtttcctgttgttggtgttgcggtggatgaaacgggagtggtggggatcagcggatcgcggcgacgttggcgccggtcacgccttcttcgggcttgaacagatccttgttcgtgttcggcagcacggtgatggcgccgcggttgctgacgtacatcacgctgctggtggaaatgtcctcctgcttcttgccgcgctgggtcggcgaagagaacttcacggtgtggtcgatctgcacctgggtctgatcgccacccaccggggtgatggtgaattccagcgtcaccttgcccttcttcgtcttggtgttgcaggcggcgacgcccagtgcggattcggcgagcgccgcggccagacgcggccccagggtgccgccgtccagttcggccatcagggtttcgatgctggtgtggttcgggttcatcgctgttgctccttcgggttggtgccagccacgcggccggcggggaaaaacgtattgaactcagtggtgcagctggcggcccggcgtctgcggaacagctgcaggcgctggtcgttggtcaaaggctggcgcggttgcttgccatggcgcaccagttccaggctggaattgcggaacatgtcatttcctccgggacgcatccacgatgaccacgaacgtggtgcccacccatatcagcatcggcaccaggttctgcatgaagaaggccgccaccagggcggggccaagaacgccatgcaaggcgcccaggaacaggccgcgcgtgcgcatcagtacatccccccttcgtggtcggcatggcgagactcgtaaagcgcttccgcggcggcctcttcggatgcggccaggtcagcatcgaccagggtttcagcatcggcgcgcagctgttcgcgcactcggtcgcgcagcttgtggaagaactgcacggcttcggcgccgaacgcggcgtcggatgacagcagcaccgcggccatgtccgccgcgaacagcgtgttgccgtcgctgcccacgtcgctgtcgcccatcaggatgtccagggcgctgctgacctcggcgctgctttccatcagttcgtccagcttggtgtcgatgaactcgccgcgcgagtcgttgcggtcctgctcggccaggtagcggttcaggtcggcggtgacggggcagtggttcactggtcacgctcctggccggcggcctgctggatgcgctttgcatcgcggcggttctgcttctcgcggcccagttcgatcatggtgcggaagtgctggatgtcgcgttcgctggtggcttggtcaggctccacgtattcgatggcgacgccttgcggactggtcttttcggtaatgcgcatgggatccctcggtggccgtagctcgtttgtgccgccaacgatacgcccttcccggaagttgtcaacccccattgcgcaattcctgttgcggctgtatggtggccccgtctcaaccaggaatagggccatccccaacatgaaaacgaagacgtggaacagggcgcagaccgcggcgcagaaggcgcagcgcgaacgcatcgccgccatcatggcgcgcgtggacaaggccgagcctgaccccatcgccgacatcgcccgcgacctcggcgtgagccggcagcgggtcagccagatcgtgaaccgcgagcgcgcccgcgccaaggtgccggcatgagcgacaaggccaccagcaaacccgattggaaggatgcgccggagtgggcgcggtggatggcccgcgacgctgatggggaatggcgcgttttcgagaatcagccgtcgcctgatcttgaagcgggcatccaccgtccgaatggcggccgtcacatgccgctcaaaccctgggcagaatctgcggagaagcggtcatgaccagcattcaagcaagggcggcgcgcgatgccggtatccagcaggccgcggaacacgccgacgacgtgaacccgaactggggtgatcgcgcgttcgaagtgctgcgcatgttcgccgcggccaagcgcgccagcggaagcagcttcaccagcgaggacgttcgcaacagcatcctgggcgcgcacctgccgcagccgccgcatctgcgcgcctggggttcggtgttccagcgcgcggcgaagcaggggatgatcgtcaaaacgggcgtcactgagtcgcgggcagcgcactgccactgcgccttcgtggcgacctggaaggcggtgtgacatggcaggggactggctgaaattcgaaaaggacacgctggacaagccggaagtgttcgccatcgcggaagccctgggcatcgacccggatgcggtgatcggcaagttgatgcgggtgtggtcctggttcgattcgcataccgtggacggtaacgctgcgcgcgttacctcatcgttgcttgatcgtgtcgctggcgttcctggcttcatcgctgcaatggcgattgagggctgggcgacggtcgatgctgctggcgtgtcgttgccgcacttcgaccggcacaacggcgaaaccgccaagcagcgggctttgacggcgaaacgggtgcagaaacacaagtcgaaaggtaacgacgcaggtaacgctgacggcgttagcggtgcgttacctagagaagagaagagaagagaagatatagaaaagcaaaaggccaccggccagcaggctggccacgacgccgagccgcaggacgaactgcccaaggacatccccacgccggacgcgccccaaccggtggatgacgcgcctgcagtggagacgcctaagcggatcaccagcaccggcaagaagcagaccgcggaacacttcccgaagttttgggcggcgtacccggtgaagaagggcaaggccgatgcgctgaaaaagtggaagctgaaaggctgcgacgcgatggccgatcagatcatcgcccacgtgcgccgcatggagcgcgaggacgacgattggctgcgcggcttcattccgcatggcagcacctacatcaacggcgagcgctgggaagacgagccgaagaaggacaaggtggccacggcgccggcaccgccgccggaatcgtttggcgcgaaggctgcgctggcgaagtccgaatccaagctggaaaacgccctgggcttcatccgccagcagcgcagcatgggcgcctatggcgagggcgaagcggcagacttggaaatgcgccggctcatggccgaagcgaccgaaaagtacagggggcagtgatgcgcgtcaggatctacaaacccaagcacgtccgcgctacgcggtctaagctggccgagcggatcgggcaggaactgccggcggaagtgatgggcctgcgcacgcggctgttgatggctgacgtgatgcggaagtaccggtgcggtcggtccaccgcggcgcatgccgtcgcgttggcgcgggtccgcgttggagtggagcgccgacaccatggctgaccatccgcattccacaacccgcaagatcgcgcgccgctacgtctacatgaagtggcgcacgatgatcgacccggcgaccggcgaggaagtgcgcgcgctggtggcctgcagcaacgtggatcggcggatcctgcaggggcgcaagttccgccccgatggccgcgtgcgctgcgaaatcaagaacccgcgcaacgaagggttccaccggctggtgcatgtgttcgggacgttcctggtgcaacacgtggacggctacgggcaccatctgaccggcaagggcacgcctgacgcgcatgccgcggtgaaggactgccaggcgcgcagcggtgccggctgcgagcgcgtcatctacgacctggacatacctgggatgggcatgacccaggtcacgcgcatggagccgcgcagcctgagctttgacgaaatggacgaagacgacttcgccgccgtgttcaagggcatgaccgaatacgtggcggaacacgactatcccgacctgacccagcagcagatcgcggatttcgaaaacctgctggaacaaccgtgaggatgcaggggatgaacgaaaaactgaaagaggcaataagcgaggcaatccgcgaagccttgggtggggcgctggactgcacgcgcgtgtggtcggcttggggtgttggcacgatgagcgaggacgatttttcgcccgttgccgatgattccgagcgagttggcgaaatagccgacgcggtgatggccgtactgaccacccggaagctggtgtgcgaaacctgcagtggctggggcatgatcggcgggccgagcttctatgcgcctgacgaaggcggcgagccgtgcccggattgcaacgcccgccaggcggtggacctgggaaggctggaacgcttcgaaaccgcaaccttcaacgagggcggaaatgtctgtccgtgcatggataaagacggcactggaacgtgggttcgtttcgatgacgtggctgctttgatcgatggcaaggggtcgcaggtatgaggcttgctattgccgatccaccgtatccccctttccatggggcgggcggtagaaagaatcgtgcttcgcgctggtatggggacgggcagaggtcagcaaaggatcggccggccgacttccaccctggtgcgtccgattgggatatgcctgaaaggcatcggaaattgttggaagatctactggacgaatatgatgggtttgtgatcgccacatccctggatggggttgctgcttacggacaactgccgtccgctgctcgcattgcagtgtggtaccgcgcgaacgcaaaccccggcgcacaccgcatcggaaccaagtgcgaggcggttattgtctacccgccgaaggggcgtaggtcgaaccgtggtggcgttgggatggtttctgaccatctttcctgtccagtgccgcgcggtggttttaccgggaggaagccggacgcctgggttgattgggtgctggatatgttgacgtggcaacctggcgacgttgtagatgatcttttccctggctcaggccaggtatcagatgctgtcgcgcgcaggcagaagtcaggtgtttcgccgtgacgttcagcggtaagtcgctgacgaagggcgacctagaacggcgaaggcttatccatgaaggtccgtgcatggcctgcatacagcgcggcatcaacatggccggcagcggctacgtgcagtggcaccacacggcagggaagaagcggcacgacctgacgtgtgggctgtgcatgtggcaccacatggcccggccgatgttcgggctttcgcatgcgcagttgcgcgagcaatacgggccgagcctggccgaaggatccaagccgttccacgctgagttcggatcgaacgaacacctgctgcagctgcagaacaactacctgggggttacatgaaaatcgtggtatacggcgatcccgcgccgcagggaagcaagtctttcaagggaacattcaccgggaaggatgggcgcacacacgcaaagctggccgagtcatcgaagcgcgtggcgccgtggcgccaggacgtgaagctggcagcagaaggagcaatcgaaggccgcggcgatcccggtgcgtgggtgccgatggatggcccgctgctgctggtggtggttttcacgctgccggcgccgctgtcgctgcccaagcgtcgcgcatcctatccgtcgaagctgcccgacctgtcgaagctggtgcgcagcaccgaagacgcactgaccgcggccggcttgtggaaggacgacgcgcgcgtggtggaatgtagggcgatcaagacgtacccgtccgacacccttggcgcgcacccggacgccctgcgtaggcctggcgccgtgatcgaagtgctgccctatgcaggggcgcaataaatattgcgcaatgggtattgacaagtcggaaatgggcgtgcgaggatggcgccgctggtggtgaagcacacggttacttctcaatgggtcgcgggttcgactcccgcagcggttcgccgcttagctcagctggtagagcaatcgacaaaagcccgtgtgcgccccattccccagcaacgaattccgtaacaacccaagagcgtgaagaattcggtggtgtaggttgcggttacttctggcaatgaaaaatgccgcagccgtttgttccccgatgttgattgccagtggtgtagtggtcggttacttcctatctcaaaggggtgacgtgggttcgaatcccaccgggtgcttcggctcccgtcgtctagtggcttaggacaccaaaaaataccgactgcgtttgttccctggcttgttgttgttttaccccgtggtgaaaggtgcggtttcatcggattaagccggcttcggccggtggtggttcaagtccaccagccgcccctgatagttcccggattcggtttcccttgctggtggtgtagtgggcagttacttcgactgttaatcgagaggtcgccggttcgaatccggccacacgccgaaaggcgcgtgtagctcagttggatagagcgctaaaatctctgcccgcgtctgttccccagcttctaccgaattcggatcactccaaccttgcgaggatccgcacatgcagcgcaacgccgcaccccgtcgtaacaccgaagtgacccatggcggttcgcccgccttcccgcacgtctccccgatccagcagcttcgccgcgccgtcctggcgtgtttgctgtgggaagacaccttctacgaatcgggcgagtccatcgccgaccgcatcgccggcctggtcggcaaggtgaagccggaagacgtggcggccctggccgtcgaagcgcgttccgaacacaacctgcgccacgtgccgctgctgctggcggtcgaattggccaagcacgcccgcggcaccggcatcgtgtccgacaccatcggcaaggtgatccagcgcgcggacgaagtggccgagttcctgaccctgtactggcgcgacggccgcacgcccatcgccaagcaggtgaagaaggggctggccgcggcgctgcgcaagttcgacgcctaccagctggcgaagtacgaccgcgaaaaggcgatccgcctgcgcgacgtgctgttcatggttcacgccaagccgaaggacgacgcccaggcggcgatctggaagcagctggtggacggtaccctgccggcgccggacacctgggaagtggccctgtccggcggcgccgacaagcgcgagacgttcgaccggatgctgcgcgaagggacgctgggctacctggccctgctgcgtaacctgcgcaacatggtcgaagccggcgtggacatgcagctggtgcgcgacgccgtgctggcccgcaagggtggcgcgaaccgcgtgctgccgttccggtacgtggccgccgcgcgcgtcgtgccgcagctggagcccgtcatcgaccaggcgctgcaggcggcgatcagcgaactgccggcgctgcctggccgcaccgtggtgctggtggacgtgtccggttcgatggacgccaagctgtcgggcaagtcggacctgacccgcatggatgccgcggccaccctggcggccgtggtgaactgcgaacagctgcgcatgttctccttctcgtacaacctggtcgaagtgcccccgcgccgcggcatggccggcgtcgatgccttgatccggtcgcagcagcacggcggcacggacctggccggtgccatcaccgcgatcaaccggcagttgcagtgtgaccgcctcatcgtcatcaccgacgaacaggcgaccaccggacgcgtgcccgatccggtcgcgccgctggcgtacatggtcaacgtcgccagctacaagaacggcgtgggctacggcaagtggacgcacatcgacggtttcagcgaaggcatcatccgctggatccaccaggccgagcggggcgattgaccgcccacgcctgacgtgcaacgctgtacccgcggccatcccctgccgcctccccgccccggcctgcctccccagcagccggggcttttcattgactggccacggcgggcgccgcatcatcacgccaccgtccgcgaaatcgtgtcccaggggaaaccatgtccgaccaagccgcgaagctcgcgctgcccatcgtcgccgagttcgaagggttccgcccgcatccgtatcccgatcccgccagcccgttggccaaggcgacccggaaagaaccgtggggccacgtccctgcccgctccatcttgaaccgcctgccggccgccaccgcggcgctgtccggcgcgccttggaccatcggctacgggcagaccggcaagttcatcacccccgataccgccccctggtccgacgctgtggcccgcgcgaacctggaagaggaagtgcagatccgcgtcgatgcggtgcgctcccgcgccaagcgcgacggcggcacgctgcaggacgcccaggtggcggccctggccagcttcctgttcaacgtcggcgagggccgcaaggccgccggcaaggatccgggcaaggacggactgttcatgctgaaatccggccggccctcgaccctgtggcgcaaggccatggaagggtgccacacctgcgccgcggaccagttccccgcctggaacaaggccggcgggcaggtaatggcgggcctcacgcgccgtcgcaccgcggagcgtagcctgtaccttcgggcgggctgacggtggacgacttcatggggccgggcaaggtcatcgggatattcggcgctgcagcgacggccggcgccaccgcggtggaagtggtcacaaagaccgaaaccgtggtgctgaacatcccgctgtcgatgctgctggtggccatcgccggcaccatgatcggctttttcatcctcccgtcgaaggacgccgcccgtatcagcccgaaccccggcgcgaccgggcgccagcgcgtgctgtacgtgctgttctcgctcgccatcatcggggcggcggtcatcgcctacgccatcatgtcggcctggatcatccaggcaggcgtgtccatcatcgccaccgtcttcaagggctggcgcgtcgaagacggggcaatcatgccctgcactggcctggtcggaatcggcatccgtctgtggcttcctacccttctgaaagcagttgagcggcgcgccgaccgcgttatcgggggttccccatgaagtggcttatgtggatcggcggcggcttggccggcgcggcggcaatcgtcgctgtgctgtacttcctcggcctgggcggtgtggtgcgtgtggtccgggcggcgggcaacttcctgggcgatgcggccgaatcgctgcgggactggctgcgcaagccgggcaacaaggtccgcggcctgtgcgcggtgttcgggttcctgttcctggccgcggggctgcagtcctggcaacgcggcacggtcatcatccagcagcgcgccgactacacggccctgcaggagaagaccacccaggagaagcgcacgctggccgagcagatcgcggaccgcgaagcgaccatccggcggttcaccgacctggccgagcgccagaagcagctgctggcccaggctgcgcaggagaacgaagtggccctggccgctgccaaggcggcagctgtgcgtgctgcggagtcggaacagaagtaccaggacgccttccagcagcggcccaccgaatgcaaggcggcgctggaagtgatggctgcagcctgcccgaccttgaaggattactgaccatgcgcgcgttgctttggcttccctccatcctgctggccgcctgcgggcgtcaggccgtcaagccggacatccccaccaccccggccggtgtgatcgaagtgcccgtggaagtgtatgtgcccatcgacgcggaactgaccgcgcgctgccagtggcgcgagtctgccccgctggaagtcatgcccagcgtggcgcgcgagcgcaagaagtgcctgcagttctacgaaggcaacctggacgccatcgagcgggtgcagggccggcccgtcccgaagctgggccaccccacccctgccatcaaacggaagaagtaacgcacgcagcgttaccttcaccgttacaacgtcgttaccggagcgtatccaatgaacctgtcgtttctcgccaccatcgccttcgccatcctggtgatcgtcggcgccttcctcgcaaacctggtggtgctggtgttcacgaacagccagtggcacgtgtcgggcgtcgtgctgtcgatcctggccgcggccgccagctactgggcgcagcacaacttcaccgcctcggccggctacgcgcaggaactgctggtgtcccccggcctgaccgggctgcacgcggccgctgatcgggccgaatccctgggcgtggcgttccagtacgtggccatcgcctgcctggtggcctcggtcgcctgcttctggctggggatgcggtaatgcgcgggctgcgctgcctcggctgggtgggtgcgtcgctggccactgtgctggtggggaccgtcgccgccagctggctgggtggatccggcggcatgggcgtggcgatcctggccaccgtgctggcgctgctcatggcccagcgtgctgaggcgacctggtaatggctgggcgccccaccgtccggcactcggatctggatgaccggatcatcggcctgttgcaggaaggcaagtccttccgctggttcgattccgaagaggctgtgggcctgccgtccacggccacgattcgccgctggcgggccgacgatgccgaattcgacgccaggtgcgtgcgcgcgtgcgaggcggccgcggacgccgactacgacgaaatggagcgcatcgaacgccaggtgctgggcctggacctggcgccgggggaaaagccgctggacccgaaggccgcgaacgtggtgctgtcgaacatgaggtggcgcatggagaagcggaagccgcgcacctacggccagaaggtcgaagtgaaggcgcaggtgacgctggaacagctggtcgctgaaagcctgggcggcaccggtaccgccgggggtggccattgaacaacacggccgaactgacgcggcagatgctggccagggccgatgcggacgccctgccggccgaccacgaactgcgcgttaaggcccaggcgttcgaccaggccgcggtcggcttctatgcccagccgcagaccaccgacgtgcggaccttc

SEQ ID NO: 29 - DNA, 42368 bp, unidentified
  source 1..42368: mol_type = genomic DNA
tgcagcgccgacaccagcgtgtcgccgtaaatctcccggtcggtgggcatcttgccgctacgcagcgcgtccaggaacgggtccacgtcgatgtccacgccgcgcgggcgggcgcgggtgtcggtggtggcgccggggatgcgcagcttgaactgctggtacagcgtccaggcgtcggtgccgacgcgctcggccaggttgcgatagaccgactgcaccacgctggcgttctgcctggccagctgttcgtcctggcgcgacagcagctgccccaccacgtcgtcgtacacctggccggccggcccgttctcgcgcgcgtcctgctgctgcgcttcggccagcccttgatcgatggcctgctggatttcttccgacgacaccgccggcagatcgtggcgaccgccgggctgcagcctcacctggtcggccacagccgcgtgcagttccggcgtgaccagggtggcgtacttcgccagcgggatcgccacttcgccgcccgtggcgatggcctcgcgcagggcgtcggaatcgaccaggccgcccaggtccgggccgccctcgctgttggccgactggaacaggcgctgggcgccatcggcagacaggtagatggtgtcctcgccctcgctggtcatgtcgcggatgagcgattcgaagcgggtggcggaacgctcgcgggtcttcgactgcgacgccaggttcaccaggtcgctgatcgcccgctgttcctggtgggcatcgaagcggtcggcgttgtgcatcgccgcgcggcgtgcttccgcgatctgcccgcggccttcggccaggaaggtgggcatttcggccgccgcttccaggaaaatgtccgactggctggtgatcttgccttcgctggccagctgcgcggtggcctcgcccgcggcgccgccgccggcctgcaccgccgcttcgcccgccacgcggccggtgatcgacaccgccgtgcgccggctgttcgcaatgaggcggcccgcgaaaccggcggtcagggcgtcgaacgtgcccacagccacaccgcgcgccagcgccttctgccgtgccttctccatcgccggcttgttgcgcaggaaggccgacaccgctgccgggtcgctggtttccacgccggcatcgcccatcacgtccaggatggtcatgccctgttcggtggcgaaggatccggtgccggccgtgacgcccgccacgacgcggctggccggcatcgccgcggacagcgccagctgcggggcggtgttgcccagcgactgcgccaccacggccatgacggcgcgcgggttcgtgaccacggcgcgcgcaatcttgcccgtgtccttcgtcttctcggcgtcggcgatttcctggaagccggcagcggtcgccgcggtttccacgtcggcggcctgcgcgcggcgcgactggtcggccacgtacacggccgtgcgggcggtgtcgtagtcggccgccgactggtagcccaggccgcgggccacctgttcttcgacggatcgggaattcgcgtcccccaggttcggcagcgggatcaagccgaacccggctttgccctgataccaaccggattggaacttgcccaccatttcgctgaaccacgacgggtccgggctggcgcgcatttccggcccgcgcgcggcggcggccttgcgttccttgtccagatccagggccgactgcggcagcgggagccacggcagcgtttccttcgccgacagcaggccgctgttgaactgccggccaaggcccgccagcacgcccgtgtcgtccttggacagcgccgagtggttagggtcgcccagccaccgcgccaggaccggggacgcgctcgcagcgtcgcccagcgcgtcctgctgctgctgctggtcatactccggcaggttgtccgctacgacgccaggcggcaggccgcgctggtcggccaggcgcatggcccggcccatcgcatcgggatccacctgcggcgccgtgacgccggccgcgcgcgcgcgggcctggtcatcttcggcctgggttgccgcgatgatttccgaatacttccccatgttcagttcgtccccgcgctgttggactgcatccgataccgtgccccaatcctaacgatttcggcttcggtcggttcgcgcccggtggacgcacggaagtcgctgatgatttcggcgcggtcggccgccggcagcgcagcaccgaacccttcgatggcgccagcacgggacagcttgccggggatgtcggtggccacgttgcgcacgacggcgcgcaggatcgaatcggcttccgccggggtaggatccttgccgtgccgctggatgaaggcgcgttcggcctcgcggtacacctgggcaaactgggcgcgctgcaccttgcgttcgtccagcttcttcttcggcggcttggccacgaattcgccttcggcgttgcggttgtcgccggcttcgtccaggcccaggatccgcagccccgattcgatgcgctgggactgggtggcccagtcggcgcgcttcgaaggatcgttcgcctgcttctgcttgcccagcagggtgcccagggtttcggtggaaatgcggtcggccagggcgtggatgtcccggcgcgcgaaggtctgcggcgacagcaccgcttcgcgttccagggtttcgaccagcacggcgtcgtcctgggtgaaggtgccggccaccttgttcttccgcaggttttccagcgtgggcagatggcccttgcgctcggcccaggcgtacacctgggcgcccaggatttcgcgcagcggcgcgttcgggttggtcgcctggttgatcgcggtgtacgcgccttccgacgcggcccggtcctcttcctgccggcgcagatccgacagctggaaccgctcgcggatcttgcccaccactgcggcgcggcggcgagggtccgggatggcctgcgcgcgcgcgatggcgtcggcctcgctcggcggtgcggtgcggcccacctgctgcacgggagcatcgccacgccagcgcgacgcccggcccatgacctcttccacgtatcgggcggtcttcgggttctcggcgcggcgcccgcgcttcacgaccgcggcggcgccgccctcgccagcgaagtgggcggccacggcgaattccacgccgccggtcttggcgcgctgggcaaactcacgggcggcagcgcgcgccgatgcgcgggcatccttccggtcgaacccctgggcgctggtggcgcggtactggaacaggccggtggcgttgtcgccgtcgtccagcacttccgggttgaccgcgttggggttgaagccggattcctgttcggccagggcgtacaggtattcccgcggcacgccagcggcgtcggcctcttcgtccaggatcttggccacggccggcgccgggccgcgccctcgctggccagggtcgcggtatgcctgcggctgcgcgccggccaggatcgcatccgcgtcgtcctgggccgcggcatcggacacgaccgggtacagcaggcggtccaccttggcccggtcttccggggtcatctgatcggcgtagcgttcgaagtaggcctgcgcttcgaacgggcgcgcggtggccatgccttcgatggtctgcgaccgcacgctggacaccaggccgcgttcctcggccttgatgagttcttcgcccatgccatcggcttcgcgccgcgcgcggttcatggccagcagttcgttcgccacacggtcctgccgggagaagtcgccggacacgccagcggacaccgcatcggcgcccaggttgtccacagccgccttctgctcggcggtgatgtagccggaatgttcccggtccatgtagccgttcaggcgtccggccacgctgtcccggaagttcatggccacgccttcgaactgctggcgctgcttcggggtcaggccggcgctgatgctgcccaccgtcttgtccaggtcgggcagcagcacttcgtcggcgcccagggcgttcttgcccttgtacttcgaaatgccgtccgggttgccggggttgaacgtgctggcctcccagtcggacagctgcttgcgcgcagccatcaccgcggtggtgtcgttgcgctcctgttcccgctgggcgtattccagggccgggcgcgcgaagctgccgatggcgccggccagcgcctgggcaccggagtcatcggcgcgcgcggtgttgcgtacctgcggaccctgctggacttcgacctggggcgcggtgacgcgcggaatgatggtggccattacccgtagaaccccccggcgctgctggcgatgctggaaatgccggaaagcaccgtggcggtgcccttggccctggtgttgaagcggtcgatgccggcctggttctggatgttgcgcacctgggagttgaagccccaggcggtgcgcgcggtgttcagccggatggcctgctggtcaacctcgccgaacagcgccgtttcgcccaggatttcggccggcgtcccgatcccggcatcgatcccgtttgccgcgatggcagcgcgctgctggcccatgatcgcgcgcgtgcgccaggtctgttgctgggattcgcggtcgcccatggcctgggctgcagccgcgtcgtcggccgccaggcgcgcgttgttggccgcaatctcggcattcgcttcgccggtcttcttgttggcgtcataggacacatacgtggccgcggcggtggccgctgctgccgcgcccagtgcccaggcggcgccggtcgaaatggtaatcggctcacacatcacacacccctgcggcgatagaagggcaggaacggcaagccgtccacgccataggcaatcggatcgctgaactggaaacccagccagcgcagccagcggatcgctgcgatgttccgctgatccacgaaattgtagagaaggttcgggaactggtcttgcatgtattcgaccacgggttccgacagccgcagcagatccttctgcgcgccatgctggttcagcacgctgctgccgatcatccaggccgaccccatgccgcccatgatggagaacggcgacgccccgaacatgcaggcggggcggccgttgtatatggcggtgaagggttcggcggtgcgttccatgccccgcagcatcgcatccagcgggtcgctgcggctgcacgcccacagttcggccaggtccgccgcccgcgggttctccgcgatggcgtgcgcatgttccacggttgccggcacgatggtggcgcggatcatcccttgcccccggcgccgccggcctggccgttggacgacacggccctggtggtgatcgacaggatttccatgggcagcgggtcatccgacacgatgcgcacgcgcccggcatccacgccccagcctgccgggatgtcgcagtcgaacacgccggttttcagatagggcggctggccgtagggttcgaagcggcgttccttcaccgggtagagcttgtccgtaacgccgccggccttcaccccgcgcgacgccagcagcaggatgctgaccttgtacgccagcttctgctgatcgcgcatcgaatcgccgcccggcgaattcagttccagggtttcgacctcgcaggcgtagggcaggccgatgttgcagacgccgccaggcgtggccaggccgatcttgccgccggtcacggtgtacgggccggccaccgcggcatcctgcagcagcacgacgcgcttgccttccaggtgccacaggttgtcgatggtgtcgcgctgtaacgtccagctggccagcggcacgccgcgcagcgacgccggcaccgtgccgatgctgcgcgccacgacgtgggtggcgtccacgtaggaatcgatcaccagccgcaccttgacgcgcgtggtgctggcgatgccgtcttccaccgtggtcacgtcgcgccacagttcgaagccgtcaccgacatccgtggcgccgacgaacagcgcggcggaagcggtgatggtcagttcgtcctgttcggtccagccggcggtgctgcccagctggatcgtggtggcggtcgcgttccggccgtcgtactgcacaccgcagtccacgaaccacagatccgattcgctgttcgcgcgggtcggcgcctgctgttcgatgcactgcaccacttcgccgtcgatcaaccgttccaccaggaaatagcattccgactccttcttgcccggcagcgcgcaggcgtccaggaacaggccatcggtgtcgtgccagtgccagcccacgacctcctgttccggcatgtacgtgcagccgatgcgcacgccgtcgtcgcgggtgaaccacaccacttgccagggcgccttccagtattcgatccactggacttcgaagccggcgaacaggtgatcggcccacacgctgatgtcgttgccgcggaacccgtccttttcgaactggtagcgcagatcgcggatcttctggccctcttcctggatgaagatggccgactcgccaatcagcttggactgcacatcgccgctgccggcgttgccctggttcttgacgccgatggtgctgggcgtcaccacgtcgtcctgcccgcccgtgaccttgtattcgccgcccgtggtcatcaccagcaggttgtccagcggcaccaggtctttcaccgtgttgacctggcgcgcgttgatgacgaacgtaaccgtgtcgctgtccacaatgggcgaggaccggccgaagttggggtaatcgccgatgcacgacgcccaaatggtttggggatccgctggcgtgccggcgaaccacagccggtcggcgaagaactccacttccgagggatagccgtagcggcccgaccaggagccgaccgcccacacgtcggtgccgccctggccagcatcggccagttcgttaaccaggatgttgttcgtgccaaccggcggcgcttcgtagaaggtgatcgtgtccgcggtgggattgaccgtccagccctgtgccatcactgaatctcctgctggacgttggtgtttccgccggggcgcacgctgccgccaccgccgccattcacgccgccgccgccgccgtagtacgggttcggctggatcggctggccatcgatgttcaccttgtagtccagggtcgaaccgctcaacgcgcccgtgatgttgaacaccttggtgctgccgtcgccgctgaacgtccaggtgttggccggtgccggtgcggtgcccacgatgctgtccggcacacgttcgatcaccaccgcctgcacgtggcgcgcgtcggtgtaggtctgcacctgcaggatgccgaaggtgttgtgcaagaactcccattcgacgccgaccgcgtagctgttcacgccgtcgtccttgatgtcctgcggcccgtcgaaggcccggccgctgtcatggatcgggcgcacgttgccggcgacccagtagggcgtgcccttgccgcccaggctcggcgggatgctgacgcagcgatacaccttgctgtccgaccggcgcaacgcgcccacgggcacgttcttttcggcggacgcccagggcttcaccccgcgcagttccttttcctcgacgtacagcagcgaccccaccatgtcggcggtgaaggtgtccacgttcgtgctgaccgtgacgatgccggtggtgccggacaccgccatgatgagggcttcgtcgctgttgaacgggcggaacgggccgcgcttgaacgcgaagtcgcgcagttcgaactggttgaccgccaggcggcgcagttccttctgcggcacctggccgtggacgatgtagagaacgtccgccgactgggtgaagcgcacgctgcgcagcttcgcttcgtcgtagggcgtggccacttccacgatgcggtcggcgctgccgccgccggcataagcggtcaggatgctggaatcgaagccagccagctggaaggtgttggccgtggccaccgtcacggtgaaggtgcggccgtttaccttggtcatgccgcgcacgccggtaatcaccacctggtcgccggcaacgtagccgtgcccggtggacgtgaccacggcggggttcgcctggctgatcccttcgatgggcttctgcgcgttggtcagcagcgcgccgttgacccaaaagcggaaatacccgtcgcccatttcgatcaagtatttgacgctggtggagtagatgaagggcaccaggcgcgtcagcttgttggagaacttcacccggccgcggaagatcgtgccggggcgcttggcgccgccgccggtcggcttggtgatgaagttgcgggccatgcccaggctgatcgcgtagcgcgccagatcgacgcggccacgcataccgggcgaaagctcgccgccggacagggaaggctgcaggaacttgggcatgtcagtacggcccccggcccggccacacgttgctgtcgcgcgcggccagggccggcgtcacgtagtcggcgtccgtccgcgattcgttcatggcgtgcgcgcccgcgttggtcagcgccagggtgtattcctgcagcagctgggtcttgttgttcaagcccacttcgccgatcaagggcggcgcggcttcggcggcgatgcggcacgccagggcgttgacgaactgcggcggataccggccggtgtcttcgacgcggcaggcgtacaccaggaaggcgttgcgcacgttcgtgttgatcgtggtggcctggtcgccgtagctggtgtcccagtcgaaggcgccggatccccacacgctggcgatgtagtcgccgttcgtgaagcgggacagcttgccggcggcggcgatgccgttggcgtccgtgaccgcgtaggcggtcaggcaatcgttcgggtacgcatagcggtagtaccagcccggttgtgcggcttccacgtccagggccagcgcctgcgagcgcacagcccagggccacacccgttcggtcagcaccaggtcgcgcatcggctcccacaggcggttcatcacgtcggcggccttggattcgtccgtgaccgccgggatggcgatggactgggccagcttgtagagcgccaggttaaaaatgtcggtctgcgtggccacggtcatcacctaaaaagaggggccggcaatacgccgaccccgactgcacgcccgccggggaggcgggaattacttggccttgtcgccggtcttcgcgtcgcccttggccttgtcggcttccgcggctgcggcgttgaccttttccagctgcgactgcgcggcggccagttcctggcgcgaggcttccagctgggcctgcagttcgtccgcgcgctgcttctcggcggtcgcctggtcggccgcggcctgggccttggcatcggacgccgccagcttggcgatggcatccgcttcggcctgggccttcgcctgggcatcggcagcggcctgcgcctgggtcgcctggtcggcggcctgcttgcggctcacgtcctcgctgttggccttcgccttgatcttggcggcggccagcacggcaaggcgctgggcgtcggactcgctggcggcggccttctcggcatcctccggggcgacttcgacgtaccagcggcccggcgtgacgcccggtgccagcgtgacgatggcgccagcgccgaccaggccgtaaccgtccacgtagtgctgcggcgcgccgtgggcgatgacgtactgctgttccccgcctgccggcgtgcgtgccgtccgcgggttcagtgctttggtgttgctcatggtgcagttccttggtcagtggaaccggccccgtagggccggatccagggcggtcagttgcgggcctgggggttgttggccgccatcttgcgccagtagccgggggtctgcgtcaggaaggcgcggatggtgccggcggtgccggtcccggtgatgtcgtagatgaggcccacgtaccgttcgtaatcgcccggcggcaccggcaggaccgccaccaccttgttcgcgcccaggttggccaccggaatggcgcccgtggaagcgtgggtggtcggcgacgtggccaggtcggcggtgctgtccgaagccagcttcacttccagcgcggtggcacccgtgaacgcggtgccggtctgcacgaccaggaacaggtcgccagcgaagccgggggagaagttggccaggaccggcgcggtggaaccgcggtcgatgacattggaaatgccatcggcaagcaccgcctggttgtcggagaagtacagcagctgatcgaggatcatggtttcgattccttgtgaatggccggcgccgtcgattagacgacgacgcgggtttcgttgagggaaatggcgtccatacgacggaccggcacgccatcgaagtccgtgaccttcttgcccgcgatttcgcgggtggacagccacacgttcgccttgttctggatctgcaggcgcatgaaggtgctgaccacgcgcggcacatagaacaccgggttcaggccgttggggttgttcagctgttccagggccatggtcatcaggttgatgagcttggcgcccgcggtgatcccggtgatggggtcgccggcctgcaggtccgaaacgtcgatgttggcgatgcggacgatgttgcggtaatcgctgacggcgataccggcattcaggtcgaaccagtcttcgaagcccaggtacttgccgcccgtgccgtcatcgatcatcgcctgcggcagcgggacgtgcttgatgccggcggtggtgcccttcgggtagaagcccatcaccgagccttcgccccagccgaccaggtagatgctggtcaggtcggcgccggtaccgcccgcgtcgatgatctgcaccgcggtgcggtcggcggcggccaggctggcgtagcgcggcgcgatgcccaggaagtcttccggcaccacgttcggatcgccgtacagcatggactggaagaaacgctggcccatcgattcgatgtggcccttgttttcgatgaagcggaaacgggccttgtccacggccagttcgaccagcttggcatcgacctggcccagggcattgaacaggccagccgattccagcacggagccgtaaccggacttcgacgggcggatgccctgattgatgcggcgcaggaaggtttccggcagcttctggcgggccgacaccttgtggccggtggtgctgttggcctcttcccacgggatgtcgttgaaagccgggttggtctgttccagcagttccgcgatggtgacagcggcgccggaatcagtggtcagggccgccgcatccgcaagggtgggctggccgttggcgagaattgccatggtgcgattcctttttcaggtggtcaggtcagggttgagggcattacatgtcggggtacatgcggttccacggcttcacgtccggcttcgcggccccaccattgccgatgccatcgacaggcgaatcccgcatcatcttgccgaacattgcgaaggccttgataagttccgggtggttgccccagcccaggttatcgaacgcctccaccagcttcgggttctgcagcgcgtgaaccgccgtggtggcgaatttcacttcggcgtcgtactggtcgcccagttcggctttcgcctgcttaccccattcgtcgcgctgctgcgccacagcggcttccatggcctgctgctgcaccgcggcgtcctcgcccaccgtcttgatgaagtggtcgatggcccgctgcgctcccgcctgggacaggcccaggtcacggaacagcgacagcgccacgtccttccgctcgccttccagctggaagccgtccggcagggtgaagtccgtgtacgcttcgggcgcgccagtcagtacaggcggttcgtcgtcggtcttgccctggccgtcgccagtcttcccttcgtcgcccgtcttgccctggtcgccctgcttgccggcgtcgtcgccggtcttctcgccaccctcgccctgacctcccgaaacagccggcgcgctggcctgctgcccgttcgggttcgctgcatcggtggctgcacctgcgccgtcgccaggattgggttgctggccggcggcgttgttggtgtcttcggtactcattgttcggattcctcttcggtgggtttcggcttggactgcgccaggccttcccggcggatctgcgcttccttctccgggcagtggtcgcgcaccaggttcagccaccacttcgccgcgtcctgcatcccgattgcgtgggactgcgccatggcgttggtggcaaacggtgaagcgtccagcccggtctgcagcatgaacagccacaggatacgacgggcggccggcatattcatcacctgctgcacgtcggcccgcagctgttcctggaaccacttttcggcctggcgggcttcgcgctgctgggcttcgatggcatcgcggtcggcggggtgcgtcatgcgaacccccaccagcacaggccaccgacgatccaacaggccgcggcggcgacgccccacacgatcaccccggcgccttccaggtcgagcttacggcggcggtcggcggtcatgctgcctgtcccccgcgcagctgttcggccaggccttcgcccaggctccccggctgcggcaccgcttcgttcagcgtcttgatcgcctgggcgccatcggccatcggcttggccgcagccagcgccgcctgctgcgcttcctgcgcggcgcgaccctggcggatggccagcacggcgtcgtcgtcgcggacgatgctggccggcgcgcccgtgcgctcgctgtattcgtccaccgcctggtcggcgtcgaacttgtccagggcggacgggccgaacacgctggccatctgcgcgacgaacccggcggtgcgttcgatgccgctggtgcccgacgccttcatggcctgggccaggatgctggtgtattcgatcttcaaggggatgctggccagcacagccggcggcggcgggatcaagccggcgcgctcgcacaggcggaacacgcgcaccacggtcgggtccaggccttcgtcggtgacgatttccagggtcggccccagcacggtcgccttctcttccttgcgctcggcgatttccgtggccgtgcggccggcggcctcgcccagggattccagcatcaggaacaggttgtaatagaacgaatcttcgatccggctttcgacctcgcggatttcctgctgcacccactgcagcgaccccggctgcggggtgtaggtggcttcgatcttcgcgctgttctgattctgcggcaggtagttcttcgtccgcggcgccaggctggccccgatgttgcgcatggtgtcgggcacgctgaccggcggttccgccatcaagtcaatcaggcgcagcttctgcccttccaggtactgcagctgtttgatgtcgcccagcgagtcggtgccggggcacgcggaatagctttcgtcgcccaccgggttgaagcggatgcacacgaacggcggttcgtagtggccgccgatgtccagcacgccgtgcttttcgtcgccgctgccgctgatccacaccacttcgcggaacgggcggaacttcggcgcctggacgcccagcggccccatgccagggcgcgcgtcggggttcggctcgtacagggcttccacggtgaaccgctggtccgggctgcgcttgtacgcctggatcacgcgctggggcagcttcgcttcgtcgggcacgcgctcgcccgtctccgggtccatgcggccgtacttctgcaccagctggcgcgcggtcttcgtgtagcagcgccacagcgaatcgaccttgccggcgtcgtccagggcgatggcatagctgccgatggtcagcgggtggaagcgcacgacctcttcggcgttctccacgatcatcatggccgccacgccgtaggacaggtcttcggtgtagcagaccggcatggccttgtagaaattcgacttggccagggtgtcgcgcaggatggtggtcacgttgtccagccacacgcgcacgtcctgcagctggcccatggccgggtccggcgtggtcaggttgaaccagggtcgggccttgctggtcatgtgcgaggacatgccggcggtggccacgcgcacgcacttggtcgcggtgccgttgatgatcttcgaccggctgcgcttcttcgtggtggtgttggtgccctcaccgttgaaccggccgcgggccgggtcgatgtactccgtcacctgcatccagtcgggcatccatgcttcgcggtcggcgatcatcgcgccccggcgccggtcgcagtgctggcgcagctgcagcgtcggctgggccgcggcggcgtcgagcttggcgcgggcggtttcgatgtccatggcttcccctgtcagatgccgaaggggcgcagatcatgcgccccctgctgcaccaggatggaacggatggcccacggcagtgcagcgaccagggggcgggcaaggtattggcgggtggtcttcatcggtcgggatcccagcacggtcttcggggcggcgaactgctgctgcgcggccagctgctgctgatagttcgcggcggcggcgcggcgctccgggccaccgttgcgcacgtcctggcgcacgcgctccgtctcggcgttgcggcgcagctggccggtcgggtcgcccaccgcggtcttcgtcaggccagcaggatcggcccagcgcgcgctgttgccggtcaggagcttggccgggtccatcaccttccccatggtggtcgaattgcacatgcgtcagacccccagggcagtcttcacgggtgcggtgggggccgtgccggtgttgccggccaggatcgtggactggcgcccgccgcggctgcggatccggttgcgctcgcggtcgcgctcggcgacagcggcatcatccacggattcggggccgaccacgggggccgatgctacgggcttcactttcggggcgctgctgcacatggtggtcagtccttcatcacgggatcgtccgcgtacatcgcggcgtatttgctggtcccggccgcggccagggccaggtcggtgatctgcagttccaggcgccggctggtcttgccgccgtccaccgtctcttccccgaccgaatacaccagggcaacgccttccagcgccaccttcgcgccggccaccggcagggacttgatgcccagggcgtccagctgttcttcggccaggttgatccgcagaccccacgggaagtcgggatgctcaccatgcacggtgtcgcagcactccgcgtccttcgtcttctcttccggcttgcgcttcatcgataccagtttcatggcgtcatcccagtgggttgtagggggtgccgggctgaccggacccatacgattcggccacctgcgcagccagcgactggatgcgagggtggccgatgttctcctggctccggtcccctggcgccacgtcgaaagcatacgtcagcgccgcggcgtccgcacgatccggcgagtggcccagttcttccttcacctggtccttctccaccacgcgcatcttgtcgccctggaaatagtaggtgtgggcggtcagttcgcgggacaggtcggggtcattgggcaggcacaggccgtcgtgcttgatggcgtgggccagccggaaatacatttcggtgcgcttgttgaagtagcgcggatcgtcggccttgccggcgaagcccaccccggtcacggtgtagttcagcgcgcgcagctggtcgatccagccggcgccccagccgcccgtgtcgtccacgaacaccgcgtctggcttggcgttggtctgatccttgtagaagtcgcgggcgtcctgggccacccagccggcgccctgcaggctttccatgttccggccgatttccagggggaacatcacattgccgttgcggcgggccttgcagctggcgtcgtcgccgaaccgggccacgtccacgccgatgatgcgggccagggcacgccacgactggtcggtgggctggcgcttcatggccgcggccacgtcgtccggtcccagcagggcgttcatgctggacggcgggaacttgccgaagacgttgaccagcacccacgggttgtcgcggccgtacttctcgatctgctggcgcgcccactcggcggacacgcgcggcgtgcgcttcgggtcatccgggtccgacgtgatttccaccagccaccacagatggcgttcgctggtggtcgcccggtacagcggcccggacaggtgcgtggggttgcccgccatcaccaggtgcgcgtgcaagttgatcccgtccgcgttggccaggccggcttcggccgcggccatcaccgcgtcggggatgccgccggcctcatcgatgatgaacatgatgttgtcggcgtgcaggcccgccagggtgtcggcctgctgttcggtgctgccgcccttggcccacgaccggaaggacatgaaccaggtttcggggttcgcgttctcgtaaatccgggtcttcgtccaggtgaaggtcgcctgcagcagcggcgcgcgcttctgccacttggacatttccgaccacaggccgtccgccaggttgtcggcggtgatcgacacggccgcgatcttcgggtgcatgtagcacagcaggaagttccagcacagccaggccagcacagcggtcttgcccggccccttacacgccttcatggccaggcgcgggttgtgcgggaaggccgccagcacgtcgtcctgccattcgtcgggggtggtgccgaacagttcccggaccatctgccccggatgctcgcgccagcggcggatgcgctggccggccgtctccgggaccggggtggtgctgatgccggtgtcgtcggtcacagcagcggttcccccgaatagtcgcaccagcagcgccgggcgcgcgcccagtgccccatgaaggactgcaccggcacggtctgcgggtcagcgtagaagccgaccgcggcctggtcgaaggcctgggccttcacgcgcagttcgtggtcggccggcaggccatcggcgtcagccctggccaccattcgccgggtcagttccgcgctggcgttcaatggccacccccgccggtaccggacccgcccaggctttccgcgaccagctgttccagggtcacggcggccttcacttcgaccttctggccgtaggtgcgcggcttccgcttctccatgcgccacctcatgttcgaaagcacgacgttcgcggccttcgggtccagcggcttttcaccaggctgcagatccaggcccagcacctggcgttcgatgcgctccatttcgtcgtagtcggcgtccgctgcagcctcgcacgcgcgcacgcacctggcgtcaaagtcggcatcgtcggcacgccagcggcgaatcgtggcggtcgagggaaggccggcagcgtcggggtcggtcgagtcgaaccaccggaaggacttgccttcctgcagcaggcgcacgatccggtcatccagatccgagtgccggacggtcgggcggccagccatcaccacacccccatgccgcgttcggtcatccacagggcgccgatgatccccagcagcgcaatgccaggaccgccaccggacggccccagccatgcacctgccaccagggagccggtgcccagcaccagcccgcccatgacccagcccgtggcgcgcagcagtcgcatcaacgcatcccgagccagaagcaggcggccgatgccaccaggcaggcgatggccaccagctggaacacctggccgaacccttccgccttgtcggcgatgccctggtacgcggtcaggcccggcgtcaccagcagctgctgttcggcgatagccgcggccgtgtagttgtgctgtgcccagtagctggcggcagcggcgacgatggccagcaggacgccggacacgtgccactggctgttcgtgaacaccagcaccaccaggttcgcaaggaaggcgccgacgatcaccaggatggcgaaggcgatggtggcgagaaacgacaggttcatgggatacgctccgataacgatggggtaacgatgcaggtaacgcttcgtgcgttacttcttccgtttgatggccggcgacggggtgcccagcttcggcaccggcttcccctggacccgctggatggcgtccaggttcgattcgtagaactgcaggcacttcttccgctcgcgggccacgctgggcatgacttccagcggcgccgtctcccgccactcgcacttcgcggtcaggtccgggtcgatgggaacgaacacctgcacgggcacttcgacaatcccggccggcgtggtcgggatgtcgggcttgatgacctggcgaccgcacgcggccagcaggatggacgggagccagagcagcgcgcgcatgtcagtagtccttcaaggtcgggcaggctgcagccatcacttccagcgccgccttgcattcgggcgggcgctgcaggaaggcgtcctggtacttctgttccgactcggcggccagcgcctgggcggccttcgccgcggccagggcggtcgcgttgtcccgtgcggcctgttccagcagcagcttctgctggcgggccaggtccgtgaaccgggcgatggtcgcttcccgatccgcgatctgctgggccagcgtgcgcttctcctggtccgtcgtctctttcaggcgggtgtagtcggcccgctgctggacgatgaccgtgccgcgctgccaggactgcaggccggcggccaggaacagcagcgcgaagaaggcgcaggcgccgcgggtcttgttgcccggttgccgcagccacttccgcgccgtctcggccgcatcgcccagggcgcccaggatcgaccggaccaccttgaccacgccgcccaggcccatgaagtacaaggccgccacggcgatgatcgccacgacggatccgccaccaacccaccacagccagttcatcggtcattctcccggcggcgccacggtgccagaagcagcacagccagcccgcacttcaataccacgatgtggaacggcggcacctggtggccggcccactggtcgcccaggatgaccagcatggggatgccgatgcacagatgaaccaccagccacagcagccactggccgatgcagccgaacgtgtgatcggtcggccggcgcgtctcgtacaggcgccagcagaccgcggagaacaccccgaaggtggcgcaaaggttgaccaggtacaggatcacgggtcgcccccgatgacacgatccgcccggcgctccacggctttcagcaggccagggagccacggacggatgccgacgcccaccaggccggtgacgggcagcaccagggattcgtccaccaccaggcgggtcagcgtcttgacgaacgcgatgccggcctggacggaccaggcggcgatgaaggagtaagccagcacgacggcgcccaggaagcccgcggtgaacagcaggtacagcaggcgacggcgcaggctggaaccggggtcagtgctgatgcgcgcggcttctttcgccggaagcagaaacacgccgatcatggtgccggcgatggccacgtacagcatcgaaatggggacgttcaggaaggcggtttcggtcttcgtgacgacttcacccacggcgccaccagcggacaccacggccatcgtcaacgctccgattttccccatgcccatgtcgtccaccgtcaacctgcccgaaggtacaggctacgttccgcggcgcgacggcgcgtgaggcccgccattacctggccgccggccttgttccagaccgggaactggtcagccgcgcaggtgtggcacccttccatggccttgcgccacatggtcgaggggcggccggatttcagcatgaacagtccgtccttgcccggatccttgccggcggccttgcggccctcgccgacgttgaacaggaagctggccagggccgccacctgggcgtcctgcagcacgccgccgtccttcttggcgcgggtgcgcacggcgttcacgcgcagctgcacttcctcttccaggttggcgcgggccacggcatcggaccagggcgcggtgtcgggggtaatgaactttcccgtttgcccgtagccgatagtccagggcgcgccggacagcgccgcagtggcagccggcaggcggttcaagatcgaacgggcggggacgtggccccagggttccttccgcgtggccttggccaacgggctggcggggtcgggatacggatgcgggcggaacccttcgaactcggcgacgatgggcagcgcgagcttcgcggcttggtcggacacaatttccccctggacacggtttcgcggacggtggcgtgatgatgggccgcgcgccgtgggcagtcaatgaaaagccccggctgctggggaggcagaccggggcggggaggcggcagaggatggccgccggaacagcgttgcacgtcaggcgcgggcggtcaatcgctccgctcgggcttgatctttgccacctttcggcaagcatccagccttgactgcagccgcctggcctggtgcagcgcatcaccgtcgccgcgcctggctgcgcgatgaagctgggccaggcgcggcgcgttgtaggcaacgaacagttcgcggtccagttcgcccaggctggccgcccactcgcggttcgcctgcgcgttgcgcttagaccgtgctgacatacggatgcacctggatcaccgcgccaggcctgcgcagcgcgtcagggtgcgcgcccagggtgtcggcgggataggtcttgatcgcccggcactccaccacgcgcgcgtcgtccttccacacgccggccgcggtcagcgcgtcttcggtgctgcgcaccagtttcgacaggtcgggcagctttgacggatacgatgcgcgccgcttgggcagcgacagcggcgccggcagcgtgaacaccaccagcagcagcagcgggccatccatcggcacccagtcgcctggatcctcgcgccgtccgatttcagcttccgccgccaccttcacgtcctggcgccagggcgccacgcgcttcgatgattcggccagcaccgcgtgcccgccgtggatgcccttgaaggacttactgccctgcggcgccgggtcgccgtacaccacgatcttcatgccagttccctggcagcgcgcgcgtcgaacttcaacacgcccaggcggatggcttccagcagcgtggccttcaccatgtccgcttcggtcttgccgtacttctccacgaacgcggccatgccggcgtgcagttcgcggtgttcctcatccgtcagcggcatggtgtcgaagtcgctgaccttgtgctgcgacagccggccaccgatgcggtggtgtgccacgcagccgatcatgccgctggccgcggacggcagcgaacggacgaacgccaagtattccggcgcttccttggggagctttgcatacaggtcgcggatcattttctttcgccttcgggttttgtgagcctggccagttcgaccaaccagtgcgccaatttttcgggggtatgttcgcgctccgctttcgaaacttccgggcgccacttcggatggcctttcttcattcttgatccatcgcgcagcgttctgttttgcgcaataacatgggtggaccctcccagcacaaaatgcatagcggggacatcctgcggttcgatcccgcacacgtacagccaggtcgccttttcggcgcgatggccgaaccagtgctgcaggatcgggatcgtaaatcctccccagctgtcccgcccagcacctggcaacggaaggccttgatgcgcccaaagcgttgacgttgccgggtgttcaagcaccccccccagcgacgaaccgcagctaccgcaaacacagccaggtcgcgttctccttccctgggcttggccaccatgcgaagccttccccaggaccggcacggcggatgcgctacaacaggcgcgccgccgtcccacgatctggcatccctgtcgatgtcataaacatcacacccggatattttcttgtagatgctgtcctgcctggcgaaaagaacggcaacggtcatggttgctccagtagggattcgaagtctgcgacctgctcgggcgacaggtcggggtagtcgtgttcggcgacgtattcggtcatcaccttgaaagcggcggcgaattcgtcttcgtccatttcatcgaaggaaatgctgcgcggctcgctgcgtgttacccgggtcatgcccatcccagggatgtcgatgtcgtaggcgatgcgttcgcaggcggcgccgctgcgcgcctgcacgtccttcaccgcggcgtgagaatccggcttgcccttgtgcgtcaggtggtggccgtagccgtccacgtgcgtgaccaggaacgtgccgaactgatgcaccaggcggtggaacccctcattgcgcgggttcttgatttcgcagcgcacgcgcccatcggggcggaacttccgcccctgcaggatccgccgatccacgttgctgctggccaccagcgcgcgcacttcctcgccggtcgccgggtcgatcatcgtgcgccacttcatgtagacgtagcgccgcgcgatcttgcgcgtggtcgaatgcggatggtcagccattgggatacccgtcatgcagcacgccgtccagggtccggccagcggcgtgctttccgaccatgaccatgcggtgcgcgcctacgtcctgcgggacgacatcgtgcccgcactgactgccgtcacgcatcaccgccatctgccgaacagggccgcaggcccacaggtcgcgcggctcccactcgccccactgcttgaacaggaacggcacgcggtatgcggcgcactggtcgcgcaacatgcgcgcccaatcaggatgcagaggcctggcgccacgcccgctttcgccaccgacaatcacccaatccaggccatacaacagcggcggatcggtgggctggccgccacatccgcattcgtgcccgctgcagcacatcgccggcccgttcgggaacaggctttcggggtaggccagatccacttcgcccagcagcggttccatcgacaggaacttgaccgccgcgcgtgtggccagcagcttcggaatgtcgcggtcggcttcggcctggttgcagatcgtcgcgcccagccacacgttcgccggccacccgccatggatgttcgccgggtccgggccgtgctggaccgggccgccgacccagggggcgggcgccatcttcgccacgttgccgatgcgcttggtcagcagcagccagtccaggttcggcgtggcttctatcaacgcgaacaggtcggcgcgccacgccgggtccacttcgttgtcgaacacgtcggccaggctcgcgcagaacacgcggcggcgccggccgttctccgagaagaactgatcgtgctgcgcgttccaccgcagcggcagctgccagttcgaaggcgcggtgcggcggcgttcctcgcctgcgccccacttcacgccgaaccggcgcgtgggcgtggacacgctggcgtagcagtggtcacacgccgggctgattttggtgcagccgatccacggattgaacgtggcgtcggtccattcgatcttgctttcgattgccatggtgttcccctctctcccgttggttattggccgctggcgcgccgctcggcggccagggcttcgaagtcacgcatttccgaatcgctcatgccctcgcggcgctggaacgccgccctggcttcctcgctggccacgtccccgaagtaggtgcgcaccagcggcggcgccggggtatcagcgtccaggctcacgcccagcagcaaacggctgaccacttcggcaggcggcagtcggtgccgaaacgccaggatgcgcagctgttccgcagcgtccgccgtgatgcgtggcccgcgcacccagccttcggccttcttcttcgcttcataccgctggttatgctcgcgcgctgccatcactgccccctgtacttttcggtcgcctcgcccatgagccggcgcatttccgtgtcggcctcttcgccttcgccataggcgccgatgctgcgctgctggcggatgaacgccagggcgttttccagcttcgattccgacttcgccagcgcggccttcgcgccgaacgattccggcggcggtgccggcgccgtggccaccttgtccttcttcggttcgtcttcccaccgctcgccgttgatgtaggtgctgccgtgcgggatgaagccgcgcagccaatcgtcgtcctcgcgctccatgcggcgcacgtgggcaatgatctgatccgccatggcatcgcagcctttcagcttccactttttcagcgcgtcagccttgcccttcttgaccgggtacgcggcccaaaacttcgggaagtgttcggcggtctgcttcttgccggtgccggtgatgcgcttgggcggcggttgctcgccttcgttatcgggcggtaccggcgcttccggcttcgggatgtccttgggcaattcgtcccgcggcgcgtcgtcgtggccagcctgctggccggtggcctttggctctttagaatcttcttttctcttctcttctttaggtaacgcaccactaacgccgccagcgttaccgccatcgttacctttcgccttgtgcttctgcactcgtttggccgtcagggcgcgctgcttggcggtttccccgttgtgccggtcgaagtgaggcagcgacacgcccgacgcatcgatgatcgcccaccgctccaccgccatcgcggcgatgaacccaggaacgccagcgacacgatcaagcaacgatgaagtaacgcgcgcagcgttaccgtccacggtgtgcgagtcgaaccacgaccacacccgcatcagctttccgatcaccgcatccgggtcgatgcccagggcttccgcgatggcgaacacttccggcttgtccagcgtgtccttttcgaatttcagccagtcccctgccatgtcacaccgccttccaggccgcaacgtgggcgcaatggcagtgcgcggcgcgcgactccacaatgcccacctttgcaatcagcccggcccgtgcagcgcgctggaacaccgaaccccaggcccgcagatgcggcggcgccggcacggccgcggcggcaatgctgctgcgcacgtcctcgctggtgaaggtggcgccgctgctacgcttgcccgccgcgaagatgcgcagggcttcgtaggccgtgtccccccagttcgggttcacgtcttcggcatgatcggcggcctgctggatcccggcatcgcgcgccgcccgcgcggccgtccaatcgaattcaggctggttcatgtggtcgctgccttgcgccgttcgcgctgcacgatctggctgacccgctgcctggtgatgtccaggtcgcgggcgatttcggcgatgctgtcgcccccttccacgcgcgccatgatggccacgatgcgttcccgctgggccttctgcgccgcggtctgcgccctgttccacgtcttcgttttcatgtcggggtcatgccctgttcctggttggtgacggcgccaccttacccccgcaacaggaattgcgcaacaggggttgacaacttccgggaacggcgtatcgttggcggcacaaacgagctacggccaccgagggatcccatgcgcatcaccgaaaagaccagtccgcaaggcgtcgccatcgaatacgtggagcctgaccaggccaccagcgaacgcgacatccagcacttccgcaccatgatcgaactgggccgggagaagcaaaaccgccgcgacgcgaagcgcccgcagcaggccgccgtccaggaaggtgccgaatgaaccactgccccgtcaccgcagacctgaaccgccacctggacgaactggaccgggccgactcgcgcagcgaatgcgtggacgccaagctggacgaactcatggaggacgcggccgaggttggcagcgccctggacatcatcatgggcgacagcgacgtgggcagcggcggcaacaccctgttcgctggcgacctggccgcggtgctgctggcgtccgatgtcgccttcggttccgaggccgtccagttcttccacaagctgcgcgagcgcgtccgcgaccagctgcgcagcgacgccgaaaccctggtggatgaagccctggccgaatccgaagacgccgcggcggaagcgcgctacgaagcccagcaggccgaccgcgaacaggggtggtactgatgcgcgcccgcggcatgttcctgggcgcgctgttcgccttctccggccccgccctggtggcggccttcttcatggacaccctggtgccgcttgtcatctggctggcggccaccgcggtggtgatcgcgtgcggacgggaggcatgatcgtggccagcgaagcgaagtggcccagctacctgggcaagccggcggatccgctggaaaacgtggtgcgcacgcgcgcccagtccatcctgacggaagtgggcgcggtcggcccgcctctcccctatgaccaggcgcgcgatgtcgtgcgctggcacgaatcgcacctgcggagactgcagggcgtcagcctgggccaccggctccggcagttgttccacctttccaccaacgacaaaggaacgcagcaatgaacccgaaccacaccagcatcgaaaccctgatggccgaactggatggcggcaccctggggccgcgcctggccgccgcgctcgccgaatccgccctgggcgtcgccgcctgcaacaccaagaccaagaagggcaaggtgacgctggaattcaccatcaccccggtgggcggcgatcagacccaggtgcagatcgaccacaccgtgaagttctcttcgccgacccagcgcggcaagaagcaggaggacatttccaccagcagcgtgatgtacgtcagcaaccgcggcgccatcaccgtgctgccgaacacgaacaaggatctgttcaagcccgaagaaggcgtgaccggcgccaacgtcgccgcgatccgctgatccccaccactcccgtttcatccaccgcaacaccaacaacaggaaaccgaaccacatggacaagagcgcaatcgaagcgatccaggattccagcgccgccgcggccaaggccacccaggaacagatcccggccagcatcgcgcacctggtcgccgtccccaacggcgtcaccctgcagaacgtggaagcccagctggccggccgcacccgcttccgcggcaagctgaccaccagcagcatcccggacttcgttacctacgtgaaggcacgcgaaggtggccacggcttcatcgacaccgacaagctgggcgccaccgtgttcttcaacctgggcgacgccgctgcgccgggccacgccgaccacaccgcccgcctgaccctgcaggcgacccccgcctacctggccatgctcgccgctggcggcaaggcgttcagccagcgcgatgccctggacttcatcgaagactggtcccacctgatcggtgcgcaccaggtcagcgacgacggggcgttcaccccgatcccgctggcccgcgccatcgcggccatccgcaaagtgaagatcaaggcggaatcgaccaccgagcagaccgaaggcaacttccagcagtcgcgcagcgtcctggaatcggtggccgcgtcgagcgatgaaggcctgccggacgtgctttcgttcaagaccgaaccgtacctgggcctgccggaacgcaccttccacctgcgcgtgtcggtgtccaccaccggccgggaaccctcgctgcgcttccgcgtgatcgccctggaacaggaacaggacgaaatcgccaagcagttcaaggcgctgctgctgggcgaggttggcgattccgccagcatgaccatcggcaccttcgccccgtaacgggcgccacaccgcgcgacgcgcaccacagccggcgggccacccccgccggcactaccacaccaaggatcgaacgatgagccacgaaatcgacccggcggccgagcagaaccaggacgccaccgacatcgcaaccgccagcgccctggcgctgcgcactgccgccatgcaggaactggacaccgtggaagcgggcctgtccgaccttgccacgaaatacaagggcgtcgtgttcgacgtgaccaccacgaagggcatggacgaagccaaggccgcgcgcgccgccatccgcgaaccgcgctacaaggccgagaacatccgcaaggaaaagaccagccagctgtccaagctgggcaaggaaatcaacgaacgcgccggcacgatcaaggacgccatcctggccatcgaagaccccatcgataagcagatcaaggccgaagaggaccggaaggaagccgagcgcgaagccaagcgccaggccgaggccgaccgcatcgccggcatgaacgcgcgcctggacaacatccgcaacatgccgctgcaggcggtgggcgccagcgccgacgaactgcagcaggccatcgaccgcgtggccaccgacgaactggaaggcttcgatgaagtctacctgccgaccgcccagcagacccgcgacaccgccctggacgccctgcgcaagatgctggccgagcgccaggcgctggacgaacaggccgcccagctggaacgccagcgccaggaacaggccgcgcgtgacgccgaagccgccgagcagcgccgcatcgcagacgaagccgcccaggccgagcgcgaccgcctggccgccgaggcgcaggccaaggccgacgccgaagccaaggcgcgccgcgagcagcaggagaaggaggacgccgaccgtgccgcccgccaggccgaggaagaccgccagcgcgccgcgcaggccgaagccgaccgggtggagcgcgagcgcgtccaggccgagcaggcggcgcgtcaggccgaactggaccgccaggcggcagagcagcgccagcgggacgaagccgccgcccaggcgcagcgggaagcccaggagaaggccgaccaggaacgccgcgaccgtgaggccgccgaacaggccgccgccgcgcaggcgcgcgcacaggccgaagccgaggcatcccgccgggctgcgctgctgtacgtggtggccatgccggacggaagccgctgggcggtgccgctgatggtcattgcgaccgaccgcgcgaagcactacgcccaggagttcgacggcgacctggaacgctccctggccgaagacaccctgccgctgttcgacgccgacccgtaccaggcccacgactgggcggccaataacatgaactggtccgacgtgaagggcgaagcccggatctacgagccggccaagccgctgggcgatgacgacttcgccgaaggctgggtgaacggcgaataccaggtggtcaacacccaggggccgcgggcatgagcatccagggctggtactacctgcacacgaacggcgaactgatcttcaagccgaaccccgacgcggcgtgcgacatccgggattccgacttcgcccgccacctttggccgatggaccccagcgaccgcgaaggcgcgtggaacatcctggtggaagcgcacgccctgggcgcgcaccaggcgcgcatcgatgacctggccgcgaagtggggatgcgacgacgccgatgccgacaactacgcccagcgcgtcggcgtcaccatccagcgcgacggcgatgcctggtgcgccaccggccccggcttccaggacatccaggcatccccggtcggcttcggcgaaaccaagctggaagcgatggccaacctggcgcgcgcactcggcatgtccgccgggaaaatgtgggcgccgaccttccgcgatcttctgaaaaaggcagcatgaccatgaccaccgaaaccaacaccatcgaaggcgaagtgctggacgccatgccagccgcacagccggcgccgtccaccgcgctgacccacgccaccaaccccttccagcagatggccgtgattgccatggagaagggcgccatggatcaattcgaaaagctgctggatctgcaactgaaatgggacgccgagcaggcgcgcaaggcgttcgtggcggccatggcatcgttcaaggccgaacccatcgacatccgcaaaacgaaggccgtgggctacagcaccagcgacggcgggttcgtcggctacaagcacgccaccctggccgacgtggtggacggcgtggtggccgccctgggcaagcacggcctgtcccaccgctgggacgtgaagcaggaagccgggcagatcaccgtggcctgcatcgtggcccaccgcgacggccacagcgagtcggtcgaaatgttcgcggcgccggacaacagcggcaagaagaacgcgattcagcaggtggccagcaccgtcgcgtacctgcagcgttacaccctgatgtcggcgaccggcgtggccgcgaaggacatggacgacgacggaatcacgggaggcgcgccccaggtcgagttcatcaccgacgaacaggtggccatcctgcgcgacctgatcgacgcctacgtggtgaacgaaggcaagttcatggactggctgcgcggcgcgtgccgtaaccagcagatccaggcgctggaagaagtgccggccgattgctacaaccgcattcacgaccagctgggccggatccgcaagcagaaggtggccgagggcaaggcgcccgcagccgaaggatccaccaatgggtgacattgccgacatgatgctggacgggacgctgtgcgaagactgcggcgtctccctggacggcgaggcgccgggttatccgcggtactgcagcaagcggtgccgcaaggaccgcgaaccggctgtgccgaaagccacgaagatcccctgcccggcgtgcggtaagcgcgtcaaggcggcgggcctgcacgaccacatgcgcgacgcgcacaccaccaaggaaccgaccgatgcttgacgaactgcagattttcgaagacctggaacagggcacgcccgaatggcacgcggcgcgctgcggcgtcgtcaccgcttcggtctttcacaccgtgctggccaagggccgcggcggcgcgccgagcgagacgcgcaagaagctgctgtaccagctggcggccgagacgatcaccggggagtacgtgccgacctgggacggcaacaagcacaccgagcgcgggcacgtgatggaaccgcaggtgcgcgacctctacatggccaccagcgcgctggactgccgccaggtcgggttcatgcgtcgcggccggatcggctgcagcccggacaccctggtgggcgacgaaggcctgctggaaatcaagaccaagctgccgcacctgcagatcgaagccgtgctggcgggcaagctgcccagcgaccacgtggcccaggtgcagggccagctgctggtgtccggccggcagtggtgcgacttccgcagctactggccgggcctgccggaactgcgcgtgcgcgtgtaccgggatctgccctacctctccaccctgaaccaggaattgcagctgttcattcgtgaactggatgccctggtcgcacagatcaaggcaatggcatgaacatcgaaaacgacgtgcgcctgatcggcaacctgggcaacgacccggaagtgaagtacacgcagggcggaatggccatcacccgcgtttccctggccaccacgtcgaagcggaaggaccgcgacggcaaccaggtcgaggaaacccagtggcaccgcgtggtgttcttcgggaagctggccgagatagccggcgaatacctgcgcaagggttcgaagatcgccgtggccgggatgatccgttacggcaaatacgacaaggacggcgtgacccactacaccaccgacatcgcgtgcgaccagatgaagatgctggacgcccgccctgccgatggcgagcgcacccagcgccaggcaccgcagcgccagcccgcccagcagcagcgccaggcgccgcccatggacgacttcgccgacgacgacattcctttttgaggatccccagccatgaacgcagcacgtatgcagtcgatcatccatggcctaaccggcatcgcccggaaggtgtacgacacggtgccgatccaagaaggttggacgctggcgcaggtgtcggccgaactggggcgccacggcctggtgtacgaacacgcgaaggtgcatgggtgccttcgttcgttgaaggaataggggctgatccgcgaatgcgacggacagttccagcgcattgagcagcgcccgcgcctggtcgccgctcgcacccccaccgccacccaccaggaagacgacatgcccgcaccgaccagcagcgacccgatggccaacctggcagagattgccgccaccctgcgcgagcaggcgcgccagctgatggccaaggccgacgccctggacgcttcggccatcgaagtggcggaagccatcgaacgcagcggcgaggacggcgcgaagctgcgccagctgcaggcgctgctgaaagacatttcgaagtaacccgacccaccaccggccaaaggaggccagcaccatggaaagtaacgaaaccagtaacgcattcggtaacgctccgcgcgttaccaccgaacaggtggaggccgccatcatcggcgaaacctacaccgtcctgccgaacggccgcaccacggtctgtcagctgacgctggacaacgggttcaccgtcgaaggcctgtccgcgtgcgtgagcatcgaaaacttcaacgccgaactgggcaacaagtattcgcgccagcgcgccgttgaccaggtgtggcagctgctgggcttccgcctgcaggacacgctgccgcgcactgccggcggcctgccggaaggtggcgtgcgcgctgctgatgcaccgcccgtcgaacagttcgcgcgcagcgccgactgaccaccacggcgccgccagcacggggcgccactacctgcaggggataccgatgacacgcgatcaatggctggaaaaatgcgcggaacgcctgcgcgagaaggccggcatggaaccgggcgaggccgcggcctacgccatcatgctgcacgacaaccaggtgaacgataacgggcgcgagccgggcagctgggacgatcccaccgacaccgccgacgaagaaatcagctacatgtccgacgatgaggatggcgacgatgagccgtgaaaccagcatggaagcagccctggaacggttgctggaagtgatcgacacgccgccggcccgcaactgcgcgtgccacatttcgccgccatgcagtgactgtgtggactggggcggcctgcgcgaagccatcgccgacgcggaaactgccatggccatgcccgcggatccgatcacccccgaccaggtgaagcgcgccgcggcggccatagccaattcgcgcggcgggcgccggggcgtgccggccatcaccaacgtcctggacatcctgccgccgcacctgcttgcggaagtgaccgaggacgcgaaggccgcgctggaagccgcaggcggtgcgtcgtgaagcgccgccgccgcaccatcacccaggccgaggcccaggccttgaagcgtcgcgtggcgcagctggaaaacgacgaagagcgccgccgcgcagcatgggtatccggctacccggacggggtgaacatcgccacccacgacttccccagcagcgacagcgtggtgccgaccgcgctgcgcacggccaggaagctggggcacgccatcgtggcggtggacgatgggcacaggctgcggttctacgcgctgccgctgccgaaggcgtaacaggaaagggccggggatcacccggcccttctttcatggcggcgtcggccgcagccggaactgcaggcggttgccgcggttcatcccgatggccaccagcgtggcattgacgccactggccagcaggtgttcgatctggaaccgctcgcgctgcatcctgaaatacaggttgttcgcgcgaacgtaggccaggatcacgtccgaattcgaagagtagatggcgcgcttttcgtcggtggtcagccgcggcgtgatggcgccagtgaaagacgaaaagaccatggccgacacctgcgtgtcgtaccagtacagccacgccaccccgttctgcacgaacgccacgaagggccgcatgttctgatcgaacgccagcgccacttcgctgatgtccggccgcgagaagtacaggaacgccggcacggacggcgccgacagccacacgtccgtgcccagcacttccaccttccacagctgcacctgcagcccctgggctgcatcgttgatcgccaccccgcccatttcgtaatcaaccagcgggatggtccgccggctgacctgttccacgaaggcagaaggctgcggcaacgtcgaaagggaattgttggtgaacattacggcgtgtacctgccccagctaacggtgacggtgatggtcaattcctgggcgttcgtcttcgacaacgtggccggggaaatgctcatctgcgtagtgcatccaccgaacgcgaaaaatgccatgttggcgttcgtgatttccgtgcccaccggccacttcgcggtcgcggtgcgctggtacgtgccggcgacgtagttacccgaagagttccacagcccgtttatggtctgcgtggcgccggtaggttcaccagtgatcgcgccgaaggacgcgccggcataaagcctggtcggcagatactgcggattctgctgcatcacattgaacgggttttgcagcccccagccgccggtgaaaatgccgtaatccgaagtgacattcgcagcccgcatttcggtggtgtaggtggtggcgccgatggagaacgaaccggcgataccatccaggaacggatagttccgaagctcgtaggtcacgtccaagatttcatcggccagcacggtgatcgtggtggggttgccactgccgtcgcggataagagcgcgcgagaagagaaccgcgccggacgaaccccagcccacgccgacttcggaaaggttgccagcagcgacgccagcaccgaagcggtaagttttgcgaacccagccgtaatacggcgcgctgggctgcactccgctgggattggacaacgcggtggacgtggacgcaacctgcgacaccagctgcgtgtcgccattgctgggagccgtggaacccgacccaacaaggcaaaactggatgttgttgtaatggtagtccgttccgagccggtccagaccctggttcgtgatgaggttttcgaaccagtcggcaacaacgcgccggccgatttcctggccatccttgtcaatgcgcaccgcttcgatcttgtagaagccggcgacgccgtggtggagttcgatgttcatgcaagggttcccgaagtaggtgccatggtggtgcggatattctccgctgcgatggtgtgggtgatgagtacagttttcagggtgccgctggtggcggccatgatgggctgcacggactcggtaccgtaatcataggtccgctggatgtcccggagagtgccggaattggggtccatgctggcggttacgaagtcttccggcggcagggtgatcgccgactgcgtgttccgaatctcgccagccagcggcgccatagccgccgataccccgtcatcgaacacggggggcaatccgagcctggccaggtacacgccaggcatctgcgccatgatgctttcgaattcgaagtacgggtacggctgcgtggtcaggtaaatggcctgttcgcccacgcacccttcccacggcgcttcacggccagccgagtcgcgcacgcgcagcaccatgcaatagtcgtcgtcgctgttctggccggtcgggtaggagtggttccataccgccttgtctgcccacagacgccggttctgccgcttccggttggcgctgaccgccagggccacgtagaaggcgccagcgggcgcggaggcggtcacggtggaggcgtgccaggcgccgttactgcccgaccgcaccaggttgccgccgttccaggaatgcccctcgccgccgggcagcatgacgccataggcgtcgtaccaaatcagcaggatccgcgcgaccacgttgcccttgctggacgcgccctgctggatctgcacgctggcggtgatgctggtgccgacgatcaccggcaccttcgtcccttccaggctggcgatgccgcggccggtgtaggccgccgagtgggtgccgtcgtaggtgtcgaagccggatccgctgccgatgagccagcccgcgcccttcgaccactgcacgtcgccgtcttcgaaactgccattgggcaccacggtggtgtccgggtcgggaacctggtagccgggccaggccaccacgacttcgctggtgctgttgtccacgcgcacggtggtgcccggcggcatcgtgccggacagccattccacggtgcagtcgccgatgttgttgacgatctgcagcctgccttcgtaggcatcgccggccacgtacccttccagctggccatcgacgcgcaacgccggaagccccacgaatcgaagggccagcgggcgggtgaaaaggatgtggtggctggtcatggtcaggcctgcgccaggtcgccgctgatgatccaggtatcgccctctgcgtactcacacacgccggagataaccgaaccttccgtgcgcgtgtaaggcaggaacccggccgggatcaccagcgtgacatcggtatccgcaacgatgcgcgcctggccatcgccgcgctgcacgatgctgaaatagctgccgtccgccatgtcgtacagatcgccctgattcgcgcgcaaggtcagcaggcacgggttgacgttggtggtgcgcagcagcgcgaattcgctggacttgtccacggtgtaggtgatgccgtccacgtcgatgatcggaatgcgcagcgtctggaccggcgtggtgccggtgaacggcttggcgtagccgcgcaggatcacgaacccttcggcgccattcggcagcggcgccgggaagcgcaccgcgaagtcggatccgtccgatgccggcaccacggtgtattcgtcgtaaggctccttcgacaggccttccaccactacatcgtagaacagcaaatccgacacgtcggagccgggcagttcgaagtcggtatcctcgccgtcgcccgtgatttcccagtatttcgggctgacgccgaccacgccgccgccgttctggatctgttcgatgaccaggtaaagcgtgcgcaggttcaccgcgtcctggtccgcgcgcgggtcgcccacgcgcacgatgcggctacccttcgcatcccacacgaattcgccgtcttcgaacaccagctggatcgtgccatcgaccagctgctggatctgcatttccagcgcgtcgaagcccttttcgatggtttcggcgtggaaggcgccctggttggtgatgtcggtttcctgggtgtacggcatcgtgcgcagcagcagcagcatttcgtcggcggccggcggcgtgtgcatcgtgacgcgggtgcccgactcgtaccccagcttttccacgtcgaaactggcgctgggcaccagggtcatcgtgttgcccttcaccaggaaggcgtacacgtgcgcgcgcgcataggccatcggcccgttgaacacctgggtgacgccgttgccctggtattcgcggcggcggctgttggcggaaacggtcattatttgggttccttcttggggccggtcaggtattcgtatggcgacacgtcgcggccgtccgcgcgcgccgcgatggcgtcgatggtcttattgacctgggtggacggcaagcccagcgtgacgcccgccgcggacactgccgccttcgccacgcccttgtccaggttcacttcgccgtcctcgccgggggtcagcttttccagcagttcggcgtaggcgcgccaggcgccggccaccacgccgctggaatcgtagccgcggaactggtcaaccagcacgccgccgccggggatcacgccgaagaacgtggacagcgcatccttgatcgcccattcgcccaggtcatcccacaggccgtcgtcgtcgtcatcgttcggcagcttcgcggtcagggccgcggtcagcaggccttccacggagaacagcatcaccatgtcggcggcccacttcatcgcctggcgcgggtttcgcagattcgccttgcgggtctgttcgtaggccagattcccctttgcgatcatgtagccttgcagggcggtggtggccttgatccattccgtttggcgcacgttgtcgcccagcgtgccgcgctgcagcggcgacttgtcgatgaactcgcccgaaccctgggcgcgcgtcaccacgtcgtcggcataggcgcgggcgcggcccacgtcgttgccgaacttggccatgcccgcctgttcggcggccagccaggtcacggtatccaccagcccctgcacgcggccgatcatccagtaaccgaaccggatgctggcggccttccccgcggcgaacctgccggcttccgcatccatcacggtctgcaccgcttcgatgtgcgtgcgcaggcggctgtccatgtacggcgacgcctcgcgcacgtagcgcgtcatcgcgcgcggcttgcccaggtactggccgatgccagccatggtgtggccctggccgatggtgacgatggtgggcacaacgcccgacagctgcagcagcgcgctggtgactttgaaggtcagcaccgacgcggtgaagttctggcgggcggcgcgcatggcgcgttcgtgccacacgcgcggcccaatctcgccggccgccgcgtccttcaaccacacttccagcgcctggcggtactcctgggtgccggtgctgtccacggcttccttgaactcctggccgttcagcacgttgtggacgtagttgaccgcatcgcccaggtggacatcgcgcagcacgtcgcgcaggtgctgctgcaccacgcccgtgtccaggcgcacggtgcgcccgcccgacccgacacgttcgatggtgtggccgttgcgggtcgcagccttcgcggtgcggccggtgcggatgctgttatagaagtcgtccgcttcgtccttcatggtcttgacggaatcggattcgtacttcaacgggtaatagccgccagggatctgcagcgttttcccgtcgctggtctgcacggtgaaggcgctggcctgcacgcgctccggcaccaggccggtgcgacgcttctgcgcgtcggcaatggccggccactgcgaatcgatcaagcgccacacgtcttccacgaacgcccagtcgcgcgaatccagcttcgacagcagggcgttcacctgttccggcgacatgcgcccgcgcgcctgggtcaggatcgcttcgcggttgccggcattgccccagttcagcgccaggccaagcaggcgggacttgctccacaggtcgccgttcacttcgggcatcggcacgcgctcggagaagccgcggatttccgccttgctgtagtgcttcacgtagacctgggccagttcgtcctgcgcctgctgcagcgccgggttcagccggttgttcaccgcgtcgcgcatcacgcccacggtgttcatccagatggcgccctgatccttgaacccatccagttcgcgggccatgtcggtggccgtggcctggatcacgcggccctgcatgaaggcctggcgcagccggtccttcggcccgcggtcgcccgtggtgatcgggcgcgcttcgtgcgcagcggccaggctggcggccatggcggcatccacttccgcggcatcgcgcacttcgccggccagcagcagcttgcccttcaatcgcgccaggtgatcgatggaacggatggcatcgcgcagcgtggccaggtccgccacggtcatttcgcggtacggaatggtgaacgcttcgtccatgatcttgggcggcaggttcacgtcgatccccttctgcgcctgcacttcgatccaggtggccagcgaggaacggcggtcggccgccttgtcgctgatcttgcggaagtcgaagcggtccagcaggccatccacctggtcgaggtagtcggcgccagccttgcccaggcgtgcgcgggtcttcgtctcgccgaacttggccaggtacttcgcggtgcgtgcggcctcatcgcgcgcgcgcacggcttcgcggaacagttcgaagttcagcagctgccggcggcgcgcggccagggcgttgccccagtcctgcttcgccgcggcttcgaaggcctcacgcccggcccttgcttcggccgaacggtaggtggccggctgcaggtggcgcagcttcttgtcctggatgatctggcgagccacgcccttgatgaccgcggcctgcgatacctggcggccgttgacgtgctgttccagcgcgcgaatctcgcgcaccatcacgtcggcctggcggtcccggtgcgccgcgatcatggcgcggtcgggcagcgtgccatccgtcatcggatccgggtggcggtccttcatgcgcgcttccgtctcgctggccacagcgtcggccaggcgcggcgcgttcaccagcgattcgatcaattcgcggccggacccgaacccgtagatggccgcggcttcgtcgccgcgcacgccgccttccaccgaatacatgccgaccaggttgcgcaggaaggactggccgaacttgtccagcagttcgtccttcgacagcttgacccgcagttcgtccggggccaggtcgccgttcggcagcttcccgttgcgcagcaggcgctgggcgcgatacaccggcagattgcggacctcttccagcacctgggcgcgcacttcgcgcttctcgcggttgtaccaggcctgttgctcgcggcgctcggccagcagcacttcggccgccacggtggcttcggcgtcggcgcgcgcggtgttcaccgcttcgttgtaggcctgcagctgttcgaaggtcatgcccacagccatgccatcggcaatcagcgcgccctggtactggccggcgcgggcgtcttcaatctcggcatcgctggccacgatgcggtccatgacgttgcgcacgtcatcggtcagttccacgttgaggctgcgcacgctgcggtacagcgcggtcagccacaccttgaacgcggcgaacgtgcggcgcagcgcagacgacggcgccttgccctcgcgcaggtaggcttcgaagccgcgggcgaactgttcgtgctggtcaacggtgaacgcggcgccggcctcgcggcccagccaggtgttcagggtggccatgtcgttggtgatctgcgcgggcgcgccatcacgcgcggccaggtcattcagcacttccaggtacacgtgccccatttcgtgcatgaaggtgctggcgtccatgcctttcagcagttcgatgttgaacacccgcgcgccgggcacaccttcgaacgtgacggcgccgcgcggcttctcgccgccctggttcagcgccgcggcgtcggtgatcggaacgcccagccggttggcctcgctcatctgcgcgaagttggccgcgcgcgggttggcctgggcgaagtccaccaggtcgctggtcgattcgatcaaggcatccagcgcggtgcgttcctgcccggtcacgcccagcatcgtcgcaatggcgtccttgaaccactgccaggccgtgcgcgattcctcgcggccagccggcgccggcacggtggcaagccattcctggaaccgcttgtcggtcatgccgtaggtcagcagttccttgatgttcgacagtgggccgcgcggatcctgcagcgtggcgcgcagcgccgccggcacatcggcgccatcggtttccatgcctgcgaagtgggcctgggcagcgcccagcaagtcgttgaactcggccacggcgcgcgccacggtcgtgttcgaccggcgcagggtcgggctggtcatcatcgccgacgtgacgccatgcaggacttcgtgcagcaccacggacgggaccgcctggtggatccagatttcgttcgtggtgttgttgtagatgccggcggcgttggcgttggccggtgccgccaccatcgtcacgttcaggtcgggcgtgatttcagccaggcgcagcgcaagcgcggcctggtcggcatcgatcccttcctgggtggcgatgccctgcagcatcttggccaggtcgccatcggccaccgcctgatccaccagcgcgcgcgtcgcggcgctttccggccggccgctcggcccggccaccaggtcgcgcacggcgtagtccacaccatcggattcgaccggctggccctgttccagggtccggttcgcgtaccccagcgcctggcgtgccgtcgcgttgtcggtctgctgcaggtcgatgccgcgctggtcaagctcatcctgcaggcccagggcgctgtcacggaacgcggcgcgctcggcgttcatcgctgccggccggtacaccgggttcccgccaagatcctgggcgagcatgtccagcagcgtgttgatgtccggcgcgtcggcgtcgtaggcgccttcctgctggttcgtcggtgcctgggtgatgaagccttcctggtaggcccacaccagcgcatcgtccaggctcatacctgccaggttgttgaccaggccggggtgcgccttcgccgcgtccatgttggccagttcgccgccggagtcgcgcaggccgccggccgcg

SEQ ID NO: 30 - DNA, 20 bp, synthetic construct
  source 1..20: mol_type = other DNA
gcgcagtcatgagatcgaga

SEQ ID NO: 31 - DNA, 20 bp, synthetic construct
  source 1..20: mol_type = other DNA
gttgagtgcaccgagagtga

SEQ ID NO: 32 - DNA, 20 bp, synthetic construct
  source 1..20: mol_type = other DNA
tgggtcacttcggtgttacg

SEQ ID NO: 33 - DNA, 20 bp, synthetic construct
  source 1..20: mol_type = other DNA
gtggtgaaaggtgcggtttc

SEQ ID NO: 34 - DNA, 20 bp, synthetic construct
  source 1..20: mol_type = other DNA
cgtagtcgcgattgtcggta

SEQ ID NO: 35 - DNA, 20 bp, synthetic construct
  source 1..20: mol_type = other DNA
accactgctgacgttcgatt

SEQ ID NO: 36 - DNA, 20 bp, synthetic construct
  source 1..20: mol_type = other DNA
gctaccggtacgactacgtg

SEQ ID NO: 37 - DNA, 20 bp, synthetic construct
  source 1..20: mol_type = other DNA
gatctggaaacagccgtcca

SEQ ID NO: 38 - DNA, 19 bp, synthetic construct
  source 1..19: mol_type = other DNA
tttcggtggcttggatttt

SEQ ID NO: 39 - DNA, 20 bp, synthetic construct
  source 1..20: mol_type = other DNA
atttgcgagaagtacaactg

SEQ ID NO: 40 - DNA, 20 bp, synthetic construct
  source 1..20: mol_type = other DNA
atcccctttgcatcttcaat

SEQ ID NO: 41 - DNA, 20 bp, synthetic construct
  source 1..20: mol_type = other DNA
ttccgtcatctaagggaatc

SEQ ID NO: 42 - DNA, 20 bp, synthetic construct
  source 1..20: mol_type = other DNA
taagcccttcgtaaagttct

SEQ ID NO: 43 - DNA, 20 bp, synthetic construct
  source 1..20: mol_type = other DNA
aagcattgaaaaacgaaacg

SEQ ID NO: 44 - DNA, 21 bp, synthetic construct
  source 1..21: mol_type = other DNA
actaggagaagattagatggc

SEQ ID NO: 45 - DNA, 16 bp, synthetic construct
  source 1..16: mol_type = other DNA
ctggtccgtaagggtg

SEQ ID NO: 46 - DNA, 20 bp, synthetic construct
  source 1..20: mol_type = other DNA
gatatacgagcaacgtcttc

SEQ ID NO: 47 - DNA, 20 bp, synthetic construct
  source 1..20: mol_type = other DNA
atttgcgagaagtacaactg

SEQ ID NO: 48 - DNA, 20 bp, synthetic construct
  source 1..20: mol_type = other DNA
gttattgcgacggttaaaga

SEQ ID NO: 49 - DNA, 20 bp, synthetic construct
  source 1..20: mol_type = other DNA
tggattaaatactacgccga

SEQ ID NO: 50 - DNA, 20 bp, synthetic construct
  source 1..20: mol_type = other DNA
ctggcaaaacaacctcatta

SEQ ID NO: 51 - DNA, 20 bp, synthetic construct
  source 1..20: mol_type = other DNA
agttaccacgaggatttcat

SEQ ID NO: 52 - DNA, 19 bp, synthetic construct
  source 1..19: mol_type = other DNA
gtagatgttcggttcggta

SEQ ID NO: 53 - DNA, 20 bp, synthetic construct
  source 1..20: mol_type = other DNA
caagccaattcacatcgtag

SEQ ID NO: 54 - DNA, 20 bp, synthetic construct
  source 1..20: mol_type = other DNA
attctgtttcaacaaccctg

SEQ ID NO: 55 - DNA, 20 bp, synthetic construct
  source 1..20: mol_type = other DNA
cagacatccaggaacttttc

SEQ ID NO: 56 - DNA, 20 bp, synthetic construct
  source 1..20: mol_type = other DNA
catacctacgatatacggca

SEQ ID NO: 57 - DNA, 20 bp, synthetic construct
  source 1..20: mol_type = other DNA
gactactcgctctacatcaa

SEQ ID NO: 58 - DNA, 20 bp, synthetic construct
  source 1..20: mol_type = other DNA
atggcctttcttcattcttg

SEQ ID NO: 59 - DNA, 20 bp, synthetic construct
  source 1..20: mol_type = other DNA
agaaaatatccgggtgtgat

SEQ ID NO: 60 - DNA, 20 bp, synthetic construct
  source 1..20: mol_type = other DNA
tagattgtgattcacgcaac

SEQ ID NO: 61 - DNA, 20 bp, synthetic construct
  source 1..20: mol_type = other DNA
gaagacgaaaaggcaaaaac

SEQ ID NO: 62 - DNA, 20 bp, synthetic construct
  source 1..20: mol_type = other DNA
atattgaactccgaagtcgt

SEQ ID NO: 63 - DNA, 19 bp, synthetic construct
  source 1..19: mol_type = other DNA
ctaccaaactgggggatag